European Patent Application EP 4 458 963 A1 - sequence listing, part 2

SEQ ID NO: 2824 - protein, 726 aa, synthetic construct
SEVEFSHEYWMRHALTLAKRARDEREVPVGAVLVLNNRAIGEGWNRAIGLHDPTAHAEIMALRQGGLVMQNYRLTDATLYVTLEPCVMCAGAMIHSRIGRVVFGVRNSKRGAAGSLMNVLNYPGMNHCVEITEGILVDECAALLCDFYRMPRQVLNAQKKAQSSISSGGSSGGSSGSETPGASGSVIPKSSGGSSAGSTKDTITKTLKLRIVRPYNSAEVEKVVADEKNNREKIALEKNKDKVKEACSKHLKVASYCTTQVERNACPFCKARKLDDKFYQKLRGQFPDAVFWQEIGEIFRQLQKQAAEIYNQSLIELYYEIFIKGKGFANASSVEHYLSDVCYTRAAELFKNAAIASGLRGKVKSNFRLKELKNMKSGLPTTKSDNFPIPLVKQKGGQYTGFEISSHNDDFIIKVPFGRWQVKKEIDKYRPWEKFDFEQVRKSPKPISLLLSTQRRKGNKGWSMDEGTEAEIRKVMNGGYQTSYIEVKRGSKVGEKSAWMLNLSIDVPKIDKGVDPSIIGGIDVGVKSPLVCAINNAFSRYSISDNDLFHFNKKMFARRRILLTKSKHKRAGHGAKNKLKPISILTGKSERFRKKLIERWACEIADFFIKNKVGTVQMENLESMKRKEDSYFNIRLRGFWPYAEMQNKIEFKLKQYGIEIRKVAPNNTSKTCSKCGHLNNYFNFEYRKKNKFPHFKCEKCNFKENADYNAALNISNPKLKSTKEKP

SEQ ID NO: 2825 - protein, 726 aa, synthetic construct
SEVEFSHEYWMRHALTLAKRARDEREVPVGAILVLNNRVIGVGWNRAIGLHDPTAHAEIMALRQGGLVMQNYRLIDATLYVTFEPCIMCAGAMIHSRIGRVVFGVRNSKRGAAGSLMNVLNYPGMNHRVEITEGVLADECAALLCDFYRMPRQVLNAQKKAQSSINSGGSSGGGSGGETPGTSESATQESSGGSSGGSAKNTITKTLKLRIVRPYNSAEVEKIVADEKNNREKIALEKNKDRVKEACSKHLKVAAYCTTQVERNACLFCKARKLDDKFYQKLRGQFPDAVFWQEISEIFRQLQKQAAVIYNQGLIELYYEIFIKGKGITNASRVEHYLSDVCYTRAAELFKNAAIASGLRNRIKSNFRLKELKNMKSGLPTTKSDNFPIPLVKQKGGQYTGFEISNHNSDFIIKIPFGRWQAKKEIDKYRPWEKFDFEQVRKSPKPISLLLSTQRRKRNRGWSKDEGTEAEVKKVMNGDYQISYIEVKRGSKIGEKSAWTLNLSIDVPKIDKGVDPSIIGGIDVGVKSPLVCAISNALSRYSINDNDLFHFNKKMFARRRILLKKSKHKRAGHGAKNKLKPITILTEKSRRFRKKLIERWACEIADFFIKNKVGTVQMENLEGMKRKEDSYFNIRLRGFWPYAEMQNKIEFKLKQYGIEIRKVAPNNTSKTCSKCGHLNNYFNFEYRKKNKFPHFKCEKCSFKENADYNAALNISNPKLKSTKEEP

SEQ ID NO: 2826 - protein, 726 aa, synthetic construct
SEDEFSHEYWMRHALTLAKRARDGREVPVGAVLVLNNRVIGEGWNRAIGLHDPTAHAEIMALRQGGLVMQNYRLIDATLYVTFEPCVMCAGAMIHSRIGRVVFGVRNNKHGAAGSLVNVLNYPGMNHRVKITEGILADECAALLCDFYRMPRQVFNARKKAQSSINPGGSSGGSSGSVTPGASESATPKSSGGSSGGSTKNTITKTLKLRIVRPYNSAEVEKIVADEKNNRERIALEKNKDKVKEACSKHLKVAAYCTTQVERNACLFCKARKLDDKFYQKLRGQFPDAVFWQEIGEIFRQLQRQAAEIYNQSLIELYYEIFIKGKGFANASNVEHYLSDVCYTRAAELFKNAAIASGLRGKVKSNFRLKELKNMKSGLPTTKSDNFPIPLVKQKGGRYTGFEISSHNDDFIIKIPFGRWQVRKEIDKYRPWEKYNFEQVRMSPKPISLLLSTQRRRRNKGWSKDEGTEAEIRKVMNGDYQTSYIEVKRGSKTGEKSAWMLNLSIDVPKIDKGVDPSIIGGIDVGVKSPLVCAINNAFSRYSISDNDLFRFNKKMFARRRILLKKNRHKRAGHGAKNKLKPITILTEKSGRFRKKLIERWACEIADFFIKNKVGTVQMENLESMKRKEDSYFNIRLRGFWPYAEMQNKIELKLKQYGIKIRKVAPNSTSKTCSKCGHLNNYFSFEYRKKNKFPHFKCEKCNFKEDADYNAALNISNPKLKSTKEEP

SEQ ID NO: 2827 - protein, 726 aa, synthetic construct
SEVEFSHEYWMRHALTLAKRARDEREVPVGAVLVLNDRVIGEGWNRAIGLHDPTAHAEIMALRQGGLVMQNYRLTDATLYVTFEPCVMCAGAMIHSRIGRVVFGVRNSKRGAAGSLMNVLNYPGMNHCVEITEGILVDECAALLCDFYRMPRQVLNAQKKAQSSINSGGSSGGSSGSETPGTSESATPEGSGGGSSGSAKNTITKTLQLRIVRPYNSAEVEKIVADEKNNREKIALEKNKGKVKEACSKHLKVASYCTTQVERSACPFCKARRLDDKFYQKLGGQFPDAVFWQELGEILRQLQKQAAEIYNQSLIELYYEIFIKGRGFANASSVEHYLSDVCYTRAAELFKNAAIASGLRGKVKSNFRLKELKNMKSGLPTTKSDNFPIPLVKQKGGQYTGFEISSHNDDFIIKIPFGRWQVKKEIDKYRPWEKFDFEQVRKSPKPISLLLSTQRRKRNKGWSKDEGTEAEIRKVMNGDYQTSYIEVKRGSKIGEKSAWMLSLSIDVPKIDKGVDPSTIGGIDVGVKSPLVCAINNAFCRYSISDNDLFHFNKKMFARRRILLKKSRHKRAGHGAKNKLKPISILTEKSKRFRKKLIERWACEIADFFIKNKVGTVQMENLESMKRKEDSYFNIRLRGFWPYAEMQNKIEFKLKQYGIEIRKVAPNNTSKTCSKCGHLNNYFNFEYRKKNKFPHFRCEKCNFKENADYNAALNISNPKLKSTKEEP

SEQ ID NO: 2828 - protein, 726 aa, synthetic construct
SEVEFSHEYWMRHALTLARRARDEREVPVGAILVLNNRVIGEGWNRAIGLHDPTAHAEIMALRQGGLVMQNYRLIDATLYVTFEPCVMCAGAMIHSRIGRVVFGVRNNKHGAAGSLVNVLNYPGMNHRVEITEGILADECAALLCDFYRMPRRVFNARKKAQSSINPGGPSGGSSGSETPGTSESATPESSGGSSAGSTKNTITKTLKLRIVRPYNSAEVEKIVADEKNSREKTALEKNKDKVEEACSKHLKVAAYCTTQVERSACLFCRARKLDDKFYQKLRGQFPEAVFWQEIGEIFRQLQKQAAEIYNQSLIELYYEIFIKGKGFANASSAEHYLSDVCYTRAAELFKNAAIASGLRGKVKSNFRLKELKNMKSGLPTTKSDNFPIPLVKQKGGKYTGFEISSHNDDFIIKIPFGRWQVKKEIDKYRPWEKFDFEQVRKSPKPISLLLSTQRRKRNKGWSKDEGTEAEIRKVMNGDYQTSYIEVKRGSKIGEKSAWMLNLSIDVPKIDKGVDPSIIGGIDVGVKSPLVCAINNAFSRYSISDNDLFHFNKKMFARRRILLKKNRHKRAGHGAKNKLKPISILTEKSKRFRKKLIERWACEIADFFIKNKVGTVQMENLESMKRKEDSYFNIRLRGLWPYAEMQNKIEFKLKQYGIEIRKVAPNNTSKTCSKCGHLNNYFNFEYRRKNKFPHFKCEKCNFKENADYNAALNISNPKLKSTKEEP

SEQ ID NO: 2829 - protein, 726 aa, synthetic construct
SEVEFSHEYWMRHALTLAKRARDEREVPVGAVLVLNNRVIGEGWNRAIGLHDPTAHAEIMALRQGGLVMQNYRLIDATLYVTFEPCVMCAGAMIHSRIGRVVFGVRNSKHGAAGSLMNVLNYPGMNHRVEITEGILADECAALLCDFYRMPRQIFNARKKARSSINPGGPSGGSSGSETPDTSEGATPESSGGNSGGSAKNTITKTLKLRIVRPYNSAEVEKIVADEKNNREKIALEKNKDKVKEACSEHLKVAAYCTTQVERNACLFCKARKLDDKFYQKLRGQFPDAVFWQELGEIFRQLQKQTAEIYNQSLIELYYEIFIKGKGFANASSVEHYLSDVCYTRAAELFKNAAIASGLRNKIKSNFRLKELRNMKSGLPTTKSDNFPIPLVRQKGGQYTGFEISSHNDDFIIKIPFGRWQVKEEIDKYRPWEKFDFEQVRKSPKPISLLLSTQRRKKNKGWSKDEGTEAEIRRVMNGDYQTSYIEVKRGSKIGEKSAWMLNLSIDVPKIDKGVDPSIIGGIDVGVKSPLVCAINNSSSRYSICDNDLFRFNKKMFARRRILLKKNRHKRAGHGAKNKLKPITILTKKSERFRKKLIERWVCEVADFFIKNKVGTVQMENLESMKRKEDSYFNIRLRGFWPYAEMQNRIELKLKQYGIEIRRVAPNNTSRTCSKCGHLNNYFSFEYRKKNKFPHFKCEKCNFKEDADYNAALNISNPKLKSTKEEP

SEQ ID NO: 2830 - protein, 726 aa, synthetic construct
SGVEFSHEYWMRHALTLAKRARDEREVPVGAVLVLNNRVIGEGWNRAIGLHDPAAHAEIMALRQGGLVMQNYRLIGATLYVTFEPCVMCAGAMIHSRVGRVVFGVRNNKHGAAGSLVNVLNYPGMNHRVEITEGILADECAALLCDFYRMPRQVLNAQKKAQSSINSGGSSGGSSSSETPGTSGSATPEGSGGSSSGSAKNTFTKTLQLRIVRPYNSAEVEKIVADEKDNREKIALEKNKDKVKEACSEHLKVAAYCTTQVERNACLFCKARKLDDKFYQKLRGQFPDAVFWQEISEIFRQLQKQAAVVYNQSLIELYYEVFIKGKGFANASSVEHYLSDVCYTRAAELFKNAAIASGLRGKVKSNFRLKELKNMKSGLPTTKSDNFPIPLVKQKGGQYTGFEISSHNDDFIIKIPFGRWQVKKEIDKYRPWEKFDFEQVRKSPKPISLLLSTQRRKRNKGWSKDEGTEAEIRKVMNGDYQTSYIEVKRGSKIGEKSAWMLNLSIDVPKIDKGVNPSIIGGIDVGVKSPLVCAINNAFSRYSISDNDLFHFNKKMFARRRILLKKNRHKRAGHGAKNKLKPISILTEKSKRFRKKLIERWACEIADFFIKNKVGTVQMENLESMKRKEDGYFNIRLRGFWPYAEMQNKIEFKLKQYGIEIRKVAPNNTSKTCSKCGHLNNYFNFEYRKMNKFPHFKCEKCNFKEDADYNAALNISNPKLKSTKEEP

SEQ ID NO: 2831 - protein, 726 aa, synthetic construct
SEVEFSHEYWMRHALTLAKRARDEREVPVGAVLVLNNRVIGEGWNRAIGLHDPTAHAEIMALRQGGLVMQNYRLTDATLYVTFEPCVMCAGAMIHSRIGRVVFGVRNSKRGAAGSLMNVLNYPGMNHCVEITEGILVDECAALLCDFYRMPRQVLNAQKKAQSSISFGGSSGGSSGSETPGASESVTPKSSGGGPAGSTKNTITKTLKLRIVRPYNSAEVEKIVADEKNSREKIALEKNKDKVKEACSKHLKVAAYCTTQVERNACLFCRARKLDDKFYQKLRGQFPDAVFWQEIGEIFRQLQRQAAEIYNQSLIELYYEIFIKGKGFANASSAEHYLSDVCYTRAAELFKNAAIASGLRGKVKSNFRLKELKNMKSGLPTTKSDNFPIPLVKQKGGQYTGFEISSHNDDFVIKIPFGRWQVKREIDKYRPWERFDFEQVRKSPKPISLLLSTQRRKRNKGWSKDEGTEAEIRKVMNGDYQTSYIEVKRGSKIGEKSAWMLNLSIDVPKIDKGVDPSIIGGIDVGVKSPLVCAINNAFSRYSISDNDLFHFNKKMFARRRILLKKTRHKRAGHGAKNKLKPISILTEKSERFRKKLIERWACEIADFFIKNKVGTVQMENLESMKRKEDSYFNIRLRGFWPYAEMQNKIEFKLKQYGIEIRKVAPNNTSKTCSKCGHLNNYFNFEYRKKNKFPHFKCEKCNFKENADYNAALNISNPKLKSTKKEP

SEQ ID NO: 2832 - protein, 726 aa, synthetic construct
SEVEFSHEYWMRHALTLAKRARDEREVPVGAILVLNNRVIGEGWNRAIGLHDPTAHAEIMALRQGGLVMQNYRLIDATLYVTFEPCVMCAGAMVHSRIGRVVFGVRNSKRGAAGSLMNVLDYPGMGHRVEVTEGILADECAALLCDFYCMPRQVFNAQKRAQSSINSGGSSGGSSGSETPGTSESATPESSGGGSSGSAKNTITKTLQLRIVRPYNSAEVEKIVADEKNNREKIALEKNKDKVREACSKHLKVASYCTTQVERNACPFCKARKLDDKFYQKLRGQFPDAVFWQELGEILRQLQRQAAEIYNQSLIELYYEIFIKGRGFANASSVEHYLSDVCYTRAAELFKNAAIASGLRSKVRSNFRLKELKNMKSGLPTTKSDNFPIPLVKQKGGQYTGFEISSHNSDFIIKIPFGRWQEKEEIGKYRPWEKFDFEQVRRSPKPISLLLSTQRRKKNKGWSKDEGTEAEIRRVMNGDYQTSYIEVKRGSKIGEKSAWMLSLSIDVPKIDKGVDPRIIGGIDVGVKSPLVCAINNAFSRYSISDNDLFHFNKKMFARRRILLKKNRHKRAGHGAKNKLKPITILTEKSVRFRKKLIERWACEIADFFVKNKVGTVQMENLESMKGKEDSYFNIRLRGFWPYAEMQNKIEFKLKQYGIKIRKVAPNNTSKTCSKCGHLNNYFSFEYRKKNKFPHFKCEKCNFKENADYNAALNISNPKLKSTKEEP

SEQ ID NO: 2833 - protein, 726 aa, synthetic construct
SEVEFSHEYWMRHALTLAKRARDEREVPVGAILVLNNRVIGEGWNRAIGLHDPTAHAEIMALRQGGLVMQNYRLIDATLYVTFEPCVMCAGAMIHSRIGRVVFGVRNSKHGAAGSLVNALNYPGMNHRVEITEGILADECAALLCDFYRMPRQVFNARKKAQSSINPSGSSGGSSGSVTPGTSESATPESSGGGFGGSAKNTITKTLQLRIVRPYNSAEVEKIVADEKNNREKIALEKNKDKVKEACSKHLKVASYCTTQVERNACLFCKARKLDDKFYQKLRGQFPDAVFWQELGEIFRQLQKQAAEIYNQSLIELYYEVFIKGKGFANASSVEHYLSDVCYTRAAELFKNAAIASGLRGKVKSNFRLKELKNMKSGLPTTKSDNFPIPLVKQKGGQYTGFEISSHNDDFIVKIPFGRWQVKKEIDKYRPWEKFDFEQVRKSPKPISLLLSTQRRKRNKGWSKDEGTEAEIRKVMNGDYQTSYIEVKRGSKIGEKSAWMLNLSIDVPKIDKGVDPSIVGGIDVGVKSPLVCAIDNALSRYSISDNDLFHFNKKMFARRRILLKKNRHKRAGHGAKNKLKPITILTEKGVRFRKKLIERWACEIADFFIKNKVGTVQMENLESMKGKEDSYFNIRLRGFWPYAEMQSKIEFKLKQYGIEIRKVAPNNTSKTCSRCGHLNNYFNFEYRRKNKFPHFKCEKCNFKENADYNAALNISNPKLKSTKEEP

SEQ ID NO: 2834 - protein, 726 aa, synthetic construct
SEVEFSHEYWMRHALTLAKRARDEREVPVGAVLVLNNRIIGEGWNRAIGLHDPTAHAEIMALRQGGLVMQNYRLTDATLYVTFEPCVMCAGAMIHSRIGRVVFGVRNSKRGAAGSLMNVLSYPGMNHCVEITEGILVDECAALLCDFYRMPRQVLSAQKKAQSSISSGGLPGGSSGSETPGVSESVTPKSSVGSSASSTKNTITKTLKLRIVRPYNSAEVEKIVADEKNNREKIALEKNKDKVKEACSKHLKVAAYCTTRVERNACLFCKARRLDDKFYQKLRGQFPDAVFWQEIGEIFRQLQKQAAEVYNQSLVELYYEILIKGKGIANASSVEHYLSDVCYTRAAKLFKNAAIASGLRNKIKSNFRLKELRNMKSGLPTTKSDNFPIPLVRQKGGQYTGFEISNHDGDFIIKIPFGRWQVKKEINKHRPWEKFDFEQVRKSPKPISLLLSTQRRKRNKGWSKDEGTEAEIRKVMDGDYQTSYIEVKRGRKIGEKSVWMLNLSIDVPKIDKGVDPSTIGGIDVGVKSPLVCAINNAFSRYSISDNDLFRFNKKMFARRRILLKKNRHKRAGHGAKNKLKPITILTEKSGRFRKKLIERWACEIADFFIKNKVGTVQMENLESMKRKGDSYFNIRLRGFWPYAEMQNKIEFKLKQYGIEIRKVAPNNTSKTCSKCGHLNNYFNFEYRKKNKFPHFKCEKCNFKENADYNAALNISNPKLKSTKGEP

SEQ ID NO: 2835 - protein, 726 aa, synthetic construct
SEVEFSHEYWMRHALTLAKRARDEREVPVGAVLVLNNRVIGEGWNRAIGLHDPTAHAEIMALRQGGLVLQNYRLVDATLYVTFEPCVLCAGAMVHSRIGRVVFGARNSKRGAAGSLMNILNYPGMNHCVEITEGILVDECAALLCDFYRMPRQVFNARKKAQSTINSGGSSGGSSGSETPGTSESATPESSGGGFGGSAKNTITKTLQLRIVRPYNSAEVEKIVADEKNNREKIALEKNKDKVKEACSKHLKVASYCTTQVERNACLFCKARKLDDKFYQKLRGQFPDAVFWQELGEIFRQLQKQAAEIYNQSLIELYYVIFIKGKGLANASSVEHYLSDVCYTRAAELFKNAAIASGLRSKVRSNFRLKELKNMKSGLPTTKSDNFPIPLVKQKGGQYTGFEISSHNSDFIIKIPFGRWQEKEEIDKYRPWEKFDFEQVRRSPKPISLLLSTQRRKRNRGWSKDEGTEAEIRKVMNGDYQTSYIEVKRGSKFGEKSAWMLNLSIDVPKIDKGVDPSIIGGIDVGVKSPLVCAINNAFSRYSISDNDLFRFNKKMFARRRILLGKNRHKRAGHGVKNKLKPITILTEKSGRFRKKLIERWACEIADFFVKNKVGTVQMENLESMKRKEDSYFNIRLRGFWPYAEMQNKIEFKLKQYGIKVRKVAPNNTSKTCSKCGHLNNYFSFEYRKKNKFPHFKCEKCNFKENADYNAALNISNPKLKSTKEEP

SEQ ID NO: 2836 - protein, 726 aa, synthetic construct
SEVEFSHEYWMRHALTLAKRARDEREVPVGAVLVLNNRVIGEGWNRAIGLHDPTAHAEIMALRQGGLVMQNYRLTDATLYVTFEPCVMCAGAMIHSRIGRVVFGVRNSKRGAAGSLMNALNYPGMNHCVEITEGILVDECAALLCDFYRMPRQVLNAQKKAQSSISPGGSSGGSSGSETPGASGSVTPKSSGGGSSGSAKNTITKTLQLRIVRPYNSAEVEKIVTDEKNNREKIALEKNKDKVKEACGEHLKVAAYCTTQVERNACLFCRARKLDDKFYQKLRGRFPDAVFWQEIGEIFRQLQKQAAEIYNQSLIELYYEIFIKGKGFANASSVEHYLSDVCYTRAAELFKNAAIASGLRGKVKSNFRLKELKNMKSGLPTTKSDNFPIPLVKQKGGQYTGFEISNRNSDFIIKIPFGRWQVKKEINKYRPWEKFDFEQVRKGPKPISLLLSTQRRKRNKGWSKDEGTEAEIRKVMNGDYQTSYIEVKRGSKIGEKSAWMLNLSIDVPKIDKGVDPSIVGGIDVGVKSPLVCAINNALGRFSISDNDLFHFNKKMFARRRILLKKNRHRRTGHGARNKLKPITVLTEKSERFRKKLIERWACEIANFFIKNKVGTVQMENLESMKRREDSYFNIRLRGLWPYAEMQNKIEFKLKQYGIKIRKVAPNNTSKTCSKCGHLNNYFSFEYRKKNKFPHFKCEKCNFKENADYNAALNISNPKLMSTKEEP

SEQ ID NO: 2837 - protein, 726 aa, synthetic construct
SEDEFSHEYWMRHALTLAKRARDGREVPVGAVLVLDNRVVGEGWNRAIGLHDPTAHAEIMALRQGGLVMQNYRLIDATLYVTFEPCVMCAGAMVHSRIGRVVFGVRNSKRGAAGSLMNVLDYPGMGHRVEITEGILADECAALLCDFYCMPRQVFNAQKRAQSSINSGGSSGGSSGSETRGTSESATPGSSGGGSSGSAKNTITKTLQLRIVRPYNSAEVEKIVADEKNNREKIALEKNKDKVKEACSKHLKVASYCTTQVERNTCPFCKARKLDDKFYQKLRGQFPDAVFWQELGEILRQLQKQAAEIYNQSLIELYYEIFIKGRGFANANSVEHYLSDVCYTRAAELFKNAAIASGLRNKVKSNFRLKELRNMKSGLPTTKSDNFPIPLVRQKGGQYTGFEISNHDGDFIIKIPFGRWQVKKEINKHRPWEKFDFEQVRKSPKPISLLLSTQRRKRNKGWSKDEGTEAEIRKVMNGDYQTSYIEVKRGSKTGEKSAWMLNLSIDVPKIDKGVDPSIIGGIDVGVKSPLVCAINNAFSRYSISDNDLFRFNKKMFARRRILLKKNRHKRAGHGAKNKLKPISILTGKSERFRKKLIERWACEIADFFIKNKVGTVQMENLESMKRKEDSYFNIRLRGFWPYAEMQNKIEFKLKQYGIEIRKVAPNNTSKTCSKCGHLNNYFNFEYRKKNKFPHFKCEKCNFKENADYNAALNISNPKLKSTKEEP

SEQ ID NO: 2838 - protein, 726 aa, synthetic construct
SEVEFSHEYWMRHALTLAKRARDEREVPVGAVLVLNNRVIGEGWNRAIGLHDPTAHAEIMALRQGGLAMQNYRLVDATLYVTFEPCVLCAGAMVHSRIGRVVFGVRNSKRGAAGSLMNVLNHPGMSHRVEITGGILADECAALLCDFYRMPRQVFNAQKKARSNINSGGSSGGSSGSETPGTSESATPESSGGSSGGSAKNTITKTLQLRIVRPYNSAEVEKIVTDEKNNREKIALEKNKDKVKEACSKHLKMASYCTTQVERNACLFCKARKLDDKFYQKLRGQFPDAVFWQEIGEIFRQLQKQAAEIYNQSLIELYYEIFIKGKGITNASRVEHYLSDVCYTRAAELFKNAAIASGLRSKVRSNFRLKELKNMKSGLPTTKSDNFPIPLVKQKGGQYTGFEISSHNSDFIIKIPFGRWQVKEEIDKYRPWEKFDFEQVRKSPKPISLLLSTQRRKKNKGWSKDEGTEAEIRRVMNGDYQTSYIEVKRGSKIGEKSAWMLNLSIDVPKIDKGVDPSIIGGIDVGVKSPLVCAINNAFSRYSISDNDLFHFNKKVFARRRILLKKTRHKRAGHGAKNKLKPISILTEKSERFRKKLIERWACEIADFFIKNKVGTVQMENLESMKRKEDSYFNIRLRGLWPYAEMQNKIEFKLKQYGIKIRKVAPNNTSKTCSKCGHLNNYFNFEYRKRNKFPHFKCEKCNFKENADYNAALNISNPKLKSTKEEP

SEQ ID NO: 2839 - protein, 726 aa, synthetic construct
SEVEFSHEYWMRHALTLAKRARDEREVPVGAILVLNNRVIGEGWNRAIGLHDPTAHAEIMALRQGGLVMQNYRLIDATLYVTFEPCVMCAGAMIHSRIGRVVFGVRNNKHGAAGSLVNVLNYPGMNHRVEITEGILADECAALLCDFYRMPRQVFNARKKAQSSINPGGSSGGSGGSETPGTSESATPENSGGSSGSSAKNTITKTLKLRIVRPYNSAEVEKIVADEKNNREKIALEKNKDKVKEACSRHLKVASYCTTQVERNACPFCKARKLDDKFYQKLRGQFPDAVFWQELGEILRQLQKQAAEIYNQSLIELYYEIFIKGKGFANASSVEHYLSDVCYTRAAELFKNAAIASGLRGKVKGNFRLKELKNMKSGLPTTKSDNFPIPLVRQKGGQYTGFEISNHNSDFIIKIPFGRWQAKKEIDKYRPWEKFDFEQVRKSPKPISLLLSTQRRKRNRGWSKDESTEAEIKKVMNGDYQTSYIEVKRGSKVGEKSAWMLNLSIDVPKIDKGVDPSIIGGIDVGVKSPLVCAINNAFSRYSISDNDLYRFNKKMFARRRILLKKSKHKRAGHGAKNKLKPISILTGKSGRFRKKLIERWACEIADFFIKNKVGTVQMENLEGMKRKEDSYFNIRLRGLWPYAEMQNKIEFKLKQYGIEIRKVAPNNTSKTCSKCGHLNNYFNFEYRRKYKFPHFKCEKCNFKEDADYNAALNISNPKLKSTKEEP

SEQ ID NO: 2840 - protein, 726 aa, synthetic construct
SEVEFSHEYWMRHALTLAKRARDGREVPVGAVLVLNNRVIGEGWNRAIGLHDPTAHAEIMALRQGGLVMQNYRLIDATLYVTFEPCVMCAGAMVHSRIGRVVFGVRNSKRGAAGSLMNVLDYPGMGHRVEITEGILADECAALLCDFYCMPRQVFNAQKRAQSSINSGGSSGGSSGSETPGTSESATPESSGGGSSGSAKNTITKTLQLRIVRPYNSAEVEKIVADEKNNREKIALERNKDKVKEACSKHLKVASYCTTQVERSACPFCKARKLDDKFYQKLGGQFPDAVFWQELGEILRQLQKQAAEIYNQSLIELYYEIFIKGRGFANASSVEHYLSDVCYTRAAELFKNAAIASGLRGKVKSNFRLKELKNMKSGLPTTKSDNFPIPLVKQKGGQYTGFEVSNHNSDFIIKIPFGRWQAKKEIDKYRPWEKFDFEQVRKSPKPISLLLGTQRRKRNRGWSKDEGTEAEIKKVMNGDYQTSYIEVKRGSKIGEKSAWMLNLSIDVPRIDKGVDPSIIGGIDVGVKSPLVCAINNAFSRYSISDNDLFRFNKKMFARRRILLKKNRHKRAGHGAKNKLKPISILTGKSERFRKKLIERWACEIADFFIKNKVGTVQMENLESMKRKEDSYFNIRLRGFWPYAEMQNKIEFKLKQYGIEIRKVAPNNTSKTCSKCGHLNNYFNFEYRKKNKFPHFKCERCNFKENADYNAALNISNPKLKSTKGEP

SEQ ID NO: 2841 - protein, 726 aa, synthetic construct
SEVEFSHEYWMRHALTLAKRARDEREVPVGAILVLNNRVIGEGWNRAIGLHDPTAHAEIMALRQGGLAMQNYRLTDATLYATFEPCVMCAGAMIHSRIGRVVFGVRNSKHGAAGSLMNVLNYPGMNHRVEITEGILADECAGLLCDFYRMPRQVFSARKKAQSSINPGGSSGGSSGGKAPGTSESATLESSGGSSGDSAKNSITKTLKLRIVRPYNSAEVEKIVADEKNNREKIALEKNKGKVEEACSKHLKVATYCTTQVERNACLFCKARKLDDKFYQKLRGQFPDAVFWQELGEIFRQLQKQAAEIYNQSLIELYYEIFIKGKGLANASSVEHYLSDVCYTRAAELFKNAAIASGLRGKVKSNFKLKELKSMKSGLPSTKSDNFPIPLVKQKGGQYTGFEISSHNDDLIIKIPFGRWQVKEEIDKYRPWEKFDFEQVRKNPKPISLLLSTQRRKGNKGWSKDEGTEAEIRKVMNGDYQTSYIEVKRGSKTGGKSAWMLNLSIDVPKIDKGVDPCIIGGIDVGVKSPLVCAINDAFSRYSISDNDLFHFNKKMFARRRILLKKNGHKRAGHGAKNKLRPITIMTEKSKRFRKKLIERWACEIADFFIKNKVGTVQMENLESMKRKEDSYFNIRLRGFWPYAEMQNKIEFKLKQYGIVVRKVAPNNTSKTCSKCGHLNNYFSFEYRKKNKFPHFKCEKCNFKENADYNAALNISNPKLKSTKEEP

SEQ ID NO: 2842 - protein, 726 aa, synthetic construct
SEVEFSHEYWMRHALTLAKRARDGREVPVGAVLVLNNRVIGEGWNRAIGLHDPTAHAEIMALRQGGLVMQNYRLIDATLYVTFEPCAMCAGAMVHSRIGRVVFGVRNSKRGAAGSLMNVLNYPGMDHRVEITGGILADECAALLCDFYRMPRRVFNAQKKAQPSINSGGPSGGSSGSETPGTSESAAPKSSGGSSAGSTKDAITKTLKLRIVRPYNSAEVEKIVADEKNNREKIAMEKNKDKVKEACSKHLKVASYCTTQVERNACLFCKARKLDDEFYQKLRGQFPDAVFWQELGGIFRQLQKQAAEIYNQSLIELYHEIFIKGKGITNASRVEHYLSDVCYTRAAELFKNAAIASGLRSKVRSNFRLKELKNMKSGLPTTKSDNFPIPLVKQKGGQYTGFEISSHNSDFIIKIPFGRWQEKEEIDKYRPWEKFDFEQVRKSPKPISLLLSTQRRKKNKGWSKDEGTEAEIRRVMNGDYQTSYIEVKRGSKIGEKSAWMLNLSIDVPKIDKGVDPSIIGGIDVGVKSPLVCAINNAFSRYSISDNDLFHFNKKMFARRRILLKKNRHRRAGHGAKNKLKPITILTEKSARFRKKLIERWACEIADFFIKNKVGTVQMENLESMKRKEDSYFNIRLRGFWPYAEMQNKIEFKLKQYGIEIRRVAPNNTSRTCSKCGHLNNYFNFEYRRKNKFPHFKCEKCNFREDADYNAALNISNPKLKSTKEEP

SEQ ID NO: 2843 - protein, 726 aa, synthetic construct
SEVEFSHEYWMRHALTLAKRARDEREVPVGAVLVLNNRVIGEGWNRTTGLHDPTAHAEIMALRQGGLVMQNHRLVDATLYVTFEPCVMCAGAMIHSRIGRVVFGVRNSKRGAAGSLTNVLNYPGMNHRVEITEGILVGECAALLCDFYRMPRQVFNAQKKAQSTINTGGSSGGSSGSETPGTSESPTPESSGSSPGGSAKNTITKTLKLRIVRPYNSAEVEKIVADEKNNREKIALEKNKDKVKEACSKHLKVAAYCTTQVERNACLFCKARKLDDKFYQKLRGQFPDAVFWQEIGEIFRQLQKQAAEIYNQSLIELYYEIFIKGKGFANACSVEHYLSDVCYTRAAELFKNAAIASGLRGKVKSNFRLKELKNMKSGLPTTKSDNFPIPLVKQKGGQYTGFEISSHNDDFIIKVPFGRWQVKKEIDKYRPWEKFDFEQVRKSPKPISLLLSTQRRKRNKGWCKDESTEAEIKKVMNGDYQTSYIEVKRGSKVGEKSVWMLSLSIDVPKIDKGVDPSIIGGIDVGVKSPLVCAINNAFSRYSISDNDLFHFNKKMFARRRILLKKNRRRRAGHGAKNKLKPITILTEKSVRFRKKLIERWACEIANFFIKNKVGTVQMENLESMKRREDSYFNIRLRGFWPYAEMQSKIEFKLKQYGIKIRKVAPNNTSKTCSKCGHLNNYFNFEFRKKNKFPHFKCEKCNFKEDADYNAALNISNPKLKSTKEEP

SEQ ID NO: 2844 - protein, 726 aa, synthetic construct
SEVEFSHEYWMRHALTLAKRARDEREVPVGAVLVLNNRVIGEGWNRTTGLHDPTAHAEIMALRQGGLVMRNYRLTDATLYVTFEPCVMCAGAMIHSRIGRVVFGVRNSKRGAAGSLMNVLNYPGMNHCVGITEGILVDECAALLCDFYHMPPQVLNARKKAQSSISSGGSSGGSNGSETPGASESATPKSSGGSSAGSTRNTITKTLQLRIVRPYNCAEVEKIVADEKNNREKIALEKNKDKVKEACSKHLKVAPYCTTQVERSACLFCKARKLDDRFYQKLRGQFPDAVFWQEVSEIFRQLQKQAAEIYNQSLIELYYEIFIKGKGFANASNVEHYLSDVCYTRAAELFKNAAIASGLRSKVKSNFRLKELKNMKSGLPTTKSDNFPIPLVKQKGGQYTGFEISSRNDDFIIKIPFGRWQAKKEIDRYRPWEKFDFEQVRKSPKPISLLLSTRRRKGNKGWSKDEGTEAEIRRVMNGDYQTSYIEVKRGSKIGEKSAWMLSLSIDVPKIDKGVDPRIIGGIDVGVKSPLVCAINNVLSRYSISDNDLFHFNKKMFARRRILLKKNGHKRAGHGAKNKLKPITIMTEKSKRFRKKLIERWACEIADFFIKNKVGTVQMENLESMKRKEDSYFNIRLRGFWPYAEMQNKIEFKLKQYGIVVRKVAPDNTSKTCSQCGHLNNYFNFEYRKKNKFPHFKCEKCNFKEDADYNAALNISNPKLKSTKEEP

SEQ ID NO: 2845 - protein, 726 aa, synthetic construct
SEVEFSHEYWMRHALTLAKRARDEREVPVGAILVLNNRVIGEGWNRAIGLNDPTAHAEIMALRQGGLVMQNYRLIDATLYVTFEPCVMCAGAMIHSRIGRVVFGVRNSKHGAAGSLVNVLNHPGMNHRVEITEGILADECAALLCDFYRMPRQVFNARKKAQSSINPGGSSGGSSGSETPGTSESATPESSGGSSGGSAKNTITKTLKLRIVRPYNSAEVEKIVADEKNNREKTALEKNKDKVKEACSEHLKVATYCTTQVERNACLFCKARKLDDKFYQKLRGQFPDAVFWQEIGEIFRQLQKQAAEIYNQSLIELYYEIFIKGKGFANASSVEHYLSDVCYTRAAELFKNAAIASGLRNKTKSNFRLKELRSMKSGLPTTKSDNFPIPLVKQKGGQYTGFEISNHNSDFIIKIPFGRWQAKKEIDKYRPWEKFDFEQVRKSPKPISLLLSTQRRKRNKGWSKDEGTEAEIEKVMNGDYRTSYIEVKRGSKTGGKSAWMLNLSIDVPKIDKGVDPCIIGGIDVGVKSPLVCAINDAFSRYSISDNDLFHFNKKMFARRRILLKKNGHKRAGHGAKNKLKPITIMTEKGKRFRKKLIERWACEIADFFIKNKVGTVQMENLESMKRKEDSYFNIRLRGFWPYAEMQNKIEFKLKQYGIVVRKVAPNNTSKTCSKCGHLNNYFNFEYRKKNKFPYFKCEKCNFKENADYNAALNISNPQLKSTKGEP

SEQ ID NO: 2846 - protein, 726 aa, synthetic construct
SEVEFSHEYWMRHALTLAKRARDEREVPVGAVLVLNNRVIGEGWNRAIGLHDPTAHAEIMALRQGGLAMQNYRLVDATLYVTFEPCVLCAGAMVHSRIGRVVFGVRNSKRGAAGSLMNVLNHPGMSHRVEITGGILADECAALLCDFYRMPRQVFNAQKKARSNINSGGSSGGSSGSETLGTSESATPESSGGSSGGSAKNTITKTLKLRIVRPYNSAEVEKIVADEKNNREKIALEKNRDKVKEACSKHLKVAAYCTTQVERNACPFCKARKLDDKFYQKLRGQFPDAVFWQELGEILRQLQKQAAEIYNQSLVELYYEIFIKGRGFANASSVEHYLSDVCYTRAAELFKNAAIASGLRGKVKSSFRLKELKNMKSGLPTTKSDNFPIPLVKQKGGQCTGFEISSHNSDFIIKIPFGRWQEKEEIDKYRPWEKFDYEQVRRSPKPISLLLSTQRRKRNKGWGKDEGTEAEIRKVMNGDYQTSYIEVKRGSKIGEKSAWMLSLSIDVPKIDKGVDPRIIGGIDVGVKSPLVCAINNAFSRYSISDNDLFHFNKKMFARRRILLKKNRHKRAGHGAKNKLKPITILTEKSVRFRKKLIERWACEIADFFIKNKVGTVQMENLESMKGKEDSYFNIRLRGFWPYAEMQNKIEFKLKQYGIEIRKVAPNNTSKTCSKCGHLNNYFNFEYRKKNKFPHFKCEKCYFKEDADYNAALNISNPRLKSTKEEP

SEQ ID NO: 2847 - protein, 726 aa, synthetic construct
SEVEFSHEYWMRHALTLAKRARDEREVPVGAVLVLNNRVIGEGWNRAIGLHDPTAHAEIMALRQGGLVMQNYRLTDATLYVTFEPCVMCAGAMIHSRIGRVVFGVRNSKRGAAGSLMNVLNYPGMNHCVEITEGILVDECAALLCDFYRMPCQVLNAQKKAQSSISSGGSSGGSSGSDTLGASESVTPKSSVGSSASSTKNTITKTLKLRIVRPYNSAEVEKIVADEKDNREKIALERNKDKVKEACSKHLKVAAYCTTQVERNACLFCKARKLDDKFYQKLRGQFPDAVFWQELGEIFRQLQKQAAEIYNQSLIELYYEIFIKGKGFANASSVEHYLSDVCYTRAAELFKNAAIASGLRGKVKSNFRLKELKNMKSGLPTTKSDNFPIPLVKQKGGQYTGFEISSHNDDFIIKIPFGRWQVKKEIDKYRPWEKFDFEQVRKSPKPISLLLSTQRRKRNKGWSRDEGTEAEIRKVMNGDYQTSHIEVKRGSKTGEKSAWMLNLSIDVPKIDKGVDPSIIGGIDVGVKSPLVCAINNAFSRYSISDNDLFRFNKKMFARRRILLKKNRHKRAGHGAKNKLKPISILTGKSERFRKKLIERWACEIADFFVKNKVGTVQMENLESMKRKEDSYFNIRLRGFWPYAEMQDKIEFKLKQYGIEIRKVAPNNTSKTCSRCGHLNNYFNFEYRKKNKFPHFKCEKCNFKENADYNAALNISNPKLKSTKEEP

SEQ ID NO: 2848 - protein, 726 aa, synthetic construct
SEVEFSHEYWMRHALTLAKRARDEREVPVGAILVLNNRVIGVGWNRAIGLHDPTAHAEIMALRQGGLVMQNYRLIDATLYVTFEPCVMCAGAMIHSRIGRVVFGVRNSKHGAAGSLVNVLNYPGMNHRVEITEGILADECAALLCDFYRMPRQVFNARKKAQSSINSGGSSGGSSGSETPGTSESATPKSSGGSSGGSAKNTITKALKLRIVRPYNSAEVEKIVADEKNNRERIALEKNKDKVKEACSKHLKVAAYCTTQVERNACLFCKARKLDDKFYQKLRGQFPDAVFWQEIGEIFRQLQKQAAEIYNQSLIELYYEILIKGKGFANASSVEHYLSDVCYTRAAELFKNAAIASGLRGKVKSNFRLKELKNMRSGLPTTKSDNFPIPLVKQKGGQCTGFEISNHNSDFIIKIPFGRWQVKKEIDKYRPWEKFDFEQVRKSPKPISLLLSTQRRKRNKGWSKDEGTEAEIRKVMNGDYQTSYIEVKRGSKIGEKSAWMLNLSIDVPKIDKGVDPSIIGGIDVGVKSPLVCAINNAFSRYSISDNDLFRFNKKMFARRRILLRKNRHKRAGHGAKNKLKPISILTGKSERFRKKLIERWACEIADFFIKNKVGTVQMENLESMKRKEDSYFNIRLRGFWPYAEMQNKIEFKLKQYGIEIRKVAPNNTSKTCSKCGHLNNYFNFEYRKKNKFPHFKCEKCYFKEDADYNAALNISNPRLKSTKEEP

SEQ ID NO: 2849 - protein, 726 aa, synthetic construct
SEVEFSHEYWMRHALTLAKRARDEREVPVGAVLVLNNRVIGEGWNRAIGQHDPTAHAEIMALRQGGLVMQNYRLVNATLYVTFEPCVMCAGAMIHSRIGRVVFGVRNSKRGAAGSLMNVLNYPGMNHRVEITEGILTDECAALLCDFYRMPHQVLNAQKKAQSSINPGGPSGGSSGSETPDTSESATPESSGGNSGGSAKNTITKTLKLRIVRPYNSAEVEKIVADEKNNREKIALEKNKDKVKEACSEHLKVAAYCTTQVERNACLFCKARKLDDKFYQKLRGQFPDAVFWQELGEIFRQLQKQTAEIYNQSLIELYYEIFIKGKGFANASSVEHYLSDVCYTRAAELFKNAAIASGLRGKVKSNFRLKELKNMRSGLPTTKSDNFPIPLVKQKGGQYTGFEISSHNDDFIIKIPFGRWQVKKEIDKYRPWEKFDFEQVRKSPKPISLLLSTQRRERNKGWSKDEGTEAEIRKVMNGDYQTSYIEVKRGSKIGEKSAWMLNLSIGVPKIDKGVNPSIIGGIDVGVKSPLVCAINNAFSRYSISDNDLFHFNKKMFARRRILLKKNRHRRAGHGAKNKLKPITILTEKSARFRKKLIERWACEIADFFIKNKVGAVQMENLESMKRKEDSYFNIRLRGFWPYAEMQNKIEFKLKQYGIEIRRVAPNNTSRTCSKCGHLNNYFNFEYRRKNKFPHFKCEKCNFKEDADYNAALNISNPKLKSTKEEP

SEQ ID NO: 2850 - protein, 726 aa, synthetic construct
SEVEFSHEYWMRHALTLAKRARDKREVPVGAVLVLNNRVIGEGWNRAIGLHDPTAHAEIIALRQGGLVMQNYRLTDATLYVTFEPCVMCAGAMIHSRIGRVVFGVRNNKRGAAGSLMNVLDYPGMGHRVEITEGILAGECAALLCDFYCMPRQVFNAQKRAQSSINSGGSSGGSSGSETPGTSESATPESSVGSSAGSTKNTITKTLKLRIVRPYNSAEVEKIVADEKNNREKIALEKNKDKVKEACSKHLKVAAYCTTQVERNACLFCKARKLDDRFYQKLRGQFPDAVFWQEISEIFRQLQKQAAEIYNQSLIELYYEIFVKGKGFANASSVEHYLSDVCYTRAAELFKNAAIASGLRGKVKSNFRLKELKNMKSGLPTTKSDNFPIPLVKQKGGQYTGFEINSHNDDFIIKIPFGRWQVKKEIDKYRPWEKFDFEQVRKGPKPISLLLSTRRRKRNKGWSKDEGTEAEIKRVMNGDYQISYIEVKRGSKIGEKSAWMLSLSVDVPKIDKGVDPSIIGGIDVGVKSPLVCAINNALSRYSISDNDLFHFNKKMFARRRILLKKNRHKRAGHGAKNKLKPISILTERSERFRKKLIERWACEIADFFIKNKVGTVQMENLESMKRKEDSYFNIRLRGFWPYAEMQDKIEFKLKQYGIEIRKVAPNNTSKTCSRCGHLNNYFNFEYRRKNKFPHFKCEKCNFKENADYNAALNISNPKLKSTKEEP

SEQ ID NO: 2851 - protein, 726 aa, synthetic construct; identical to SEQ ID NO: 684

SEQ ID NO: 2852 - protein, 726 aa, synthetic construct
SEVEFSHEYWMRHALTLAKRARDGREVPVGAILVLNNRVIGEGWNRAIGLHDPTAHAEIMALRQGGLVMQNYRLIDATLYVTFEPCAMCAGAMIHSRIGRVVFGVRNSKHGAAGSLVNVLNYPGMNHRVEITEGILADECAALLCDFYRMPRQVFNAQKKAQSSINPGGSSGGSSGSETPGTSESATPESSGGSSGSSAKNTITKTLKLRIVRPYNSAEVEKIVADEKNNREKIALEKNKDKVKEACSKHLKVAAYCTTQVERNACLFCKARRLDDKFYQKLRGQFPDAVFWQEIGEIFRQLQKQAAEIYNQSLVELYYEILIKGKGIANASSVEHYLSDVCYTRAAGLFKNAAIASGLRNKIKSNFRLKELRNMKSGLPTTKSDNFPIPLVKQKGGQYTGFEISNHDGDFIIKIPFGRWQVKREINKHRPWEKFDFEQVRKSPKPISLLLSTQRRKRNKGWSKDEGTEAEIRKVMNGDYQTSYIEVKRGSKIGEKSAWMLNLSIDVPKIDKGVDPSIIGGIDVGVKSPLVCAINNAFSRYSISDNDLFHFNKKMFARRRILLKKNRHKRAGHGAKNKLKPISILTEKSGRFRKKLIEKWACEIADFFIKNKVGTVQMENLESMKKREDSYFNIRLRGFWPYAEMQNKIEFKLKQYGIVVRKVAPNNTSKTCSKCGHLNNYFNFEYRKKNKFPHFKCEKCNFKEDADYNAALNISNPKLKSAKEEP

SEQ ID NO: 2853 - protein, 726 aa, synthetic construct
SEVEFSHEYWMRRALTLAKRARDEREVPVGAVLVLNNRVIGEGWNRAIGLHDPTAHAEIMALRQGGLVMQNYRLTDATLYVTFEPCVMCAGAMIHSRISRVVFGVRNSKHGAAGSLVNVLNYPGMNHRVEITEGILADECAALLCDFYRMPRQVFSARKKAQSSINSGGSSGGNSGNKTPGTSESATPESSGGSSGSSAKNTITKTLKLRIVRPYNSAEVEKIVADEKNNREKIALEKNKDKVKEACSKHLKVAAYCTTQVERNACLFCRARRLDDKFYQKLRGQFPDAVFWQEIGEIFRQLQKQAAEIYNQSLIELYYEIFIKGRGFANASSVEHYLSDVCYTRAAELFKNAAIASGLRGKVKSNFRLKELKNMKSGLPTTKSDNFPIPLVKQKGGQYTGFEISSHNDDFIIKIPFGRWQVKKEIDKYRPWEKFDFEQVRKSPKPISLLLSTQRRKRNKGWSKDEGTEAEIRKVMNGDYQTSYIEVKRGSKTGEKSAWMLNLSIDVPKIDKGVDPCIIGGIDVGVKSPLVCAINNAFSRYNISDNDLFHFNKKMFARRRILLKENGHKRAGHGAKNKLKPITIMTEKSKRFRKKLIERWACEIADFFIKNKVGTVQMENLESMKRKEDSYFNIRLRGFWPYAEMQNKIEFKLKQYGIVVRKVAPNNTSKTCSECGHLNNYFNFEYRKKNKFPLFKCEKCNFKENADYNAALNISNPKLKSTKGEP

SEQ ID NO: 2854 - protein, 726 aa, synthetic construct
SEVEFSHEYWMRHALTLAKRARDEREVPVGAVLVLNNRVIGEGWNRAIGLHDPTAHAEIMALRQGGLVMQNYRLTDATLYVTFEPCVMCAGAMIHSRIGRVVFGVRNSKRGAAGSLMNVLNYPGMNHCVEITEGILVDECAALLCDFYRMPRQVLNAQKKAQSSISSGGSSGGSSGSETPGASGSVTPKSSGGSSAGSTKDTITKTLKLRIVRPYNSAEVEKVVADEKNNREKIAMEKNKDKVKEACSKHLKVASYCTTQVERNACLFCKARKLDDKFYQKLRGQFPDAVFWQELGEILRQLQKQAAEIYNQSLIELYYEIFIKGRGFANASSVEHYLSDVCYTRAAELFKNAAIASGLRGKVKSNFRLKELRNMKSGLPTTKSDNFPIPLVRQKGGQYTGFEISNHDGDFIIKIPFGRWQVKKEIDKYRPWEKFDFEQVRKSPKPISLLLSTQRRKRNKGWSKDEGTEAEIRKVMSGDYQTSYIEVKRGSKIGEKSAWMLNLSIDVPKIDKGVDPSIIGGIDVGVKSPLVCAINNAFSRYSISDNDLFHFNKKMFARRRILLKKNRHRRAGHGAKNKLKPIAVLAEKSEGFRKKLIERWACEIADFFIKNKVGTVQMENLESMKRKEDSYFNIRLRGFWPYAEMQNRIELKLKQYGIEIRRVAPNNTSRTCSKCGHLNNYFNFEYRKKNKFPHFKCEKCNFREDADYNAALNISNPKLKSTKEEP

SEQ ID NO: 2855 - protein, 726 aa, synthetic construct
SEVEFSHEYWMRHALTLAKRARDEREVPVGAVLVLNNRVIGEGWNRTTGLHDPTAHAEIMALRQGGLVMRNYRLTDATLYVTFEPCVMCAGAMIHSRIGRVVFGVRNNKRGAAGSLMNVLNYPGMNHHVEITEGILADECAALLCDFYRMPHQVLNAQKKARSCINPGGSSGGSSGSETPGTSESATPKSSGGSSGGSAKNTITKTLKLRIVRPYNSAEVEKIVADEKNNRERIALEKNKDKVKEACSEHLKVASYCTTQVERNACLFCKARKLDDKFYQKLRGQFPDAVFWQELGEIFRQLQKQAAEIYNQSLIELYYEIFIKGKGFANASSVEHYLSDVCYTRAAELFKNAAIASGLRGKVKSNFRLKELKNMKSGLPTTKSDNFPIPLVKQKGGQYTGFEISNHNDDFIIKIPFGRWQVKEEIDRYRPWEKFDFEQVRKNPKPISLLLSTQRRRGNKGWSKDEGTEAEIRKVMNGDYQTSYIEVKRGSKIGEKSAWMLNLSIDVPKIDKGVDPSIIGGIDVGVKSPLVCAINNASSRLSISDNDLFRFNKKMFARRRILLKKNGHKRAGHGAKNKLKPISILTGKSERFRKKLIERWACEIADFFIKNKVGTVQMENLESMKRREDSYFNIRLRGFWPYAEMQNKIEFKLKQYGIEIRKVAPNNTSKTCGKCGHLNNYFNFEYRKKNKFPHFKCEKCNFKENADYNAALNISNPKLKSTKEEP

SEQ ID NO: 2856 - protein, 726 aa, synthetic construct
SEVEFSHEYWMRHALTLAKRARDEREVPVGAILVLNNRVIGVGWNRAIGLHDPTAHAEIMALRQGGLVTQNYRLIDATLYVTFEPCVMCAGAMIHSRIGRVVFGVRNSKHGAAGSLVNVLNYPGMNHRVEITEGILADECAALLCDFYRMPRQVFNARKKAQSSINSGGSSGGSSGSETPGTSESATPKSSGGSSGGSAKNTITKALKLRIVRPYNSAEVEKIVADEKNNRERIALEKNKDKVKEACSKHLKVATYCTTQVERNACLFCKARKLDDKFYQKLRGQFPDAVFWQEIGEIFRQLQKQAAEIYNQSLIELYYEILIKGKGFANAGSVEHYLSGVCYTRAAELFKNAAIASGLRGKVKSNFRLKELKNMKSGLPTTKSDNFPIPLVKQKGGQYTGFEISSHNDDFIIKIPFGRWQVKKEIDKYRPWEKFDFEQVRKSPKPISLLLSTQRRKRNKGWSKDEGTEAEIRKVMNGDYQTSYIEVKRGSKTGEKSAWMLNLSIDVPKIDKGVDPSIIGGIDVGVKSPLVCAINNAFSRYSISDNDLFRFNKKMFARRRILLGKNRHKRAGHGVKNKLKPITILTEKSGRFRKKLIERWACEVADFFIKNKVGTVQMENLESMKRKEDSYFNIRLRGFWPYAEMQNRIELKLKQYGIEIRRVAPNNTSRTCSKCGHLNNYFNFEYRKKNKFPHFKCEKCNFREDADYNAALNISNPKLKSTKEEP

SEQ ID NO: 2857 - protein, 726 aa, synthetic construct
SEVEFSHEYWMRRALTLAKRARDEREVPVGAVLVLSNRVIGVGWNRAVGLHDPTAHAEIMALRQGGLVMQNYRLIEATLYVTFEPCIMCAGAMIHSRIGRVVFGVRNSKRGAAGSLMNVLNYPGMNHRVEITEGILADECAALLCDFYRMPRQVFNARKKAQSSISSGGSSGGSSGNETPGASESATPKSSSGSSAGSTKNTITKTLKLRIVRPYNSAEVEKIVADEKNNRERIALEKNKDKVKEACSKHLKVAAYCTTQVERNACLFCKARKLDDKFYQKLRGQFPDAVFWQETGEIFRQLQRQAAEIYNQSLIELYYEIFIKGKGFANASSVEHYLSDVCYTRAAELFKNAAIASGLRGKVKSNFRLKELKNMKSGLPTTKSDNFPIPLVKQKGGQYTGFEISSHNDNFIIKIPFGRWQVKKEIDKYRPWEKFDFEQVRKSPKPISLLLSTQRRKRNKGWSKDEGTEAEIRKVMSGDYQTSYIEVKRGSKTGEKSAWMLNLSIDVPKIDKGVDPSIIGGVDVGVKSPLVCAINNAFSRYSISDNDLFRFNKKMFARRRILLKKNRHKRAGHGAKNKLKPISILTGKSERFRKKLIERWACEIADFFIKNKVGTVQMENLESMKRKEDSYFNIRLRGFWPYAEMQNKIEFKLKQYGIEIRRVAPNNTSKTCSKCGHLNNYFNFEYRKKNKFPHFKCEKCNFKENADYNAALNISNPKLKSTKEEP

SEQ ID NO: 2858 - protein, 726 aa, synthetic construct
SEAEFSHEYWMRHALTLAERARDEREVPVGAILVLNNRVIGEGWNRAIGLHDPTAHAEIMALRQGGLVTQNYRLTDATLYATFEPCVMCAGAMIHSRIGRVVFGVRNSKRGAAGSLMNVLNYPGMNHCVEITGGILADECAALLCDFYRMPRQVFNAQKKAQSNINPGGSSGGSSDSETPGTSENATPGSSGGSSGGSAKNTITKTLKLRIVRPYNSAEVEKIVADEKNNREKIALEKNKDKVKEACSKHLKVASYCTTQVERNACLFCKARKLDDKFYQKLRGQFPDAVFWQELGEIFRQLQKQAAEIYNQSLIELYYEIFIKGKGFANASSVEHYLSDVCYTRAAELFKNAAIASGLRGKVKSNFRLKELKNMKSGLPTTKSDNFPIPLVKQKGGQYTGFEINSHNDDFIIKIPFGRWQVKKEIDKYRPWEKFDFEQVRKGPKPISLLLSTRRRKRNKGWSKDEGTEAEIRKVMNGDYQTSYIEVKRGSKIGEKSAWMLNLSIDVPKIDKGVDPSIIGGIDVGVRSPLVCAINNAFSRYSISDNDLFHFNKKVFARRRILLKKNRHKRAGHGAKNKLKPISILTEKSKRFRKKLIEKWACEIADFFIKNKVGTVQMENLESIKRKEDSYFNIRLRGFWPYAEMQSKIEFKLKQYGIKIRKVAPNNTSKTCSKCGHLNNYFNFEYRKKNKFPHFKCEKCSFKENADYNAALNISNPKLKSTKEEP

SEQ ID NO: 2859 - protein, 726 aa, synthetic construct
SEVEFSHEYWMRHALTLAKRARDEREVPVGAILVLNNRVIGEGWNRAIGLHDPTAHAEIMALRQGGLVMQNYRLIDATLYVTFEPCVMCAGAMVHSRIGRVVFGVRNSKRGAAGSLMNVLNYPGMNHCIEITEGILVDECAALLCDFYRMPRQVLSAQKKAQSSISSGGSSGGSSGSETPGASGSVTPKSSVGSSAGSTKNTITKTLKLRIVRPYNSAEVEKIVADEKNNREKIALEKNKDKVKEACSEHLKVAAYCTTQVERNACLFCKARKLDDKFYQKLRGQFPDAVFWQEIGEIFRQLQKQAAEIYNQSLIELYYEIFIKGKGFANASSVEHYLSDVCYTRAAELFKNAAIASGLRGKVKSNFRLKELKNMKSGLPTTKGDNFPIPLVKQKGGQYTGFEISSHNDDFIIKIPFGRWQVKKEIDKYRPWEKFDFEQVRKSPKPISLLLSTQRRKRNKGWSKDEGTEAEIRKVMNGDYQTSYIEVKRGRKIGEKSAWMLNLSIDVPKIDKGVDPSTIGGIDVGVKSPLVCAINNALSRYSISDNDLFRFNKKMFARRRILLKKNRHKRAGHGAKNKLKPITIMTEKSKRFRKKLIERWACEIADFFIKNKVGTVQMEDLESMKRKEDSYFNIRLRGFWPYAEMQNKIEFKLKQYGIEIRKVAPNNTSKTCSRCGHLNNYFNFEYRKKNKSPHFKCEKCNFKEDADYNAALNISNPKLKSTKEEP

SEQ ID NO: 2860 - protein, 726 aa, synthetic construct
SEVEFSHEYWMRHALTLAKRARDEREVPVGAVLVLNNRVIGEGWNRAIGLHDPTAHAEIMALRQGGLVLQNYRLVDATLYVTFEPCVLCAGAMVHSRIGRVVFGARNSKRGAAGSLMNILNYPGMNHRVEITEGILADECAALLCDFYRMPRQVFNAQKKAQSSINSGGSSGGSSGSETPSTSESATPESSGACSGGSAKNTITKTLQLRIVRPYNSAEVEKIVTDEKNNREKIALEKNKDKVKEACSKHLKMASYCTTQVERNACLFCKARKLDDKFYQKLRGQFPDAVFWQELGGIFRQLQKQAAEIYNQSLIELYYEIFIKGKGITNASRVEHYLSDVCYTRAAELFKNAAIASGLRSKVRSNFRLKELKNMKSGLPTTKSDNFPIPLVKQKGGQYTGFEISSHNSDFIIKIPFGRWQVKEEIDKYRPWEKFDFEQVRKSPKPISLLLSTQRRKKNKGWSKDEGTEAEIRRVMNGDYQTSYIEVKRGSKIGEKSAWMLNLSIDVPKIDKGVDPSIIGGIDVGVKSPLVCAINNAFSRYSISDNDLFRFNKKMFARRRILLKKNRHKRAGHGAKNKLKPISILTGKSERFRKKLIERWACEIADFFIKNKVGTVQMENLESMKKKEDSYFNIRLRGFWPYAEMQNRIEFKLKQYGIEIRKVAPNNTSKTCSKCGHLNNYFDFEYRKKNKFPHFKCEKCNFKENADYNAALNISNPKLRSTKEEP

SEQ ID NO: 2861 - protein, 726 aa, synthetic construct
SEVEFSHEYWMRHALTLAKRARDEREVPVGAILVLNNRVIGEGWNRAIGLHDPTAHAEIMALRQGGLVMQNYRLIDATLYVTFEPCVMCAGAMIHSRIGRVVFGVRNNKHGAAGSLVNVLNYPGMNHRVEITEGILADECAALLCDFYRMPRQVFNARKKAQSSINPGGSSGGSSGSETPGTSESATPESSGGSSGSSAKNTITKTLKLRIVRPYNSAEVEKIVADEKNNREKTALEKNKGKVKEACSKHLKVATYCTTQVERNACLFCKARRLDDEFYQKLRGQFPDAVFWQELGGIFRQLQKQAAEIYNQSLIELYYEIFIKGKGITNASRVEHYLSDVCYTRAAELFKNAAIASGLRSKVRSNFRLKELKNMKSGLPTTKSDNFPIPLVKQKGGQYTGFEISSHNSDFIIKIPFGRWRVKEEIDKYRPWEKFDFEQVRKSPKPISLLLSTQRRKKNKGWSKDESTEAEIRRVMNGDYQTSYIEVKRGSKIGEKSAWMLNLSIDVPKIDKGVDPSIIGGIDVGVKSPLVCAINNAFSRYSISDNDLFHFNKKMFARRRILLKKNGHKRAGHGAKNKLKPITILTEKSVRFRKKLIERWACEIADFFVKNKVGTVQMENLESMKRKEDSYFNIRLRGFWPYAEMQNKIEFKLKQYGIEIRKVAPNNTSKTCSKCGHLNSYFNFEYRKKNKFPHFKCEKCNFKENADYNAALNISNPKLKSTKEEH

SEQ ID NO: 2862 - protein, 726 aa, synthetic construct
SEVEFSHEYWMRHALTLAKRARDEREVPVGAILVLNNRVIGEGWNRTTGLHDPTAHAEIMALRQGGLVMQNHRLVDATLYVTFEPCVMCAGAMIHSRIGRVVFGVRNSKRGAAGSLTNVLSYPGMNHRVEITEGILADECAALLCDFYRMPRRVFNAQKKAQSSINSGGSSGGGSGSETPGTSESATPESSGGSSGSSAKNTITKTLKLRIVRPYNSAEVEKIVADEKNNREKTALEKNKDKVKEACSKHLKVAAYCTTQVERNACLFCKARKLDDKFYQKLRGQFPDAVFWQEVGEIFRQLQKQAAEIYNQSLIELYYEIFIKGKGFANASSVEHYLSDVCYTRAAELFKNAAIASGLRGKVKSNFRLKELKNMKSGLPTTKSDNFPIPLVKQKGGQYTGFEISSHNDDFIIKIPFGRWQVKKEIDKYRPWEKFDFEQVRKSPKPISLLLSTQRRKRNKGWSKDEGTEAEIRRVMNGDYQTSYIEVKRGSKIDEKSAWMLNLSIDVPKIDKGVDPSIIGGIDVGVRSPLVCAINNAFSRYSISDNDLFRFNKKMFARRRILLKKNRHKRAGHGAKNKLKPITILTEKSRRFRKKLIERWACEIADFFIKNKVGTVQMESLESMKRKEDSYFNIRLRGFWPYAEMQNKIEFKLKQYGIKIRKVAPNNTSKTCSMCGHLNNYFNFEYRKKNKFPHFKCVKCNFKENADYNAALNICNPKLKSTKEEP

SEQ ID NO: 2863 - protein, 726 aa, synthetic construct
SEVEFSHEYWMRHALTLAKRARDEREVPVGAVLVLNNRAIGEGWNRAIGLHDPTAHAEIMALHQGGLVMQNYRLIDATLYVTFEPCVMCAGAMIHSRIGRVVFGARNSKRGAAGSLMNVLSYPGMNHRVEITEGILADECAALLCDFYRMPRRVFNAQKKAQSSINSGGSSGGGSGSETPSTSENTTPESSGGSSGGPAKNTITKTLKLRIVRPYNSAEVEKIVADEKNSREKIALEKNKDKVKEACGKHLKVASYCTTQVERNACLFCKARKLDDKFYQKLRGQFPDAVFWQELGEIFRQLQKQAAEIYNQSLIELYYEIFIKGKGLANASSVEHYLSDVCYTRAAELFKNAAIASGLRGKVKSNFKLKELKSMKSGLPSTKSDNFPIPLVKQKGGQYTGFEISSHNDDLIIKIPFGRWQVKKEIDKYRPWEKFDFEQVRKSPKPISLLLSTQRRKRNKGWSKDEGTEAEIRKVMNGDYQTSYIEVKRGSKAGEKSAWMLNLSIDVPKIGKGVDPSIIGGIDVGVKSPLVCAINNAFSRYSISDNDLFRFNKKMFARRRILLKKNRHKRAGHGAKNKLKPVSILTEKSERFRKKLIERWACEIADFFIKNKVGTVQMENLESMKRREDSYFNIRLRGFWPYAKMQNKIEFKLKQYGIEIRKVAPNNTSKTCSKCGHLNNYFDFEYRKKNKFPHFKCEKCNFKESADYNAALNISNPKLKSTKEEP

SEQ ID NO: 2864 - protein, 726 aa, synthetic construct
GEVEFSHEYWMRRALTLAKRARDEREVPVGAVLVLNNRVIGEGWNRAIGLHDPAAHAEIMALRQGGLVMQNYRLIGATLYVTFEPCVMCAGAMIHSRVGRVVFGVRNNKHGAAGSLVNVLNYPGMNHRVEITEGILADECAALLCDFYRMPRQVFNARKKAQSSINPGSSSGGSGGSETPGTSESATPESSGGSSGSSAKNTITKTLKLRIVRPYNSAEVEKIVADEKNNREKIALEKNKDKVKEACSKHLKVAAYCTTQVERNACLFCKARKLDDKFYQKLRGQFPDAVFWQEIGEIFRQLQKQAAEIYNQSLIELYYEIFIKGKGFANTSSVEHYLSDVCYTRAAELFKNAAIASGLRGKVKSNFRLKELKNMKSGLPTTKGDNFPIPLVKQKGGQYTGFEISSHNDDFIIKIPFGRWQVKKEIDKYRPWEKFDFEQVRKSPRPISLLLSTQRRKRNKGWSKDEGTEAEIRKVMNGDYQTSYIEVKRGRKIGEKSVWMLNLSIDVPKIDKGVDPSTIGGIDVGVKSPLVCAINNALSRYSISDNDLFRFNKKMFARRRILLKKNRHKRAGHGAKNKLKPITILTEKSGRFRKKLIERWACEIADFFIKNKVGTVQMENLESMKRKEDNYFNIRLRGFWPYAEMQNKIELKLKQYGIKIRKVAPNNTSKTCSKCGHLNDYFNFEYRKKNKFPHFKCEECNFKEDADYNAALNISNPKLKSTREEP

SEQ ID NO: 2865 - protein, 726 aa, synthetic construct
SEDEFSHEYWMRHALTLAKRARDEREVPVGAILVLNNRVIGEGWNRAIGLHDPTAHAEIMALRQGGLVMQNYRLIDATLYVTFEPCVMCAGAMIHSRIGRVVFGVRNSKHGAAGSLMNVLNYPGMNHRVEITEGILADECAALLCDFYRMPHQVFSARKKAQSSINPGGSSGGSSGSKTPGTSESATPESSGGSSGGSAKNSITKTLKLRIVRPYNSAEVEKIVADEKNNREKIALEKNKGKVKEACSKHLKVATYCTTQVERNACLFCKARKLDDKFYQKLRGQFPDAVFWQEIGEIFRQLQKQAAEIYNQSLIELYYEIFIKGKGITNASRVEHYLSDVCYTRAAELFKNAAIASGLRSKVRSNFRLKELKNMKSGLPTTKSDNFPIPLVKQKGGQYTGFEISSHNDDLIIKIPFGRWQVKREIDKYRPWEKFDFEQVRKGPKPISLLLSTQRRKRNKGWSKDEGTEAEIRKVMNGDYQTSYIEVKRGSKIGEKSAWMLNLSIDVPKIDKGVDPSVIGGIDVGVKSPLVCAINNAFSRYSISDNDLFHFNKKMFARRRILLKKSRHKRAGHGAKNKLKPISILTEKSERFRKKLIERWACEIANFFIKNKVGTVQMENLEGMKRKEDSYFNIRLRGFWPYAEMQNKIEFKLKQYGIVIRKVAPNNTSKTCSKCGHLNNYFNFEYRKKNKFPHFKCEKCNFKENADYNAALNISNPKLKSTKEEP

SEQ ID NO: 2866 - protein, 725 aa, synthetic construct
SEVEFSHEYWMRHALTLAKRARDEREVPVGAVLVLNNRVIGEGWNRAIGLHDPTAHAEIMALRQGGLVMQNYRLTDATLYVTFEPCVMCAGAMIHSRIGRVVFGVRNSKRGAAGSLMNVLNYPGMNHCVEITEGILMDECAALLCDFYRMPRQVLNAQKKAQSSISSGGPSGGSSCSETPGASESVTPKSSGGSSTGSTKNTITKTLKLRIVRPYNSAEVEKIVADEKNSREKIALEKNKDKVKEACSKHLKVAAYCTTQVERNACLFCKARRLDDKFYQKLRGQFPDAVFWQEIGEIFRQLQKQAAEIYNQSLIELYYEIFIKGKGIAGASRVGHYLSDVCYTRAAELFKNAAIASGLRSKIKSNFRLKELKNMKSGLPTTKSDNFPIPLVKQKGGQYTGFEISSHNDDFIIKIPFGRWVKKEIDKYRPWEKFDFEQVRKSPKPISLLLSTQRRKRNKGWSKDEGTEAEIRKVMNGDYQTSYIEVKRGSKTGEKSAWMLNLSIDVPKIDKGVDPCIIGGIDVGVKSPLVCAINDAFSRYSISDNDLFHFNKKMFARRRILLKRNRHKRAGHGAKNKLKPISILTEKSGRFRKKLIERWACEIADFFIKNKVGTVQMENLESMKRKEDSYFNIRLRGFWPYAEMQNKIEFKLKQYGIEIRKVAPNNTSKTCSKCGHLNNYFNFEYRKKNKFPHFKCEKCNFKEDADYNAALNISNPKLKSTKEEP

SEQ ID NO: 2867 - protein, 726 aa, synthetic construct
SEVEFSHEYWMRHALTLAKRARDEREVPVGAVLVLNNRVIGVGWNRTIGLHDPTAHAEIMALRQGGLVMRNYRLIDATLYVTFEPCAMCAGAMIHSRIGRVVFGVRNSKRGAAGSLMNVLDYPGMNHCVEITEGILVDECAALLCDFYRMPRQVLNAQKKAQSSISSGGSSGGSSGSETPGASESATPKSSVGSSAGSTKNTITKTLKLRIVRPYNSAEVEKIVADEKNSREKIALEKNKDKVKEACSEHLKVAAYCTTQVERNACLFCKARKLDDRFYQKLRGQFPDAVFWQEIGEIFRQLQKQAAEIYNQSLIELYYEIFIKGKGFANASSVEHYLSDVCYTRAAGLFKNAAIASGLRGKVKSNFRLKELKNMKSGLPTTKSDNFPIPLVKQKGGQYTGFEISNHNSDFIIKIPFGRWQVKKEINKYRPWEKFDFEQVRKSPKPISLLLSTQRRKRNKGWSKDEGTEAEIRKVMNGDYQTSYIEVKRGSRIGEKSAWMLSLSIDVPKIDRGVDPSIIGGIDVGVKSPLVCAINNALSRYSISDNDLFRFNKKMFARRRILLKKNRHKRAGHGAKNKLKPISILTGKGERFRKKLIERWACEIADFFVKNKVGTVQMENLESMKRKEDSYFNIRLRGFWPYAEMQNKIEYKLKQYGIKVRKVAPNNTSKTCSKCGHLNNYFSFEYRKKNKFLHFKCEKCNFKENADYNAALNISNPKLKSTKEEP

SEQ ID NO: 2868 - protein, 726 aa, synthetic construct
SEVEFSHEYWMRHALTLAKRARDEREVPVGAILVLNNRVIGEGWNRAIGLHDPTAHAEIMALRQGGLVMQNYRLIDATLYVTFEPCVMCAGAMVHSRIGRVVFGVRNSKRGAAGSLMNVLDYPGMGHRVEITEGILADECAALLCDFYCMPRQVFNAQKRAQSSINSGGSSGGSSGSETPGTSGSVTPKSSGGSSAGSTKDTITKTLKLRIVRPYNSAEVEKIVADEKNNREKIALEKNKDKVKEACSKHLKVAAYCTTQVERNACLFCRARKLDDKFYQKLRGQFPDAVFWQEIGEIFRQLQKQAAEIYNQSLIELYYEIFIKGKGFANASSVEHYLSDVCYTRAAELFKNAAIASGLRGKVKSNFRLKELKNMKSGLPTTKSDNFPIPLVKQKGGQYTGFEISSHNGDFIIKIPFGMWQVKKEINKHRPWEKFDFEQVRKSPKPISLLLSTQRRKSNRGWSKDEGTEAEVKKVMNGDYQISYIEVKRGSKIGEKSAWMLNLSIDVPKIDKGVDPSIIGGIDVGVKSPLVCAISNAFGRYSISDNDLFHFNKKMFAMRRILLKKNRHKRAGHGAKNKLKPITILTEKSKRFRKKLIERWACEIADFFIKNKVGTVQMENLESMKRKEDSYFNIRLRGFWPYAEMQDKIEFKLKQYGIEIRKVAPNNTSKTCSRCGHLNNYFNFEYRRKNKFPHFKCEKCNFKENADYNAALNISNPKLKSTKEEP

SEQ ID NO: 2869 - protein, 726 aa, synthetic construct
SEVEFSHEYWMRHALTLAKRARDEREVPVGAVLVLNNRVIGEGWNRAIGLHDPTAHAEIMALRQGGLVMQNYRLTDATLYVTFEPCVMCAGAMIHSRIGRVVFGIRNSKRGAAGSLMNVLNYPGMNHRVEITEGILADECAALLCDYYRMPRQVFNARKKAQSSINSGGSSDGGSGSETPGASESVTPKSSVGSSAGSTKNTITKTLKLRIVRPYNSAEVEKIVADEKNNREKIALEKNKDKVKEACSKHLKVAAYCTTQVERNACLFCKARRLDDKFYQKLRGQFPDAVFWQEIGEIFRQLQKQAAEIYNQSLIELYYEIFIKGKGITNASRVEHYLSDVCYTRAAELFKNAAIASGLRSKVRSNFRLKELKNMKSGLPTTKSDNFPIPLVKQKGGQYTGFEISSHNSDFIIKIPFGRWQEKEEIGKYRPWEKFDFEQVRRSPKPISLLLSTQRRKKNKGWSKDEGTEAEIRRVMNGDYQTSYIEVKRGSKIGEKSAWMLNLSIDVPKIDKGVDPSIIGGIDVGVKSPLVCAINNAFSRYSISDNDLFHFNKKMFARRRILLKKNRRRRAGHGAKNKLKPITILTEKSVRFRKKLIERWACEIADFFIKNKVGTVQMENLESMKRKEDSYFNIRLRGFWPYAEMQNKIEFKLKQYGIEIRRVAPNNTSRTCSKCGHLNNYFSFEYRKKNKFPHFRCEKCNFKENADYNAALNISNPKLKSTKEEP

SEQ ID NO: 2870 - protein, 726 aa, synthetic construct
SEDEFSHEYWMRHALTLAKRARDGREVPVGAVLVLNNRVIGEGWNRAIGLHDPTAHAEIMALRQGGLVMQSYRLIDATLYVTFEPCVMCAGAMVHSRIGRVVFGVRNSKRGAAGSLMNVLDCPGMGHRVEITEGILADECAALLCDFYCMPRQVFNAQKRAQSSISPGGSSGGSSGSETPGASESVTPKSSGGSSGGSAKNTITKTLKLRIVRPYNSAEVEKIVADEKNNREKIALEKNKGKVKEACSKHLEVAAYCTTQVERNACLFCRARKLDDKFYQKLRGQFPDAVFWQELGEIFRQLQKQAAEIYNQSLIELYYEIFIKGRGFANASSVEHYLSDVCYTRAAELFKNAAIASGLRGKVKGNFRLKELKNMKSGLPTTKSDNFPIPLVKQKGGQYTGFEISNHNSDFTIKIPFGRWQAKKEIDKYRPWEKFDFEQVRKSPKPISLLLSTQRRKRNRGWSKDESTEAEIKKVMNGDYQTSYIEVKRGSKIGEKSAWMLNLSIDVPKIDKGVDPSIIGGIDVGVKSPLVCAIDNAFSRYSISDNDLYRFNKKMFARRRILLKKNRHKRAGHGAMNKLKPITILTEKSGRFRKKLIERWACEIADFFIKNKVGTVQMENLESMKRREDSYFNIRLRGLWPYAEMQNKIEFKLKQYGIKIRKVAPNNTSKTCSKCGHLNNYFSFEYRKKNKFPHFKCEKCNFKENADYNAALNISNPKLKSTKEGP

SEQ ID NO: 2871 - protein, 726 aa, synthetic construct
SEVEFSHEYWMRHALSLAKRARDEREVPVGAVLVLNNRVIGEGWNRAIGLHDPTAHAEIMALRQGGLVLQNHRLVDATLYVTFEPCVMCAGAMIHSRIGRVVFGVRNSKRGAAGSLTNVLNYPGMNHRVEITEGILVDECAALLCDFYRMPRQVFNAQKKAQSAINSGSSSGGSSGSETPGTSESPTPESSGGSPGGSAKSTITKTLQLRIVRPYNSAEVEKIVADEKNNREKIALEKNKGKVKEACSKHLEVAAYCTTQVERNACLFCKARRLDDKFYQRLRGQFPDAVFWQEIGEIFRQLQKQTAEIYNQSLIELYYEIFIKGKGFANASSVEHYLSDVCYTRAAELFKNAAIASGLRGKVKSNFRLKELKNMKSGLPTTKSDNFPIPLVKQKGGQYTGFEISNHNSDFIIKIPFGRWQEKEEIDKYRPWEKFDFEQVRKSPKPISLLLSTQRRKRNKGWSKDEGTEAEIRRVMNGDYQTSYIEVKRGSKIGEKSAWMLNLSIDVPKIDKGVDPSIIGGIDVGVRSPLVCAINNAFSRYSISDNDLFRFNKKMFARRRILLKKNRHRRAGHGAKSKLKPISILTEKSKRFRKKLIERWACEIADFFIKNKVGTVQMENLESMKRKEDSYFNIRLRGFWPYAEMQNKIEFKLKQYGIEIRRVAPNNTSRTCSKCGHLNNYFNFEYRRKYKFPHFKCEKCNFKEDADYNAALNISNPKLKSTKEEP

SEQ ID NO: 2872 - protein, 726 aa, synthetic construct
SEDEFSHEYWMRHALTLAKRARDRREVPVGAVLVLNNRVIGEGWNRAIGLHDPTAHAEIMALRQGGLVMQNYRLTDATLYATFEPCVMCAGAMIHSRIGRVVFGVRNSKHGAAGSLMNVLNYPGMNHRVEITEGILADECAGLLCDFYRMPRQVFSARKKAQSSINPGGSSGGSSGGKAPGTSESATLESSGGSSGGSAKNSITKTLKLRIVRPYNSAEVEKIVADEKNNREKTALEKNKGKVKEACSKHLKVATYCTTQVERNACLFCKARKLDDKFYQKLRGQFPDAVFWQEIGEIFRQLQKQAAEIYNQSLIELYYEIFIKGKGFANASSAEHYLSDVCYTRAAELFKNAAIASGLRGKVKSNFRLKELKNMKSGLPTTKSDNFPIPLVKQKGGKYTGFEISSHNDDFIIKIPFGRWQVKKEIDKYRPWEKFDFEQVRKSPKPISLLLSTQRRKRNKGWSKDEGTEAEIRKVMNGDYQTSYIEVKRGSKIGEKSAWMLNLSIDVPKIDKGVDPSIIGGIDVGVKSPLVCAINNAFSRYSISDNDLFHFNKKMFARRRILLKKNRHKRAGHGVKNKLKPISILTGKSERFRKKLIERWACEIANFFIKNKVGTVQMENLEGMKRKEDSYFNIRLRGFWPYAEMQNKIEFKLKQYGIEIRKVAPNNTSKTCSKCGHLNNYFNFEYRKRNKFPHFRCEKCNFKEDADYNAALNISNPKLKSTKEEP

SEQ ID NO: 2873 - protein, 726 aa, synthetic construct
SEDEFSHEYWMRHALTLAKRARDRREVPVGAVLVLNNRVIGEGWNRAIGLHDPTAHAEIMALRQGGLAMQNYRLVDATLYVTFEPCVLCAGAMVHSRIGRVVFGVRNSKRGAAGSLMNVLNHPGMNHRVEITGGILADECAALLCDFYRMPRQVFNAQKKARSNINSGGSSGGSSGSETLGTSESATPESSGGSSGGSAKNTITKTLKLRIVRPYNSAEVEKIVADEKNNREKIALEKNKDKVKEACSEHLKVAAYCTTQVERNACLFCKARKLDDKFYQKLRGQFPDAVFWQEIGEIFRQLQKQAAEIYNQSLIELYYEIFVKGKGFANASSVEHYLSDVCYTRAAELFKNAAIASGLRGKVKSNFRLRELKSMRSGLPTTKSDNFPIPLVKQKGGQYTGFEISSHNDDFIIKIPFGRWQVKKEIDRYRPWEKFDFEQVRKSPKPISLLLSTQRRKRNKGWSKDEGTEAEIRRVMNGDYQTSYIEVKRGSKTGEKSAWMLNLSIDVPKIDKGVDPSIIGGIDVGVKSPLVCAINNAFSRYSISDNDLFRFNKKMFARRRILLRKNRHKRAGHGAKNKLKPISILTGKSERFRKKLIERWACEIADFFIKNKVGTVQMENLESMKRREDSYFNIRLRGFWPYAEMQNKIEFKLKQYGIEIRKVAPNNTSKTCSKCGHLNNYFSFEYRKKNKFPHFKCEKCNFKENADYNAALNISNPKLKSTKEEP

SEQ ID NO: 2874 - protein, 726 aa, synthetic construct
SEVEFSHEYWMRHALTLAKRARDEREVPVGAVLVLNNRVIGEGWNRAIGLHDPTAHAEVMALRQGGLVMQNYRLTDATLYATFEPCVMCAGAMIHSRIGRVVFGVRNSKRGAAGSLMNVLNYPGMNHCVEITEGILVDECAALLCDFYRMPRQVLNAQKKAQPSISPGGSSGGSSGSETPGASGSVTPKSSGGSSAGSTKDTITKTLKLRIVRPYNSAEVEKIVADEKNNREKIALEKNKDKVKEACSKHLKVAAYCTTQVERNACLFCRARRLDDKFYQKLRGQFPDAVFWQEIGEIFRQLQKQAAETYNQSLIELYYEIFIKGKGIANASNVEHYLSDVCYTRAAELFKNAAIASGLRNKIKSNFRLKELKNMRSGLPTTKSDNFPIPLVRQKGGQYTGFEISNHNGDFIIKIPFGRWQVKKEIDKRRPWEKFDFEQVRKSPKPISLLLSTQRRKRNKGWSKDEGTEAEIRKVMNGDYQTSYIEVKRGGKIGEKSAWMLNLSIDVPKIDKGVDPSIIGGIDVGVKSPLVCAINNAFSRYSISDNDLFHFNKKMFARRRILLGKNRHKRAGHGVKNKLKPITILTEKSGRFRKKLIERWACEIADFFVKNKVGTVQMENLESMKRKEDSYFNIRLRGFWPYAEMQNKIEFKLKQYGIKIRKVAPNNTSKTCSRCGHLNNYFSFEYRKKNKFPYFKCEKCNFKENADYNAALNISNPQLKSTKGEP

SEQ ID NO: 2875 - protein, 726 aa, synthetic construct
SEVEFSHEYWMRHALTLAKRARDEREVPVGAILVLNNRVIGEGWNRAIGLHDPTAHAEIMALRQGGLVMQNYRLIGATLYVTFEPCVMCAGAMIHSRIGRVVFGVRNNKHGAAGSLVNVLNYPGMNHRVEITEGILADECAALLCDFYRMPRQVFNARKKAQSSTNPGGSSGDSSGSETPGTSESATPESSGGGSGGSAKSTITKTLQLRIVRPYNSAEVEKIVADEKNNREKIALEKNKDKVKEACSKHLKVASYCTTQVERNACPFCKARKLDDKFYQKLRGQFPDAVFWQEIGEIFRQLQKQAAEIYNQSLIELYYEIFIKGKGFANASSVEHYLSDVCYTRAAELFKNAAIASGLRGKVKSNLRLKELKNMKSGLPTTKSDNFPIPLVKQKGGQYTGFEISSHNDDFIIKIPFGRWQVKKEIDKYRPWEKFDFERVRKSPKPISLLLSTQRRKRNKGWGKDEGTEAEIRKVMNGDYQTSYIEVKRGSRIGEKSAWMLSLSIDVPKIDRGVDPSIIGGIDVGVKSPLVCAINNALSRYSISDNDLFHFNKKMFARRRILLKKNRHRRAGHGARNKLKPITVLTEKSKRFRKKLIERWACEIANFFIKNKVGTVQMENLESMKRKEDSYFNIRLRGLWPYAEMQNKIEFKLKQYGIEIRKVAPNNTSKTCSKCGHLNNYFNFEYRKRNKFPHFKCEKCNFKEDADYNAALNISNPKLKSTKGEP

SEQ ID NO: 2876 - protein, 726 aa, synthetic construct
SEVEFSHEYWMRHALTLAKRARDEREVPVGAILVLNNRVIGEGWNRAIGLHDPTAHAEIMALRQGGLVMQNYRLIDATLYVTFEPCVMCAGAMIHSRIGRVVFGVRNNKHGAAGSLVNVLNYPGMNHRVEITEGILADECAALLCDFYRMPRQVFNARKKAQSSINPGGSSGGSSGSETPGTSESATPESPGGSSGGSAKNTITKTLQLRIVRPYNSAEVEKIVADEKNNREKIALEKNKGKVREACSKHLKVASYCTTQVERNACPFCKARKLDDKFYQKLRGQFPDAVFWQELGEILRQLQKQAAEIYNQSLIELYYEIFIKGRGFANASNVEHYLSDVCYTRAAELFKNAAIASGLRGKVKGNFRLKELKNMKSGLPTTKSDNFPIPLVKQKGGQYTGFEISSHNDDFIIKIPFGRWQVKKEIDKYRPWEKFDFEQVRKSPKPISLLLSTQRRKRNKGWSKDEGTEAEIRKVMNGDYQTSYIEVKRGSKIGEKSAWMLSLSIDVPKIDRGVDPSIIGGIDVGVKSPLICAINNAFSRYGISDNDLFRFNKKVFARRRILLKKNRHKRAGHGTKNKLKPITILTEKSGRFRKKLIERWACEIANFFIKNKVGTVQMENLESMKRKEDSYFNIRLRGFWPYAEMQNKIEFKLKQYGIKIRKVAPNNTSKTCSKCGHLNNYFSFEYRKKNKFPHFKCEKCNFKENADYNAALNICNPKLKSTKEEP

SEQ ID NO: 2877 - protein, 726 aa, synthetic construct
SEVEFSHEYWMRHALTLAKRARDEREVPVGAVLVLNNRVIGVGWNRAIGLHDPSAHAEIMALRQGGLVMQNYRLTDATLYVTFEPCVMCAGAMVHSRIGRVVFGVRNSKRGAAGSLMNVLNYPGMSHCVEITEGILVDECAALLCDFYRMPRQVLNAQKKAQSSISSGGSSGGSGGGETPGASESVTPKSSGGSSAGSTKNTITKTLKLRIVRPYNSAEVEKIVADEKNSREKIALEKNKGKVKEACSKHLKVATYCTTQVERNACLFCKARKLDDKFYQKLRGQFPDAVFWQEIGEIFRQLQKQAAEIYNQSLIELYYEIFIKGKGFANASSVEHYLSDVCYTRAAELFKNAAIASGLRGKVKSSFRLKELKNMKSGLPTTKSDNFPIPLVKQKGGQYTGFEISSHNDDFIIKIPFGRWQVKKEIDKYRPWEKFDFEQVRKSPKPISLLLSTQRRKRNKGWSKDEGTEAEIRKVMNGDYLTSYIEVKRGSKTGEKSAWMLNLSIDVPKIDKGVDPSIIGGIDVGVKSPLVCAISNAFSRYSISDNDLFHFNKKMFARRRILLKKNRHKRAGHGAKNKLKPISILTEKSKRFRKKLIERWACEIADFFIKNKVGTVQMENLESMKRKEDSYFNIRLRGFWPYAEMQNKIEFKLKQYGIEIRKVAPNNTSKTCSKCGHLNNYFNFEYRRKNKFPHFKCEKCNFKEDADYNAALNISNPKLKSTKEEP

SEQ ID NO: 2878 - protein, 726 aa, synthetic construct
SEVEFSHEYWMRHALSLAKRARDEREVPVGAVLVLNNRIIGEGWNRAIGLHDPTAHAEIMALRQGGLVMQNNRLTDATLYVTFEPCVMCAGAMVHSRIGRVVFGVRNSKRGAAGSLLNVLNYPGVNHCVEITEGILVDECAALLCDFYRMPRQVLNAQKKAQSSISSGGSSGGCSGSEMPSASESVTPKSSGGSSAGSTKNTITKTLKLRIVRPYNSAEVEKIVADEKNSREKIALERNKDKVKEACSEHLKVAAYCTTQVERSACLFCKARKLDDKFYQKLRGQFPDAVFWQEIGEIFRQLQKQAAEIYNQSLIELYYEIFIKGKGFANASSVEHYLSDVCYTRAAELFKNAAIASGLRGKVKSNFRLKELKNMKSGLPTTKSDNFPIPLVKQKGGQYTGFEISSHNDDFIIKIPFGRWQVKKEIDKYRPWEKFDFEQVRKSPKPISLLLSTQRRRRNKGWSRDEGTEAEIKKVMNGDYQASYIEVKRGSKIGEKSAWMLNLSIDVPKIDRGVDPSIIGGIDVGVKSPLVCAINNAFSRYSISDNDLFHFNKKVFARRRILLKKNRHKRAGHGAKNKLKPITILTEKSKRFRKKLIERWACEIANFFIKNKVGTVQMENLESMKRKEDSYFNIRLRGFWPYAEMQNKIEFKLKQYGIEIRKVAPNNTSRTCSRCGHLNNYFNFEYRKKNKFPHFKCEKCNFKEDADYNAALNISNPKLKGTKEEP

SEQ ID NO: 2879 - protein, 726 aa, synthetic construct
SEDEFSHEYWMRHALTLAKRARDGREVPVGAVLVLNNRVIGEGWNRAIGLHDPTAHAEIMALRQGGLVMQNYRLIDATLYVTFEPCVMCAGAMVHSRIGRVVFGVRNSKRGAAGSLMNVLDHPGMGHRVEITEGILADECATLLCDFYCMPRQVFNAQKRAQSSINSGGSSGGGSGSETPSTSESTTPESSGGSSGGPAKNTITKTLKLRIVRPYNSAEVEKIVADEKNNREKTALEKNKDKVKEACSKHLKVAAYCTTQVERNACLFCKARKLDDKFYQKLRGQFPDAVFWQEVGEIFRQLQKQAAEIYNQSLIELYYEIFIKGRGFANASSVEHYLSDVCYTRAAELFKNAAIASGLRGKVKSNFRLKELKNMKSGLPTTKSDNFPIPLVKQKGGQYTGFEISNHNSDFIIKIPFGRWQVKKEINKYRPWEKFDFEQVRKSPKPISLLLSTQRRKRNKGWSKDEGTEAEIRKVMNGDYQTSYIEVKRGSRIGEKSAWMLSLSIDVPKIDRGVDPSIIGGIDVGVKSPLVCAINNALSRYSISDNDLFHFNKKMFARRRILLKKNRHRRAGHGARNKLKPVTVLTEKSKRFRKKLIERWACEIANFFIKNKVGTVQMENLESMKRKEDSYFNIRLRGLWPYAEMQNKIEFKLKQYGIEIRKVAPNNTSKTCSKCGHLNNYFNFEYRKRNKFPHFKCEKCNFKENADYNAALNISNPKLKGTKEEP

SEQ ID NO: 2880 - protein, 726 aa, synthetic construct
SEDEFSHEYWMRHALTLAKRARDGREVPVGAVLVLNNRVIGEGWNRAIGLHDPTAHAEIMALRQGGLVMQNYRLIDATLYVTFEPCVMCAGAMVHSRIGRVVFGVRNSKRGAAGSLVNVLNYPGMNHRVEITEGILADECAALLCDFYRMPRQVFNARKKAQSSINSGGSSGGSSGSETPGTSESATPESSGGGSSGSAKNTITKTLQLRIVRPYNSAEVEKIVADEKNNREKIALEKNKDKVKEACSKHLKMASYCTTQVERNACPFCKARKLDDKFYQKLRGQFPDAVFWQELGEILRQLQKQAAEIYNQSLIELYYEIFIKGRGFANASSVEHYLSDVCYTRAAGLFKNAAIASGLRGKVKSNFRLKELKNMKSGLPTTKSDNFPIPLVKQKGGQYAGFEISSHNDDFIIKIPFGRWQVKKEIDKYRPWEKFDFEQVRKSPKPISLLLSTQRRKRNKGWSKDEGTEAEIRKVMNGDYQTSYIEVKRGSKTGEKSAWMLNLSIDVPKIDKGVDPSIIGGIDVGVKSPLVCAINNAFSRYSISDNDLFRFNKKMFARRRILLKKTRHKRAGHGAKNKLKPISILTEKSERFRKKLIERWACEIADFFVKNKVGTVQMENLESMKRREDSYFNIRLRGFWPYAKMQNKIEFKLKQYGIEIRKVAPNNTSKTCSKCGHLNNYFNFEYRKKNKFPHFKCEKCNFKENADYNAALNISSPKLKSTKEEP

SEQ ID NO: 2881 - protein, 726 aa, synthetic construct; identical to SEQ ID NO: 2809

SEQ ID NO: 2882 - protein, 726 aa, synthetic construct
SEDEFSHEYWMRHALTLAKRARDRREVPVGAVLVLNNRVIGEGWNRAIGLHDPTAHAEIMALRQGGLVMQNYRLIDATLYVTFEPCVMCAGAMIHSRIGRVVFGVRNNKHGAAGSLVNVLNYPGMNHRVEITEGILAGECAALLCDFYRMPRRVLNAQKKAQSNINSGGPSGGSSGSETPGTSESPTSEGSSGSSGGSARNTITKTLKLRIVRPYNSAEVEKIVADEKNNREKIALEKNKDKVKEACSKHLKVAAYCTTQVERNACLFCKARKLDDKFYQKLRGQFPDAVFWQEIGEIFRQLQKQAAEIYNQSLIELYYEIFIKGKGFANASSVEHYLSDVCYARAAELFKNAAIASGLRGKVKSNFRLKELKNMKSGLPTTKSDNFPIPLVKQKGGQYTGFEISSHNDDFIIKIPFGRWQVKKEIDKYRPWEKFDFEQVRKSPKPISLLLSTQRRRRNKGWSKDEGTEAEIRKVMYGDYQTSYIEVKRGSKIGEKSAWMLNLSIDVPKIDKAADPSIIGGIDVGVKSPLVCAINNAFSRYSISDNDLFHFNKKVFARRRILLKKNRHRRAGHGAKNKLRPITILTEKSKRFRKKLIERWACEIADFFIKNKVGTVQMENLESMKRKEDSYFNIRLRGFWPYAEMQNKIEFKLKQYGIKIKKVAPNNTSRTCSECGHLNNYFSFEYRKKNKFPHFKCEKCNFKEDADYNAALNISNPKLKGTKEEL

SEQ ID NO: 2883 - protein, 726 aa, synthetic construct
SEVEFSHEYWMRHALTLAKRARDEREVPVGAVLVLNNRVIGEGWNRAIGLHDPTAHAEIMALRQGGLVMQNYRLVDATLYVTFEPCVLCAGAMVHSRIGRVVFGVRNSKRGAAGSLMNVLNYPGMNHRVEITEGVLADECAALLCDYYRMPRQVFNARKKAQSSINSGGLSDGGSGSETPGTSKSATPESSGGSSGGSAKNTITKTLKLRIVRPYNSAEVEKIVADEKSNREKIALEKNKDKVKEACSEHLKVAAYCTTQVERSACLFCKARKLDDKFYQRLRGQFPDAVFWQEIGEIFRQLQKQAAEIYNQSLIELYYEIFIKGKGFANASSVEHYLSDVCYTRAAELFKNAAIASGLRGKVKSNFRLKELKNMRSSLPTAKSDNFPIPLVKQKGGQYTGFEISSHNDDFIIKIPFGRWQAKKEIDRYRPWEKFDFEQVRKSPKPISLLLSTQRRKRNKGWSKDEGTEAEIRKVMNGDYQTSYIEVKRGSKIGEKSAWMLNLSIDVPKIDKGVDPSIIGGIDVGVKSPLVCAINNAFSRYSISDNDLFHFNKKMFARRRILLKKNRHRRAGHGAKNKLKPIAVLAEKSEGFRKKLIERWACEVADFFIKNKVGTVQMENLESMKRREDSYFNIRLRGFWPYAEMQNKIEFKLRQYGIEIRKVAPNNTSKTCSKCGHLNNYFNFEYRKRNKFPHFKCEKCNFKENADYNAALNISNPKLKGTKEEP

SEQ ID NO: 2884 - protein, 726 aa, synthetic construct
SEVEFSHEYWMRHALTLAKRARDRREVPVGAVLVLNNRVIGEGWNRAIGLHDPTAHAEIMALRQGGLVMQNYRLIDATLYVTFEPCVMCAGAMVHSRIGRVVFGVRNGKRGAAGSLMNVLNYPGMNHCVEITEGILVDECAALLCDFYRMSRRVLNAQKKAQSSISSGGSSGGSNGSETRGASESATPKSSGGSSAGSTKNTITKTLKLRIVRPYNSAEVEKIVTDEKNNREKIALEKNKDKVKEACSKHLKVAAYCTTQVERNACLFCKARKLDDGFYQKLRGQFPDAVFWQEIGEIFRQLQKQAAEIYNQSLIELYYEIFIKGKGFASASSVEHYLSDVCYTRAAELFKNAAIASGLRGKVKSNFRLKELKNMKSGLPTTKSDNFPIPLVKQKGGQYTGFEISSHNDDFIIKIPFGRWQVKKEIDKYRPWEKFDFEQVRKSPKPISLLLSTQRRKRNKGWSKDEGTEAEIRKVMNGDYQTSYIEVKRGSKTGEKSAWVLNLSIDVPKIDKGVDPSIIGGIDVGVKSPLVCAVNNAFSRYSISDNDLFRFNKKMFARRRILLRRNRHKRAGHGAKNKLKPISILTGKSERFRKKLIERWACEIADFFIKNKVGTVQMENLESMKRKEDSYFNIRLRGFWPYAEMQNKIEFKLKQYGIEIRKVAPNNTSKTCSKCGHLNNYFNFEFRKKNKFPHFKCEKCNFKENADYNAALNISNPKLKSTKEEP

SEQ ID NO: 2885 - protein, 726 aa, synthetic construct; identical to SEQ ID NO: 684

SEQ ID NO: 2886 - protein, 726 aa, synthetic construct
SEVEFSHEYWMRRALTLAKRARDEREVPVGAVLVLNNRVIGEGWNRAIGQHDPTAHAEIMALRQGGLVMQNYRLVDATLYVTFEPCVLCAGAMVHSRIGRVVFGVRNSKRGAAGSLMNVLNYPGMNHRVEITEGILADECAALLCDFYRMPRQVFNAQKKARSNTNSGGSSGGSSGSETPGTREGATPESSGGGSGGSAKNTITKTLKLRIVRPYNSAEVEKIVTDEKNNREKIALEKNRDKVREACSEHLKVAAYCTTQVGRNACLFCKARKLDDKFYQKLRGQFPDAVFWQEISEIFRQLQKQAAEVYNQSLIELYYEIFIKGKGFANASSVEHYLSDVCYTRAAELFKNSAIASGLRGKVKSNFRLKELKSMKSGLPTTRSDNFPIPLVKQKGGRYTGFEISSHNDDFIIKIPFGRWQEKKEINKYRPWEKFDFEQVRKSPKPISLLLSTQRRKRNKGWSKDEGTEAEIRKVMNGNYQTSYIEVKRGSKIGGKSAWMLSLSIDVPKIDKGVDPSIVGGIDVGVKSPLVCAINNALSRYSISDNDLFHFNKKMFARRRILLRKNRHKRAGHGARNKLRPITVLTEKSERFRKKLIERWACEIANFFIKNKVGTVQMEDLESMKRKEDSYFNIRLRGFWPYAEMQNKIEFKLKQYGIEIRKVAPNNTSKTCSKCGHLNNYFNFEYRKKSKFPHFKCEKCNFKENADYNAALNISNPKLKSTKEEP

SEQ ID NO: 2887 - protein, 726 aa, synthetic construct
GGVEFSHEYWMRRALTLAKRARDEREVPVGAILVLNNRVIGEGWNRAISLHDPTAHAEITALRQGGLVMQNYRLIDATLYVTFEPCVMCAGAMIHSRIGRVVFGVRNSKHGAAGSLVNVLNYPGMNHRVEITEGILADECAALLCDFYRMPRQVFNARKKAQPSINPGGSSGGSGGGETPGASESVTPKSSGGSSAGSAKNTITKALKLRIVRPYNSAEVEKIVADEKNNRERIALEKNKDKVKEACSKHLKVAAYCTTQVERNACLFCKARKLDDRFYQKLRGQFPDAVFWQETGEIFRQLQRQAAEIYNQSLIELYYEIFIKGKGFANASSVEHYLSDVCYTRAAELFKNAAIASGLRGKVKSNFRLKELKNMKSGLPTTKSDNFPIPLVKQKGGQYTGFEISSHDDDFIIKIPFGRWQVKKEICKHRPWEKFDFEQVRKSPKPISLLLSTQRRKRNKGWSKDEGTEAEIRKVMNGDYQTSYIEVKRGSKTGEKSAWMLNLSIDVPKIDKGVDPSIIGGIDVGVKSPLVCAINNAFGRYSISDNDLFRFNKKMFARRRILLKKNRHKRAGHGAKNKLKPISILTGKSERFRKKLIERWACEIADFFIKNKVGTVQMENLESMKRKEDSYFNIRLRGFWPYAEMQNKIEFKLKQYGIEIRKVAPNNTSKTCSKCGHLNNYFNFEYRKKNKFPHFKCEKCNFKENADYNAALNISNPKLKSTKEKP

SEQ ID NO: 2888 - protein, 726 aa, synthetic construct
SEVEFSHEYWMRHALTLAKRARDEREVPVGAVLVLDNRVIGEGWNRAIGLHDPTAHAEIMALRQGGLVMQNYRLIDATLYVTFEPCVMCAGAMIHSRVGRVVFGVRNNKHGAAGSLVNVLNYPGMNHRVEITEGILADECAALLCDFYRMPRQVFNARKKAQSSINPGGSSGGSSGSETLGTSENATPESSGGSSGSSAKNTITKTLKLRIVRPYNSAEVEKIVADEKNNREKIALEKNKDKVKEACSKHLKVAAYCTTQVERNACLFCKARRLDDKFYQKLRGQFPDAVFWQEIGEIFRQLQKQAAEIYNQSLIELYYEIFIKGKGFANASSVEHYLSDVCYTRAAELFKNAAIASGLRGKVKSNFRLKELKNMKSGLPTTKSDNFPIPLVKQKGGQYTGFEISSHNDDFIIKIPFGRWQVRKEIDKYRPWEKFNFEQVRMSPKPISLLLSTQRRKGNKGWSKDEGTEAEIRKVMNGDYQTSYIEVKRGSKIGEKSAWMLSLSIDVPKIDKGVDPSIVGGIDVGVKSPLVCAINNVLSRYSISDNDLFHFNKKMFARRRILLKKNGHKRAGHGAKNKLKPITIMTEKSKRFRKKLIERWACEIADFFTKNKVGTVQMENLESMKGKEDSYFNIRLRGFWPYAEMQSKIEFKLKQYGIEVRKVAPNNTSKTCSKCGHLNNYFNFEYRKKSKFPHFKCEKCNFREDADYNAALNISNPKLRSTKEEP

SEQ ID NO: 2889 - protein, 726 aa, synthetic construct
SEDEFSHEYWMRHALTLAKRARDGREVPVGAVLVLNNRVIGEGWNRAIGLHDPTAHAEILALRQGGLVMQNYRLIDATLYVTFEPCAMCAGAMVHSRIGRVVFGVRNSKRGAAGSLMNVLNYPGMDHRVEITGGILADECAALLCDFYRMPRRVFNAQKKAQSSINSGGSSGGSNSSVTPGTSESATPESSGGSFGGSAKNTVTKTLQLRIVRPYNSAEVEKIVADEKNSREKIALEKNKDRVKEACGKHLKVASYCTTQVERNACLFCKARKLDDKFYQKLRGQFPDAVFWQELGEIFRQLQKQAAEIYNQSLIELYYEIFIKGKGFANASSVEHYLSDVCYTRAAELFKNAAIASGLRGKVKSNFKLRELKSMKSGLPSTKSDNFPIPLVKQKGGQYTGFEISSHNDDFIIKIPFGRWQAKKEIDKYRPWEKFDFEQVRKSPKPISLLLSTQRRKRNKGWSKDEGTEAEIRKVMNGDYQTSYIEVKRGSKIGEKSAWMLSLSIDVPKIDKGVDPRIIGGIDVGVKSPLVCAINNVLSRYSISDNDLFHFNKKMFARRRILLKKNGHKRAGHGAKNKLKPISILTEKSKRFRKKLIERWACEIADFFIKNKVGTVQMENLESMKRKEDSYFNIRLRGFWPYAEMQNKIEFKLKQYGIEIRKVAPNNTSKTCSKCGHLNNYFNFEYRKKNKFPHFKCEKCNFKENADYNAALNISNPKLKSTKEEP

SEQ ID NO: 2890 - protein, 726 aa, synthetic construct
SEVEFSHEYWMRRALTLAKRARDEREVPVGAILVLNNRVIGEGWNRAIGLHDPTAHAEITALRQGGLVMQNYRLIDATLYVTFEPCVMCAGAMIHSRIGRVVFGVRNNKHGAAGSLVNVLNYPGMNHRVEITEGVLADECAALLCDFYRMPRQVFNARKKAQSSINPGGSSGGSSGSETPGTSESATPESSGGSSGGSAKNTITKTLKLRIVRPYNSAEVERILADEKDNREKIALERNKDKVKEACSKHLKVAAYCTTQVERNACLFCRARKLDDKFYQKLRGQFPDAVFWQEIGEIFRQLQKQAAEIYNQSLIELYYEIFIKGKGFANASSVEHYLSDVCYTRAAELFKNAAIASGLRGKVKSNFRLKELKNMKSGLPTTKSDNFPIPLVKQKGGQYTGFEISSHNDDFIIKIPFGRWQVKKEIDKYRPWEKFDFEQVRKSPKPISLLLSTQRRKRNKGWSKDEGTEAEIRKVMNGDYQTSYIEVKRGSKIGEKSAWMLSLSIDVPKIDKGVDPSIIGGIDVGVKSPLVCAINNAFCRYSISDNDLFHFNKKMFARRRILLKKSRHKRAGHGARNKLKPISILTEKSKRFRKKLIERWACEIADFFIKNKVGTVQMENLESMKRKEDSYFNIRLRGFWPYAEMQNKIEFKLKQYGIETRKVAPNNTSKTCSKCGHLNNYFSFEYRKKNKFPHFKCEKCNFKEDADYNAALNISNPKLKSTKEEP

SEQ ID NO: 2891 - protein, 726 aa, synthetic construct
SEVEFSHEYWMRHALTLAKRARDEREVPVGAVLVLNNRAIGEGWNRAIGLHDPTAHAEIMALRQGGLVMQNYRLTDATLYVTFEPCVMCAGAMIHSRIGRVVFGVRNSKRGAAGSLMNVLNYPGMNHCVEITEGILVDECAALLCDFYRMPRQVLNAQKKARPNINSGGSSGGRSGSETPGTSGSATPESSGGSSGGSAKNTITKTLRLRIVRPYNSAEVEKIVADEKNNREKVALEKNRDKVKEACSEHLRVAAYCTTQVERNACLFCKARKLDDKFYQKLRGQFPDAVFWQEIGEIFRQLQKQAAAIYNQSLIELYYEIFIKGRGFANASSVEHYLSDVCYTRAAELFKNAAIASGLRGKVKSNFRLKELKNMRSGLPTAKSDNFPIPLVKQKGGQYTGFEISSHNDDFIIKIPFGRWQVKKEIDKYRPWEKFDFEQVRRSPKPISLLLSTQRRKKNKGWSKDEGTEAEIRRVMNGDYQTSYIEVKRGSKIGEKSAWMLNLTIDVPKIDKGADPSIIGGIDVGVKSPLVCAISNAFGRYSISDNDLFHFNKKMFARRRILLKKNRHKRAGHGAKNKLKPITIMTEKSKRFRKKLIERWACEIADFFIKNKVGTVQMENLESMKRREDSYFNIRLRGFWPYAEMQNKIEFKLKQYGIKVRKVAPNNTSKTCSKCGHLNNYFSFEYRKKNKFPHFKCEKCNFKEDADYNAALNISNPKLKSTKGEP

SEQ ID NO: 2892 - protein, 726 aa, synthetic construct
SEVEFSHEYWMRHALTLAKRARDEREVPVGAVLVLNNRVIGEGWNRAIGLHDPTAHAEIMALRQGGLVMQNYRLVDATLYVTFEPCVLCAGAMVHSRIGRVVFGVRNSKRGAAGSLMNVLNYPGMNHRVEITEGILADECAALLCDFYRMPRQVLNAQKKAQSSISSGGSSGGSSGSETPGASGSVTPKSSGGSFGGSAKNTITKTLKLRIVRPYNSAEVEKIVADEKNNREKIALEKNKGKVKEACSKHLEVAAYCTTQVERNVCLFCKARKLDDKFYQKLRGQFPDAVFWQELGEIFRQLQRQAAEIYNQSLIELYYEIFIKGKGFANASSVEHYLSDVCYTRAAELFKNAAIASGLRGKVKSNFRLKELKNMKSGLPTTKSVNFPIPLVKQKGGRYTGFEISSHNDDFIIKIPFGRWQVKKEIDKYRPWEKFDFEPVRKSPKPISLLLSTQRRKRNKGWSKDEGTEAEIRKVMNGDYQTSYIEVKRGSKVGEKSAWMLNLSIDVPKIDKGVDPSIVGGIDVGVKSPLVCAINNAFSRYSISDNDLFRFNKKMFARRRILLKKNRHKRAGHGAKNKLKPISILTGKSERFRKKLIERWACEIADFFIKNKVGTVQMENLESMKRKEDSYFNIRLRGLWPYAEMQNKIEFKLKQYGIEIRKVAPNNTSKTCSKCGHLNNYFNFEYRKKNKFPHFKCEKCNFKENADYNAALNISNPMLKGTKEEP

SEQ ID NO: 2893 - protein, 726 aa, synthetic construct
SEVEFSHEYWMRHALILAKRARDEREVPVGAVLVLNNRVIGEGWNRAIGLHDPTAHAEIMALRQGGLVMQNYRLIDATLYVTFEPCVMCAGAMIHSRIGRVVFGVRNNKHGAAGSLVNVLNYPGINHRVEITEGILANECAALLCDFYRMPRQVFNARKKAQSSINPGGSSGGSSGSGIPGTSESATPESSGGSSGGSAKNTITKTLKLRIVRPYNSAEVEKIVADEKNNREKIALEKNKDKVKEACSKHLKVAAYCTTQVGRNACLFCKARRLDDKFYQKLRGQFPDAVFWQEIGEIFRQLQKQAAEIYNQSLVELYYEILIKGKGIANASSVEHYLSDVCYTRAAELFKNAAIASGLRNKIKSNFRLKELRNMKSGLPTTKSDNFPIPLVRQKGGQYTGFEISNHDGDFIIKIPFGRWQVKKEINKHRPWEKFDFEQVRKSPKPISLLLSTQRRKRNKGWSKDEGTEAEIRKVMNGDYQTSYIEVKRGSKTGEKSAWMLNLSIDVPKIDKGVDPSIIGGIDVGVRSPLVCAINNAFSRYSISDNDLFRFNKKMFARRRILLRKNRHKRAGHGAKNKLKPISILTGKSERFRKKLIERWACEIADFFIKNKVGTVQMENLESMKRKEDSYFNIRLRGFWPYAEMQNKIEFKLKQYGIEIRKVAPNNTSKTCSKCGHLNNYFNFEYRKKNKFPHFKCEKCNFKENADYNAALNISNPMLKSTKEEP

SEQ ID NO: 2894 - protein, 726 aa, synthetic construct
SEVEFSHEYWMRHALTLAKRARDGREVPVGAVLVLNNRVIGEGWNRAIGLHDPTAHAEIMALRQGGLVMQNYRLTGATLYVTFEPCVMCAGAMIHSRIGRVVFGVRNSKRGAAGSLMNVLNYPGMDHCVEITEGILVDECAALLCDFYRMPRQVLNAQKKAQSSISSGGSSGGSSGSVTPGASGSVTPKSSGGGSAGSTKNTITKTLKLRIVRPYNSAEVEKIVADEKNSREKIALEKNKDKVKEACSKHLKVAAYCTTQVERNACPFCKARKLDDKFYQKLRGQFPDAVFWQELGEILRQLQKQAAEIYNQSLIELYYEIFIKGRGFANASSVEHYLSDVCYTRAAELFRNAAIASGLRGKVKSNFRLKELKNMKSGLPTTKSDNFPIPLVKQKGGQYTGFEISSHNDDFIIKIPFGRWQVKKEIDKYRPWEKFDFEQVRKSPKPISLLLSTQRRRRNKGWSKDEGTEAEIRKVMNGDYRTSYIEVKRGSKTGEKSAWMLNLSIDVPKIDKGVDPSIIGGIDVGVKSPLVCAINNAFSRYSISDNDLFRFNKKMFARRRILLKKSRHKRAGHGAKNKLKPISILTEKSKRFRKKLIERWACEIADFFIKNKVGTVQMENLESMKRKEDSYFNIRLRGFWPYAEMQNKIEFKLKQYGIVVRKVAPDNTSKTCSKCGHLNNHFNFEYRKKNKFPHFKCEKCNFKEDADYNAALNISNPKLKSTKGEP

SEQ ID NO: 2895 - protein, 726 aa, synthetic construct
SEVEFSHEYWMRHALTLAKRARDEREVPVGAVLVLNNRVIGEGWNRTTGLHDPTAHAEIMALRQGGLVMQNHRLVDATLYVTFEPCVMCAGAMIHSRIGRVVFGVRNSKRGAAGSLTNVLNYPGMNHRVEITEGILVDECAALLCDFYRMPRQVFNAQKKAQSTINSGGSSGGGSGSETPGTSESPTPKSSGGSSAGSTKNTITKTLKLRIVRPYNSAEVEKIVADEKNSREKIVLERNKDKVREACSRHLKVAAYCTTQVERNACLFCKARKLDDRFYQKLRGQFPDAVFWQEIGEIFRQLQRQAAEIYNQSLIELYYEIFIKGKGFANASSVEHYLSDVCYTRAAELFKNAAIASGLRNKVKSNFRLKELRSMKSGLPTTKSDNFPIPLVRQKGGQYTGFEISSHNDDFIIKIPFGRWQVKKEIDKYRPWEKFDFEQVRKSPKPISLLLSTQRRKKNKGWSKDEGTEAEIRRVMNGDYQTSYIEVKRGSKIGEKSAWMLNLSIDVPKIDKGVDPSIIGGIDVGVKSPLVCAINNSSSRYSICDNDLFRFNKKMFARRRILLKKSKHKRAGHGAKNKLKPITILTGKSRRFRKKLIERWACEIADFFIKNKVGTVQMENLEGMKRKEDSYFNIRLRGFWPYAEMQNKIEFKLKQYGIEIRKVAPNNTSKTCSKCGHLNNYFDFEYRKKNKFPHFKCEKCNFKENADYNAALNISNPKLKSTKEEP

SEQ ID NO: 2896 - protein, 726 aa, synthetic construct
SEVEFSHEYWMRHALTLAKRARDEREVPVGAILVLNNRVIGEGWNRAIGLHDPTAHAEIMALRQGGLVMQNYRLIDATLYVTFEPCVMCAGAMIHSRIGRVVFGVRNSKHGAAGSLVNVLNYPGMNHRVEITEGILADECAALLCDFYRMPRQVFNARKKAQSSINPSGSSGGSSGSVTPGTSESATPESSGGGFGGSAKNTITKTLKLRIVRPYNSAEVEKIVADEKDNREKIALEKNKDKVKEACSKHLKVAAYCTTQVERNACLFCKARKLDDKFYQKLRGQFPDAVFWQEIGEIFRQLQKQAAEIYNQSLIELYYEIFIKGKGFANASSVEHYLSDVCYTRAAELFKNAAIASGLRNKIKSNFRLKELRNMKSGLPTTKSDNFPIPLVRQKGGQYTGFEISNHDGDFIIKIPFGRWQVKKEINKHRPWEKFDFEQVRKSPKPISLLLSTQRRKRNKGWSKDEGTEAEIRKVMNGDYQTSYIEVKRGSKIGEKSAWMLNLSIDVPKIDKGVDPGIIGGIDVGVKSPLVCAINNASGRYSISDNDLFHFNKKMFARRRILLKKNRHKRAGHGAKSKLKPISILTEKSERFRKKLIERWACEIADFFIKNKVGTVQMENLESMKRREDSYFNIRLRGFWPYAKMLNKIEFKLKQYGIKIRKVAPNNTSKTCSKCGHLNYYFNFEYRKRNKFPHFKCEKCNFKEDADYNAALNISNPKLKSTKEEP

SEQ ID NO: 2897 - protein, 726 aa, synthetic construct
SEVEFSHEYWMRHALTLAKRARDEREVPVGAVLVLNNRVIGEGWNRAIGLHDPTAHAEIMALRQGGLVMQNYRLVDATLYVTFEPCVLCAGAMVHSRIGRVVFGVRNSKRGAAGSLMNVLNYPGMNHRVEITEGVLADECAALLCDFYRMPRQVFNAQKKARSNINSGGSSGGSSGSETPGTSESATPESSGGSSGGSAKNTITKTLKLRIVRPYNSAEVEKIVADEKNNREKIALEENKDKVKEACSEHLKVTAYCTTQVEKNACLFCKARKLDDKFYQKLRGQFPDAVFWQELGGIFRQLQKQAAEIYNQSLIELYYEIFIKGKGITNASRVEHYLSDVCYTRAAELFKNAAIASGLRSKVRSNFRLKELKNMKSGLPTTKSDNFPIPLVKQKGGQYTGFEISSHNSDFIIKIPFGRWQEKEEIDKYRPWEKFDFEQVRKSPKPISLLLSTQRRKKNKGWSKDEGTEAEIRRVMNGDYQTSYIEVKRGSKIGEKSAWMLNLSIDVPKIDKGVDPSIIGGIDVGVKSPLVCAINNAFSRYSISDNDLFHFNKKMFARRRVLLKKNRHRRAGHGARNKLKPITILTEKSERFRKKLIERWACEIANFFIKNKVGTVQMENLEGMKRKEDSYFNIRLRGFWPYAEMQNKIEFKLKQYGIEIRKVAPNNTSKTCSRCGHLNNYFNFEYRRKNKFPHFKCEKCNFKENADYNAALNISNPKLKSTKEEP

SEQ ID NO: 2898 - protein, 726 aa, synthetic construct
SEVEFSHEYWMRHALTLAKRARDEREVPVGAVLVLNNRVIGEGWNRAIGLHDPTAHAEIMALRQGSLVMQNYRLTDATLYVTFEPCVMCAGAMIHSRIGRVVFGVRNNKRGAAGSLMNVLDYPGMDHRVEITGGILMDECAALLCDFYRMPRQVLNAQKKAQSSISSGGPSGGSSCSETPGASESVTPKSSGGSSTGSTKNTITKTLKLRIVRPYNSAEVEKIVADEKNSREKIALEKNKDKVKEACSEHLKVAAYCTTQVERNACLFCKARKLDDRFYQKLRGQFPDAVFWQEIGEIFRQLQKQAAEIYNQSLIELYYEIFIKGKGFAIASSVEHYLSCVCYTRAAELFKNAAIASGLRGKVKSNFRLKELKNMKSGLPTTKSDNFPIPLVKQKGGQYTGFEISSHNDDFIIKIPFGRWQVKKEIDKYRPWEKFDFEQVRKSPKPISLLLSTQRRKRNKGWSKDEGTEAEIRKVMNGDYQTSYIEVKRGSKVGEKSAWMLNLSIDVPKIDKGVDPSIIGGIDVGVRSPLVCAIDNAFSRFSISDNDLFHFNKKMFARRRILLKKNRRRRAGHGAKNKLKPITILTEKSVRFRKKLIERWACEIADFFIKNKVGTVQMENLESMKRKEDSYFNIRLRGFWPYAEMQNKIEFKLKQYGIEIRRVAPNNTSRTCSKCGHLNDYFNFEYRRKYKFPHFKCEKCNFKEDADYNAALNISNPKLKSTKEEP

SEQ ID NO: 2899 - protein, 726 aa, synthetic construct
SEVEFSHEYWMRHALTLAKRARDEREVPVGAVLVLNNRVIGEGWNRAIGLNDPTAHAEIMALRQGGLVMQNYRLIDATLYVTFEPCVMCAGAMIHSRIGRVVFGVRNNKHGAAGSLVNVLNYPGMNHRVEITEGILADECAALLCDFYRMPRQVFNARKKAQSSINPGGSSGGSGGSETPGTSESATPESSGGSSGSSAKNTITKTLKLRIVRPYNSAEVEKIVADEKNNREKIALEKNKDKVKEACSEHLKVAAYCTTQVERNACLFCKARKLDDRFYQKLRGQFPDAVFWQETGEIFRQLQRQAAEIYNQSLIELYYEIFIKGKGFANASSVEHYLSDVCYTRAAELFKNAAIASGLRGKVKSNFRLKELKNMKSGLPTTKSDNFPIPLVRQKGGQYTGFEISNHNGDFIIKIPFGRWQVKKEISKHRPWEKFDFEQVRKSPKPISLLLSTQRRKRNKGWGKDEGTEAEIRKVMNGDYRTSYIEVKRGSKTGEKSAWMLNLSIDVPKIDKGVDPSIIGGIDVGVKSPLVCAINNAFSRYSISDNDLFRFNKKVFARRRILLKKNRHKRAGHGTKNKLKPITILTEKSGRFRKKLIERWACEIADFFIKNKVGTVQMENLESMKRKEDSYFNIRLRGFWPYAEMQNRIEFKLKQYGIEIRKVAPNNTSKTCSKCGHLNNYFNFEYRKKNKFPHFKCEKCNFKEDADYNAALNISNPKLKSTKEEL

SEQ ID NO: 2900 - protein, 726 aa, synthetic construct
SEDEFSHEYWMRHALTLAKRARDGREVPVGAVLVLNNRVIGEGWNRAIGLHDPTAHAEIMALRQGGLVTQNYRLIDATLYVTFEPCVMCAGAMIHSRIGRVVFGVRNNKHGAAGSLVNVLNYPGMNHRVEITEGILADECAALLCDFYRMPRQVFNARKKAQSSISPGGSSGGSSGGETPGTSESATPESSGGSSGGSAKNTITKTLKLRIVRPYNSAEVEKIVADEKDNREKIALEKNKDKVKEACSKHLKVAAYCTTQVERNACLFCKARKLDDKFYQKLRGQFPDAVFWQEISEIFRQLQKQAAEIYNQSLIELYYEIFIKGKGFANASSVEHYLSDVCYTRAAELFKNAAIASGLRGKVKSNFRLKELKNMKSGLPTTKSDNFPIPLVKQKGGQYTGFEISNHDGDFIIKIPFGRWQVKKEINKHRPWEKFDFEQVRKNPKPISLLLSTQRRKRNKGWSKDESTEAEIRKVMNGDYQTSYIEVKRGSKIGEKGAWMLNLSIDVPKIDKGVDPSIIGGIDVGVKSPLVCAINNALSRYSISDNDLFHFNKKMFARRRILLRKNRHKRAGHGAKNKLKPISILTEKSERFRKKLIERWACEIADFFIKNKVGTVQMENLESMKRREDSYFNIRLRGFWPYAKMLNKIEFKLKQYGIKIRKVAPNNTSKTCSKCGHLNNYFNFEYRKKNKFPHFKCEKCNFKENADYNAALNISNPKLKSTKEEP

SEQ ID NO: 2901 - protein, 725 aa, synthetic construct
SEVEFSHEYWMRHALTLAKRARVEREVPVGAVLVLNNRVIGEGWNRAIGLHDPTAHAEIVALRQGGLVMQNYRLTDATLYVTFEPCVMCAGAMIHSRIGRVVFGVRNSKRGAAGSLMNVLNYPGMNHCVEITEGILVDECAALLCDFYRMPRQVLNAQKKAQSSISSGGSSGGSGGSEPPGASESVTPKSSAGSSAGSTKNTITKTLKLRVVRPYNSAEVEKIVADEKNNREKIALEKNKDKVKEACSKHLKVAAYCTTQVERNACLFCKARKLDDKFYQKLRGQFPDAVFWQEISEIFRQLQKQAAEIYNQSLIELYYEIFIKGKGFANASSVEHYLSDVCYTRAAELFKNAAIASGLRGKVKSNFRLKELKNMKSGLPTTKSDNFPIPLVKQKGGQYTGFEISSHNDDFIIKIPFGRWQMKKEIDKYRPWEKFDFEQVRKSPKPISLLLSTQRRKRNKGWSKDEGTEAEIKKVMNGDYQTSYIEVKRGSKIGEKSAWMLNLSIDVPKIDKGVDPNIIGGIDVGVKSPLVCAINNAFSRYSISDNDLFRFNKKMFARRRILLEKNRHKRAGHGVKNKLKPITILTEKSRRFRKKLIERWACEIADFFVKNKVGTVQMENLEGMRRKEDSYFNIRLRGFWPYAEMQNKIEFKLKQYGIKVRKVAPNNTSKTCSKCGHLNNYFSFEYRKKNKFPHFKCKKCNFENADYNAALNISNPKLKSTKEEP

SEQ ID NO: 2902 - protein, 726 aa, synthetic construct
SEVEFSHEYWMRHALMLAKRARDEREVPVGAVLVLNNRVIGEGWNRAIGLHDPTAHAEIVALRQGGLVMQNYRLVDATLYVTFEPCVLCAGAMVHSRIGRVVFGVRNSKRGAAGSLMNVLNYPGMNHRVEITEGILADECAALLCDFYRMPRQVFNAQKKARSNINSGGSSGGSSGSETLGTSESATPESSGGSPGGSAKNTITKTLKLRIVRPYNSAEVEKIVADEKNNREKIALEKNKDKVKEACSEHLKVAAYCTTQVERNACLFCKARKLDDKFYQKLRGQFPDAVFWQEISGIFRQLQKQAAEIYNQSLIELYYEIFIKGKGFANASSVEHYLSDVCYTRAAELFKNAAIASGLRGKVKSNFRLKELKSMKSGLPTTKSDNFPIPLVKQKGGQYTGFEISSHNDDFIIKIPFGRWQVKKEIDKYRPWEKFDFEQVRKSPKPISLLLSTQRRKRNKGWGKDEGTEAEIWKVMNGDYQTSYIEVKRGSKIGEKSAWMLNLSIDVPKIDKGVDPSIIGGIDVGVKSPLVCAINNAFSRYSISDNDLFRFNKKMFARRRILLRNNRHKRAGHGAKSKLKPITILTEKGERFRKKLIERWACEIANFFIKNKVGTVQMENLESMKRKEDSYFNVRLRGFWPYAEMQNKIEFKLKQYGIEIRKVAPNNTSKTCSRCGHLNNYFNFEYRKRNKFPHFKCEKCNYKEDADYNAALNISNPKLKSTKEEP

SEQ ID NO: 2903 - protein, 726 aa, synthetic construct
SEVEFSHEYWMRHALTLAKRARDEREVPVGAILVLNNRVIGVGWNRAIGLHDPTAHAEIMALRQGGLVTQNYRLIDATLYVTFEPCVMCAGAMIHSRIGRVVFGVRNSKHGAAGSLVNVLNYPGMNHRVEITEGILADECAALLCDFYRMPRQVFNARKKAQSSVNSGGSSGGSSGGDTLGASESVTPKSSGGSSAGSTKNTITKTLKLRIVRPYNSAEVEKIVADEKNSREKIALERNKDKVKEACSEHLKVAAYCTTQVERNACLFCKARKLDDRFYQKLRGQFPDAVFWQETGEIFRQLQRQAAEIYNQSLIELYYEIFIKGMGFANASSVEHYLSDVCYTRAAELFKNAAIASGLRGKVKSNFRLKELKNMKSGLPTTKSDNFPIPLVKQKGGQYTGFEISSHNDDFIIKIPFGRWQVKKEIDKYRPWEKFDFEQVRKSPKPISLLLSTQRRKRNKGWSKDEGTEAEIRKVMNGDYQTSYIEVKRGSKTGEKSAWMLNLSIDVPKIDKGVDPCIIGGIDVGVKSPLVCAINNAFSRYSISDNDLFHFNKRMFARRRILLKENGHKRAGHGAKNKLKPITIMTEKSKRFRKKLIERWACEIADFFIKNKVGTVQMENLESMKRKEDSYFNIRLRGFWPYAEMQNRIEFKLKQYGIKIRKVAPNNTSKTCSKCGHLNNYFSFEYRKKNKFPHFKCEKCNFKENADYNAALNISNPKLKSTKEGL

SEQ ID NO: 2904 - protein, 726 aa, synthetic construct
SEVEFSHEYWMRHALSLAKRARDEREVPVGAVLVLNNRIIGEGWNRAIGLHDPTAHAEIMALRQGGLVMQDYRLTDATLYVTFEPCVMCAGAMVHSRIGRVVFGVRNSKRGAAGSLMNVLNYPGVNHRVEITEGILANECAALLCDFYRMPRQVFNARKKAQSSINPGGSSGGSSGGDTLGASESVTPKSSVGSSASSTKNTITKTLKLRIVRPYNSAEVEKIVADEKDNREKIALEKNKDKVKEACSKHLKVASYCTTQVERNACPFCKARKLDDKFYQKLRGQFPDAVFWQELGEIFRQLQKQAAEIYNQSLIELYYEIFIKGKGFANASSVEHYLSDVCYTRAAELFRNAAIASGLRGKVKSNFRLKELKNMKSGLPTTRSDNFPIPLVKQKGGQYTGFEISSHNDDFIIKIPFGRWQVRKEIDKYRPWEKFDFEQVRKSPKPISLLLSTQRRKRNRGWSKDEGTEAEIKKVMNGDYQTSYIEVKRGSKTGEKSAWMLNLSIDVPKIDKGVDPSIIGGIDVGVKSPLVCAINNAFSRYSISDNDLFHFNKKMFARRRILLKKTRHKRAGHGAKNKLKPVSILTEKSERFRKKLIERWACEIADFFIKNKVGTVQMENLESMKRREDSYFNIRLRGFWPYAKMQNKIEFKLKQYGIEIRKVAPNNTSKTCSKCGHLNNYFDFEYRKKNKFPHFKCEKCNFKESADYNAALNISNPKLKSTKEEP

SEQ ID NO: 2905 - protein, 726 aa, synthetic construct
GEDEFSHEYWMRHALTLAKRARDGREVPVGAVLVLNNRVIGEGWNRAIGLHDPTAHAEIMALRQGGLVMQNYRLIDATLYVTFEPCVMCAGAMVHSRIGRVVFGVRNSKRGAAGSLMNVLDYPGMGHRVEITEGILVDECAALLCDFYRMPRQVLNAQKKAQSSISSGGSSGGCSGSKMPGASESVTPKSSGGGSSGSAKNTITKTLQLRIVRPYNSAEVEKIVADEKNNREKIALEKNKDKVKEACSKHLKVASYCTTQVERNACPFCKARKLDDKFYQKLRGQFPDAVFWQELGGILRQLQKQAAEIYNQSLIELYYEIFIKGRGFANASSVEHYLSDVCYTRAAELFKNAAIASGLRGKVKSNFRLKELKNMKSGLPTTKSDNFPIPLVKQKGGQYTGFEISSHNDDFIIKIPFGRWQVKKEIDKYRPWEKFDFEQVRKSPKPISLLLSTQRRKRNKGWSKDEGTEAEIRKVMSGDYQTSYIEVKRGSKTGEKSAWMLNLSIDVPKIDKGADPSIIGGIDVGVRSPLVCAVNNAFSRYSISDNDLFRFNKKMFARKRILLKKNRHKRAGHGAKNKLKPISILTGKSERFRKKLIERWACEIADFFIKNKVGTVQMENLESMKRKEDSYFNIRLRGFWPYAEMQNKIEFKLKQYGIEIRKVAPNNTSKTCSKCGHLNNYFNFEYRKKNKFPHFKCEKCNFKENADYNAALNISNPKLKSTKEKP

SEQ ID NO: 2906 - protein, 726 aa, synthetic construct
SEVEFSHEYWMRHALILAKRARDEREVPVGAVLVLNNRVIGVGWNRAIGLHDPTAHAEIMALRQGGLVMRNYRLIDATLYVTFEPCAMCAGAMIHSRIGSVVFGVRNSKRGAAGSLMNVLNYPGMNHRVEITEGILAGECAALLCDFYRMPRQVFNAQKKAPSTINSGGSSGGSSGSETPGTGKSPTPESPGGSSGSSAKNIITKTLKLRIVRPYNSAEVEKIVADEKNNREKIALEKNKDKVKEACSKHLKVAAYCTTQVERNACLFCKARKLDDKFYQKLRGQFPDAVFWQEIGEIFRQLQKQAAEIYNQSLIELYYEIFIKGRGFANASSVEHYLSDVCYTRAAELFKNAAIASGLRGKVKSNFRLKELKNMKSGLPTTKSDNFPIPLVKQKGGQYTGFEISSHNDDFIIKIPFGRWQAKEEIDKYRPWEKFDFEQVRKSPKPISLLLSTQRRKRNKGWSKDEGTEAEIRKVMNGDYRTSYIEVKRGSKIGEKSAWMLNLSIDVPKIDKGVDPSIIGGIDVGVKSPLVCAINNALSRYSISDNDLFHFNKKMFARRRILLKKNGHKRAGHGAKNKLKPISVLTEKSGRFRKKLIERWACEIADFFIKNKVGIVQMENLESMKRREDSYFNIRLRGFWPYAEMQNKIEFKLKQYGIGIRKVAPNNTSKTCSRCGHLNNYFNFEHRKKNKFPRFKCEKCNFKENADYNAALNISNPKLKSTKEEP

SEQ ID NO: 2907 - protein, 726 aa, synthetic construct
SEVEFSHEYWMRHALTLAKRARDEREVPVGAVLVLNNRVIGEGWNRAIGLHDPTAHAEIMALRQGGLAMQNYRLVDATLYVTFEPCVLCAGAMVHSRIGRVVFGVRNSKRGAAGSLMNVLNYPGMNHRVEITEGILADECAALLCDFYRMPRQVFNAQKKAQSSISSGGSSGGSSGSETPGASESATPKSSGGSSASSTKNTITKTLKLRIVRPYNSAEVEKIVADEKNNRERIALEKNKDKVKEACSKHLKVAAYCTTQVERNACLFCKARKLDDKFYQKLRGQFPDAVFWQETGEIFRQLQRQAAEIYNQSLIELYYEIFIKGKGFANASSVEHYLSDVCYTRAAELFKNAAIASGLRGKVKGNFRLKELKNMKSGLPTTKSDNFPIPLVKQKGGQYTGFEISSHNDGFIIKIPFGRWQAKKEIDKYRPWEKFDFEQVRKSPKPISLLLSTQRRKRNKGWSKDEGTEAEIRKVVNGVYQTSYIEVKRGSKIGEKSAWMLNLSIDVPKIDKGVDSSIIGGIDVGVKSPLVCAINNALSRYSISDNDLFHFNKKMFARRRILLRKNGHKRAGHGAKNKLKPISILTGKSERFRRKLIERWACEIADFFIKNKVGTVQMENLESMKRKEDSYFNIRLRGFWPYAEMQNKIEFKLKQYGIKIRKVAPNNTSKTCSKCGHLNNYFNFEFRKKNKFPHFKCEKCNFKEDADYNAALNISNPKLKSTKEEP

SEQ ID NO: 2908 - protein, 726 aa, synthetic construct
SEVEFSHEYWMRHALTLAKRARDKREVPVGAVLVLNNRVIGEGWNRAIGLHDPTAHAEIIALRQGGLVMQNYRLTDATLYVTFEPCVMCAGAMIHSRIGRVVFGVRNNKRGAAGSLMNVLDYPGMGHRVEITEGILAGECAALLCDFYCMPRQVFNAQKRAQSSINSGGSSGGSSGSETPGTSESATPESSVGSSAGSTKNTITKTLKLRIVRPYNSAEVEKIVADEKNNREKIALEKNKDKVKEACSKHLKVAAYCTTQVERNACLFCKARKLDDRFYQKLRGQFPDAVFWQEISEIFRQLQKQAAEIYNQSLIELYYEIFVKGKGFANASSVEHYLSDVCYTRAAELFKNAAIASGLRGKVKSNFRLKELKNMKSGLPTTKSDNFPIPLVKQKGGQYTGFEINSHNDDFIIKIPFGRWQVKKEIDKYRPWEKFDFEQVRKGPKPISLLLSTRRRKRNKGWSKDEGTEAEIKRVMNGDYQISYIEVKRGSKIGEKSAWMLSLSVDVPKIDKGVDPSIIGGIDVGVKSPLVCAINNALSRYSISDNDLFHFNKKMFARRRILLKKNRHKRAGHGAKNKLKPISILTERSERFRKKLIERWACEIADFFIKNKVGTVQMENLESMKRKEDSYFNIRLRGFWPYTEMQNKIEFKLKQYGIEIRKVAPNNTSKTCSKCGHLNSYFNFEYRKKNKFPHFKCEKCNFKENADYNAALNISNPKLKSTKEEP

SEQ ID NO: 2909 - protein, 726 aa, synthetic construct
SEVEFSHEYWMRHALTLAKRARDEREVPVGAILVLNNRVIGEGWNRAIGLHDPTAHAEIMALRQGGLVMQNHRLTDATLYVTFEPCVMCAGAMIHSRIGRVVFGVRNSKRGAAGSLMNVLNYPGMNHCVEITEGILVGECAALLCDFYRMPRQVFNARKKAQSSINPGGSSGGSSGSETPGTSGSATPESSGDSSGGSAKNTITKTLKLRIVRPYNSAEVEKIVADEKNSREKIALEKNKDKVKEACSEHLKVAAYCTTQVERNACLFCKARRLDDKFYQKLRGQFPDAVFWQEIGEIFRQLQKQAAEIYNQSLIELYYEIFIEGKGFANASSVEHYLSDVCYTRAAELFKNAAIASGLRGKVKSNFRLKELKNMKSGLPTTKSDNFPIPLVKQKGGQYTGFEISSHNDDFIIKIPFGRWQVKKEIDKYRPWEKVDFEQVRKSPKPISLLLSTQRRKRNKGWSKDEGTEAEIRKVMNGDYQTSYIEVKRGSKIGEKSAWMLNLSIDVPKIDKGVDPSIIGGIDVGVKSPLVCAINNAFSRYSIGDNDLFHYNKKMFARRRILLKKNRHKRAGHGAKNKLKPISILTEKSKRFRKKLIERWACEIADFFIKNKVGTVQMENLESMKRREDSYFNIRLRGFWPYAEMQNKIEFKLKQYGIEIRKVAPNNTSKTCSKCGHLNNYFNFEYRKKNKFPHFKCEKCNFKENADYNAALNISNPKLKSTKEEP

SEQ ID NO: 2910 - protein, 726 aa, synthetic construct
SEVEFSHEYWMRHALTLAKRARDEREVPVGAVLVLNNRVIGEGWNRAIGLHDPTAHAEIMALRQGGLVMQNYRLTDATLYVTFEPCVMCAGAMTHSRIGRVVFGVRNSKRGAAGSLMNVLNYPGMNHCVEITEGILVDECAALLCDFYRMPRQVLNAQRRAQSSINSGGSSGGSSGSETPGTSESATPESSGGGSGGSAKNTITKTLQLRIVRPYNSAEVEKIVTDEKNNREKIALEKNKDKVKEACSKHLKMASYCTTQVERNACLFCKARKLDDKFYQKLRGQFPDAVFWQELGGIFRQLQKQAAEIYNQSLIELYYEIFIKGKGITNASRVEHYLSDVCYTRAAELFKNAAIASGLRSKVRSNFRLKELKNMKSGLPTTKSDNFPIPLVKQKGGQYTGFEISSHNSDFIIKIPFGRWQVKEEIDKYRPWEKFDFEQVRKSPKPISLLLGTQRRKRNKGWSKDEGTEAEIRKVMNGDYQTSYIEVKRGSKIGEKSAWMLSLSIDVPRIDKGVDPSIIGGIDVGVKSPLVCAINNAFCRYSISDNDLFHFNKKVFARRRILLKKNRHKRAGHGTKNKLKPITILTEKSGRFRKKLIERWACEIADFFIKNKVGTVQMENLESMKRREDSYFNIRLRGFWPYAEMQNKIEFKLKQYGIEIRKVAPNNTSKTCSKCGHLNNYFNFEYRKKNKFPHFKCEKCNFKENADYNAALNISNPKLKSTKEEP

SEQ ID NO: 2911 - protein, 726 aa, synthetic construct
SEIEFSHEYWMRHALTLARRARDEREVPVGAILVLNNRVIGEGWNRAIGLHDPTAHAEIMALRQGGLVMQNYRLTDATLYVTFEPCVMCAGAMIHSRIGRVVFGVRNSKHGAAGSLVNVLNYPGMNHRVEITEGILADECAALLCDFYRMPRQVFNARKKAQSSINPGGSSGGSSGSKTPGTSESATPESSGGSSGGSAKNSITKTLKLRIVRPYNSAEVEKIVADEKNNREKIALEKNKDKVKEACSKHLKVASYCTTQVERNACPFCKARKLDDKFYQKLRGQFPDAVFWQELGEILRQLQKQAAEIYNQSLIELYYEIFIKGRGFANASSVEHYLSDVCYTRAAELFKNAAIASGLRGKVKSNFRLKELKNMKSGLPTTKSDNFPIPLVKQKGGQYTGFEISSHNDDFIIKIPFGRWQVKKEIDKYRPWEKFDFEQVRKSPKPISLLLSTQRRKRNKGWSKDEGTEAEIRKVMNGDYQTSYVEVKRGSKIGEKSAWMLNLSIDVPKIDKGVDPSIIGGIDVGVKSPLVCAINNAFSRYSISDNDLFHYNKKMFARRRILLKKNRRKRAGHGAKNKLKPITTLTEKSGRFRKKLIERWACEIANFFIKNKVGTVQMENLESMKRKEDSYFNIRLRGFWPYAEMQNKIEFKLKQYGIEIRKVAPNNTSKTCSKCGHLNNYFNFEYRRKNKFPHFKCEKCNFKENADYNAALNISSPKLKSTKEEP

SEQ ID NO: 2912 - protein, 726 aa, synthetic construct
SEVEFSHEYWMRHALTLAKRARDEREVPVGAVLVLNNRVIGEGWNRAIGLHDPTAHAEIMALRQGGLVMQNYRLTDATLYVTFEPCAMCAGAMIHSRIGRVVFGVRNSKHGAAGSLMNVLNYPGMNHCVEITEGILVDECAALLCDFYRMPRQVLNAQKKAQSSTSSGGSSGGSSGSETPGASGSVTPKSSGGSSAGLTKDTITKTLKLRIVRPYNSAEVEKIVADEKNSREKIALEKNKDKVKEACSEHLKVAAYCTTQVERNACLFCKARKLDDGFYQKLRDQFPDAVFWQEIGEIFRQLQKQAAEIYNQSLVELYYEIFIKGKGFANASSVEHYLSDVCYTRAAELFKNAAIASGLRGKVKSNFRLKELKNMKSGLPTTKSDNFPIPLVKQKGGQYTGFEISNHNSDFIIKIPFGRWQVKEEINKYRPWEKFDFEQVRKSPKPISLLLSTQRRKRNKGWSKDEGTEAEIRKVMNGDYQTSYIEVRRGSKIGERSAWMLNLSIDVPKIDKGVNPSIIGGIDVGVKSPLVCAINNAFSRYSISDNDLFRFNKKMFARRRILLGKNRHKRAGHGVKNKLKPITILTEKSGRFRKKLIERWACEIADFFVKNKVGTVQMENLESMKRKEDSYFNIRLRGFWPYAEMQNKIEFKLRQYGIKVRKVAPNNTSKTCSKCGHLNNYFSFEYRKKNKFPHFKCEKCNFKENADYNAALNISNPKLKSTKEEP

SEQ ID NO: 2913 - protein, 726 aa, synthetic construct
SEVEFSHEYWMRHALTLAKRARDEREVPVGAVLVLNNRVIGEGWNRTTGLHDPTAHAEIMALRQGGLVMQNHRLVDATLYVTFEPCVMCAGAMIHSRIGRVVFGVRNSKRGAAGSLMNVLNYPGMNHCVEITEGILVDECAALLCDFYRMPRQVLNAQKKAQSSISSGGSSGGCSGSEMPGASESVTPKSSGGSSAGSTKNTITKTLKLRIVRPYNSAEVEKIVADEKNSREKIALERNKDKVKEACSEHLKVATYCTTQVERNACLFCKARKLDDRFYQKLRGQFPDAVFWQETGEIFRQLQRQAAEIYNRSLIELYYEIFIKGKGITNASRVEHYLSDVCYTRAAELFKNAAIASGLRSKVRSNFRLKELKNMKSGLPTTKSDNFPIPLVKQKGGQYTGFEISSHNSDFIIKIPFGRWQEKEEIDKYRPWEKFDFEQVRRSPKPISLLLSTQRRKKNKGWSKDEGTEAEIRRVMNGDYQTSYIEVKRGSKIGEKSAWMLNLSIDVPKIDKGVDPSIIGGIDVGVKSPLVCAVNNAFSRYSISDNDLFHFNKKMFARRRILLKKNRRRRAGHGAKNKLKPITILTEKSVRFRKKLIERWACEIADFFIKNKVGTVQMENLEGMKRKEDSYFNIRLRGFWPYAEMQNKIEFKLKQYGIEIRKVAPNNTSRTCSKCGHLNNYFNFEYRKKNKFPHFKCERCNFREDADYNAALNISNPKLKSTKEEP

SEQ ID NO: 2914 - protein, 726 aa, synthetic construct
SEVEFSHEYWMRHALTLAKRARDEREVPVGAILVLNNRVIGVGWNRAIGLHDPTAHAEIMALRQGGLVMQNYRLIDATLYVTFEPCVMCAGAMIHSRIGRVVFGVRNSKHGAAGSLVNVLNYPGMNHRVEITEGILADECAALLCDFYRMPRQVFNARKKAQSSINSGGSSGGSSGSETPGTSESATPESSGGSSGGPAKNTITKTLKLRIVRPYNSAEVEKIVADEKNNREKIALERNKDKVKEACSKHLKVAAYCTTQVGRNACLFCKARRLDDKFYQKLRGQFPDAVFWQEIGEIFRQLQKQAAEVYNQSLVELYYEILIKGKGIANASSVEHYLSDVCYTRAAELFKNAAIASGLRNKIKSNFRLKELRNMKSGLPTTKSDNFPIPLVRQKGGQYTGFEISNHNGDFIIKIPFGRWQVKKEISKHRPWEKFDFEQVRKSPKPISLLLSTQRRKRNKGWGKDEGTEAEIRKVMNGDYQTSYIEVKRGSKIGEKSAWMLNLSIDVPKIDKGVDPSIIGGIDVGVKSPLVCAINNAFSRYSISDNDLFRFNKKVFARRRILLKKNRHKRAGHGTKNKLKPITTLTEKSGRFRKKLIERWACEIADFFIKNKVGTVQMENLESMKRKEDSYFNIRLRGFWPYAEMQNKIEFKLKRYGIEIRKVAPNNTSKTCSRCGHLNNYFNFEYRKKNKFPHFKCEKCNFKENADYNAALNISNPKLKSTKEKP

SEQ ID NO: 2915 - protein, 726 aa, synthetic construct
SEVEFSHEYWMRHALTLAKRARDEREVPVGAVLVLNNRVIGEGWNRAIGLHDPTAHAEIMALRQGGLVMQNYRLTDATLYVTFEPCVMCAGAMIHSRIGRVVFGVRNSKRGAAGSLMNVLNYPGMNHCVEITEGILVDECAALLCDFYRMPRQVLNAQKKAQSSINSGGSSGGSSGSETPGTSESATPVSSSGSSGGSAKNTITKTLKLRIVRPYNSAEVEKIVADEKNNREKIALEKNKDKVKEACSEHLKVAAYCTTQVERNACLFCKARKLDDKFYQKLRGQFPDAVSWQEIGEIFRQLQKQAAEIYNQSLIELYYEIFIKGKGFANASSVEHYLSDVCYTRAAELFKNAAIASGLRGKVKSNFRLKELKNMKSGLPTTKSDNFPIPLVKQKGGQYTGFEISSHNDDFIIKIPFGRWQVKKEIDKYRPWEKFDFEQVRKSPKPISLLLSTQRRKRNKGWSKDEGTEAEIRKVMNGDYQTSYIEVKRGSKIGEKSAWMLNLSIDVPKIDKGVDPRIIGGIDVGVKSPLVCAINNAFSRYSISDNDLFRFNKKMFARRRILLKKNRHKRAGHGAKNKLKPFTILTEKSGRFRKKLIERWACEIADFFVKNKVGTVQMENLESMKRKEDSYFNIRLRGFWPYAEMQNRIEFKLKQYGIKVRKVAPNNTSKTCSKCGHLNSYFSFEYRKKNKFPHFKCEKCNFKENADYNAALNISNPKMKSTKEEP

SEQ ID NO: 2916 - protein, 726 aa, synthetic construct
SEVEFSHEYWMRHALTLAKRARDEREVPVGAVLVLNNRVIGEGWNRAIGLHDPTAHAEIMALRQGGLVMQNYRLIDATLYVTFEPCVMCAGAMVHSRIGRVVFGVRNSKHGAAGSLVNVLNYPGMNHRVEITEGILADECAALLCDFYRMPRQVFNARKKAQSSINPSGSSGGSSGSVTPGTSESATPESSGGGFGGSAKNTITKTLQLRIVRPYNSAEVEKIVADEKNNREKIALEKNKDKVKEACSKHLKVASYCTTQVERNACLFCKARKLDDKFYQKLRGQFPDAVFWQELGEIFRQLQKQAAEIYNQSLIELYYEIFIKGKGLANASSVEHYLSDVCYTRAAELFKNAAIASGLRGKVKSNFKLKELKSMKSGLPSTKSDNFPIPLVKQRGGQYTGFEISSHNDDFIIKIPFGRWLAKKEIDKYRPWEKFDFEQVRKSPKPISLLLSTQRRKRNRGWSKDEGTEAEIRKVMNGDYQTSYVEVKRGSKIGEKSAWMLNLSIDVPKIDKGVDPSIVGGIDVGVKSPLVCAINNAFSRYSISDNDLFRFNKKMFARRRILLGKNRHKRAGHGVKNKLKPITILTEKSGRFRKKLIERWACEIADFFVKNKVGTVQMENLESMKRKEDSYFNIRLRGFWPYAEMQNRIEFKLKQYGIKVRKVAPNNTSKTCSKCGHLNNYFSFEYRKKNKFPHFKCEKCNFKENADYNAALNISNPKLKSTKEEP

SEQ ID NO: 2917 - protein, 726 aa, synthetic construct
SEVEFSHEYWMRHALTLAKRARDEREVPVGAILVLNNRVIGVGWNRAIGLHDPTAHAEIMALRQGGLVMQNYRLIDATLYVTFEPCVMCAGAMIHSRIGRVVFGVRNSKHGAAGSLVNVLNYPGMNHRVEITEGILADECAALLCDYYRMPRQVFNARKKAQSSINSGGSSDGGSGSETPGTCESVTPESSGGSSGGSAKNTITKTLKLRIVRPYNSAEVEKIVADEKNNREKIALEKNEDKVKEACSEHLKVAAYCTTQVERSACLFCKARKLDDRFYQKLRGQFPDAVFWQEIGEIFRQLQKQAAEIYNQSLIELYYEIFIKGKGFANASNVEHYLSDVCYTRAAELFKNAAIASGLRSKVRSNFRLKELKNMKSGLPTTKSDNFPIPLVKQKGGQYTGFEISSHNDDFIIKIPFGRWQVKKEIDKYRPWEKFDFEQVRKSPKPISLLLSTQRRKRNKGWSKDEGTEAEIRKVMNGDYQTSYIEVKRGSKIGEKSAWMLSLSIDVPKIDKGVDPSIIGGIDVGVKSPLVCAINNAFCRYSISDNDLFHFNKKMFARRRILLKKSRHKRAGHGAKNKLKPISILTEKSKRFRKKLIERWACEIADFFIKNKVGTVQMENLESMKRKEDSYFNIRLRGFWPYAEMQNKIEFKLKQYGIKIRKVAPNNTSKTCSKCGHLNNYFSFEYRKKNKFPHFKCEKCNFKEDADYNAALNISNPKLKSTKEEP

SEQ ID NO: 2918 - protein, 726 aa, synthetic construct
SEVEFSHEYWMRHALTLAKRARDEREVPVGAVLVLNNRVIGEGWNRTTGLHDPTAHAEIMALRQGGLVMQNHRLVDATLYVTFEPCVMCAGAMIHSRIGRVVFGVRNNKHGAAGSLVNVLNCLGMNHRVEITEGILADECAALLCDFYRMPRQVFNARKKAQSSINPGGSFGGGSGSETPGTSESATLESSGGSSGGSAKNTITKTLKLRIVRPYNSAEVERIVADEKNSREKIALEKNKDKVREACSKHLKVASYCTTQVERNACPFCKARKLDDKFYQKLRGQFPDAVFWQELGEILRQLQKQAAEIYNQSLIELYYEIFIKGRGFANASSVEHYLSDVCYTRAAELFKNAAIASGLRGKVKGNFRLKELKNMKSGLPTTKSDNFPIPLVKQKGGQYTGFEISSHNDDFIIKIPFGRWQVKKEIDKYRPWEKFDFEQVRKSPKPISLLLSTQRRRRNKGWGKDEGTEAEIRRVMNGDYQTSYIEVKRGSKTGEKSAWMLNLSIDVPKIDKGVDPSIIGGIDVGVKSPLVCAINNALSRYSISDNDLFHFNKKMFARRRILLKKNRHRRAGHGARNKLKPITVLTEKSKRFRKKLIERWACEIANFFIKNKVGTVQMENLESMKRKEDSYFNIRLRGLWPYAEMQNKIEFKLKQYGIEIRKVAPNNTSKTCSKCGHLNNYFNFEYRKRNKFPHFKCEKCNFKENADYNAALNISNPKLKGTKEEP

SEQ ID NO: 2919 - protein, 726 aa, synthetic construct
SEVEFSHEYWMRHALTLAKRARDGREVPVGAVLVLNNRVIGEGWNRAIGLHDPTAHAEIMALRQGGLVMQNYRLIDATLYVTFEPCVMCAGAMVHSRIGRVVFGVRNSKRGAAGSLMNVLDHPGMNHRVEITEGILADECAALLCDFYRMPRQVFNTRKKAQSSINPGGSSGGSSGSEMPGASESVTPKSSGGSSAGSTKNTITKTLKLRIVRPYNSAEVEKIVADEKNNREKIALEKNKDKVKEACSKHLKVAAYCTTQVERNACLFCKARKLDDKFYQKLRGQFPDAVFWQETGEIFRQLQRQAAEIYNQSLIVLYYEIFIKGKGIANASSVEHYLSDVCYTRAAELFKNAAIASGLRGKVKGNFRLKELRNMKSGLPTTKSDNFPIPLVKQKGGQYTGFEISSHNDDFIIKIPFGRWQVKKEIDKYRPWEKFDFEQVRKSPKPISLLLSTQRRKRNKGWSKDEGTEAEIRKVMNGDYQTSYIEVKRGSRIGEKSAWMLSLSIDVPKIDRGVDPSIIGGIDVGVRSPLVCAINNALSRYSISDNDLFHFNKKMFARRRILLKKNRHRRAGHGARNKLKPITVLTEKSKRFRKKLIERWACEIANFFIKNKVGTVQMENLESMKRKEDSYFNIRLRGLWPYAEMQNKIEFKLKQYGIEIRKVAPNNTSKTCSRCGHLNNYFNFEYRKRNKFPYFKCEKCNLKENADYNAALNISNPKLKGTKEEP

SEQ ID NO: 2920 - protein, 726 aa, synthetic construct
SEVEFSHEYWMRHALTLAKRARDEREVPVGAVLVLNNRVIGEGWNRAIGLHDPTAHAEIMALRQGGLVMQDYRLTDATLYVTFEPCVMCAGAMIHSRIGRVVFGVRNSKRGAAGSLMNVLNYPGMNHCVEITEGILVDECAALLCDFYRMPRQVLNAQKKAQSSISSGGSSGGSSGSETPGASGSVTPKSSGGSSAGSTKDTVTKTLKLRIVRPYNSAEVEKIVADEKNSREKIALEKNKDKVKEACSEHLKVAAYCTTQVERSACLFCKARKLDDGFYQKLRGQFPDAVFWQEIGEIFRQLQKQAAEIYNQSLIELYYEIFIKGKGFANASSVEHYLSDVCYTRAAELFKNAAIASGLRGKVKSNFKLKELKSMKSGLPSTKSDNFPIPLVKQKGGQYTGFEISSHNDDLIIKVPFGRWQVKKEIDKYRPWEKFDFEQVRKSPKPISLLLSTQRRKRNKGWSKDEGTEAEIRKVMNGDYQTSYIEVKRGSKIGEKSAWMLNLSIDVPKIDKGVDPSIIGGIDVGVKSPLVCAIDNAFSRYSISDNDLFHFNKKMFARRRILLKKSRHKRAGHGTKNKLMPITILTEKSKRFRKKLIERWACEIADFFIKNKVGTVQMENLESMKRKEDSYFNTRLRGFWPYAEMQNKIEFKLKQYGIEIRKVAPNNTSKTCSKCGHLNNYFNFEYRKKNKFPPFKCEKCNFKEDADYNAALNISNPKLKSTKEEH

SEQ ID NO: 2921 - protein, 726 aa, synthetic construct
SEVEFSHEYWMRHALTLAKRARDEREVPVGAVLVLNNRVIGEGWNRAIGLHDPTAHAEIMALRQGGLVTQNYRLIDATLYVTFEPCVMCAGAMVHSRIGRVVFGVRNSKRGAAGSLMNVLDYPGMGHRVEITEGILADECAALLCDFYCMPRQVFNAQKRAQSSINSGGSSGGSSGSETPGTSESATPESSGGSSGGSAKNTITKTLQLRIVRPYNSAEVEKIVTDEKNNREKIALEKNKDKVKEACSKHLKMASYCTTQVERNACLFCKARKLDDKFYQKLRGQFPDAVFWQEIGEIFRQLQKQAAEVYNQSLVELYYEILIKGKGIANASSVEHYLSDVCYTRAAELFKNAAIASGLRNKIKSNFRLKELRNMKSGLPTTKSDNFPIPLVRQKGGQYTGFEISNHNGDFIIKIPFGRWQVKKEVNKHRPWEKFDFEQVRKSPKPISLLLSTQRRKRNKGWSKDEGTEAEIRKVMNGDYQTSYIEVKRGSKTGEKSAWMLNLSIDVPKIDKGVDPSIVGGIDVGVKSPLVCAINNAFSRYSISDNDLFRFNKKMFARRRILLKKNGHKRAGHGAKNKLKPISILTGKSERFRKKLIERWACEIADFFIKNKVGTVQMENLESMRRKEDSYFNIRLRGFWPYAEMQNKIEFKLKQYGIEIRKVAPNNTSKTCSKCGHLNNYFSFEYRKKNKFPHFKCEKCNLKENADYNAALNISNPKLKSTKGEP

SEQ ID NO: 2922 - protein, 726 aa, synthetic construct
SEVEFSHEYWMRHALTLAKRARDEREVPVGAILVLNNRVIGEGWNRAVGLHDPTAHAEIMALRQGGLVMQNYRLIEATLYVTFEPCIMCAGAMIHSRIGRVVFGVRNSKRGAAGSLMNVLNYPGMNHRVEITEGILADECAALICDYYRMPRQVFNARKKAQSSINSGGSSDGGSGSETPGTSESATPESSGDSSGGSAKNTITKTLKLRIVRPYNSAEVEKIVADEKNNREKIALEKNKDKVKEACSEHLKVAAYCTTQVERNACLFCKARKLDDKFYQKLRGQFPDAVFWQEIGEIFRQLQKQAAEVYNQSLVELYYEIFIKGKGIANASSVEHYLSDVCYTRAAELFKNAAIASGLRGKVRSNFRLKELKNMKSGLPTTKSDNFPIPLVKQKGGQYTGFEISSHNDDFIIKIPFGRWQVKKEIDKYRPWEKFDFEQVRKSPKPISLLLSTQRRKRNKGWSKDEGTEAEIRKVMNGDYQTSYIEVKRGSKIGEKSAWMLSLSIDVPKIDKGADPSIIGGIDVGVKSPLVCAINNAFCRYSISDNDLFHFNKKMFARRRILLKKSRHKRAGHGAKNKLKPISILTEKSKRFRKKLIERWACEIADFFIKNKVGTVQMENLESMKRKEDSYFNIRLRGFWPYAEMQNKIEFKLKQYGIEIRKVAPNNTSKTCSRCGHLNNYFDFEYRKMNKFPHFKCEKCNFKENADYNAALNISNPKLKSTKEEP

SEQ ID NO: 2923 - protein, 726 aa, synthetic construct
SEVEFSHEYWMRHALTLAKRARDEREVPVGAILVLNNRVIGEGWNRAIGLHDPTAHAEIMALRQGGLAMQNYRLVDATLYVTFEPCVLCAGAMVHSRIGRVVFGVRNSKRGAAGSLMNVLNHPGMSHRVEITGGILADECAALLCDFYRMPRQVFNAQKKARSNINSGGSSGGSSGSETLGTSESATPESSGGSSGGPAKNTITKTLKLRIVRPYNSAEVEKIVADEKNNREKTALEKNKDKVKEACSEHLKVAAYCTTQVERSACLFCKARKLDDKFYQKLRGQFPDAVFWQEIGEIFRQLQKQAAEIYNQSLIELYYEIFIKGKGFANASSVEHYLSNVCYTRAAELFKNAAIASGLRGKVKSNFRLKELKNMKSGLPTTKSDNFPIPLVKQKGGQYTGFEINSHNDDFIIKIPFGRWQVKKEIDKYRPWEKFDFEQVRKGPKPISLLLSTRRRKRNKGWSKDEGTEAEIRKVMNGDYQTSYIEVKRGSKIGEKSAWMLNLSIDVPKIDKGVDPSIIGGIDVGVKSPLVCAINNAFSRYSISDNELFHFNKKMFARRRILLKKNRHKRAGHGAKNKLKPISILTEKSGRFRKKLIERWACEIANFFIKNKVGTVQMENLGSMKRREDSYFNIRLRGLWPYAEMQNKIEFKLKQYGIEVRKVAPNNTSKTCSKCGHLNNYFNFEYRKKNKLPLFKCEKCNFKENADYNAALNISNPKLKSTKGEP

SEQ ID NO: 2924 - protein, 726 aa, synthetic construct
SEVEFSHEYWMRHALTLAKRARDEREVPVGAVLVLNNRVIGEGWNRAIGLHDPTAHAEIMALRQGGLVMQNYRLVDATLYVTFEPCVLCAGAMVHSRIGRVVFGVRNSKRGAAGSLMNVLDYPGMGHRVEITEGILADECAALLCDFYCMPRQVFNAQKRAQSSINSGGSSGGSSGSETPGTSESATPESSGGGSSGSAKNTITKTLQLRIVRPYNSAEVEKIVADEKNNREKIALEENKDKVREACNKHLKAASYCTTQVERNACPFCKARKLDDKFYQKLRGQFPDAVFWQELGEILRQLQKQAAEIYNQSLIELYYEIFIKGRGFANASSVEHYLSDVCYTRAAELFKNAAIASGLRGKVKSNFRLKELKNMKSGLPTTKSDNFPIPLVKQKGGQYTGFEISSHNDDFIIKIPFGRWQAKEEIDKYRPWERFDFEQVRKSPKPISLLLSTQRRKRNRGWSKDEGTEAEIRKVMNGDYQTSYIEVKRGSKIGEKSAWMLNLSIDVPKIDKGVDPSIIGGIDVGVKSPLVCAINNAFNRYSISDNDLFRFNKKMFARRRILLEKNRHKRAGHGVKNKLKPITILTEKSGRFRKKLIERWACEIADFFVKNKVGTVQMENLESMKRKEDSYFNIRLRGFWPYAEMQNKIEFKLKQYGIKVRKVAPNNTSKTCSKCGHLNNYFSFEYRKKNKFPHFKCEKCNFKEDADYNAALNISNPKLKSTKEKP

SEQ ID NO: 2925 - protein, 726 aa, synthetic construct
SEVEFSHEYWMRHALTLAKRARDEREVPVGAVLVLNNRVIGEGWNRAIGLHDPTAHAEIMALRQGGLVMQNYRLIDATLYVTFEPCVMCAGAMVHSRIGRVVFGVRNSKRGAAGSLMNVLDCPGMGHRVEITEGILVDECAALLCDFYRMPHQVLNAQKKARSSISSGGSSGGSSCSETPGASESVTPKSSGSSSAGSTRNTITKTLKLRIVRPYNSAEVEKIVADEKNSREKIALEKNKDKVKEACSEHLKVAAYCTTQVERNACLFCKARKLDDRFYQKLRGQFPDAVFWQEIGEIFRQLQKQAAEIYNQSLIELYYEIFIKGKGFANASSVEHYLSDVCYTRAAELFKNAAIASGLRGKVKSNFRLKELKNMKSGLPTTKSDNFPIPLVKQKGGQYTGFEVSSHNDDFIIKIPFGRWQVKKGIDKYRPWEKFDFEQVRKSPRPISLLLSTQRRKRNKGWSKDEGTEAEIRKVMNGDYQTSYIEVKRGSKIGEKSAWMLNLSIDVPKIDKGVDPSIIGGIDVGVKSPLVCAIDNAFSRYSISDNDLYHFNKKMFAKRRILLKKNRHKRAGHGAKNKLKPISILTEKSKRFRKKLIERWACEIADFFIKNKVGTVQMENLESMKRKEDSYFNIRLRGFWPYAEMQNKIEFKLKQYGIEIRKVAPNNTSKTCSKCGHLNNYFNFEYRKKNKFPHFRCEKCNFKENADYNAALNISNPKLKSTKEEP

SEQ ID NO: 2926 - protein, 726 aa, synthetic construct
SEVEFSHEYWMRHALTLAKRARDEREVPVGAVLVLNNRVIGEGWNRAIGLHDPTAHAEIMALRQGGLVMQNYRLIDATLYVTFEPCVMCAGAMIHSRIGRVVFGVRNNKHGAAGSLVNVLNYPGMNHRVEITEGILADECAALLCDFYCMPRQVLNAQKRAQSSINSGGSSGGSSGSETPGTSESATPESSGGCSAGSTKDTITKTLKLRIVRPYNSAEVEKIVADEKNNRERIALEKNKDKVKEACSKHLKVAAYCTTQVERNACLFCKARRLDDKFYQKLRGQFPDAVFWQEIGEIFRQLQKQAAEIYNQSLVELYYEIFIKGKGIANASSVEHYLSDVCYTRAAELFRNAAIASGLRNKIKSNFRLKELRNMKSGLPTTKSDNFPIPLVKQKGGQYTGFEISSHNDDFIIKIPFGRWQVKEEIDKYRPWEKFDFEQVRKSPKPISLLLSTQRRRRNKGWSKDEGTEAEIRKVMNGDYQTSYIEVKRGSKIGEKSAWMLNLSIDVPKIDKGVDPSIIGGIDVGVKSPLVCAINNAFSRHSISDNDLFHFNKKMFARRRILLKKNRHKRAGHGAKNKLKPISILTGKSKRFRKKLIERWACEIADFFIKNKVGTVQMENLESMKRKEDSYFNIRLRGFWPYAEMQNKIEFKLKQYGIEIRKVAPNNTSKTCSKCGHLNNYFDFEYRKKNKFPHFKCEKCNFKENADYNAALNISNPKLKSTKEEP

SEQ ID NO: 2927 - protein, 726 aa, synthetic construct
SEVEFSHEYWMRRALTLAKRARDEREVPVGAVLVLNNRVIGVGWNRAAGLHDPTAHAEIMALRQGGLVMQNYRLVEATLYVTFEPCIMCAGAMIHSRIGRVVFGVRNSKRGAAGSLMNVLNYPGMNHRVEITEGILADECAALLCDYYRMPRQVFNAREKAQSSINSGGSSDGGSGSETPGTSESATPESSGGSSGGSAKNTITKTLKLRIVRPYNSAEVEKIVADEKNDREKIALEKNKDKVKEACSEHLKVAAYCTTQVERNACLFCKARKLDDRFYQKLRGQFPDAVFWQETGEIFRQLQRQAAEIYNQSLIELYYEIFIKGKGFANASSVEHYLSDVCYTRAAELFKNAAIASGLRGKVKSNFRLKELKNMKSGLPTTKSDNFPIPLVKQKGGQYTGFEISSRNDDFIIKIPFGRWQVKKEIDRYRPWEKFDFEQVRKSPKPISLLLSTQRRKRNKGWSKDEGTEAEIRKVMNGDYQTSYIEVKRGSKIGEKSAWMLSLSIDVPKIDKGVDPSTIGGIDVGVKSPLVCAINNAFCRYSISDNDLFHFNKKVFARRRILLKNNRHRRAGHGAKNKLKPITILTEKSKRFRKKLIERWACEIADFFIKNKVGTVQMENLESMKRKEDSYFNIRLRGFWPYAEMQNKIEFKLKQYGIEIRKVAPNNTSRTCSKCGHLNNYFNFEYRKKNKFPHFKCEKCNFKEDADYNAALNISNPKLKSTKEEP

SEQ ID NO: 2928 - protein, 726 aa, synthetic construct
SEVEFSHEYWMRHALTLAKRARDEREVPVGAVLVLNNRVIGEGWNRAIGLHDPTAHAEIMALRQGGLVMQNYRLTDATLYVTFEPCIMCAGAMIHSRIGRVVFGVRNSKRGAAGSLMNVLNYPGMNHCVEITEGILVDECAALLCDFYRMPRQVLNAQKKAQSSISSGGSSGGSSGSETPGASGSVTPKSSGGSSAGSTKDTITKTLKLRIVRPYNSAEVEKVVADEKNNREKIAMEKNKDKVKEACSKHLKVASYCTTQVERNACLFCKARKLDDKFYQKLRGQFPDAVFWQELGGIFRQLQKQAAEIYNQSLIELYYEIFIKGRGFANASSVEHYLSDVCYTRAAELFKNAAIASGLRNKIKSNFRLKELRNMKSGLPTTKSDNFPIPLVRQKGGQYTGFEISNHDGDFIIKIPFGRWQVKKEINKHRPWEKFDFEQVRKSPKPISLLLSTQRRKRNKGWSKDEGTEAEIRKVMNGDYQTSYIEVKRGSKIGEKSAWMLNLSIDVPKIDKGVDPGIIGGIDVGVKSPLVCAINNASSRYNISDNDLFHFNKKMFARRRILLKKNRHRRAGHGVKNKLKPITILAEKSKRFRKKLIERWACEIADFFVKNKVGTVQMENLESMKRKEDSYFNIRLRGFWPYAEMQNKIEFKLKQYGIEIRKVAPNNTSRTCSKCGHLNNYFNFEYRKKNKFPHFKCEKCNFKENADYNAALNISNPKLKSTKGEP

SEQ ID NO: 2929 - protein, 726 aa, synthetic construct
SEVEFSHEYWMRHALTLAKRARDEREVPVGAILVLNNRVIGEGWNRTIGLHDPTAHAEIMALRQGGLVMQNYRLIDATLYVTFEPCVMCAGAMIHSRIGRVVFGVRNSKRGAAGSLMNVLDYPGMNHRVEITEGILADECAALLCDFYRMPRQVFNAQKKARPNINSGGSSGGRSGSETPGTSESATPESSGGSSSGSAKNTITKTLKLRIVRPYNSAEVEKIVADEKNNREKIALEKNKDKVKEACSKHLKVATYCTTQVERDACLFCKARRLDDKFYQKLRGQFPDAVFWQEVGEIFRQLQKQAAEIYNQSLIELYYEIFIKGKGFANASSVEHYLSDVCYTRAAELFKNAAIASGLRGKVKSNFKLKELKNMKSGLPTTKSDNFPIPLVKQKGGQYTGFEISNHNGDFIIKIPFGRWQAKKEIDKRRPWEKYDFEQVRKSPKPISLLLSTQRRKRNKGWSKDEGTEAEIMKVMRGDYQTSYIEVKRGSKIGEKSAWMLNLSIDVPKIDRGVDPSIIGGIDVGVKSPLVCAINNSSSRYSICDNDLFRFNKKMFARRRILLKKNRHKRAGHGAKNKLKPITILTKKSERFRKKLIERWVCEVADFFIKNKVGTVQMENLESMKRKEDSYFNIRLRGFWPYAEMQNKIEFKLKQYGIGIRKVTPNNTSKTCSKCGHLNNYFNFEYRKKNKFPHFKCEKCNFKENADYNAALNISNPKLKSTKEEP

SEQ ID NO: 2930 - protein, 726 aa, synthetic construct
SEVEFSHEYWMRRALTLAKRARDEREVPVGAVLVLNNRVIGEGWNRAIGLHDPTAHAEIMALRQGGLVMQNYRLTDATLYVTFEPCVMCAGAMIHSRIGRVVFGVRNSKRGAAGSLMNVLNYPGMNHCVEITEGILVDECAALLCDFYRMPRQVLSAQKKAQSNISSGGSSGGSSGSETPGARGSVTPKSSGGGFGGSAKNTITKTLQLRIVRPYNSAEVEKIVADEKNNREKIALEKNKDKVKEACSKHLKVASYCTTQVERNACLFCKARKLDDKFYQKLRGQFPDAVFWQEIGEIFRQLQKQAAEIYNQSLIELYYEIFIKGKGSANASSVEHYLSDVCYTRAAELFKNAAIASGLRGKVKSNFRLKELKNMRSGLPTTKSDNFPIPLVKQKGGQYAGFEISSHNDDFIIKIPFGRWQVKKEIDKYRPWEKFDFEQVRKSPKPISLLLSTRRRKRNKGWSKDEGTEAEIRKVMNGDYQTSYIEVRRGNKIGERSAWMLNLSIDVPKIDKGVNPSIIGGIDVGVKSPLVCAINNAFSRYSISDNDLFHFNKKMFARRRILLKKNRHRRAGHGAKNKLKPISILTEKSKRFRKKLIERWACEIADFFIKNKVGTVQMENLESMKRKEDSYFNIRLRGFWPYAEMQNKIEFKLKQYGIEIRKVAPNNTSKTCSKCGHLNNYFNFEYRRKNKFPHFKCEKCNFKEDADYNAALNISNPKLKSTKEEP

SEQ ID NO: 2931 - protein, 725 aa, synthetic construct
SEVEFSHEYWMRHALTLAKRARDEREVPVGAVLVLNNRVIGEGWNRAIGLHDPTAHAEIMALRQGGLVMQNYRLTDATLYVTFEPCVMCAGAMIHSRIGRVVFGVRNSKRGAAGSLMSVLNYPGMNHCVEITEGILVDECAALLCDFYRMPRQVLNAQKKAQSSISSGGSSGGSSGSETPGASGNVTPKSSGGSSAGSTKDTITKTLKLRIVRPYNSAEVEKVVADEKNNREKIAMEKNKDKVKEACSKHLKVASYCTTQVERNACLFCKARKLDDKFYQKLRGQFPDAVFWQELGGIFRQLQKQAAEIYNQSLIELYYEIFIKGKGITNASRVEHYLSDVCYTRAAELFKNAAIASGLRSKVRSNFRLKELKNMKSGLPTTKSDNFPIPLVKQKGGQYTGFEISSHNSDFIIKIPFGRWQEKEEIDKYRPWEKFDFEQVRRSPKPISLLLSTQRRKKNKGWSKDEGTEAEIRRVMNGDYQTSYIEVKRGSKIGEKSAWMLNLSIDVPKIDKGVDPSIIGGIDVGVKSPLVCAINSAFSRYSISDNDLFRFNKKMFARRRILLKKNRHKRAGHGAKNKLRPISILTGKSERFRKKLIERWACEIADFFIKNKVGTVQMENLESMKRKEDSYFNIRLRGFWPYAEMQNKIEFKLKQYGIEIRKVAPNDTSKTCSKCGHLNNYFNFEYRKKNKFPHFKCEKCNFKENADYNAALNISNPKLKSTEEP

SEQ ID NO: 2932 - protein, 726 aa, synthetic construct
SEVEFSHEYWMRHALTLAKRARDEREVPVGAVLVLNNRVIGEGWNRTTGLHDPTAHAEIMALRQGGLVMQNHRLVDATLYVTFEPCVMCAGAMIHSRIGRVVFGVRNSKRGAAGSLTNVLNYPGMNHRVEITEGILVDECAALLCDFYRMPRQVFNAQKKAQSAINSGSSSGGSSGSETPGTSESPTPESSGGSPGGSAKSTITKTLKLRIVRPYNSAEVEKIVADEKNNREKIALEKNKDKVKEACSKHLKVAAYCTTQVERNACLFCKARKLDDKFYQKLRGQFPDAVFWQEIGEIFRQLQKQAAEIYNQSLIELYYEIFIKGKGFANASSVEHYLSDVCYTRAAELFKNAAIASGLRGKVKSNFRLKELKNMKSGLPTTKSDNFPIPLVRQKGGQYTGFEISSHNDDFIIKIPFGRWQVKKEIDKYRPWEKFNFEQVRKSPKPISLLLSTQRRKRNKGWSKDEGTEAEIRKVMNGDYQTSYIEVKRGSKTGEKSAWMLNLSIDVPKIDKGVDPSIIGGIDVGVKSPLVCAINNAFSRYSISDNDLFRFNKKMFARRRILLMKNRHKRAGHGAKNKLKPITILTKKSERFRKKLIERWACEIADFFVKNKVGTVQMENLESMKRREDSYFNIRLRGFWPYAKMQNKIEFKLKQYGIEIRKVAPNNTSKTCSKCGHLNNYFNFEYRKKNKFPHFKCEKCNFKENADYNAALNISSPKLKSTKEEP

SEQ ID NO: 2933 - protein, 726 aa, synthetic construct
NEDEFSHEYWMRHALTLAKRARDGREVPVGAVLVLNNRVIGEGWNRAIGLHDPTAHAEIMALRQGGLVMQNYRLIDATLYVTFEPCVMCAGAMVHSRIGRVVFGVRNSKRGAAGSLMNVLDYPGMGHRVEITEGILADECAALLCDFYCMPRQVFNAQKRAQSSINSGGSSGGSSGSETQGTSESATPESSGGSSGGSTKNTITKTLKLRIVRPYNSAEVEKIVADEKNNRERTALEKNKDKVKEACSKHLKVAAYCTTQVERNACLFCKARKLDDKFYQKLRGQFPDAVFWQELGEILRQLQKQAAEIYNQSLIELYYEIFIKGRGFANASSVEHYLSDVCYTRAAELFKNAAIASGLRGKVKSNFRLKELRNMKSGLPTTKSDNFPIPLVRQKGGQYTGFEISNHDGDFILKIPFGRWQVKKEINKHRPWEKFDFEQVRKSPKPISLLLSTQRRKRNKGWSKDEGTEAEIRRVMNGDYQTSYIEVKRGSKIGEKSAWMLNLSIDVPKIDKGVDPSIIGGIDVGVKSPLVCAINNAFSRYSISDNDLFHFNKKMFARRRILLKKNRRRRAGHGAKNKLKPITILTEKSVRFRKKLIERWACEIADFFIKNRVGTVQMENLESMKRREDSYFNIRLRGFWPYAEMQNKIEFKLKQYGIEIRKVAPNNTSKTCNKCGHLNNYFNFEYRKKNKFPHFRCEKCNFKENADYNAALNISDPKLKSTKEEP

SEQ ID NO: 2934 - protein, 726 aa, synthetic construct
SEVEFSHEYWMRHALALAKRARDEREVPVGAVLVLNNRAIGEGWNRAIGLHDPTAHAEIMALRQGGLVMQNYRLTDATLYVTFEPCVMCAGAMIHSRIGRVVFGVRNSKRGAAGSLMNVLNYPGMTHRVEITEGILADECAALLCDFYRMPRQVFNARKKAQSSISPGGSSGGSSDSETPGTSESATPESSGGSSGGSAKNIITKTLKLRIVRPYNSAEVEKIVADEKDIRERIALEKNKGKVKEACSKHLKVAAYCTTQVERNACLFCKARKLDDKFYQKLRGRFPDAVLWQEIGEIFRQLQKQAAEIYNQSLIELYYEIFIKGKGFANASSVEHYLSDVCYTRAAELFKNAAIASGLRNKIKSNFRLKELRNMRSGLPTTKSDNFPIPLVRQKGGQYTGFEISNHDGDFIIKIPFGRWQVKKEINKHRPWEKFDFEQVRKSPKPISLLLSTQRRKRNKGWSKDEGTEAEIRKVMNGDYQTSYIEVKRGSKTGEKSAWMLNLSIDVPKIDKGVDPSIIGGIDVGVKSPLVCAINNAFSRYSISDNDLFHFNKKMFARRRILLGKNRHKRAGHGARNKLKPITVLTEKSERFRKKLIERWACEIANFFIKNKVGTVQMENLESMKRREDSYFNIRLRGFWPYAEMQSKIEFKLKQYGIKIRKVAPNNTSKTCSKCGHLNNYFNFEFRKKNKFPHLKCEKCNFKEDADYNAALNISNPKLKSTKEEP

SEQ ID NO: 2935 - protein, 726 aa, synthetic construct
SEVEFSHEYWMRHALTLAKRARDEREVPVGAVLVLNNRAIGEGWNRAVGLHDPTAHAEIMALRQGGLVMQSYRLTDATLYVTFEPCVMCAGAMIHSRIGRVVFGVRNSKRGAAGSLMNVLNYPGMNHRVEITEGILADECAALLCDFYRMPRQVFSAQRKARSNINSGGSSGGSSGSETPGTSESATPESSGGSSGGSAKNTITKTLKLRIVRPYNSAEVEKIVADEKNNREKVALEKNKDKVKEACSKHLKVATYCTTQVERNACLFCKARKLDDKFYQKLRGQFPDAVFWQEVGEIFRQLQKQAAEIYNQSLIELYYEIFIKGKGIANASSVGHYLSDVCYTRAAELFKNAAIASGLRGKIKSNFRLKELKNMKSGLPTTKSDNFPIPLVKQKGGQYTGFEISNHNGDFIIKIPFGRWQVKKEINKYRPWEKFDFEQVRKSPKPISLLLSTQRRRRNKGWSKDEGTEAEIRKVMNGDYQASYIEVKRGSKIGEKSAWMLNLSIDVPKIDKGVDPSIIGGIDVGVKSPLVCAINNAFSRYSISDNDLFRFNKKMFARRRILLGKNRHKRAGHGVKNKLKPITILTEKSGRFRKKLIERWACEIADFFVKNKVGTVQMENLESMKRKEDSYFNIRLRGFWPYAEMQNKIEFKLKQYGIKVRKVAPNNTSKTCSKCGHLNNYFSFEYRKKNKFPHFKCEKCNFKEDADYNAALNISNPKLKSTKEEP

SEQ ID NO: 2936 - protein, 726 aa, synthetic construct
SEVEFSHEYWMRHALTLAKRARDEREVPVGAILVLNNRVIGEGWNRAIGLHDPTAHAEIMALRQGGLVMQNYRLIDATLYVTFEPCVMCAGAMIHSRIGRVVFGVRNNKHGAAGSLVNVLNYPGMNHRVEITEGILADECAALLCDFYRMPRQVFNARKKAQSSINPGGSSGGSRGSETPGASESATPKSSGGSSGGSAKNTITKTLKLRIVRPYNSTEVEKIVADEKNNREKIALEKNKDKVKEACSKHLKVAAYCTTQVERNACLFCRARKLDDKFYQKLRGQFPDAVFWQELGGIFRQLQKQAAEIYNQSLIELYYEIFIKGKGITNASRVEHYLSDVCYTRAAELFKNAAIASGLRSKVRSNFRLKELKNMKSGLPTTKSDNFPIPLVKQKGGQYTGFEISSHNSDFIIKIPFGRWQVKKEICKHRPWEKFDFEQVRKSPKPISLLLSTQRRKRNKGWGKDEGTEAEIRKVMNGDYQTSYIEVKRGSKIGEKSAWMLSLSIDVPKIDKGVDPSIVGGIDVGVKSPLVCAINNALGRFSISDNDLFHFNKKMFARRRILLRKNRHKRAGHGAKNKLKPISILTEKSRRFRKKLIERWACEIADFFTKNKVGTVQMENLESMKRKEDSYFNIRLRGFWPYAEMQNKIEFKLKQYGIEIRKVAPNNTSKTCSKCGHLNNYFNFEFRKKNKFPHFKCEKCNFKEDADYNAALNISNPKLKSTKEEP

SEQ ID NO: 2937 - protein, 726 aa, synthetic construct
SEVEFSHEYWMRHALTLAKRARDEREVPVGAILVLNNRVIGEGWNRAIGQHDPTAHAEIMALRQGGLVLQNYRLTDATLYVTFEPCVMCAGAMIHSRIGRVVFGVRNSKRGAAGSLMNVLNYPGMNHRVEITEGILVDECAALLCDFYRMPRQVLNAQKKAQSSISPGGSSGGSSGSETPGASESVTPKSSGGSSGGSAKNTITKTLQLRIVRPYNSAEVEKIVTDEKNNREKIALEKNKGKVKEACSKHLKMASYCTTQVEKNACLFCKARKLDDKFYQKLRGQFPDAVFWQELGEIFRQLQKQAAEIYNQSLIELYYEIFIKGKGFANASSVEHYLSDVCYTRAAELFKNAAIASGLRGKVKSNFRLKELKNMKSGLPTTKSDNFPIPLVKQKGGQYTGFEISSHNDDFIITIPFGRWQVKKEIDKYRPWEKFDFAQVRKSPKPISLLLSTQRRKRNKGWSKDEGTEAEIRKVMNGDYQTSYIEVKRGSKIGEKSAWMLNLSIDVPKIDKGVDPSIIGGIDVGVKSPLVCAINNAFSRYSISDNDLFHFNKKMFARRRILLKKTRHKRAGHGAKHKLKPISILTEKSERFRKKLIERWACEIADFFIKNKVGTVQMENLESMKRREDSYFNIRLRGFWPYAKMQNKIEFKLKQYGIEIRKVAPNNTSKTCSKCGHLNNYFNFEYRKKNKFPHFKCEKCNFKENADYNAALNISNPKLKSTKEEP

SEQ ID NO: 2938 - protein, 726 aa, synthetic construct
SEVEFSHEYWMRHALTLAKRARDEREVPVGAVLVLNNRVIGEGWNRAIGLHDPTAHAEIMALHQGGLVMQNYRLIDATLYVTFEPCVMCAGAMIHSRIGRVVFGARNSKRGAAGSLMNVLSYPGMNHRVEITEGILVDECAALLCDFYRMPRQVFNAQKKAQSSVSSGGSSGGSSGSETPGASGSVTPKSSVGSSAGSTKNTITKTLKLRIVRPYNSAEVEKIVADEKNNREKIALEKNRDKVKEACSKHLKVAAYCTTQVERNACLFCKARKLDDKFYQKLRGQFPDAVFWQEISEVFRQLQKQAAEIYNQSLIELYYEIFIKGKGFANASSVEHYLSDVCYTRAAELFKNAAIASGLRGKVKSNFRLKELKNMKSGLPTTKSDNFPIPLVKQKGGQYTGFEISSHNDDFIIKIPFGRWQVKKEISKHRPWEKFDFEQVRKSPKPISLLLSTQRRKRNKGWGKDEGTEAEIRKVLNGDYQTSYIEVKRGSKTGEKSAWMLNLSIDVPKIDKGVDPSIIGGIDVGVKSPLVCAINNAFSRYSISDNDLFRFNKRMFARRRILLKKNRHKRAGHGAKNKLKPISILTGKSERFRKKLIERWACEIADFFIKNKVGTVQMENLESMKRKEDSYFNIRLRGFWPYAEMQNKIEFKLKQYGIVVRKVAPNNTSKTCSECGHLNNYFNFEYRKKNKFPLFKCEKCNFKENADYNAALNISNPKLKSTKGEP

SEQ ID NO: 2939 - protein, 726 aa, synthetic construct
NEDEFSHEYWMRHALTLAKRARDGREVPVGAVLVLNNRVIGEGWNRAIGLHDPTAHAEIMALRQGGLVMQNYRLIDATLYVTFEPCVMCAGAMVHSRIGRVVFGVRNSKRGAAGSLMNVLNFPGMSHCVEITEGILVDECAALLCDFYRMPRQVLNAQKKAQSSISSGGSSGGSGGGETPGASESVTPKNSGGSSASSTKNTITKTLKLRIVRPYNSAEVEKIVADEKNSREKIALEKNKDKVKEACREHLKVAAYCTTQVERSACLFCKARKLDDRFYQKLRGQFPDAVFWQEISEIFRQLQKQAAEIYNQSLIELYYEVLIKGKGIANASRVEHYLSDVCYTRAAELFKNAAIASGLRSKIKSNFRLKELRNMKSGLPTTKSDNFPIPLVKQKGGQCTGFEISNHNSNFIIKIPFGRWQVKKEIDKYRPWEKFDFEQVRKSPKPISLLLSTQRRRRNKGWSKDEGTEAEIRKVMYGDYQTSYIEVKRGSKIGEKSAWMLNLSIDVPKIDKGVDPSIIGGIDVGVKSPLVCAINNAFSRYSISDNDLFHFNKKVFARRRILLKKNRHRRAGHGAKNKLKPITILTEKSKRFRKKLIERWACEIADFFIKNKVGTVQMENLESMKRKEDSYFNIRLRGFWPYAEMQNKIEFKLKQYGIKIRKVAPNNTSRTCSECGHLNNYFSFEYRKKNKFPHFKCEKCNFKEDADYNAALNISNPKLKGTKEEL

SEQ ID NO: 2940 - protein, 726 aa, synthetic construct
SEVEFSHEYWMRHALTLAKRARDEREVPVGAILVLNNRVIGEGWNRAIGLHDPTAHAEIMALRQGGLVMQNYRLIDATLYVTFEPCVMCAGAMIHSRIGRVVFGVRNSKHGAAGSLVNVLNYPGMNHRVEVTEGILADECAALLCDFYRMPRQVFGARRKAQSSINPGGSSGGSSGSETPGTSESATPESSGGSTGGSAKNTITKTLKLRIVRPYNSAEVEKIVADEKNNREKIALEKNKDKVKEACSEHLKVAAYCTTQVERSACLFCKARKLDDKFYQKLRGQFPDAVFWQEIGEIFRQLQKQAAEIYNQSLIELYYEIFIKGKGFANASSVEHYLSDVCYTRAAELFKNAAIASGLRGKVKSNFRLKELKNMKSGLPTTKSDNFPIPLVKQKGGQYTGFEISSHHDDFIIKIPFGRWQVKKEIDKYRPWEKFDFEQVRKSPKPISLLLSTQRRKRNKGWSKDEGTEAEIRKVMNGDYQTSYIEVKRGSKIGEKSAWMLSLSIDVPKIDKGVDPSIVGGIDVGVKSPLVCAINNALGRYSISDNDLFHFNKKMFARRRILLRKNRHKRAGHGARNKLKPISILTGKSERFRKKLIERWACEIADFFIKNKVGTVQMENLESMKRKEDSYFNIRLRGFWPYAEMQNKIEFKLKQYGIEIRKVAPNNTSKICSKCGHLNNYFNFEYRRMNKFPHFKCEECNFKENADYNAALNISNPKLESTKEEP

SEQ ID NO: 2941 - protein, 726 aa, synthetic construct
SEVEFSHEYWMRRALTLAKRARDEREVPVGAVLVLNNRVIGVGWNRAVGLHDPTAHAEIMALRQGGLVMQNYRLIEATLYVTFEPCIMCAGAMIHSRIGRVVFGVRNSKRGAAGSLMNVLNYPGMNHRVEITEGILADECAALLCDYYRMPRQVFNARKKAQSSINSGGSSGGGSGGETPGTSESATQESSGGSSGGSAKNTITKTLKLRIVRPYNSAEVEKIVADEKNNREKIALEKNKDKVKEACSKHLKVAAYCTTQVERNACLFCKARKLDDKFYQKLRGQFPDAVFWQEISEIFRQLQKQAAVIYNQGLIELYYEIFIKGKGFANASSVEHYLSDVCYTRAAELFKNAAIASGLRGKVKSNFRLKELKNMKSGLPTTKSDNFPIPLVKQKGGQYTGFEISNHNSDFIIKIPFGRWQVKKEIDKYRPWEKFDFEQVRKSPKPISLLLSTQRRRRNKGWSKDEGTEAEIRKVMNGDYQASYIEVKRGSRIGEKSAWMLNLSIDVPKIDKGVDPSIIGGIDVGVKSPLVCAINNAISRYSISDNDLFHFNKKVFARRRILLKKNRHRRAGHGTKNKLKPITILTEKSKRFRKKLIERWACEIADFFIKNKVGTVQMENLESMKRKEDSYFNIRLRGFWPYAEMQSKIEFKLKQYGIKIRKVAPNNTSKTCSKCGHLNNYFNFEYRKKNKFPHFKCEKCNFKEDADYNAALNISNPKLKSTKDEP

SEQ ID NO: 2942 - protein, 726 aa, synthetic construct
SEVEFSHEYWMRHALTLAKRARDKHEVPVGAVLVLDNRVIGEGWNRATGQNDPTAHAEIMALRQGGLVMQNHRLIDATLYVTFEPCVMCAGAMIHSRIGRVVIGVRNSKRGAAGSLMNVLNHPGMNHRVEITEGILADECAALLCDFYRMPRQVLNAQEKAQSSINSGGSSGGSSGSETPGTSESATPGSSGGGSSGSAKNTITKTLQLRIVRPYNSAEVEKIVADEKNNREKIALEKNKDKVREACSKHLKVASYCTTQVERNACPFCKARKLDDKFYQKLRGQFPDAVFWQELGEILRQLQKQAAEIYNQSLIELYYEIFIKGRGFANASSVEHYLSDVCYTRAAELFKNAAIASGLRGKVRSNFRLKELKSMKSGLPTTKSDNFPIPLVKQKGGQYTGFEISNHNSDFIIKIPFGRWQVKKEIDKYRPWEKFDFEQVRKSPKPISLLLSTRRRKRNKGWSKDEGTEAEIRKVMNADYQTSYIEVKRGSKTGEKSTWMLNLSIDVPKIDKGVDPSIIGGIDVGVKSPLVCAINNAFSRYSISDNDLFRFNKKMFARRRILLKKNRHKRAGHGAKNKLKPISILTGKSERFRKKLIERWACEIADFFIKNKVGTVQMENLESMKRKEDSYFNIRLRGFWPYAEMQDKIEFKLKQYGIEIRKVAPNNTSKTCSRCGHLNSYFNFEYRRENKFPHFKCEKCNFKENADYNAALNISNPKLKSTKEEP

SEQ ID NO: 2943 - protein, 726 aa, synthetic construct
SEVEFSHEYWMRHALTLAKRARDEREVPVGAVLVLNNRVIGEGWNRAIGLHDPTAHAEIMALRQGGLVMQNYRLTDATLYVTFEPCVMCAGAMIHSRIGRVVFGVRNSKRGAAGSRMNVLNYPGMNHCVEITEGILVDECAALLCDFYRMPRQVLNAQKKAQSSISSGGSSGGSSGSETPGASESVTPKSSVGSSAGSTKNTITKTLKLRIVRPYNSAEVEKIVADEKNNREKIALEKNKDKVKEACSKHLKVASYCTTQVERNACPFCKARKLDDKFYQKLRGQFPDAVFWQELGEILRQLQKQAAEIYNQSLIELYYEIFIKGRGFANASSVEHYLSDVCYTRAAELFKNAAIASGLRGKVKSNFRLKELRNMRGGLPTTKSDNFPIPLVKQKGGQYTGFEISSHNDDFIIKIPFGRWQVKKEIDKYRPWEKFDFEQVRKSPKPISLLLSTQRRKRNKGWSKDEGTEAEIRKVMNGDYQTSYIEVKRGSKIGEKSAWMLNLSIDVPKIDKGVDPSIVGGIDVGVKSPLVCAINNAFSRYSISDNDLFRFNKKMFARRRILLGKNRHKRAGHGAKNKLKPITILTEKSGRFRKKLIERWACEIADFFIKNKVGTVQMENLESMKRKEDSYFNIRLRGFWPYAEMQNKIELKLKRYGIKIRKVAPNNTSKTCSKCGHLNNYFNFEYRKTNKFPHFKCEKCNFKEDADYNAALNISNPKLKSTKEEP

SEQ ID NO: 2944 - protein, 726 aa, synthetic construct
SEVEFSHEYWMRHALTLAKRARDEREVPVGAILVLNNRVIGEGWNRAIGLHDPTAHAEIMALRQGGLMMQNCRLIDATLYVTFEPCVMCAGAMIHSRIGRVVFGVRNNKHGAAGSLMNVLNYPGMNHCVEITEGILVDECAALLCDFYRMPRQVLNAQKKAQSSISSGGSSGGSSGSETPGASGSVTPKSSGGSSAGSTKDAITKTLKLRIVRPYNSAEVEKIVADEKNNREKIAMEKNKDKVKEACSKHLKVASYCTTQVERNACLFCKARKLDDKFYQKLRGQFPDAVFWQELGGIFRQLQKQAAEIYNQSLIELYYEIFIKGKGITNASRVEHYLSDVCYTRAAELFKNAAIASGLRGKVKSNFRLKELKNMKSGLPTTKSDNFPIPLVKQKGGQYTGFEISNRNSDFIIKIPFGRWQVKKEINKYRPWEKFDFEQVRKSPKPISLLLSTQRRKRNKGWSKDEGTEAEIRKVMNGDYQTSYIEVKRGSRIGEKSAWMLSLSIDVPKIDRGVDPSIIGGIDVGVKSPLVCAINNALSRYSISDNDLFHFNKKMFARRRILLKKNRHRRAGHGARNKLKPITVLTEKSKRFRKKLIERWACEIANFFIKNKVGTVQMENLESMKRKEDSYFNIRLRGLWPYAEMQNKIEFKLKQYGIEIRKVAPNNTSKTCSKCGHLNNYFNFEYRKRNKFPHFKCEKCNFKENADYNAALNISNPKLKGTKEEP

SEQ ID NO: 2945 - protein, 726 aa, synthetic construct
SEVEFSHEYWMRHALTLAKRARDEREVPVGAVLVLNNRVIGEGWNRAIGLHDPTAHAEIMALRQGGLVMQNCRLVDATLYVTFEPCVMCAGAMIHSRIGRVVFGVRNSKRGAAGSLMNILNYPGMNHRVEITEGILADECAALLCDFYRMPRQVFNAQKKAQSSINPGGSSGGSSGSETPSTSESATPESSGGSSGGSAKNTITKTLQLRIVRPYNSAEVEKIVTDEKNNREKIALEKNKDKVKEACSKHLKMASYCTTQVERNACLFCKARELDDKFYQKLRGQFPDAVFWQELGGIFRQLQKQAAEIYNQSLIELYYEIFIKGKGITNASRVEHYLSDVCYTRAAELFKNAAIASGLRSKVRSNFRLKELKNMKSGLPTTKSDNFPIPLVRQKGGQYTGFEISNYNGDFIIKIPFGRWQVKKEINKHRPWEKFDFEQVRKSPKPISLLLSTQRRKRNKGWSKDEGTEAEIRKVMNGDYQTSYIEVKRGSKIGEKSAWMLNLSIDVPKIDKGVDPSIIGGIDVGVKSPLVCAINNALSRYSISDNDLFHFNKKMFARRRILLRKNRHKRAGHGARNKLKPITVLTEKSERFRKKLIERWACEIANFFIKNKVGTVQMENLESMKRREDSYFNIRLRGFWPYAEMQNKIEFKLKQYGIEIRKVAPNNTSKTCSKCGHLNNYFNFEFRKKNKFPHFKCEKCNFKENADYNAALNISNPKLKSTKEEP

SEQ ID NO: 2946 - protein, 726 aa, synthetic construct
SEVEFSHEYWMRHALTLAKRARDEREVPVGAVLVLNNRVIGEGWNRAIGLHDPTAHAEIMALRQGGLVLQNYRLVDATLYVTFEPCVLCAGAMVHSRIGRVVFGARNSKRGAAGSLMNILNYPGMNHRVEITEGILADECAALLCDFYRMPRQVFNAQKKAQSSINSGGSSGGSSGSETPSTSESATPESSGGSSGGSAKNTITKTLKLRIVRPYNSAEVEKIVADEKNNREKTALEKNKGKVKEACSEHLKVAAYCTTQVERNACLFCKARKLDDKFYQKLRGQFPDAVFWQEISEILRQLQKQAAEIYNQSLIGLYYEIFIKGKGIANANGVEHYLSDVCYTRAAELFRNAAIASGLRSKVKSNFRLKELKNMKSGLPTTKSDNFPIPLVKQKGGQYTGFEISNHNSDFIIKIPFGRWQVKEEIDKYRPWEKFDFEQVRKSPKPISLLLSTQRRKKNKGWSKDEGTEAEIRRVMNGDYQTSYIEVKRGSKIGEKSAWMLNLSIDVPKIDKGVDPSIIGGIDVGVKSPLVCAINNSSSRYSICDNDLFRFNKKMFARRRILLKKNRHKRAGHGAKNKLKPISILTEKSERFRKKLIERWACEIADFFIKNKVGTVQMENLESMKRKEDSYFNIRLRGFWPYAEMQNKIEFKLKQYGIKIRKVAPNNTSKACSKCGHLNNYFSFEYRKKNKFPHFKCEKCNFKENADYNAALNISNPKLRSTKEKP

SEQ ID NO: 2947 - protein, 726 aa, synthetic construct
SEVEFSHEYWMRYALTLAKRARDEREVPVGAVLVLNNRVIGEGWNRAIGLHDPTAHAEIMALRQGGLVMQNYRLVDATLYVTFEPCVMCAGAMVHSRIGRVVFGVRNSKRGAAGSLMNVLDYPGMGHRVEITEGILADECAALLCDFYRMPRQVLNAQKKAQSSISSGGSSGGSGGGETPGASESVTPKSSGGSSAGSTKNTITKTLKLRIVRPYNSAEVEKIVADEKNSREKIALEKNKGKVKEACSEHLKVAAYCTTQVERSACPFCKARKLDDRFYQKLRGQFPDAVFWQEISEIFRQLQKQAAEIYNQSLIELYYEIFIKGRGFANASSVEHYLSDVCYTRAAELFKNAAIASGLRSKVRSNFRLKELKNMKSGLPTTKSDNFPIPLVKQKGGQYTGFEISSHNSDFIIKIPFGRWQVREEIDKYRPWEKFDFEQVRKSPKPISLLLSTQRRKKNKGWSKDEGTEAEIRRVMNGDYRTSYIEVKRGSKIGEKSAWMLNLSIDVPKIDKGVDPSIIGGIDVGVKSPLVCAINNSSSRYSICDNDLFRFNKKMFARRRILLKKNRHKRAGHGAKNKLKPITILTKKSERFRKKLIERWVCEVADFFIKNKVGTVQMENLESMKRKEDSYFNIRLRGFWPYAEMQNKIELKLKQYGIEIRKVAPNNTSKTCSMCGHLNDYFNFEYRKKNKFPHFKCEKCNFKENADYNAALNISNPKLKSTREEP

SEQ ID NO: 2948 - protein, 726 aa, synthetic construct
SEVEFSHEYWMRHALTLAKRARDEREVPVGAVLVLNNRVIGEGWNRAIGLHDPTAHAEIMALRQGGLVMQNYRLVDATLYVTFEPCVLCAGAMVHSRIGRVVFGVRNSKRGAAGSLMNVLNYPGMNHRVEITEGILADECAALLCDFYRMPRQVFNARKKARSNINSSGSSGGSSGSETPGTSESATPESSGGSSGGSAKNTITKTLKLRIVRPYNSAEVEKIVADEKNNREKIALEKNKDKVKEACSEHLKVAAYCTTQVERNACLFCRARKLDDKFYQKLRGQFPDAVFWQEIGEIFRQLQKQAAEIYNQSLIELYYEIFIKGKGFANASSVEHYLSDVCYTRAAELFKNAAIASGLRGKVKSNLRLKELKNMKSGLPTTKSDNFPIPLVKQKGGQYTGFEISSHNDDFIIKIPFGRWQVKKEIDKYRPWEKFDFERVRKSPKPISLLLSTQRRKRNKGWGKDEGTEAEIRKVMNGDYQTSYIEVKRGSKIGEKSAWMLSLSIDVPKIDKGVDPRIIGGIDVGVKSPLVCAINNAFSRYSISDNDLFHFNKKMFARRRILLKKNRHKRAGHGAKNKLKPITILTEKSVRFRKKLIERWACEIADFFIKNKVGTVQMENLESMKGKEDSYFNIRLRGFWPYAEMQNKIEFKLKQYGIEIRKVAPNNTSKTCSKCGHLNNYFNFEYRKKNQFPYFKCEKCNFKENADYNAALNISNPQLKSTKGEP

SEQ ID NO: 2949 - protein, 726 aa, synthetic construct
SEVEFSHEYWMRRALTLAKRARDEREVPVGAVLVLNNRVIGEGWNRAIGLHDPTAHAEIMALRQGGLVMQNYRLTDATLYVTFEPCVMCAGAMIHSRIGRVVFGVRNSKRGAAGSLMNVLNYPGMNHCVEIMEGILVDECAALLCDFYRMPRQVLNAQKKAQSSISSGGSSGGCSGSEMPGASESVTPKSSGGSSGGSAKNTITKTLKLRIVRPYNSAEVEKIVADEKSNREKIALEKNKDKVKEACSEHLKVAAYCTTRVERSACLFCKARKLDDKFYQKLRGQFPDAVFWQEIGEIFRQLQRQAAEIYNQSLIELYYEIFIKGKGFANASSVEHYLSDVCYTRAAELFKNAAIASGLRGKVKSNFRLKELKNMKSGLPTTKSDNFPIPLVKQKGGQYTGFEISSHNDDFIIKIPFGRWQVRKEIGKYRPWEKFNFEQVRKSPKPISLLLSTQRRKRNKGWSKDEGTGAEIRKVMNGDYQTSYIEVKRGSKTGEKSAWMLNLSIDVPKIDKGVDPSIIGGIDVGVKSPLVCAINNALSRYSISDNDLFHFNKKMFARRRILLKKNRHKRAGHGAKNKLKPISILTEKSERFRKKLIERWACEIADFFIRNKVGTVQMENLEGMKRKEDSYFNIRLRGFWPYAEMQNKIEFKLKQYGIEIRKVAPNNTSKTCSKCGHLNNYFNFEYRKKSKFPHFKCEKCSFKEDADYNAALNISNPKLKSTKEEP

SEQ ID NO: 2950 - protein, 726 aa, synthetic construct
SEVEFSHEYWMRHALTLAKRARDEREVPVGAVLVLNNRVIGEGWNRAIGLHDPTAHAEIMALRQGGLVMQNYRLTDATLYVTFEPCVMCAGAMIHSRIGRVVFGVRNSKRGAAGSLMNVLNYPGMNHCVEITEGILVDECAALLCDFYRMPRQVLNAQKKAQPSISSGGSSGGSSGSETPGASGSVTPESSGGSSGGSAKNTITKTLKLGIVRPYNSAEVEKIVADEKNNREKIALEKNKDKVKEACSEHLKVAAYCTTLVERNACLFCKARKLDDKFYQKLRGQFPDAVFWQEIGEIFRQLQKQAAEIYNQSLIELYYEIFIKGKGFANASSVEHYLSDVCYTRAAELFKNAAIASGLRGKVKSNFRLKELKNMKSGLPTTKSDNFPIPLVKQKGGQYTGFEINSHNDDFVIKIPFGRWRVKKEIDKYRPWEKFDFEQVRKSPKTISLLLSTQRRKRNKGWSKDEGTEAEIRKVMNGDYQTSYIEVKRGSKIGEKSAWMLNLSIDVPKIDKGVDPSIIGGIDVGVKSPLVCAVNNAFSRYSISDNDLFRFNKKMFARRRILLKKNRHQRAGHGAKNKLKPITILTEKSGRFRKKLIERWACEIADFFIKNKVGTVQMENLESMKRKEDSYFNIRLRGFWPYAEMQNKIEFKLKQYGIKIRKVAPNNTSRTCSKCGHLNNYFSFEYRKKNKFPHFKCEKCNFKENADYNAALNISNPKLMSTKEEP

SEQ ID NO: 2951 - protein, 726 aa, synthetic construct
SEVEFSHEYWMRHALTLAKRARDEREVPVGAILVLNNRVIGEGWNRAIGLHDPTAHAEIMALRQGGLVMQNYRLIDATLYVTFEPCVMCAGAMIHSRIGRVVFGVRNSKHGAAGSLVNVLNYPGMNHRVEITEGILADECAALLCDFYRMPRRVFNARMKAQSSISPGGSSGGSSGSETPGTSESPTPESSGGSSGGSAKNTITKTLKLRIVRPYNSAEVEKIVADEKNNREKIALEKNKDKVREACSEHLKVAAYCTTQVERNACLFCKARKLDDKFYQKLRGQFPDAVFWQEIGEIFRQLQKQAAEIYNQSLIELYYEIFIKGRGFANASSVEHYLSDVCYTRAAELFKNAAIASGLRGKVKSNFRLKELKNMKSGLPTTKSDNFPIPLVKQKGGQYTGFEISSHNDDFIIKIPFGRWQVRKEIDKYRPWEKFNFEQVRKSPKPISLLLSTQRRKRNKGWSKDEGTEAEIRKAMNGDYQTSYIEVKRGSKIGEKSAWMLNLSIDVPKIDKGVDPSIIGGIDVGVKSPLVCAINNAFSRYSISDNDLFHFNKKMFARRRILLKKNRHKRAGHGAKNKLKPISILTEKSERFRKKLIEKWACEIADFFIKNKVGTVQMENLESMKRKEDSYFNIRLRGFWPYAEMQSKIEFKLKQYGIEIRKVAPNNTSKTCSKCGHLNNYFNFEYRKKNKFPHFKCEKCNFKENADYNAALNISNPKLKSTKEEP

SEQ ID NO: 2952 - protein, 726 aa, synthetic construct
SEVEFSHEYWMRHALTLAKRARDEREVPVGAVLVLNNRVIGVGWNRAIGLHDPTAHAEIMALRQGGLVMQNYRLIDATLYVTFEPCIMCAGAMIHSRISRVVFGVRNSKRGAAGSLMNVLNYPGMNHRVEITEGVLADECAALLCDFYRMPRQVFNAQKKAQSNINPGGSSGSSRGSETPGTSESAAPGSSGGGSSGSAKNTITKTLKLRIVRPYNSAEVEKIVADEKNNREKIALEKNKDKVKEACSEHLKVAAYCTTQVERNACLFCKARKLDDKFYQKLRGQFPDAVFWQELGEILRQLQKQAAEIYNQSLIELYYEIFIKGRGFANASSVEHYLSDVCYTRAAELFKNAAIASGLRGKVKSNFRLKELKNMKSGLPTTKSDNFPIPLVKQKGGQYTGFEISDHNSDFIIKIPFGRWQAKKEIDKYRPWEKFDFEQVRKSPKPISLLLSTQRRKKNRGWSKDEGTEAEIKKVMNGDYQTSYIEVKRGSKIGEKSAWMLSLSIDVPKIDKGVDPSIIGGIDVGVKSPLVCAISNAFSRYSISDNDLFHFNKKMFARRRILLKKSRHKRAGHGAKNKLKPITILTEKSRRFRKKLIERWACEIADFFIKNKVGTVQMENLESMKRREDSYFNIRLRGFWPYAEMQNKIEFKLKQYGIEIRKVAPNNTSKTCSKCSHLNNYFNFEYRKKNKFPLFKCEKCNFKENADYNAALNISSPKLKGTKEEP

SEQ ID NO: 2953 - protein, 726 aa, synthetic construct
SEVEFSHEYWMRRALTLAKRARDEREVPVGAVLVLNNRVIGVGWNRAVGLHDPTAHAEIIALRQGGLVMQNYRLIEATLYVTFEPCIMCAGAMIHSRIGRVVFGVRNSKRGAAGSLMNVLDYPGMGHRVEITEGILADECAALLCDFYCMPRQVFNAQKRAQSSINSGGSSGGSSGNETPGTSESATPESSGGGSSGSAKNTITKTLQLRIVRPYNSAEVEKIVADEKNNREKIALEKNKGKVKEACSKHLKVASYCTTQVERNACPFCKARKLDDKFYQKLRGQFPDAVFWQELGEILRQLQKQAAEIYNQSLIELYYEIFIEGRGFANASSVEHYLSDVCYTRAAELFKNAAIASGLRSKVRSNFRLKELKNMKSGLPTTKSDNFPIPLVKQKGGQYTGFEISSHNSDFIIKIPFGRWQEKEEIDKYRPWEKFDFEQVRRSPKPISLLLSTQRRKKNKGWSKDEGTEAEIRRVMNGDYQTSYIEVKRGSKIGEKSAWMLNLSIDVPKIDKGVDPSIIGGIDVGVKSPLVCAINNAFSRYSISDNDLFHFNKKMFARRRILLRKNRHKRAGHGARNKLKPITVLTEKSERFRKKLIERWACEIANFFIKNKVGTVQMENLESMKRKEDSYFNIRLRGFWPYAEMQNKIEFKLKQYGIEIRKVAPNNTSKTCSKCGHLNNYFNFEYRKKNKFPHFKCEKCNFKENADYNAALNISNPKLKSTKEEP

SEQ ID NO: 2954 - protein, 726 aa, synthetic construct
SEVEFSHEYWMRHALTLAKRARDEREVPVGAVLVLNNRIIGEGWNRAIGQHDPTAHAEIMALRQGGLVMQNNRLTDATLYVTFEPCVMCAGAMVHSRIGRVVFGVRNSKRGAAGSLMNVLNYPGVNHCVEITEGILVDECAALLCDFYRMPRQVLNAQKKARSSISSGGSSGGCSGSEMPGASESVTPKSSGGSSAGSTKNTITKTLKLRIVRPYNSAEVEKIVADEKNSREKIALERNKDKVKEACSEHLKVAAYCTTQVERNACLFCKARKLDDRFYQKLRGQFPDAVFWQETGEIFRQLQRQAAEIYNQSLIELYYEIFIKGKGFANASSVEHYLSDVCYTRAAELFKNAAIASGLRSKIKSNFRLKELRNMKSGLPTTKSDNFPIPLVKQKGGQCTGFEINNHNSDFIIKIPFGRWQVKKEIDKYRPWEKFDFEQVRKSPKPISLLLSTQRRKKNKGWSKDEGTEAEIRRVMNGDYQTSYIEVKRGSKIGEKSAWMLNLSIDVPKIDKGVDPSIIGGIDVGVKSPLVCAINNSSSRYSICDNDLFRFNKKMFARRRILLKKNRHKRAGHGAKNKLKPISILTGKSERFRKKLIERWACEIADFFIKNKVGTVQMENLESMKRKEDSYFNIRLRGFWPYAEMQNKIEFKLKQYGIEIRKVAPNNTSKTCSKCGHLNYYFNFEYRKRNKFPHFKCEKCNFKEDADYNAALNISNPKLKSTKEEP

SEQ ID NO: 2955 - protein, 726 aa, synthetic construct
SEVEFSHEYWMRHALTLAKRARDEREVPVGAILVLNNRVIGEGWNRAIGLHDPTAHAEIMALRQGGLVMQNYRLIDATLYVTFEPCVMCAGAMIHSRIGRVVFGVRNSKHGAAGSLVNVLNYPGMNHRVEITEGILADECAALLCDFYRMPRQVFNARKKAQSSINPGGSSGGSSGSETPGTSESATPESSGGSSGGSAKNTITKTLKLRIVRPYNSAEVEKIVADEKNNREKIALEKNKDKVKEACSKHLKVAAYCTTQVESNACLFCKARRLDGKFYQKLRGQFPDAVFWQEIGEIFRQLQKQAAEIYNQSLIELYYEIFIKGKGLANASSVEHYLSDVCYTRAAELFKNAAIASGLRGKVKSNFKLKELKSMKSGLPSTKSDNFPIPLVKQKGGQYTGFEISSHNDDLIIKIPFGRWQVKREIDKYRPWEKFDFEQVRKSPKPISLLLSTRRRKRNKGWSKDEGTEAEIRKVMNGDYQTSYIEVKRGSKIGEKSAWMLNLSIDVPKIDKGVDPSIIGGIDVGVKSPLVCAINNAFSRYSISDNDLFRFNKKMFARRRILLKKNRHKRAGHGARNKLKPITVLTEKSERFRKKLIERWACEIANFFIKNKVGTVQMENLESMKRRGDSYFNIRLRGFWPYAEMQSKIEFKLKQYGIKIRKVAPNNTSKTCSKCGHLNNYFNFEFRKKNKFPHFKCEKCNFKEDADYNAALNISNPKLKSTKEEP

SEQ ID NO: 2956 - protein, 726 aa, synthetic construct
SEDEFSHEYWMRHALTLAKRARDGHEVPVGAILVLNNRVIGEGWNRAIGLHDPTAHAEIMALRQGGLVMQNYRLIDATLYVTFEPCVMCAGAMIHSRIGRVVFGVRNNKHGAAGSLVNVLNYPGMNHRVEITEGILADECAALLCDFYRMPRQVFNARKKAQSSINPGGSSGGSSGSETPGTSESATPESSGGSSGGSAKNTITKTLKLRIVRPYNSAEVEKIVADEKDNREKIALEKNKGKVKEACSKHLEVAAYCTTQVERNACLFCKARKLDDKFYQKLRGQFPDAVFWQELGEIFRQLQKQAAEIYNQSLIELYYEIFIKGKGFANASSVEHYLSDVCYTRAAELFKNAAIASGLRGKVKGNFRLKELKSMKSGLPTTKSDNFPIPLVKQKGGQYTGFEISSHNDDFIIKIPFGRWQVKKEIDKYRPWEKFDFEQVRKSPKPISLLLSTQRRKRNKGWSKDEGTEAEIRKVMSGGYQTSYIEVKRGSKTGEKSAWMLNLSIDVPKIDRGVDPSIIGGIDVGVKSPLVCAINNALSRYSISDNDLFHFNKKMFARRRILLKKNRHKRAGHGAKNKLRPISILTEKSERFRKKLIEKWACEIADFFIKNKVGTVQMENLESMKRKEDSYFNIRLRGFWPYAEMQNKIEFKLKQYGIEIRKVAPYNTSKTCSKCGHLNNYFNFEYRKKNKFPHFRCEKCNFKENADYNAALNISNPKLKGTKEEP

SEQ ID NO: 2957 - protein, 726 aa, synthetic construct
SEVELGHEYWMRHALTLAKRARDEREVPVGAVLVLNNRVIGEGWNRTTGLHDPTAHAEIMALRQGGLVMRNYRLIDATLYVTFEPCVMCAGAMIHSRIGRVVFGVRNSKHGAAGSLVNVLNYPGMNHRVGITEGILADECAALLCDFYRMPRQVFNARKKAQSSINPGGSSGGSSGSETPGTSESATPESSGGSSGGSAKNTITKTLKLRIVRPYNSAEVEKIVADEKNNRERIALEKNKDKVKEACSKHLKVAAYCTTQVERNACLFCKARRLDDKFYQKLRGQFPDAVFWQEIGEIFRQLQKQAAETYNQSLIELYYEILIKGKGIANASRVEHYLSDVCYTRAAELFKNAAIASGLRNKIKSNFRLKELRNMKSGLPTTKSDNFPIPLVKQKGGQYTGFEISNHNSDFIIKIPFGRWQAKKEIDKYRPWEKFDFEQVRKSPKPISLLLSTQRRKRNKGWSKEEGTEAEIRKVMNGDYQTSYIEVKRGSKIGEKSAWMLNLSIDVPKIDKGVDPSIIGGIDVGVKSPLVCAINNAFSRYSISDNDLFHFNKKVFARRRILLKKNRHRRAGHGAKNKLKPITVLSEKSKRFRKKLIERWACEIADFFIKNKVGTVQMENLESMKRKEDSYFNIRLRGFWPYAEMQNKIEFKLKQYGIEIRKVAPNNTSKTCSKCGHLNNYFNFEYRKKNKFPHFKCEKCNFKENADYNAALNISNPKLKSTKEEP

SEQ ID NO: 2958 - protein, 726 aa, synthetic construct
SEVGFSHEYWMRHALTLAKRARDEREVPVGAVLVLNNRVIGEGWNRAIGLHDPTAHAEIMALRQGGLVMQNYRLSDATLYVTFEPCVMCAGAMIHSRIGRVVFGVRNSKRGAAGSLMNVLNYPGMNHCVEITEGILVDECAALLCDFYRMPRQVLNAQKKAQSSISSGGSSGGSNGSETPGASGSVTPKSSGGSSTGSTKNTITKTLKLRIVRPYNSAEVEKIVADEKNNREKIALEKNKDKVKEACSKHLKVAAYCTTQVERNACLFCKARKLDDKFYQKLRGQFPDAVFWQEIGEIFRQLQKQAAEIYNQSLIELYYEIFIKGRGFANASSVEHYLSDVCYTRAAELFKNAAIASGLRGKVKSNFRLKELKNMRSGLPTAKSDNFPIPLVKQKGGQYTGFEISSHNDDFIIKIPFGRWQVKKEIDKYRPWEKFDFEQVRKSPKPISLLLSTQRRKRNKGWSKDEGTEAEIRKVMNGDYQTSYIEVKRGSKTGEKSAWMLNLSIDVPKIDKGVDPCIIGGIDVGVKSPLVCAINNAFSRYSISDNDLFHFNKKMFARRRILLKENGHKRAGHGAKNKLKPLTIMTEKSKRFRKKLIERWACEIADFFIKNKVGTVQMENLESMKRKEDSYFNIRLRGFWPYAEMQNKIEFKLKQYGIVVKKVAPNNTSKTCSECGHLNNYFNFEYRKKNKFPHFKCEKCNFKENADYNAALNISNPKLKSTKGEP

SEQ ID NO: 2959 - protein, 726 aa, synthetic construct
SEVEFSHEYWMRHALTLAKRARDEREVPVGAVLVLNNRVIGEGWNRAIGLHDPTAHAEIMALRQGGLVMQNYRLTDATLYVTFEPCVMCAGAMIHSRIGRVVFGVHNSKRGAAGSLMNVLNYPGMNHCVEITEGILVDECAALLCDFYRMPRQVLNAQKKAQSSISSGGSSGGSSGSETPGASGSVTPKSSVGSSAGSTKNTITKTLKLRIVRPYNSAEVEKIVADEKNNREKIALEKNKDKVKEACSKHLKVAAYCTTQVERNACPFCKARRLDDKFYQKLRDQFPDAVFWREIGEIFRQLQKQAAEIYNQSLIELYYEILIKGKGFANASSVEHYLSDVCYTRAAELFKNAAIASGLRGKVKSNFKLKELKSMKSGLPTTKSDNFPIPLVKQKGGQYTGFEISSHHDDFIIKIPFGRWQVKKEIDKYRPWEKFDFEQVRKSPKPISLLLSTQRRKRNKGWSKDEGTEAEIKKVMNGDYQTSYIEVTRGSKIGEKSAWMLNLSIDVPKIDKGVDPSIIGGIDVGVKSPLVCAINNAFSRYSISDNDLFHFNKKMFARRRILLKKNGHKRAGHGAKNKLKPITILTEKSKRFRKKLIERWACEIADFFVKNKVGTVQMENLESMKRKEDSYFNIRLRGFWPYAEMQNKIEFKLKQYGIEIRKVAPNNTSKTCSKCGHLNNYFNFEYRKKNKFPHFKCEKCNFKENADYNAALNICNPKLKSTKEEP

SEQ ID NO: 2960 - protein, 726 aa, synthetic construct
SEVEFSHEYWMRHALTLAKRARDEREVPVGAVLVLNNRVIGEGWNRAIGLHDPTAHAEIMALRQGGLVMQNYRLIDATLYVTFEPCVMCAGAMVHSRIGRVVFGVRNSKRGAAGSLMNVLNYPGMSHCVEITEGILVDECAALLCDFYRMPRQVLNAQKRAQSSINPGGSSGGCSGSEMPGASESVTPKSSGGGSSGSAKNTFTKTLQLRIVRPYNSAEVEKIVADEKDNREKIALEKNKDKVREACSRHLKVASYCTTQVERNACPFCKARKLDDKFYQKLRGQFPDAVFWQELGEILRQLQKQAAEIYNQSLIELYYEIFIKGRGFANASSVEHYLSDVCYTRAAELFKNAAIASGLRGKVKSNFRLKELKNMKSGLPTTKSDNFPIPLVKQKGGQYTGFEISSHNDDFIIKIPFGRWQVKKEINKFRPWEKFDFEQVRKSPKPISLLLSTQRRKRNKGWSRDEGTEAEIRKVMNGDYQTSYIEVKRGSKIGEKSAWMLNLSIDVPKIDKGVDPSIIGGIDVGVKSPLVCAINNAFSRYSISDNDLFHFNKKMFARRRILLKKTRHKRAGHGAKNKLKPISILTEKSMRFRKKLIERWACEIANFFIRNRVGTVQMENLESMKRKEDSYFNIRLRGLWPYAEMQNKIEFKLKQYGIVIRKVAPNNTSKTCSKCGHLNNYFNFEYRKRNKFPHFKCEKCNFKENADYNAALNISNPKLKGTKEEP

SEQ ID NO: 2961 - protein, 726 aa, synthetic construct
SEVEFSHEYWMRHALTLAKRARDEREVPVGAVLVLNNRVIGEGWNRTTGLHDPTAHAEIMALRQGGLVMQNHRLVDATLYVTFEPCVMCAGAMIHSRIGRVVFGVRNSKRGAAGSLTNVLNYPGMNHRVEITEGILVDECAALLCDFYRMPRQVFNARKKAQSNIHPGGSSGSSSGSETPGTSESATPGSSCGSSGGSAKNTITKTLKLRIVRPYNSAEVEKIVADEKNSREKIALEKNKDKVKEACSEHLKVAAYCTTQVERNACLFCKARKLDDRFYQKLRGQFPDAVFWQEIGEIFRQLQKQAAEIYNQSLIELYYEIFIKGKGFAIASSVEHYLSCVCYTRAAELFKNAAIASGLRGKVKSNFRLKELKNMKSGLPTTKSDNFPIPLVKQKGGQYTGFEISSHNDDFIIKIPFGRWQVKKEIDKYRPWEKFDFEQVRKSPKPISLLLSTQRRKRNKGWSKDEGTEAEIRKVMNGDYQTSYIEVKRGSKTGEKSAWMLNLSIDVPKIDKGVDPTIIGGIDVGVKSPLVCAINNAFSRYSISDNDLFRFNKKMFARRRILLKKNRHKRAGHGAKNKLKPISILTGKGERFRKKLIERWACEIADFFIKNKVGTVQMENLESMKRKEDSYFNIRLRGFWPYAEMQNKIEFKLKQYGIEIRKVAPNNTSKTCSKCGHLNNYFNFEYRKKNKFPHFKCVKCNFKENADYNAALNISNPKLKNTKEEP

SEQ ID NO: 2962 - protein, 726 aa, synthetic construct
SEVEFSHEYWMRHALTLAKRARDEREVPVGAVLVLNNRVIGEGWNRAIGLHDPTAHAEIMALRQGGLVMQNYRLTDATLYVTFEPCVMCAGAMVHSRIGRVVFGVRNSKRGAAGSLMNVLNYPGVNHCVEITEGILVDECAALLCDFYRMPRQVLNAQKKAQSSISSGGSSDGSSGSETPGTSESATPESSGGGSSGSAKNTITKTLQLRIVRPYNSAEVEKIVADEKNNREKIALEKNKDKVKEACSEHLKVAAYCTTQVERNACLFCKARRLDDKFYQKLRGQFPDAVFWQETGEIFRQLQRQAAEIYNQSLIELYYEIFIKGRGFANASSVEHYLSDVCYTRAAELFKNAAIASGLRGKVKSNFRLKELKNMKSGLPTTKSDNFPIPLVRQKGGQYTGFEISSHNDDFIIKIPFGRWQAKKEIDKYRPWEKFDFEQVRKSPKPISLLLSTQRRKRNKGWSKDEGTEAEIRKVMNGDYQTSYIEVKRGSKIGEKSAWMLNLSIDVPKIDKGVDPSIIGGIDVGVQSPLVCAINNAFSRYSISDNDLFHFNKKMFARRRILLKKNGHKRAGHGAKNKLKPITIMTEKSRRFRKKLIERWACEIADFFIKNKVGTVQMENLESMKRKEDSYFNIRLRGFWPYAEMQNKIEFKLKQYGIEIRKVAPNNTSKTCSKCGHLNSYFNFEYRKKNKFPHFKCEKCNFKENADYNAALNISNPKLRSTKEEP

SEQ ID NO: 2963 - protein, 726 aa, synthetic construct
SEVEFSHEYWMRHALTLAKRARDEREVPVGAVLVLNNRAIGEGWNRTTGLHDPTAHAEIMALRQGGLVMQNHRLVDATLYVTFEPCVMCAGAMIHSRIGRVVFGVRNSKRGAAGSLTNVLNYPGMNHRVEITEGILVDECAALLCDFYRMPRQVFNAQKKAQSTINSGGSSGGSSGSETPGTSESPTPESSGGSPGGSAKNTITKTLKLRIVRPYNSTEVEKIVADEKNNREKIALEKNKDKVKEACSKHLKVASYCTTQVERNACPFCKARKLDDKFYQKLRGQFPDAVFWQELGGILRQLQKQAAEIYNQSLIELYYEIFIKGRGFANASSVEHYLSDVCYTRAAELFKNAAIASGLRGKVKSNFRLKELKNMKSGLPTTKSDNFPIPLVKQKGGQYTGFEICSHNDDFIIKIPFGRWQVKKEICKHRPWEKFDFEQVRKSPKPISLLLSTQRRKRNKGWGKDEGTEAEIRKVMNGDYQTSYIEVKRGSKTGEKSAWMLNLSIDVPKIDKGVDPSIIGGIDVGVKSPLVCAINNAFSRYSISDNDLFRFNKKMFARRRILLKKNRHKRAGHGARNKLKPITILTEKSVRFRKKLIERWACEIADFFIKNKVGTVQMENLESMKRKEDSYFNIRLRGFWPYAEMQNKIEFKLKQYGIVVRKVAPNNTSKTCSQCGHLNNYFNFEYRKKNKFPYFKCEKCNFKENADYNAALNISNPQLKSTKGEP

SEQ ID NO: 2964 - protein, 726 aa, synthetic construct
SEVEFSHEYWMRHALTLAKRARDEREVPVGAILVLNNRVIGEGWNRAIGLHDPTAHAEIMALRQGGLVMQNYRLIDATLYVTFEPCVMCAGAMIHSRIGRVVFGVRNNKHGAAGSLVNVLNYPGMDHRVEITGGILADECAALLCDFYRMPRQVFNAQKKAQSSINSGGSSGGSSGSETPGTSESATPESSGGSSGDSARNTITKTLQLRIVRPYNSAEVEKIVADEKNRREKIALEKNKDKVKEACSKHLMVASYCTTQVERNACLFCKARELDGKFYQKLRGQFPDAVFWQELGEILRQLQKQAAEIYNQSLIELYYEIFIKGRGFANASSVEHYLSDVCYTRAAELFKNAAIASGLRGKVKSNFRLKELKNMKSGLPTTKSDNFPIPLVKQKGGQYTGFEISSHNDDFIIKIPFGRWQVKKEINKYRPWEKFDFEQVRKSPKPISLLLSTQRRKRNKGWSKDEGTEAEIKKVMNGDYQTSYIEVKRGSKIGEKSAWMLNLSIDVPKIDKGVDPSIIGGIDVGVKSPLVCAINNAFSRYSISDNELFHFNKKMFARRRILLKKNRHKRAGHGAKNKLKPISILTEKSKRFRKKLIEKWACEIADFFIKNKVGTVQMENLESIKRKEDSYFNIRLRGFWPYAEMQNKIEFKLKQYGIEIRKVAPNNTSKTCSKCGHLNNYFNFEYRKKNKFPHFKCEKCNFKENADYNAALNISNPKLKSTKEGP

SEQ ID NO: 2965 - protein, 726 aa, synthetic construct
SEDEFSHEYWMRHALTLAKRARDGREVPVGAVLVLDNRVIGEGWNRAIGLHDPTAHAEIMALRQGGLVMQNYRLIDATLYVTFEPCVMCAGAMVHSRIGRVVFGVRNSKRGAAGSLMNVLDYPGMGHRVEITEGILADECAALLCDFYCMPRQVFNAQKRAQSSINSGGSSGGSSGSETPGTSENATPESSGGGSSGSAKNTITKTLQLRIVRPYNSAEVEKIVADEKNNREKIALEKNKDKVKEACSKHLKVASYCTTQVERNACPFCKARKLDDKFYQKLRGQFPDAVFWQELGEILRQLQKQAAEIYNQSLIELYYEIFIKGKGIVNASSVEHYLSDVCYTRAAELFKNAAIASGLRNKIKSNFRLKELRNMKSGLPTTKSDNFPIPLVRQKGGQYTGFEISNHNGDFIIKIPFGRWQVKKEIDKYRPWEKFDFAQVRKSPKPISLLLSTQRRKRNRGWSKDEGAEAEIKKVMNGDYQTSYIEVKRGSKTGEKSAWMLNLGIDVPKIDKGVDPSIIGGIDVGVKSPLVCAINNAFSRHSISDNDLFHFNKKMFARRRILLKKNRHKRAGHGTKNKLKPISILTEKSKRFRKKLIERWACEIADFFIKNKVGTVQMENLESMKRKEDSYFNIRLRGFWPYAEMQNKIEFKLKQYGIEIRKVAPNNTSKTCSKCGHLNNYFDFEYRKKNKFPHFKCEKCNFKENADYNAALNISNPKLKSTKEGP

SEQ ID NO: 2966 - protein, 726 aa, synthetic construct
SEVEFSHEYWMRHALTLAKRARDEREVPVGAVLVLNNRIIGEGWNRAIGLHDPTAHAEIMALRQGGLVMQNYRLTDATLYVTFEPCVMCAGAMVHSRIGRVVFGVRNSKRGAAGSLMNVLNYPGVNHCVEITEGILVDECAALLCDFYRMPRQVLNAQKKAQSSISSGGSSGGCSGSEMSGASESVTPKSSGGSSAGSTKNTITKTLKLRIVRPYNSAEVEKIVADEKNSREKIALERNKDKVKEACSEHLKVAAYCTTQVERNACLFCKARKLDDRFYQKLRGQFPDAVFWQETGEIFRQLQRQAAEIYNQSLIELYYEILIKGKGFANASSVEHYLSDVCYTRAAELFKNAAIASGLRGKVKSNFRLKELRNMKSGLPTTKSDNFPIPLVRQKGGQYTGFEISNHNSDFIIKIPFGRWQAKKEIDKYRPWEKFDFEQVRKSPKPISLLLSTQRRKRNRGWSKDEGTEAEIRKVMNGDYQTSYIEVKRGSKIGEKSAWMLNLSIDVPKIDKGVDPSIIGGIDVGVRSPLVCAINNAFSRYSISDNDLFHFNKKMFARRRILLKKSKHKRAGHGAKNKLKPITILTEKSGRFRKKLIERWACEIADFFIKNKVGTVQMENLESMKRKEDSYFNIRLRGFWPYAEMQNKIEFKLKQYGIEIRKVAPNNTSKTCSKCGHLNNYFNFEYRKKNKFPHFKCERCNFKENADYNAALNISNPKLKGTKEEP

SEQ ID NO: 2967 - protein, 726 aa, synthetic construct
SEDEFSHEYWMRHALTLAKRARDGREVPVGAVLVLNNRVIGEGWNRAIGLHDPTAHAEIMALRQGGLVMQNYRLIDATLYVTFEPCVMCAGAMVHSRIGRVVFGVRNSKRGAAGSLMNVLDYPGMNHRVEITEGILADECAALLCDYYRMPRQVFNARKKAQSSINSGGSSDGGSGSETPGTSESATPESSGGSSGGSAKNTITKALKLRIVRPYNSAEVEKIVADEKNNRERIALEKNKDKVKEACSKHLKVAAYCTTQVERNACLFCKARKLDDKFYQKLRGQFPDAVFWQEIGEIFRQLQKQAAEIYNQSLIELYYEIFIKGKGFANASSVEHYLSDVCYTRAAELFKNAAIASGLRGKVKSNFRLKELKNMRSGLPTTKSDNFPIPLVKQKGGQYAGFEISSHNDDFIIKIPFGRWQVKKEINKHRPWEKFDFEQVRKSPKPISLLLSTQRRKRNKGWGKDEGTEAEIRKVMNGDYQISYIEVKRGSKIGEKSAWMLNLSIDVPKIDKGVDPSIIGGIDVGVKSPLVCAINNAFGRYSISDNDLFRFNKKVFARRRILLKKNRHKRAGHGTKNKLKPITILTEKSGRFRKKLIERWACEIANFFIKNKVGTVQMENLESMKRKEDSYFNIRLRGFWPYAEMQNKIEFKLKQYGIKIRKVAPNNTSKTCSKCGHLNNYFGFEYRKKNKFPHFKCEKCNFKEDADYNAALNISNPKLKSTKEEP

SEQ ID NO: 2968 - protein, 726 aa, synthetic construct
SEVEFSHEYWMRHALTLAKRARDEREVPVGAILVLNNRVIGEGWNRAIGLHDPTAHAEIMALRQGGLVMQNYRLVDATLYVTFEPCVLCAGAMVHSRIGRVVFGARNSKRGAAGSLMNILNYPGMNHRVEITEGILADECAALLCDFYRMPRQVFNAQKKAQSSINSGGSSGGSSGSETPSTSESATPESSGGSSGGSAKNTITKTLQLRIVRPYNSAEVEKIVADEKSNREKIALEKNKDKVKEACSKHLKVAAYCTTQVERNACLFCKARKLDDKFYQKLRGQFPDAVFWQETGEIFRQLQRQAAEIYNQSLIELYYEIFIKGKGFANASSVEHYLSDVCYTRAAERFKNAAIASGLRGKVKSNFRLRELKNMKSGLPTTKSDNFPIPLVKQKGGQYTGFEISSHNDDFIIKIPFGRWQVKKEIDKYRPWEKFDFEQVRKSPKPISLLLSTQRRKRNKGWSKDEGTEAEIRKVMNGDYQTSYIEVKRGSKIGEKSAWMLSLSIDVPKIDKGVDPSIIGGIDVGVKSPLVCAINNALSRYSISDNDLFHFNKKMFARRRILLKKNRHKRAGHGAENKLKPISILTGKGERFRKKLIERWACEIADFFIKNKVGTVQMENLESMKRKEDSYFNIRLRGFWPYAEMQNKIEFKLKQYGIEIRKVAPNNTSKTCSKCGHLNNYFNFEYRKKNKFPHFKCEKCNFKENADYNAALNISNPKLKSTKEEP

SEQ ID NO: 2969 - protein, 725 aa, synthetic construct
SEVEFSHEYWMRHALTLAKRARDEREVPVGAVLVLNNRVIGVGWNRAVGLHDPTAHAEIMALRQGGLVMQNYRLVEATLYVTFEPCIMCAGAMVHSRIGRVVFGVRNSKRGAAGSLMNVLNYPGMNHRVEITEGILADECAALLCDFYRMPRQVLNAQKKAQSSISSGGSSGGSSGSETPGASGSVTPKSSGGSSAGSTKDTITKTLKLRIVRPYNSAEVEKVVADEKNNREIALEKNKDKVKEACSKHLKVAAYCTTQVERNACLFCKARKLDDKFYQKLRGQFPDAVFWQEIGEIFRQLQKQAAEIYNQSLIELYYEIFIKGKGFANASSVEHYLSDVCYTRAAELFKNAAIASGLRGKVKSNFRLKELKNMKSGLPTTKSDNFPIPLVKQKGGQYTGFEISSHNDDFIIKIPFGRWQVKKEIDKYRPWEKFDFEQVRKSPKPISLLLSTQRRKRNKGWSKDEGTEAEIRKVMNGDYQTSYIEVKRGSKTGEKSAWMLNLSIDVPKIDKGVDPSIIGGIDVGVKSPLVCAINNAFSRHSISDNDLFRFNKKMFARRRILLKKNRHKRAGHGAKNKLKPISILTGKSERFRKKLIERWACEIADFFIKNKVGTVQMENLESMKRKEDSYFNIRLRGFWPYAEMQNKIEFKLKQYGIGIRKVAPNNTSKTCSKCGHLNNYFNFEYRRKNKFPHFKCEKCNFKEDADYNAALNISNPKLKSTKEEP

SEQ ID NO: 2970 - protein, 726 aa, synthetic construct
SEDEFSHEYWMRHALTLAKRARDGREVPVGAVLVLNNRVIGEGWNRAIGLHDPTAHAEIMALRQGGLVMQNYRLIDATLYVTFEPCVMCAGAMIHSRIGRVVFGVRNNKHGAAGSLVNVLNYPGMNHRVEFTEGILADECAALLCDFYRMPRQVFNARKKAQSSISPGGSSGSSSGSETPGSNESATPESSGGGSSGSAKNTITKTLQLRIVRPYNSAEVEKIVADEKNNREKIALEKNKDKVKEACSKHLKVASYCTTQVERNACLFCKARKLDDKFYQKLRGQFPDAVFWQEIGEIFRQLQKQATEIYNRSLIELYYEIFIKGKGIANASRVGHYLSDVCYTRAAELFKNAAIASGLRNKIKSNFRLKELKNMKSGLPTTKSDNFPIPLVKQKGGQYTGFEISNHNGDFIIKIPFGRWQVKKEVDKYRPWEKFDFEQVRKSPKPISLLLSTQRRKRNKGWSKDEGTEAEIRKVMNGDYQTSYIEVKRGSKTGEKSAWMLNLSIDVPKIDKGVDPSIIGGIDVGVKSPLVCAINNALSRYSISDNDLFHFNKKMFARRRILLRKNRHKRAGHGAKNKLKPITIMTEKSKRFRKKLIERWACEIADFFIKNKVGTVQMENLESMKRREDSYFNIRLRGFWPYAEMQNKIEFKLKQYGIVVRKVAPNNTSKTCSKCGHLNNYFNFEYRKKNKFPHFKCEKCNFKEDADYNAALNISNPKLKSTKGEP

SEQ ID NO: 2971 - protein, 726 aa, synthetic construct
SEVEFSHEYWMRHALTLAKRARDEREVPVGAVLVLNNRVIGEGWNRAIGLHDPTAHAEIMALRQGGLVMQNYRLVNATLYVTFEPCVMCAGAMIHSRIGRVAFGVRNSKRGAAGSLMNVLNYPGMNHRVEITEGILAGECAALLSDFYRMPRQVFNAQKKARSYINSGGSSGGSSGSGTPGTSESPTPESSGGSSGGSAKNTITKTLKLRIVRPYNSAEVEKIVADEKNNREKIALEKNKDKVKEACSKHLKVAAYCTTQVERNACLFCKARKLDDKFYQKLRGQFPDAVFWQEIGEIFRQLQKQAAEIYNQSLIELYYEIFIKGRGFANASSVEHYLSDVCYTRAAELFKNAAIASGLRGKVKSNFRLKELKNMKSGLPTTKSDNFPIPLVKQKGGRYTGFEISSHNDDFIIKIPFGRWQVKKEIDKYRPWEKFDFEQVRKCPKPISLLLSTQRRKRNKGWSKDEGTEAEIRKVLNGDYQTSYIEVKRGSKIGEKSAWMLSLSIDVPKIDKGVDPSIIGGIDVGVKSPLVCAINNAFCRYSISDNDLFHFNKKMFARRRILLKKSRHKRAGHGAKNKLKPISILTEKSKRFRKKLIERWACEIADFFIKNKVGTVQMENLESMKRKEDSYFNIRLRGFWPYAEMQNKIEFKLKQYGIEIRKVAPNNTSKTCSKCGHLNNYFNFEYRKKNKFPHFKCEKCNFKEIADYNAALNISNPKLKSTKEEP

SEQ ID NO: 2972 - protein, 726 aa, synthetic construct
SEVVFSHEYWMRHALSLAKRARDEREVPVGAVLVLNNRIIGEGWNRAIGLHDPTAHAEIMALRQGGLVMQNYRLVEATLYVTFEPCIMCAGAMIHSRIGRVVFGVRNSKRGAAGSLMNVLSYPGMNHRVEITEGILADECAALLCDYYRMPRQVFNARKKAQSSINPGGPSGGSSGSETPGASESVTPKSSGGSSGGSAKNTITKTLKLRIVRPYNSAEVEKIVADEKNNREKIALEKNKGKVKEACSKHLEVAAYCTTQVERNACLFCKARKLDDKFYQRLRGQFPDAVFWQELGEIFRQLQKQAAEIYNQSLIELYYEIFIKGKGFANASSVEHYLSDVCYTRAAELFKNAAIASGLRGKVKSNFRLKELKNMKSGLPTTKSDNFPIPLVKQKGGQYTGFEISDHNSDFIIKIPFGRWQAKKEIDKYRPWEKFDFEQVRKSPKPISLLLSTQRRRGNKGWSKDEGTEAEIRRVMNGDYQASYIEVKRGSKIGEKSAWMLNLSIDVPKIDKGVDPSIIGGIDVGVKSPLVCAVNNVLSRYSISDNDLFHFNKKMFARRRILLKKNGHKRAGHGAKNKLKPITIMTEKSRRFRKKLIERWACEIADFFIKNKVGTVQMENLESMKRKEDSYFNIRLRGFWPYAEMQNKIEFKLKQYGIEIRKVAPNNTSKTCSKCGHLNSYFNFEYRKKNKFPHFKCEKCNFKEDADYNAALNISNPKLKSTKEEP

SEQ ID NO: 2973 - protein, 726 aa, synthetic construct
SEVEFSHEYWMRHALTLAKRARDEREVPVGAVLVLNNRVIGEGRNRAIGLHDPTAHAEIMALRQGGLVMQNYRLTDATLYVTFEPCVMCAGAMIHSRIGRVVFGVRNSKRGAAGSLMNVLNYPGMNHCVEITEGILVDECAALLCDFYRMPRQVLNAQKKARSCINSGGSSGGSSGSETPGTSESATPESSGGGSSGSAKNTITKTLQLRIVRPYNSAEVEKIVADEKNNREKIALEKNKDKVKEACSKHLKVASYCTTQVERNACPFCKARKLDDKFYQKLRGQFPDAVFWQELGEILRQLQKQAAEIYNQSLIELYYEIFIKGKGFANASSVEHYLSDVCYTRAAELFKNAAIASGLRGKVKSNFRLKELKNMKSGLPTTKSDNFPIPLVKQKGGQYTGFEISSHNDDFIIKIPFGRWQVKKEIDKYRPWEKFDFEQVRKSPKPISLLLSTQRRKRNKGWSKDEGTEAEIRKVMNGDYQTSYIEVKRGSKIGEKGAWMLNLSIDVPKIDKDVDPSIIGGIDVGVKSPLVCAIDNAFSRYSISDNDLFHFNKKMFARRRILLKKNRHRRAGHGAKNKLKPIAVLAKKSEGFRKKLIERWACEVADFFIKNKVGTVQMENLEGMKRKEDSYFNIRLRGFWPYAEMQNRIEFKLKQYGIEIRKVAPNNTSRTCSKCGHLNNYFNFEYRKKNKFPHFKCEKCNFREDADYNAALNISNPKLKSTKEEP

SEQ ID NO: 2974 - protein, 726 aa, synthetic construct
SEVEFSHEYWMRHALTLAKRARDEREVPVGAVLVLNNRVIGEGWNRAIGLHDPTAHAEIMALRQGGLVMQNHRLIDATLYVTFEPCVMCAGAMVHSRIGRVVFGVRNSKRGAAGSLTNVLDYPGMGHRVEITEGILADECAALLCDFYCMPRQVFNAQKRAQPSINSGGSSGDSSGSETPGTSESATPESFGGGSSGSAKNTITKTLQLRIVRPYNSAEVEKIVADEKNNREKIALEKNKDKVKEACSKHLKVAAYCTTQVERSACLFCKARKLDDKFYQKLRGQFPDAVFWQEIGEIFRQLQKQAAEIYNQSLIELYYEIFIKGKGFANASSVEHYLSDVCYSRAAELFKNAAIASGLRGKVKSNFKLKELKSMKSGLPTTKSDNFPIPLVKQKGGQYTGFEISSHNDDFIIKIPFGRWQVRKEIDKYRPWEKFNFEQVRKSPKPISLLLSTQRRKRNRGWSKDEGTEAEIRKVMNGDYQTSYIEVKRGSKIGEKSAWMLSLSIDVPKIDKGVDPSIIGGIDVGVKSPLVCAINNAFSRYSISDNELFHFNKKMFARRRILLKKNRHRRAGHGARNKLKPITVLTEKSERFRKKLIERWACEIADFFIRNKVGTVQMENLEGMKRKEDSYFNIRLRGFWPYAEMQNKIEFKLKQYGIEVRKVAPNNTSKTCSKCGHLNNYFNFEYRKKNKFPHFKCEKCNFKENADYNAALNISNPKLKSTKEEP

SEQ ID NO: 2975 - protein, 726 aa, synthetic construct
SEVEFSHEYWMRHALTLAKRARDEREVPVGAVLVLNNRVIGEGWNRAIGLHDPTAHAEIMALRQGGLVMQNYRLVDATLYVTFEPCVLCAGAMIHSRIGRVVFGVRNSKRGAAGSLMNVLNYPGMNHRVEITEGILADECAALLCDFYRMPRQVFNARKKARSNINSGGSSGGSSGSETLGTREGATPESTGGSSGGSAKSTITKTLKLRIVRPYNSAEVEKIVVDEKNSREKIAVEKNKDKVKEACSKHLKVASYCTTQVERNACLFCKARKLDDKFYQKLRGQFPDAVFWQELGGIFRQLQKQAAEIYNQSLIELYYEIFIKGKGITNASRVEHYLSDVCYTRAAELFKNAAIASGLRSKVRSNFRLKELKNMKSGLPTTKSDNFPIPLVKQKGGQYTGFEISSHNCDFIIKIPFGRWQEKEEIDKYRPWEKFDFGQVRKSPKPISLLLSTQRRKKNKGWSKDEGTEAEIRRVMNGDYQTSYIEVKRGSKIGEKSAWMLNLSIDVPKIDKGVDPSIIGGIDVGVKSPLVCAINNAFSRYSISDNDLFHFNKKMFARRRILLKKNRHRRAGHGAKNKLKPIAILTEKSERFRKKLIERWACEIANFFIKNKVGTVQMENLESMKRREDSYFNIRLRGFWPYAEMQSRIEFKLRQYGIKIRKVAPNNTSKTCSKCGHLSNYFNFEFRKKNKFPHFKCEKCSFKEDADYNAALNISNPKLKGTKEEL

SEQ ID NO: 2976 - protein, 726 aa, synthetic construct
GEVEFSHEYWMRRALTLAKRARDEREVPVGAILVLNNRVIGEGWNRAIGLHDPTAHAEITALRQGGLVMQNYRLIDATLYVTFEPCVMCAGAMIHSRIGRVVFGARNSKRGAAGSLMNVLSYPGMNHRVEITEGILADECAALLCDFYRMPRQVFNARRKAQPSINPGGSSGGSSGSETPGTSESATPESSGGNSGGSAKNTITKTLKLRIVRPYNSAEVEKIVADEKNNREKIALEKNKDKVKEACSKHLKVAAYCTTQVERNACLFCKARRLDDKFYQKLRGQFPDAVFWQEIGEIFRQLQKQAAEIYNQSLIELYYEIFIKGKGFANASSVEHYLSDVCYTRAAELFKNAAIASGLRGKVKSNFRLKELKNMRSGLPTTKSDNFPIPLVKQKGGQYTGFEISSHNDDFIIKIPFGRWQVKKEIDKYRPWEKFNFEQVRKSPKPISLLLSTQRRKRSKGWSKDEGTEAEIRKVMNGDYQTSYIEVKRGSKIGEKSAWMLNLSIDVPKIDKGVDPSIIGGIDVGVKSPLVCAINNAFSRYSISDNDLFRFNKKMFARRRILLGKNRHKRAGHGVKNKLKPITILTEKSGRFRKKLIERWACEIADFFIKNKVGTVQMENLESMKRKEDSYFNIRLRGFWPYAEMQNKIEFKLKQYGIVVRKVAPNNTSMTCSECGHLNNYFNFEYRKKNKFPHFKCEKCNFKENADYNAALNISNPKLKSTKGEP

SEQ ID NO: 2977 - protein, 726 aa, synthetic construct
SEVEFSHEYWMRHALTLAKRARDGREVPVGAVLVLNNRVIGEGWNRAIGLHDPTAHAEIMALRQGGLVMQNYRLIDATLYVTFEPCVMCAGAMVHSRIGRVVFGVRNSKRGAAGSLMNVLDYPGMGHRVEITEGILADECAALLCDFYCMPRQVFNAQKRAQSSINSGGSSGGSSGSETPGTSESATPGSFGGGSSGSARNTITKTLQLRIVRPYNSAEVEKIVADEKNNREKTALEKNKGKVKEACSEHLKVAAYCTTQVERNACLFCKARKLDDKFYQKLRGQFPDAVFWQEISEILRQLQKQAAEIYNQSLIGLYYEIFIKGKGIANANGVEHYLSDVCYTRAAELFRNAAIASGLRSKVKSNFRLKELKNMKSGLPTTKSDNFPIPLVKQKGGQYTGFEISNHNSDFIIKIPFGRWQVKKEIDKFRPWEKFDFEQVRKSPKPISLLLSTQRRKRNKGWGKDEGTEAEIKKVMNGDYQTSYIEVKRSSKIGEKGAWMLSLSIDVPKIDKGVDPSIIGGIDVGVKSPLVCAINNAFSRYSISDNDLFHFNKKMFARRRILLKKNRHKRAGHGAKNKLKPISILTERSKRFREKLIERWACEIANFFIKNKVGTVQMENLESMKRKEDSYFNIRLRGFWPYAEMQNKIVFKLKQYGIEIRKVAPNNTSKTCSKCGHLNNYFNFEYRKKNKFPHFKCEKCNFKENADYNAALNISNPKLKSNKEEA

SEQ ID NO: 2978 - protein, 726 aa, synthetic construct
SEVEFSHEYWMRHALTLAKRARDEREVPVGAVLVLNNRVIGEGWNRAIGLHDPTAHAEIMALRQGGLVMQNHRLVDATLYVTFEPCVLCAGAMVHSRIGRVVFGVRNSKRGAAGSLMNVLSYPGMNHRVEITEGILADECAALLCDFYRMPRQVFNAQKKARSNINSGGSSGGSSGSETPGTSESATPESSGGGFGGSAKNTITKTLQLRIVRPYNSAEVEKIVADEKNNREKIALEKNKDKVKEACSKHLKVASYCTTQVERNACLFCKARKLDDKFYQKLRGQFPDAVFWQEIGEIFRQLQKQAAEIYNQSLIELYYEIFIKGKGFANASSMEHHLSDVCYARAAELFKNAAIASGLRGKVKSNFRLKELKNMRSGLPTTKSDNFPIPLVKQKGGQYTGFEISSHNDDFIIKIPFGRWQVKKEIDKYRPWEKFDFEQVRKNPKPISLLLSTQRRKRNKGWSKDEGTEAEIRKVMNGDYQTSYIEVKRGSKIGEKSAWMLNLSIDVPKIDKGVDPSIIGGIDVGVKSPLVCAINNAFSRYSICDNDLFRFNKKMFARRRILLKKNRHKRAGHGAKNKLKPITILTKKSERFRKKLIERWVCEVADFFIKNKVGTVQMENLESMKRKEDSYFNIRLRGFWPYAEMQNRIEFKLKQYGIEIRKVAPNNTSKTCSKCGHLNNYFNFEYRKKNKFPHFKCEKCNFKENADYNAALNISNPKLKSTKEEP

SEQ ID NO: 2979 - protein, 726 aa, synthetic construct
SEVEFSHEYWMRHALTLAKRARDEREVPVGAVLVLNDRVIGEGWNRAIGLHDPTAHAEIMALRQGGLVTQNYRLINATLYVTFEPCAMCAGAMVHSRIGRVVFGVHNSKRGAAGSLMNVLNYPGMDHRVEITGGILADECAALLCDFYRMPRRVFNAQKKAQSSINSGGSSGGSSGSVTPGTSESATPESSGGSSAGSTKDTITKTLKLRIVRPYNSAEVEKVVADEKNNREKIAIEKYKDMVKEACSKHLKVASYCTTQVERNACLFCKARKLDDKFYQKLRGQFPDAVFWQELGGIFRQLQKQAAEIYNQSLIELYYEIFIKGKGITNASRVEHYLSDVCYTRAAELFKNAAIASGLRSKVRSNFRLKELKNMKSGLPTTKSDNFPIPLVKQKGGQYTGFEISSHNSDFIIKIPFGRWQEKEEIGKYRPWEKFDFEQVRRSPKPISLLLSTQRRKKNKGWSKDEGTEAEIRRVMNGDYQTSYIEVKRGSKIGEKSAWMLNLSIDVPKIDKGVDPSIIGGIDVGVKSPLVCAIYNAFSRYSISDNDLFHFNKKMFARRRILLKKNRHKRAGHGAKNKLKPISILTEKSKRFRKKLIERWACEIAGFFIKNKVGTVQMENLESMKRKEDSYFNIRLRGFWPYAEMQNKVEFKLKQYGIEIRKVAPNNTSKTCSKCGHLNNYFNFEYRKKNKFPHFKCEKCNFKENADYNAALNISNPKLKSTKEEP

SEQ ID NO: 2980 - protein, 726 aa, synthetic construct
SEVEFSHEYWMRHALTLAKRARDEREVPVGAILVLNNRVIGEGWNRAIGLHDPTAHAEIMALRQGGLVMQNYRLIDATLYVTFEPCVMCAGAMIHSRIGRVVFGVRNNKHGAAGSLVNVLNYPGMNHRVEITEGILADECAALLCDFYRMPRQVFNARKKAQSSINPGGSSGGSGGSETPGTSESATPENSGGSSGSSAKNTITKTLKLRIVRPYNSAEVEKIVADEKNNREKIALEKNKDKVKEACSKHLKVAAYCTTRVDRNACLFCKARRLDDKFYQKLRGQFPDAVFWQEIGEIFRQLQKQAAEVYNQSLVELYYEIFIKGKGIANASSVGHYLSDVCYTRAAELFKNAAIASGLRSKVRSNFRLKELKNMKSGLPTTKSDNFPIPLVKQKGGQYTGFEISSHNDDFIIKIPFGRWQAKKEIDKYRPWEKFDFEQVRKSPKPISLLLSTQRRKRNRGWSKDEGTEAEIKKVMNGDYQTSYIEVKRGSKIGEKSAWMLNLSIDVPKIDKGVDPSIIGGIDVGVKSPLVCAISNAFSRYSISDNDLFHFNKKMFARRRILLKKNRRRRAGHGAKSKLKPITILTEKSVRFRKKLIERWACEIADFFIKNKVGTVQMENLESMKRKEDSYFNIRLRGFWPYAEMQNKIEFKLKQYGIEIRKVAPNNTSKTCSKCGHLNNYFNFEYRRKNKFPHFKCEKCNFKEDADYNAALNISNPKLKSTKGEP

SEQ ID NO: 2981 - protein, 726 aa, synthetic construct
SEVEFSHEYWMRHALTLAKRARDEREVPVGAILVLNNRVIGEGWNRAIGLHDPTAHAEIMALRQGGLVMQNYRLIDATLYVTFEPCVMCAGAMIHSRIGRVVFGVRNNKHGAAGSLVNVLNYPGMNHRVEITEGILADECAALLCDFYRMPRQVFNARKKAQSSINPGGSSGGSSGSETPGTSESATPESSGGSSGSSAKNTITKTLKLRIVRPYNSAEVEKIVADEKNNREKIALEKHKDKVKEACSKHLKVAAYCTTQVERNACLFCKARRLDDKFYQKLRGQFPDAVFWQEIGEIFRQLQKQAAEVYNQSLVELYYEILIKGKGIANASSVEHYLSDVCYTRAAELFKNAAIASGLRNKIKSNFRLKELRNMKSGLPTTKSDNFPIPLVRQKGGQYTGFEISNHDGDFIIKIPFGRWQVKKGINKHRPWEKFDFEQVRKSPKPISLLLSTQRRKRNKGWSKDEGTEAEIRKVMNGDYQTSYIEVKRGSKIGEKSAWMLNLSIDVPKIDKGVDPSIIGGIDVGVKSPLVCAINNALSRYSISDNDLFHFNKKMFARRRILLRKNRHKRAGHGAKNKLKPITIMTEKSKRFRMKLIERWACEIADFFIKNKVGTVQMENLESMKRKEDSYFNIRLRGFWPYAEMQNKIEFKLKQYGIVVRKVAPNNTSKTCSKCGHLNNYFNFEYRKKNKFPHFKCEKCNFKEDADYNAALNISNPKLKSTKGEP

SEQ ID NO: 2982 - protein, 726 aa, synthetic construct
SEVEFSHEYWMRHALTLAKRARDEREVPVGAVLVLNNRVIGEGWNRAIGLHDPTAHAEIMALRQGGLVMQNHRLIDATLYVTFEPCVLCAGAMVHSRIGRVVFGVRNSKRGAAGSLMNVLNYPGMNHRVEITEGVLADECAALLCDFYRMPRQVFNAQKKAQSSINSGGSSGGSSGSETPGTSESATPESSGGGSSGSAKNTITKTLQLRIVRPYNSAEVEKIVTDEKNNREKIALEKNKDKVKEACSKHLKMASYCTTQVERNACLFCKARKLDDKFYQKLRGQFPDAVFWQELGEILRQLQKQAAEIYNQSLIELYYEIFIKGRGFANASSVEHYLSDVCYTRAAELFKNAAIASGLRGKVKSNFRLRELKNMKSGLPTTKSDNFPIPLVKQKGGQYTGFEISSHNDDFIIKIPFGRWQVKEEIDKYRPWEKFDFEQVRKNPKPISLLLSTQRRKRNKGWSKDEGTEAEIRKVMNGDYQTSYIEVKRGSKIGEKSAWMLNLSIDVPKIDKGVDPSIVGGIDVGVKSPLVCAINNSFSRYSICDNDLFRFNKKMFARRRVLLKKNRHKRAGHGAKNKLKPITILTKKSERFRKKLIERWVCEVADFFIKNKVGTVQMENLESMKRKEDSYFNIRLRGFWPYAEMQNRIELKLKQYGIEIRRVAPNNTSRTCSKCGHLNNYFNFEYRKKNKFPHFKCEKCNFKENADYNAALNISNPKQKSTKEEP

SEQ ID NO: 2983 - protein, 726 aa, synthetic construct
SEVEFSHEYWMRHALTLAKRARDEHEVPVGAVLVLDNRVIGEGWNRAIGLHDPTAHAEIMALRQGGLVMQNYRLVNATLYVTFEPCVMCAGAMIHSRIGRVAFGVRNSKRGAAGSLMNVLNYPGMNHRVEITEGILAGECAALLCDFYRMPRRVFNAQKKAQSNINSGGLSGGSSGSETPGASESVTPKSSGGSSAGSTKNTITKTLKLRIVRPYNCAEVEKIVADEKNNREKIALEKNRDKVKEACSKHLKVAAYCTTQVERNACLFCKARKLDDKFYQKLRGQFPDAVFWQEVGGIFRQLQKQAAEIYNQSLIELYYEIFIKGKGFANASSVEHYLSDVCYTRAAELFKNAAIASGLRGKVKSNFRLKELKNMKSGLPTTKSDNFPIPLVKQKGGQYTGFEISSHSDDFIIKIPFGRWQVKEEIDKYRPWEKFDFEQVRKSPKPISLLLSTQRRKRNKGWSKDEGTEAEIRKVMNGDYQTSYIEVKRGSKTGEKSAWMLNLSIDVPKVDKGVDPSIIGGIDVGVKSPLVCAINNAFSRYSISDNDLFHFNKKMFARRRILLKKNRHKRAGHGAKNKLKPISILTEKSKRFRKKLIERWACEIADFFIKNKVGTVQVENLESMKRKEDSYFNIRLRGFWPYAEMQNKIEFKLRQYGIEIRKVAPNNTSKTCSKCGHLNNYFNFEYRKMNKFPHFKCEKCNFKENADYNAALNISNPKLKSTKEEP

SEQ ID NO: 2984 - protein, 726 aa, synthetic construct
SEVEFSHEYWMRHALTLAKRARDEREVPVGAVLVLNNRAIGEGWNRAIGLHDPTAHAEIMALRQGGLVMQNYRLIDATLYVTFEPCVMCAGAMIHSRIGRVVFGVRNSKRGAAGSLMNVLNHPGMNHRVEITEGILAGECAALLCDFYRMPRQVFNAQKKAQSTINSGGSSGGSSSSETPGTSGSATPEGSGGSSGGSAKNTITKTLKLRIVRPYNSAEVEKIVADEKNNREKIALEKNKDKVKEACSKHLKVASYCTTQVERNACLFCKARKLDDKFYQKLRGQFPDAVFWQELGEIFRQLQKQAAEIYNQSLIELYYEIFIKGKGFANASSVEHYLSDVCYTRAAELFKNAAIASGLRGKVKSNFRLKELKNMKSGLPTTKSDNFPIPLVKQKGGQYTGFEISSHNDDFIIKIPFGRWQVKKEIDKYRPWEKFDFGQVRKSPKPISLLLSTQRRKRNKGWSKDEGTEAEIRKVMSGDYQTSYIEVKRGSKIGEKSAWMLNLSIDVPKIDKGVDPSIIGGIDVGVKSPLVCAINNAFSRYSISDNDLFHFNKKMFARRRILLKKTRHKRAGHGAKNKLKPISILTEKSERFRKKLIERWACEIADFFIKNKVGTVQMENLESMKRREDSYFNIRLRGFWPYAKMQNKIEFKLRQYGIEIRKVAPNNTSKTCSKCGHLNDYFNFEYRKKNKFPHFKCERCNFKENADYNAALNISNPKLKSTKEEP

SEQ ID NO: 2985 - protein, 726 aa, synthetic construct
SGVEFSHEYWMRHALTLAKRARDGREVPVGAVLVLNNRVIGEGWNRAIGLHDPTAHAEIMALRQGGLVMQNYRLPDATLYVTFEPCVMCAGAMIHSRIGRVVFGVRNSKRGAAGSLMNVLNYPGMNHCVEITEGILVDECAALLCDFYRMPRQVLSAQKKAQSGISSGGSSGGSSGCETPGASGSVTPKSSVGSSAGSTKDTITKTLKLRIVRPYNSAEVEKVVADEKNNREKIAMEKNKDKVKEACSKHLKVASYCTTQVERNACLFCKARKLDDKFYQKLRGQFPDAVFWQELGGIFRQLQKQAAEIYNQSLIELYYEIFIKGKGITNASRVEHYLSDVCYTRAAELFKNAAIASGLRSKVRSNFRLKELKNMKSGLPTTKSDNFPIPLVRQKGGQYTGFEISSRNDDFIIKIPFGRWQVKKEIDKYRPWEKFDFEQVRKSPKPISLLLSTQRRKRNRGWGKDEGTEAEIKRVMNGDYQTSYIEVKRGSKIGEKSAWMLNLSIDVPKIDKGVDPRIIGGIDVGVKSPLVCAINNAFSRYSISDNDLFHFNKKMFARRRILLKKNRHKRAGHGAKNKLKPITILTEKSVRFRKKLIERWACEIADFFIKNKVGTVQMENLESMKGKEDSYFNIRLRGFWPYAEMQNKIEFKLKQYGIEIRKVAPNNTSKTCSKCGHLNNYFSFEYRKKNKFPHFKCEKCNFKEDADYNAALNISNPKLKSTKEEP

SEQ ID NO: 2986 - protein, 726 aa, synthetic construct
SEVEFSHEYWMRHALTLAKRARDEREVPVGAILVLNNRVIGEGWNRAIGLHDPTAHAEIMALRQGGLVMQNYRLIDATLYVTFEPCVMCAGAMIHGRIGRVVFGVRNSKHGAAGSLMNVLNYPGMNHRVEITEGILADECAALLCDFYRMPRQVFSARKKAQSSINSGGSSGGSSGSETPGTSESATPESSGGSPGGSAKNTITKTLKLRIVRPYNSAEVEKIVADEKDNREKIALEKNKDKVKEACSKHLKVAAYCTTQVERNACLFCKARKLDDKFYQKLRGQFPDAVFWQEIGEIFRQLQKQAAEIYNQSLIELYYEIFIKGKGFANASSVEHYLSDVCYTRAAEQFKNAAIASGLRGKVKSNFRLKELKNMKSGLPTTKSDNFPIPLVKQKGGQYTGFEISNHNSDFIIKIPFGRWQVKKEIDRYRPWERFDFEQVRKSPKPISLLLSTQRRKRNKGWSKDEGTEAEIKRVMSGDYQISYIEVKRGSKIGEKSAWMLNLSIDVPKIDKGVDPSIIGGIDVGVKSPLVCAIDNALSRYSISDNDLFHFNKKMFARRRILLKKNRHKRAGHGARNKLKPIAVLTEKSRRFRKKLIERWACEIANFFIKNKVGTVQMENLESMKRKEDSYFNIRLRGFWPYAEMQNKIEFKLRQYGIEIRKVAPNNTSKTCSKCGHLNNYFNFEYRKKNKFPYFKCEKCNFKENADYNAALNVSNPKLKSTKEEP

SEQ ID NO: 2987 - protein, 726 aa, synthetic construct
SEVEFSHEYWMRHALTLAKRARDEREVPVGAILVLNNRVIGEGWNRAIGLHDPTAHAEIMALRQGGLVMQNYRLVDATLYVTFEPCVLCAGAMVHSRIGRVVFGVRNSKRGAAGSLMNILNYPGMNHRVEITEGILADECAALLCDFYRMPRQVFNAQKKARSNIDSGGSSGGSSGSETPGTSESPTPESSGGSSGGSAKNTITKTLKLRIVRPYNSAEVEKIVADEKNNREKIALEKNKDKVKEACSEHLKVAAYCTTQVERNACLFCKARKLDDKFYQKLRGQFPGAVFWQEIGEIFRQLQKQAAEVYNQSLIELYYEIFIKGKGIANASSVEHYLSDVCYTRAAELFKNAAIASGLRNKIKSNFRLKELRNMKSGLPTTKSDNFPIPLVRQKGGQYTGFEISNHNGDFIIKIPFGRWQVKKEICKHRPWEKFDFEQVRKSPKPISLLLSTQRRKRNKGWGKDEGTEAEIRKVMNGDYQTSYIEVKRGSKIGEKSAWMLNLSIDVPKTDKGVDPSIIGGIDVGVKSPLVCAINNALSRYSISDNDLFHFNKKMFARRRILLRKNRHKRAGHGARNKLKPITVLTEKSERFRKKLIERWACEIANFFIKNKVGTVQMENLESMKRREDSYFNIRLRGFWPYAEMQSKIEFKLKQYGIKIRKVAPNNTSKTCSKCGHLNNYFNFEFRKKNKFPHFKCEKCNFKEDADYNAALNISNPKLKGTKEEP

SEQ ID NO: 2988 - protein, 726 aa, synthetic construct
SEVEFSHEYWMRRALTLAKRARDEREVPVGAVLVLNNRVIGVGWNRAVGLHDPTAHAEIMALRQGGLVMQNYRLIEATLYVTFEPCIMCAGAMIHSRIGRVVFGVRNSKRGAAGSLMNVLNYPGMNHHVEITEGILADECAALICDYYRMPRQVFSARKKAQSSINSGGSSDGGSGGETPGTSESATPESSGGSSGGSAKNTITKTLKLRIVRPYNSAEVEKIVAGEKNNREKIALEKNKDKVKEACSEHLKVAAYCTTQVERSACLFCKARKLDDKFYQKLRGQFPDAVFWQEISEIFRQLQKQAAEIYNQSLIELYYEIFIKGKGSANASSVEHYLSDVCYTRAAELFKNAAIASGLRGKVKSNFRLKELKNMKSGLPTTKSDNFPIPLVKQKGGQYTGFEISSHNSDFIIKIPFGRWQVKEEIDKFRPWEKFDFEQVRKSPKPISLLLSTQRRKKNKGWSKDEGTEAEIKKVMNGDYQTSYIEVKRGSKTGEKSAWMLNLSIDVPKIDKGVDPCIIGGIDVGVKSPLVCAINNALSRYSISDNDLFRFNKKMFARRRILLKKNGHKRAGHGAKNKLKPITIMTEKSKRFRKKLIERWACEIADFFIKNKVGTVQMENLESMKRKEDSYFNIRLRGFWPYAEMQNKIEFKLKQYGIVVRKVAPNNTSKTCSKCGHLNNYFNFEYRKKNKFPHFKCERCNFKENADYNAALNISNPKLKSTKGEP

SEQ ID NO: 2989 - protein, 726 aa, synthetic construct
SEVEFSHEYWMRHALTLAKRARDEREVPVGAILVLNNRVIGEGWNRAIGLHDPTAHAEIMALRQGGLVMQNYRLIDATLYVTFEPCVMCAGAMIHSRIGRVVFGVRNSKHGAAGSLVNVLNYPGMNHRVEITEGILADECAALLCDFYRMPRQVFGARRKAQSSINPGGSSGGSSGSETPGTSESPTPESPGGSSGGSAKNTITKTLKLRIVRPYNSAEVEKIVADEKNNREKIALEKNKDKVKEACSKHLKVAAYCTTQVERNACLFCKARKLDDKFYQKLRGQFPDAVFWQEIGEIFRQLQKQAAEIYNQSLIELYYEIFIKGRGFANASSVEHYLSDVCYTRAAELFKNAAIASGLRGKVKSNFRLKELKNMKSGLPTTKSDNFPIPLVKQKGGQYTGFEISNHNSDFIIKIPFGRWQAKKEIDKYRPWEKFDFEQVRKSPKPISLLLSTQRRKKNRGWSKDEGTEAEIKKVMNGDYQTSYIEVKRGSKIGEKSAWMLNLSIDVPKIDKGVDPSIIGGIDVGVKSPLVCAISNAFSRYSISDNDLFHFNKKMFARRRILLKKNRHKRAGHGAKNKLKPISILTEKSKRFRKKLIEKWACEIADFFIRNKVGTVQMENLESMKRKEDSYFNIRLRGFWPYAEMQNKIEFKLEQYGIEIRKVAPNNTSKTCSKCGHLNNYFNFEYRKKNKFPHFKCEKCNFKENADYNAALNISNPMLKSTKEEP

SEQ ID NO: 2990 - protein, 726 aa, synthetic construct
SEVEFSHEYWMRHALTLAKRARDEREVPVGAVLVLNNRVIGEGWNRAIGLHDPTAHAEIMALRQGGLVMQNYRLVDATLYVTFEPCVMCAGAMIHSRIGRVVFGVRNNKHGAAGSLVNVLNYPGMNHRVEITEGILADECAALLCDFYRMPRQVLNAQKKAQSSISSGGSSGGSSCSETSGASESVTPKSSGGSSAGTTKNTITKTLKLRIVRPYNSAEVEKIVADEKNSREKIALEKNKDKVKEACSEHLKVVAYCTTQVERNACLFCKARKLDDKFYQKLRGQFPDAVFWQELGEIFRQLQKQAAEIYNQSLIELYYEILIKGKGFANASSVEHYLSDVCYTRAAELFKNAAIASGLRGKVKSNFRLKELKNMKSGLPTTKSDNFPIPLVKQKGGQYTGFEISSHNDDFIIKIPFGRWQVKKEIDKYRPWEKFDFEQVRKSPKPISLLLSTQRRKRNKGWSKDEGTEAEIRKVMNGDYQTSYIEVKRGSKTGEKSAWMLNLSIDVPKIDKGVDPSIIGGIDVGVKSPLVCAINNAFSRYSISDNDLFRFNKKMFARRRILLGKNRHKRAGHGAKNKLKPISILTGKSERFRKKLIERWACEIADFFIKNKVGTVQMENLEGMKRKEDSYFNIRLRGFWPYAEMQNKIEFKLKQYGIEIRKVAPNNTSKTCSKCGHLNNYFNFGYRKRNKFPHFECEKCNFKEDADYNAALNISNPKLKSTKEEP

SEQ ID NO: 2991 - protein, 725 aa, synthetic construct
SEAEFSHEYWMRHALTLAKRARDEREVPVGAVLVLNNRVIGEGWNRAIGLHDPTAHAEIMALRQGGLVMQNYRLADATLYVTFEPCVLCAGAMVHSRIGRVVFGVRNSKRGAAGSLMNVLNYPGMNHRVEITEGILADECAALLCDFYRMPRQVFNARKKARSNINSGGSSGGSSGSETPGTSESATPESSGGGSSGSAKNTITKTLQLRIVRPYNSAEVEKIVADEKNNREKIALEKNKDKVKEACSKHLKVASYCTTQVERSACPFCKARKLDDKFYQKLGGQFPDAVFWQELGEILRQLQKQAAEIYNQSLIELYYEIFIKGRGFANASSVEHYLSDVCYTRAAELFKNAAIASGLRGKVKSNFRLKELKNMKSGLPTTKSDNFPIPLVKQKGGQYTGFEISSHNDDFIIKIPFGRWVKKEIDKYRPWEKFDFEQVRKSPKPISLLLSTQRRKKNKGWSKDEGTEAEIRRVMNGDYRTSYIEVKRGSKIGEKSAWMLNLSIDVPKIDKGVDPSIIGGIDVGVKSPLVCAINNSSSRYSICDNDLFRFNKKMFARRRILLKKNRHKRAGHGAKNKLKPITILTKKSERFRKKLIERWVCEVADFFIKNKVGTVQMENLESMKRKEDSYFNIRLRGFWPYAEMQNKIEFKLKQYGIEIRKVAPNNTSKTCSKCGHLNSYFNFEYRKKNKFPHFKCEKCNFKENADYNAALNISNPKLKSTKEEP

SEQ ID NO: 2992 - protein, 726 aa, synthetic construct
SEVEFSHEYWMRHALTLAKRARDEREVPVGAVLVLNNRVIGEGWNRAIGLHDPTAHAEIMALRQGGLVMQNYRLTDATLYVTFEPCVMCAGAMIHSRIGRVVFGVRNSKRGAAGSLMNVLNYPGMNHCVEITEGILVDECAALLCDFYRMPRQVLNAQKKAQSSVSSGGSSGGSSGSETPGASGSVTPKSSVGSSAGSTKNTITKTLKLRIVRPYNSAEVEKIVADEKNNREKIALEKNKDKVKEACSKHLRVAAYCTTQVERNACLFCKARRLDDKFYQKLRGQFPDAVFWQEIGEIFRQLQKQAAEIYNQSLIELYYEIFIKGKGFANASSVEHYLSDVCYTRAAELFKNAAIASGLRGKVKSNFRPKELKNMKSGLPTTKSDNFPIPLVKQKGGQYTGFEISSHDDDFVIKIPFGRWQVKKEIDKYRPWEKFDFEQVRKSPKPISLLLSTQRRKRNKGWSKDVGTEAEIRKVMNGDYQTSYIEVKRGSKIGKKSAWMLNLSIDVPKIDKGVDPSIIGGIDVGVKSPLVCAINNAFSRYSISDNDLFHFNKKVFARRRILLKRNGHKRAGHGTKNKLKPITILAEKSGRFRKKLIERWACEIANFFIKNKAGTVQMENLESMKRKEDSYFNIRLRGFWPYAEMQNKIEFKLKQYGIKIRKVAPNNTSKTCSKCGHLNNYFSFEYRKKNKFPHFKCEKCNFKEDADYNAALNISNPKLKSTKEEP

SEQ ID NO: 2993 - protein, 726 aa, synthetic construct
SEVEFSHEYWMRHALTLAKRARDEREVPVGAVLVLNNRVIGEGWNRAIGLHDPTAHAEIMALRQGGLVMQNYRLVDATLYVTFEPCVLCAGAMVHSRIGRVVFGVRNSKRGAAGSLMNVLNYPGMNHRVEITEGILADECAALLCDFYRMPRQVFNAQKKARSNINPGGSSGGSSGSETLGTSESATPESSGGSSGGSAKNTITKTLKLRIVRPYNSAEVEKIVADEKNNREKIALEKNKDKVKEACGKHLKVASYCTTQVERNACLFCKARKLDDKFYQKLRGQFPDAVFWQELGEIFRQLQKQAAEIYNQSLIELYYEIFIKGQGLANASSVEHYLSDVCYTRAAELFKNAAIASGLRGKVKSNFKLKELKNMKSGLPTTKSDNFPIPLVRQKGGRYTGFEISSHNDDFIIKIPFGRWQVRKEISRHRPWEKFDFEQVRKSPKPISLLLSTQRRKRNKGWGKDEGTEAEIRKVMNGDYQTSYIEVKRGSKIGEKSAWMLNLSIDVPKIDKGVDPSIIGGIDVGVKSPLVCAINSALSRYSISDNDLFHFNKKMFARRRILLRKNRHKRAGHGARNKLKPITVLTEKSERFRKKLIERWACEIANFFIKNKVGTVQMENLESMKRREDSYFNIRLRGFWPYAEMQSKIEFKLKQYGIKIRKVAPNNTSKTCSKCGHLNNYFNFEFRKKNKFPHFKCEKCNFKENADYNAALNISNPKLKSAKEEP

SEQ ID NO: 2994 - protein, 726 aa, synthetic construct
SEVEFSHEYWMRHALTLAKRARDGREVPVGAVLVLNNRVIGEGWNRAIGLHDPTAHAEIMALRQGGLVTQNYRLIDATLYVTFEPCAMCAGAMIHSRIGRVVFGVRNSKHGAAGSLVNVLNYPGMNHRVETTEGILADECAALLCDFYRMPRRVFNARMKAQSSINPGGSSGGSGGSETPGTSESATPESFGGSSGGSAKNTITKTLKLRIVRPYNSAEVEKIVADEKNNREKIALEKNKDKVKEACSKHLKVAAYCTTQVERNACLFCKARKLDDKFYQKLRGQFPDAVFWQEIGEIFRQLQKQAAEIYNQSLIELYYEIFIKGKGFANASSVEHYLSDVCYTRAAELFKNAAIASGLRGKVKSNFRLKELKNMKSGLPTTKSDNFPIPLVKQKGGQYTGFEVSSHNDDFIIKIPFGRWQVKKEIDKYRPWEKFDFEQVRKSPRPISLLLSTQRRKRNRGWSKDEGTEAEIRKVMNGDYQTSYIEVKRGSKIGEKSAWMLNLSIDVPKIDKGVDPGIIGGIDVGVKSPLVCAINNALSRYSISDNDLFHFNKKMFARRRILLRKNRHKRAGHGAKNKLKPITIMTEKSKRFRKKLIERWACEIADFFIKNKVGTVQMENLESMKRKEDSYFNIRLRGFWPYAEMQNKIEFKLKQYGIEIRKVAPNNTSKTCSKCGHLNNYFNFEYRKKNKFPHFKCEKCNFKENADYNAALNISNPKLKGTKEEP

SEQ ID NO: 2995 - protein, 726 aa, synthetic construct
SEVEFSHEYWMRHALTLAKRARDEREVPVGAILVLNNRVIGGGWNRAIGLHDPTAHAEIMALRQGGLVMQNYRLIDATLYVTFEPCVMCAGAMIHSRIGRVVFGVRNNKHGAAGSLMNVLDYPGMNHRVEITEGILADECAALLCDFYRMPRQVFNARKKAQSSISPGGSSGGSSGSETPGTSESATPESSGGSSGSSAKNTITKTLKLRIVRPYNSAEVEKIVADEKNNREKIALEKNKDKVKEACSKHLKVASYCTTQVERNACPFCKARKLDDKFYQKLRGQFPDAVFWQELGEILRQLQKQAAEIYNQSLIELYYEIFIKGRGFANASSVEHYLSDVCYTRAAELFKNAAIASGLRGKVKSNFRLKELKNMKSGLPTTKSDNFPIPLVKQKGGQYAGFEISSHNGDFIIKIPFGRWQVKKEIDKYRPWEKFDFEQVRRSPKPISLLLSTQRRKKNKGWSKDEGTEAEIRRVMNGDYQTSYIEVKRGSKIGEKSAWMLNLSIDVPKIDKGVDPSIIGGIDVGVKSPLVCAINNAFSRYSISDNDLFHFNKKMFARRRILLKKNRRRRAGHGAKNKLKPISILTGKGERFRKKLIERWACEIADFFIKNKVGTVQMENLESMKRKEDSYFNIRLRGFWPYAEMQNKIEFKLKQYGIKIRKVAPNNTSKTCSKCGHLNNYFNFEYRKKNKFPHFKCEKCNFKENADYNAALNISNPKLKSTKEEP

SEQ ID NO: 2996 - protein, 726 aa, synthetic construct
SEVEFSHEYWMRHALTLAKRARDEREVPVGAILVLNNRVIGEGWNRAIGLHDPTAHAEIMALRQGGLVMQNYRLIDATLYVTFEPCVMCAGAMIHSRIGRVVFGVRNSKHGAAGSLMNVLNYPGMNHRVEITEGVLADECAALLCDFYRMPRRVFSAQKKAQSSINPGGPSGGSSGSETPGTSESATPESSGGSSGGSTKGTITKTLKLRIVRPYNSAEVEKIVADEKNSREKIALEKNKDKVKEACSKHLKVAAYCTTQVERNACLFCKARKLDDKFYQKLRGQFPDAVFWQEVSEIFRQLQKQAAEIYNQSLIELYYEIFIKGKGFANASSVEHYLSDVCYTRAAELFKNAAIASGLRGKVKSNFRLKELKNMKSGLPTTKSDNFPIPLVKQKGGQYTGFEISSHNDDFIIKIPFGRWQVKKEVDKYRPWEKFDFEQVRKSPKPISLLLSTQRRKKNKGWGKDEGTEAEIRRVMNGDYQTSYIEVKRGSKIGEKSAWMLNLSIDVPKIDKGVDPSIIGGIDVGVISPLVCAINNSSSRYSICDNDLFRFNKKMFARRRILLKKNRHKRAGHGAKNKLKPITILTKKSERFRKKLIERWVCEVADFFIKNKVGTVQMENLESLKRKEDSYFNIRLRGFWPYAEMQNRIELKLKQYGIEIRRVAPNNTSRTCSKCGHLNNYFNFEYRKKNKFPHFKCEKCNFREDADYNAALNISNPKLKSTKEEP

SEQ ID NO: 2997 - protein, 726 aa, synthetic construct
SEVEFSHEYWMRHALTLAKRARDEREVPVGAILVLNNRVIGEGWNRAIGLHDPTAHAEIMALRQGGLVMQNYRLIDATLYVTFEPCVMCAGAMIHSRIGRVVFGVRNSKHGAAGSLVNVLNYPGMNHRVEITEGILADECAALLCDFYRMPRQVFNARKKAQSSINPSGSSGGSSGSVTPGASGSVTPKSSGGGSSGSARNTITKTLQLRIVRPYNSAEVEKIVADEKNNREKIALEKNKGKVREACNKHLKVASYCTTQVERNACPFCKARKLDDRFYQKLRGQFPDAVFWQETGEIFRQLQRQAAEIYNQSLIELYYEIFIKGKGFANASSVEHYLSDVCYTRAAELFKNAAIASGLRGKVKSNFRLKELKNMKSGLPTTKSDNFPIPLVKQKGGQYTGFEISNHNGDFIIKIPFGRWQVKKEISKHRPWEKLDFEQVRKSPRPISLLLSTQRRKRNKGWGKDEGTEAEIRKVMNGDYQTSYIEVKRGSKIGEKSAWMLNLSIDVPKIDKGVDPSIIGGIDVGVKSPLVCAINNALSRYSISDNDLFHFNKKMFARRRILLRKNRHKRAGHGARNKLKPITVLTEKSERFRKKLIERWACEIANFFIKNKVGTVQMENLESMKRREDSYFNIRLRGFWPYAEMQSKIEFKLKQYGIEIRKVAPNNTSKTCSKCGHLNNYFNFEFRKKNKFPHFKCEKCNFKEDADYNAALNISNPKLKSTKEEP

SEQ ID NO: 2998 - protein, 726 aa, synthetic construct
SEVEFSHEYWMRHALTLAKRARDEREVPVGAVLVLNNRVIGEGWNRAIGLHDPTAHAEIMALHQGGLVMQNYRLIDATLYVTFEPCVMCAGAMIHSRIGRVVFGARNSKRGAAGSLMNVLSYPGMNHRVEITEGVLADECAALLCDFYRMPRRVFNAQKKAQSSINSGGSSGGGSGSETPSTSESTTPESSGGSSGGPAKNTITKTLKLRIVRPYNSAEVEKIVADEKNNREKTALEKNKDKVKEACSMHLKVAAYCTTQVERNACLFCKARKLDDKFYQKLRGQFPDAVFWQEVGEIFRQLQKQAAEIYNQSLIELYYEIFIKGKGFANASSVEHFLSDVCYTRAAELFKNAAIASGLRNKTKSNFRLKELRSMKSGLPTTKSDNFPIPLVKQKGGQYTGFEISNHNSDFIIKIPFGRWQVKKEINKYRPWEKFDFEQVRKSPKPISLLLSTQRRKRNKGWSKDEGTEAEIRKVMNGDYQTSYIEVKRGSKIREKSAWMLNLSIDVPKIDKGVDPSIIGGIDVGVKSPLVCAINNAFSRYSISDNDLFRFNKKVFARRRILLKKNRHKRAGHGTKNKLKPITILTEKSGRFRKKLIERWACEIANFFIKNKVGTVQMENLESMKRKEDSYFNIRLRGFWPYAEMQNKIEFKLKQYGIKIRKVAPNNTSKTCSKCGHLNNYFNFEYRRKNKFPHFKCEKCNFKEDADYNAALNISNPKLKSTKEEP

SEQ ID NO: 2999 - protein, 726 aa, synthetic construct; identical to SEQ ID NO: 2904

SEQ ID NO: 3000 - protein, 726 aa, synthetic construct; identical to SEQ ID NO: 684

SEQ ID NO: 3001 - protein, 726 aa, synthetic construct
SEVEFSHEYWMRRALTLAKRARDEREVPVGAVLVLNNRVIGVGWNRAVGLHDPTAHAEIMALRQGGLVMQNYRLIEATLYVTFEPCIMCAGAMIHSRIGRVVFGVRNSKRGAAGSLMNVLDYPGMGHRVEITEGILADECAALLCDFYCMPRQVFNAQKRAQSSINSGGSSGGSSGSETPGTSESATPESSSGGSSGSAKNTITKTLQLRIVRPYNSAEVEKIVADEKNNREKIALEKNKDKVKEACSKHLKVASYCTTQVERNACPFCKARKLDDKFYQKLRGQFPDAVFWQELGGIFRQLQKQAAEIYNQSLIELYYEIFIKGKGITNASRVEHYLSDVCYTRAAELFKNAAIASGLRSKVRSNFRLKELKNMKSGLPTTKSDNFPIPLVKQKGGQYTGFEISSHNSDFIIKIPFGRWRVKEEIDKYRPWEKFDFEQVRKSPKPISLLLSTQRRKKNKGWSKDEGTEAEIRRVMNGDYQTSYIEVKRGSKIGEKSAWMLNLSIDVPKIDKGVDPSIIGGIDVGVKSPLVCAINNSSSRYSICDNDLFRFNKKMFARRRILLKKNRHKRAGHGAKNKLKPITIPTEKSRRFRKKLIERWACEIADFFIKNKVGTVQMESLESMKRKEDSYFNIRLRGFWPYAEMQNKIEFKLKQYGIKIRKVAPDNTSKTCSKCGHLNNYFSFEYRKKNKFPHFKCEKCNFKEDADYNAALNISNPKLKSTKEEP

SEQ ID NO: 3002 - protein, 726 aa, synthetic construct
SEVEFSHEYWMRHALALAKRARDGREVPVGAVLVLNNRVIGEGWNRAIGLHDPTAHAEIMALRQGGLVMQNYRLIDATLYVTFEPCVMCAGAMIHSRIGRVVFGVRNSKHGAAGSLVNVLNYPGMNHRVEITEGILADECAALLCDFYRMPRQVFNARKKAQSSINSGDSSGGSSGSETPGTSESATPKSSGGSSGGSAKNTITKALKLRIVRPYNSAEVEKIVADEKNNRERIALEKNKDKVKEACSKHLKVAAYCTTQVERNACLFCKARKLDDKFYQKLRGQFPDAVFWQEIGEIFRQLQKQAAEIYNQSLIELYYEILIKGKGFANASRVGHYLSDVCYTRAAELFKNAAIASGLRSKIKSNFRLKELKNMKSGLPTTKSDNFPIPLVKQKGGQYTGFEISNHNSDFIIKIPFGRWQVKKEIDKYRPWEKFDFEQVRKSPKPISLLLSTQRRKRNKGWSKDEGTEAEIRKVMNGDYQTSYIEVKRGSKIGEKSAWMLNLSIDVPKIDKGVDPSIIGGIDVGVKSPLVCAINNALSRYSISDNDLFHFNKKMFARRRILLRKNRHKRAGHGAKNKLKPITMMTEKSKRFRKKLIERWACEIADFFIKNKVGTVQMENLESMKRKEDSYFNIRLRGFWPYAEMQNKIEFKLKQYGIRVRKVAPNNTSKTCSKCGHLNNYFNFEYRKTNKFPHFKCEKCNFKEDADYNAALNISNPKLKSTKEEP

SEQ ID NO: 3003 - protein, 726 aa, synthetic construct
SEVEFSHEYWMRHALTLAKRARDEREVPVGAVLVLNNRVIGVGWNRAIGLHDPTAHAEIMALRQGGLVMQNYRLINATLYVTFEPCVMCAGAMIHSRIGRVVFGVRNSKHGAAGSLMNVLNYPGMNHRVEITEGILADECAALLCDFYRMPRQVLNAQKKAQSSISFGGSSGGSSGSETPGTSESATPGSSGGSSGGSAKNTITKTLKLRIVRPYNSAEVEKIVADEKNNREKIALEKNKGKVKEACSEHLKVAAYCTTQVERNACLFCKARKLDDKFYQKLRGQFPDAVFWQEIGEIFRQLQKQAAEIYNQSLIELYYEIFIKGKGFANASSVEHYLSDVCYTRAAELFKNAAIASGLRGKVKSNFRLKELKNMKSGLPTTKSDNFPIPLVKQKGGQYTGFEISSHNDDFIIKIPFGRWQEKEEIGKYRPWEKFDFEQVRKGPRPISLLLSTQRRKRNKGWSKDEGTEAEIRKVMNGDYQTSYIEVKRGSKIGEKSAWMLNLSIDVPKIDKGVDPSIIGGIDVGVKSPLVCAINNALSRYSISDNDLFHFNKKMFARRRILLRKNRHKRAGHGARNKLKPITVLTEKSKRFRKKLIERWACEIANFFIKNRVGTVQMENLESMKRKEDSYFNIRLRGFWPYAEMQNRIEFKLKQYGIEIRKVAPNNTSKTCSKCGHLNNYFNFEYRKKNKFPHFRCEKCNFKENADYNAALNISNPKLKSTKEEP

SEQ ID NO: 3004 - protein, 725 aa, synthetic construct
SEVEFTHEYWMRHALTLAKRARDEREVPVGAILVLNNRVIGEGWNRAIGLHDPTAHAEIMALRQGGLVMQNYRLIDATLYVTFEPCVMCAGAMIHSRIGRVVFGVRNNKHGAAGSLVNVLNYPGMNHRVEITEGILANECAALLCDFYRMPRQVFNARKKAQSSINPGGSSGGSSGSETPGASGSVTPKSSGGSSAGSTKDTITKTLKLRIVRPYNSAEVEKIVADEKNSREKIALEKNKDKVKEACSEHLKVAAYCTTQVERNACLFCKARKLDDGFYQKLRGQFPDAVFWQEIGEIFRQLQKQAAEIYNQSLIELYYEIFIKGKGFANASSVEHYLSDVCYTRAAELFKNAAIASGLRGKVKSNFRLKELKNMKSGLPTTKSDNFPIPLVKQKGGQYTGFEISSHNDDLIVKIPFGRWQVKKEIDRYRPWEKFDFEQVRKSPKPISLLLSTRRKRNKGWSKDEGTEAEIRKVMNGDYQISYIEVKRGSKIGEKNAWMLNLSIDVPKVDKGVDPSIIGGIDVGVKSPLVCAINNALSRYSISDNDLFRFNKKMFARRRILLKKNRHKRAGHGAKNKLKPISILTGKSERFRKKLIERWACEIADFFIKNKVGTVQMENLESMKRKEDSYFNIRLRGFWPYAEMQNKIEFKLKQYGIEIRKVAPSNTSKTCSRCGHLNNYFNFEYRKKSKFPHFKCEKCNFKENADYNAALNISNPKLKSSKEEP

SEQ ID NO: 3005 - protein, 726 aa, synthetic construct
SEVEFSHEYWMRHALTLAKRARDEREVPVGAILVLNNRVIGVGWNRAIGLHDPTAHAEIMALRQGGLVMQNYRLIDATLYVTFEPCVMCAGAMIHSRIGRVVFGVRNSKHGAAGSLTNVLNYPGMNHCVEITEGILVDECAALLCDFYRMPRQVLNARKKAQSSINPSGSSGGSSGSETPGTSESVAPESSGGSSGGSAKNTITKTLKLRIVRPYNSAEVEKIVADEKNNREKIALEKNKDKVKEACSKHLKVAAYCTTQVERNACPFCKARKLDDKFYQKLRGQFPDAVFWQELGEILRQLQKQAAEIYNQSLIELYYEIFIKGRGFANASSVEHYLSDVCYTRAAELFKNAAIASGLRNKIKGNFRLKELRNMKSGLPTTKSDNFPIPLVRQKGGQYTGFEISNHNGDFIIKIPFGRWLVKKEINKHRPWEKFDFEQVRKSPKPISLLLSTQRRKRNKGWSKDEGTEAEIRKVMNGDYQTSYIEVKRGSKIGEKSAWMLNLSIDVPKIDKGVDPSIIGGIDVGVKSPLVCAINNAFSRYSISDNDLFRFNKKMFARRRILLKKNRHKRAGHGAKNKLKPISILTGKSERFRKKLIERWACEIADFFIKNKVGTVQMENLESMKRREDSYFNIRLRGFWPYAEMQNKIEFKLKQYGIEIRKVAPNNTSKTCSKCGHLNNYFNFEYRRKNKFPHFKCEKCNFKEDADYNAALNISNPKLKSTKEEP

SEQ ID NO: 3006 - protein, 726 aa, synthetic construct
SEVEFSHEYWMRHALTLAKRARDEREVPVGAILVLNNRVIGEGWNRAIGLHDPTAHAEIMALRQGGLVMQNYRLIDATLYVTFEPCVMCAGAMIHSRIGRVVFGVRNSKHGAAGSLVNVLNYPGMNHRVEITEGILADECAALLCDFYRMPRQVFNARKKAQSSINPGGSSGGSGGSETPGTSESATPESSGGSSSGSTKNTITKTLKLRIVRPYNSAEVEKIVADEKNNREKIALEKNKDRVKEACSKHLKVASYCTTQVERNACPFCKARKLDDKFYQKLRDQFPDAVFWQELGEILRQLQKQAAEIYNQSLIELYYEIFIKGRGFANASSVEHYLSDVCYTRAAELFKNAAIASGLRGKVKSNFRLKELKNMKSGLPTTKSDNFPIPLVKQKGGQYTGFEISSRNDDFIIKIPFGRWQVKKEIDKYRPWEKFDFEQVRKSPKPISLLLSTQRRKRNKGWSKDEGTEAEIRKVMNGDYQTSYIEVKRGSKTGEKSAWMLNLSIDVPKIDKGVDPSIIGGIDVGVKSPLICAINNAFSRYGISDNDLFRFNKKVFARRRILLKKNRHKRAGHGAKNKLKPISILTEKSKRFRKKLIERWACEIADFFIKNKVGTVQMENLESMKRKEDSYFNIRLRGFWPYAEMQNKIEFKLKQYGIEIRKVAPNNTSKTCSKCGHLNNYFNFEYRKMNKFPHFKCEKCNFKENADYNAALNISNPKLKGTKEEP

SEQ ID NO: 3007 - protein, 726 aa, synthetic construct
SEVEFSHEYWMRHALTLAKRARDEREVPVGAILVLNNRVIGEGWNRAIGLHDPTAHAEIMALRQGGLVMQNYRLIDATLYVTFEPCVMCAGAMIHSRIGRVVFGVRNSKHGAAGSLMNVLNYPGMNHRVEITEGVLADECAALLCDFYRMPRQVFSARKKAQSSINPGGSSGGSSGSKTPGTSESATPESSGGSSGGSAKNSITKTLKLRIVRPYNSAEVEKIVADEKNNREKIALEKNKGKVKEACSKHLKVATYCTTQVERNACLFCKARKLDDKFYQKLRGQFPDAVFWQEIGEIFRQLQKQAAEIYNQSLIELYYEIFIKGKGFANASSVEHYLSDVCYTRAAELFKNAAIASGLRNKIKSNFRLKELRNMKSGLPTTKSDNFPIPLVRQKGGQYTGFEISNHNGDFIIKIPFGRWQVKKEINKHRPWEKFDFEQVQKSPKPISLLLSTQRRKRNKGWSKDEGTEAEIKRVMNGDYQTSYIEVTRGSKIGEKSAWMLSLSIDAPKIDKGVDPSIIGGIDVGVKSPLVCAINNAFSRYSISDNDLFHFNKKMFARRRILLKKNRHKRAGHGAKNKLKPITILTEKSKRFRKKLIERWACEIADFFIKNKVGTVQMENLESMKRKEDSYFNIRLRGFWPYAEMQNKIEFKLKQYGIVVRKVAPNNTSKTCSKCGHLNNYFNFEYRKKNKFPHFKCEKCNFKENADYNAALNISNPKLKNTKGEP

SEQ ID NO: 3008 - protein, 726 aa, synthetic construct
SEVEFSHEYWMRHALTLAKRARDEREVPVGAVLVLNNRVIGEGWNRAIGLHDPTAHAEIMALRQGGLVMQNYRLTDATLYVTFEPCVMCAGAMIHSRIGRVVFGVRNSKRGAAGSLMNVLNYPGMNHCVEITEGILVDECAALLCDFYRMPRQVLNAQKKAQSSISSGGSSGGSSGSETPCASESATPKSSGGSSAGSTKNTLTKTLKLRIVRPYNSAEVEKIVADEKNNREKIALEKNKDKVKEACSKHLKVAAYCTTQVERNACLFCKARKLDDKFYQKLRGQFPDAVFWQEISEILRQLQKQAAEIYNQSLIELYYEIFIKGRGFANASNVEHYLSDVCYTRAAELFKNAAIASGLRGKVKGNFRPKELKNMKSGLPTTKSDNFPIPLVKQKGGQYTGFEISSHNDDFIIKIPFGRWQVKKEIDKYRPWEKFDFEQVRKSPKPISLLLSTQRRKRNKGWSKDEGTEAEIRKAMNGDYQTSYIEVKRGSKIGEKSAWMLSLSIDVPKIDKGVDPRIIGGIDVGVKSPLVCAINNVLSRYSISDNDLFHFNKKVFARRRILLKKNGHKRAGHGAKNKLKPITIMTEKSKRFRKKLIERWACEIADFFIKNKVGTVQMENLESMKRKEDSYFNIRLRGFWPYAEMQNKIEFKLKQYGIVVRKVAPNNTSKTCSQCGHLNNYFNFEYRKKNKFPHFKCEKCNFKENADYNAALNISNPKLKSTKEEP

SEQ ID NO: 3009 - protein, 726 aa, synthetic construct
SEDEFSHEYWMRHALTLAKRARDGREVPVGAVLVLNNRVIGEGWNRAIGLHDPTAHAEIMALRQGGLVMQNYRLIDATLYVTFEPCVMCAGAMIHSRIGRVVFGVRNNKHGAAGSLVNVLNYPGMNHRVEITEGILADECAALLCDFYRMPRQVFNARKKAQSSINPGGSSGGSGGSVTPGTSESATPKSSGGSSGGSAKNTITKALKLRIVRPYNSAEVEKIVADEKNNRERIALEKNKDKVKEACSKHLKVAAYCTTQVERNACLFCKARKLDDKFYQKLRGQFPDAVFWQEIGEIFRQLQKQAAEIYNQSLIELYYEIFIKGRGFANASSVEHYLSDVCYTRAAELFKNAAIASGLRGKVKSNFRLKELKNMKSGLPTTKSDNFPIPLVKQKGGQYTGFEVSSHNDDFIIKIPFGRWQVKKEIDKYRPWEKFDFEQVRKSPRPISLLLSTQRRKRNKGWSKDEGTEAEIRKVMNGDYQTSYIEVKRGSKIGEKSTWMLNLSIDVPKIDKGVDPSIIGGIDVGVKSPLVCAIDNAFSRYSISDNDLYHFNKKMFAKRRILLRKNRHKRAGHGAKNKLKPISILTEKSERFRKKLIERWACEIADFFIKNKVGTVQMENLESMKRREDSYFNTRLRGFWPYAEMQNKIEFKLKQYGIEIRKVAPNNTSKTCSKCGHLNNYFNFEYRKKNKFPHFKCEKCNFKENADYNAALNISNPKLKSTKEEP

SEQ ID NO: 3010 - protein, 726 aa, synthetic construct
SEVEFSHEYWMRHALTLAKRARDEREVPVGAILVLNNRVIGVGWNRAIGLHDPTAHAEIMALRQGGLVMQNYRLIDATLYVTFEPCVMCAGAMIHSRIGRVVFGVSNSKHGAAGSLVNVLNYPGMNHRVEVTEGILADECAALLCDFYRMPRQVFNARKKAQSSINSGGSSGGSSGSETPGTSESATPKSSGGSSGGSAKNTITKALKLRIVRPYNSAEVEKIVADEKNNRERIALEKNKDKVKEACSKHLKVAAYCTTQVERNACLFCKARKLDDKFYQKLRGQFPDAVFWQEIGEIFRQLQRQAAEIYNQSLIELYYKIFIKGKGFANASSVEHYLSDVCYTRAAELFKNAAIASGLRGKVKSNFRLKELKNMRSGLPTTKSDNFPIPLVKQKGGQYAGFEISSHNDDFIIKIPFGRWQVKKEIDKYRPWEKFDFEQVRKSPKPISLLLSTRRRKRNKGWSKDEGTEAEIRKVMNGDYQTSYIEVKRGSKIGEKSAWMLNLSIDVPKIDKGVDPSIIGGIDVGVKSPLVCAINNAFSRYSISDNDLFHFNKKMFARRRILLKKTRHKRAGHGAKNKLKPISILTEKSERFRKKLIERWACEIADFFIKNKVGTVQMENLESMKRREDSYFNIRLRGFWPYAEMQNKIEFKLKQYGIEIRKVAPNNTSKTCSKCGHLNNYFNFEYRKKNKFPHFKCEKCNFKEDADYNAALNISNPKLKSTKEEP

SEQ ID NO: 3011 - protein, 726 aa, synthetic construct
SEVEFSHEYWMRHALTLAKRARDEREVPVGAVLVLNNRVIGEGWNRAIGLHDPTAHAEIMALRQGGLVMQNYRLADATLYVTFEPCVMCAGAMIHSRIGRVVFGVRNSKRGAAGSLMNVLNYPGMNHCVEITEGILVDECAALLCDFYRMPRQVLNAQKKAQSSISSGGSSGGSSGSETPGASGSVTPKSSGGSSAGSAKDTITKTLKLRIVRPYNSAEVEKIVADEKNSREKIALEKNKDKVKEACSEHLKVAAYCTTQVERNACLFCKARRLDDKFYQKLRGQFPDAVFWQEIGEIFRQLQKQAAEIYNQSLIELYYEIFIKGRGFANASSVEHYLSDVCYTRAAELFKNAAIASGLRGKVKSNFRLKELKNMKSGLPTTKSDNFPIPLVKQKGGQYTGFEISSHNDDFIIKIPFGRWQVKKEIGKYRPWEKFDFEQVRKSPKPISLLLSTQRRKMNKGWSKDEGTEAEIRKVMNGNYQTSYIEVKRGSKTGEKSAWMLNLSIDVPKIDKGVDPSIIGGIDVGVKSPLVCAINNAFSRYSISDNDLFRFNKKMFARRRILLKKNRHKRAGHGAKNKLKPISILTGKSERFRKKLIERWACEIADFFIKNKVGTVQMENLESMKRKEDSYFNIRLRGFWPYAEMQNKIEFKLKQYGIEIRKVAPNNTSKTCSKCGHLNNYFNFEYRKKNKFPHFKCEKCNFKENADYNAALNISNPKLKSTKEEP

SEQ ID NO: 3012 - protein, 726 aa, synthetic construct
SEAEFSHEYWMRHALTLAKRARDEREVPVGAVLVLNNRVIGEGWNRAIGLQDPTAHAEVMALRQGGLVMQNYRLTDATLYVTFEPCVMCAGAMIHSRIGRVVFGVRNSKRGAAGSLMNVLNHPGMNHRVEITEGILAGECAALLCDFYRMPRQVLSAQKKAQSSISSGGSSGGSSGSETPGASGSVTPKSSVGSSAGSTKNTITKTLKLRIVRPYNSAEVEKIVADEKNNREKIALEKNKDKVKEACSKHLKVAAYCTTQVERNACLFCKARRLDDKFYQKLRGQFPDAVFWQEISEIFRQLQKQAAEIYNQSLIELYYEIFIKGKGFANASSVEHYLSDVCYTRAAELFKNAAIASGLRGKVKSNFRLKELKNMKSGLPTTKSDNFPIPLVKQKGGQYTGFEISSHNDDFIIKIPFGRWQVKKEIDKYRPWEKFDFEQVRKSPKPISLLLSTQRRKRNKGWSKDEGTEAEIKKVMNGDYQTSYIEVKRSSKIGEKGAWMLSLSIDVPKIDKGVDPSIVGGVDVGVKSPLVCAINNALSRYSISDNDLYRFNKKMFARRRILLKKNRHKRAGHGAKNKLKPITILTEKSERFRKKLIERWACEIADFFIKNKVGTVQMENLEGMKRKEDSYFNIRLRGLWPYAEMQNKIEFKLKQYGIVVRKVAPNNTSKTCSQCGHLNNYFNFEYRKKNKFPYFKCEKCNFKENADYNAALNISNPQLKSTKGEP

SEQ ID NO: 3013 - protein, 726 aa, synthetic construct
SEDEFSHEYWMRHALTLAKRARDGREVPVGAVLVLNNRVIGEGWNRAIGLHDPTAHAEIMALRQGGLVMQNYRLIDATLYVTFEPCVMCAGAMVHSRIGRVVFGVRNSKRGAAGSLMNVLDYPGMGHRVEITEGILADECAALLCDFYRMPHQVFNAQKKAQSSINSGGSSGGSSGSVTPGPSESATPESSGGSSGSSAKNTITKTLQLRIVRPYNSAEVEKIVADEKNNREKIALEKNKDKVKEACSKHLKVASYCTTQVERNACLFCKARKLDDKFYQRLRGQFPDAVFWQELGEIFRQLQKQAAEIYNQSLIELYYEIFIKGKGFANANSVEHYLSDVCYTRAAELFKNAAIASGLRGKVKSNFRLKELKNMKSGLPTTKSDNFPIPLVKQKGGQYTGFEISSHNSDFIIKIPFGRWQEKEEIDKYRPWEKFDFEQVRRSPKPISLLLSTQRRKKNKGWSKDEGTEAEIRRVMNGDYQTSYIEVKRGSKIGEKSAWMLSLSIDVPKIDKGVDPSIIGGIDVGVKSPLVCAINNAFNRYSISDNNLFHFNKKMFARRRILLKKNRHKRAGHGAKNKLKPISILTGKSKRFRKKLIERWACEIADFFIKNKVGTVQMENLESMKRKEDSYFNIRLRGFWPYAEMQNKIEFKLKQYGIEIRKVAPNNTSKTCSKCGHLNNYFNFEYRKKNKFPHFKCEKCSFKENADYNAALNISNPRLKSTKEEP

SEQ ID NO: 3014 - protein, 726 aa, synthetic construct
SEVEFSHEYWMRHALTLAKRARDEREVPVGAILVLNNRVIGEGWNRAIGQHDPTAHAEIMALRQGGLVMQNNRLTDATLYVTFEPCVMCAGAMVHSRIGRVVFGVRNSKRGAAGSLMNVLNYPGVNHCVEITEGILVDECAALLCDFYRMPRQVLNAQKKARSSISSGGSSGGCSGSEMPGASESVTPKSSGGSPGGSAKNTITKTLKLRIVRPYNSAEVEKIVADEKNNREKIALEKNKDKVKEACSKHLKVAAYCTTQVERNACLFCKARKLDDKFYRKLRGQFPDAVFWQEIGEIFRQLQKQAAEIYNQSLIELYYEIFIKGKGFANASSVEHYLSDVCYTRAAELFKNAAIASGLRGKVKSNFRLKELKNMKSGLPTTKSDNFPIPLVKQKGGQYTGFEISNHNGDFIIKIPFGRWQVKKEVDKYRPWEKLDFEQVRKSPKPISLLLSTQRRKRNKGWSKDEGTEAEIKKVMNGDYQTSYIEVKRGSKTGEKSAWMLNLSIEVPKIDKGVDPCIIGGIDVGVKSPLVCAINNAFSRYSISDNDLFHFNKKMFARRRILLKKNGHKRAGHGAKNKLRPITIMTEKSKRFRKKLIERWACEIADFFIKNKVGTVQMEDLESMKRKEDSYFNIRLRGFWPYAEMQNKIEFKLKQYGIEIRKVAPDNTSKTCSKCGHLNNYFNFEYRKKNKFPHFKCEKCNFKENADYNAALNISNPKLKSTKGEP

SEQ ID NO: 3015 - protein, 725 aa, synthetic construct
SEVEFSHEYWMRHALTLAKRARDEREVPVGAVLVLNNRAIGEGWNRAIGLHDPTAHAEIMALRQGGLVMQNYRLIDATLYVTFEPCVMCAGAMIHSRIGRVVFGVRNNKHGAAGSLVNVLNYPGMNHRVEITEGILADECAALLCDFYRMPRQVFNARKKARSNINSGCSSGGSSGSETPGTSESATPESSGGSSGGSTKNTITKTLKLRIVRPYNSAEVEKIVADEKNNREIALEKNKDKVREACSKHLKVAAYCTTQVERNACLFCKARKLDDKFYQKLRGQFPDAVFWQEIGEVFRQLQKQAAEIYNQSLIELYYEIFIKGKGFANASSVEHYLSDVCYTRAAELFKNAAIASGLRGKVKSNFRLKELKNMKSGLPTTKSDNFPIPLVKQKGGQYTGFEISSHNDDFIIKIPFGRWQVKKEINKHRPWEKFDFEQVRKSPKPISLLLSTQRRKRNKGWSKDEGTEAEIRKVMNGDYQTSYIEVKRGSKIGEKSAWMLNLSIDVPKIDKGVDPSIIGGIDVGVKSPLVCAINNALSRYSISDNDLFHFNKKMFARRRILLRKNRHKRAGHGARSKLKPITVLTEKSERFRKKLIERWACEIANFFIKNKVGTVQMENLESMKRREDSYFNTRLRGFWPYAEMQNKIEFKLKQYGIEIRKVAPNNTSKTCSKCGHLNNYFNFEYRKKNKFPHFKCEKCNFKENADYNAALNISNPRLKSTKEEP

SEQ ID NO: 3016 - protein, 726 aa, synthetic construct
SEVEFSHEYWMRHALTLAKRARDEREVPVGAVLVLNNRVIGEGWNRAIGLHDPTAHAEIMALRQGGLVLQNYRLVDATLYVTFEPCVLCAGAMVHSRIGRVVFGARNSKRGAAGSLMNILNYPGMNHRVEITEGILADECAALLCDFYRMPRQVFNAQKKARSNINSGGSSGGSSGSETLGTSESATPESSGGSSGGSAKNTITKTLKLRIVRPYNSAEVEKIVADEKNNREKIALEKNKDKVKEACSKHLKVAAYCTTQVERNACLFCKARKLDDKFYQKLRGQFPDAVFWQEIGEVFRQLQKQAAEIYNQSLIELYYEIFIKGKGFANASSAEHYLSDVCYTRAAELFKNAAIASGLRGKVKSNFRLKELKNMKSGLPTTKSDNFPIPLVKQKGGQYTGFEISSHNDDFIIKIPFGRWQVKKEIDKYRPWEKFDFEQVRKSPKPISLLLSTQRRKRNKGWSKDEGTEAEIRKVMNGDYQTSYIEVKRGSKIGEKSAWMLNLSIDVPKIDKGVDPSIIGGIDVGVKSPLVCAISNAFSRYSISDNDLFHFNKKMFARRRILLKKSKHKRAGHGAKNKLKPITILTEKSRRFRKKLIERWACEIADFFIKNKVGTVQMENLEGMKRKEDSYFNIRLRGLWPYAEMQNKIEFKLEQYGIRIRKVAPNNTSKTCSKCGHLNNYFNFEYRKKNKFPHFKCERCSFKENADYNAALNISNPKLKSTKEEP

SEQ ID NO: 3017 - protein, 726 aa, synthetic construct; identical to SEQ ID NO: 684

SEQ ID NO: 3018 - protein, 726 aa, synthetic construct
SEDEFSHEYWMRHALTLAKRARDGREVPVGAVLVLNNRVIGEGWNRTTGLHDPTAHAEIMALRQGGLVMQNHRLVDATLYVTFEPCVMCAGAMIHSRIGRVVFGVRNGKRGAAGSLTNVLNYPGMNHRVEITEGILVDECAALLCDFYRMPRQVFNAQKKAQSTINSGGSSGGSSGSETPGTSESPTPESSGGSPGGSAKNTITKTLKLRIVRPYNSAEVEKIVADEKNNREKIALEKNKDKVKEACSKHLKVAAYCTTQVERNACLFCKARKLDDKFYQKLRGQFPDAVFWQEIGEIFRQLQKQAAEIYNQSLIELYYEIFIKGKGFANASSVEHYLSDVCYTRAAGLFKNAAIASGLRGKVKSNFRLKELKNTKSGLPTTKSDNFPIPLVKQKGGQYTGFEISSHNDDFIIKIPFGRWQAKEEIDKYRPWEKFDFEQVRKNPKPISLLLSTQRRKRNKGWSKDEGTEAEIRRVMNGDYQTSYIEVKRGSKIGEKSAWMLNLSIDVPKIDKGVDPSIIGGIDVGVKSPLVCAINNAFSRYSISDNDLFHFNKKMFARRRILLKENGHRRAGHGAKNKLKPITIMTEKSKRFRKKLIERWACEIADFFIKNKVGTVQMENLESMKRKEDSYFNIRLRGFWPYAEMQNKIEFKLKQYGIKIRKVAPNNTSKTCSKCGHLNNYFSFEYRKKNKFPHFKCEKCNFKEDADYNAALNISNPKLKSTKEEP

SEQ ID NO: 3019 - protein, 726 aa, synthetic construct
SEDEFSHEYWMRHALTLAKRARDGREVPVGAVLVLNNRVIGEGWNRAIGLHDPTAHAEIMALRQGGLVMQNYRLIDATLYVTFEPCVMCAGAMVHSRIGRVVFGVRNSKRGAAGSLMNVLDYPGMGHRVEITEGILADECAALLCGFYCMPRQVFNAQKKAQSSINSGGSSGGSSGSETPGTSESATPESSGGGSSGSAKNTITKTLQLRIVRPYNSAEVEKIVADEKNNREKTALEKNKDKVKEACSEHLKVAAYCTTQVERNACLFCKARKLDDKFYQKLRGQFPDAVFWQEIGEIFRQLQKQAAEIYNQSLIELYYEIFIKGKGFANASSVEHYLSDVCYTRAAELFKNAAIASGLRGKVKSNFRLKELKNMKSGLPTTRSDNFPIPLVKQKGGQYTGFEISSHNDDFIIKIPFGRWQVKKEIDKYRPWEKFDFEQVRKSPRPISLLLSTQRRKRNKGWSRDEGTEAEIRKVMNGDYQTSYIEVKRGSKIGEKSAWMLNLSIDVPKIDKGVDPSIIGGIDVGVKSPLVCAINNAYSRYSISDNDLFHFNKKMFARRRILLKKTRHKRAGHGAKNKLKPVSILTEKSERFRKKLIERWACEIADFFIKNKVGTVQMENLESMKRREDSYFNIRLRGFWPYAKMQNKIEFKLKQYGIEIRKVAPNNTSKTCSKCGHLNNYFNFEYRKKNKFPHFKCEKCNFKESADYNAALNISNPKLKSTKEEP

SEQ ID NO: 3020 - protein, 725 aa, synthetic construct
SEVEFSHEYWMRHALTLAKRARDEREVPVGAILVLNNRVIGEGWNRAIGLHDPTAHAEIMALRQGGLVMQNYRLIDATLYVTFEPCVMCAGAMIHSRIGRVVFGVRNSKHGAAGSLVNVLNYPGMNHRVEITEGILADECAALLCDFYRMPRRVFNARKKAQSSIDPGGTSGGSSGSETPGTSECATPESSGGRSGGSAKNTITKTLKLRIVRPYNSTEVEKIVADEKNNREKIALEKNKDKVKEACSKHLKVASYCTTQVERNACLFCKARKLDDKFYQKLRGQFPDAVFWQELGEIFRQLQKQAAEIYNQSLIELYYEIFIKGKGFANASSVEHYLSNVCYTRAAELFKNAAIASGLRGKVKSNFRLKELKNMKSGLPTTKSDNFPIPLVKQKGGQYTGFEISSHNDDFIIKIPFGRWQVKREIDKYRPWEKFDFEQVRKSPKPISLLLSTQRRKRNKGWSKDEGTEAEIRKVMNGDYQTSYIEVKRGSKIGEKSAWMLNLSIDVPKIDKGVDPSIIGGVDVGVKSPLVCAINNAFSRYSISDNDLFRFNKRMFARRRILLKKNRHKRAGHGAKSKLKPISILTEKSERFRKKLIERWACEIADFFIKNKVGTVMENLESMKRKEDSYFNIRLRGFWPYAEMQNKIEFKLKQYGIEIRKVAPNNTSKTCSKCGHLNNYFNFEYRKKNKFPHFKCEKCNFKENADYNAALNISNPKLKSTKEEP

SEQ ID NO: 3021 - protein, 726 aa, synthetic construct
SEVEFSHEYWMRHALTLAKRARDEREVPVGAVLVLNNRVIGEGWNRAIGLHDPTAHAEIMALHQGGLVTQNYRLIDATLYVTFEPCVMCAGAMIHSRIGRVVFGARNSKRGAAGSLMNVLSNPGMNHRVEITEGILADECAALLCDFYRMPRRVFNAQKKAQSSINSVGSSGGGSGSETPSTSESATPESSGGSSGGPVKNTITKTLQLRIVRPYNSAEVEKIVADEKNNREKIALEKNKDKVKEACSKHLKVAAYCTTQVERNACLFCKARKLDDRFYQKLRGQFPDAVFWQEVGEIFRQLQKQAAETYNQSLIELYYEIFIKGKGFANASSVEHYLSDVCYTRAAELFKNAAIASGLRGKVKSNFRLKELKNMKSGLPTTKSDNFPIPLVKQKGGQYTGFEISSHNDDFIIKIPFGRWQVKKEIDKYRPWEKFGFEQVRKSPKPISLLLSTQRRKRNKGWSKDEGTEAEIRKVMNGDYQTSYIEVKRGSKIGEKSAWMLSLSIDVPKIDKGVDPNIIGGIDVGVKSPLVCAINNAFCRYSISDNDLFHFNKKMFARRRILLKKSRHKRAGHGAKNKLKPISILTEKSKRFRKKLIERWACEIADFFIKNKVGTVQMENLESMKRKEDSYFNIRLRGFWPYAEMQNKIEFKLKQYGIEIRKVAPNNTSKTCSMCGHLNNYFNFEYRKKNKFPHFKCEKCNFKENADYNAALNISNPKLKSTKEEP

SEQ ID NO: 3022 - protein, 726 aa, synthetic construct
SEVEFSHEYWMRHALTLAKRARDEREVPVGAVLVLNNRVIGEGWNRTTGLHDPTAHAEIMALRQGGLVMRNYRLTDATLYVTFEPCVMCAGAMIHSRIGRVVFGVRNSKRGAAGSLMNVLNYPGMNHCVEITEGILVDECAALLCDFYRMPRQVLNAQRKAQSSISPGGSSGGSSGSVTPGASESVTPESSGGGSSGSAKNTITKTLQLRIVRPYNSAEVEKIVADEKNNREKIAMEKNKDKVKEACSKHLKVASYCTTQVERNACLFCKARKLDDKFYQKLRGQFPDAVFWQELGGIFRQLQKQSAEIYNQSLIELYYEIFIKGKGITNASRVEHYLSDVCYTRAAELFKNAAIASGLRSKVRSNFRLKELKNMKSGLPTTKSDNFPIPLVKQKGGQYTGFEISSHNDDFIIKIPFGRWQVKEEIDKYRPWEKFDFEQVRKNPKPISLLLSTLRRKRNKGWSKDEGTEAEIRKVMNGDYQTSYIEVKRGSKIGEKSAWMLNLSIDVPKIDKGADPSVIGGIDVGVKSPLVCAINNAFSRYSISDNDLFRFNKKVFARRRILLKKNRHKRAGHGTKNKLKPITILTEKSGRFRKKLIERWACEIANFFIKNKVGTVQMENLEGMKRKEDSYFNIRLRGFWPYAEMQNKIEFKLKQYGIKIRKVAPNNTSKTCSKCGHLNSYFNFEYRKKNKFPHFKCKKCNFKENADYNAALNISNPKLKSTKEEP

SEQ ID NO: 3023 - protein, 726 aa, synthetic construct
SEVEFSHEYWMRRALTLAKRARDEREVPVGAVLVLNNRVIGVGWNRAVGLHDPTAHAEIMALRQGGLVMQNYRLIEATLYVTFEPCIMCAGAMIHSRIGRVVFGVRNSKHGAAGSLVNVLDYPGMNRRVKITEGILADECAALLCDFYRMPRQVFNARKRAQSSINPGGSSGGSSGSETPGTSESATPKSSGGSSGGSAKNTITKTLKLRIVRPYNSAEVEKIVADEKDNREKIALEKNKDKVQEACSKHLKVASYCTTQVERNACLFCKARKLDDKFYQKLRGQFPDAVFWQELGEIFRQLQKQAAEIYNQSLIELYYEIFIKGKGFANASSVEHYLSDVCYTRAAELFKNAAIASGLRGKVKSNFRLKELKNMKSGLPTTKSDNFPIPLVKQKGGQYTGFEISSHNDDFIIKIPFGRWQVKKEIDKYKPWEKFDFEQVRKSPKPISLLLSTQRRKGNKGWSKDEGTEAEIRKVMNGDYQTSYIEVKRGSKIGEKSAWMLNLSIDVPKIDKGVDPSIIGGIDVGVRSPLVCAIDNSFSRYSISDNDLFHFNKKMFARRRILLKKNRHKRAGHGAKNKLRPISILTEKSKRFRKKLIERWACEIADFFIKNKVGTVQMENLESMKRKEDSCFNIRLRGFWPYAEMQNKIKFKLKQYGIEIRKVAPNNTSKTCSKCGHLNNYFNFEYRKKNKFPHFKCEKCNFKEDADYNAALNISNPKLKSTKEEP

SEQ ID NO: 3024 - protein, 726 aa, synthetic construct
SEVEFSHEYWMRHALTLAKRARDEREVPVGAILVLNNRVIGEGWNRAIGLHDPTAHAEIMALRQGGLVMQNYRLIDATLYVTFEPCVMCAGAMIHSRIGRVVFGVRNNKHGAAGSLMNVLNHPGMNHRVEITGGILADECAALLCDFYRMPRQVFNAQKKARSNINSGGSSGGSSGSETLGTSESATPESSGGSSGGSAKNTITKTLKLRIVRPYNSAEVEKIVADEKNSREKIALEKNKDKVKEACSKHLKVAAYCTTQVERNACLFCKARKLDDKFYQKLRGQFPDAVFWQEIGEVFRQLQKQAAEIYNQSLIELYYVIFIKGKGLANASSVEHYLSDVCYTRAAELFKNAAIASGLRGKVKSNFKLKELKSMKSGLPSTKSDNFPIPLVKQRGGQYTGFKISSHNDDFIVKIPFGRWQVKKEIDKYRPWEKFDFEQVRKSPKPISLLLSTQRRKRNKGWSKDEGTEAEIKKVMSGDYQTSYIEVKRGRKIGEKSVWMLNLSIDVPKIDKGVDPSTIGGIDVGVKSPLVCAINNAFSRYSISDNDLFRFNKKMFARRRILLKKNRHKRAGHGAKNKLKPITILTEKSGRFRKKLIERWACEIADFFIKNKVGTVQMENLESMKRKEDSYFNIRLRGFWPYAEMQNKIEFKLKQYGIEVRKVAPDNTSKTCSKCGHLNNYFNFEYRKKNKFPHFKCEKCNFKENADYNAALNISNPKLKSTKEEP

SEQ ID NO: 3025 - protein, 726 aa, synthetic construct
SEVEFSHEYWMRHALTLAKRARDEREVPVGAVLVLNNRVIGEGWNRAIGLHDPTAHAEIMALRQGGLVMQNYRLVDATLYVTFEPCVLCAGAMVHSRIGRVVFGVRNSKRGAAGSLMNVLNYPGMNHRVEITEGILADECAALLCDFYRMPRQVFNAQKKARSNINSGGSSGGSSGSETPGTSESATPESSGGSSGGSAKNTITKTLQLRIVRPYNSAEVEKIVADEKNSREKIALEKNKDKVKEACSKHLMVASYCTTQVERSACLFCKARELDGKFYQKLRGQFPDAVFWQELGEIFRQLQKQAAEIYNQSLIELYYEIFVKGKGIANTSRMEHYLSDVCYTRAAGLFKNAAIASGLRGKIKSNFRLKELKSMKSGLPTTRSDNFPIPLVKQKGGQYTGFEISSHNSDFIIKIPFGRWQVKEEIDKFRPWEKFDFEQVRKSPKPISLLLSTQRRKKNKGWSKDEGTEAEIRRVMNGDYQTSYIEVKRGSKIGEKSAWMLNLSIDVPKIDKGVDPSIIGGIDVGVKSPLVCAINNSSSRYSICDNDLFRFNKKMFARRRILLKKNRHKRAGHGAKNKLKPITILTEKSKRFRKKLIERWVCEVADFFIKNKVGTVQMENLESMKRKEDSYFNIRLRGFWPYAEMQNRIELKLKQYGIEIRRVAPNNTSRTCSKCGHLNNYFNFEYRKRSKFPHFKCEKCNFREDADYNAALNISNPKLKSTKEEP

SEQ ID NO: 3026 - protein, 726 aa, synthetic construct
SEVEFSHEYWMRHALTLAKRARDEREVPVGAILVLNNRVIGEGWNRAIGLHDPTAHAEIMALRQGGLAMQNYRLVDATLYVTFEPCVLCAGAMVHSRIGRVVFGVRNSKRGAAGSLMNVLNYPGMNHRVEITEGILADECAALLCDFYRMPRQVFNAQKKARSNINSGGSSGGSSGGKAPGTSESATLESSGGSSGDSAKNSITKTLKLRIVRPYNSAEVEKIVADEKNNREKIALEKNKGKVEEACSKHLKVATYCTTQVERNACLFCKARKLDDKFYQKLRGQFPDAVFWQEIGEIFRQLQKQAAEIYNQSLIELYYEIFIKGKGFTNASSVEHYLSDVCYTRAAELFKNAAIASGLRGKVKSNFRLKELKNMKSGLPTTKSDNFPIPLVKQKGGQYTGFEISSLNDDFIIKIPFGRWQVKKEIDKYRPWEKFDFEQVRKSPKPISLLLSTQRRKKNKGWSKDEGTEAEIRRVMNGDYQTSYIEVKRGSKTGEKSAWMLNLSVDVPKIDKGVDPSIIGGIDVGVKSPLVCAINNALSRYSISDNDLFHFNKKMFARRRILLRKNRHKRAGHGARNKLKPITVLTEKSERFRKKLIERWACEIANFFIKNKVGTVQMENLESMKRREDSYFNIRLRGFWPYAEMQSKIEFKLKQYGIKIRKVAPNNTSKTCSKCGHLNNYFNFEFRKKNKFPHFKCEKCNFKEDADYNAALNISNPKLKSTKEEP

SEQ ID NO: 3027 - protein, 726 aa, synthetic construct
SEVEFSHEYWMRHALTLAKRARDEREVPVGAVLVLNNRVIGVGWNRTTGLHDPTAHAEIMALRQGGLVMQNHRLVDATLYVTFEPCVMCAGAMIHSRIGRVVFGVRNSKHGAAGSLVNVLNYPGMNHRVEITEGILADECAALLCDFYCMPRQVFNAQKRAQSSINSGGSSGGSSGSETPGTSESATPESSGGGSSGSAKNTITKTLQLRIVRPYNSAEVEKIVADEKNSREKIALEKNKDKVKEACSKHLMVASYCTTQVERSACLFCKARELDGKFYQKLRGQFPDAVFWQELGEIFRQLQKQAAEIYNQSLIELYYEIFVKGKGIANTSRMEHYLSDVCYTRAAGLFKNAAIASGLRGKIKSNFRLKELKSMKSGLPTTRSDNFPIPLVKQKGGQYTGFEISSHNDDFIIKIPFGRWQVKKEIDKYRPWEKFDFEQVRKSPKPISLLLSTQRRKRNKGWSKDEGTEAEIEKVMNGDYQTSYIEVKRGSKTGGKSAWMLNLSIDVPKIDKGVDPCIIGGIDVGVKSPLVCAINDAFSRYSISDNDLFHFNKKMFARRRILLKKNGHKRAGHGAKNKLKPITIMTEKSKRFRKKLIERWACEIADFFIKNKVGTVQMENLESMKRKEDSYFNIRLRGFWPYAEMQNKIEFKLKQYGIVVRKVAPNNTSKTCSECGHLNNYFNFEYRKKNKFPHFKCEKCNFKENADYNAALNISNPKLKSTKKEP

SEQ ID NO: 3028 - protein, 725 aa, synthetic construct
SEVEFSHEYWMRHALTLAKRARDAREVPVGAILVLNNRVIGEGWNRAIGQHDPTAHAEIMALRQGGLVMQNYRLTDATLYVTFEPCVMCAGAMIHSRIGRVVFGVRNSKHGAAGSLMNVLNYPGMNHRVEITEGILADECAALLCDFYRMPRQVFNGRKKAQSSINSGGSSGGSSGSETPSTSESATPKSSGGSSGGSAKNTITKTLKLRIVRPYNSAEVEKIVADEKNNRERIALEKNKDKVKEACSKHLKVAAYCTTQVERNACLFCKARKLDDKFYQKLRGQFPDAVFWQEIGEIFRQLQKQAAEIYNQSLIELYYEIFIKGKGFANASSVEHYLSDVCYTRAAELFKNAAIASGLRSKIKSNFRLKELRNMRGGLPTTKSDNFPIPLVKQKGGQYTGFEISSHNDDFIIKIPFGRWQVKKEIDKYRPWGKFDFEQVRKSPKPISLLLSTQRRKRNKGWSKDEGTEAEIRKVMNGDYQTSYIEVKRGSKIGEKSAWMLNLSIDVPKIDKGVDPSIVGGIDVGVKSPLVCAIDNALSRYSISDNDLFHFNKKMFARRRILLKKNGHRRAGHGAKNKLKPISILTEKSKRFRKKLIERWACEIADFFIKNKVGTVMENLESMKRKEDSYFNTRLRGIWPYAEMQNKIEFKLKQYGIEIRKVAPNNTSKTCSKCGHLNNYFNFEYRKKNKFPHFKCEKCNFKENADYNAALNISNPKLKSTKEEP

SEQ ID NO: 3029 - protein, 726 aa, synthetic construct
SEDEFSHEYWMRHALTLAKRARDGREVPVGAILVLNNRVIGEGWNRAIGLHDPTAHAEIMALRQGGLVMQNYRLIDATLYVTFEPCVMCAGAMIHSRIGRVVFGVRNSKHGAAGSLVNVLSYPGMNHRVEVTEGILADECAALLCDFYRMPRRVFNARKKAQSSINPGDSFGGSSGSETPGTSESATPESSGGSSGRSAKNAITKTLKLRIVRPYNSAEVEKIVADEKNNREKIALEKNKGKVKEACSKHLKVAAYCTTQVERNACLFCKARRLDDKFYQKLRGQFPDAVFWQEIGEIFRQLQKQAAEIYNQSLIELYYEIFIKGKGFASASSVEHYLSDVCYTRAAELFKNAAIASGLRGKVKSNFRLKELKNMKSGLPTTKSDNFPIPLVKQKGGQYTGFEISSHNDDFIIKIPFGRWQVKKEIDKYRPWEKFDFEQVRKSPKPISLLLSTQRRKRNKGWSKDEGTEAEIRKVMNGDYQTSYIEVKRGSKIGEKSAWMLNLSIDVPKIDKGVDPSIIGGIDVGVKSPLVCAINNALSRYSISDNDLFHFNKKMFARRRILLKKNRHRRAGHGAKNKLKPIAVLAEKSEGFRKKLIERWACEVADFFIKNKVGTVQMENLESMKRREDSYFNIRLRGFWPYAEMQNKIEFKLRQYGIEIRKVAPDNTSKTCSKCGHLNNYFNFEYRKKNKFPHFKCEKCNFKENADYNAALNISNPKLKSAKEEP

SEQ ID NO: 3030 - protein, 726 aa, synthetic construct
SEVEFSHEYWMRHALALAKRARDEREVPVGAILVLNNRVIGEGWNRAIGLHDPTAHAEIMALRQGGLVMQNYRLIDATLYVTFEPCVMCAGAMIHSRIGRVVFGVRNSKHGAAGSLVNVLNYPGMNHRVEITEGILADECAALLCDFYRMPRQVFNARKKAQSSINPSGSSGGSSGSVTPGTSESATPESSGGGFGGSAKNTITKTLQLRIVRPYNSAEVEKIVADEKNNREKIALEKNKDKVKEACSKHLKVASYCTTQVERNACLFCKARKLDDKFYQKLRGQFPDAVFWQELGEIFRQLQKQAAEIYNQSLIELYYVIFIKGKGLANASSVEHYLSDVCYTRAAELFKNAAIASGLRGKVKSNFKLKELKSMKSGLPSTKSDNFPIPLVKQRGGQYTGFEISSHNDDFIIKIPFGRWQAKKEIDKYRPWEKFDFEQVRKSPKPISLLLSTQRRKRNKGWSKDEGTEAEIKKVMNGDYQISYIEVKRGSKIGEKSAWTLNLSIDVPKIDKGVDPSIIGGIDVGVKSPLVCAINNSFSRYSICDNDLFRFNKKMFARRRILLKKNRHKRAGHGAKNKLKPITILTKKSERFRKKLIERWVCEVADFFIKNKVGTVQMENLESMKRKEDSYFNIRLRGFWPYAEMQNRIELKLKQYGIEIRRVAPDNTSRTCSKCGHLNNYFNFEYRKKNKFPHFKCEKCNFREDADYNAALNISNPKLKSTKEEP

SEQ ID NO: 3031 - protein, 726 aa, synthetic construct
SEVEFSHEYWMRHALTLAKRARDEREVPVGAVLVLNNRVIGEGWNRAVGLHDPTAHAEIMALRQGGLVMQNYRLVDATLYVTFEPCVLCAGAMVHSRIGRVVFGVRNSKRGAAGSLMNVLDYPGMNHRVEITEGILADECAALLCDFYRMPRQVFNAQKKARPNINSGGSSGGRSGSETPGTSESATPESSGGSSGDSAKNTITKTLKLRIVRPYNSAEVEKIVADEKNNRERVALEKNKDKVKEACSEHLRVAAYCTTQVERNACLFCKARKLDDKFYQKLRGQFPDAVFWQEIGEIFRQLQKQAAEIYNQSLIELYYEIFIKGKGFANASSVEHYLSDVCYTRAAELFKNAAIASGLRGKVKSNFRLKELKNMKSGLPTTKSDNFPIPLVKQKGGQYTGFEISSHNDDFIIKIPFGRWQVKEEIDKYRPWEKFDFEQVRKSPKPISLLLSTQRRKRNKGWSKDEGTEAEIRKVMNGDYQTSYIEVKRGSKIGEKSAWVLNLSIDVPKIDKGVDPSIIGGIDVGVKSPLVCAINNAFSRYSISDNDLFRFNKKMFARRRILLKKNRHKRAGHGAKNKLKPISILTGKSERFRKKLIERWACEIADFFIKNKVGTVQMENLESMKKKEDSYFNIRLRGFWPYAEMQNRIEFKLKQYGIEIRKVAPNNTSKTCSKCGHLNNYFNFEYRKKNKFPHFKCEKCNFKENADYNAALNISNPKLKSTKEEP

SEQ ID NO: 3032 - protein, 726 aa, synthetic construct
SEVEFSHEYWMRRALTLAKRARDEREVPVGAVLVLNNRVIGEGWNRAIGLHDPTAHAEIMALRQGGLVLQNYRLVDATLYVTFEPCVLCAGAMVHSRIGRVVFGARNSKRGAAGSLMNILNYPGMNHRVEITEGILADECAALLCDFYRMPRQVFNAQKKAQSSINSGGSSGGSSGSETPSTSESATPESSGGSSGGSAKNTITKTLQLRIVRPYNSAEVEKIVADEKNNRERIALEKNKDKVKEACSKHLKVAAYCTTQVERNACLFCKARKLDDKFYQKLRGQFPDAVFWQEIGEIFRQLQKQAAEIYNQSLIELYYEIFIKGKGFANASSVEHYLSDVCYTRAAELFKNAAIASGLRGKVKSNFRLKELKNMRSGLPTTKSDNFPIPLVKQKGGQYAGFEISSHNDDFIIKIPFGRWQVKKEIDKYRPWEKFDFGQVRKSPKPISLLLSTRRRKRNKGWSKDEGTEAEIRKVMNGDYQTSYIEVKRGSKIGEKSAWMLSLSIDVPKIDKGVDPSIIGGIDVGVKSPLVCAINNAFGRYSISDNDLFHFNKKMFAMRRILLKKNRHKRAGHGAKNKLKPITILTEKSKRFRKKLIERWACEIADFFIKNKVGTVQMENLESMKRKEDSYFNIRLRGFWPYAEMQDKIEFKLKQYGIEIRKVAPNNTSKTCSRCGHLNNYFNFEYRKKNKFPHFKCEKCNFKEDADYNAALNISNPKLKSPKEEP

SEQ ID NO: 3033 - protein, 726 aa, synthetic construct
SEVEFSHEYWMRRALTLAKRARDEREVPVGAVLVLNNRVIGVGWNRAVGLHDPTAHAEIMALRQGGLVMQNYRLIEATLYVTFEPCIMCAGAMIHSRIGRVVFGVRNSKRGAAGSLMNVLNYPGMNHRVEITKGILADECAALLCDYYRMPRQVFNARKKAQSSINSGGSSGGSSGSETPGASESVTPKSSVGSSAGSTKNTITKTLKLRIVRPYNSAEVEKIVADEKDNRERIALEKNKDKVKEACSKHLRVAAYCTTQVERNACLFCKARRLDDKFYQKLRGQFPDAVFWQEIGEIFRQLQKQAAEIYNQSLVELYYEILIKGKGIANASSVEHYLSDVCYTRAAELFKNAAIASGLRNKIKSNFRLKELRNMKSGLPTTKSDNFPIPLVRQKGGQYTGFEISNHNDDFIIKIPFGRWQVKKEIDKYRPWEKFDFEQVRKSPKPISLLLSTQRRKKNKGWSKDEGTEAEIRRVMNGDYQTSYIEVKRGSKIGEKSAWMLNLSIDVPRIDKGVDPSIIGGIDVGVKSPLVCAINNAFSRYSISDNDLFHFNKKMFARRRILLKKNRHKRAGHGAKNKLKPISILTEKSKRFRKKLIERWACEIADFFIKNKVGTVQMENLESMKRKEDSYFNIRLRGFWPYAEMQDRIEFKLKQYGIEIRRVAPNNTSRTCSKCGHLNNYFNFEYRKKSKFPHFKCEKCNFREDADYNAALNISNPKLKSTKEEP

SEQ ID NO: 3034 - protein, 726 aa, synthetic construct
SEVEFSHEYWMRHALTLAKRARDEREVPVGAILVLNNRVIGEGWNRAIGQHDPTAHAEIMALRQGGLVMQNYRLIDATLYVTFEPCVMCAGAMIHGRIGRVVFGVRNSKHGAAGSLMNVLNYPGMNHRVEITEGILADECAALLCDFYRMPRQVFNARKKAQSSTNPGGLSGGSSGGETPGTSESPTPESSGGSSGGSAKNTITKTLKLRIVRPYNSAEVEKIVADEKNNREKIALEKNKDKVREACSKHLKVASYCTTLVERNACPFCKARKLDDKFYQKLRGQFPDAVFWQELGEILRQLQKQAAEIYNQSLIELYYEIFIKGRGFANAGSVEHYLSDVCYTRAAELFKNAAIASGLRNKIKSNFRLKELRNMKSGLPTTKSDNFPIPLVRQKGGQYTGFEISNHDGDFIIKIPFGRWRVKKEINKHRPWEKFDFEQVRKSPKPISLLLSTQRRKRNRGWSKDEGTEAEIRRVMNGDYQTSYIEVKRGSKIGEKSAWMLNLSIDVPKIDKGVDPSIIGGIDVGVKSPLVCAINNAFSRYSISDNELFHFNKKMFARRRILLKKNRHKRAGHGAKNKLKPISILTGKSERFRKKLIERWACEIADFFTKNKVGTVQMENLESMKRKEDSYFNIRLRGFWPYAEMQNKIEFKLKQYGIEIRKVAPNNTSKTCSKCGHLNNYFNFEFRKKNKFPHFKCERCNFKENADYNAALNISNPKLKSTKEEP

SEQ ID NO: 3035 - protein, 726 aa, synthetic construct
SEVEFSHEYWMRHALTLAKRARDEREVPVGAILVLNNRVIGEGWNRAIGLHDPTAHAEIMALRQGGLEMQNYRLIDATLYVTFEPCVMCAGAMIHSRIGRVVFGVRNNKHGAAGSLVNVLNYPGMNHRVEITEGILADECAALLCDFYRMPRQVFNARKKAQSSINPGGSSGGSSGSETPGTSESATPESSGGSSGSSAKNTITKTLKLRIVRPYNSAEVEKIVADEKNNREKIALEKNKDKVKEACSKHLKVAAYCTTQVERNACLFCKARRLDDKFYQKLRGQFPDAVFWQEIGEIFRQLQKQAAEVYNQSLVELYYEILIKGKGIANASSVEHYLSDVCYTRAAELFKNAAIASGLRNKIKSNFRLKELRNMRSGLPTTKSDNFPIPLVRQKGGQYTGFEISNHDGDFIIKIPFGRWQVKEEINKHRPWEKFDFEQVRKSPKPISLLLSTQRRKRNKGWSKDEGTEAEIKKVMSGDYQTSYIEVKRGSKTGEKSAWMLNLSIDVPKIDKGVDPCIIGGIDVGVKSPLVCAINNAFSRYSISDNDLFRFNKKVFARRRILLKKNRHKRAGHGTKNKLKPITILTEKSGRFRKKLIERWACEITNFFIKNKVGTVQMENLESMKRKEDSYFNIRLRGFWPYAEMQNRIEFKLKQYGIKIRRVAPNNTSKTCSKCGHLNNYFSFEYRKKNKFPHFKCEKCNFKEDADYNAALNISNPKLKSTKEEP

SEQ ID NO: 3036 - protein, 726 aa, synthetic construct
SEVEFSHEYWMRHALTLAKRARDEREVPVGAVLVLNNRVIGEGWNRAIGLHDPTAHAEIMALRQGGLVMQNYRLVNATLYVTFEPCVMCAGAMIHSRIGRVAFGVRNSKRGAAGSLMNVLNYPGMNHRVEITEGILAEECAALLCDFYRMPRQVFSARKKAQPSINPGGSSGGSSGSETPGASESVTPESSGGSSGGSAKDTITKTLKLRIVRPYNSAEVEKIVADEKNNREKIALEKNKDKVKEACSRHLEVAAYCTTQVERNACLFCKARKLDDKFYQKLRGQFPDAVFWQELGEIFRQLQKQAAEIYNQSLIELYYEIFIKGKGFANASSVEHYLSDVCYTRAAELFKNAAIASGLRGKVKSNFRLKELKNMKSGLPTTKSDNFPIPLVKQKGGQYTGFEISSHNDDFVIKIPFGRWQVKKEIDKYRPWEKFDFEQVRKGPKPISLLLSTQRRKRNKGWSKDEGTEAEIRKVMSGDYQTSYIEVKRGSKTGEKSAWMLNLSIDVPKIDKGVDPSIIGGIDVGVKSPLVCAINNALSRYSISDNDLFHFNKKMFARRRILLKRNRHKRAGHGAKNKLKPITILTEKSKRFRKKLIERWACEIADFFIKNKVGTVQMENLESMKRKEDSYFNIRLRGFWPYAELQNKIEFKLKQYGIVVRKVAPNNTSKTCSKCGHLNNYFNFEYRKMNKFPHFKCEKCNFKENADYNAALNISNPKLKSTKEEP

SEQ ID NO: 3037 - protein, 726 aa, synthetic construct
SEDEFSHEYWMRHALTLAKRARDGREVPVGAVLVLNNRIIGEGWNRAIGLHDPTAHAEIMALRQGGLVMQNYRLTDATLYVTFEPCVMCAGAMVHSRIGRVVFGVRNSKRGAAGSLMNVLNYPGVNHCVEITEGILVDECAALLCDFYRMPRQVLNAQKKAQSSISSGGSSGGCSGSEMPGASESVTPKSSGGSSGGSAKNTITKTLKLRIVRPYNSAEVERIVADEKDYREKVALEKNKDKVKEACSEHLKVAAYCTTQVERNACLFCKARKLDDKFYQKLRGRFPDAVFWQEIGEIFRQLQKQAAEIYNQSLIELYYEIFIKGKGITNASRVEHYLSDVCYTRAAELFKNAAIASGLRSKVRSNFRLKELKNMKSGLPTTKSDNFPIPLVKQKGGQYTGFEISSHNSDFIIKIPFGRWQVKEEIDKYRPWEKFDFEQVRKSPKPISLLLSTQRRKKNKGWSKDEGTEAEIRRVMNGDYQTSYIEVKRGSKIGEKSAWMLNLSIDVPKIDKGVDPSIIGGIDVGVKSPLVCAINNSSSRYSICDNDLFRFNKKMFARRRILLKKNGHKRAGHGAKNKLKPITILTKKSERFRKKLIERWVCEVADFFIKNKVGTVQMENLESMKRREDSYFNIRLRGFWPYAEMQNRIELKLKQYGIEIRKVAPNNTSKTCSKCGHLNDYFNFEYRRKNKFPHFKCEKCNFKENADYNAALNISNPKLKSTKEEP

SEQ ID NO: 3038 - protein, 726 aa, synthetic construct
SEVEFSHEYWMRHALALAKRARDEREVPVGAILVLNDRVIGEGWNRAIGLHDPTAHAEIMALRQGGLVMQNYRLIDATLYVTFEPCVMCAGAMIHSRIGRVVFGVRNNKHGAAGSLVNVLNYPGMNHRVEITEGILADECAALLCDFYRMPCQVFNARKKAQSSISPGGPSGGSSGSETPGTSESAAPESSGGSSGVSAKNTITKTLKLRIVRPYNSAEVEKIVADEKNNREKIALEKNKDKVKEACSKHLKVAAYCTTRVDRNACLFCKARRLDDKFYQKLRGQFPDAVFWQEIGEIFRQLQKQAAEVYNQSLVELYYEILIKGKGIANASSVEHYLSNVCYTRAAELFKNAAIASGLRNKIKSNFRLKELRNMKSGLPTTKSDNFPIPLVRQKGGQYTGFEISNHDGDFIIKIPFGRWRVKKEINKHRPWEKFDFEQVRKSPKPISLLLSTQRRKRNKGWSRDEGTEAEIRKVMNGDYQTSYIEVKRGSKIGEKSAWMLNLSIDVPKIDKGVDPGIIGGIDVGVKSPLVCAINNAFSRYSISDNDLFHFNKKMFARRRILLRENGHKRAGHGAKNKLKPITIMTEKSKRFRKKLIERWACEIADFFIKNKVGTVQMENLESMKRKEDSYFNIRLRGFWPYAEMQNKIEFKLKQYGIVVRKVAPNNTSKTCSECGHLNNYFNFEYRKKNKFPHFKCEKCNFKENADYNAALNISNPKLKSTKEEP

SEQ ID NO: 3039 - protein, 726 aa, synthetic construct
SEVEFSHEYWMRHALALAKRARDEREVPVGAVLVLNNRVIGEGWNRAIGLHDPTAHAEIMALRQGGLVMQNYRLVDATLYVTFEPCVLCAGAMVHSRIGRVVFGVRNSKRGAAGSLMNVLNYPGMNHRVEITEGILADECAALLCDFYRMPRQVFNAQKKAQSSINSGGSSGGSSGSETPSTSESATPESSGGSSGGSAKNTITKTLQLRIVRPYNSAEVEKIVTDEKNNREKIALEKNKDMVKEACSKHLKVASYCTTQVERNACLFCKARKLDDKFYQKLRGQFPDAVFWQEIGEIFRQLQKQAAEIYNQSLVELYYEILIKGKGIANASSVEHYLSDVCYTRAAELFKNAAIASGLRNKIKSNFRLKELRNMKSGLPTTKSDNFPIPLVRQKGGQYTGFEISDHNGDFIIKIPFGMWQVKKEFNKHRPWEKFDFEQVRKSPKPISLLLSTQRRKKNKGWSKDEGTEAEIRRVMNGDYQTSYIEVKRGSKIGEKSAWMLNLSIDVPKIDKGVDPRIIGGIDVGVKSPLVCAINNVLSRYSISDNDLFHFNKKMFARRRILLKKNGHKRAGHGAKNKLKPISILTEKSKRFRKKLIERWACEIADFFIKNKVGTVQIENLESMKRKEDSYFNIRLRGFWPYAEMQNKIEFKLKQYGIEIRKVAPNNTSKTCSKCGHLNNYFSFEYRKKNKFPHFKCEKCNFKEDADYNAALNISNPKLKSTKEEP

SEQ ID NO: 3040 - protein, 726 aa, synthetic construct
SEVEFSHEYWMRHALTLAERARDEREVPVGAVLVLNNRVIGEGWNRAIGLHDPTAHAEIMALRQGGLVMQNYRLTDATLYVTFEPCVMCAGAMIHSRIGRVVFGVRNSKRGAAGSLMNVLNYPGMNHCVEITEGILVDECAALLCDFYRMPRQVLNAQKKAQSSISSGGSSGGSSGSVTPGASGSVTPKSSGGSSAGSTKDTITKTLKLRIVRPYNSAEVEKIVADEKNNREEIALEKNKDKVKEACSKHLKVASYCTTQVERNACPFCKARKLDDKFYQRLRGQFPDAVFWQELGEILRQLQKQAAEIYNQSLIELYYEIFIEGRGFANASSVEHYLSDVCYTRAAELFKNAAIASGLRGKVKSNFRLKELKNMKSGLPTTKSDNFPIPLVKQKGGQYTGFEISSHNDDFIIKIPFGRWQVKKEIDKYRPWEKFDFEQVRKSPKPISLLLSTQRRKRNKGWSKDEGTEAEIRKVMNGDYQTSYIEVKRGSKTGEKSAWMLNLSIDVPKIDKGVDPCIIGGIDVGVKSPLVCAINNAFSRYSISDNDLFHFNKKMFARRRILLKENGHKRAGHGAKNKLKPITIMTEKSKRFRKKLIERWACEIADFFIKNKVGTVQMENLESMKRKEDSYFNIRLRGFWPYAEMQNKIEFKLKQYGIVVRKVAPNNTSKTCSECGHLNNYFNFEYRKKNKFPHFKCEKCNFKENADYNAALNISNPKLKSTKGEP

SEQ ID NO: 3041 - protein, 726 aa, synthetic construct
SEVEFSHEYWMRHALTLAKRARDGREVPVGAVLVLNNRVIGEGWNRAIGLHDPTAHAEIMALRQGGLVMQNYRLIDATLYVTFEPCVMCAGAMVHSRIGRVVFGVRNSKRGAAGSLMNVLDYPGMGHHVEITEGILADECAALLCDFYRMPRQVLNAQKKAQSSISSGGSSGGSSGSETPGASESATPKSSGGSTASSTKNTITKTLKLRIVRPYNSAEVEKIVADEKNNRERIALEKNKDKVKEACSKHLKVAAYCTTQVERNACLFCKARKLDDKFYQKLRGQFPDAVFWQETGEIFRQLQRQAAEIYNQSLIELYYEIFIKGKGFANASSVEHYLSDVCYTRAAELFKNAAIASGLRGKVKGNFRLKELRNMKSGLPTTKSDNFPIPLVKQKGGQYTGFEISSHNDDFIIKIPFGRWQARKEIDKYRPWEKFNFAQVRKSPKPISLLLSTQRRKRSKGWSKDEGTEAEIRKVMNGDYQTSYIEVKRGSKIGEKSAWMLSLSIDVPKIDKGVDPSIIGGIDVGVKSPLVCAINNAFNRYSISDNNLFHFNKKMFARRRILLKKNRHKRAGHGAKNKLKPISILTEKSERFRKKLIERWACEIADFFIRNKVGTVQMENLEGMKRKEDSYFNIRLRGFWPYAEMQNKIEFKLKQYGIEVRKVAPNNTSKTCSKCGHLNNYFNFEYRKKNKFPHFKCEKCNFKENADYNAALNISNPKLKSTKEEP

SEQ ID NO: 3042 - protein, 726 aa, synthetic construct
SEVEFSHEYWMRHALTLAKRARDEREVPVGAVLVLNNRVIGEGWNRAIGLHDPTAHAEIMALRQGGLVMQNYRLTDATLYVTFEPCVMCAGAMIHSRIGRVVFGVRNSRRGAAGSLMNVLNYPGMNHCVEITEGILMDECAALLCDFYRMPRQVLNAQKKAQSSISSGGPSGGSSCSETPGASESVTPKSSGGSSTGSTKNTITKTLKLRIVRPYNSAEVEKIVADEKNSREKIALEKNKDKVKEACSEHLKVAAYCTTQVERSACLFCKARKLDDKFYQKLRGQFPDAVFWQEIGEIFRQLQKQAAETYNQSLIELYYEIFIKGKGITNASRVEHYLSDVCYTRAAELFKNAAIASGLRSKVRSNFRLKELKNMKSGLPTTKSDNFPIPLVKQKGGQYTGFEISSHNSDFIIKIPFGRWQVKEEIDKYRPWEKFDFEQVRKSPKPISLLLSTQRRKKNKGWSKDEGTEAEIRRVMNGDYQTSYIEVKRGSKIGEKSAWMLNLSIDVPKIDKGVDPSITGGIDVGVKSPLVCAINNSFSRYSICDNDLFRFNKKMFARRRILLKRNRHKRAGHGAKNKLKPITILTKKSERFRKKLIERWVCEVADFFIKNKVGTVQMENLESMKRKEDSYFNIRLRGFWPYAEMQNRIELKLKQYGIEIRRVAPNNTSRTCSKCGHLNNYFNFEYRKKNKFPHFKCEKCNFREDADYNAALNISNPKLKSTKEEP

SEQ ID NO: 3043 - protein, 726 aa, synthetic construct
SEDEFSHEYWMRHALTLAKRARDGREVPVGAVLVLNNRVIGEGWNRAIGLHDPTAHAEIMALRQGGLVMQNYRLVDATLYVTFEPCVMCAGAMVHSRIGRVVFGVRNGKRGAAGSLMNILDYPGMGHRVEITEGILADECAALLCDFYCMPRQVFNAQRRAQSSINSGGSSGGSSGSVTPGTSESATPESSGGSSGGPAKNTITKTLKLRIVRPYNSAEVEKIVADEKNNREKTALEKNKDKVKEACSKHLKVAAYCTTQVERNACLFCKARRLDDKFYQKLRSQFPDAVFWQEIGEIFRQLQKQAAEIYNQSLVELYYEILIKGKGIANASSVEHYLSDVCYTRAAELFKNAAIASGLRGKVKSNFRLKELKSMKSGLPTTKSDNFPIPLVKQKGGQYTGFEISSRNSDFIIKIPFGRWQVKKEINKYRPWEKFDFEQVRKSPKPISLLLSTQRRKRNKGWSKDEGTEAEIRKVMNGDYQTSYIEVKRGSRIGEKSAWMLSLSIDVPKIDRGVDPSIIGGIDVGVKSPLVCAINNALSRYSIGDNDLFHFNKKMFARRRILLKKNRHRRAGHGARNKLKPITVLTEKSKRFRKKLIERWACEIADFFIRNKVGTVQIENLESMKRKEDSYFNIRLRGFWPYAEMQNKIEFKLKQYGIEIRKVAPNNTSKTCSKCGHLNNYFDFEYRKKNKFPRFKCEKCNFKENADYNAALNISNPKLKSTKEEP

SEQ ID NO: 3044 - protein, 726 aa, synthetic construct
SEVEFSHEYWMRHALTLAKRARDKHEVPVGAVLVLNNRVIGEGWNRATGQNDPTAHAEIMALRQGGLVMQNHRLIDATLYVTFEPCVMCAGAMIHSRIGRVVIGVRNSKRGAAGSLMNVLNYPGMNHRVEITEGILADECAALLCDFYRMPRQVFNARKKAQSSINSGGSSGGSSGSETPGTSESATPKSSGGSSGGSAKNTITKALKLRIVRPYNSAEVEKIVADEKNNREKIALEKNKDKVQEACSKHLKVASYCITQVERNACLFCKARKLDDKFYQKLRGQFPDAVFWQELGEIFRQLQKQAAEIYNQSLIELYYEIFIKGKGLANASSVEHYLSDVCYTRAAELFKNAAIASGLRGKVKSNFKLKELKSMKSGLPSTKSDNFPIPLVKQKGGQYTGFEIRGHNDDLIIKIPFGRWQVKKEIDKYRPWEKFDFEQVRKSPKPISLLLSTQRRKRNKGWSKDEGTEAEIRKVMNGDYQTSYIEVKRGSKIGEKSAWMLNLSIDVPKIDKGVDPGIIGGIDVGVQSPLVCAINNAFSRYSISDNDLFHFNKKMFARRRILLKKNGHKRAGHGAKNKLKPITIMTEKSKRFRKKLIERWACEIADFFIKNKVGTVQMENLESMKRKEDSYFNIRLRGFWPYAEMQNKIEFKLKQYGIEIRKVAPNNTSKTCSKCGHLNNYFNFEYRKENKFPHFKCEKCNFREDADYNAALNISNPKLKSTEEEP

SEQ ID NO: 3045 - protein, 726 aa, synthetic construct
SEDEFSHEYWMRHALTLAKRARDGREVPVGAVLVLNNRVIGEGWNRAIGLHDPTAHAEIMALRQGGLVMQNYRLIDATLYVTFEPCVMCAGAMIHSRIGRVVFGVRNSKHGAAGSLMNVLNYPGMNHRVEITEGILVDECAALLCDFYRMPRQVFNARKKAQSSINPGGSFGGGSGSETPGTSESATLESSGGSSGGSAKNTITKTLKLRIVRPYNSAEVERIVADEKDSREKIALEKNKDKVKEACSRHLRVAAYCTTQVERNACLFCKARKLDDKFYQKLRGQFPDAVFWQEISEIFRQLQKQAAEIYNQSLIELYYEIFIKGKGIANASSVEHYLSDVCYTRAAELFKNAAIASGLRNKIKSNFRLKELRNMKSGLPTTKSDNFPIPLVRQKGGQYTGFEISNYNGDFIIKIPFGRWQVKKEINKHRPWEKFDFEQVRKSPKPISLLLSTQRRKRNKGWSKDEGTEAEIRRVMNGDYQTSYIEVKRGSKIGEKSAWMLNLSIDVPKIDKGVDPSIIGGIDVGVKSPLVCAINNALSRYSISDNDLFHFNKKMFARRRILLRKNRHKRAGHGARNKLKPITVLTEKCERFRKKLIERWACEIANFFIKNKVGTVQMENLESMKGKEDSYFNIRLRGFWPYAEMQNKIEFKLKQYGIEIRKVAPNNTSKTCSKCGHLNNYFNFEYRKKNKFPHFKCEKCYFKEDADYNAALNISNPKLKSTKEEP

SEQ ID NO: 3046 - protein, 726 aa, synthetic construct
SEVEFSHEYWMRHALTLAKRARDEREVPVGAVLVLNNRVIGVGWNRAIGLHDPTAHAEIMALRQGGLVMQNYRLTDATLYVTFEPCVMCAGAMVHSRIGRVVFGVRNSKRGAAGSLMNVLNYPGMSHCVEITEGILVDECAALLCDFYRMPRQVLNAQKKAQSSISSGGSSEGSGGSETPGTSESATPESSGGGSSGSAKNTITKTLQLRIVRPYNSAEVEKIVADEKNYREKIALEKNKDKVKEACSKHLKVASYCTTQVERNACPFCKARKLDDKFYQKLRGQFPDAVFWQEIGEIFRQLQKQAAEIYNQSLIELYYEIFIKGKGIANAGSVEHYLSDVCYTRAAELFKNAAIASGLRNKIKSNFRPKELKNMKSGLPTTKSDNFPIPLVKQKGGQYTGFEISNHNSDFIIKIPFGRWQAKEEIDKYRPWERFDFEQVRKSPKPISLLLSTQRRKRNRGWSKDEGTEAEIRKVMNGDYQTSYIEVKRGGKIGEKSAWMLNLSIDVPKIDKGVDPSIIGGIDVGVKSPLVCAINNAFNRYSISDNDLFRFNKKMFARRRILLEKNRHKRAGHGVKNKLKPISILTEKSKRFRKKLIERWACEIADFFIKNKVGTVQMENLESIKRREDSYFNIRLRGFWPYAKMQNKIEFKLKQYGIKIRKVAPNNTSKTCSKCGHLNNYFNFEYRKRNKFPHFKCEKCNFKEDADYNAALNISNPKLKSTKEEP

SEQ ID NO: 3047 - protein, 726 aa, synthetic construct
SEAEFSHEYWMRHALTLARRARDEREVPVGAILVLDNRVIGGGWNRAIGLHDPTAHAEIMALRQGGLVMQSYRLADATLYVTFEPCVMCAGAMIHSRIGRVVFGVRNSKHGAAGSLMNVLSYPGMNHRVEITEGILADECAALLCDFYRMPRRVFNAQKKAQSSINSGGSSDGSSSSETPGTSGSATPEGSGGSSGGSAKNTITKTLKLRIVRPYNSAEVEKIVADEKNNREKIALEKNKDKVKEACSKHLKVASYCTTQVERNACLFCKARKLDDKFYQKLRGQFPDAVFWQELGEIFRQLQKQAAEIYNQSLIELYYEIFIKGKGFANASSVEHYLSDVCYTRAAELFKNAAIASGLRSKVRSNFRLKELKNMKSGLPTTKSDNFPIPLVKQKGGQYTGFEISSHNSDFIIKIPFGRWQVKEEIDKYRPWEKFDFEQVRKSPKPISLLLSTQRRKKNKGWSKDEGTEAEIRRVMNGDYQTSYIEVKRGSKIGEKSAWMLNLSVDVPKIDKGVDPSIIGGIDVGVKSPLVCAINNSFSRYSICDNDLFRFNKKMFARRRILLKKNRHKRAGHGAKNKLKPISILTEKSERFRKKLIERWACEIADFFVRNKVGTVQMENLESMKRKEDSYFNIRLRGFWPYAEMQNKIEFKLEQYGIKIRKVAPNNTSKTCSKCGHLNNYFNFEYRKKNKFPHFKCEKCNFKEDADYNAALNISNPKLKSTKGEP

SEQ ID NO: 3048 - protein, 726 aa, synthetic construct
SEVEFSHEYWMRHALTLAKRARDEREVPVGAVLVLNNRVIGVGWNRAIGLHDPTAHAEIMALRQGGLVMQNYRLTDATLYVTFEPCVMCAGAMVHSRIGRVVFGVRNSKRGAAGSLMNVLNYPGMSHCVEITEGILVDECAALLCDFYRMPRQVLNAQKKAQSSISSGGSSGGSGGGETPGASESVTPKSSGGSSAGSTKNTITKTLKLRIVRPYNSAEVEKIVADEKNSREKIALEKNKDKVKEACSEHLKVAAYCTTQVERSACLFCKARKLDDRFYQKLRGQFPDAVFWQEISEIFRQLQKQAAVIYNQSLIELYYEIFIKGKGFANASSVEHYLSDVCYTRAAELFRNAAIASGLRGKVKSNFRLKELKNMKSGLPTTKSDNFPIPLVKQKGGQYTGFEISSHNDDLIIKIPFGRWQVKKEINKYRPWEKFDFEQVRRSPKPISLLLSTQRRKRNKGWSKDEGTEAEIRKVMNGDYQTSYIEVKRGSKIGEKSAWMLNLSIDVPKIDKGVDPSIIGGIDVGVKSPLVCAINNALSRYSISDNDLFRFNKKMFARRRILLKKNRHRRAGHGAKNKLKPIAVLAEKSEGFRKKLIERWACEVADFFVKNKVGTVQMENLESMKRKEDSYFNIRLRGFWPYAEMQNKIEFKLKQYGIKVRKVAPNNTSKTCSKCGHLNNYFNFEYRKKNKFPHFKCEKCNFREDADYNAALNISNPKLKSTKEEP

SEQ ID NO: 3049 - protein, 726 aa, synthetic construct
SEVEFSHEYWMRHALTLARRARDEREVPVGAVLVLNNRVIGEGWNRAIGLHDPTAHAEIMALRQGGLVMQNYRLTDATLYVTFEPCVMCAGAMIHSRIGRVVFGVRNSKRGAAGSLMNVLDYRGMDHCVEITEGILVDECAALLCDFYRMPRQVLNAQKKAQSSISPGGSSGGSSGSETPGASGSVTPKSSGGSSAGSTKDTITKTLKLRIVRPYNSAEVEKIVADEKNNREKIALEKNKDKVKEACSKHLKVASYCTTQVERNACLFCKARKLDDKFYQKLRGQFPDAVFWQELGEIFRQLQKQAAEVYNQSLVELYYEILIKGKGIANASSVEHYMSDVCYTRAAELFKNAAIASGLRNKIKSNFRLKELRNMKSGLPTTKSDNFPIPLVRQKGGQYAGFEISNHDGDFIIKIPFGRWQVKKEINKHRPWEKFDFEQVRKSPKPISLLLSTQRRKRNKGWSKDEGTEAEIRKVMNGDYQTSYIEVKRGSKIGEKSAWMLNLSIDVPKIDKGVDPSIIGGIDVGVKSPLVCAINNALSRYSISDNDLFHFNKKMFARRRILLRKNRHKRAGHGAKNKLKPITMMTEKSKRFRKKLIERWACEIADFFIKNKVGTVQMENLESMKRREDSYFNIRLRGFWPYAKMQNKIEFKLKQYGIEIRKVAPNNTSKTCSKCGHLNNYFNFEYRRKNKFPHFKCEKCNFKEDADYNAALNISNPKLKSTKEKP

SEQ ID NO: 3050 - protein, 726 aa, synthetic construct
SEVEFSHEYWMRHALTLAKRARDEREVPVGAILVLNNRVIGEGWNRAIGLHDPTAHAEIMALRQGGLVMQNYRLTDATLYATFEPCVMCAGAMIHSRIGRVVFGVRNSKHGAAGSLMNVLNYPGMNHRVEITEGILADECAGLLCDFYRMPRQVFSARKKAQSSINPGGSSGGSSGGKAPGTSESATLESSGGSSGDSAKNSITKTLKLRIVRPYNSAEVEKIVADEKNNREKIALEKNKGKVEEACSKHLKVATYCTTQVERNACPFCKARKLDDKFYQKLRGQFPDAVFWQEIGEIFRQLQKQAAEIYNQSLIELYYEIFIEGKGSANARSVEHYLSDVCYTRAAELFKNAAIASGLRGKVKGNFRLKELKSMKSGLPTTKSDNFPIPLVKQKGGQYTGFEISSHNDDFIIKIPFGRWQVKKEIDKYRPWEKFDFEQVRKSPRPISLLLSTQRRKRNKGWSKDEGTEAEIRKVMNGDYQTSYIEVKRGSKIGEKSAWMLNLSIDVPKIDKGVDPSIIGGIDVGVRSPLVCAIDNAFSRYSISDNDLFHFNKKMFARRRILLKKNGHRRAGHGAKNKLKPISILTEKSKRFRKKLIERWACEIADFFIKNKVGTVQMENLESMKRKEDSYFNIRLRGLWPYAEMQSKIEFKLKQYGIEIRKVAPNNTSKTCSKCGHLNNYFDFEYRKKNKFPHFKCEKCNFKENADYNAALNISNPKLRSTKEEP

SEQ ID NO: 3051 - protein, 726 aa, synthetic construct
SEVEFSHEYWMRHALTLAKRARDGREVPVGAVLVLNNRVIGEGWNRAIGLHDPSAHAEIMALRQGGLVMQNYRLIDATLYVTFEPCVMCAGAMVHSRIGRVVFGVRNSKRGAAGSLMNVLDCPGMGHRVEITEGILADECAALLCDFYCMPRQVFNAQKRAQSSINSGGSSGGSSGSETPGTSESATPGSSGGGSSGSAKNTITKTLQLRIVRPYNSAEVEKIVADEKNNREKIALEKNKDKVKEACSKHLKVASYCTTQVERNACPFCKARKLDDKFYQKLRGQFPDAVFWQELGEILRQLQKQAAEIYNQSLIELYYEIFIKGKGFANASSVEHYLSDVCYTRAAELFKNAAIASGLRGKVKSNFRLKELKNMKSGLPTTKSDNFPIPLVKQKGGQYTGFEISNHNSDFIIKIPFGRWQAKKEIDKYRPWEKFDFEQVRKSPKPISLLLSTQRRKKNRGWSKDEGTEAEIKKVMNGDYQTSYIEVKRGSKIGEKSAWMLNLSIDVPKIDKGVDPSIIGGIDVGVKSPLVCAINNSSSRYSICDNDLFRFNKKMFARRRILLKKNRHKRAGHGAKNKLKPITILTKKSERFRKKLIERWVCEVADFFIKNKVGTVQMENLESMKRKEDSYFNIRLRGFWPYAEMQNRIELKLKQYGIEIRRVAPNNTSRTCSKCGHLNNYFNFEYRKRNKFPHFKCEKCNFKENADYNAALNISNPKLKGTKEEP

SEQ ID NO: 3052 - protein, 726 aa, synthetic construct
SEVEFSHEYWMRHALTLAKRARDEREVPVGAVLVLNNRVIGEGWNRAIGLHDPTAHAEVMALRQGGLVMQNYRLTDATLYVTFEPCVMCAGAMIHSRIGRVVFGVRNSKRGAAGSLMNVLNYPGMNHCVEITEGILVDECAALLCDFYRMPRQVLNAQKKAQSSISPGGSSGGSSGSETPGASESVTPKSSGGSSGGSAKNTITKTLKLRIVRPYNSAEVEKIVADEKNNREKIALAKNKDKVKEACSEHLKVAAYCTTQVERNACLFCKARKLDDRFYQKLRGQFPDAVFWQEIGEIFRQLQKQAAEIYNQSLIELYYEIFIKGKGFANASSVEHYLSDVCYTRAAELFKNAAIASGLRGKVKSNFRLKELKNMKSGLPTTKSDNFPIPLVRQKGGQYTGFEVSSHNDDFIIKIPFGRWQVKKEIDKYRPWEKFDFEQVRKSPKPISLLLSTQRRKRNKGWSKDESTEAEIRKVMNGDYQTSYIEVKRGSKIGEKSAWMLNLSIDVPKIDKGVDPSIIGGVDVGVKSPLVCAINNAFSRYSISDNDLFRFNKRMFARRRILLKKNRHKRAGHGAKNKLKPISILTEKSERFRKKLIERWACEIANFFIKNKVGTVQMENLGSMKRKEDSYFNIRLRGFWPYAEMQNKIEFKLKQYGIEIRKVAPNNTSRTCSKCGHLNNYFNFEYRKKNKFPHFKCEKCNFKENADYNAALNISNPKLKSTKEEP

SEQ ID NO: 3053 - protein, 726 aa, synthetic construct
SEDEFSHEYWMRHALTLAKRARDGREVPVGAVLVLNNRVIGEGWNRAIGLHDPTAHAEIMALRQGGLVMQNYRLIDATLYVTFEPCVMCAGAMIHSRIGRVVFGARNSKRGAAGSLMNVLSYPGMNHRVEITEGILADECAALLCDFYRMPRRVFNAQKKAQSSINSGGSSGGGSGSDTPSTSESTTPESSGGSSGGPAKNTITKTLKLRIVRPYNSAEVEKIVADEKNNREKTALEKNKDKVKEACSKHLKVAAYCTTQVERNACLFCKARKLDDKFYQKLRGQFPDAVLWQEIGEIFRQLQKQAAEIYNQSLIELYYEIFIKGKGFANASSVEHYLSDVCYTRAAELFKNAAIASGLRGKVKSNFRLKELKNMKSGLPTTKSDNFPIPLVRQKGGQYTGFEISSHNDDFIIKIPFGRWQMRKEIDKYRPWEKFDFEQVRKSPKPISLLLSTQRRKRNKGWSKDEGTEAEIRKVMNGDYQTSYIEVKRGSKIGEKSAWMLNLSIDVPKIDKGVDPSIIGGIDVGVKSPLVCAINNAFSRYSIGDNDLFHYNKKMFARRRILLKKNGHKRAGHGAKNKLKPITILTKKSERFRKKLIERWACEIANFFIKNKVGTVQMENLESMKRKEDSYFNIRLRGFWPYAEMQNKIEFKLKQYGIKIRKVAPNNTSKTCSKCGHLNNYFSFEYRKKNKFPHFKCEKCNFKENADYNAALNISNPKLKSTKEEP

SEQ ID NO: 3054 - protein, 726 aa, synthetic construct
SEVEFSHEYWMRHALTLAKRARDEREVPVGAVLVLNNRVIGEGWNRTTGLHDPTAHAEIMALRQGGLATQNHRLVDATLYVTFEPCVMCAGAMIHSRIGRVVFGVRNSKRGAAGSLTNVLNYPGMNHRVEITEGILVDECAALLCDFYRMPRQVFNARKKAQSTINSGGSSGGSSGSETPGTSESPTPESPGGSSGGSAKNSITKTLKLRIVRPYNSAEVEKIVADEKNNREKIALEKNKGKVKEACSKHLKVATYCTTQVERNACLFCKARKLDDKFYQKLRGQFPDAVFWQETGEIFRQLQRQAAEIYNRSLIELYYEIFIKGKGFANASSVEHYLSDVCYTRAAELFKNAAIASGLRGKVKSNFRLKELKNMKSGLPTTKSDNFPIPLVKQKGGQYTGFEISSHNDDFIIKIPFGRWQVKKEIDRYRSWEKFDFEQVRKSPKAISLLLSTQRRKRNKGWSKDEGTEAEIRKVMNGDYQTSYIEVKRGSKIGEKSAWMLSLSIDVPKIDKGVDPSTIGGIDVGVKSPLVCAINNAFCRYSISDNDLFHFNKKMFARRRILLKKSRHKRAGHGAKNKLKPISILTEKSKRFRKKLIERWASEIADFFIKNKVGTVQMENLESMKRKEDSYFNIRLRGFWPYAEMQNKIEFKLKQYGIEIRKVAPNNTSKTCSKCGHLNNYFNFEYRKKNKFPHFKCEKCNFKENADYNAALNISNPKLKSTKEEP

SEQ ID NO: 3055 - protein, 726 aa, synthetic construct
SEVEFSHEYWMRHALTLAKRARDEREVPVGAVLVLNNRVIGAGWNRTTGLHDPTAHAEIMALRQGGLVIQNYRLSDATLYVTFEPCVMCAGAMIHSRIGRVVFGARNSKRGAAGSLMNVLNYPGMDHRVEITGGILADECAALLCDFYRMPRRVFNAQKKAHSSINSGGSSGGSSGSVTPGTSESATPESSGGSSGGSAKNTITKTLKLRIVRPYNSAEVEKIVADEKNNREKIALEKNKDKVKEACSEHLKVAAYCTTQVERSACLFCKARKLDDKFYQKLRGQFPDAVFWQEIGEIFRQLQKQAAEIYNQSLIELYYEIFIKGKGITNASRVEHYLSDVCYTRAAELFKNAAIASGLRGKVKSNFRLKELRNMKSGLPTTKSDNFPIPLVKQKGGQYTGFEISSHNDDFIIKIPFGRWQVKKEIDKHRPWEKFDFEQVRKSPKPISLLLSTQRRKRNRGWGKDEGTEAEIRKVMNGDYQTSYIEVKRGSKIGEKSAWMLNLSIDVPKIDKGVDPSIIGGIDVGVKSPLVCAINNAFSRYGISDNDLFRFNKKMFARRRILLKKNRHKRAGHGAKNKLKPISILTEKSKRFRKKLIERWACEIADFFIKNKVGTVQMENLESMKRKEDSYFNIRLRGFWPYAEMQNKIEFKLKQYGIEIRKVAPNNTSKTCSKCGHLNNYFNFEYRKMNKFPHFKCEKCNFKENADYNAALNISNPKLKSTKEEP

SEQ ID NO: 3056 - protein, 726 aa, synthetic construct
SEVEFSHEYWMRRALTLAKRARDEREVPVGAVLVLNNRVIGVGWNRAAGLHDPTAHAEIMALRQGGLVMQNYRLVGATLYVTFEPCIMCAGAMIHSRIGRVVFGVRNSKRGAAGSLMNVLNYPGMNHRVEITEGILADECAALLCDYYRMPRQVFNARKKAQSSINSGGSSDGGSGSETPGTSESATPESSGGSSGGSAKNTITKTLKLRIVRPYNSAEVERIVADEKNSREKIALERNKDKVKEACSKHLRVAAYCTTQVERNACLFCKARKLDDKFYQRLRGQFPDAVFWQELGEIFRQLQKQAAEIYNQSLIELYYEIFIKGKGFANASSVEHYLSDVCYTRAAELFKNAAIASGLRGKVKSNFRLKELKNMRSGLPTAKSDNFPIPLVKQKGGRYTGFEISSHNDDFIIKIPFGRWRVKKEINKHRPWEKFDFEQVRKSPKPISLLLSTQRRKRNKGWSKDEGTEAEIRKVMNGDYQTSYIEVKRGSKIGEKSAWMLNLSIDVPKIDKGVDPGIIGGIDVGVKSPLVCAINSASSRYSISDNDLFHFNKKMFARRRILLKKNGHKRAGHGAKNKLKPITIMTEKSKRFRKKLIERWACEIADFFIKNKVGTVQMENLESMRRKEDSYFNIRLRGFWPYAEMQNKIEFKLKQYGIEIRKVAPNNTSKTCSKCGHLNNYFSFEYRKKNKFPHFKCEKCNFKEDADYNAALNISNPKLKSTKEEP

SEQ ID NO: 3057 - protein, 726 aa, synthetic construct
SEVEFSHEYWMHHALSLAKRARDEREVPVGAVLVLNNRIIGEGWNRAIGLHDPTAHAEIMALRQGGLVMQNYRLDDATLYVTFEPCVLCAGAMVHSRIGRVVFGVRNSKRGAAGSLMNVLNYPGMNHRVEITEGILADECAALLCDFYRMPRQVFNARKKAQSSISPGGSSGGSSGSETPGTSESATPESSGGSSGGSAKNTITKTLKLRIVRPYNSAEVEEIVADEKNNREKIALEKNKDKVKEACSEHLKVVAYCTTQVERSACLFCKARKLDDKFYQKLRGQFPDAVFWQEIGEIFRQLQKQAAEIYNQSLIELYYEIFIKGKGFANASSVEHYLSDVCYTRAAELFKNAAIASGLRGKVKSNFRLKELKNMKSGLPTTKSDNFPIPLVKQKGGQYTGFEISNHNDDFIIKIPFGRWQVKEEIDKYRPWEKFDFEQVRKNPKPISLLLSTQRRKGNKGWSKDEGTEAEIRKVMNGDYQTSYIEVKRGSKIGEKSAWMLNLSIDVPKIDKGVDPSIIGGIDVGVKSPLVCAINSAFSRYSISDNDLFRFNKKVFARRRILLKKNRHKRAGHGTKNKLKPIAILTEKSGRFRKKLIERWACEIANFFIKNKVGTVQMENLESMKRKEDSYFNIRLRGFWPYAEMQNKIEFKLKQYGIKIRKVAPNNTSKTCSKCGHLNNHFSFEYRKKNKFPHFKCEKCNFKEDADYNAALNISNPKLKSTKEEP

SEQ ID NO: 3058 - protein, 726 aa, synthetic construct
SEVEFSHEYWMRHALTLAKRARDEREVPVGAVLVLNNRVIGGGWNRAIGLHDPTAHAEIMALRQGGLVMQNCRLVDATLYVTFEPCVMCAGAMIHSRIGRVVFGVRNSKRGAAGSLMNVLNYPGMNHRVEITEGILAGECAALLCDFYRMPRQVFNAQKKAQSTINSGGSSGGSSSSETPGISGSATPEGSGGSSGGSAKNTITKTLKLRIVRPYNSAEVEKIVADEKNNREKIALEKNKDKVKEACSKHLKVASYCTTQVERNACLFCKARKLDDKFYQKLRGQFPDAVFWQELGEIFRQLQKQATEIYNQSLIELYYEIFIKGKGITNASRVEHYLSDVCYTRAAELFKNAAIASGLRSKVRSNFRLKELKNMKSGLPTTKSDNFPIPLVKQKGGQYTGFEISSHNSDLIIKIPFGRWQVKEEIDKYRPWEKFDFEQVRKSPKPISLLLSTQRRKRNKGWSKDEGTEAEIRKVMNGDYQTSYIEVKRGSKTGEKSAWMLNLSIDVPKIDKGVDPSIIGGIDVGVKSPLVCAIDNAFSRYSISDNDLFRFNKKMFARRRILLKKNRHKRAGHGAKNKLKPISILTGKSERFRKKLIERWACEIADFFIKNKVGTVQMENLESMKRKEDSYFNIRLRGFWPYAEMQNKIEFKLKQYGIEIRKVAPNNTSKICSKCGHLNNYFNFEYRKKNKFPHFKCEKCNFKENADYNAALNISNPKLKSTKEEP

SEQ ID NO: 3059 - protein, 726 aa, synthetic construct
SEVEFSHEYWMRHALTLAKRARDEREVPVGAVLVLNNRVIGVGWNRAIGLHDPTAHAEIMALRQGGLVMQNYRLIDATLYVTFEPCVMCAGAMIHSRIGRVVFGVRNSKRGAAGSLTNVLNYPGMNHRVEITEGILVDECAALLCDFYRMPRQVFNAQKKAQSTINSGSSSGGSSGSETPGTSESPTPESSGGSPGGSAKNTITKTLKLRIVRPYNSAEVEKIVADEKNNREKIALEKNKDKVKEACSKHLKVAAYCTTQVERNACLFCKARKLDDKFYQKLRGQFPDAVFWQEIGEIFRQLQKQAAEIYNQSLIELYYEIFIKGKGFANASSVEHYLSDVCYTRAAELFKNAAIASGLRNKIKSNFRLKELKNMKSGLPTTKSDNFPIPLVKQKGGQYTGFEISDHNSDFIIKIPFGRWQVKKEINRYRPWEKFDFEQVRKSPKPISLLLSTQRRKRNKGWSKDEGTEAEIRKVMNGGYQTSYIEVKRGSKVGEKSAWMVNLSIDVPKIDKGVDPSIIGGIDVGVKSPLVCAVNNALSRYSIDDNDLFHFNKKMFARRRILLKKNRHRRAGHGARNKLKPITVLTEKSKRFRKKLIERWACEIANFFVKNKVGTVQMENLESMKRKEDSYFNIRLRGLWPYAEMQNKIEFKLKQYGIEVRKVAPNNTSKTCSKCGHLNNYFSFEYRKKNKFPHFKCEKCNFKENADYNAALNISNPKLKSTKEEP

SEQ ID NO: 3060 - protein, 726 aa, synthetic construct
SEVEFSHEYWMRHALTLAKRARDEREVPVGAVLVLNNRVIGVGWNRAIGLHDPTAHAEIMALRQGGLVMQNYRLIEATLYVTFEPCIMCAGAMIHSRIGRVVFGVRNSKRGAAGSLMDVLNYPGMNHRVEITEGILADECAALLCDYYRMPRQVFITQRKAQSSINSGGSSDGGSGSETPGTSESATPESSGGSSGGSAKNTITKTLKLRIVRPYNSAEVEKIVADEKNNREKIALEKNKDKVKEACSEHLKVAAYCTTQVERSACLFCKARKLDDKFYQKLRGQFSDAVFWQELGEIFRQLQKQAAEIYNQSLIELYYEIFIKGKGIANASSVEHYLSDVCYTRAAELFKNAAIASGLRNKIKSNFRLKELRNMKSGLPTTKSDNFPIPLVRQKGGQYTGFEISNHDGDFIIKIPFGRWQVKKEINKHRPWEKFDFEQVRKSPKPISLLLSTQRRKGNKGWSKDEGTEAEIRKVMNGDYQTSYIEVKRGSKIGEKSAWMLNLSIDVPKIDKGVDPSIIGGIDVGVKSPLVCAINNALSRYSISDNDLFHFNKKMFARRRILLKKNRHKRDGHGARNKLKPITVLAEKSERFRKKLIERWACEIANFFIKNKVGTVQMENLESMKRKEDSYFNNRLRGFWPYAEMQNKIEFKLKQYGIEVRKVAPNNTSKTCSKCGHLNNYFNFEYRKKNKYPYFKCEKCNFKENADYNAALNISNPKLRSTKEEP

SEQ ID NO: 3061 - protein, 726 aa, synthetic construct
SEVEFSHEYWMRHALTLAKRARDEREVPVGAILVLNNRVIGEGWNRAIGLHDPTAHAEIMALRQGGLVMQNHRLIDATLYVTFEPCVMCAGAMIHSRIGRVVFGVRNNKHGAAGSLVNVLNYPGMNHRVEVTEGILVDECAALLCDFYRMPRQVLNAQKMAQSSISSGGSSGDSSGSETPGTSESATPKSSGGSSGGSAKNTITKALKLRIVRPYNSAEVEKIVADEKNNRERIALEKNKDKVKEACSKHLKVAAYCTTQVERNACLFCKARKLDDKFYQKLRGQFPDAVFWQEIGEIFRQLQKQAAEIYNQSLIELYYEILIKGKGFANASSVEHYLSDVCYTRAAELFKNAAIASGLRGKVKSNFRLKELKNMRSGLPTTKSDNFPIPLVKQKGGQYAGFEISSHNDDFIIKIPFGRWQVKKEIDKYRPWEKFDFGQVRKSPKPISLLLSTRRRKRNKGWSKDEGTEAEIMKVMRGDYQTSYIEVKRGSKIGEKSAWMLSLSIDVPKIDKGVDPSIIGGIDVGVKSPLVCAINNAFNRYSISDNDLFRFNKKMFARRRILLKKNRHQRAGHGAKNKLKPITILTEKSGRFRKKLIERWACEIADFFVKNKVGTVQMENLESMKGKEDSYFNIRLRGFWPYAEMQNKIEFKLKQYGIVVRKVAPNNTSKTCSKCGHLNNYFNFEYRKMNKFPHFKCEKCNFKENADYNAALNISNPKLKSTKEEP

SEQ ID NO: 3062 - protein, 726 aa, synthetic construct
SEVEFSHEYWMRRALTLAKRARDEREVPVGAVLVLNNRVIGVGWNRAVGLHDPTAHAEIMALRQGGLVMQNYRLIEATLYVTFEPCIMCTGAMIHSRIGRVVFGVRNSKRGAAGSLMNVLNYPGMNHRVEITEGILADECAALLCDYYRMPRQVFNARKKAQSSINSGGSSDGGSGSETPGTSGSATPESSGGSSGGSAKNTITKTLKLRIVRPYNSAEVEKIVADEKNNREKIALEKNKDKVKEACSKHLKVAPYCTTQVERNACPFCKARKLDDKFYQKLRGQFPDAVFWQEIGEIFRQLQKQAAEIYNQSLIELYYEIFIEGKGFANASSVEHYLSDVCYTRAAELFKNAAIASGLRGKVKGNFRLKELKSMKSGLPTTKSDNFPIPLVKQKGGQYTGFEISSHNDDFIIKIPFGRWQVKKEIDRYRPWEKFDFEQVRKSPKPISLLLSTQRRKRNKGWSKDEGTEAEIRKVMNGDYQTSYIEVKRGSKIGEKSTWMLSLSIDVPKIDKGVDPSIIGGIDVGVRSPLVCAIDNAFSRYSISDNDLFHFNKKMFARRRILLKKTRHKRAGHGVKNKLKPITILTEKSGRFRKKLIERWACEIADFFVKNKVGTVQMENLESMKRKEDSYFNIRLRGFWPYAEMQNKIEFKLKQYGIKVRKVAPNNTSKTCSKCGHLNNYFSFEYRKKNKFPRFKCEKCNFKEDADYNAALNICNPKLKSTKEEP

SEQ ID NO: 3063 - protein, 726 aa, synthetic construct
SEDEFSHEYWMRHALTLAKRARDGREVPVGAVLVLNNRVIGEGWNRAIGLHDPTAHAEIMALRQGGLVMQNYRLIDATLYVTFEPCVMCAGAMVHSRIGRVVFGVRNSKRGAAGSLMNVLDYPGMGHRVEITEGILADECAALLCDFYCMPRQVFNAQEKAQSSVSSGGSSGGCSGSEMPGASESVTPKSSGGSSAGSTKNTITKTLKLRIVRPYNSAEVEKIVADEKNSREKIALERNKDKVKEACSEHLKVATYCTTQVERNACLFCKARKLDDRFYQKLRGQFPDAVFWQETGEIFRQLQKQAAEIYNQSLIELYYEIIIKGKGITNASRVEHYLSDVCYTRAAELFKNAAIASGLRSKVRSNFRLKELKNMKSGLPTTKSDNFPIPLVKQKGGQYTGFEISSHNSDFIIKIPFGRWQEKEEIDKYRPWEKFDFEQVRRSPKPISLLLSTQRRKKNKGWSKDEGTEAEIRKVMNGDYQTSYIEVKRGSKTGEKSAWMLNLSIDVPKIDKGVDPSIIGGIDVGVKSPLVCAINNSSSRYSICDNDLFHFNKKMFARRRILLKKNRHKRAGHGAKNKLKPITILTEKSKRFRKKLIERWVCEVADFFIKNKVGTVQMENLESMKRKEDSYFNIRLRGFWPYAEMQSRIELKLKQYGIEIRRVAPNNTSRTCSKCGHLNNYFNFEYRKRSKFPHFKCEKCNFREDADYNAALNISNPKLKSTKEEP

SEQ ID NO: 3064 - protein, 726 aa, synthetic construct
SEVEFSHEYWMRHALTLAKRARDEREVPVGAVLVLNNRVIGEGWNRTTGLHDPTAHAEIMALRQGGLVMRNYRLTDATLYVTFEPCIMCAGAMIHSRIGRVVFGVRNSKRGAAGSLMNVLNYPGMNHCVEITGGILADECAALLCDFYRMPHQVFNARKKAQSSINPGGPSGGSSGSETPDTSESATPESSGGNSGGSAKNTITKTLKLRIVRPYNSAEVEKIVADEKNNREKIALEKNKDKVKEACSEHLKVAAYCTTQVERNACLFCKARKLDDKFYQKLRGQFPDAVFWQEIGEIFRQLQKQAAEAYNQGLVELYYEIFIKGKGIANASNVEHYLSDVCYTRAAELFKNAAIASGLRNKIKSNFRLKELRNMKSGLPTTKSDNFPIPLVRQKGGQYTGFEISNHNSDFIIKIPFGRWQVKKEINKYRPWEKFDFEQVRKSPKPISLLLSTQRRKRNKGWNKDEGTEAEIRKVMNGDYQISYIEVKRGSKIGEKSAWMLNLSIDVPKIDKGVDPSIIGGIDVGVKSPLVCAINNAFCRYSISDNDLFHFNKKMFARRRILLKKSRHRRAGHGAKNKLKPISILTEKSKRFRKKLIERWACEIADFFIKNKVGTVQMENLESMKRKEDSYFNIRLRGFWPYAEMQNKIEFKLKQYGIEIRKVAPNNTSKTCSKCGHLNNYFNFEYRKKNKFPHFKCEKCNFKENADYNAALNISNPKLKSTKEEP

SEQ ID NO: 3065 - protein, 726 aa, synthetic construct
SEVEFSHEYWMRRALTLAKRARDEREVPVGAVLVLNNRVIGVGWNRAVGLHDPTAHAEIMALRQGGLVMQNYRLVEATLYVTFEPCIMCAGAMIHSRIGRVVFGVRNSKRGAAGSLMNVLNYPGMNHRVEITEGILADECAALLCDYYRMPHQVFNARKKAQSSINSGGSSDGGSGSETPGTSESATPESSGGSSGGSAKNTITKTLKLRIVRPYNSAEVEKIVADEKNNREKIALEKNKDKVKEACSKHLKVASYCTTQVERNACPFCKARKLDDKFYQKLRGQFPDAVFWQELGEILRQLQKQAAEIYNQSLIELYYEIFIKGKGFANASSVEHYLSDVCYTRAAELFKNAAIASGLRGKVKSNFRLKELKNMKSGLPTTKSDNFPIPLVKQKGGQYTGFEISSHNDDFIIKIPFGRWQVKKEIDKYRPWEKFDFEQVRKSPKPISLLLSTQRRKRNKGWSKDEGTEAEIRKVMNGDYQTSYIEVERGSKIGEKSTWMLNLSIDVPKIDKGVDPSIVGGIDVGVKSPLVCAINNALSRYSISDNDLFRFNKKMFARRRILLKKNRHKRAGHGAKNKLKPISILTGKSERFRKKLIERWACEIADFFIKNKVGTVQMENLESMKRKEDSYFNIRLRGFWPYAEMQNKIEFKLKQYGIEIRKVAPNNTSKTCSKCGHLNNYFNFEYRKKNKFPHFKCEKCNFKENADYNAALNISNPRLKSTKEEP

SEQ ID NO: 3066 - protein, 726 aa, synthetic construct
SEVEFSHEYWMRHALTLAKRARDEREVPVGAVLVLNNRVIGVGWNRAIGLHDPTAHAEIMALRQGGLVLQNYRQTDATLYVTFEPCVMCAGAMIHSRIGRVVFGVRNSKRGAAGSLMNVLDYPGMGHRVEITEGILADECAALLCDFYCMPRQVFNAQKRAQSSISPGGSSGGSSGSETPGASESVIPKSSGGSSGGSAKNTITKTLKLRIVRPYNSAEVEKVVADEKNNREKIAIEKNKDKVKEACSKHLKVASYCTTQVERNACPFCKARKLDDKFYQKLRGQFPDAVFWQEIGEIFRQLQKQAAGIYNQSLIELYYEIFIKGRGFANASSVEHYLSDVCYTRAAELFKNAAIASGLRGKVKSNFKLKELKSMKSGLPTTKSDNFPIPLVKQKGGQYTGFEISSHNDDFIIKIPFGRWQMKKEIDRYRPWEKFDFEQVRKSPKPISLLLSTQRRKRNKGWSKDEGTEAEIRKVMNGDYQTSYIEVKRGSKIGEKSAWMLSLSIDVPKIDKGVDPSIIGGIDVGVKSPLVCAINNAFCRYSISDNDLFHFNKKVFARRRILLKKNRHRRAGHGAKNKLKPITILTEKSKRFRKKLIERWACEIANFFIKNKVGTVQMENLESMKRKEDSYFNIRLRGFWPYAEMQNKIEFKLKQYGIKIRKVAPNNTSRTCSKCGHLNNYFSYEYRKKNKFPHFKCEKCNFKEDADYNAALNISNPKLKGTKEEL

SEQ ID NO: 3067 - protein, 726 aa, synthetic construct
SEVEFSHEYWMRHALILAKRARDEREVPVGAVLVLNNRVIGEGWNRAIGLHDPTAHAEIMALRQGGLVMQNYRLIDATLYVTFEPCVMCAGAMVHSRIGRVVFGVRNSKRGAAGSLMNVLDYPGMGHRVEITEGILADECAALLCDFYCMPRQVFNAQKRAQSSINSGGSSDGSSGSETPGTSESPTPESSGGSPGGSAKNTITKTLQLRIVRPYNSAEVEKIVADEKNNREKIALEKNKDKVREACNKHLKVASYCTTQVERNACPFCKARKLDDKFYQKLRGQFPDAVFWQELGEILRQLQKQAAEIYNQSLIELYYEIFIKGKGITNASRVEHYLSDVCYTRAAELFKNAAIASGLRSKVRSNFRLKELKNMKSGLPTTKSDNFPIPLVKQKGGQYTGFEISSHNSDFIIKIPFGRWQVKEEIDKFRPWEKFDFEQVRKSPKPISLLLSTQRRKKNKGWSKDEGTEAEIKKVMNGDYQTSYIEVKRGSKTGEKSAWMLNLSIDVPKIDKGVDPCIIGGIDVGVKSPLVCAINNALSRYSISDNDLFRFNKKMFARRRILLKKNGHKRAGHGAKNKLKPITIMTEKSKRFRKKLIERWACEIADFFIKNKVGTVQMENLESMKRKEDSYFNIRLRGFWPYAEMQNKIEFKLKQYGIVVRKVAPNNTSKTCSKCGHLNNYFSFEYRKKNKFPHFKCEKCNFKENADYNAALNISNPKLKSTKEEP

SEQ ID NO: 3068 - protein, 726 aa, synthetic construct
SEVEFSHEYWMRHALTLAKRARDEREVPVGAVLVLNNRVIGVGWNRAIGLHDPTAHAEIMALRQGGLVMQNYRLTDATLYVTFEPCVMCAGAMVHSRIGRVVFGVRNSKRGAAGSLMNVLNFPGMSHCVEITEGILVDECAALLCDFYRMPRQVLNAQKKAQSSISSGGSSGGSGGGETPGASESVTPKNSGGSSASSTKNTITKALKLKIVRPYNSAEVEKIVADEKNNRERIALEKNKDKVKEACSKHLKVAAYCTTQVERNACLFCKARKLDDKFYQKLRGQFPDAVFWQEIGEIFRQLQKQAAEIYNQSLIELYYEIFIKGKGFANASSVEHYLSDVCYTRAAELFKNAAIASGLRGKVKSNFRLKELKNMKSGLPTTKSDNFPIPLVRQKGGQYTGFEVSSHNDDFIIKIPFGRWQVKKEIDKYRPWEKFDFEQVRKSPRPISLLLSTQRRKRNKGWSKDEGTEAEIRKVMNGDYQTSYIEVKRGSKIGEKNVWMLNLSIDVPKIDKGVDPSIIGGIDVGVKSPLVCAINNAFSRYSISDNDLFHFNKKMFARRRILLKKNRHKRAGHGAKNKLRPITILAERSERFRKKLIEKWACEIADFFIKNKVGTVQMENLESMKRKEDSYFNIRLRGFWPYAEMQNKIEFKLKQYGIKIRKVAPNNTSRTCSECGHLNNYFSFEYRKKNKFPHFKCEKCNFKEDADYNAALNISNPKLKGTKEEL

SEQ ID NO: 3069 - protein, 726 aa, synthetic construct
SEVEFSHEYWMRHALTLAKRARDEREVPVGAVLVLNNRVIGEGWNRAIGLHDPTAHAEIMALRQGGLVMQNYRLVDATLYVTFEPCVLCAGAMVHSRIGRVVFGVRNSKRGAAGSLMNVLNYPGMNHRVEITEGILADECAALLCDFYRMSRRVFNAQKKAQSNINPGGSSGGSGGSETPGTSESATPKSSGGSSGGSAKNTITKTLKLRIVRPYNSAEVEKIVADEKNNREKIALEKNKDKVKEACSKHLKVASYCTTQVERNACLFCKARKLDDKFYQKLRGQFPDAVFWQELGEIFRQLQKQAAEIYNQSLIELYYEIFIKGKGFANASSVEHYLSDVCYTRAAELFKNAAIASGLRGKVKSNFRLKELKNMKSGLPTTKSDNFPIPLVKQKGGQYTGFEISSHNDDFIIKIPFGRWQVKKEINKFRPWEKFDFEQVRKSPKPISLLLSTQRRKRNKGWNRDEGTEAEIRKVMNGDYQTSYIEVKRGSKIGEKSAWMLNLSIDVPKIDKGVDPSIIGGIDVGVKSPLVCAINSAFSRYSISDNDLFHFNKKMFARRRILLKKTRHKRAGHGAKNKLKPISILTEKSERFRKKLIERWACEIADFFIKNKVGTVQMENLESMKRKEDSYFNIRLRGFWPYAEMQNKIEFKLKQYGIKVRKVAPNNTSKTCSKCGHLNNYFSFEYRKKNKFPHFKCEKCNFKENADYSAALNISNPKLKSTKEEP

SEQ ID NO: 3070 - protein, 726 aa, synthetic construct
SEDEFSHEYWMRHALTLAKRARDGREVPVGAVLVLNNRVIGEGWNRAIGLHDPTAHAEIMALRQGGLVMQNYRLIDATLYVTFEPCVMCAGAMVHSRIGRVVFGVRNSKRGAAGSLMNVLDYPGMGHRVEITEGILADECAALLCDFYCMPRQVFNAQKRAQSSTNPGGSSGGSSGSETPGTSESATPESSSGSSGGSTKNTITKALKLRIVRPYNSAEVEKIVADEKNNREKIALEKNKDKVKEACSKHLKVAAYCTTQVERNACLFCKARRLDDKFYQKLRGQFPDAVFWQEIGEIFRQLQKQAAEIYNQSLIELYYEIFIKGKGFANASSVEHYLSDVCYARAAELFKNAAIASGLRGKVKGNFRLKELKSMKSGLPTTKSDNFPIPLVKQKGGQYTGFEISSHNDDFIIKIPFGRWQVKKEIDKYRPWEKFDFEQVRKSPKPISLLLSTQRRKRNKGWSKDEGTEAEIRKVMNGDYQTSYIEVKRGSKIGEKNAWMLNLSIDVPKIDKGVDPSIIGGIDVGVKSPLVCAINNAFSRYSISDNDLFRFNKKMFARRRILLKKNRHKRAGHGAKNKLKPISILTGKSERFRKKLIERWACEIADFFIRNKVGTVQMENLESMKRKEDSYFNIRLRGFWPYAEMQNRIEFKLKQHGIEIRKVAPNNTSKTCSKCGHLNNYFSFEYRKKNKFPHFKCEKCNFKEDADYNAALNISNPKLKGTKEEL

SEQ ID NO: 3071 - protein, 726 aa, synthetic construct
SEVEFSHEYWMRHALTLAKRARDEREVPVGAILVLNNRVIGEGWNRAIGLHDPTAHAEIMALRQGGLVMQNYRLINATLYVTFEPCVMCAGAMIHSRIGRVVFGVRNNKHGAAGSLMNVLNYPGMNHRVEITEGILADECAALLCDFYRMPRQVFNARKKAQSSINPGGPPGGSSGSETPGTSESATPESSGGSSGGSAKNTITKTLKLRIVRPYNSAEVEKIVADEKNNREKIALEKNKDKVKEACSEHLKVAAYCTTQVERSACLFCKARKLDDKFYQKLRGQFPDAVFWQEIGEIFRQLQKQAAEIYNQSLIELYYEIFIKGKGIANASSVEHYLSDVCYTRAAELFKNAAIASGLRGKVKSNFRLKELRNMKSGLPTTKSDNFPIPLVRQKGGQYTGFEISNHDGDFIIKIPFGRWQVKKEINKHRPWEKFDFEQVRKSPKPISLLLSTQRRKRDKGWSKDEGTEAEIRKVMNGDYQTSYIEVKRGSKIGEKSAWMLNLSIDVPKIDKGVDPSIIGGIDVGVKSPLVCAINNAFSRYSIGDNDLFHYNKKMFARRRILLKKNRHKRAGHGTKNKLKPITILTEKSGRFRKKLIERWACEIADFFIKNKVGTVQMENLEGMKRKEDSYFNIRLRGFWPYAEMQNKIEFKLKQYGIKIRKVAPNNTSKTCSKCGHLNNYFNFEYRKRNKLPHFKCEKCNFKENADYNAALNISNPKLKGTKEEP

SEQ ID NO: 3072 - protein, 726 aa, synthetic construct
SEVEFSHEYWMRHALTLAKRARDEREVPVGAVLVLNNRVIGEGWNRAIGLHDPTAHAEIMALRQGGLAMQNYRLVDATLYVTFEPCVLCAGAMVHSRIGRVVFGVRNSKRGAAGSLMNVLNHPGMNHRVEITEGILTDECAALLCDFYRMPHQVLNAQKKAQSSINSGGSAGGSSGSETPGTSGSTTPVSSGGSSGGSAKNTITKALKLRIVRPYNSAEVEKIVADEKNNREKIALEKNKDKVKEACSKHLKVAAYCTTQVERNACLFCKARKLDDKFYQKLRGQFPDAVFWQEIGEIFRQLQRQAAEIYNQSLIELYYEILIKGKGFANASSVEHYLSDVCYTRAAELFKNAAIASGLRGKVKSNFRLKELKNMKSGLPTTKSDNFPIPLVKQKGGQYTGFEISSHNDDFIIKIPFGRWQVKKEIDKYRPWEKFDFEQVRKSPKPISLLLSTQRRKRNKGWSKDDGTEAEVRKVMNGDYRTSYIEVKRGSKTGEKSAWMLNLSIDVPKIDKGVDPSIIGGIDVGVKSPLVCAINNAFSRYSISDNDLFRFNKKMFARRRILLKKNRHKRAGHGAKNKLKPISILTEKSKRFRKKLIERWACEIADFFIKNKVGTVQMENLESMKRKEDGYFNIRLRGFWPYAEMQNKIEFKLKQYGIEIRKVAPNNTSKTCSKCGHLNNYFNFEYRKTNKFPHFKCEKCNFKEDADYNAALNISNPKLKSTKEEP

SEQ ID NO: 3073 - protein, 726 aa, synthetic construct
SEVEFSHEYWMRHALTLAKRARDEREVPVGAVLVLNNRVIGGGWNRAVSLRDPTAHAEIMALRQGGLVMQNHRLTDATLYVTFEPCVMCAGAMVHSRIGRVVFGVRNSRRGAAGSLMNVLNYPGMNHCVEITEGILVDECAALLCDYYRMPRQVLSAQKKARSSISSGGSSGGSSGSETPGASGSVTPKSSVGSSAGSTKNTITKTLKLRIVRPYNSAEVEKIVADEKNNREKIALEKNKGKVKEACSKHLEVAAYCTTQVERNACLFCKARKLDDKFYQKLRDQFPDAVFWQELGEIFRQLQKQAAEIYNQSLIELYYEIFIKGKGFANASNVEHYLSDVCYTRAAELFKNAAIASGLRGKVKSNFRLKELKNMKSGLPTTKSDNFPIPLVKQKGGQYTGFEISSHNDDFIIKIPFGRWQVRKEIDKYRPWEKFNFEQVRKSPKPISLLLSTQRRKRNKGWSKDEGTEAEIRKVMNGDYQTSYIEVKRGSKIGEKSAWMLCLSIDVPKIDKGVDPSIIGGIDVGVKSPLVCAINNAFNRYSISDNDLFHFNKKMFARRRILLKKNRHKRAGHGARNKLKPITVLTGKSERFRKKLIERWACEIANFFIKNKVGTVQMENLESMKRKEDSYFNNRLRGFWPYAEMQNKIEYKLKQYGIEVRKVAPNNTSKTCSKCGHLNDYFNFEYRKKNKFPHFKCEKCNFKENADYNAALNISNPKLKSTKEEP

SEQ ID NO: 3074 - protein, 726 aa, synthetic construct
SEDEFSHEYWMRHALTLAKRARDGREVPVGAVLVLNNRVIGEGWNRAIGLHDPTAHAEIMALRQGGLVMQNYRLIDATLYVTFEPCVMCAGAMVHSRIGRVVFGVRNSKRGAAGSLMNVLDYPGMGHHVEITEGILADECAALLCDFYCMPRQVFNARKKAQSSINPSGSSGGSSGSVTPGTSESATPESSGGGFGGSAKNTITKTLQLRIVRPYNSAEVEKIVADEKNSREKIALEKNKDKVKEACSEHLKVAAYCTTQVERSACLFCKARKLDDRFYQKLRGQFPDAVFWQEIGEIFRQLQKQAAEIYNQSLIELYYEIFIKGKGLANASSVEHYLSDVCYTRAAESFKNAAIASGLRGKVKSNFKLKELKSMKSGLPSTKSDNFPIPLVKQRGGQYTGFEISSHNDDFIIKIPFGRWQAKKEIDKYRPWEKFDFEQVRKSPKPISLLLSTQRRKRNRGWSKDEGTEAEIRKVMNGDYQTSYIEVKRGSKFGEKSAWMLNLSIDVPKIDKGVDPSIIGGIDVGVKSPLVCAINNAFSRYSISDNDLFRFNKKMFARRRILLGKNRHKRAGHGVKNKLKPITILTEKSGRFRKKLIERWACEIADFFVKNKVGTVQMENLESMKRKEDSYFNIRLRGFWPYAEMQNKIEFKLKQYGIKVRKVAPNNTSKTCSKCGHLNNYFSFEYRKKNKFPHFKCEKCNFKENADYNAALNISNPKLKSTKEEP

SEQ ID NO: 3075 - protein, 726 aa, synthetic construct
SEVEFSHEYWMRHALTLAKRARDEHEVPVGAVLVLDNRVIGEGWNRAVGLHDPTAHAEIMALRQGGLVMQNHRLVDATLYVTFEPCVLCAGAMVHSRIGRVVFGVRNSKRGAAGSLMNVLNHPDMNHRVEITEGILVDECAALLCDFYRMPRQVLNAQKKAQSSINPGGSSSGSSGSETPGTSESATPESSGGSSGGSAKNTITKALKLRIVRPYNSAEVEKIVADEKNNRERIALEKNKDKVKEACSKHLKVAAYCTTQVERNACLFCKARKLDDKFYRKLRGQFPDAVFWQEIGEIFRQLQKQAAEIYNQSLIELYYEIFIKGKGFANASSVEHYLSDVCYTRAAELFKNAAIASGLRGKVKSNFRLKELKNMKSGLPTTKSDNFPIPLVKQKGGQYTGFEISSHNSDFIIKIPFGRWQVKEEIDKYRPWEKFDFEQVRKSPKPISLLLSTQRRKKNKGWSKDEGTEAEIRRVMNGDYQTSYIEVKRGSKIGEKSAWMLNLSIDVPKIDKGVDPSIIGGIDVGVKSPLVCAINNALSRYSISDNDLFHFNKKMFARRRILLRKNRHKRAGHGAKNKLKPITMMTEKSKRFRKKLIERWACEIADFFIKNKVGTVQMENLESMKRKEDSYFNIRLRGFWPYAEMQDKIEFKLKQYGIVVRKVAPNNTSKTCSKCGHLNHYFNFEYRKKNKFPHFKCEKCNFKEDADYNAALNISNPKLKSTKGEP

SEQ ID NO: 3076 - protein, 726 aa, synthetic construct
GEVEFSHEYWMRHALTLAKRARDEREVPVGAVLVLNNRAIGEGWNRAIGLHDPTAHAEIMALRQGGLVMQNYRLTDATLYVTFEPCVMCAGAMIHSRIGRVVFGVRNSKRGAAGSLMNVLNYPGMNHRVEITEGVLADECAALLSDFYRMPRQVFNAQKKARPYINSGGSSGGSSGSETPGTSESPTPESSGGSSGGSAKNTITKTLKLRIVRPYNSAEVEKIVADEKNNREKIALEQNKDKVREACSKHLKVAAYCTTQVERNACLFCKARRLDDKFYQKLRGQFPDAVFWQEIGEIFRQLQKQAAEIYNQSLVELYYEIFIKGKGFANASSVEHYLSDVCYTRAAELFKNAAIASGLRGKVKSNLRLKELKNMKSGLPTTKSDNFPIPLVKQKGGQYTGFEISSHNDDFIIKIPFGRWQVKEEIDKYRPWEKFDFEQVRKNPKPISLLLSTQRRKRNKGWSKDEGTEAEIRKVMNGDYQTSYIEVKRGSKVGEKSAWMLNLSIDVPKIDKGVDPSIIGGIDVGVKSPLVCAINSAFSRYSISDNDLFHFNKKVFARRRILLKKNRHRRAGHGAKNKLKPISILTEKSERFRKKLIERWACEIADFFIKNKVGTVQMENLESMKRREDSYFNIRLRGFWPYAKMLNKIEFKLKQYGIKIRKVAPNNTSKTCSKCGHLNNYFNFEYRKKNKFPHFKCEKCNFKENADYNAALNISNPKLKSTKGEP

SEQ ID NO: 3077 - protein, 726 aa, synthetic construct
SEVEFSHEYWMRHALTLAKRARDEREVPVGAILVLNNRVIGEGWNRAIGLHDPTAHAEIMALRQGGLVMQNYRLIDATLYVTFEPCVMCAGAMIHSRIGRVVFGVRNNKHGAAGSLVNVLDYPGMNHRVEITEGILADECAALLCDFYRMPRQVFNARKKAQSSISPGGSSDGGSGSETPGTCESVTPESSGGSSGGSAKNTITKTLKLRIVRPYNSAEVEKIVADEKNSREKIALEKNKDKVKEACSEHLKVAAYCTTQVERNACLFCKARKLDDRFYQKLRGQFPDAVFWQEIGEIFRQLQKQAAEIYNQSLIELYYEIFIKGKGFANASSVEHYLSDVCYTRAAELFKNAAIASGLRGKVKSNFRLKELKNMRSGLPTTKSDNFPIPLVKQKGGQYTGFEISDHNSDFIIKIPFGRWQVKKEIDKYRPWEKFDFEQVRKSPKPISLLLSTQERKKNKGWSRDEGTEAEIRKVMNGDYQTSYIEVKRGSKIGEKSAWMLNLSIDVPKIDKGVDPSIIGGIDVGVKSPLVCAINNAFSRYSISDNDLFRFNKKMFARRRILLKKNRHKRAGHGAKNKLKPISILTGKSERFRRKLIERWACEIADFFIKNKVGTVQMENLESMKRKEDSYFNIRLRGFWPYAEMQNKIEFKLKQYGIEIRKVAPNNTSRTCSKCGHLNNYFNFEYRRKYKFPHFKCEKCNFKEDADYNAALNISNPKLKSTKEEP

SEQ ID NO: 3078 - protein, 726 aa, synthetic construct
SEVEFSHEYWMRHALTLAKRARDEREVPVGAILVLNNRVIGEGWNRAIGLHDPTAHAEIMALRQGGLVMQNYRLIDATLYVTFEPCVMCAGAMIHSRIGRVVFGARNSKHGAAGSLMNVLNYPGMNHRVEITEGILADECAALLCDYYRMPRQVFNARKKVQSSINSGGSSDGGSSSETPGTSESATPESSGGGSGGSAKNTITKTLKLRIVRPYNSAEVEKIVADEKNNREKIALEKNKDKVKEACSEHLKVAAYCTTQVERSACLFCKARKLDDKFYQELRGQFPDAVFWQELGEILRQLQKQAAEIYNQSLIELYYEIFIKGKGFANASSVEHYLSDVCYTRAAELFKNAAIASGLRGKVKSNFRLKELKNMKSGLPTTKSDNFPIPLVKQKGGQYTGFEISSHNDDFIIKIPFGRWQVKKEIDKYRPWEKFDFEQVRKSPKPISLLLSTQRRKRNKGWSKDEGTEAEIRKVMNGDYQTSYIEVKRGSKTGEKSAWMLNLSIDVPKIDKGVDPSIIGGIDVGVKSPLVCAINNSSSRYSICDNDLFRFNKKMFARRRILLKKNRHKRAGHGAKNKLKPITILTKKSERFRKKLIERWVCEVADFFIKNKVGTVQMENLESMKRKEDSYFNIRLRGFWPYAEMQNRIELKLKQYGIEIRRVAANNTSRTCSKCGHLNNYFNFEYRKKSKFPHFKCEKCNFREDADYNAALNISNPKLKSTKEEP

SEQ ID NO: 3079 - protein, 726 aa, synthetic construct
SEVEFSHEYWMRHALSLAKRARDEREVPVGAVLVLNNRIIGEGWNRAIGLHDPTAHAEIMALRQGGLVMQNYRLTDATLYVTFEPCVMCAGAMVHSRIGRVVFGVRNSKRGAAGSLMNVLNYPGVNHCVEITEGILVDECAALLCDFYRMPRQVLNAQKKAQSSISSGGSSGGCSGSEMPGASESVTPKSSGGSSAGSTKNTITKTLKLRIVRPYNSAEVEKIVADEKNSREKIALERNKGKVKEACSEHLKVAAYCTTQVERNACLFCKARKLDDRFYQKLRGQFPDAVFWQETGEILRQLQKQAAEIYNQSLIELYYEIFIKGRGFANASSVEHYLSDVCYTRAAELFKNAAIASGLRGKVKSNFRLKELKNMKSGLPTTKSDNFPIPLVKQKGGQYTGFEISSHNDDFIIKIPFGRWQVKKEIDKYRPWEKFDFEQVRKSPKPISLLLSTQRRRKNKGWSKDEGTEAEIRRVMNGDYQTSYIEVKRGSKIGEKSAWMLNLSIDVPKIDKGVDPSIIGGIDVGVKSPLVCAINNTLSRYSISDNDLFHFNKKMFARRRILLKKNRHKRAGHGARNKLKPITVLTGKSERFRKKLIERWACEIANFFIKNKVGTVQMENLESMKRKEDSYFNNRLRGFWPYAEMQNKIEYKLKQYGIEVRKVAPNNTSKTCSKCGHLNNYFNFEYRKKNKYPYFKCEKCNFKEDADYNAALNISNPKLKSTGEEP

SEQ ID NO: 3080 - protein, 725 aa, synthetic construct
SEVEFSHEYWMRHALTLAKRARDEREVPVGAILVLNNRVIGEGWNRAIGLHDPTAHAEIMALRQGGQVMQNYRLIDATLYVTFEPCVMCAGAMIHSRIGRVVFGVRNNKHGAAGSLVNVLNHPGMNHCIEITEGILVDECAALLCDFYRMPRQVLSAQKKAQSSINSGGSSGGSSGSETPGTSSATPESSGGGSSGSAKNTITKTLQLRIVRPYNSAEVEKIVADEKNNREKIALEKNKDKVKEACSKHLKVASYCTTQVERNACLFCKARKLDDKFYQKLRGQFPDAVFWQELGEIFRQLQKQAAEIYNQSLIELYYEIFIKGKGLASASSVEHYLSDVCYTRAAELFKNAAIASGLRGKVKSNFKLKELKSMKSGLPSTKSDNFPIPLVKQRGGQYTGFKISSHNGDFIIKIPFGRWQAKKEIDKYRPWEKFDFEQVRKSPKPISLLLSTQRRKRNRGWSKDEGTEAEIRKVMNGDYQTSYIEVKRGSKIGEKSAWMLNLSIDVPKIDKGVDPSIIGGIDVGVKSPLVCAINNAFSRYSISDNDLFRFNKKMFARRRILLGKNRHKRAGHGVKNKLKPITILTEKSGRFRKKLIERWACEIADFFVKNKVGTVQMENLESMKRKEDSYFNIRLRGFWPYAEMQNKIEFKLKQYGIKVRKVAPNNTSKTCSKCGHLNNYFSFEYRKKNKLPHFKCEKCNFKENADYNAALNISNPKLKSTKEEP

SEQ ID NO: 3081 - protein, 726 aa, synthetic construct
SEVEFSHEYWMRHALTLAKRARDEREVPVGAILVLNNRVIGEGWNRAIGLHDPTAHAEIMALRQGGLMMQNYRLIDATLYVTFEPCVMCAGAMIHSRIGRVVFGVRNSKHGAAGSLVNVLNYPGMNHRVEITEGILADECAALLCDFYRMPRQVFSARKKAQSSISPGDSSGGSSGSEAPGASGSVTPKSSGGSSAGSTKDTITKTLKLRIVRPYNSAEVEKIVADEKNSREKIALEKNKDKVKEACSEHLKVAAYCTTQVERNACLFCKARRLDDKFYQKLRGQFPDAVFWQEIGEIFRQLQKQAAEVYNQSLVELYYEILIKGKGIANASSVEHYLSDVCYTRAAELFKNAAIASGLRNKIKSNFRLKELRNMRSGLPTTKSDNFPIPLVRQKGGQYTGFEISNHDGDFIIKIPFGRWQVKKEIDKYRPWEKFDFEQVRKSPKPISLLLSTQRRKGNKGWSKDEGTEAEIKKVMNGDYQVSYIEVKRGSKIGEKSAWMLNLSVDVPKIDKGVDPSIIGGINVGVKSPLVCAINDALSRYSISDNDLFHFNKKMFARRRILLRKNRHKRAGHGAKNKLKPVTILTEKSERFRKKLIERWACEIANFFIKNKVGTVQMEDLESMKRKEDSYFNIRLRGFWPYAEMQNKIEFKLKQFGIEIRKVAPNDTSKTCSKCGHLNNYFNFEYRKKNKFPHFKCEKCNFKENADYNAAQNISNPQLKSTKEEP

SEQ ID NO: 3082 - protein, 726 aa, synthetic construct
SEDEFSHEYWMRHALTLAKRARDGREVPVGAVLVLNNRIIGEGWNRAIGLHDPTAHAEIMALRQGGLVLQNYRLIDATLYVTFEPCVMCAGAMVHSRIGRVVFGVRNSKRGAAGSLMNVLDYPGMGHRVEITEGILADECAALLCDFYCMPRQVFNAQKRAQSSINSGGSSGGSSGSETPGTSESATPESSGGGPSGSAKNTITKTLQLRIVRPYNSAEVEKVVADEKNNREKIALEKNKDKVKEACSKHLKMASYCTTQVERNACLFCKARKLDDKFYQKLRGQFPDAVFWQELGGIFRQLQKQAAEIYNQSLIELYYEIFIKGKGITNASRVEHYLSDVCYTRAAELFKNAAIASGLRGKVKSNFKLKELKSMKSGLPSTRSDNFPIPLVKQKGGQYTGFEISSHNDDFIIKIPFGRWQAKKEIDKHRPWEKFDFEQVRKSPKPISLLLSTQRRKRSKGWSKDEGTEAEIRKVMNGDYQTSYIEVKRGSKIGEKSAWMLNLSIDVPKIDKGVDPSIIGGIDVGVKSPLVCAINNAFSRYSISDNDLFHFNKKMFARRRILLKKNRHRRAGHGAENKLKPISILTEKSKRFRKKLIERWACEIADFFIKNKVGTVQMENLESMKRKEDSYFNIRLRGFWPYAEMQNKIEFKLKQYGIKIRKVAPNNTSKTCSKCGHLNSYFNFEYRKKNKFPHFKCEKCNFKENADYNAALNISNPKLKNTKEEP

SEQ ID NO: 3083 - protein, 726 aa, synthetic construct
SEVEFSHEYWMRHALTLAKRARDEREVPVGAILVLNNRVIGEGWNRAIGLHDPTAHAEIMALRQGGLVMQNYRLIDATLYVTFEPCVMCAGAMIHSRIGRVVFGVRNSKHGAAGSLMNVLNYPGMNHRVEITEGILVDECAALLCDFYRMPRQVFNARKKAQSSINPGGSSGGSSGSEMPGSSESATPESSGGSSSGSAKNTITKTLQLRIVRPYNSAEVEKIVADEKNNREKIALEKNKDKVKEACSKHLKVASYCTTQVERNACPFCKARKLDDKFYQKLGGQFPDAVFWQELGEILRQLQKQAAEIYNQSLIELYYEIFIKGKGITNASRVEHYLSDVCYTRAAELFKNAAIASGLRSKVRSNFRLKELKNMKSGLPTTKSDNFPIPLVKQKGGQYTGFEISSHNSDFIIKIPFGRWQVKEEIDKYRPWEKFDFEQVRKSPKPISLLLSTQRRKRNKGWSKDEGTEAEIRKVMNGDYQTSYIEVKRGSKTGEKSAWVLNLSIDVPKIDKGVDPSIIGGIDVGVKSPLVCAINNALSRYSISDNDLFHFNKKMFARRRILLKKNRHRRAGHGARNKLKPITVLTEKSKRFRKKLIERWACEIANFFIKNKVGTVQMENLESMKRKEDSYFNIRLRGLWPYAEMQNKIEFKLKQYGIEIRKVAPNNTSKTCSKCGHLNDYFNFEYRKRNKFPHFKCEKCNFKENADYNAALNISNPKLKGTKEEP

SEQ ID NO: 3084 - protein, 726 aa, synthetic construct
SEVEFSHEYWMRHALTLAKRARDEREVPVGAVLVLNNSVIGEGWNRAIGLHDPTAHAEIMALRQGGLVMQNCRLVDATLYVTFEPCVMCAGAMIHSRIGRVVFGVRNSKRGAAGSLMNVLNYPGMNHRVEITEGILADECAALLCDFYRMPRQVLSARRKAQSSISPGGSSGGSSGSETPGTSKSPTPESPGGSSGGSAKNTITKTLKLRIVRPYNSAEVEKIVADEKNNREKIALEKNKDKVKEACSKHLKVAAYCTTQVERNACLFCKARKLDDKFYQKLRGQFPDAVFWQEIGEIFRQLQKQAAEIYNQSLIELYYEIFIKGRGFANASSVEHYLSDVCYTRAAELFKNAAIASGLRGKVKSNFRLKELKNMKSGLPTTKSDNFPIPLVKQKGGQYTGFEISSHNDDFIIKIPFGRWQVRKEIDKYRPWEKFDFEQVRKSPKPISLLLSTRRRKRNKGWSKDEGTEAEIRKVMNGDYQTSYIEVKRGSKIGEKSAWMLSLSIDVPKLDRGADPSIIGGIDVGVRSPLVCAIDNSFSRYSISDNDLFHFNKKMFARRRILLKKNRHKRAGHGAKNKLKPITILTKKSERFRKKLIERWACEVADFFIKNKVGTVQMENLESMKRKEDSYFNIRLRGFWPYAEMQDRIEFKLKQYGIEIRRVAPNNTSRTCSKCGHLNNYFNFEYRKTNKFPLFKCEKCNFREDADYNAAMNISNPKLKSTKEEP

SEQ ID NO: 3085 - protein, 726 aa, synthetic construct
GEDEFSHEYWMRHALTLAKRARDGREVPVGAVLVLNNRVIGEGWNRAIGLHDPTAHAEIMALRQGGLVVQNYRLIDATLYVTFEPCVMCAGAMIHSRIGRVVFGVRNSKHGAAGSLMNVLNYPGMNHRVEITEGILADECAALLCDFYRMPRQVFNARKKAQSSINPGGPSGGSSGSETPDTSESATPESSGGNSGGSAKNTITKTLKLRIVRPYNSAEVEKIVADEKNNREKIALEKNKDKVKEACSEHLKVAAYCTTQVERSACLFCKARKLDDKFYQKLGGQFPDAVFWQETGEIFRQLQRQAAEIYNQSLIELYYEIFIKGKGFANASSVEHYLSDVCYTRAAELFKNAAVASGLRGKVKSNFRLKELKNMKSGLPTTKSDNFPIPLVRQKGGQYTGFEISNHDGDFIIKIPFGRWQVKKEIDKYRPWEKFDFEQVRKSPKPISLLLSTQRRKRNKGWSKDEGTEAEIRKVMNGDYQTSYIEVKRGSKIGEKSAWMLNLSIDVPKIDKGVDPSIIGGIDVGVKSPLVCAISNAFSRYSISDNDLFHFNKKMFARRRILLKKNRHKRAGHGAKNKLKPISILTEKSVRFRKKLIERWACEIADFFIKNKVGTVQMENLEGMKMKEDSYFNIRLRGFWPYAEMQSKIEFKLKQYGIKIRKVAPNNTSKTCSKCGHLNNYFNFEFRKKNKFPHFKCEKCNFKEDADYNAALNISNPKLKSTKEEP

SEQ ID NO: 3086 - protein, 726 aa, synthetic construct
SEVEFSHEYWMRHALTLAKRARDEREVPVGAVLVLNNRVIGEGWNRAIGLHDPTAHAEIMALRQGGLVLQNYRLVDATLYVTFEPCVLCAGAMVHSRIGRVVFGARNSKRGAAGSLMNILNYPGMNHRVEITEGILADECAALLCDFYRMPRQVFNAQKKAQSSINTGGSSGGSSGSETPSTSESATPESSGGSSGGSVKNTITKTLQLRIVRPYNSAEVEKIVTDEKNNREKIALEKNKDKVKEACSEHLKVAAYCTTQVERNACLFCKARKLDDKFYQKLRGQFPDAVFWQEVGEIFRQLQKQAAEIYNQSLIELYYEIFIKGKGFANASSVEHYLSDVCYTRAAELFKNAAIASGLRGKVKSNFRLKELKNMKSGLPTTKSDNFPIPLVKQKGGQYTGFEISNHNSDFIIKIPFGRWQVKKEINKYRPWEKFDFEQVRKSPKPISLLLSTQRRKRNKGWSKDEGTEAEIRKVMNGDYQTSYIEVKRGSRIGEKSAWMLSLSIDVPKIDRGVDPSIIGGIDVGVKSPLVCAINNAFSRYSISDNDLFHFNKKMFARRRILLKKNRRRRAGHGAKNKLKPITILTEKSVRFRKKLIERWACEIADFFIKNKVGTVQMENLESMKRKEDSYFNIRLRGFWPYAEMQNKVEFKLKQYGIEIRRVAPNNTSRTCSKCGHLNNYFNFEYRRKYKFPHFKCEKCNFKEDADYNAALNISNPKLKSTKEEP

SEQ ID NO: 3087 - protein, 726 aa, synthetic construct
SEVEFSHEYWMRHALTLAKRARDGREVPVGAVLVLNNRVIGEGWNRATGLHDPTAHAEIMALRQGGLVMQNYRLIDATLYVTFEPCVMCAGAMVHSRIGRVVFGVRNSKRGAAGSLMNVLDYPGMGHRVEITEGILADECAALLCDFYCMPRQVFNAQKRAQSSINSGGSSGGSSGSETPGTSESATPESSGGGSSGSAKNTITKTLQLRIVRPYNSAEVEKIVADEKNNREKIALEKNKDKVKEACSKHLKVASYCTTQVERSACPFCKARKLDDKFYQKLGGQFPDAVFWQELGEIFRQLQKQAAEIYNQSLVELYYEILIKGKGIANASSVEHYLSDVCYTRAAELFKNAAIASGLRGKVKSNFRLKELKNMKSGLPTTKSDNFPIPLMKQKGGQYTGFEISSHNDDFIIKIPFGRWQVKKEIDRYRPWEKFDFEQVRKSPKPISLLLSTQRRKRNKGWSKDEGTEAEIRKVMNGDYQTSYIEVRRGSKIGEKNTWMLSLSIDVPKIDKGVDPSIIGGIDVGVKSPLVCAINNAFSRYSISDNDLFHFNKKMFARRRILLRKNRHKRAGHGAKNKLKPITILTEKSRRFRKKLIERWVCEVADFFIKNKVGTVQMENLESMKRREDSYFNIRLRGFWPYAEMQNKIEFKLKQYGIEIRKVAPNNTSKTCSKCGYLNNYFNFEYRKKNKFPHFKCEKCNFKENADYNAALNISNPKLKSTKEEP

SEQ ID NO: 3088 - protein, 726 aa, synthetic construct
SEVEFSHEYWMRHALTLAKRARDEREVPVGAVLVLNNRVIGEGWNRAIGLHDPTAHAEIMALRQGGLVMQNYRLVDATLYVTFEPCVLCAGAMVHSRIGRVVFGARNSKRGAAGSLMNILNYPGMNHRVEITEGILADECAALLCDFYRMPRQVFNAQKKAQSSINSGGSSGGSSGSETPSTSESATPESSGGSSGGSAKNTITKTLQLRIVRPYNSAEVEKIVTDEKNNREKIALEKNKDKVKEACSKHLEVAAYCTTQVERNACLFCKARKLDDKFYQKLRGQFPDAVFWQEIGEIFRQLQKQAAEIYNQSLIELYYEILIKGKGFANASSVEHYLSDVCYTRAAELFKNAAIASGLRGKVKSNFRLKELKNMKSGLPTTKSDNFPIPLVKQKGGQYTGFEISSHNSDFIIKIPFGRWQEKEEIDKYRPWEKFDFEQVRKSPKPISLLLSTRRRKRNKGWSKDEGTEAEIRKVMNGDYQTSYIEVTRGSKIGEKSAWMLNLSIDVPKIDKGVDPSIIGGIDVGVKSPLVCAINNAFSRYSISDNDLFHFNKKMFARRRILLKKNRHKRAGHGAKNKLKPITILTEKSKRFRKKLIERWACEIADFFVKNKVGTVQMENLESMKRKEDSYFNIRLRGFWPYAEMQNKIEFKLKQYGIEIRKVAPNNTSKTCSKCGHLNNYFNFEYRKKNKFPHFKCEKCNFKENADYNAALNICNPKLKSTKEEP

SEQ ID NO: 3089 - protein, 726 aa, synthetic construct
SEVEFSHEYWMRRALTLAKRARDEREVPVGAVLVLNNRVIGVGWNRAVGLHDPTAHAEIMALRQGGLVMQNYRLIEATLYVTFEPCIMCAGAMIHSRIGRVVFGVRNSKHGAAGSLVNVLNYPGMNHRVEITEGILADECAALLCDFYRMPRQVFNARKKAQSSINSGGSSGGSSSSGTPGTSESATPKSSGGSSGGSAKNTITKALKLRIVRPYNSAEVEKIVADEKNNRERIALEKNKDKVKEACSKHLKVAAYCTTQVERNACLFCKARKLDDKFYQKLRGQFPDAVFWQEIGEIFRQLQKQAAEIYNQSLIELYYEILIKGKGFANASSVEHYLSDVCYTRAAELFKNAAIASGLRGKVKSNFRLKELKNMKSGLPTTKSDNFPIPLVKQKGGQYTGFEISSHNSDFIIKIPFGRWQEKEEIDKYRPWEKFDFEQVRRSPKPISLLLSTQRRKKNKGWSKDEGTEAEIRRVMNGDYQTSYIEVKRGSKIGEKSAWMLNLSIDVPKIDKGVDPSIIGGIDVGVKSPLVCAINNAFSRYSISDNDLFHFNKKMFARRRILLKKNRHKRAGHGAKNKLKPISILTEKSKRFRKKLIERWACEIADFFIKNKVGTVQIENLESMKRKEDSYFNIRLRGFWPYAEMQNKIEFKLKQYGIEIRKVAPNNTSKTCSKCGHLNNYFNFEYRKKNKFPHFKCEKCNFKEDADYNAALNISNPKLKSTKGEP

SEQ ID NO: 3090 - protein, 726 aa, synthetic construct
SEVEFSHEYWMRHALTLAKRARDEREVPVGAVLVLNNRVIGEGWNRAIGLHDPTAHAEIMALRQGGLVMQNYRLIDATLYVTFEPCVMCAGAMIHSRIGRVVFGVRNNKHGAAGSLVNVLNYPGMNHRVEITEGILADECAGLLCDFYRMPRQVFNAQKKAQSSINSGGSSGGSSSSETPGTSESPTPESSGGSPGGSAKNTITKTLKLRIVRPYNSAEVEKIVADEKNSREKIALERNKDKVKEACSEHLKVAAYCTTQVERNACLFCKARKLDDRFYQKLRGQFPDAVFWQETGEIFRQLQRQAAEIYNQSLIELYYEIFIKGKGFANASSVEHYLSDVCYTRAAELFKNAAIASGLRGKVKSNFRLKELKNMKSGLPTTKSDNFPIPLVKQKGGQYTGFEISNHNDDFIIKIPFGRWQVKKEIDKYRPWEKYDFEQVRKSPKPISLLLSTQRRKRNKGWSKDEGTEAEIRKVMNGDYQTSYIEVKRGSKTGEKSAWMLNLSIDVPKIDKGVDPSIIGGIDVGVKSPLVCAINNAFSRYSISDNDLFRFNKKMFARRRILLKKNGHKRAGHGARNKLKPITVLTEKSKRFRKKLIERWACEIANFFIKNRVGTVQMENLESMKRKEDSYFNIRLRGFWPYAEMQNRIEFKLKQYGIEIRKVAPNNTSKTCSKCGHLNNYFNFEYRKKNKFPHFKCEKCNFKENADYNAALNICDPKLKGTKEEP

SEQ ID NO: 3091 - protein, 726 aa, synthetic construct
SEVEFSHEYWMRHALTLAKCARDEREVPVGAILVLNNRVIGEGWNRAIGLHDPTAHAEIMALRQGGLVMQNYRLTDATLYVTFEPCVMCAGAMIHSRIGRVVFGVRNNKHGAAGSLVNVLNYPGMNHRVEITEGILADECAALLCDFYRMPRQVFNARKKAQSSINPGGLSGGSSGSETPGTSESATPESSGGSSSGSAKNTITKTLQLRIVRPYNSAEVEKIVADEKNDRERIALEKNKGKVKEACSKHLEVAAYCTTQVERNACLFCKARTLDDKFYQKLRGQFPDAVFWQELGEILRQLQKQAAEIYNQSLIELYYEIFIKGRGFANASSVEHYLSDVCYTRAAELFKNAAIASGLRGKVKSNFRLKELKNMKSGLPTTKSDNFPIPLVRQKGGQYTGFEISSHNDDFIIKIPFGRWQVKKEINKYRPWEKFDFEQVRKSPKPISLLLSTQRRKRNKGWSKDEGTEAEIRRVMSGDYQTSHIEVKRGSKTGEKSAWMLSLSIDVPKIDKGVDPSIIGGIDVGVKSPLVCAINNAFSRYSISDNDLFRFNKKLFARRRILLKKNRHKRAGHGAKNKLKPISILTGKSERFRKKLIERWACEIADFFIKNKVGTVQMENLESMKRKEDSYFNIRLRGFWPYAEMQNKIEFKLKQYGIEIRKVAPNNTSKTCSKCGHLNNYFNFEYRKKNKFPHFKCEKCNFKENADYNAALNISNPKLKSTKEKP

SEQ ID NO: 3092 - protein, 726 aa, synthetic construct
GEVEFSHEYWMRRALTLAKRARDEREVPVGAILVLNNHVIGEGWNRAIGLHDPTAHAEITALRQGGLVMQNYRLIDATLYVTFEPCVMCAGAMIHSRIGRVVFGVRNSKHGAAGSLVNVLNYPGMNHRVGITEGILADECAALLCDFYRMPRQVFNARKKAQSSINPGGSSGGSSGSETPGTSESATPESSGGGSSGSAKNTITKTLQLRIVRPYNSAEVEKIVADEKNNREKIALERNKDKVKEACSEHLKVAAYCTTQVERNACLFCKARKLDDKFYQKLRGQFPDAVFWQELGEILRQLQKQAAEIYNQSLVELYYEIFIKGRGFANASSVEHYLSDVCYTRAAELFKNAAIASGLRGKVKSNFRLKELKNMRSGLPTTKSDNFPIPLVKQKGGQYTGFEISSHNDDFIIKIPFGRWQVKKEIDKYRPWEKFDFEQVRKSPKPISLLLSTQRRRRNKGWSKDEGTEAEIRKVMYGDYQTSYIEVKRGSKIGEKSAWMLNLSIDVPKIDKGVDPSIIGGIDVGVKSPLVCAINNAFSRYSISDNDLFRFNKKVFARRRILLKKNRHKRAGHGTKNKLKPITILTEKSGRFRKKLIERWACEIANFFIKNKVGTVQMENLESMKRKEDSYFNIRLRGFWPYAEMQNKIEFKLKQYGIKIRRVAPNNTSKTCSKCGHLNNYFSFEYRKKNKFPHFKCEKCNFKEDADYNAALNISNPKLKSTKEEP

SEQ ID NO: 3093 - protein, 726 aa, synthetic construct
SEVEFSHEYWMRHALTLAKRARDEREVPVGAVLVLNNRVIGEGWNRAIGLHDPTAHAEIMALRQGGLVMQNYRLTDATLYVTFEPCVMCAGAMIHSRISRVVFGVRNSKRGAAGSLMNVLNHPGMNHRVEITEGILADECAALLCDFYRMPRQVFNAQKKARSNINSGGSSGGSSGSETPSTSESATPKSSGGSSGGSAKNTITKALKLRIVRPYNSAEVEKIVADEKNNRERIALEKNKDKVKEACSKHLKVAAYCTTQVERNACLFCKARKLDDKFYQKLRGQFPDAVFWQEIGEIFRQLQKQAAEIYNQSLIELYYEILIKGKGIANASSVEHYLSDVCYTRAAELFKNAAIASGLRNKIKSNFRLKELRNMKSGLPTTKSDNFPIPLVKQKGGQCTGFEISNHNSDFIIKIPFGRWQVKKEIDKYRPWEKFDFEQVRKSPKPISLLLSTQRRRRNKGWSKDEGTEAEIRKVMNGDYQASYIEVKRGSKIGEKSAWMLNLSIDVPKIDKGVDPSIIGGIDVGVRSPLVCAIDNAFSRYSISDNDLFHFNKKMFARRRILLKKNRHKRVGHGAKNKLKPISILTEKSKRFRKKLIERWACEIADFFIKNKVGTVQMENLVSMKRKEDSYFNIRLRGLWPYAEMQNKIEFKLKQYGIKIRKVAPNNTSKTCSKCGHLNNYFNFEYRKKNKFPHFKCEKCNFKEDADYNAALNISNPKLKSTKEEP

SEQ ID NO: 3094 - protein, 726 aa, synthetic construct
SEVEFSHEYWMRHALTLAKRARDEREVPVGAVLVLNNRVIGEGWNRAIGLHDPTAHAEIMALRQGGLVMQNYRLVDATLYVTFEPCVLCAGAMVHSRIGRVVFGVRNSKRGAAGSLMNVLDYPGMGHRVEITEGILADECAALLCDFYCMPRRVFNAQKRAQSSINSGGSSGGSSGSETPGTSESATPESSGGGSSGSAKNTITKTLQLRIVRPYNSAEVEKIVTDEKNNREKIALEKNKDKVKEACSKHLKVAAYCTTQVERNACLFCKARKLDDKFYRKLRGQFPDAVFWQEIGEIFRQLQKQAAEIYNQSLIELYYEIFIKGKGFANASSVEHYLSDVCYTRAAELFKNAAIASGLRGKVKSNFRLKELKNMKSGLPTTKSDNFPVPLVKQKGGQYTGFEISNHNSDFIIKIPFGRWQVKEEINKYRPWEKFDFEQVRKSPKPISLLLSTQRRKRNKGWSKDEGTEAEIRKVMNGDYQTSYIEVRRGSKIGERSAWMLNLSIDVPKIDKGVNPSIIGGIDVGVKSPLVCAINNAFSRYSISDNDLFRFNKKMFARRRILLGKNRHKRAGHGVKNKLKPITILTEKSGRFRKKLIERWACEIADFFVKNKVGTVQMENLESMKRKEDSYFNIRLRGFWPYAEMQNKIEFKLKQYGIKVRKVAPNNTSKTCSKCGHLNNYFSFEYRKKNKFPHFKCEKCNFKENADYNAALNISNPKLKSTKEEP

SEQ ID NO: 3095 - protein, 725 aa, synthetic construct
SEVEFSHEYWMRRALTLAKRARDGREVPVGAVLVLNNRVIGVGWNRVVGLHDPTAHAEIMALRQGGLVMQNYRLVEATLYVTFEPCIMCAGAMIHSRIGRVVFGVRNSKRGAAGSLMNVLNYPGMNHRVEITEGILADECAALLCDYYRMPRQVFNARKKAQSSINSGGSSDGGSGSETPGTSESATPESSGGSSGGSAKNTITKTLKLRIVRPYNSAEVEKIVADEKNNREKIALEKNKDKVKEACSKHLKVAAYCTTLVERNACPFCKARKLDDGFYQKLRGQFPDAVFWQEIGEIFRQLQKQAAEIYNQSLIELYYEIFIRGKGFANASSVEHYLSDVCYTRAAELFKNAAIASGLRGKVKSNFRLKELKNMKSGLPTTKSDNFPIPLVKQKGGQYTGFEISSHNDDLIVKIPFGRWQVKKEIDRYRPWEKFDFEQVRKSPKPISLLLSTRRKRNKGWSKDEGTEAEIRKVMNGDYQISYIEVKRGSKIGEKSAWMLNLSIDVPKIDKGVDPSIIGGIDVGVKSPLVCAINNSSSRYSICDNDLFRFNKKMFARRRILLKKNRHKRAGHGAKNKLKPITILTKKSERFRKKLIERWVCEVADFFIKNKVGTVQMENLESMKRKEDSYFNIRLRGFWPYAEMQNRIELKLKQYGIEIRRVAPNNTSRTCSKCGHLNNYFNFEYRKKNQFPYFKCEKCNFREDADYNAALNISNPKLKSTKEEP

SEQ ID NO: 3096 - protein, 726 aa, synthetic construct
SEVEFSHEYWMRHALTLAKRARDEREVPVGAVLVLNNRVIGEGWNRAIGLHDPTAHAEIMALRQGGLVMQNYRLTDATLYVTFEPCVMCAGAMIHSRIGRVVFGIRNSKRGAAGSLMNVLNYPGMNHCVEITEGILVDECAALLCDFYRMPRQVLNAQKRAQSSISSGGSSGGSSGSGTPGASESVAPKSSVGSSAGSAKSTITKTLKLRIVRPYNSAEVEKIVADEKNNREKTALEKNKDKVKEACSEHLKVAAYCTTQVERSACLFCKARKLDDKFYQKLRGQFPDAVFWQELGEILRQLQKQAAEIYNQSLVELYYEIFIKGKGFANASSVEHHLSDVCYTRAAELFKNAAIASGLRGKVKSNFRLKELKNMKSGLPTTKSDNFPIPLVKQKGGQYTGFEISSHNDDFIIKIPFGRWQVKKEINKYRPWEKFDFEQVRKSPKPISLLLSTQRRKRNKGWSKDEGTEAEIRKVMNGDYQTSYIEVKRGSKVGEKSAWMLSLSIDVPKIDRGVDPSIIGGIDVGVKSPLVCAINNALSRYSISDNDLFHFNKKMFARRRILLKKNRHRRAGHGARNKLKPITVLTEKSKRFRKKLIERWACEIANFFIKNKVGTVQMENLESMKRKEDSYFNIRLRGLWPYAEMQNKIEFKLKQYGIEIRKVAPNNTSKTCSKCGHLNNYFNFEYRKRNKFPHFKCEECNFKENADYNAALNISNPKLKGTKEEP

SEQ ID NO: 3097 - protein, 726 aa, synthetic construct
SEVEFSHEYWMRHALTLAKRARDEREVPVGAILVLNNRVIGEGWNRAIGLHDPTAHAEIMALRQGGLVMQNYRLIDATLYVTFEPCVMCAGAMIHSRIGRVVFGVRNSKHGAAGSLVNVLNYPGMNHRVEITEGILADECAALLCDFYRMPRQVFNARKKAQSSINPSGSSGGSSGSKTPGTSESATPEGSSGSSGGSAKNTITKTLKLRIVRPYNSAEVEKIVADEKNNREKIALEKNKDKVKEACSKHLKVAAYCTTQVERNACLFCKARRLDDKFYQKLRGQFPDAVFWQEIGEIFRQLQKQAAEIYNQSLIELYYEIFIKGKGITNASRVEHYLSDVCYTRAAELFKNAAIASGLRGKIKSNFRLKELKNMKSGLPTTKSDNFPIPLVKQKGGQYTGFEISSHNSDFIIKIPFGRWQVKEEIDKYRPWEKFDFEQVRKSPKPISLLLSTQRRKKNKGWSKDEGTEAEIRRVMNGDYQTSYIEVKRGSKIGEKSAWMLNLSIDVPKIDKGVDPSIIGGIDVGVKSPLVCAINNSSSRYSICDNDLFRFNKKMFARRRILLKKNRHKRAGHGAKNKLKPITILTKKSERFRKKLIERWVCEVADFFIKNKVGTVQMENLESMKRKEDSYFNIRLRGFWPYAEMQNRIELKLKQYGIEIRRVAPNNTSRTCSKCGHLNNYFNFEYRKKSKFPHFKCEKCNFREDADYNAALNISNPKLKSTKEEP

SEQ ID NO: 3098 - protein, 726 aa, synthetic construct
SEVEFSHEYWMRHALALAKRARDEREVPVGAVLVLNNRVIGEGWNRAIGLHDPTAHAEIMALRQGGLVMQNYRLTDATLYVTFEPCVMCAGAMVHSRIGRVVFGVRNSKRGAAGSLMNVLNYPDMNHCVEITEGILVDECAALLCDFYRMPRQVLNSQKKAQSSISSGGSSGGSSGSETPGASESATPKSSGGSSGGSTKNTITKTLKLRIVRPYNSAEVEKIVADEKNNRERTALEKNKDKVKEACSKHLKVAAYCTTQVERNACLFCKARKLDDKFYQKLRGQFPDAVFWQEIGEIFRQLQRQAAEIYNQSLIELYYEIFIKGKGFANASNVEHYLSDVCYTRAAELFKNAAIASGLRGKVKSNFRLKELKNMKSGLPTTKSDNFPIPLVKQKGGQYAGFEISSHNGDFIIKIPFGRWQVKKEIDKYRPWEKFDFEQVRKSPKPISLLLSTRRRKRNKGWSKDEGTEAEIRKVMNGDYQTSYIEVKRGSKTGEKSAWMLNLSIDVPKIDKGVDPSIIGGIDVGVKSPLVCAINNAFSRYSISDNDLFRFNKKMFARRRILLRKNRHKRAGHGARNKLKPISILTGKSERFRKKLIERWACEIADFFIKNKAGTVQMENLESMKRKEDSYFNIRLRGFWPYAEMQNKIEFKLKQYGIEIRKVAPNNTSKTCSKCGHLNNYFDFEYRKKNKFPHFKCEKCNFKENADYNAALNISNPKLKSTKEEP

SEQ ID NO: 3099 - protein, 726 aa, synthetic construct
SEVEFSHEYWMRHALTLAKRARDEREVPVGAVLVLNNRVIGGGWNRAIGLHDPTAHAEIMALRQGGLVMQNCRLVDATLYVTFEPCVMCAGAMIHSRIGRVVFGVRNSKRGAAGSLMNVLNYPGMNHRVEITEGILADECAALLCDFYRMPRRVFNAQKKAQSNINPGGSYGGSGGSETPGTSESATPKSSGGSSGGSAKNTITKTLKLRIVRPYNSAEVEKLVADEKNNREKIALEKNKGKVKEACSRHLEVAAYCTTQVERNACLFCKARKLDDKFYQKLRGQFPDAVFWQELGEIFRQLQKQAAEIYNQSLIELYYEIFIKGKGFANASSVEHYLSDVCYTRAAELFKNAAIASGLRGKVKSNFRLKELKNMKSGLPTTKSDNFPIPLVKQKGGQYTGFEISSHNDDFIIKIPFGRWQVRKEIDKYRPWEKFNFEQVRKSPKPISLLLSTQRRKRNKGWSKDEGTEAEIRKVMNGDYQTSYIEVKRGSKIGEKSAWMLSLSIDVPKIDKGVDPSIIGGIDVGVKSPLVCAINNAFNRYSISDNNLFHFNKKMFARRRILLKKNRHKRAGHGAKNRLKPISILTEKSERFRKKLIERWACEIADFFIRNKVGTVQMENLEGMKRKEDSYFNIRLRGFWPYAEMQNKIEFKLKQYGIEVRKVAPNNTSKTCSKCGHLNNYFNFEYRKKNKFPHFKCEKCNFKENADYNAALNISNPKLKSTKEEP

SEQ ID NO: 3100 - protein, 725 aa, synthetic construct
SEGEFSHEYWMRHALTLAKRARDGREVPVGAVLVLNNRVIGEGWNRAIGLHDPTAHAEIMALRQGGLVMQNYRLIDATLYVTFEPCVMCAGAMVHSRIGRVVFGVRNSKRGAAGSLMNVLDYPGMGHRVEITEGILADECAALLCDFYCMPRQVFNAQKRAQSSINSGGSSDGSSGSETPGTSSATPESSGGSSGGSAKNTITKTLKLRIVRPYNSAEVEKIVADEKNNREKIALEKNKDKVKEACSKHLKVASYCTTQVERNACPFCKARKLDDKFYQKLRGQFPDAVFWQELGEILRQLQKQAAEIYNQSLIELYYEIFIKGRGFANASSVEHYLSDVCYTRAAGLFKNAAIASGLRGKVKSNFRLKELKNMKSGLPTTKSDNFPIPLVKQKGGQYTGFEISSHNSDFIIKIPFGRWQVKEEIDKYRPWEKFDFEQVRKSPKPISLLLSTQRRQKNKGWSKDEGTEAEIRRVMNGDYQTSYIEVKRGSKIGEKSTWMLNLSIDVPKIDKGVDPSIVGGIDVGVKSPLVCAINNSFSRYSICDNDLFRFNKKMFARRRILLKKNRHKRAGHGAKNKLKPITILTKKSERFRKKLIERWVCEVADFFIKNKVGTVQMENLESMKRKEDSYFNIRLRGFWPYAEMQNRIELKLKQYGIEIRRVAPNNTSRTCSKCGHLNNYFNFEYRKKNKFPHFKCEKCNFREDADYNAALNISNPKLKSTKEEP

SEQ ID NO: 3101 - protein, 726 aa, synthetic construct
SEVEFSHEYWMRHALTLAERARDAREVPVGAILVLNNRVIGEGWNRAIGQHDPTAHAEIMALRQGGLVMQNYRLIDATLYVTFEPCVMCAGAMIHSRIGRVVFGVRNSKHGAAGSLMNVLNYPGMNHRVEITEGILADECAGLLCDFYRMPRQVFSARKKAQSSTNPGGSSGGSSGGKAPGTSESATLESSGGSSGGSAKNSITKALKLRIVRPYNSAEVEKIVADEKNNREKTALEKNKGKVKEACSKHLKVATYCTTQVERNACLFCKARKLDNKFYQKLRGQFPDAVFWQEIGEIFRQLQKQAAEIYNQSLIELYYEIFIEGKGSANARSVEHYLSDVCYTRAAELFKNAAIASGLRGKVKGNFRLKELKSMKSGLPTTKSDNFPIPLVKQKGGQYTGFEISSHNDDFIIKIPFGRWQVKKEIDKYRPWEKFDFEQVRKSPKPISLLLSTQRRKRNKGWSKDEGTEAEIRKVMNGDYQTSYIEVKRGSKIGEKSAWMLNLSIDVPKIDKGVDPSIIGGIDVGVKSPLVCAINNAFSRYSISDNDLFRFNKKMFARRRILLKKNRHKRAGHGAKNKLKPISILTGKSERFRKKLIERWACEIADFFIKNKVGTVQMENLESMKRKEDSYFNIRLRGFWPYAEMQNKIEFKLKQYGIEVRKVAPNNTSKTCSKCGHLNNYFNFEYRKKNKFPHFKCEKCNFKENADYNAALNISNPKLKSTKEKP

SEQ ID NO: 3102 - protein, 725 aa, synthetic construct
SEVEFSHEYWMRHALTLAKRARDEREVPVGAVLVLNNRVIGEGWNRAIGLHDPTAHAEIMALRQGGLVMQNYRLVDATLYVTFEPCVLCAGAMVHSRIGRVVFGVRNSKRGAAGSLMNVLDYPGMNHRVEITEGILADECAALLCDFYRMPRQVFNAQKKARPNINSGGSSGGRSGSETPGTSESATPESSGSSSGGSAKNTITKTLKLRIVRPYNSAEVEKIVADEKNNREKVALEKNKDRVREACSEHLRVAAYCTTQVERNACLFCKARKLDDKFYQKLRGQFPDAVFWQEISEIFRQLQKQAAEVYNQSLIELYYEIFIKGKGFANASSVEHYLSDVCYTRAAELFKNAAIASGLRGKVKSNFRLKELKNMKSGLPTTKGDNFPIPLVKQKGGQYTGFEISSHNDDFIIKIPFGRWVKKEIDKYRPWEKFDFEQVRKSPKPISLLLSTLRRKRNKGWSKDEGTEAEIRKVMNGDYQTSYIEVKRGRKIGEKSAWMLNLSIDVPKVDKGVDPSTIGGIDVGVKSPLVCAINNAFSRYSISDNDLFRFNKKMFARRRILLKKNKHKRAGHGAKNKLKPITILTEKSGRFRKKLIERWACEIADFFIKNRVGTVQMENLESMKRKEDSYFNIRLRGFWPYAEMQNKIEFKLKQYGIEIRKVAPNNTSKTCSKCGHLNNYFNFEYRRKNKFPHFKCEKCNFKEDADYNAALNISNPKLKSTKERP

SEQ ID NO: 3103 - protein, 726 aa, synthetic construct; identical to SEQ ID NO: 684

SEQ ID NO: 3104 - protein, 726 aa, synthetic construct
SEVEFSHEYWMRHALTLAKRARDEREVPVGAILVLNNRVIGEGWNRAIGLHDPTAHAEIMALRQGGLVMQNYRLIDATLYVTFEPCVMCAGAMIHSRIGRVVFGVRNSKHGAAGSLVNVLNYPGMNHRVEITEGILADECAALLCDFYRMPRQVLSARRKTQSSINPGGSSGGSSGSETPGTSESPTPESPGGSSGGSAKNTITKTLKLRIVRPYNSAVVEKIVADEKNNREKIALEKNRDKVKEACSKHLKVAAYCTTQVERNACLFCKVRKLDDKFYQKLRGQFPDAVFWQEIGEIFRQLQKQAAEIYNQSLIELYYEIFIKGRGFANASSVEHYLSDVCYTRAAKLFKNAAIASGLRGKVKSNFRLKELKNMKSGLPTTKSDNFPIPLVKQKGGQYTGFEISSHNDDFIIKIPFGRWQVKKEINKHRPWEKFDFEQVRKSPKPISLLLSTQRRKRNKGWSKDEGTEAEIRKVMNGDYQTSYIEVKRGSKIGEKSAWMLNLSIDVPKIDKGVDPSIIGGIDVGVKSPLVCAINNALSRYSISDNDLFHFNKKMFARRRILLRKNRHKRAGHGARSKLKPITVLTEKSERFRKKLIERWACEIANFFIKNKVGTVQMENLESMKRREDSYFNTRLRGFWPYAEMQNKIEFKLKQYGIEIRKVAPNNTSKTCSKCGHLNNYFNFEYRKKNKFPHFKCEKCNFKENADYNAALNISNPRLKSTKEEP

SEQ ID NO: 3105 - protein, 726 aa, synthetic construct
SEVEFSHEYWMRHALTLARRARDEREVPVGAILVLNNRVIGEGWNRAIGLHDPTAHAEIMALRQGGLVMQNYRLVDATLYVTFEPCVMCAGAMIHSRIGRVVFGVRNNKHGAAGSLMNVLNYPGMNHRVEITEGILADECAALLCDFYRMPRQVFSARKKAQSSINPGGPSGGSSGSKTPGTSESATPEGSGGGSSGSAKNTITKTLQLRIVRPYNSAEVEKIVADEKNNREKIALEKNKDKVREACNKHLRVASYCTTQVERSACPFCKARKLDDKFYQKLRGQFPDAVFWQELGEILRQLQKQAAEIYNQSLIELYYEIFIKGRGFANASSVEHYLSDVCYTRAAELFKNAAIASGLRGKVKGNFRLKELKNMKSGLPTTKSDNFPIPLVKQKGGQYTGFEISSHNDDFIIKIPFGRWQVKKEIDKYRPWEKFDFEQVRKSPKPISLLLSTQRRKRNKGWSKDEGTEAEVRKVMNGDYQTSYIEVKRGSRTGEKSAWMLNLSIDVPKIDKGVDPSIIGGIDVGVKSPLVCAINNAFSRYSISDNDLFRFNKKMFARRRILLKKNRHKRAGHGAKNKLKPISILTGKSERFRKKLIERWACEIADFFTKNKVGTVQMENLESMKRKEDSYFNIRLRGFWPYAEMQNKIEFKLKQYGIEIRKVAPNYTSKTCSKCGHLNNYFNFEYRKRNKFPHFKCEKCNFKENADYNAALNISNPKLKSAKEEP

SEQ ID NO: 3106 - protein, 726 aa, synthetic construct
SEVEFSHEYWMRRALTLAKRARDEREVPVGAVLVLNNRVIGEGWNRTTGLHDPTAHAEIMALRQGGLVMQNHRLVDATLYVTFEPCVMCAGAMIHSRIGRVVFGVRNSKRGAAGSLTNVLNYPGMSHRVEITEGILADECAALLCDFYRMPRQVFNAQKKAQSNINPGGSSGGSSGSETPSTSESATPGSSGGSSGGSAKNTITKTLKLRIVRPYNSAEVEKIVADEKNNREKIALEKNKDKVKEACSEHLKVATYCTTQVERNACLFCKARKLDDKFYQKLRGQFPDAVFWQELGEILRQLQKQAAEIYNQSLVELYYEILIKGKGIANASSVEHYLSDVCYTRAAELFKNAAIASGLRNKIKSNFRLKELRNMKSGLPTTKSDNFPIPLVRQKGGQYTGFEISNHNGDFIIKIPFGRWQVKKEINKHRPWEKFDFEQVRKSPKPISLLLSTQRRKRNKGWSKDEGTEAEVRKVMNGDYQTSYIEVKRGSKIGEKSAWMLNLSIDVPKIDKGVDPGIIGGIDVGVKSPLVCAINNSSSRYSICDNDLFRFNKKMFARRRILLKKNRHKRAGHGAKNKLKPITILTKKSERFRKKLIERWVCEVADFFIKNKVGTVQMENLESMKRKEDSYFNIRLRGFWPYAEMQNRIELKLKQYGIEIRRVAPNNTSRTCSKCGHLNNYFNFEYRKKSKFPHFKCEKCNFREDADYNAALNISNPKLKSTKEEP

SEQ ID NO: 3107 - protein, 726 aa, synthetic construct
SEDEFSHEYWMRHALTLAKRARDGREVPVGAVLVLNNRVIGEGWNRAIGLHDPTAHAETMALRQGGLVMQNYRLIDATLYVTFEPCVMCAGAMVHSRIGRVVFGVRNNKRGAAGSLMNVLDYPGMGHRVEITEGILADECAALLCDFYCMPRQVFNAQKRAQSSINSGGSSGGSSGSETPGTSESATPESSGGGSSGSAKNTITKTLQLRIVRPYNSAEVEKIVADEKNNREKIALEKNKDKVKEACSKHLKVASYCTTQVERNACPFCKARKLDDKFYQKLRGQFPDAVFWQELGEILRQLQKQAAEIYNQSLIELYYEIFIKGRGFANASSVEHYLSDVCYTRAAELFKNAAIASGLRNKIKSNFRLKELRNMRSGLPTTKSDNFPIPLVRQKGGQYTGFEISNHDGDFIIKIPFGRWQVKKEINKHRPWEKFDFEQVRKGPKPISLLLSTQRRKRNRGWSKDEGTEAEIRKVMNGDYQTSYIEVKRGSKIGEKSAWMLNLSIDVPKIDKGVDPSIIGGIDVGVKSPLVCAINNAFSRYSISDNDLFRFNKKMFARRRILLGKNRHKRAGHGVKNKLKPITILTEKSGRFRKKLIERWACEIADFFVKNKVGTVQMENLESMKRKEDSYFNIRLRGFWPYAEMQNKIEFKLKQYGIKVRKVAPNNTSKTCSKCGHLNNYFSFEYRKKNKFPHFKCEKCNFKEDADYNAALNISNPKLKSTKEEP

SEQ ID NO: 3108 - protein, 726 aa, synthetic construct
SEVEFSHEYWMRHALILAKRARDEREVPVGAVLVLNNRVIGVGWNRAIGLHDPTAHAEIMALRQGGLVMQNYRLIDATLYVTFEPCVMCAGAMVHSRIGRVVFGVRNSKRGAAGSLMNVLNYPGMGHRVEITEGILADECAALLCDFYRMPRQVFNARKKAQSSINPGGSSGGSSGSETPGASGSVIPRSSGGSSAGSTKDTITKTLKLRIVRPYNSAEVEKVVADEKNNREKIAMEKNKDKVREACSKHLKVASYCTTQVERNACLFCKARKLDDKFYQKLRGQFPDAVFWQELGGIFRQLQKQAAEIYNQSLIELYYEIFIKGKGITNASRVEHYLSDVCYTRAAELFKNAAIASGLRSKVRSNFRLKELKNMKSGLPTTKSDNFPIPLVKQKGGQYTGFEISNHNDDFIIKIPFGRWQVKKEIDKYRPWEKFDFEQVRKSPKPISLLLSTQRRKRNKGWSKDEGTEAEIRKVMNGDYQTSYIEVRRGSKIGEKNAWMLNLSIDVPKIDKGVDPSIIGGIDVGVKSPLVCAINNAFSKYSISDNDLFRFNKKMFARRRILLGKNRHKRAGHGVKNKLKPITILTEKSGRFRKKLIERWACEIADFFVKNKVGTVQMENLESMKRREDSYFNIRLRGFWPYAKMQNKIEFKLKQYGIEIRKVAPNNTSKTCSKCGHLNNYFSFEYRKKNKFPHFKCEKCNFKENADYNAALNISNPKLKSTKEEP

SEQ ID NO: 3109 - protein, 726 aa, synthetic construct
SEVEFSHEYWMRHALTLAKRARDEREVPVGAILVLNNRVIGEGWNRAIGLHDPTAHAEIMAMRQGGLVLQNYRLIDATLYVTFEPCVMCAGAMIHSRIGRVVFGVRNNKHGAAGSLVNVLNYPGMNHRVEITEGILADECAALLCDFYRMPRQVFNARKKAQSSINPGGSSGGSSGSETPGTSESATPVSSGGSSGSSAKNTITKTLKLRIVRPYNSAEVEKIVADEKNNREKIALEKNKDKVKEACSKHLKVAAYCTTQVERNACLFCKARRLDDKFYQKLRGQFPDAVFWQEIGEIFRQLQKQAAEVYNQSLVELYYEILIKGKGIANASSVEHYLSDVCYTRAAELFKNAAIASGLRNKIKSNFRLKELRNMKSGLPTTKSDNFPIPLVRQKGGQYTGFEISNHDGDFIIKIPFGRWQVKKEINKHRPWEKFDFEQVRKSPKPISLLLSTQRRKRNKGWSKDEGTEAEIRKVMNGDYQTSYIEVKRGSKIGEKSAWMLNLSIDVPKIDKGVDPSIIGGIDVGVKSPLVCAINNALSRYSISDNDLFHFNKKMFARRRILLRKNRHKRAGHGAKNKLKPISILTEKSKRFRKKLIERWACEIADFFIKNKVGTVQMENLERMKRKEDGYFNIRLRGFWPYAEMQNKIEFKLKQYGIEIRKVAPNNTSKTCSKCGHLNNYFNFEYRKTNKFPHFKCEKCNFKEDADYNAALNISNPKLKSTKEEP

SEQ ID NO: 3110 - protein, 726 aa, synthetic construct
SEVEFSHEYWMRRALTLAKRARDEREVPVGAVLVLNNRVIGVGWNRAVGLHDPTAHAEIMALRQGGLVMQNYRLIEATLYVTFEPCIMCAGAMIHSRISRVVFGVRNSKRGAAGSLMNVLNYPGMNHRVEITEGILADECAALLCDFYRMPRQVFSARKKAQSSINSGGSSGGNSGSKTPGTSESATPESSGGSSGGSAKNTITKTLKLRIVRPYNSAEVEKIVADEKNNREKIALEKNKDKVKEACSKHLKVAAYCTTQVERNACQFCKARKLDDKFYQKLRGQFPDAVFWQEIGEIFRQLQKQAAEIYNQSLIELYYEIFIKGKGFANASSVEHYLSDVCYTRAAELFKNAAIASGLRGKVKSSFRLKELKNMKSGLPTTKSDNFPIPLVRQKGGQYTGFEISNHDGDFIIKIPFGRWQVKKEISKHRPWEKFDFEQVRKSPKPISLLLSTQRRKRNKGWGKDEGTEAEIRKVMNGDYQTSYIEVKRGSKIGEKSAWMLNLSIDVPKIDKGVDPSIIGGIDVGVKSPLVCAINNAFSRYSISDNDLFHFNKKMFARRRILLKKNRHKRAGHGAKNKLKPISILTEKSKRFRKKLIERWACEIANFFIKNKVGTVQMENLEGMKRKEDSYFNIRLRGLWPYAEMQNKIEFKLKQYGIEIRKVAPNNTSKTCSKCGHLNNYFNFEYRRKNKFPHFKCEKCNFKENADYNAALNISNPKLKSTKEEP

SEQ ID NO: 3111 - protein, 726 aa, synthetic construct
SEVEFSHEYWMRHALTLAKRARDGREVPVGAVLVLNNRVIGEGWNRAIGLHDPTAHAEIMALRQGGLVMQNYRLVDATLYVTFEPCVMCAGAMVHSRIGRVVFGVRNSKRGAAGSLMNVLDYPGMGHRVEITEGILADECAALLCDFYCMPRQVFNAQKRAQSSINSGGSSGGSSGSDTPGTSESATPESSGGGSSGSAKNTITKTLQLRIVRPYNSAEVEKIVADEKNNREKIALEKNKDKVREACSKHLKVAAYCTTQVERNACLFCKARKLDDKFYQKLRGQFPDAVFWQELGEILRQLQKQAAEIYNQSLIELYYEIFIKGRGFANASSVEHYLSDVCYTRAADLFKNAAIASGLRGKVKSNFRLKELKNMRSGLPTAKSDNFPIPLVKQKGGQYTGFEISSHNDDFIIKIPFGRWQVKKEIDKYRPWEKFDFEQVRKSPKPISLLLSTQRRKRNKGWSKDEGTEAEIRKVMNGDYQTSYIEVKRGSKTGEKSAWMLNLSIDVPKIDKGVDPCIIGGIDVGVKSPLVCAINNAFSRYSISDNDLFHFNKKMFARRRILLKENGHKRAGHGAKNKLKPITIMTEKSKRFRKKLIERWACEIADFFIKNKVGTVQMENLESMKRKEDSYFNIRLRGFWPYAEMQNKIEFKLKQYGIVVRKVAPNNTSKTCSECGHLNNYFNFEYRKMNKFPHFKCEKCNFKEDADYNAALNISNPKLKSTKEEP

SEQ ID NO: 3112 - protein, 726 aa, synthetic construct
SEVEFSHEYWMRHALTLAKRARDEREVPVGAVLVLNNRVIGGGWNRAIGLHDPTAHAEIMALRQGGLVTQNYRLIDATLYVTFEPCVMCAGAMIHSRIGRVVFGVRNNKHGAAGSLVNVLNYPGMNHRVEITEGILADECAALLCDFYRMPRQVFNARKKAQSSINPGGSSGGSGGSETPGTSESPTPESSGGSSGGSAKNTITKTLKLRIVRPYNSAEVEKIVAEEKDNREKIALETNKDKVREACSKHLKVAAYCTTQVERNACLFCKARRLDDKFYQKLRGQFPDAVFWQEIGEIFRQLQKQAAEVYNQSLVELYYEILIKGKGIANASSVEHYLSDVCYTRAAELFKNAAIASGLRNKIKSNFRLKELKNMKSGLPTTKSDNFPIPLVKQKGGQYTGFEISSHNSDFIIKIPFGRWQVKEEIDKYRPWEKFDFEQVRKSPKPISLLLSTQRRKKNKGWSKDEGTEAEIRRVMNGDYQTSYIEVKRGSKIGEKSAWMLNLSIDVPTIDKGVDPSIIGGIDVGVKSPLVCAINNSSSRYSICDNDLFRFNKKMFARRRILLKKNRHKRAGHGTKNKLKPITILTKKSERFRKKLIERWVCEVADFFIKNKVGTVQMENLESMKRKEDSYFNIRLRGFWPYAEMQNRIELKLKQYGIEIRRVAPNNTSRTCSKCGHLNNYFNFEYRKKNKFPHFKCEKCNFREDADYNAALNISNPKLKSTKEEP

SEQ ID NO: 3113 - protein, 726 aa, synthetic construct
SEVEFSHEYWMRHALTLAKRARDEREVPVGAVLVLNNRVIGEGWNRTTGLHDPTAHAEIMALRQGGLVMQNHRLVDATLYVTFEPCVMCAGAMIHSRIGRVVFGVRNSKRGAAGSLTNVLNYPGMNHRVEITEGILVDECAALLCDFYRMPRQVFNAQKRAQSTINTGGSSGSSSGSETPGTSESPTPESSGGSPGGSAKNTITKTLKLRIVRPYNSAEVEKIVADEKNNRERIALEKNKDKVKEACSKHLKVASYCTTQVERNACLFCKARKLDDKFYQKLRGQFPDAVFWQELGEIFRQLQKQAAEIYNQSLIELYYEIFIKGKGFANASSVEHYLSDVCYTRAAELFKNAAIASGLRGKVKSNFRLKELKNMKSGLPTTKSDNFPIPLVKQKGGQYTGFEVSSHNDDFIIKIPFGRWQVRKEIDKYRPWEKFNFEQVRKSPKPISLLLSTQRRKRNKGWSKDEGTEAEIRKVMNGDYQTSYIEVKRGSKIGEKSAWMLSLSIDVPKIDKGVDPSIIGGIDVGVKSPLVCAINNAFNRYSISDNSLFHFNKKMFARRRILLKKNRHKRAGHGAKNKLKPISILTERSERFRKKLIERWACEIASFFIKNKVGTVQMENLESMKRREDSYFNIRLRGFWPYAEMQNKIVFKLKQYGIEIRKVAPNNTSKTCSKCGHLNNYFNFEYRKMNKFPHFKCEKCNFKENADYNAALNISNPKLKSTKEEP

SEQ ID NO: 3114 - protein, 726 aa, synthetic construct; identical to SEQ ID NO: 3029

SEQ ID NO: 3115 - protein, 726 aa, synthetic construct
SEVEFSHEYWMRHALILAKRARDEREVPVGAVLVLNNRVIGVGWNRAIGLHDPTAHAEIMALRQGGLVMQNYRLIGATLYVTFEPCAMCAGAMVHSRIGRVVFGVRNSKRGAAGSLMNVLNYPGMDHRVEITGGILADECAALLCDFYRMPRRVFDAQKKAQSSINSGGSSGGSSGSVTPGTSESATPESSGGGFGSSAKNTITKTLQLRIVRPYNSAEVEKIVADEKNNREKIALEKNKDKVQEACSKHLKVASYCTTQVERNACLFCKARKLDDKFYQKLRGQFPDAVFWQELGEIFRQLQKQAAEIYNQSLIELYYKIFIKGKGLANASNVEHYLSDVCYTRAAELFKNAAIASGLRGKVKSNFRLKELKNMKSGLPTTKSDNFPIPLVKQKGGQYTGFEISNHNSDFIIKIPFGRWQAKKEIDKYRPWEKFDFEQVRKSPKPVSLLLSTQRRKKNRGWSKDEGTEAEIKKVMNGDYQTSYIEVKRGSKIGEKSAWMLSLSIDVPKIDKGVDPSIIGGIDVGVKSPLVCAINNALSRYSISDNDLFHFNKKLFARRRILLGKNRHKRAGHGVKNKLKPITILTEKSGRFRKKLIERWACEIADFFVKNKVGTVQMENLESMKRKEDSYFNIRLRGFWPYAEMQNKIEFKLEQYGIEVRKVAPDNTSKTCSKCGHLNNYFNFEYRRKNKFPHFKCEKCNFKEDADYNAALNISNPKLKSTKEEP

SEQ ID NO: 3116 - protein, 726 aa, synthetic construct
SEVEFSHEYWMRHALTLAKRARDEREVPVGAVLVLDNRVIGEGWNRAIGLHDPTAHAEIMALRQGGLVMQNYRLIDATLYVTFEPCVMCAGAMVHSRIGRVVFGVRNNKRGAAGSLMNVLDYPGMDHRVEITEGILADECAALLCDFYRMPRQVFNAQRKAQSSINSGGSSGGSSGSETPGTSESATPESSGGSSGGSAKNTITKTLQLRIVRPYNSAEVEKIVADEKNNREKIALEKNKDKVKEACSKHLKVAAYCTTQVERNACLFCKARKLDDKFYQELRGQFPDAVFWQEIGEIFRQLQKQAAEIYNQSLIELYYEIFIKGKGIANASSVGHYLSDVCYTRAAELFKNAAIASGLRSKIKSNFRLKELKSMKSGLPSTKSDNFPIPLVKQKGGQYTGFEISSHNDDLIIKIPFGRWQVKKEIDKYRPWEKFDFEQVRKSPKPISLLLSTQRRKRNKGWGKDEGTEAEIRKVMNGDYQTSYIEVKRGSKIGEKSAWMLNLSIDVPKIDKGVDPSIIGGIDVGVKSPLVCAINNAFSRYSISDNDLFHFNKKMFARRRILLRKNRHKRAGHGAKNKLKPISVLAEKSGRFRKKLIERWACEIADFFIKNKVGTVQMENLGSMKRKEDSYFNIRLRGFWPYAEMQNKIEFKLKQYGIEIRKVAPDNTSKTCSKCGHLNNYFNFEYRKKNKFPHFKCEKCNFKEDADYNAALNISNPKLKSTKEEP

SEQ ID NO: 3117 - protein, 726 aa, synthetic construct
SEVEFSHEYWMRHALTLAKRARDEREVPVGAILVLNNRVIGEGWNRAIGLHDPTAHAEIMALRQGGLVMQNYRLIDATLYVTFEPCVMCAGAMIHSRIGRVVFGVRNNKHGAAGSLVNVLDYPGMNHRVEITEGILADECAALLCDFYRMPRQVFNARKKAQSSISPGGSSGGSSGSETPGTSESATPESSGGSSGGSAKNTITKTLKLRIVRPYNSAEVEKVVADEKNNRERIALEKNKDKVKEACSKHLKVAAYCTTQVERNACLFCKARKLDDKFYQKLRGQFPDAVFWQEIGEIFRQLQKQAAEIYNQSLIELYYEIFIKGKGFANASSVEHYLSDVCYTRAAELFKNAAIASGLRGKVKSNFRLKELKNMKSGLPTTKSDNFPIPLVKQKGGQYTGFEISSHNDDFIIKIPFGKWQAKKEINKHRPWEKFDFEQVRKSPKPISLLLSTQRRKKNKGWSKDEGTEAEIRRVMNGDYQTSYIEVKRGSKIGEKSAWMLNLSIDVPKIDKGVNPSIIGGIDVGVKSPLVCAINNSSSRYSICDNDLFRFNKKMFARRRILLKKNRHKRAGHGAKNKLKPITILTKKSERFRKKLIERWVCEVADFFIKNKVGTVQIENLESMKRKEDSYFNIRLRGFWPYAEMQNRIEFKLKQYGIEIRKVAPNNTSKTCSKCGHLNNYFNFEYRKKNKFPHFKCEKCNFKENADYNAALNICNPKLKGTREEP

SEQ ID NO: 3118 - protein, 726 aa, synthetic construct
SEDEFSHEYWMRHALTLAKRARDEREVPVGAVLVLNNRVIGEGWNRAIGLHDPTAHAEIMALHQGGLVMQNYRLIDATLYVTFEPCVMCAGAMIHSRIGRVVFGARNSKRGAAGSLMNVLSYPGMNHRVKITEGILVDECAALLCDFYRMPRQVLSAQKKAQSSVSSGGSSGGSSGSETPSASGSVTPKSSVGSSAGSTKNTITKTLKLRIVRPYNSAEVEKIVADEKNNREKIALEKNRDKVKEACSKHLKVAAYCTTQVERNACLFCKARKLDDKFYQKLRGQFPDAVFWQEIGEIFRQLQKQSAEIYNQSLIELYYEIFIKGKGFANTSSVEHYLSDVCYTRAAELFKNAAIASGLRGKVKSNFRLKELKNMNSGLPTTKSDNFPIPLVKQKGGQYTGFEISNHNDDFIIKIPFGRWQVKKEIDKYRPWEKFDFEQVRKSPKPISLLLSTQRRKRNKGWSKDEGTEAEIRKVMNGDYQTSYIEVKRGSKIGEKSAWMLNLSIDVPKIDKGVDPSIIGGIDVGVKSPLVCAINNAFSRYSISDNDLFRFNKKMFARRRILLKKNRHKRAGHGARNKLKPITVLTEKSKRFRKKLIERWACEIANFFVKNKVGTVQMENLESMKRKEDSYFNIRLRGLWPYAEMQNKIEFKLKQYGIEVRKVAPNNTSKTCSKCGHLNNYFNFEYRKKNKFPHFKCEKCNFKENADYNAALNISNPKLKSTKEEP

SEQ ID NO: 3119 - protein, 726 aa, synthetic construct
SEVEFSHEYWMRHALTLAKRARDGREVPVGAILVLNNRVIGEGWNRAIGLHDPTAHAEIMALRQGGLVMQNYRLIDATLYVTFEPCVMCAGAMIHSRIGRVVFGVRNSKHGAAGSLVNVLNYPGMNHRVEITEGILADECAALLCDFYCMPRQVFNAQKRAQSGINSGGSSGGSSGSETPGTSESATPESSGGGSSGSAKNTITKTLQLRIVRPYNSAEVEKIVADEKNNREKIALEKNKDKVKEACSKHLKVASYCTTQVERNACLFCKARKLDDKFYQGLRGQFPDAVFWQELGEIFRQLQKQAAEIYNQSLIELYYEIFIKGKGFANASSVEHYLSDVCYARAAELFKNAAIASGLRGKVKSNFRLKELKNMRSGLPTTKSDNFPIPLVKQKGGQYTGFEISSHNDDFIIKIPFGRWQVKKEIDKYRHWEKFDFEQVRKSPKPISLLLSTQRRKRNKGWSKDEGTEAEIRKVMNGDYQTSYIEVKRGSKTGEKSAWMLNLSIDVPKIDKGVDPSIIGGIDVGVKSPLVCAINNAFSRYSISDNDLFRFNKKMFARRRILLKKNRHKRAGHGAKNKLKPISILTGKSERFRKKLIERWACEIADFFIKNKVGTVQMENLESMKRKEDSYFNIRLRGFWPYAEMQNKIEFKLKQYGIEIRKVAPNNTSKTCSKCGHQNNYFNFEYRRKNKFPHFKCEKCNFKENADYNAALNISNPMLKSAKEEP

SEQ ID NO: 3120 - protein, 726 aa, synthetic construct
SEVEFSHEYWMRHALTLAKRARDEREVPVGAVLVLNNRVIGEGWNRAIGLHDPTAHAEIMALRQGGLVMQNYRLIDATLYVTFEPCVMCAGAMVHSRIGRVVFGVRNSKRGAAGSLMNVLDYPGMGHRVEITEGILADECAALLCDFYCMPRQVFNAQKRAQSSINSGGSSGGSGGSETPGTSESATPESSGGGSSGSAKNTITKTLQLRIVRPYNSAEVEKIVADEKNNREKIALEKNKDKVKEACSRHLKVASYCTTQVERNACPFCKARKLDDKFYQKLRGQFPDAVFWQELGEILRQLQKQAAEIYNQSLIELYYEIFIKGRGFANAGSVEHYLSDVCYTRAAGLFKNAAIASGLRGKVKSNFRLKELRNMKSGLPTTKSDNFPIPLVKQKGGQCTGFEISNHNSDFIIKIPFGRWQVKEEIDKYRPWEKFDFEQVRKNPKPISLLLSTQRRKRSKGWSKDEGTEAEIRKVMNGDYQTSYIEVKRGSKIGEKSAWMLNLSIDVPKIDKGVDPSIIGGIDVGVKSPLVCAINNAFSRYSISDNDLFRFNKKVFARRRILLKKNRHKRAGHGTKNKLKPITILTEKSGRFRKKLIERWACEIANFFIKNKVGTVQMENLESMKRKEDSYFNIRLRGFWPYAEMQNKIEFKLKRYGIEIRKVAPNNTSKTCSKCGHLNNYFNFEYRKRNKFPHFKCEKCNFKENADYNAALNISDPKLKGTKEEP

SEQ ID NO: 3121 - protein, 726 aa, synthetic construct
SEDEFSHEYWMRHALTLAKRARDGREVPVGAVLVLNNRVIGEGWNRAIGLHDPTAHAEIMALRQGGLVMQNYRLIDATLYVTFEPCVMCAGAMVHSRIGRVVFGVRNSKRGAAGSLMNVLNYPGMGHRVEITEGILADECAALLCDFYCMPRQVFNAQKRAQFSINSGGSSGGSSGSETPGSSESATPESSGGGSSGSAKNTITKALQLRIVRPYNSAEVEKIVADEKNNREKIALEKNKDKVKEACSKHLKVASYCTTQVERNACPFCKARKLDDKFYQKLRGQFPDAVFWQELGEILRQLQKQAAEIYNQSLIELYYEIFIKGRGFANAGSVEHYLSDVCYTRAAELFKNAAIASGLRGKVKSNFRLKELKNMKSGLPTTKSDNFPIPLVKQKGGQYTGFEISSHNDDFIIKIPFGRWQVKKEIDKYRPWEKFDFEQVRKSPKPISLLLSTQRRKRNKGWSKDEGTEAEIRKVMNGDYQTSYIEVKRGSKTGEKSAWMLNLSIDVPKIDKGVDPSIIGGIDVGVKSPLVCAINNAFSRYSISDNDLFRFNKKMFARRRILLKKNRHKRAGHGAKNKLKPISILTGKSERFRKKLIERWACEITDFFIKNKVGTVQMENLESMKRKEDSYFNIRLRGFWPYAEMQNKIEFKLKQYGIEIRRVAPNNTSKTCSKCGHLNNYFNFEYRKKNKFPHFKCEKCNFKENADYNAALNISNPELKSTKEEP

SEQ ID NO: 3122 - protein, 726 aa, synthetic construct
SEVEFSHEYWMRHALTLAKRARDEREVPVGAILVLNNRVIGEGWNRAIGLHDPTAHAEIMALRQGGLVMQHYRLIDATLYVTFEPCVMCAGAMIHSRIGRVVFGVRNNKHGAAGSLVNVLNYPGMNHRVEITEGILANECAALLCDFYRMPRQVFNARKKAQSSINPGGSSGGSSGSETPGTSESATPESSGGSSGGSAKNTITKTLKLRIVRPYNSAEVEKIVADEKNNREKIALEENKDKVKEACSKHLKVAAYCTTQVERNACLFCKARRLDDKFYQKLRGQFPDAVFWQEIGEIFRQLQKQAAEIYNQSLVELYYEIFIKGKGIANASSVEHYLSDVCYTRAAELFKNAAIASGLRNKIKSNFRLKELRNMRSGLPTTKSDNFPIPLVRQKGGQYTGFEISNHDGDFIIKIPFGRWQVKKEINKHRPWEKFDFEQVRKSPKPISLLLSTQRRKRNKGWSKDEGTEAEIRKVMNGDYQTSYIEVKRGSKIGEKSAWMLNLSIDVPKIDKGVDPSIIGGIDVGVKSPLVCAINNALGRYSISDNDLFHFNKKMFARRRILLKKNRHKRAGHGAKNKLKPITILTKKSERFRKKLIERWVCEVADFFIKNKVGTVQMENLEGMKRKEDSYFNIRLRGFWPYAEMQNKIEFKLKQYGIEIRKVAPNNTSKTCSKCGHLNNYFNFEYRKKNKFPHFKCEKCNFKENADYNAALNISNPKLKSTKEEP

SEQ ID NO: 3123 - protein, 726 aa, synthetic construct
SEVEFSHEYWMRHALTLAKRARDEREVPVGAILVLNNRVIGEGWNRAIGLHDPTAHAEIMALRQGGLVMQNYRLIDATLYVTFEPCVMCAGAMVHSRIGRVVFGVRNSKRGAAGSLMNVLDYPGMNHRVEITEGILTDECAALLCDFYRMPHQVLNAQKKAQSSINSGGSAGGSGGSETPGTSGSTTPVSSGGSSGGSAKNTITKALKLRIVRPYNSAEVEKIVADEKNNREKIALEKNKDKVKEACSKHLKVAAYCTTQVERNACLFCKARKLDDKFYQKLRGQFPDAVFWQEIGEIFRQLQRQAAEIYNQSLIELYYEILIKGKGFANASSVEHYLSDVCYTRAAELFKNAAIASGLRGKVKSNFRLKELKNMKSGLPTTKSDNFPVPLVKQKGGQYTGFEISSHNDDFIIKIPFGRWQVKKEIDKYRPWEKFDFEQVRKSPKPISLLLSTQRRKRNKGWSKDEGTEAEIRKVMNGDYQTSYIEVKRGSKTGEKSAWMLNLSIDVPKIDKGVDPSIIGGIDVGVKSPLVCAINNAFSRYSISDNDLFRFNKKMFARRRILLKKNRHKRAGHGAKNKLKPISILTGKSERFRKKLIERWACEIADFFIKNKVGTVQMENLESMKRKEDSYFNIRLRGFWPYAEMQNKIEFKLKQYGIEIRKVAPNNTSKTCSKCGHLNNYFNFEYRKKNKFPHFKCEKCNFKENADYNAALNISNPKLKSTREEP

SEQ ID NO: 3124 - protein, 726 aa, synthetic construct
SEVEFSHEYWMRHAMSLAKRARDEREVPVGAVLVLNNRIIGEGWNRAIGLHDPTAHAEIMALRQGGLVMQNNRLTDATLYVTFEPCVMCAGAMVHSRIGRVVFGVRNSKRGAAGSLMNVLNYPGVNHCVEITEGILVDECAALLCDFYRMPRHVLNAQKKAQSSISSGGSSGGCSGSEMPGASESVTPKSSGGSSAGSTKNTITKTLKLRIVRPYNSAEVEKIVADEKNSREKIALERNKDKVKEACSEHLKVAAYCTTQVERNACLFCKARKLDDRFYQKLRGQFPDAVFWQETGEIFRQLQRQAAEIYNQSLIELYYEIFIKGKGFANASSVEHYLSDVCYTRAAELFKNAAIASGLRGKVKSNFRLKELKNMKSGLPTTKSDNFPIPLVKQKGGQYTGFEVSSHNDDFIIKIPFGRWQVKEEIDKYRPWEKFDFEQVRKGPKPISLLLSTQRRKRNKGWSKDEGTEAEIRKVMNGDYQTSYIEVKRGSRIGEKSAWMLSLSIDVPKVDRGVDPSIIGGIDVGVKSPLVCAINNAFSRYSISDNDLFHFNKKVFARRRILLKKNRHKRAGHGVKNKLKSISILTEKSKRFRKKLIERWACEIADFFIKNKVGTVQMENLESMKRKEDSYFNIRLRGFWPYAEMQNKIEFKLKQYGIEIRKVAPNNTSKTCSKCGHLNNYFNFEYRKKNKFPHFKCEKCNFKEDADYNAALNISNPKLKSTKEEP

SEQ ID NO: 3125 - protein, 726 aa, synthetic construct
SEVEFSHEYWMRRALTLAKRARDEREVPVGAVLVLNDRVIGEGWNRAVGLHDPTAHAEIMALRQGGLVMQNHRLIEATLYVTFEPCIMCAGAMIHSRIGRVVFGVRNGKRGAAGSLMNVLNYPGMNHRVEITEGILADECAALLCDFYRMPRQVFNAQKKAQSNINPGGSSGGSSGSETPGTSESPTPESSGGSSGGSAKSTITKTLKLRIVRPYNSAEVEKIVADEKNNREKIALEKNKDKVKEACSKHLKVAAYCTTQVERNACLFCKARRLDDKFYQKLRGQFPDAVFWQEIGEIFRQLQKQAAEVYNQSLVELYYEILIKGKGIANASSVEHYLSDVCYTRAAELFKNAAIASGLRNKIKSNFRLKELRNMRSGLPTTKSDNFPIPLVRQKGGQYTGFEISNHDGDFIIKIPFGRWQVKKEIDKYRPWEKFDFEQVRKSPKPISLLLSTQRRKGNKGWSKDEGTEAEIKKVMNGDYQVSYIEVKRGSKIGEKSAWMLNLSVDVPKIDKGVDPSIIGGINVGVKSPLVCAINDALSRYSISDNDLFHFNKKMFARRRILLRKNRHKRAGHGAKNKLKPVTILTEKSERFRKKLIERWACEIANFFIKNKVGTVQMEDLESMKRKEDSYFNIRLRGFWPYAEMQNKIEFKLKQFGIEIRKVAPNDTSKTCSKCGHLNNYFNFEYRKKNKFPHFKCEKCNFKENADYNAAQNISNPQLKSTKEEP

SEQ ID NO: 3126 - protein, 726 aa, synthetic construct
SEVEFSHEYWMRHALTLAKRARDEREVPVGAILVLNNRVIGVGWNRAIGLHDPTAHAEIMALRQGGLVMQNYRLIDATLYVTFEPCVMCAGAMIHSRIGRVVFGVRNSKHGAAGSLVNVLNYPGMNHRVETTEGILADECAALLCDFYRMPRRVFNARMKAQSSINPGGSSGGSGGSETPGTSESATPESFGGSSGGSAKNTITKTLRLRIVRPYNSAEVEKIVADEKNNREKIALEKNKDKVKEACSKHLKVAAYCTTQVERNACLFCKARRLDDKFYQKLRGQFPDAVFWQEIGEIFRQLQKQAAEIYNQSLIELYYEIFIKGKGIAGASRVGHYLSDVCYTRAAELFKNAAIASGLRSKIKSNFRLKELKNMKSGLPTTKSDNFPIPLVKQKGGQYTGFEISNHNGDFIIKIPFGRWQVKKEIDKYRPWEKFDFEQVRKSPKPISLLLSTQRRKRNKGWSKDEGTEAEIRKVMNGDYQTSYIEVKRGSKIGEKSAWMLSLSIDVPKIDKGVDPSTIGGIDVGVKSPLVCAINNAFCRYSISDNDLFHFNKKMFARRRILLKKSRHKRAGHGAKNKLKPISILTEKSKRFRKKLIERWACEIADFFIKNKVGTVQMENLESLKRKEDSYFNIRLRGFWPYAEMQNKIEFKLKQYGIEIRKVAPNNTSKTCSKCGHLNNYFNFEYRKKNKFPHFKCEKCNFKENADYNAALNISNPKLKSTREEP

SEQ ID NO: 3127 - protein, 726 aa, synthetic construct
SEVEFSHEYWMRHALTLAKRARDEREVPVGAVLVLNNRVIGEGWNRAIGLHDPTAHAEIMALRQGGLVMQNYRLSDATLYVTFEPCVMCAGAMIHSRIGRVVFGVRNSKRGAAGSLMNVLNYPGMNHRVEITEGILTDECAALLCDFYRMPHQVLNAQKKAQSSINSGGSSDGSSGSVTPGTSGSATPEGSGGSSSGFAKNTITKSLKLRIVRPYNSAEVEKIVADEKNNREKVALEKSKGKVKEACSKHLKVVSYCTTQVERNACPFCKARKLDDKFYQKLRGQFPDAVFWQELGEILRQLQKQAAEIYNQSLIELYYEIFIKGRGFANASSVEHYLSDVCYTRAAELFKNAAIASGLRGKVKSNFRLKELKNMKSGLPTTKSDNFPIPLVKQKGGQYTGFEISSHNDDFIIKIPFGRWQVKKEVGKYRPWEKFDFEQVRKSPKPISLLLSTQRRKRNKGWSKDEGTEAEIRKVMNGDYQTSYIEVKRGSKIGEKSAWMLNLSIDVPKIDKGVDPSITGGIDVGVKSPLVCAINNAHSRYSVSDNDLFHFNKKMFARRRILLKKNGHKRAGHGARNKLKPITALTEKSGRFRKKLIERWACEIANFFIKNKVGTVQMENLESMKRKEDSYFNIRLRGFWPYAEMQNKIEFKLKQYGIEIRKVAPNNTSKTCSRCGHLNNYFNFEYRKKNKFPHFKCEKCNFKEDADYNAALNISNPKLKSTKEEP

SEQ ID NO: 3128 - protein, 726 aa, synthetic construct
GEDEFSHEYWMRHALTLAKRARDGREVPVGAVLVLNNRVIGEGWNRAIGLHDPTAHAEIMALRQGGLVMQNYRLIDATLYVTFEPCVMCAGAMVHSRIGRVVFGVRNSKRGAAGSLMNVLDYPGMGHRVEITEGILADECAALLCDFYCMPRQVFNAQKRAQSSISSGGSSGGSSGSETPGTSESATPESSGGGSSGSAKNTITKTLQLRIVRPYNSAEVEKIVADEKNNRERIALEKNKDKVKEACSKHLKVAAYCTTQVERNACLFCKARKLDDKFYQKLRGQFPDAVFWQETGEIFRQLQRQAAEIYNQSLIELYYEIFIKGKGFANASSVEHYLSDVCYTRAAELFKNAAIASGLRGKVKGNFRLKELKNMKSGLPTTKSDNFPIPLVKQKGGQYTGFEISSHNDDFIIKIPFGRWQARKEIDKYRPWEKFDFEQVRKSPKPISLLLSTQRRKRNKGWSKDEGTEAEIRKVMNGDYQTSYIEVKRGNKIGEKSAWMLNLSIDVPKIDKGVDPSIIGGIDVGVKSPLVCAINNAFSRYSISDNDLFHFNKKMFARRRILLKKNGHKRAGHGAKNKLKPIAIMTEKSKRFRKKLIERWACEIADFFIKNKVGTVQMEDLESMKRKEDSYFNIRLRGFWPYAEMQNKIEFKLKQYGIVVRKVAPNNTSKTCSKCGHLNNYFNFEYRKKNKFPHFKCEKCNFKEDADYNAALNISNPKLKSTKGEP

SEQ ID NO: 3129 - protein, 726 aa, synthetic construct
SEVEFSHEYWMRHALTLAKRARDEREVPVGAILVLNNRVIGEGWNRAIGLHDPTAHAEIMALRQGGLVMQNYRLIDATLYVTFEPCVMCAGAMIHSRIGRVVFGVRNNKHGAAGSLVNVLNYPGMNHRVGITEGILADECAALLCDFYRMPRQVFNARKKAQSSISPGGSSGGSSGSETPGTSESATPESSGGSSGGSAKNTITKTLKLRIVRPYNSAEVEKIVADEKNNREKIALEKNKDKVKEACSKHLKVAAYCTTQVERNACLFCKARRLDDKFYQKLRGQFPDAVFWQEIGEIFRQLQKQAAEVYNQSLVELYYEILIKGKGIANASSVEHYLSDVCYTRAAELFKNAAIASGLRNKIKSNFRLKELRNMKSGLPTTKSDNFPIPLVRQKGGQYTGFEISNHDGDFIIKIPFGRWQVKKEINKHRPWEKFDFEQVRKSPKPISLLLSTQRRKRNKGWSKDEGTEAEIRKVMNGDYQTSYIEVKRGSKIGEKSAWMLNLSIDVPKIDKGVDPSIVGGIDVGVKSPLVCAIDNALSRYSISDNDLFHFNKKMFARRRILLKKNRHRRAGHGAKNKLKPISILTEKSKRFRKKLIERWACEIADFFIKNKVGTVQMENLESMKRKEDSYFNIRLRGFWPYAEMQNKIEFKLKQYGIKVRMVAPNNTSKTCSKCGHLNNYFSFEHRKKNKFPHFKCKKCNFKENADYNAALNISNPKLKSTKEEP

SEQ ID NO: 3130 - protein, 726 aa, synthetic construct
SEVEFSHEYWMRHALTLAKRARDEREVPVGAVLVLNNRVIGEGWNRAIGLHDPTAHAEIMALRQGGLVMQNYRLVDATLYVTFEPCVMCAGAMIHSRIGRVVFGVRNNKHGAAGSLVNVLNYPGMNHRVEITEGILADECAALLCDFYRMPRQVFNARKKAQSSINPGGSSGGSSGSETLGTSENATPESSGGSSGSSARNTITKTLKLRIVRPYNSAEVEKVVADEKNNREKIAIEKNKDMVKEACSKHLKVASYCTTQVERNACLFCKARKLDDKFYQKLRGQFPDAVFWQELGGIFRQLQKQAAEIYNQSLIELYYEIFIKGKGIANASSVEHYLSDVCYTRAAELFKNAAIASGLRNKIKSNFRLKELRNMKSGLPTTKSDNFPIPLVRQKGGQYTGFEISNHNSDFIIKIPFGRWQVKKEIDKYRPWEKFDFAQVRKSPKPISLLLSTQRRKRNRGWSKDEGTEAEIKKVMNGDYRTSYIEVKRGSKTGEKSAWMLNLSIDVPKIDKGVDPSTIGGIDVGVKSPLVCAINNAFSRYSISDNDLFRFNKKMFARRRILLGKNRHKRAGHGAKNKLKPISILTEKSGRFRKKLIERWACEIANFFVKNKVGTVQMENLESMKRKEDSYFNIRLRGFWPYAEMQNKIEFKLKQYGIKIRKVAPNNTSKTCSKCGHLNNYFSFEYRRKNKFPHFKCEKCNFKEDADYNAALNISNPKLKSTKEEP

SEQ ID NO: 3131 - protein, 726 aa, synthetic construct
SEVEFSHEYWMRHALTLAKRARDEREVPVGAVLVLNNRVIGEGWNRAIGLNDPTAHAEIMALRQGGLVMQNYRLIDATLYVTFEPCVMCAGAMIHSRIGRVVFGVRNNKHGAAGSLVNVLNYPGMNHRVEITEGILADECAALLCDFYRMPRQVFNARKKAQSSINPGGSSGGSGGSETPGTSESATPESSGGSSGSSAKNTITKTLKLRIVRPYNSAEVEKIVADEKNNREKIALEKNKDKVKEACSKHLKVAAYCTTQVERNACLFCKARRLDDKFYQKLRGQFPDAVFWQEIGEIFRQLQKQAAEIYNQSLVELYYEILIKGKGIANASSVEHYLSDVCYTRAAELFKNAAIASGLRNKIKSNFRLKELRNMKSGLPTTKSDNFPIPLVRQKGGQYTGFEVSNHNSDFIIKIPFGRWQAKKEIDKYRPWEKFDFEQVRKSPKPISLLLSTQRRKRNRGWSKDEGTEAEIKKVMNGDYQTSYIEVKRGSKIGEKSAWMLNLSIDVPKIDKGVDPSIIGGIDVGVKSPLVCAINNAFSRYSISDNDLFHFNKKMFARRRILLKKDRLKRAGHGAKNKLKPISILTGKSERFRKKLIERWACEIADFFIKNKVGTVQMENLESMKRKEDSYFNIRLRGFWPYAEMQNKIEFKLKQYGIEIRRVAPNNTSRTCSKCGHLNNYFNFEYRRKYKFPHFKCEKCNFKEDADYNAALNISNPKLKSTKEEP

SEQ ID NO: 3132 - protein, 726 aa, synthetic construct
SEDEFSHEYWMRHALTLAKRARDGREVPVGAVLVLNNRVIGEGWNRAIGLHDPTAHAEIMALRQGGLVMQNYRLIDATLYVTFEPCVMCAGAMVHSRIGRVVFGVRNSKRGAAGSLMNVLDCPGMGHRVEITEGILADECAALLCDFYCMPRQVFNAQKRAQSSINSGGSSGGSSGSETPGTSESATPESSGGGSSGSAKNTITKTLQLRIVRPYNSAEVEKIVADEKNNREKIALEKNKDKVKEACSKHLKVASYCTTQVERNACPFCKARKLDDKFYQKLRGQFPDAVFWQELGEILRQLQKQAAEIYNQSLIELYYEIFIKGRGFANASSVEHYLSDVCYTRAAELFKNAAIASGLRGKVKGNFRLKVLKNMKSGLPTTKSDNFPIPLVKQKGGQYTGFEISSHNDDFIVKIPFGRWQVKKEIDKYRPWEKFDFEQVRKSPKPISLLLSTQRRKRNKGWSKDEGTEAEVRKVMNGDYQISYIEVKRGSKIGEKSAWMLNLSIDVPKIDKGVDPSIIGGIDVGVKSPLVCAINNAFSRYSISDNDLFRFNKKMFARRRILLKKSKHKRAGHGAKNKLKPISILTGKSERFRKKLIERWACEIADFFIKNKVGTVQMENLESMKGKEDSYFNIRLRGFWPYAEMQNKIEFKLKQYGIEIRKVAPNNTSKTCSKCGHLNNYFNFEYRKKNKFPHFKCEKCYFKEDADYNAALNISNPKLKSTKEEP

SEQ ID NO: 3133 - protein, 726 aa, synthetic construct
SEVEFSHEYWMRHALALAKRARDEREVPVGAVLVLNNRIIGVGWNRAIGLHDPTAHAEIMALRQGGLVMQNYRLIDATLYVTFEPCVMCAGAMIHSRIGRVVFGVRNSKRGAAGSLMNVLNYPGMNHRVEITEGILADECAALLCDYYRMPRQVFNARKKAQSSINSGGSSDGGSGSETPGTSESATPESSGGSSGGSAKNTITKTLKLRIVRPYNSAEVEKIVADEKNNREKIALEKNKDKVKEACSEHLKVAAYCTTQVERSACLFCKARKLDDKFYQKLRGQFPDAVFWQEIGEIFRQLQKQAAEIYNQSLIELYYEIFIKGKGSANASSVEHYLSDVCYTRAAEQFKNAAIASGLRGKVKSNFRLKELKSMKSGLPTTKSDNFPIPLVRQKGGQYTGFEISSHSDDFIIKIPFGRWQVKKEIDKYRPWEKFDFEQVRKSPKPISLLLSTQRRQKNKGWSKDEGTEAEIRRVMNGDYQTSYIEVKRGSKIGEKSAWMLNLSIDVPKIDKGVDPSIIGGIDVGVKSPLVCAINNAFSRYCISDNDLFHFNKKMFARRRILLKKNRRRRAGHGAKNKLKPITILTEKSVRFRKKLIERWACEIANFFIKNKVGTVQMENLESMKRREDSYFNIRLRGFWPYAEMQSKIEFKLKQYGIEVRKVAPDNTSKTCSKCGHLNNYFNFEFRKKNKFPHFKCEKCNFKEDADYNAALNISNPKLKSTKEVP

SEQ ID NO: 3134 - protein, 726 aa, synthetic construct
SEVEFSHEYWMRHALTLAKRARDEREVPVGAVLVLNNRVIGEGWNRAIGLHDPTAHAEIMALRQGGLVMQNYRLVNATLYVTFEPCVMCAGAMIHSRIGRVAFGVRNSKRGAAGSLMNVLNYPGMNHRVEITEGILAEECAALLCDFYRMPRQVFSARKKAQPSINPGGSSDGGSGSETPGTSESATPESSSGSSGGSAKNTITKTLKLRIVRPYNSAEVEKIVADEKDNREKIALEKNKDKVKEACSKHLKVAAYCTTQVERNACLFCKARKLDGKFYQKLRGQFPDAVFWQEIGEIFRQLQKQAAEIYNQSLIELYYEIFIKGKGFANASSVEHYLSDVCYTRAAGLFKNAAIASGLRGKVKSNFRLKELKNMKSGLPTTKSDNFPIPLVKQKGGQYTGFEISSHNDDFIIRIPFGRWQVKEETDKYRPWEKFDFEQVRKSPKPISLLLSTQRRKRNRGWSKDEGTEAEIKKVMNGDYQTSYIEVKRGSKIGEKSAWMLNLSIDVPKIDKGVDPSIIGGIDVGVKAPLVCAINNAFSRYSISDNDLFRFNKKMFARRRILLKESKHKRAGHGAKNKLKPITILTEKSGRFRKKLIERWACEIADFFIKNKVGTVQMENLESMKRREDSYFNTRLRGFWPYAEMQNKIEFKLKQYGIEIRKVAPNNTSKTCSKCGHLNNYFNFEYRRKYKFPHFKCEKCNFKEDADYNAALNISNPKLKSTKEEP

SEQ ID NO: 3135 - protein, 726 aa, synthetic construct
SEVEFSHEYWMRHALALAKRARDGREVPVGAVLVLNNRVIGEGWNRAIGLNDPTAHAEIMALRQGGLVMQNYRLIDATLYVTFEPCVMCAGAMVHSRIGRVVFGVRNSKRGAAGSLMNVLDYPGMGHRVEITEGILVDECAALLCDFYRMPRQVLNAQKKAQSSISPGGSSGGCSGSEMPGASESVTPKSSGGSSAGSTKNTITKTLKLRIVRPYNSAEVEKIVADEKNSREKIALERNKDKVKEACSEHLKVAAYCTTQVERNACLFCKARKLDDRFYQKLRGQFPDAVFWQETGEIFRQLQRQAAEIYNQSLIELYYEIFIKGKGFANASSVEHYLSDVCYTRAAELFKNAAIASGLRNKIKSNFRLKELRNMRSGLPTTKSDNFPIPLVRQKGGQYTGFEISNHDGDFIIKIPFGRWQVKKEINKHRPWEKFDFEQVRKSPKPISLLLSTQRRKRNKGWSKDEGTEAEIRKVMNGDYQTSYIEVKRGSKIGEKSAWMLNLSIDVPKIDKGVDPGIIGGIDVGVKSPLVCAINNASSRYSISDNDLFHFNKKMFARRRILLKKNRHKRAGHGAKNKLKPITIMTEKSKRFRKKLIERWACEIADFFIKNKVGTVQMENLESMKRKEDSYFNIRLRGFWPYAEMQNKIEFKLKQYGIEIRKVAPNNTSKTCSKCGHLSNYFNFEYRKKNKFPHFKCEKCNFKEDADYNAALNISNPKLKSTKEEP

SEQ ID NO: 3136 - protein, 726 aa, synthetic construct
GEVEFSHEYWMRRALTLAKRARDEREVPVGAILVLNNHVIGEGWNRAIGLHDPTAHAEITALRQGGLVMQNYRLIDATLYVTFEPCVMCAGAMIHSRIGRVVFGVRNSKHGAAGSLVNVLNYPGMNHRVGITEGILADECAALLCDFYRMPRQVFNARKKAQPSINPGGSSGGSSGSETPGTSESATPESPGGSPGGSAKNTITKTLKLRIVRPYNSAEVEKIVADEKNNREKIALEKNKDKVKEACSKHLKVAAYCTTQVERNACLFCKARRLDDKFYQKLRGQFPDAVFWQEIGEIFRQLQKQAAEIYNQSLIELYYEIFIKGKGIANASSVEHYLSDVCYTRAAELFKNAAIASGLRNKVKSNFRLKELRSMKSGLPTTKSDNFPIPLVRQKGGQYTGFEISNHNSDFTIKIPFGRWQAKKEIDKYRPWEKFDFEQVRKSPKPISLLLSTQRRKRNRGWSKDESTEAEIKKVMNGDYQTSYIEVKRGSKVGEKSAWMLNLSIDVPKIDKGVDPSIIGGIDVGVKSPLVCAINNAFSRYSISDNELFHFNKKMFARRRILLKKNRHKRAGHGAKNKLKPISVLTEKSGRYRKKLIERWACEIADFFIKNKVGTVQMENLGSMKRKEDSYFNIRLRGFWPYAEMQNKIEFKLKQYGIEIRKVAPDNTSKTCSKCGHLNNYFNFEYRKKNKFPHFKCEKCNFKEDADYNAALNISNPKLKSTKEEP

SEQ ID NO: 3137 - protein, 726 aa, synthetic construct
SEVEFSHEYWMRHALTLAKRARDEREVPVGATLVLNNRVIGEGWNRAIGLHDPTAHAEIMALRQGGLVMQNYRLIDATLYVTFEPCVMCAGAMIHSRIGRVVFGVRNSKHGAAGSLVNVLNYPGMNHRVEITEGILADECAALLCDFYRMPRQVFNARKKAQSSINPSGSSGGSSGSVTPGTSESATPESSGGGFGGSAKNTITKTLQLRIVRPYNSAEVEKIVADEKNNREKIALEKNKDKVKEACSKHLKVASYCTTQVERNACLFCKARKLDDKFYQKLRGQFPDAVFWPEISEIFRQLQKQAAEIYNQSLIELYYEIFIKGKGFANASSVEHYLSDVCYTRAAELFKNAAIASGLRGKVKSNFRLKELRNMKSGLPTTKSDNFPIPLVRQKGGQYTGFEISNYNGDFIIKIPFGRWQVKKEINKHRPWEKFDFEQVRKSPKPISLLLSTQRRKRNKGWSKDEGTEAEIRKAMNGDYQTSYIEVKRGSKIGEKSAWMLSLSIDVPKIDKGVDPRIIGGIDVGVKSPLVCAINNVLSRYSISDNDLFHFNKKMFARRRILLKKNGHKRAGHGAKNKLKPITIMTEKSKRFRKKLIERWACEIADFFIKNKVGTVQMENLESMKRKEDSYFNIRLRGFWPYAEMQNKIEFKLKQYGIVVRKVAPNNTSKTCSQCGHLNNYFNFEYRKKNKFPYFKCEKCNFKENADYNAALNISNPQLKSTKGEP

SEQ ID NO: 3138 - protein, 726 aa, synthetic construct
SEDEFSHEYWMRHALTLAKRARDEREVPVGAILVLNNRVIGEGWNRAIGLHDPTAHAEIMALRQGGLVMQNYRLIDATLYVTFEPCVMCAGAMIHSRIGRVVFGVRNSRRGAAGSLMNVLGYPGMNHRVEITEGILADECAALLCDFYRMPRQVFNTQKKAQSGFNSGGSSGCGSGSETPGTSESATPESSGGSSGGSAKSTITKTLKLRIVRPYNSAEVEKIVADEKNNREKIALEKNKDKVKEACSEHLKVATYCTTQVERNACLFCKARKLDDKFYQKLRGQFPDAVFWQELGEIFRQLQKQAAEIYNQSLIELYYEIFIKGKGLANASSVEHYLSDVCYTRAAELFKNAAIASGLRGKVKSNFKLKELKSMKSGLPSTKSDNFPIPLVKQKGGQYTGFEIRGHNDDLIIKIPFGRWQVKKEIDKYRPWEMFDFEQVRKSPKPISLLLSTQRRKRNKGWSKDEGTEAEIRKVMNGDYQTSYIEVKRGSKIGEKSTWMLNLSIDVPKIDKGVDPSIIGGIDVGVKSPLVCAINNAFSRYSISDNDLFRFNKKVFARRRILLKKNRHKRAGHGTKNKLKPITILTEKSGRFRKKLIERWACEIANFFIKNKVGTVQMENLESMKRKEDSYFNIRLRGFWPYAEMQNKIEFKLKQYGIKIRKVAPNNTSRTCSKCGHLNNYFNFEYRKKNKFPHFKCEKCSFKENADYNAALNISNPKLKSTKEEP

SEQ ID NO: 3139 - protein, 726 aa, synthetic construct
SEVEFSHEYWMRHALTLAKRARDEREVPVGAVLVLNNRVIGEGWNRAIGLHDPTAHAEIMALRQGGLVMQNHRLTDATLYVTFEPCVMCAGAMIHSRIGRVVFGVRNSKRGAAGSLMNVLNYPGMNHRVEITEGILADECAALLCDFYHMPRQVFSAQKKAQFSINSGGSSGGSSGGETPGTSESATPKSSGGSSGGSAKNTITKALKLRIVRPYNSAEVEKIVADEKNNREKIALEKNRGKVKEACSEHLKVAAYCTTQVERNACLFCKARKLDDKFYQKLRGQFPDAVFWQEISEIFRQLQKQAAEIYNQSLIELYYEIFIKGKGFANASSVEHYLSDVCYTRAAELFKNAAIASGLRGKVKSNFRLKELKSMKSGLPTTKSDNFPIPLVKQKGGQYTGFEISSHNDDFIIKIPFGRWQVRKEIDKYRPWEKFNFEQVRKSPKPISLLLSTQRRRRNKGWSKDEGTEAEIRKVMNGDYQTSYIEVKRGSKIGEKSAWMLSLSIDVPKIDKGVDPSIIGGIDVGVKSPLVCAINNAFNRYSISDNNLFHFNKKVFARRRILLKKNRHKRAGHGAKNKLKPISILTEKSKRFRKKLIERWACEIADFFIKNKVGTVQMENLESMKRKEDSYFNIRLRGFWPYAEMQNKIEFKLKQYGIEIRKVAPNNTSKTCSKCGHLNNYFNFEYRRKNKFPYFKCEKCNFKEDADYNAALNISNPKLRSTKEKP

SEQ ID NO: 3140 - protein, 726 aa, synthetic construct
SEVEFSHEYWMRHALTLAERARDAREVPVGAILVLNNRVIGEGWNRAIGQHDPTAHAEIMALRQGGLVMQNYRLIDATLYVTFEPCVMCAGAMIHSRIGRVVFGVRNSKHGAAGSLMNVLNYPGMNHRVEITEGILADECAALLCDFYRMPRQVFNGRKKAQSSINSGGSSGGSSGSETPGTSESATPESSGGSSSGSTKNTITKTLKLRIVRPYNSTEVEKIVADEKNNREKIALEKNKDKVKEACSRHLKVAAYCTTQVERNACLFCKARKLDDKFYQKLRGQFPDAVFWQEIGEIFRQLQKQAAEIYNQSLIELYYEIFIKGKGFANASSAEHYLSDVCYTRAAELFKNAAIASGLRGKVKSNFRPKELKNMRSGLPTTKSDNFPIPLVKQKGGQYTGFEISSHNDDFIIKIPFGRWQVKKEIDKYRPWEKFDFEQVRKSPKPISLLLSTQRRKRNRGWSKDEGTEAEIKKVMNGDYQTSYIEVKRGSKIGEKSAWMLNLSIDVPKIDKGVDPSIIGGIDVGVKAPLVCAINNAFSRYSISDNDLFRFNKKMFARRRILLKKNGRKRAGHGAKNKLKPITILTEKSGRFRKKLIERWACEIANFFIKNKVGTVQMENLESMKRKEDSYFNIRLRGFWPYAEMQSKIEFKLKQYGIKIRKVAPNNTSKTCSKCGHLNNYFSFEYRKKNKFPHFKCEKCNFKESADYNAALNISNPKLKSTKEEP

SEQ ID NO: 3141 - protein, 726 aa, synthetic construct
SEVEFSHEYWMRHALTLAKRARDEREVPVGAVLVLNNRVIGEGWNRTTGLHDPTAHAEIMALRQGGLVMQNHRLVDATLYVTFEPCVMCAGAMIHSRIGRVVFGVRNSKRGAAGSLTNVLNYPGMNHRVEITEGILVDECAALLCDFYRMPRQVLNAQKKAQSSISPGGSSGGSSGSETPGASESVTPKSSGGSSGGSAKNTITKTLKLRIVRPYNSAEVEKIVADEKNNREKIALEKNKDKVKEACSKHLKVAAYCTTQVERNACPFCKARRLDDKFYQKLRGQFPDAVFWQEIGEIFRQLQKQAAEIYNQSLVELYYEILIKGKGIANASSVEHYLSDVCYTRAAELFKNAAIASGLRGKVRSNFRLKELKNMKSGLPTTKSDNFPIPLVKQKGGQYTGFEISSHNDDFIIKIPFGRWQVKKEIDKYRPWEKFDFEQVRKSPKPISLLLSTQRRKRNKGWSKDEGTEAEIRRVMNGDYQTSYIEVKRGSKIGERSAWMLNLSIDVPKIDKGVDPSIIGGIDVGVKSPLVCAINNSSSRYSISDNDLFHFNKKMFARRRILLKKNRHKRAGHGAKNKLKPISILTEKSKRFRKKLIERWACEIADFFIKNKVGTVQMENLESVKRKEDSYFNIRLRGFWPYAEMQNKIEFKLRQYGIEIRKVAPNNTSRTCSKCGHLNNYFSFEYRKKNKFPHFKCKKCNFKEDADYNAALNISNPKLKSTKEEP

SEQ ID NO: 3142 - protein, 725 aa, synthetic construct
SGVELSHEYWMRHALTLAKRARDGREVPVGAVLVLNNRVIGEGWNRAIGLNDPTAHAEIMALRQGGLVMQNHRLIDATLYVTFEPCVMCAGAMVHSRIGRVVFGVRNSKRGAAGSLMNVLDHPGMDHRVEITEGILADECAALLCDFYRMPRQVFNAQKKAQSSINSGGSSGGSSGSETPGTSESATPECPGGSSGGSAKNTITKTLKLRIVRPYNSAEVEKIVADEKNNREKIALEKNKDKVKEACSEHLKVAAYCTTQVERSACLFCKARKLDDKFYQKLRGQFPDAVFWQEIGEIFRQLQKQAAEIYNQSLIELYYEIFIKGKGFANASSVEHYLSDVCYTRAAELFKNAAIASGLRGKVKSNFRLKELKNMKSGLPTTKSDNFPIPLVKQKGGQYTGFEISCHNDDFIIKIPFGRWQVKKEIDRYRPWEKFDFEQVRKSPKPISLLLSTQRRKRNKGWSKDEGTEAEIRKVMNGDYQTSYIEVKRGSKTGEKSAWMLNLSIDVPKIDKGVDPCVIGGIDVGVKSPLVCAINNAFSRYSISDNDLFHFNKKMFARRRILLKENGHKRAGHGAKNKLKPITIMTEKSKRFRKKLIERWACEIADFFIKNKVGTVQMENLESMKRKEDSYFNIRLRGFWPYAEMQNKIEFKLKQYGIEIRKVAPNNTSKTCSKCGHLNNYFNFEYRKKNKFPHFKCEKCNFKENADYNAALNISNPKLKSTEEP

SEQ ID NO: 3143 - protein, 725 aa, synthetic construct
SEVEFSHEYWMRHALTLARRARGEREVPVGAILVLNNRVIGEGWNRAIGLHDPTAHAEIMALRQGGLAMQNYRLTDATLYVTFEPCVMCAGAMIHSRIGRVVFGVRNSKRGAAGSLMNVLNYPGMNHCVEITEGILVDECAALLCDFYRMPRQVLNAQKKAQSSISSGGSSGGSSGSVTPGASGSVTPSSGGSSAGSTKDTITKTLKLRIVRPYNSAEVEKIVADEKNNREKIALEKNKDKVKEACSKHLKVASYCTTQVERNACPFCKARKLDDKFYQKLRGQFPDAVFWQELGEILRQLQKQAAETYNQSLIELYYEIFIKGKGFANASSVEHYLSDVCYTRAAELFKNAAIASGLRGKVKSNFRLKELKNMKSGLPTTKSDNFPIPLVKQKGGQYTGFEISSHNDDFIIKIPFGRWQVKEEIDKYRPWEKFDFEQVRKNPKPISLLLSTQRRKRNKGWSKDEGTEAEIRKVMNGDYQTSYIEVKRGSKIGEKSAWMLNLSIDVPKIDKGVDPSIIGGIDVGVKSPLVCAINNAFSRYSISDNDLFRFNKKVFARRRILLKKSRYKRAGHGTKNKLKPITILTEKSGRFRKKLIERWACEIANFFIKNKVGTVQMENLESMKRKEDSYFNIRLRGFWPYAEMQNKIEFKLKQYGIKIRKVAPNNTSKTCSKCGHLNNYFSFEYRKKNKFPHFKCEKCNFKEDADYNAALNISNPKLKSTKEEP

SEQ ID NO: 3144 - protein, 725 aa, synthetic construct
SEVEFSHEYWMRHALTLAERARDGREVPVGAVLVLNNRVIGEGWNRAIGLHDPTAHAEIMALRQGGLVMQNYRLIDATLYVTFEPCVMCAGAMIHSRIGRVVFGVRNSKRGAAGSLMNVLNYPGMGHRVEITEGILADECAALLCDFYCMPCQVFNAQKRAQSSINSGGSSGGSSGSVTPGTSESATPESSGGGSAGSTKNTITKTLKLRIVRPYNSAEVEKIVADEKNSREKIALERNKGKVKEACSEHLKVAAYCTTQVERNACLFCKARKLDDRFYQKLRGQFPDAVFWQETGEIFRQLQRQAAEIYNQSLIELYYEIFIKGKGFANASSVEHYLSDVCYTRAAELFKNAAIASGLRGKVKSNFRLKELKNMKSGLPTTKSDNFPIPLVKQKGGQYTGFEISSHNDDFIIKIPFGRWQVRKEIDKYRPWEKFDFEQVRKSPKPISLLLSTRRRKRNKGWSKDEGTEAEIRKVMNGDYQTSYIEVKRGSKIGEKSAWMLNLSIDVPKIDKGVDPSIIGGIDVGVKSPLVCAINNAFGRYSISDNDLFHFNKKMFARRRILLKKNRHKRAGHGAKNKLKPITILTEKSKRFRKKLIERWACEIADFFIKNKVGTVQMENLESMKRKEDSYFNIRLRGFWPYAEMDKIEFKLKQYGIEIRKVAPNNTSKTCSKCGHLNNYFNFEYRRKNKFPHFKCEKCNFKENADYNAALNISNPKLKSTKEEH

SEQ ID NO: 3145 - protein, 726 aa, synthetic construct
SEVEFSHEYWMRHALTLAKRARDEREVPVGAILVLNNRVIGEGWNRAIGLHDPTAHAEIMALRQGGLVMQNYRLIDATLYVTFEPCVMCAGAMIHSRIGRVVFGVRNNKHGAAGSLVNVLDYPGMGHRVEITEGILADECAALLCDFYCMPRQVFNARKRAQSSISSGGSSGGSSGSETPGTSESATPESSGGGSSGSAKNTFTKTLQLRIVRPYNSAEVEKIVADEKNNREKIALEKNKDKVREACSRHLKVASYCTTQVERNACPFCRARKLDDKFYQKLGGQFPDAVFWQELSEILRQLQKQAAEIYNQSLIELYYEIFIKGKGITNASRVEHYLSDVCYTRAAELFKNAAIASGLRSKVRSNFRLKELKNMKSSLPTTKSDNFPIPLVKQKGGQYTGFEISSHNSDFIIKIPFGRWQVKEEIDKYRPWEKFDFEQVRKSPKPISLLLSTQRRKKNKGWSKDEGTEAEIRRVMNGDYQTSYIEVKRGSKIGEKSAWMLNLSIDVPKIDKGVDPSIVGGIDVGVKSPLVCAINNAFSRYSISDNDLFHFNKKMFARRRILLKKNRHRRAGHGAKNKLKPITILTEKSVRFRKKLIERWACEIADFFIKNKVGTVQMENLESMKRKEDSYFNIRLRGFWPYAEMQNKIEFKLKQYGIEIRRVAPNNTSRTCSKCGHLNNYFNFEYRRKNKFPHFKCEKCNFKEDADYNAALNISNPKLKSTKEEP

SEQ ID NO: 3146 - protein, 726 aa, synthetic construct
SEVEFSHEYWMRHALTLAKRARDEREVPVGAVLVLNNRVIGEGWNRTTGLHDPTAHAEIMALRQGGLVMRNYRLTDATLYVTFEPCVMCAGAMIHSRIGRVVFGARNSKRGAAGSLMNVLSYPGMNHRVEITEGILADECAALLCDFYRMPRRVLNAQKKAQSSINSGGSSGGSSGSETPGTSESATLESSGSSSGGSAKNTITKTLKLRIVRPYNSAEVEKIVADEKNNREKIALEKNKDKVKEACSKHLKVAAYCTTQVERNACLFCKARRLDEKFYQKLRGQFPGAVFWQEIGEIFRQLQKQAAETYNQSLIELYYEIFVKGKGIANASNVEHYLSDVCYTRAAELFKNAAIASGLRNKIKSNFRLKELRNMKSGLPTTKSDNFPIPLVKQKGGQYTGFEISNHNGDFIIKIPFGRWQAKKEIDKYRPWEKYDFEQVRKSPKPISLLLSTQRRKRNRGWGKDEGTEAEIKRVMNGDYQTSYIEVKRGSKIGEKSAWMLSLSIDVPKIDKGVDPSTIGGIDVGVKSPLVCAINNAFCRYSISDNDLFHFNKKMFARRRILLKKSRHKRAGHGAKNKLKPISILTEKSKRFRKKLIERWACEIADFFVKNKVGTVQMENLESMKRKEDSYFNIRLRGFWPYAEMQNKIEFKLKQYGIEIRKVAPNNTSKTCSKCGHLNNYFNFEYRRKNKFPHFKCEKCNFKENADYNAALNISNPKLKSTKEEP

SEQ ID NO: 3147 - protein, 726 aa, synthetic construct
GEVEFSHEYWMRRALTLAKRARDEREVPVGAVLVLNNRVIGVGWNRAVGLHDPTAHAEIMALRQGGLVMQNYRLVEATLYVTFEPCVMCAGAMIHSRIGRVVFGVRNNKHGAAGSLVNVLNYPGMNHRVEITEGILADECTALLCDFYRMPRQVFNARKKAQSSISPDGSSDGSSGSETPGTSESATPESSSGSSGGSAKNTITKTLKLRIVRPYNSAEVEKIVADEKSNREKIALEKNKDKVKEACSEHLKVAAYCTTQVERSACLFCKARRLDDKFYQKLRGQFPDAVFWQEIGEIFRQLQKQAAEIYNQSLVELYYEIFIKGKGIANASSVEHYLSDVCYTRAAELFKNAAIASGLRNKIKSNFRLKELRNMKSGLPTTKSDNFPIPLVRQKGGQYTGFEISNHNGDFIIKIPFGRWQVKKEISKHRPWEKFDFEQVRKSPKPISLLLSTQRRKRNKGWGKDEGTEAEIRKVMNGDYQTSYIEVKRGSKIGEKSAWMLNLSIDVPKIDKGVDPSIIGGIDVGVKSPLVCAINNAFSRYSISDNDLFHFNKKMFARRRILLKKNRRRRAGHGAKNKLKPITILTEKSVRFRKKLIERWACEIADFFIKNKVGTVQMENLESMKRKEDSYFNIRLRGFWPYAEMQNKIEFKLKQYGIEIRRVAPNNTSRTCSKCGHLNNYFNFEYRRKYKFPHFKCEKCNFKEDADYNAALNISNPKLKSTKEEP

SEQ ID NO: 3148 - protein, 726 aa, synthetic construct
SEVEFSHEYWMRRALTLAKRARDEREVPVGAVLVLNNRVIGVGWNRAVGLHDPTAHAEIMALRQGGLVMQNYRLIEATLYVTFEPCIMCAGAMIHSRIGRVVFGVRNSKRGAAGSLMNVLNYPGMNHHVEITEGILVDECAALLCDFYRMPRQVLNAQKKAQSSISSGGSSGGCSGSEMPGASESVTPKSSGGSSAGSTKNTITKTLKLRIVRPYNSAEVEKIVADEKNSREKIALERNKDKVKEACSEHLKVAAYCTTQVERNACLFCKARRLDDKFYQKLRGQFPDAVFWQEIGEIFRQLQKQAAEIYNQSLVELYYEILIKGKGIANASSVEHYLSDVCYTRAAELFKNAAIASGLRNKIKSNFRLKELRNMRSGLPTTKSDNFPIPLVRQKGGQYTGFEISNHDGDFIIKIPFGRWQVKKEINKHRPWEKFDFEQVRKSPKPISLLLSTQRRKRNKGWSKDEGTEAEIRKVMNGDYQTSYIEVKRGSKIGEKSAWMLNLSIDVPKIDKGVDPSIIGGIDVGVKSPLVCAINNSSSRYSICDNDLFRFNKKMFARRRILLKKNRHKRAGHGAKNKLKPITILTKKSERFRKKLIERWVCEVAEFFIKNKVGTVQMENLESMKRKEDSYFNIRLRGFWPYAEMQNRIELKLKQYGIEIRRVAPNNTSRTCSKCGHLNNYFSFEYRKRSKFPHFKCEKCNYREDADYNAALNISNPKLKSTKEEP

SEQ ID NO: 3149 - protein, 726 aa, synthetic construct
SEVEFSHEYWMRHALTLAKRARGEREVPVGAVLVLNNRVIGEGWNRAIGLHDPTAHAEIMALRQGGLVMQNYRLTDATLYVTFEPCVMCAGAMIHSRIGRVVFGVRNSKRGAAGSLMNVLNYPGMNHCVEITEGILVDECAALLCDFYRMPRQVLNAQKKAQSSISSGGSSGGSSGSETPSTSESATPESSGGSSSGSAKNTITKTLQLRIVRPYNSAEVEKIVADEKNNREKIALEKNKDKVREACNKHLKVASYCTTQVERNACPFCKARKLDDKFYQKLRGQFPDAVFWQEIGEIFRQLQKQAAEIYNQSLIELYYEIFIKGKGFANASSVEHYLSDVCYTRAAELFRNAAIASGLRGKVKSNFRLKELKNMKSGLPTTKSDNFPIPLVRQKGGQYTGFEISSHNDDFIIKIPFGRWQVRKEIDRYRPWEKFGFEQVRKSPKPISLLLSTQRRKRNKGWSKDEGTEAEIRKVMNGDYQTSYIEVKRGSKTGEKSAWMLNLSIDVPKIDKGVDPSVTGGIDVGVKSPLVCAINNAFSRFSISDNDLFHFNKKMFARRRILLKKNGRKRAGHGAKNKLKPISILTEKSGRFRKKLIERWACEIANFFIKNKVGTVQMENLESMKRKGDSYFNIRLRGFWPYAEMQNKIEFKLKQYGIKIRKVAPNNTSKTCSKCGHLNNYFSFEYRKKNKFPHFKCEKCNFKEDADYNAALNISNPKLKSTKEEP

SEQ ID NO: 3150 - protein, 726 aa, synthetic construct
SEVEFSHEYWMRHALTLAKRARDEREVPVGAILVLNNRVIGEGWNRAIGLHDPTAHAEIMALRQGGLVMQNYRLIDATLYVTFEPCVMCAGAMIHSRIGRVVFGVRNNKHGAAGSLVNVLNYPGMNHRVEITEGILADECAALLCDFYRMPRQVFNARKKAQSSTNPGGSPGGSSGSKMPGTSGSATPGSSGGSSGGSAKNTITKTLKLRIVRPYNSAEVEKIVADEKNNREKVALEKNKDKVKEACSEHLKVAAYCTTQVERSACLFCKARKLDDKFYQKLRGQFPDAVFWQEIGEIFRQLQKQAAEIYNQSLIELYYEVFIKGKGFANASSVEHYLSDVCYTRAAELFKNAAIASGLRGKVKSNFRLKELKNMKSGLPTTKSDNFPIPLVRQKGGQYTGFEISNHDGDFIIKIPFGRWQVKKEINKHRPWEKFDFEQVRKSPKPISLLLSTQRRKRNKGWSKDEGTEAEIRKVMNGDYQTSYIEVKRGSKTGEKSAWMLNLSIDVPKIDKGVDPSIIGGIDVGVKSPLVCAINNAFSRYSISDNDLFRFNKKMFARRRILLKKSKHKRAGHGAKNKLKPISILTEKSERFRKKLIERWACEIADFFVKNKVGTVQMENLESMKRKEDSYFNIRLRGFWPYAEMQNKIEFKLKQYGIEIRKVAPNNTSRTCSKCGHLNNYFNFEYRKKNKFPHFKCEKCNFKENADYNAALNISNPKLKSTKEEP

SEQ ID NO: 3151 - protein, 726 aa, synthetic construct
SEVEFSHEYWMRHALTLAKRARDEREVPVGAILVLNNRVIGEGWNRTIGLHDPTAHAEIMALRQGGLVMQNYRLIDATLYVTFEPCVMCAGAMIHSRIGRVVFGVRNNKHGAAGSLVNVLDYPGMNHRVEITEGILADECAALLCDFYRMPRQVFSAQKKAQSSISSGGSSGGSSGSETPGTSESATQESSGGSPGGSAKNTITKTLKLRIVRPYNSAEVEKIVADEKNSREKIALEENKDKVEEACSQHLKMASYCTTQVERNACLFCKARKLDDKFYQKLRGQFPDAVFWQEIGEIFRQLQKQAAEIYNQSLVELYYEILIKGKGIANASSVEHYLSDVCYTRAAELFKNAAIASGLRNKVKSNFRLKELRNMKSGLPTTKSDNFPIPLVRQKGGQYTGFEISSHNDDFIIKIPFGRWQVKKEIDKYRPWEKFDFEQVRKSPKPISLLLSTQRRKRNKGWSRDEGTEAEIRKVMNGDYQTSYIEVKRGSKIGEKSAWMLNLSIDVPKIDKGVDPSIIGGIDVGVKSPLVCAINNAFSRYSISDNDLFHFNKKMFARRRILLKKNRHKRAGHGAKNKLKPISILTEKSKRFRKKLIERWACEIADFFIKNKVGTVQMENLESMKRKEDSYFNIRLRGFWPYAEMQNRIEFKLKQYGIEIRRVAPNNTSRACSKCGHLNNYFNFEYRKKNKFPHFKCEKCNFREDADYNAALNISNPKLKSTKEEP

SEQ ID NO: 3152 - protein, 726 aa, synthetic construct
SEDEFSHEYWMRHALTLAKRARDGREVPVGAVLVLNNRVIGEGWNRAIGLHDPTAHAEVMALRQGGLVMQNYRLTDATLYVTFEPCVMCAGAMIHSRIGRVVFGVRNSKRGAAGSLMNVLNYPGMNHCVEITEGILMDECAALLCDFYRMPRQVLNAQKKAQSSISSGGPSGSSSCSETPGASESVTPKSSGGSSTGSAKNTITKALKLRIVRPYNSAEVEKIVADEKSNREKIALEKNKGKVKEACSKHLKVAAYCTTQVERNACLFCKARRLDDEFYQKLRGQFPDAVFWQEIGEIFRQLQKQAAEVYNQSLVELYYEIFIKGRGFANASSVEHYLSDVCYTRAAELFKNAAIASGLRSKVKSNFRLKELKNMKSGLPTTKGDNFPIPLVKQKGGQYAGFEISSHNDDFIIKIPFGRWQVKKEIDRYRPWEKFDFEQVRKSPKPISLLLSTQRRKKNRGWSKDEGTEAEIKKVMNGDYQTSYIEVKRGSKIGEKSAWMLNLSIDVPKIDKGVDPSIIGGIDVGVKSPLVCAISNAFSRYSISDNDLFHFNKKMFARRRILLKKSKHKRAGHGAKNKLKPITILTEKSRRFRKKLIERWACEIADFFIKNKVGTVQMENLESMKRREDSYFNIRLRGFWPYAEMQDKIEFKLKQYGIKVRKVAPNNTSKTCSRCGHLNNYFNFEYRRKNKFPHFKCEKCNFKEDADYNAALNISNPKLKSTKEEP

SEQ ID NO: 3153 - protein, 726 aa, synthetic construct
SEVEFSHEYWMRHALTLAKRARDEREVPVGAVLVLNNRVIGEGWNRAIGLHDPTAHAEIMALRQGGLVMQNYRLTDATLYVTFEPCVMCAGAMIHSRIGRVVFGVRNSKRGAAGSLMNVLNYPGINHCVEITEGILVDECAALLCDFYRMPRQVLNAQKKAQSSISSGGSSGGSSGSETPGASESVTPKSSVGSSAGPTKNTITKTLKLRIVRPYNSAEVEKIVADEKNNRERIALEKNKDKVKEACSEHLKVAAYCTTQVERNACLFCKARKLDDKFYQKLRGQFPDAVFWQEIGEIFRQLQKQAAEIYNQSLIELYYEIFIKGKGFANASSVEHYLSDVCYTRAAELFKNAAIASGLRGKVKSNFRLKELKNMKSGLPTTKSDNFPIPLVKQKGGQYTGFEICSHNDDFIIKIPFGRWRVKKEIDKYRPWEKFDFEQVRKSPKPISLLLSTQRRKRNKGWSKDEGTEAEIRKVMNGDYQTSYIEVKRGSKIGEKSAWMLNLSIDVPKIDKGVDPGITGGIDVGVKSPLVCAINNAFSRYSISDNDLFRFNKKVFARRRILLKKNRHKRAGHGTKNKLKPITILTEKSGRFRRKLIERWACEIANFFIKNKVGTVQMENLESMKRKEDSYFNIRLRGFWPYAEMQNKIEFKLKQYGIEIRKVAPNNTSKTCSKCGHLNNYFNFEYRKMNKFPHFKCEKCNFKENADYNAALNISNPKLKSTKEEP

SEQ ID NO: 3154 - protein, 726 aa, synthetic construct
SEVEFSHEYWMRHALTLARRARDKREVPVGAILVLNNRVIGEGWNRAIGLHDPTAHAEIMALRQGGLVMQNYRLVDATLYVTFEPCVMCAGAMIHSRIGRVVFGVRNNKHGAAGSLMNVLNYPGMNHRVEITEGILADECAALLCDFYCMPRQVFNARKKAQSSINPGGPSGGSSGSKTPGTSESATPEGSGGSSGGSAKNTITKTLKLRIVRPYNSAEVEKIVADEKNNREKIALEKNKDKVKEACSKHLKVAAYCTTQVERNACLFCKARKLDDKFYQKLRGQFPDAVFWQEIGEIFRQLQKQAAEIYNQSLIELYYEIFIKGKGFANASSAEHYLSDVCYTRAAELFKNAAIASGLRGKVKSNFRLKELKNMKSGLPTTKSDNFPIPLVKQKGGQYTGFEISSHNSDFIIKIPFGRWQVKEEIDKYRPWEKFDFEQVRKSPKPISLLLSTQRRRKNKGWSKDEGTEAEIRRVMNGDYQTSYIEVKRGSKIGEKSAWMLNLSIDVPKVDKGVDPSIIGGIDVGVKSPLVCAINNSFSRYSICDNDLFRFNKRMFARRRILLKKNGHKRAGHGAKNKLKPITIMTEKSKRFRKKLIERWACEIADFFIKNKVGTVQMENLESMKRKEDSYFNIRLRGFWPYAEMQNKIEFKLKQYGIVVRKVAPNNTSRTCSRCGHQNNYFNFEYRKKNKFPHFKCEKCNFKENADYNAALNISNPKLKSTKGEP

SEQ ID NO: 3155 - protein, 726 aa, synthetic construct
SEVEFSHEYWMRHALTLAKRARDEREVPVGAVLVLNNRAIGEGWNRAIGLHDPTAHAEIMALRQGGLVMQNYRLVDATLYVTFEPCVMCAGAMIHSRIGRVVFGVRNNKHGAAGSLMNVLNYPGMNHRVEITEGILADECAALLCDFYRMPRQVFNARKKAQSSINPGGPSGGSSGSKTPGTSESATPESSGGSSGGSAKNTITKTLQLRIVRPYNSAEVEKIVADEKNNREKIALEKNKGKVKEACSKHLEVAAYCTTQVERNACLFCKARKLDDKFYQKLRGQFPDAVFWQELGEIFRQLQKQAAEIYNQSLIELYYEIFIKGKGLANASSVEHYLSDVCYTRAAELFKNAAIASGLRGKVKSNFKLKELKSMKSGLPSTKSDNFPIPLVKQRGGQYTGFEISSHNDDFIIKIPFGRWQAKKEIDKYRPWEKFDFEQVRKSPKPISLLLSTQRRKRNRGWSKDEGTEAEIRRVMNGDYQTSYIEVKRGSKIGEKSAWMLNLSIDVPKIDKGVDPSIIGGIDVGVKSPLVCAINNAFSRYSISDNDLFRFNKKMFARRRVLLKKNRHRRAGHGAKNKLKPITILTEKSGRFRRKLIERWACEIANFFIKNKVGTVQMENLESMKRKEDSYFNIRLRGFWPYAEMQNKIEFKLKQYGIKIRKVAPNNTSKTCGKCGHLNNYFSFEYRKKNKFPHFKCEKCNFKEDADYNAALNISNPKLKSTKEEP

SEQ ID NO: 3156 - protein, 726 aa, synthetic construct
SEVEFSHEYWMRHALTLAKRARDEREVPVGAVLVLNNRVIGEGWNRAIGLHDPTAHAEIMALRQGGLVMQNYRLIDATLYVTFEPCVMCAGAMIHSRIGRVVFGARNSKRGAAGSLMNVLDYPGMNHCVEITEGILVDECAALLCDFYRMPRQVLNAQKKAQSSISSGGSPGGSSGSETPGASESVTPKSSGGGSAGSTKNTITKTLKLRIVRPYNSAEVEKIVADEKNSREKIALEKNKDKVKEACSKHLKVAAYCTTQVERNACLFCKARKLDDRFYQKLRGQFPDAVFWQEISEIFRQLQKQAAEIYNQSLIELYYEIFIKGKGLANASSVEHYLSDVCYTRAAELFKNAAIASGLRGKIKSNFRLKELKNMKSGLPTTKSDNFPIPLVKQKGGQYTGFEISNHNSDFIIKIPFGRWQVKEEIDKYRPWEKFDFEQVRKSPKPISLLLSTQRRQKNKGWSKDEGTEAEIRRVMNGDYQTSYIEVKRGSKIGEKSAWMLNLSIDVPKIDKGVDPSIIGGIDVGVKSPLVCAINNAFSRYSVSDNDLFRFNKKMFARRRILLGKNRHKRAGHGTKNKLKPITILTEKSGRFRKKLIERWACEIANFFIKNKVGTVQMENLESMKRKEDSYFNIRLRGFWPYAEMQNKIEFKLKQYGIEIRKVAPNNTSKTCSKCGHLNNYFSFEYRKKNKFPHFKCEKCNFKEDADYNAALNISNPKLKSTKEEP

SEQ ID NO: 3157 - protein, 725 aa, synthetic construct
SEVEFSHEYWMRHALTLAKRARDEREVPVGAILVLNNRVIGEGWNRAIGLHDPTAHAEIMALRQGGLVMQNYRLIDATLYVTFEPCVMCAGAMIHSRIGRVVFGVRNSKHGAAGSLVNVLNYPGMNHRVEITEGVLADECAALLCDFYRMPRQVFNARKKAQSSINPGGSSGGSSGSETPGTSESATPESSGGSSGGSAKNTITKTLKLRIVRPYNSAEVEIVADEKNSREKIALEKNKDKVKEACSEHLKVAAYCTTQVERSACLFCKARKLDDKFYQKLRGQFPDAVSWQEIGEIFRQLQKQAAEIYNQSLIELYYEIFIKGKGFANASSVEHYLSDVCYTRAAELFKNAAIASGLRGKVKSNFRLKELKNMKSGLPTTKSDNFPIPLVKQKGGQYTGFEISSHNGDFIIKIPFGRWQVKKEIDRYRPWEKFDFEQVRKSPKPISLLLSTQRRKRNKGWSKDEGTEAEIRKVMNGDYQTSYIEVKRGSKVGEKSAWMLNLSIDVPKIDKGVDPSIIGGIDVGVKSPLVCAINNAFSRYSISDNDLYRFNKKMFARRRILLKKSKHKRAGHGAKNKLKPITILTEKSGRFRKKLIERWACEIADFFIKNKVGTVQMENLEGMKRKEDSYFNIRLRGFWPYAEMQNKIEFKLKQYGIEIRKVAPNNTSKTCSKCGHLNNYFNFEYRKKNKFPHFKCEKCNFKENADYNAALNISNPVLKSTKEEP

SEQ ID NO: 3158 - protein, 726 aa, synthetic construct
SEVEFSHEYWMRRALTLAKRARDEREVPVGAVLVLNNRVIGVGWNRAVGLHDPTAHAEIMALRQGGLVMQNYRLIEATLYVTFEPCIMCAGAMIHSRIGRVVFGVRNSKRGAAGSLMNVLNYPGMNHRVEITEGILADECAALLCDYYRMPRQVFNARKKAQSSINSGGSFDGGSGSETPGTSESATSESSGGSSDGSAKNTITKTLKLRIVRPYNSAEVEKIVADEKNNREKIALEKNKDKVKEACSKHLKVAAYCTTQVERNACLFCKARKLDDKFYQKLGGQFPDAVFWQEISEIFRQLQKQAAEIYNQSLIELYYEILIKGKGITNASSVEHYLSDVCYTRAAELFKNAAIASGLRGKIKSNFRLKELKNMKSGLPTTKSDNFPIPLVKQKGGQYTGFEISSHNDDFIIKIPFGRWQVKKEIDKYRPWEKFDFEQVRKSPKPISLLLSTQRRKRNKGWSKDEGTEAEIRKVMNGDYQTSYIEVKRGSKIGEKSAWMLNLSIDVPKIDKGVDPSVVGGIDVGVKSPLVCAIDNALSRYSISDNDLFRFNKKMFARRRILLKRNRHKRAGHGAKNKLKPISILTGKSERFRRKLIERWACEIADFFIKNKVGTVQMENLESMKRKEDSYFNIRLRGFWPYAEMQNKIEFKLKQYGIEIRKVAPNNTSKTCSKCGHLNNYFNFEYRKKNKFPHFKCEKCNFKENADYNAALNISNPKLKSTKEEP

SEQ ID NO: 3159 - protein, 726 aa, synthetic construct
SEVEFSHEYWMRHALTLAKRARDEREVPVGAILVLNNCVIGEGWNRAIGLHDPTAHAEIMALRQGGLVMQNYRLIDATLYVTFEPCVMCAGAMIHSRIGRVVFGVRNNKHGAAGSLVNVLDYPGMNHRVEITEGILADECAALLCDFYRMPRQVFNARKKAQSSISPGGSSGGSSGSETPGTSESATPESSGGSSGGSAKNTITKTLKLRIVRPYNSTEVEKIVADEKNNREKVALEKNKDKVKEACSKHLKVAAYCTTQVERNACLFCKARRLDDKFYQKLRGQFPDAVFWQEIGEIFRQLQKQAAEIYNQSLVELYYEILIKGKGIANASSVEHYLSDVCYTRAAELFKNAAIASGLRNKIKSNFRLKELRNMKSGLPTTKSDNFPIPLVRQKGGQYTGFEISNHDGDFIIKIPFGRWQVKEEIDKYRPWEKFDFEQVRKYPKPISLLLSTQRRKRNKGWSKDEGTEAEIRRVMNGDYQTSYIEVKRGSKIGEKSAWMLNLSIDVPKIDKGVDPSIIGGIDVGVKSPLVCAINNAFGRYSISDNDLFHFNKKMFARRRILLKKNRHKRAGHGAKNKLKPITILTEKSKRFRKKLIERWACEIADFFIKNKVGTVQMENLESMKRREDSYFNIRLRGFWPYAKMQNKIEFKLKQYGIEIRKVAPNNTSKTCSKCGHLNNYFNFEYRKKNKFPHFKCEKCNFKENADYNAALNISNPKLKSTKEEP

SEQ ID NO: 3160 - protein, 726 aa, synthetic construct
SEVEFSHEYWMRHALTLAKRARDEREVPVGAILVLNNHVIGEGWNRAVGLHDPTAHAEIMALRQGGLVMQNYRLIDATLYVTFEPCVMCAGAMIHSRIGRVVFGVRNNKHGAAGSLVNVLDYPGMNHRVEITEGILADECAALLCDFYRMPRQVFNARKKAQSSISSGGSSGGSSGSETPGASESATPKSSGGSSAGSTKNTITKTLKLRIVRPYNSAEVEKIVADEKNNRERIALEKNKDKVKEACSKHLKVAAYCTTQVERNACLFCKARKLDDKFYQKLRGQFPDAVFWQETGEIFRQLQRQAAEIYNQSLIELYYEIFIKGKGFANASSVEHYLSDVCYTRAAELFKNAAIASGLRGKVKSNFRLKELKNMKSGLPTTKSDNFPIPLVKQKGGQYTGFEISSHSDDFIIKIPFGRWQVRKEIDKYRPWEKFDFEQVRKSPKPISLLLSTQRRKRNKGWSKDEGTEAEIRKVMNGDYQTSYIEVKRGGKIGEKSAWMLSLSIDVPKIDKGVDPRIIGGIDVGVKSPLVCAINDAFSRYSISDNDLFHFNKKVFARRRILLKKSKHKRAGHGAKNKLRPITILTEKSRRFRKKLIERWACEIADFFIKNKVGTVQMENLESMKRREDSYFNIRLRGFWPYAEMQNKIEFKLKQYGIEIRKVAPNNTSKTCSKCGHLNNHFNFEYRRKNKFPHFKCEKCNFKENADYNAALNISNPKLKGTKEEP

SEQ ID NO: 3161 - protein, 726 aa, synthetic construct
SEVEFSHEYWMRHALTLAKRARDEREVPVGAILVLNNRVIGVGWNRAIGLHDPTAHAEIMALRQGGLVMQNYRLIDATLYVTFEPCVMCAGAMIHSRIGRVVFGVRNSKHGAAGSLVNVLNYPGMNHRVETTEGILADECAALLCDFYRMPRRVFNARMKAQSSINPGGSSGGSGGSETPGTSESATPESFGGSSGGSAKNTITKTLRLRIVRPYNSAEVEKIVADEKNNREKIALEKNKDKVKEACSKHLKVAAYCTTQVERNACLFCKARRLDDKFYQKLRGQFPDAVFWQEIGEIFRQLQKQAAEIYNQSLIELYYEIFIKGKGIAGASRVGHYLSDVCYTRAAELFKNAAIASGLRSKIKSNFRLKELKNMKSGLPTTKSDNFPIPLVKQKGGQYTGFEISNHNGDFIIKIPFGRWQVKKEIDKYRPWEKFDFEQVRKSPKPISLLLSTQRRKRNKGWSKDEGTEAEIRKVMNGDYQTSYIEVKRGSKIGEKSAWMLSLSIDVPKIDKGVDPSTIGGIDVGVKSPLVCAINNAFCRYSISDNDLFHFNKKMFARRRILLKKSRHKRAGHGAKNKLKPISILTEKSKRFRKKLIERWACEIADFFIKNKVGTVQMENLESLKRKEDSYFNIRLRGFWPYAEMQNKIEFKLKQYGIEIRKVAPNNTSKTCSKCGHLNNYFNFEYRKKNKFPYFKCEKCNFKENADYNAALNISNPKLKSTREEP

SEQ ID NO: 3162 - protein, 726 aa, synthetic construct
SEVEFSHEYWMRHALSLAKRARDEREVPVGAVLVLNNRIIGEGWNRAIGQHDPTAHAEIMALRQGGLVMQNNRLTDATLYVTFEPCVMCAGAMVHSRIGRVVFGVRNSKRGAAGSLMNVLDYPGMGHRVEITEGILADECAALLCDFYCMPRQVFSAQKRAQSSINSGGSSGGSSGSDTPGTSESATPESSGGGSGGSAKNTITKTLQLRIVRPYNSAEVEKIVTDEKNNREKIALEKNKDKVKEACSKHLKMASYCTTQVERNACLFCKARKLDDKFYQKLRGQFPDAVFWQELGGIFRQLQKQTAEIYNQSLIELYYEIFIKGKGFANASSVEHYLSDVCYTRAAELFKNAAIASGLRGKVKSNFRLKELKNMRSGLPTTKSDNFPIPLVKQKGGQYTGFEISSHNDDFIIKIPFGRWQVKKEIDKYRPWEKFDFEQVRKSPKPISLLLSTQRRERNKGWSKDEGTEAEIRKVMNGDYQTSYIEVKRGSKIGEKSAWMLNLSIGVPKIDKGVNPSIIGGIDVGVKSPLVCAINNAFSRYSISDNDLFHFNKKMFARRRILLGKNRHKRAGHGVKNKLKPISILTGKSERFRKKLIERWACEIADFFIKNKVGTVQMENLESMKRKEDSYFNIRLRGFWPYAEMQNKIEFKLKQYGIEIRKVAPNNTSKTCSKCGHLNSYFNFEYRKKNKFPHFKCEKCNFKENADYNAALNISNPRLKSTKEEP

SEQ ID NO: 3163 - protein, 726 aa, synthetic construct
SEVEFSHEYWMRHALTLAKRARDEREVPVGAVLVLNNRVIGEGWNRAIGLHDPTAHAEVMALRQGGLVMQNYRLTDATLYVTFEPCVMCAGAMIHGRIGRVVFGVRNSKHGAAGSLVNVLNYPGMNHRVEITEGILADECAALLCDFYRMPRQVFNARKKAQSSISPGGSSGGSSGSETPGTSESATPESSGGSSGGSAKNTITKTLKLRVVRPYNSAEVEKIVADEKNNREKIALEKNKDKVKEACSKHLKVAAYCTTQVERNACLFCKARKLDDKFYQKLRGQFPDAVFWQEIGEIFRQLQKQAAEIYNQSLIELYYEIFIKGKGFANASSVEHYLSDVCYTRAAELFKNAAIASGLRGKVKSNFRLKELKNMKSGLPTTKSDNFPIPLVKQKGGQYTGFEISSHNDDFIIKIPFGRWQVKEEIDKYRPWEKFDFEQVRKNPKPISLLLSIQRRKRNKGWSRDEGTEAEIRKVMNGDYQTSYIEVKRGSKIGEKSAWMLNLSIDVPKIDKGVDPSIIGGIDVGVKSPLTCAINNAFSRYGISDNDLFRFNKKVFARRRILLKKNRHKRAGHGAKNKLKPISILTEKSKRFRKKLIERWACEIADFFIKNKVGTVQMENLESMTRKEDSYFNIRLRGFWPYAEMQNKIEFKLKQYGIEIRKVAPNNTSKTCSKCGHLNNYFNFEYRKKNKFPHFKCEKCNFKENADYNAALNISNPKLKSTKEEP

SEQ ID NO: 3164 - protein, 725 aa, synthetic construct
SEVEFSHEYWMRHALTLAKRARDEREVPVGAVLVLNNRVIGEGWNRAIGLHDPTAHAEIMALRQGGLVMQNYRLTDATLYVTFEPCVMCAGAMIHSRIGRVVFGVRNSKHGAAGSLVNVLNYPGMNHRVEITEGILADECAALLCDFYRMPRQVFNARKKAQSSINPSGLSGGSSGSVTPGTSESATPESSGGGFGGPAKNTITKTLQLRIVRPYNSAEVEKIVADEKNNREKIALEKNKDKVKEACSRHLKVASYCTTQVERNACLFCKARKLDDRFYQKLRGQFPDAVFWQELGEIFRQLKQAAEIYNQSLIELYYEIFIKGKGLANASSVEHYLSDVCYTRAAGLFKNAAIASGLRGKVKSNFKLKELKSMKSGLPSTKSDNFPIPLVKQRGGQYTGFEISSHNDDFIIKIPFGRWQAKKEIDRYRPWEKFDFEQVRKSPKPISLLLSTQRRKRNKGWSKDEGTEAEIRKVMNGDYQTSYIEVKRGSRIGEKSAWMLSLSIDVPKIDRGVDPSIIGGIDVGVKSPLVCAINNAFSRYSISDNDLFRFNKKMFARRRILLGKNRHKRAGHGVKNKLKPITILTEKSGRFRKKLIERWACEIANFFIKNKVGTVQMENLESMKRREDSYFNIRLRGFWPYAEMQSKIEFKLKQYGIKIRKVAPNNTSKTCSKCGHLNNYFNFEFRKKNKFPHFKCEKCNFKEDADYNAALNISNPKLKGTKEEP

SEQ ID NO: 3165 - protein, 726 aa, synthetic construct
SEVEFSHEYWMRHALTLAKRARDEREVPVGAILVLNNRVIGEGWNRAIGLHDPTAHAEIMALRQGGLVMQNYRLIDATLYVTFEPCVMCAGAMIHSRIGRVVFGVRNNKHGAAGSLVNVLNYPGMNHRVEITEGILADECAALLCDFYRMPRQVFNARKKAQSSINPGGSSGGSSGSETPGTSESATPESSGGSSAGPTKDTITKTLKLRIVRPYNSAVVEKIVADEKNSREKIALEKNKDKVKEACSEHLKVAAYCTTQVERNACLFCKARKLDDGFYQKLRGQFPDAVFWQEIGEIFRQLQRQAAEIYNQSLIELYYEIFIKGKGFANASSVEHYLSDVCYTRAAELFKNAAIASGLRGKVKSNFRLKELKNMRSGLPTTKSDNFPIPLVKQKGGQYTGFEISSHNDDFIIKIPFGRWQVKKETDKYRPWEKFDFEQVRKSPKPISLLLSTRRRKRNKGWSKDEGTEAEIRKVMNGDYQTSYIEVKRGSKVGEKSAWMLNLSIDVPKIDKGVDPGIIGGIDVGVKSPLVCAINNASSRYSISDNDLFRFNKKMFARRRILLGKNRHKRAGHGVKNKLKPITILTEKSGRFRKKLIERWACEIANFFIKNKVGTVQMENLESMKRKEDSYFNNRLRGFWPYAEMQNKIEFKLKQYGIEIRKVAPNNTSKTCSKCGHLNNYFNFEYRKKNKFPPFKCEKCNFKENADYNAALNISNPKLKSTKEES

SEQ ID NO: 3166 - protein, 726 aa, synthetic construct
SEVEFSHEYWMRHALTLAKRARDEREVPVGAILVLNNRVIGEGWNRAIGLHDPTAHAEIMALRQGGLVMQNYRLTDATLYVTFEPCVMCAGAMIHSRIGRVVFGVRNSKHGAAGSLMNVLNYPGMNHRVEITEGILADECAGLLSDFYRMPRQVFSARKKAQSSINPGGSSGGSSGSETPGTSESATPVSSSGGSSGSAKNTITKTLQLRIVRPYNSAEVEKIVADEKNNREKIALEKNKDKVKEACSKHLKVASYCTTQVERNACPFCKARKLDDKFYQKLRGQFPDAVFWQELGEILRQLQKQAAEIYNQGLIELYYEIFIKGRGFANASSVEHYLSDVCYTRAAELFKNAAIASGLRGKVKSNFRLKELKNMKSGLPTTKSDNFPIPLVKQKGGQYTGFEISSHNDDFIIKIPFGRWQVKKEIDKYRPWEKFDFEQVRKSPKPISLLLSTQRRKRNKGWSKDEGTEAEIRKVMNGDYQTSYIEVKRGSKTGEKNAWMLNLSIDVPKIDKGVDPSIIGGIDVGVKSPLVCAINNAFGRYSISDNDLFHYNKKMFARRRILQKKNRHKRAGHGAKNKLKPISILTEKSKRFRKKLIERWACEIADFFIKNRVGTVQMESLESMKRKEDSYFNTRLRGFWPYAEMQNKIEFKLKQYGIKIRKVAPNNTSKTCSKCGHLNDYFSFEYRKKNKFPHFKCEKCNFKESADYNAALNISNPKLMSSKEEP

SEQ ID NO: 3167 - protein, 726 aa, synthetic construct
SEVEFSHEYWMRHALTLAKRARDEREVPVGAILVLNNRVIGEGWNRAIGLHDPTAHAEIMALRQGGLVMQNYRLIDATLYVTFEPCVMCAGAMIHSRIGRVVFGVRNNKHGAAGSLVNVLNYPGMNHRVEITEGILADECAALLCDFYCMPRQVFNAQKRAQSSISSGGSSGGSSGSETPGTSESATPESSGGGSSGSAKNTITKTLQLRIVRPYNSAEVEKIVADEKSNREKIALEKNKDKVKEACSKHLKVAAYCTTQVERNACLFCKARKLDDKFYQKLRGQFPDAVFWQEVGEIFRQLQKQAAEIYNQSLIELYYEIFIKGRGFANASSVEHYLSDVCYTRAADLFKNAAIASGLRGKVKGNFRLKELKNMKSGLPTTKSDNFPIPLVKQKGGQYTGFEISSHNDDFIIKIPFGRWQVKKEIDKYRPWEKFDFEQVRKSPKPISLLLSTQRRKRNKGWSKDEGTEAEIRKVMNGDYQTSYIEVKRGSRIGEKSAWMLCLSIDVPKIDRGVDPSIIGGIDVGVKSPLVCAINNALSRYSISDNDLFRFNKKMFARRRILLGKNRHKRAGHGVKNKLKPITILTEKSGRFRKKLIERWACEIADFFVKNKVGTVQMENLESMKRKEDSYFNIRLRGFWPYAEMQNRIEFKLKQYGIEIRKVAPNNTSKTCSRCGHLNNYFNFEYRKKNKFPHFKCEKCNFKENADYNAALNICNPKLKGTKEEP

SEQ ID NO: 3168 - protein, 726 aa, synthetic construct
SEVEFSHEYWMRHALTLAKRARDEREVPVGAILVLNNRVIGEGWNRAIGLHDPTAHAEIMALRQGGLVMQNYRLIDATLYVTFEPCVMCAGAMIHSRIGRVVFGVRNSKRGAAGSLTNVLDHPGMNHRVEITEGILTDECAALLCDFYRMPHQVLNAQKKTQSSINSGGSSGGSSGRETPVTSGSATPEGSGGSSAGLTKDTITKTLKLRIVRPYNSAEVEKIVADEKNNREKIALEKNKDKVKEACSKHLKVAAYCTTQVERNACLFCKARKLDDKFYQKLRGQFPDAVFWQELGEILRQLQKQAAEIYNQSLIELYYEILIKGRGFANASSVEHYLSDVCYTRAAELFKNAAIASGLRGKVKSNFRLKELKNMKSGLPTTKSDNFPIPLVKQKGGQYTGFEINSHNDDFIIKIPFGRWQVKKEIDKYRPWEKFDFEQVRKGPKPISLLLSTRRRKRNKGWSKDEGTEAEIRKVMNGDYQTSYIEVKRGSKIGEKSAWMLNLSIDVPKIDKGVDPSIIGGIDVGVKSPLVCAINNACSRYSISDNDLFHFNKKMFARRRILLKKNRHKRAGHGAKNKLKPITILTEKSKRFRKKLIERWACEIADFFIKNKVGTVQMENLESMKRKEDSYFNTRLRGFWPYAEMQNKIEFKLKQYGIEIRKVAPNDTSKTCSKCGHLNNYFNFEYRKKNKFPHFKCEKCSFKENADYNAALNISNPKLKSTKEEP

SEQ ID NO: 3169 - protein, 726 aa, synthetic construct
SEVEFSHEYWMRHALTLAKRARDEREVPVGAILVLNNRVIGEGWNRTTGLHDPTAHAEIMALRQGGLVMQNHRLVNATLYVTFEPCVMCAGAMIHSRIGRVVFGVRNSKRGAAGSLTNVLNYPGMNHRVEITEGILVDECAALLCDFYRMPRQVFNAQKKAQSTINSGGSSGGSSGSETPGASGSVIPKSSGGGSSGSAKNTITKALQLRIVRPYNSAEVEKIVADEKNNREKIALEKNKDKVKEACSKHLKVASYCTTQVERNACPFCKARKLDDKFYQKLRGQFPDAVFWQEIGEILRQLQKQAAEIYNQSLVELYYEILIKGKGIANASSVEHYLSDVCYTRAAELFKNAAIASGLRNKIKSNFRLKELRNMRSGLPTTKSDNFPIPLVRQKGGQYTGFEISNHDGDFIIKIPFGRWQVKKEINKHRPWEKFDFEQVRKSPKPISLLLSTQRRKRNKGWSKDEGTEAEIRKVMNGDYQTSYIEVKRGSKIGEKSAWMLNLSIDVPKIDKGVDPGIIGGIDVGVKSPLVCAINNAFSRYSISDNDLFHFNKKMFARRRILLKKNRRKRAGHGAKNKLKPISVLTEKSGRFRKKLIERWACEIADFFIKNKVGTVQMENLGSMKRKEDSYFNIRLRGFWPYAEMQNKIEFKLKQYGIEIRKVAPDNTSKTCSKCGHLNNYFNFEYRKKNKFPHFKCEKCNFKEDADYNAALNISNPKLKSTKEEP

SEQ ID NO: 3170 - protein, 726 aa, synthetic construct
SEVEFSHEYWMRHALTLAKRARDEREVPVGAVLVLNNRVIGEGWNRAIGLHDPTAHAEIMALRQGGLVMQNYRLTDATLYVTFEPCVMCAGAMIHSRIGRVVFGVRNSKRGAAGSLMNVLNYPGMNHCVEITEGILVDECAALLCDFYRMPRQVLTAQKKAQSSISSGGSSGGSSGSETPGASESVTPKSSGGSSAGSTKNTITKTLKLRIVRPYNSAEVEKIVADEKNSREKIALEKNKDKVKEACSKHLKVAAYCTTQVERNACLFCKARKLDDKFYQKLRGQFPDAVFWQETGEIFRQLQRQAAEIYNQSLIELYYEIFIKGKGFANASSVEHYLSDVCYTKAAELFKNAAIASGLRGKVKSNFRLKELKNMKSGLPTTKSDNFPIPLVRQKGGQYTGFEISSHNDDFIIKIPFGRWQVKKEIDKYRPWEKFDFEQVRKSPKPISLLLSTQRRKRNRGWSKDEGTEAEIRRVMNGDYQTSYIEVKRGSKTGEKSAWMLNLSIDVPKIDKGVDPSIIGGIDVGVKSPLVCAINNAFSRYSISDNDLFRFNKKMFARRRILLKKNRHKRAGHGAKNKLKPISILTGKSERFRKKLIERWACEIADFFIKNKVGTVQMENLESMKRKEDSYFNIRLRGFWPYAEMQNKVEFKLKQYGIKIRRVAPNNTSRTCSMCGHLNNYFSFEYRKKNKFPHFKCEKCNFKENADYNAALNISNPKLMSTKEGP

SEQ ID NO: 3171 - protein, 726 aa, synthetic construct
SEVEFGHEYWMRRALTLAKRARDEREVPVGAVLVLNNRVIGVGWNRAVGLHDPTAHAEIMALRQGGLVMQNYRLIEATLYVTFEPCIMCAGAMIHSRIGRVVFGVRNSKRGAAGSLMNVLNYPGMNHRVEITEGILADECAALICDYYRMPRQVLNARRKAQSSINSGGSSDGSSGSETPGTSESATPESSGGSSAGSTKNTITKTLKLRIVRPYNSAEVEKIVADEKNSREKIALEKNKDKVKEACSEHLKVAAYCTTQVERSACLFCKARKLDDRFYQKLRGQFPDAVFWQEISEIFRQLQKQAAEIYNQSLIELYYEIFIKGKGLANASSVEHYLSDVCYTRAAELFKNAAIASGLRNKIKSNFRLKELRNMKSGLPTTKSDNFPIPLVRQKGGQYTGFEISSHNDDFIIKIPFGRWQVKKEINKYRPWEKFDFEQVRKSPKPISLLLSTQRRKRNKGWSKDEGTEAEIRKVMNGDYQTSYIEVKRGSKIGEKSAWMLNLSIDVPKIDKGVDPSIIGGIDVGVKSPLVCAIHNAFSRYSISDNDLFHFNKKVFAKRRILLKKNRHKRAGHGAKNKLKPIFILTEKSERFRRKLIERWACEIADFFIKNKVGTVQMENLESMKRRGDSYFNTRLRGLWPYAEMQNKIEFKLRQYGVKIRKVAPSNTSKTCSKCGHLNNYFNFEYRKKNKFPHFKCEKCNFKENADYNAALNISNPRLKSTKEEP

SEQ ID NO: 3172 - protein, 726 aa, synthetic construct
SEVEFSHEYWMRHALTLAKRARDEREVPVGAVLVLNNRVIGEGWNRAIGLHDPTAHAEIMALRQGGLVMQNYRLIDATLYVTFEPCVMCAGAMIHSRIGRVVFGVRNSKRGAAGSLMNVLNYPGMNHRVEITEGILADECAALLCDFYRMPRQVFNAQKKAQSSINSGGSSGGSSGSETPGTSESATPESSGGSSGGSAKNTITKTLKLRIVRPYNSAEVEKIVADEKNNREKIALEKNKDKVKEACSKHLKVAAYCTTQVERNACLFCKARKLDDEFYQKLRGQFPDAVFWQEISEIFRQLQKQAAEIYNQSLIELYYEIFIKGKGIANASSVEHYLSDVCYTRAAELFKNAAIASGLRSKIKSNFRLKELKNMKSGLPTTKSDNFPIPLVKQKGGQYTGFEISNHNSDFIIKIPFGRWQVKKEIDKYRPWEKFDFEQVQKSPKPISLLLSTQRRKRNKGWSKDEGTEAEIKKVMNGDYQTSYIEVKRGSKIGEKSAWMLNLSIDVPKIDKGVDPSIIGGIDVGVKSPLVCAINNAFSRYSISDNDLFHFNKKMFARRRILLKKNRHKRAGHGAKNKLKPITILTEKSERFRKKLIERWACEIADFFIKNKVGTVQMENLESMKRKEDSYFNIRLRGFWPYAEMQNKIEFKLKQYGIEIRKVAPNNTSKTCSKCGHLNNYFNFEYRKKNKFPHFKCEKCNFKENADYNAALNISNPKLKSTKEEP

SEQ ID NO: 3173 - protein, 726 aa, synthetic construct
SEVEFSHEYWMRHALTLAKRARDEREVPVGAILVLNNRVIGEGWNRAIGLHDPTAHAEIMALRQGGLVMQNYRLIDATLYVTFEPCVMCAGAMIHSRIGRVVFGARNSKRGAAGSLMNVLSYPGMNHRVEITEGILADECAALLCDFYRMPRRVFNAQKKAQSSINSGGSSGGGSSSDTPSTSESTTPESSGGSSGGPAKNTITKTLQLRIVRPYNSAEVEKIVADEKNNREKIALEKNKDKVKEACSKHLKVASYCTTQVERNACPFCKARKLDDKFYQKLRGQFPDAVFWQELGEILRQLQKQAAETYNQSLIELYYEIFIKGRGFANASSVEHYLSDVCYTRAAELFKNAAIASGLRNKIKSNFRLKELKNMKSGLPTTKSDNFPIPLVKQKGGQYTGFEISSHNDDFIIKIPFGRWQVKREIDKYRPWEKFDFEQVRKSPKPISLLLSTQRRKRNKGWSKDEGTEAEIRKVMNGDYQTSYIEVKRGSRTGEKSTWMLNLSIDVPKIDKGVDPSIIGGIDVGVKSPLVCAINNAFSRYSISDNDLFRFNKKMFARRRILLKKNRHKRAGHGAKNKLKPITVLTEKSKRFRKKLIERWACEIVNFFIKNKVGTVQMENLEGMKRKEDSYFNIRLRGLWPYAEMQNKIEFKLKQYGIEIRKVAPNNTSKTCSKCGHLNNYFSFEYRKRNKFPHFKCEKCNFKENADYNAALNISNPKLKGTKEEP

SEQ ID NO: 3174 - protein, 726 aa, synthetic construct
SEVEFSHEYWMRHALTLAKRARDEREVPVGAILVLNNRVIGEGWNRAIGLHDPTAHAEIMALRQGGLVMQNYRLTDATLYVTFEPCVMCAGAMIHSRIGRVVFGVRNSKRGAAGSLMNVLNYPGMNHCVEITEGILVDECAALLCDFYRMPRQVLNAQKKAQSSVSSGGSSGGSSCSETPGASESVTPKSSGGGSAGSTKNTITKTLQLRIVRPYNSAEVEKIVADEKNSREKIALEKNKDKVKEACSKHLKVAAYCTTQVERNACLFCKARKLDDKFYQKLRGQFPDAVFWQEIGEIFRQLQKQAAEVYNQSLVELYYEILIKGKGIANASSVEHYLSDVCYTRAAELFKNAAIASGLRNKIKSNFRLKELRNMKSGLPTTKSDNFPIPLVRQKGGQYTGFEISNHNSDFIIKIPFGRWQVKKEIDKYRPWEKFDFEQVRKNPKPISLLLSTQRRKRNKGWSKDEGTEAEIRKVMNGDYQTSYIEVKRGSKIGEKSAWMLSLSIDVPKIDRGVDPSIIGGIDVGVKSPLVCAINNALSRYSISDNDLFHFNKKMFARRRILLKKNRHRRAGHGARNKLKPITVLTEKSKRFRKKLIERWACEIANFFIKNKVGTVQMENLESMKRKEDSYFNIRLRGLWPYAEMQNKIEFKLKQYGIEVRKVAPNNTSKTCSKCGHLNDYFNFEYRKRNKFPHFKCEKCNFKENADYNAALNISNPKLKGTKEEP

SEQ ID NO: 3175 - protein, 726 aa, synthetic construct
SEVEFSHEYWMRHALTLAKRARDEREVPVGAVLVLNNRVIGEGWNRAIGLHDPTAHAEIMALRQGGLVMQNYRLVDATLYVTFEPCVLCAGAMVHSRIGRVVFGVRNSKRGAAGSLMNVLNYPGMNHRVEITEGILADECAALLCDFYRMPRQVFNARKKARSNINSGGSSGGSSGSETLGTREGATPESSGGSSGGSAKNTITKTLKLRIVRPYNSAEVEKIVVDEKNNREKVALEKNKDKVKEACSKHLKVAAYCTTQVERNACLFCKARKLDDKFYQKLRGQFPDAVFWQEIGEIFRQLQKQAAEIYNQSLIELYYEIFIKGKGFANACSVEHYLSDVCYTRAAELFKNAAIASGLRGKVKSNFRLKELRNMKSGLPTTKSDNFPIPLVRQKGGQYTGFEISSRNDDFIIKIPFGRWQVKKEVDKYRPWEKFDFEQVRKSPKPISLLLSTQRRKRNRGWGKDEGTEAEIKRVMNGDYQTSYIEVKRGSKIGEKSAWMLNLSIDVPKIDKGVDPRIIGGIDVGVKSPLVCAINNAFSRYSVSDNDLFHFNKKMFARRRILLKKNRHKRAGHGAKNKLKPITILTEKGVRFRKKLIERWACEIADFFIKNKVGTVQMENLESMKGKEDSYFNIRLRGFWPYAEMQNKIEFKLKQYGIEIRKVAPNNTSKTCSKCGHLNNYFNFEYRKKNKFPHFKCERCNFKENADYNAALNISNPKLKSTKEEP

SEQ ID NO: 3176 - protein, 726 aa, synthetic construct
SEVEFSHEYWMRHALTLAKRARDEREVPVGAVLVLNNRVIGEGWNRAIGLHDPTAHAEIMALRQGGLVMQNYRLTDATLYVTFEPCVMCAGAMVHSRIGRVVFGVRNSKRGAAGSLMNVLNYPDMNHCVEITEGILVDECAALLCDFYRMPRQVLNSQKKAQSSIGSGGSSGGSSGSETPGTSESATPESSGGSSGGSAKNTITKTLKLRIVRPYNSAEVEKIVDDEKNNREKIALEKNKDKVKEACSKHLKVAAYCTTQVERNACLFCKARKLDDKFYQRLRGQFPDAVFWQEIGEIFRQLQKQAAEVYNQSLVELYYEILIKGKGIANASSVEHYLSDVCYTRAAELFKNAAIASGLRGKVKSNFRLKELKNMKSGLPTTKSDNFPIPLVKQKGGQYTGFEISSHNSDFIIKIPFGRWQEKEEIDKYRPWEKFDFEQVRKNPKPISLLLSIQRRKRNKGWSRDEGTEAEIRKVMNGDYQTSYIEVKRGSKIGEKSAWMLNLSIDVPKIDKGVDPSIIGGIDVGVKSPLICAIYNAFSRYGISDNDLFRFNKKVFARRRILLKKNRHKRAGHGTKNKLKPITILTEKSGRFRKKLIERWACEIANFFIKNKVGTVQMENLESMKRKEDSYFNIRLRGFWPYAEMQNKIEFKLKQYGIVVRKVAPNNTSKTCSKCGHLNNYFNFEYRKKNKFPHFKCEECNFKENADYNAALNISNPKLKSAKEEP

SEQ ID NO: 3177 - protein, 726 aa, synthetic construct
SEVEFSHEYWMRRALTLAKRARDEREVPVGAVLVLNNRVIGGGWNRAIGLHDPTAHAEIMALRQGGLVMQNYRLTDATLYVTFEPCVMCAGAMIHSRIGRVVFGVRNSKRGAAGSLTNVLNYPGMNHRVEITEGILVDECAALLCDFYRMPRQVFNAQRKAQSTINSGGSSDGSSGSETPGTSESATPESSGGGSSGSAKNTITKTLQLRIVRPYNSAEVEKIVADEKNNREKIALEKNKDKVREACSKHLKVASYCTTQVERNACPFCKARKLDDKFYQKLRGQFPDAVFWQELGEILRQLQKQAAEIYNQSLIELYYEIFIKGKGFANASSVEHYLSDVCYSRAAELFKNAAIASGLRSKVRSNFRLKELKSMKSGLPTTKSDNFPIPLVKQKGGQYTGFEIRSHNSDFIIKIPFGRWQAKKEINKFRPWEKFDFEQVRKSPKPISLLLSTQRRKRNKGWSRDEGTEAEIRKVMNGDYQTSYIEVKRGSKIGEKGAWMLNLSIDVPKIDKGVDPSIIGGIDVGVKSPLVCAINNALSRYSISDNDLFHFNKKMFARRRILLKKNRHRRAGHGARNKLKPIAVLTEKSKRFRKKLIERWACEIANFFIKNKVGTVQMENLESMKRKEDSYFNIRLRGFWPYAEMQNKIEFKLRQYGIEIRKVAPSNTSKTCSKCGHLNNYFNFEYRKKNKFPYFKCEKCNFKENADYNAALNISNPKLKSTKEEP

SEQ ID NO: 3178 - protein, 726 aa, synthetic construct
SEVEFSHEYWMRHALTLAKRARDEREVPVGAVLVLNNRVIGEGWNRAIGLHDPTAHAEIMALRQGGLVMQNYRLIDATLYVTFEPCVMCAGAMVHSRIGRVVFGVRNSKRGAAGSLMNVLDYPGMGHRVEITEGILADECAALLCDFYCMPRQVFNAQRRAQSSINSGGSSGGSSGSDMPGTSESATPESSGGSSGGSAKNTITKTLKLRIVRPYNSAEVEKIVADEKNNREKVALEKNRDKVKEACSEHLKVAAYCTTQVERNACLFCKARKLDDKFYQKLRGQFPDAVFWQEIGEIFRQLQKQAAEIYNQSLIELYYEIFIKGKGFANASSVEHYLSDVCYTRAAELFKNAAIASGLRGKVKGNFRLKELKNMKSGLPTTKSDNFPIPLVKQKGGQYTGFEISSHNDDFIIKIPFGRWQVKKEIDKYRPWEKLDFEQVRKSPKPISLLLSTQRRKRNRGWSKDEGTEAEVKKVMNGDYQISYIEVKRGSKIGEKSAWTLNLSIDVPKIDKGVDPSIIGGIDVGVKSPLVCAISNAFSRYSISDNDLFHFNKKMFARRRILLKKSKHKRAGHGAKNKLKPITILTEKSKRFRKKLIERWACEIADFFIKNKVGTVQMENLESMKRKEDSYFNIRLRGFWPYAEMQNKIEFKLRQYGIEIRKVAPNNTSRTCSKCGHLNNYFNFEYRRKNKFPLFKCEKCNFKEDADYNAALNISNPKLKSTKEEP

SEQ ID NO: 3179 - protein, 726 aa, synthetic construct
SEVEFSHEYWMRHALTLAKRARDEREVPVGAVLVLNNRVIGEGWNRATGLHDPTAHAEIMALRQGGLVMQNYRLFDATLYVTFEPCVMCAGAMIHSRIGRVVFGVRNNKHGAAGSLVNVLNYPGMNHRVEITEGILADECAALLCDFYRMPRQVFNARRKAQSSINPGGSSGGSSGSETLGTSESATPESSGGSSGASAKNTITKALKLRIVRPYNSAEVEKIVADEKNNREKIALEQNKDKVREACSKHLKVAAYCTTQVERNACLFCKARRLDDKFYQKLRGQFPDAVFWQEIGEIFRQLQKQAAEIYNQSLVELYYEIFIKGKGIANASSVEHYLSDVCYTGAAELFKNAAIASGLRNKIKSNFRLKELRNMKSGLPTTKSDNFPIPLVKQKGGQYTGFEISNHNDDFIIKIPFGRWQVKKEIDRYRPWEKFDFEQVRKSPKPISLLLSTQRRKRNKGWSKDEGTEAEIRKVMNGDYQTSYIEVKRGSKTGEKSAWMLNLSIDVPKIDKGVDPSIIGGIDVGVKSPLVCAINNAFSRYSISDNDLFRFNKKMFARRRILLKKNRHKRAGHGAKNKLKPISILTGKSERFRKKLIERWACEIADFFIKNKVGTVQMENLEGMKRKEDSYFNIRLRGFWPYAEMQNKIEFKLKQYGIEIRKVAPNNTSKTCSKCGHLNNYFNFEYRRKNKFPHFKCEKCNFKENADYNAALNISNPKLKSTKEEP

SEQ ID NO: 3180 - protein, 726 aa, synthetic construct
SEDEFSHEYWMRHALTLAKRARDGREVPVGAVLVLNNRVIGVGWNRAIGLHDPTAHAEIMALRQGGLVMQNYRLIDATLYVTFEPCVMCAGAMVHSRIGRVVFGVRNSKRGAAGSLMNVLDYPGMGHRVEITEGILADECAALLCDFYCMPRQVFNAQKRAQPSINSGGSSGGGSSSDTPSTSESTTPESSGGSSGGPAKNTITKTLKLRIVRPYNSAEVEKIVADEKNNREKTALEKNKDKVKEACSKHLKVAAYCTTQVERNACLFCKARKLDDKFYQKLRGQFPDAVFWQEVGEIFRQLQKQAAEIYNQSLIELYYEIFIKGKGFANASSVEHYLSDVCYTRAAELFKNAAIASGLRGKVKSNFRLKELKNMKSGLPTTKSDNFPIPLVKQKGGQYTGFEISNRNSDFIIKIPFGRWQVKKEINKYRPWEKFDFEQVRKSPKPISLLLSTQRRKRNKGWSKDEGTEAEIRKVMNGDYQTSYIEVKRGSRIGEKSAWMLSLSIDVPKIDRGVDPSIIGGIDVGVKSPLVCAINNALSRYSISDNDLFHFNKKMFARRRILLKKNGHKRAGHGAKNKLKPITIMTEKSKRFRKKLIERWACEIADFFIKNKVGTVQMENLESMKRKEDSYFNIRLRGFWPYAEMQNKIEFKLKQYGIVVRKVAPNNTGKTCSQCGHLNNYFNFEYRKKNKFPYFKCEKCNFKENADYNAALNISNPQLKSTKGEP

SEQ ID NO: 3181 - protein, 726 aa, synthetic construct
SEVEFSHEYWMRHALTLAKRARVEREVPVGAVLVLNNRVIGEGWNRAIGLHDPTAHAEIMALRQGGLVMQNYRLTDATLYVTFEPCVMCAGAMIHSRVGRVVFGVRNSKRGAAGSLMNVLNYPGMNHCVEITEGILVDECAALLCDFYRMPRQVLNARKKAQSSINPGGSSGGSSGSETPGTSESATPESSGGSSGGSAKNTITKTLKLRIVRPYNSAEVEKIVADEKNNREKIALKKNKDKVREACSKHLKVAAYCTTQVERSACLFCKARRLDDKFYQKLKGQFPDAVFWQEIGEIFRQLQKQAAEIYNQSLIELYYEIFIKGKGIANASSVEHHLSDVCYTRAAELFKNAAIASGLRNKIKSNFRLKELRNMKSGLPTTRSDNFPIPLVKQKGGQYTGFEISNHNGDFIIKIPFGRWQAKKEIDKYRPWEKFDFEQVRKSPKPISLLLSTQGRKRNRGWSKDEGTEAEIRKVMNGDYQASYIEVKRGSKIGEKSAWMLNLSIDVPKIDKGVDPSIIGGIDVGVKSPLVCAVNNAFSRYSISDNDLFHFNKKVFARRRILLKKNRHRRAGHGAKNKLKPITILTEKSKRFRKKLIERWACEIADFFIKNKVGTVQMENLESMKRKEDSYFNIRLRGFWPYAEMQNKIEFKLKQYGIKIRKVAPNNTSRTCSKCGHLNNYFSFEYRKKNKFPHFKCEKCNFKEDADYNAALNISNPKLKGTKGEL

SEQ ID NO: 3182 - protein, 726 aa, synthetic construct
SEVEFSHEYWMRHALTLAERARDAREVPVGAILVLNNRVIGEGWNRAIGLNDPTVHAEIMALRQGGLVMQNHRLIDATLYVTFEPCVMCAGAMIHSRIGRVVFGVRNSKHGAAGSLVNVLNYPGMNHRVEITEGILADECAALLCDFYRMPRQVFIAQKKAQSSINPGGSSGGSSGSETPGTSESATPGSSGGGSSGSAKNTITKTLQLRIVRPYNSAEVEKIVADEKNNREKIALEKNKDKVKEACSKHLKVASYCTTQVERNACPFCKARKLDDKFYQKLRGQFPDAVFWQEIGEVFRQLQKQAAEIYNQSLIELYYEIFIKGRGFANASSVEHYLSDVCYTRAAELFKNAAIASGLRGKVKSNFRLKELKNMKSGLPTTKSDNFPIPLVKQKGGQYTGFEISSHNDDFIIKIPFGRWQVKKEIDRYRPWEKFDFEQVRKSPKPISLLLSTRRRKRNKGWSKDEGTEAEIRRVMNGDYQTSYIEVKRGSKIGEKSAWMLSLSIDVPKIDKGVDPRIIGGIDVGVKSPLVCAINNVPSRYSISDNDLFHYNKKMFARRRILLKKNRHRRAGHGAKNKLKPISILTEKSERFRKKLIERWACEIADFFIKNKVGTVQMENLESMKRREDSYFNIRLRGFWPYAKMQNKIEFKLKQYGIKIRKVAPNNTSKTCSKCGHLNNYFSFEYRKKNKFPHFKCEKCNFKESADYNAALNISNPKLKSTKGEP

SEQ ID NO: 3183 - protein, 725 aa, synthetic construct
SEVEFSHEYWMRHALTLAKRARDEREVPVGAVLVLNNRVIGEGWNRAIGLHDPTAHAEIMALRQGGLVMQNYRLVDATLYVTFEPCVLCAGAMVHSRIGRVVFGVRNSKRGAAGSLMNVLNYPGMNHRVEITEGILADECAALLCDFYRMPRQVFNARKKARSNINSGGSSGGSSGSETLGTREGATPESSGGSSGGSAKNTITKTLKLRIVRPYNSAEVEKIVADEKNNREKVALEKNKDKVKEACSEHLKVAAYCTTQVERSACLFCKARKLDDKFYQKLRGQFPDAVFWQEVGEIFRQLQKQAAEIYNQSLIELYYEIFIKGKGFANASSVEHYLSDVCYTRAAELFKNAAIASGLRGKVKSNFRLKELKNMKSGLPTTKSDNFPIPLVKQKGGQYTGFEISNHNSDFIIKIPFGRWVKKEINKYRPWEKFDFEQVRKSPKPISLLLSTQRRKRNKGWSKDEGTEAEIRKVMNGDYQTSYIEVKRGSKTGEKSAWMLNLSIDVPKIDKGVDPSIIGGIDVGVKSPLVCAINNAFSRYSISDNDLFHFNKKMFARRRILLKKSRHKRAGHGAKNKLKPISILTEKSKRFRKKLIERWACEIADFFIKNKVGTVQMENLESMKRKEDSYFNIRLRGFWPYAEMQNKIEFKLKQYGIEIRKVAPNNTSKTCSKCGHLNNYFNFEYRKKNKFPHFKCEKCNFKENADYNAALNISNPRLKSTKEEP

SEQ ID NO: 3184 - protein, 726 aa, synthetic construct
SEVEFSHEYWMRRALTLAKRARDEREVPVGAILVLNNRVIGEGWNRAIGLHDPTAHAEITALRQGGLVMQNYRLIDATLYVTFEPCVMCAGAMIHSRIGRVVFGVRNNKHGAAGSLVNVLNYPGMNHRVEITEGVLADECAALLCDFYRMPRQVFNARKKAQSSINPGGSSGGSSGSETPGTSESATPESSGGSSGGSAKNTITKTLKLRIVRPYNSAEVERILADEKDNREKIALERNKDKVKEACSKHLKVAAYCTTQVERNACLFCRARKLDDKFYQKLRGQFPDAVFWQEIGEIFRQLQKQAAEIYNQSLIELYYEIFIKGKGFANASSVEHYLSDVCYTRAAELFKNAAIASGLRGKVKSNFRLKELKNMKSGLPTTKSDNFPIPLVRQKGGQYTGFEISSHNDDFIIKIPFGRWQVRKEIDKYRPWEKFDFEQVRKSPKPISLLLSTQRRKRNKGWSKDEGTEAEIRKVMNGDYQTSYIEVKRGSKTGEKSAWMLNLSIDVPKIDKGVDPSVIGGIDVGVKSPLVCAINNAFSRYSISDNDLFHFNKKMFARRRILLKKNRHKRAGHGAKNKLKPITILTEKSVRFRKKLIERWACEIADFFIKNKVGTVQMENLESMKGKEDSYFNIRLRGFWPYAEMQNKIEFKLKQYGIEIRKVAPNNTSKTCSKCGHLNNYFNFEYRKKNKFPHFKCEKCNFKENADYNAALNISNPMLKSTKEEP

SEQ ID NO: 3185 - protein, 726 aa, synthetic construct
SEVEFSHEYWMRHALTLAKRARDEREVPVGAVLVLNNRVIGEGWNRAIGLHDPTAHAEIMALRQGGLVMQNYRLINATLYVTFEPCAMCAGAMVHSRIGRVVFGVRNSKRGAAGSLMNVLNYPGMDHRVEITGGILADECAALLCDFYRMPRRVFNAQKKAQSSINSGGSSGGSSGSVTPGTSESATPESSGGSFGGSAKNTITKTLQLRIVRPYNCAEVEKIVADEKNNREKIALEKNKDKVKEACSKHLKVAAYCTTQVERNACLFCRARKLDDKFYQKLRGQFPDAVFWQEIGEIFRQLQRQAAEIYNQSLIELYYEIFIKGKGFANASSAEHYLSDVCYTRAAELFKNAAIASGLRGKVKSNFRLKELKNMKSGLPTTKSDNFPIPLVKQKGGQYTGFEISSHNDDFIIKIPFGRWQVKEEIDKYRPWEKFDFEQVRKSPKPISLLLSTQRRKRNKGWSKDEGTEAEIRKVMNGDYQTSYIEVKRGSKIGEKSAWMLNLSIDVPKIDKGVDPSIIGGIDVGVKSPLVCAINNAFSRYSISDNDLFHFNKKMFARRRILLKKNRHKRAGHGAKNKLKPISILTEKSKRFRKKLIERWACEIADFFIKNKVGTVQMENLESMKRKEDSYFNIRLRGFWPYAEMQNKVEFKLKQYGIEIRKVAPNNTSKTCSKCGHLNNYFNFEYRRRNKFPHFKCEKCNFKENADYNAALNISNPKLKSTKEEP

SEQ ID NO: 3186 - protein, 726 aa, synthetic construct
SEVEFSHEYWMRHALTLAKRARDEREVPVGAILVLNNRVIGEGWNRAIGLHDPTAHAEIMAMRQGGLVLQNYRLIDATLYVTFEPCVMCAGAMIHSRIGRVVFGVRNNKHGAAGSLVNVLNYPGMNHRVEITEGILADECAALLCDFYRMPRQVFNARKKAQSSISSGGSSGGSSGSETPGTSESATPESSGGSSGGSAKNTITKTLKLRIVRPYNSAEVEKIVADEKNNREKIALEKNKDKVKEACSKHLKVAAYCTTQVERNACLFCKARRLDDKFYQKLRGQFPDAVFWQEIGEIFRQLQKQAAEIYNQSLIELYYEIFIRGKGTANASSVEHYLSDVCYTRAAELFKNAAIASGLRSKIKSNFRLKELRNMKSGLPTTKSDNFPIPLVKQKGGQYTGFEISSHNDDFIIKIPFGRWQVKKEIDKYRPWEKFDFEQVRKSPKPISLLLSTQRRKRNKGWSKDEGTEAEIRKVMNGDYQTSYIEVKRGSKIGEKSAWMLSLSIDVPKIDKGVDPSTIGGIDVGVKSPLVCAINNAFCRYSISDNDLFHFNKKMFARRRILLKKSRHKRAGHGAKNKLKPISILTERSKRFRKKLIERWACEIADFFIKNKVGTVQMENLESMKRKEDSYFNIRLRGFWPYAEMQNKIEFKLKQYGIEIRKVAPNNTSKTCSKCGHLNSYFNYEYRKKNKFPHFKCEKCNFKENADYNAALNISNPKLKSTKGEP

SEQ ID NO: 3187 - protein, 726 aa, synthetic construct
SEVEFSHEYWMRHALTLAKRARDGREVPVGAVLVLNNRVIGEGWNRAIGLHDPTAHAEIMALRQGGLVMQNYRLIDATLYVTFEPCVMCAGAMVHSRIGRVVFGVRNSKRGAAGSLMNVLDYPGMGHRVEITEGILADECAALLCDFYCMPRQVFNAQKRAQSSINSGGSSGGSSGSETPGTSESATPESPGGGSSGSAKNTVTKALKLRIVRPYNSAEVEKIVADEKNNREKIALEKNKDKVKEACSEHLKVAAYCTTQVERNACLFCKARKLDDKFYQKLRGQFPDAVFWQELGEIFRQLQKQAAEIYNQSLIELYYEIFIKGKGFANASSVEHYLSDVCYTRAAELFKNAAIASGLRGKVKSNFRMKELKNMKSGLPTTKSDNFPIPLVKQKGGQYTGFEISSHNDDFIIKIPFGRWQVKKEIDKYRPWEKFDFEQVRKSPKPISLLLSTQRRKRNKGWSKDEGTEAEIRKVMNGDYQTSYIEVKRGSKIGEKSAWMLNLSIDVPKIDKGVDPSIIGGIDVGVKSPLVCAINNAFGRYSISDNDLFHYNKKMFARRRILQKKNRYKRAGHGAKNKLKPISILTEKSKRFRKKLIERWACEIADFFIKNKVGTVQMENLESMKRKEDSYFNTRLRGFWPHAEMQNKIEFKLKQFGIEIRKVAPNNTSKTCSKCGHLNNYFNFEYRKKNKFPPFKCEKCNFKENADYNAALNISNPKLKGTKEEP

SEQ ID NO: 3188 - protein, 726 aa, synthetic construct
SEVEFSHEYWMRHALTLARRARDEREVPVGAILVLNNRVIGEGWNRAIGLHDPTAHAEIMALHQGGLVMQNYRLIDATLYVTFEPCVMCAGAMIHSRIGRVVFGARNSKRGAAGSLMNVLSYPGMNHRVEITEGILADECAALLSDFYRMPRRVFNAQKKAQSSINSGGSSGGSSGSETPGTSESATPKSSGGSSGGSAKNTITKALKLRIVRPYNSAEVEKIVADEKNNRERIALEKNKDKVKEACSKHLKVAAYCTTQVERNACLFCKARKLDDKFYQKLRGQFPDAVFWQEIGEIFRQLQKQAAEIYNQSLIELYYEIFIEGKGSANARSVEHYLSDVCYTRAAELFKNAAIASGLRGKVKGNFRLKELKSMKSGLPTTKSDNFPIPLVKQKGGQYTGFEISSHNDDFIIKIPFGRWQVKKEIDKYRPWEKFDFEQVRKSPKPISLLLSTQRRKRNKGWSKDEGTEAEIRKVMNGDYQTSYIEVKRGSKIGEKSAWMLNLSIDVPKIDKGVDPSITGGIDVGVKSPLVCAINDALSRYSISDNDLFHFNKKMFARRRILLKKNRHKRAGHGAKNKLKPLTILTGKSKRFRKKLIERWACEIAGFFIKNKVGTVQMENLESMKRREDSYFNIRLRGFWPYAEMQNKIEFKLKQYGIEIRKVAPNNTSKTCSRCGHLNNYFNFEYRKRNKFPHFKCEKCNFKENADYNAALNISNPRLKSPKEEP

SEQ ID NO: 3189 - protein, 726 aa, synthetic construct
SEVEFSHEYWMRHALTLARRARDGREVPVGAVLVLNNRVIGEGWNRAIGLHDPTAHAEIMALRQGGLVMQNYRLIDATLYVTFEPCVMCAGAMVHSRIGRVVFGVRNSKRGAAGSLMNVLNYPGMDHRVEITGGILADECAALLCDFYCMPRQVFNAQKRTQSSINSGGSSGGSSGSETPGTSESATPKSSGGSSGGSAKNTITKALKLRIVRPYNSAEVEKIVADEKNNRERIALEKNKDKVKEACSKHLKVAAYCTTQVERNACLFCKARELDDKFYQKLRGQFPDAVFWQEIGEIFRQLQKQAAEIYNQSLIELYYEIFIKGKGFANASSVEHYLSDVCYTRAAELFKNAAIASGLRGKVKSNFRLKELKNMKSGLPTTKSDNFPIPLVKQKGGQYTGFEISSHNDDFIIKIPFGRWQVKKEIDKYRPWEKFDFEQVRKSPKPISLLLSTQRRKKNKGWSRDEGTEAEIKKVMNGDYQTSYIEVKRGNKIGEKSAWMLNLSIDVPKIDKGVDPSIIGGIDVGVKSPLVCAISNAFSRYSISDNDLFHFNKKMFARRRILLKKSKHKRAGHGAKNKLKPITILTEKSRRFRKKLIERWACEIADFFIKNKVGTVQMENLESMKRREDSYFNIRLRGFWPYAEMQNKIEFKLKQYGIEIRKVAPNNTSKTCSKCGHLNNYFNFEYRKKNKFPHFKCEKCNFKENADYNAALNISNPKLKGTKEEP

SEQ ID NO: 3190 - protein, 726 aa, synthetic construct
SEVEFSHEYWMRHALTLAKRARDEREVPVGAVLVLNNRVIGEGWNRAIGLHDPTAHAEIMALRQGGLVMQNYRLIDATLYVTFEPCVMCAGAMVHSRIGHVVFGVRNSKRGAAGSLMNVLDYPGMGHRVEITEGILADECAALLCDFYCMPRQVFNAQKRAQSSINSGGSSGGSCGSDTPGTSGSATPESSGGGSSGSAKNTITKTLQLRIVRPYNSAEVEKIVADEKNNREKIALEKNKDKVREACSKHLKVASYCTTQVERNACPFCKARKLDDKFYQKLGGQFPDAVFWQELGEILRQLQKQAAEIYNQSLIELYYEIFIKGRGFANAGSVEHYLSDVCYTRAAELFKNAAIASGLRGKVKSNFRLKELKNMKSGLPTTKSDNFPIPLVKQKGGQYTGFEISSHNDDFIIKIPFGRWQVKKEIDKYRPWEKFDFEQVRKSPRPISLLLSTQRRKRNKGWSKDEGTEAEIRKVMNGDYQTSYIEVKRGSKIGEKSAWMLNLSIDVPKIDMGVDPSIIGGIDVGVKSPLVCAIDNAFSRYSISDNDLYHFNKKMFAKRRILLKKNRHKRTGHGAKNKLKPITILTGKSERFRKKLIERWACEIADFFIKNKVGTVQMENLESMKRKEDSYFNIRLRGFWPYAEMQNKIEFKLKQYGIEIRKVAPNNTSKTCSKCGHLNNYFSFEYRKKNKFPHFKCEKCNFKENADYNAALNISNPKLKSTKEEP

SEQ ID NO: 3191 - protein, 726 aa, synthetic construct
SEVEFSHEYWMRHALTLAKRARDEREVPVGAILVLNNRVIGEGWNRAIGLHDPTAHAEIMALRQGGLVMQNYRLIDATLYVTFEPCVMCAGAMIHSRIGRVVFGVRNNKHGAAGSLVNVLNYPGMNHRVEITEGILADECAALLCDFYRMPRQVFNARKKAQSSINPGGSSGGSSGSETPGTSENATPESSGGSSGSSAKNTITKTLKLRIVRPCNSAEVEKIVADEKNNREKIALEKNKDKVKEACSKHLKVADYCTTQVERNACLFCKARRLDDKFYQKLRGQFPDAVFWQEIGEIFRQLQKQAAEIYNQSLIELYYEIFIKGKGFANASSVEHYLSDVCYTRAAELFKNAAIASGLRSKVRSNFRLKELKNMKSGLPTTKSDNFPIPLVKQKGGQYTGFEISSHNDDFIIKIPFGRWQVKKEINKFRPWEKFDFEQVRKSPKPLSLLLSTQRRKRNKGWSRDEGTEAEIRKVMNGDYQTSYIEVKRGSKIGEKSAWMLNLSIDVPKIDKGVDPSIIGGIDVGVKSPLVCAINNAFSRYSISDNDLFHFNKKMFARRRILLKKTRHKRAGHGAKNKLKPISILTEKSERFRKKLIERWACEIADFFIKNKVGTVQMENLESMKRREDSYFNIRLRGFWPYAKMQNKIEFKLKQYGIEIRKVAPNNTSKTCSKCGHLNNYFNFEYRKKNKFPHFKCEKCNFKESADYNAALNISNPKLKSTKEEP

SEQ ID NO: 3192 - protein, 725 aa, synthetic construct
SEVEFSHEHWMRHALALAKRARDEREVPVGAVLVLNNRAIGEGWNRAIGLHDPTAHAEIMALRQGGLVMQNYRLVNATLYVTFEPCVMCAGAMIHSRIGRVVFGVRNGKRGAAGSLMNVLNYPGMNHRVEITEGILADECAALLCDFYRMPRQVFNARKKAQSSINPGGPSGGSSGSKTPGTSESATPEGSGGSSGGSAKNTITKTLKLRIVRPYNSAEVEKIVADEKNNREKIALEKNRDKVKEACSKHLKVAAYCTTQVERNACLFCKARKLDDKFYQKLRGQFPDAVFWQEIGEIFRQLQKQAAEIYNQSLIELYYEIFIKGRGFANASSVEHYLSDVCYTRAAELFKNAAIASGLRNKIKSNFRLKELRNMKSGLPTTKSDNFPIPLVRQKGGQYTGFEISNHDGDFIIKIPFGRWQVKKEINKHRPWEKFDFEQVRRSPKPISLLLSTQRRKRNKGWSKDEGTEAEIRKVMNGDYQTSYIEVKRGSKTGEKSAWMLNLSIDVPKIDKGVDPSIIGGIDVGVKSPLVCAINNSSSRYSICDNDLFRFNKKMFARRRILLKKNRHKRAGHGAKNKLKPITILTKKSERFRKKLIERWVCEVADFFIKNKVGTVQMENLESMKRKEDSYFNIRLRGFWPYAEMQNRIELKLKQYGIEIRRVAPNNTSRTCSKCGHLNNYFNFEYRKKNKFPHFKCEKCNFKENADYNAALNISNPKLKSTEGP

SEQ ID NO: 3193 - protein, 726 aa, synthetic construct
SEVEFSHEYWMRHALTLAKRARDAREVPVGAILVLNNRVIGEGWNRAIGLHDPTAHAEIMALRQGGLVMQNYRLIDATLYVTFEPCVMCAGAMIHSRIGRVVFGVRNSKHGAAGSLMNVLNYSGMNHRVEITEGILADECAALLCDFYRMPRQVFNGRKKAQSSINSGGSSGGSSGSETPGTSESATPESSGGSSGGSAKNTITKTLKLRIVRPYNSAEVEKIVADEKNNREKIALEKNKGKVKEACSKHLEVAAYCTTQVERNACLFCRARKLDDKFYQKLRGQFPDAVFWQELGEIFRQLQKQAAEIYNQSLIELYYEIFIKGKGFANASSVEHYLSDVCYTRAAELFKNAAIASGLRGKVKSNFRLKELKNMKSGLPTTKSDNFPIPLVKQKGGQYTGFEISSHNDDFIIKIPFGRWQVKKEIDKYRPWEKFDFEQVRKSPKPISLLLSTQRRKRNKGWSKDEGTEAEIRKVLNGDYQTSYIEVKRGSKIGEKSAWMLNLSIDVPKIDKGVDPSIIGGIDVGVKSPLVCAINNAFSRYSISDNDLFHFNKKMFARRRILLKKNRHKRDGHGARNKLKPITVLAEKSERFRKKLIERWACEIANFFIKNKVGTVQMENLESMKRKEDSYFNIRLRGFWPYAEMQDKIEFKLKQYGIEIRKVAPNNTSKTCSRCGHLNNYFNFEYRRKNKFPHFKCEKCNFKENADYNAALNISNPKLKSTKEEP

SEQ ID NO: 3194 - protein, 726 aa, synthetic construct
SEVEFSHEYWMRHALTLAKRARDEREVPVGAVLVLNNRVIGEGWNRAIGLHDPTAHAEIMALRQGGLVMQNYRLIDATLYVTFEPCVMCAGAMIHSRIGRVVFGVRNNKHGAAGSLVNVLNYPGMNHRVEITEGILADECAALLCDFYRMPRQVFNARKKAQSSINPGGSSGGSGGSETPGTSESATPESSGGSSGSSAKNTITKTLKLRIVRPYNSAEVEKIVADEKNNRERIALEKNKDKVKEACSKHLKVAAYCTTQVGRNACLFCKARRLDDKFYQKLRGQFPDAVFWQEIGEIFRQLQKQAAEVYNQSLVELYYEILIKGKGFANASSVEHYLSDVCYTRAAELFKNAAIASGLRGKIKSNFRLKELRNMKSGLPTTKSDNFPIPLVKQKGGQCTGFEISNHNSDFIIKIPFGRWQVKKEIDKYRPWEKFDFAQVRKSPKPISLLLSTQRRKRNRGWSKDESTEAEIRKVMNGDYQSSYIEVKRGSKIGEKSAWMLNLSIDVPKIDKGVDPSIIGGIDVGVKSPLVCAINNAFSRYSISDNDLFHFNKKMFARRRILLKKNRHKRAGHGAKNKLKPISILTEKSKRFRKKLIERWACEIADFFIKNKVGTVQMENLESMKRKEDGYFNIRLRGFWPYAEMQNKIEFKLKQYGIEIRRVAPNNTSRTCSKCGHLNNYFNFEYRRKYKFPHFKCEKCNFKEDADYNAALNISNPKLKSTKEEP

SEQ ID NO: 3195 - protein, 726 aa, synthetic construct
SEVEFSHEYWMRHALSLAKRARDEREVPVGAVLVLNNRIIGEGWNRAIGLHDPTAHAEIMALRQGGLVMQNNRLTDATLYVTFEPCVMCAGAMVHSRIGRVVFGVRNSKRGAAGSLMNVLNYPGVNHCVEITEGILVDECAALLCDFYRMPRHVLNAQKKAQSSISSGGSSGGCSGSEMPGASESVTPKSSGGGSSGSAKNTITKTLQLRIVRPYNSAEVEKIVADEKNNREKIALEKNKDKVKEACSKHLKVAAYCTTQVERNACLFCKARKLDDKFYQKLRGQFPDAVFWQETGEIFRQLQRQAAEIYNQSLIELYYEIFIKGRGFANASSVEHYLSDVCYTRAAELFKNAAIASGLRGKVKSNFRLKELKSMRSGLPTTKSDNFPIPLVKQKGGQYAGFEISSHNDDFIIKIPFGRWQVKKEIDKYRPWEKFDFEQVRKSPKPISLLLSTRRRKRNKGWSKDEGTEAEIRKVMNGDYQTSYIEVKRGSKIGEKSAWMLNLSIDVPKIDKGVDPGIIGGIDVGVKSPLVCAINNAFGRYSISDNDLFHFNKKMFARRRILLKKSKHKRAGHGAKNKLKPITILTEKSGRFRKKLIERWACEIADFFIKNKVGTVQMENLECMKRKEDSYFNIRLRGFWPYAEMQNKIEFKLKQYGIEIRKVAPNNTSKTCSKCGHLNYYFNFEYRKKNKFPHFKCEKCNFKEDADYNAALNISSPKLKSTKGEP

SEQ ID NO: 3196 - protein, 726 aa, synthetic construct
SEDEFSHEYWMRHALTLAKRARDGREVPVGAVLVLNNRVIGEGWNRAIGLHDPTAHAEIMALRQGGLVMQNYRLIDATLYVTFEPCVMCAGAMVHSRIGRVVFGVRNSKRGAAGSLMNVLDYPGMGHRVEITEGILADECAALLCDFYCMPRQVFNAQKRAQSTINSGSSSGGSSGSETPGTSESPTPESSGGIPGGSAKNTITKTLKLRIVRPYNSAEVEKIVADEKNNREKIALEKNKDKVKEACSKHLKVAAYCTTQVERNACLFCKARKLDDKFYRKLRGQFPDAVFWQELGEILRQLQKQAAEIYNQSLIELYYEIFIKGKGFANASSVEHYLSDVCYTRAAELFKNAAIASGLRGKVKSNFRLKELKNMKSGLPTTKSDNFPIPLVKQKGGQYTGFEISSHNDDFIIKIPFGRWQVKKEIDKYRPWEKFDFEQVRKSPKPISLLLSTQRRKRNKGWSKDEGTEAEIRKVMNGDYQTSYIEVKRGSKIGEKSAWMLSLSIDVPKIDKGVDPSIIGGIDVGVKSPLVCAINNAFNRYSISDNNLFHFNKKMFARRRILLKKNRHKRAGHGAKNRLKPISILTEKSERFRKKLIERWACEIADFFIRNKVGTVQMENLEGMKRKEDSYFNIRLRGFWPYAEMQNKIEFKLKQYGIEIRKVAPNNTSKTCSKCGHLNNYFNFEYRKKNKFPYFKCEKCNFKENADYNAALNISNPQLKSTKGEP

SEQ ID NO: 3197 - protein, 726 aa, synthetic construct
SEVEFSHEYWMRHALTLAKRARDEREVPVGAILVLNNRVIGVGWNRAIGLHDPTAHAEIMALRQGGLVTQNYRLINATLYVTFEPCVMCAGAMIHSRIGRVVFGVRNSKHGAAGSLVNVLNYPGMNHRVEITEGILADECAALLCDFYRMPRQVFNAQKRAQSTINSGGSSGGSSGSETPGTSESPTPESSGGSPGGSAKNTITKTLKLRIVRPYNSAEVEKIVADEKNNREKIALEKNKDKVKEACSKHLKVAAYCTTQVERNACLFCRARKLDDKFYQKLRGQFPDAVFWQEIGEIFRQLQKQAAEIYNQSLIELYYEIFIKGRGFANASSVEHYLSDVCYTRAAELFKNAAIASGLRGKVKSNFRLKELKNMKSGLPTTKSDNFPIPLVKQKGGQYTGFEISSHNDDFIIKIPFGRWQVKKEINKYRPWEKFDFEQVRRSPKPISLLLSTQRRKRNKGWSKDEGTEAEIRKVMNGDYQTSYIEVKRGSKTGEKSAWMLNLSIDVPKIDKGVDPSIIGGIDVGVKSPLVCAINNAFSRYSISDNDLFRFNKKMFARRRILLRKNRHKRAGHGAKNKLKPISILTGKSERFRKKLIERWACEIADFFIKNKVGTVQMENLESMKRKEDSYFNIRLRGFWPYAKMQNKIEFKLKQYGIEIRKVAPNNTSKTCSKCGHLNNYFNFEYRKKNKFPHFKCEKCNFKESADYNAALNISNPKLKSTKEEP

SEQ ID NO: 3198 - protein, 726 aa, synthetic construct
SEVEFSHEYWMRHALTLAKRARDEREVPVGAILVLNNRVIGEGWNRAIGLHDPTAHAEIMALRQGGLVMQNYRLIDATLYVTFEPCVMCAGAMIHSRIGRVVFGVRNNKHGAAGSLMNVLNCPGMNHRVEVTEGILADECAALLCDFYRMPRQVFNAQKKARSNINSGGSSGGSSGSETPGTSESASPESSGGSSGGSAKNTITKTLKLRIVRPYNSAEVEKIVADEKNNREKVALEKNKDKVREACSEHLKVAAYCTTQVERNACLFCKARKLDDKFYQKLRGQFPDAVFWQEISEIFRQLQKQTAEIYNQSLIELYYEIFIKGKGFANASRVEHYLSDVCYARAAKLFKNAAIASGLRGKVKSNFRLKELKNMKSGLPSTKSDNFPIPLVKQKGGQYTGFEISSHNDDFIIKIPFGRWQVKKEIDRYRPWEKFDFEQVRKSPKPISLLLSTQRRKRNKGWSKDEGTEAEIRKVMNGDYQTSYIEVKRGSKTGEKSAWMLNLSIDVPKIDKGVDPSIIGGIDVGVKSPLVCAINNAFSRYSISDNDLFRFNKKMFARRRILLRKNRHKRAGHGAKNKLKPVTIMTEKSKRFRKKLIERWACEIADFFIKNKVGTVQMENLESMKRKEDSYFNIRLRGFWPYAEMQSKIEFKLKQYGIVVRKVAPNNTSKTCSKCGHLNNYFNFEYRKKNKFPHFKCEKCNLKEDADYNAALNISNPKLKSTKGEP

SEQ ID NO: 3199 - protein, 726 aa, synthetic construct
SEDEFSHEYWMRHALTLAKRARDGREVPVGAVLVLNNRVIGEGWNRAIGLHDPTAHAEIMALRQGGLVMQNYRLIDATLYVTFEPCVMCAGAMVHSRIGRVVFGVRNSKRGAAGSLMNVLNYPGMGHRVEITEGILADECAALLCDFYCMPRQVFNAQKRAQFSINSGGSSGGSSGSETPGSSESATPESSGGGSSGSAKNTITKALQLRIVRPYNSAEVEKIVADEKNNREKIALEKNKDKVKEACSKHLKVASYCTTQVERNACPFCKARKLDDKFYQKLRGQFPDAVFWQELGEILRQLQKQAAEIYNQSLIELYYEIFIKGRGFANAGSVEHYLSDVCYTRAAELFKNAAIASGLRGKVKSNFRLKELKNMKSGLPTTKSDNFPIPLVKQKGGQYTGFEISSHNDDFIIKIPFGRWQVKKEIDKYRPWEKFDFEQVRKSPKPISLLLSTQRRKRNKGWSKDEGTEAEIRKVMNGDYQTSYIEVKRGSKTGEKSAWMLNLSIDVPKIDKGVDPSIIGGIDVGVKSPLVCAINNAFSRYSISDNDLFRFNKKMFARRRILLKKNRHKRAGHGAKNKLKPISILTGKSERFRKKLIERWACEIADFFIKNKVGTVQMENLESMKRKEDSYFNIRLRGFWPYAEMQNKIEFKLKQYGIEIRRVAPNNTSKTCSKCGHLNNYLNFEYRKKNKFPHFKCEKCNFKENADYNAALNISNPELKSTKEEP

SEQ ID NO: 3200 - protein, 726 aa, synthetic construct
SEVEFSHEYWMRHALTLARRARDEREVPVGAILVLNNRVIGEGWNRANGLHDPTAHAEIMALRQGGLVMQNYRLIGATLYVTFEPCVMCAGAMVHSRIGRVVFGVRNSKRGAAGSLMNVLDYPGMGHRVEITEGILADECAALLCDFYRMPRQIFNAQKKARSNINSGGSSGGSSGSETLGTSEGATPESSGSSSGGSAKNTITKTLQLRIVRPYNSADVEKIVADEKNNREKAALEKNKDKVKEACSKHLKVATYCTTQVGRNACLFCKARKLDDKFYQKLRGQFPDAVFWQEISGIFRQLQKQAAEIYNQSLIELYYEIFIKGKGFANASSVEHYLSDVCYTRAAELFKNAAIASGLRSKVKSNFRLKELKTMKSGLPTTKGDNFPIPLVKQKGGQYAGFEISSHNDDFIIKIPFGRWQVKKEINKHRPWEKFDFEQVRKSPKPISLLLSTQRRKRNKGWSKDEGTEAEIRKVMNGDYQTSYIEVKRGSKIGEKSAWMLNLSIDVPKIDKGVDPGIIGGIDVGVKSPLVCAINNASSRYSISDNDLFHFNKKMFARRRILLKKNRHKRAGHGARNKLKPITVLAEKSRRFRKKLIERWACEIANFFIKNKVGTVQMENLESMKRKEDSYFNIRLRGFWPYAEMQNKIEFKLKQYGIEIRKVAPNNTSKTCSKCGHLNNYFNFEYRKKNKFPHFKCEKCNFKESADYNAALNISNPKLKSTKEEP

SEQ ID NO: 3201 - protein, 726 aa, synthetic construct
SEVEFSHEYWMRHALTLAKRARDEREVPVGAILVLNNRVIGEGWNRAIGLHDPTAHAEIMALRQGGLVMQNYRLIDATLYVTFEPCVMCAGAMIHSRIGRVVFGVRNSKHGAAGSLVNVLNYPGMNHRVEITEGILADECAALLCDFYRMPRQVFNARKKAQSSINPSGSSGGSSGSVTPGTSESATPESSGGSSTGSTKNTITKTLQLRIVRPYNSAEVEKIVADEKSNREKIALEKNKDKVKEACSEHLKVAAYCTTQVERNACLFCKARKLDDKFYQKLRGQFPDAVFWQELGGIFRQLQKQAAEIYNQSLIELYYEIFIKGKGITNASRVEHYLSDVCYTRAAELFKNAAIASGLRSKVRSNFRLKELKNMKSGLPTTKSDNFPIPLVKQKGGQYTGFEISSHNSDFIIKIPFGRWQVKEEIDKYRPWEKFDFEQVRKSPKPISLLLSTQRRKKNKGWSKDEGTEAEIRRVMNGDYQTSYIEVRRGSKIGEKSAWMLSLSIDVPKIDKGVDPSIIGGIDVGVKSPLVCAINNAFCRYSICDNDLFRFNKKMFARRRILLKNNRHKRAGHGAKNKLKPITILTKKSERFRKKLIERWVCEVADFFIKNKVGTVQMENLESMKRKEDSYFNIRLRGFWPYAEMQNRIELKLKQYGIEIRRVAPNNTSRTCSKCGHLNNYFNFEYRKKNKFPHFKCEKCNFREDADYNAALNISNPKLKSTKEEP

SEQ ID NO: 3202 - protein, 726 aa, synthetic construct
SEVEFSHEYWMRHALTLAKRARDEREVPVGAVLVLDNRVIGEGWNRAIGLHDPTAHAEIMALRQGGLVLQNYRLVDATLYVTFEPCVLCAGAMVHSRIGRVVFGARNSKRGAAGSLMNILNYPGMNHRVEITEGILADECAALLCDFYRMPRQVFNAQKKAQSSINSGGSSGGSSGSETPSTSESATPESSGGSSGGSAKNTITKTLQLRIVRPYNSAEVEKIVTDEKNNREKIALEKNKDKVKEACSKHLKMASYCTTQVERNACLFCRARKLDDKFYQKLRGQFPDAVFWQEIGEIFRQLQKQATEIYNQGLIELYYEIFIKGKGFANASSVEHYLSDVCYTRAAELFKNAAIASGLRGKVKSNFRLKELKNMKSGLPTTKSDNFPIPLVKQKGGQYTGFEISSHNDDFIIKIPFGRWQVKKEIDKYRPWEKFDFEQVRKSPKPISLLLSTQRRKRNKGWSKDEGTEAEIRKVMNGDYQTSYIEVKRGSKIGEKSAWMLNLSIDVPKIDKGVDPSIIGGIDVGVKSPLVCAINNAFSRYSIGDNDLFHYNKKMFARRRILLKKNRHKRAGHGAKNKLKPISILTGKSKRFRKKLIERWACEIADFFIKNKVGTVQIENLESMKRKEDSYFNIRLRGFWPYAEMQNKIEFKLKQYGIEIRKVAPNNTSKTCSKCGHLNSYFNFEYRKKNKFPHFKCEKCNFKENADYNAALNISNPKLKSTKEEP

SEQ ID NO: 3203 - protein, 726 aa, synthetic construct
SEVEFSHEYWMRRALTLAKRARDEREVPVGAVLVLNNRVIGVGWNRAVGLHDPTAHAEIMALRQGGLVMQNYRLVEATLYVTFEPCVMCAGAMIHSRIGRVVFGVRNSKRGAAGSLMNVLNYPGMNHRVEITEGILADECAALLCDYYRMPRQVFNARKKAQSSISSGGSSDGGSGSGTPGTSESATPKSSGGSSGGSAKNTITKALKLRIVRPYNSAEVEKIVADDKNNRERIALEKNKDKVKEACSKHLKVASYCTTQVERNACPFCKARKLDDKFYQKLRGQFPDAVFWQEIGEIFRQLQKQAAEIYNQSLIELYYEIFIKGRGFANASSVEHYLSDVCYTRAAELFKNAAIASGLRGKVKSNFRLKELKNMKSGLPTTKSDNFPIPLVKQKGGQYTGFEISSHNDDFIIKIPFGRWQVKKEIDKYRPWEKFDFEQVRKSPKPISLLLSTQRRKRNKGWSKDEGTEAEIRKVMNGDYQTSYIEVKRGSKIGEKSAWMLNLSIDVPKIDKGVDPRIIGGIDVGVKSPLVCAINNAFSRYSISDNDLFHYNKKMFARRRILLKKNGHKRAGHGAKNKLKPISILTEKSKRFRKKLIERWACEIADFFIKNKVGTVQMENLESMKRKEDSYFNIRLRGFWPYAEMQNKIEFKLKQYGIVIRKVAPNNTSKTCSKCGHLNNYFNFEYRKKNKFPHFKCEKCNFKENADYNAALNISNPKLKSTKEEP

SEQ ID NO: 3204 - protein, 726 aa, synthetic construct
SEVEFSDEYWMRHALTLAKRARDEREVPVGAVLVLNNRVIGEGWNRAIGLHDPTAHAEIMALRQGGLAMQNYRLIDATLYVTFEPCVMCAGALIHSRIGRVVFGVRNSRRGAAGSLMNVLNYPGMNHRAEITEGILADECAALLCDFYRMPRQVFNAQKKAQSSFNSGGSSGCSSGGETLGTSESATPESSGGSSGGSAKNTITKTLKLRIVRPYNSAEVEMIVADEKNNREKIALEKNEDKVKEACSEHLKVAAYCTTQVERSACLFCKARKLDDRFYQKLRGQFPDAVFWQEIGEIFRQLQKQAAEIYNQSLIELYYEIFIKGKGFANASSVEHYLSDVCYARAAELFKNAAIASGLRGKVKSNFRLKELKNMKSGLPTTKSDNFPIPLVKQKGGQYTGFEISSHNDDFIIKIPFGRWQVKKEIDKYRPWEKFDFERVRKNPKPISLLLSTQRRKRNKGWSKDEGTEAEIRKVMNGDYQTSYIEVKRGSKIGEKSAWVLNLSIDVPKIDKGVDPSIIGGIDVGVKSPLVCAINNAFSRYSISDNDLFRFNKKVFARRRILLKKNRHKRAGHGTKNKLRPITILAEKSGRFRKKLIERWACEIANFFIKNKVGTVQMENLESMKRKEDSYFNIRLRGFWPYAEMQNKIEFKLKQYGIKIRKVAPNNTSKTCSRCGHLNNYFSFEYRKKNKFPRFKCEKCNFKEDADYNAALNISNPKLKSTKEEP

SEQ ID NO: 3205 - protein, 726 aa, synthetic construct
SEVEFSHEYWMRHALTLAKRARDEREVPVGAILVLNNRVIGEGWNRAIGLNDPTAHAEIMALRQGGLVMQNYRLIDATLYVTFEPCVMCAGAMIHSRIGRVVFGVRNNKHGAAGSLVNVLNYPGVNHCVEITEGILVDECAALLCDFYRMPRQVLNAQKRAQSSINSGGSSGGSCGSDTPGTSGSATPESSGGGSSGSAKNTITKTLQLRIVRPYNSAEVERIVADEKNNREKIALEKNKDKVKEACSKHLKVAAYCTTQVGRNACLFCKARKLDDKFYQKLRGQFPDAVFWQEVGEIFRQLQRQAAEIYNQSLIELYYEIFIKGKGFANASNVEHYLSDVCYTRAAELFRNAAIASGLRGKVKSNFRLKELKNMKSGLPTTKSDNFPIPLVKQKGGQYTGFEISSHNDDFIIKIPFGRWQAKKEIDRYRPWEKFDFEQVRKSPKPISLLLSTQRRKRNKGWSKDEGTEAEIRKVMNGDYQTSYIEVKRGSKIGEKGAWMLNLSIDVPKIDKGVDPSIIGGIDVGVKSPLVCAINNAFSRYSISDNDLFHFNKKMFARRRILLRKNRHKRAGHGARNKLKPISILTEKSKRFRKKLIERWACEIADFFIKNKVGTVQMENLESMKRKEDSYFNVRLRGFWPYAEMQNKIEFKLKQYGIEIRKVAPSNTSKTCSKCGHLNNYFNFEYRRKNKFPHFKCEKCNFKEDADYNAALNISNPKLKSTKEEP

SEQ ID NO: 3206 - protein, 726 aa, synthetic construct
SEVEFSHEYWMRHALTLAKRARDEREVPVGAVLVLDNRVIGEGWNRAIGLHDPTAHAEIMALRQGGLVMQNYRLIDATLYVTFEPCVMCAGTMVHSRIGRVVFGVRNNKRGAAGSLMNVLDYPGMDHRVEITEGILADECAALLCDFYRMPRQVFNAQRKAQSSINSGGSSGGSSGSETPGTSESATPESSGGSSGGSAKNTITKTLQLRIVRPYNSAEVEKIVADEKNNRERIALEKNKDKVKEACSKHLKAASYCTTQVERNACLFCKARKLDDKFYQRLRGQFPDAVFWQELGGIFRQLQKQAAEIYNQSLIELYYEIFIKGKGITNASRVEHYLSDVCYTRAAELFKNAAIASGLRSKVRSNFRLKELKNMKSGLPTTKSDNFPIPLVKQKGGQYTGFEISNHDGDFIIKIPFGRWQVKKEINKHRPWEKFDFEQVRKSPKPISLLLSTQRRKRNKGWSKDEGTEAEIRRVMNGDYQTSYIEVKRGSKIGEKSAWMLNLSIDVPKIDKGVDPSIIGGIDVGVKSPLVCAINNALSRYSISDNDLFRFNKKVFARRRILLKKNRHKRAGHGTKNKLKPITILTEKSGRFRKKLIERWACEIANFFIKNKVGTVQMENLESMKRKEDSYFNIRLRGFWPYAEMQNKIEFKLKQYGIEIRKVAPNNTSKTCSRCGHLNNYFSFEYRKKNKFPHFKCEKCNFKENADYNAALNISNPKLKSTKEEP

SEQ ID NO: 3207 - protein, 726 aa, synthetic construct
SEVEFSHEYWMRHALTLAKRARDEREVPVGAILVLNNRVIGVGWNRAIGLHDPTAHAEIMALRQGGLVTQNYRLIDATLYVTFEPCVMCAGAMIHSRIGRVVFGVRNSKHGAAGSLVNVLNYPGMNHRVEITEGILADECAALLCDFYRMPRQVFNARKKAQSSINSGGSSGGSSGSETPGTSESATPKSSGGSSGGSAKNTITKALKLRIVRPYNSAEVEKIVADEKNNRERIALEKNKDKVKEACSKHLKVAAYCTTQVERNACLFCKARKLDDKFYQKLRGQFPDAVFWQEIGEIFRQLQRQAAEIYNQSLIELYYEIFIKGKGFANASSVEHYLSDVCYTRAAELFKNAAIASGLRSKVRSNFRLKELKNMKSGLPTTKSDNFPIPLVKQKGGQYTGFEISSHNSDFIIKIPFGRWQEKEEVDRYRPWEKFDFEQVRKSPKSISLLLSTQRRKRNKGWSKDEGTEAEIKKVMNGDYQTSYIEVKRGSKIGEKSAWMLSLSIDVPKIDKGVDPSIIGGIDVGVKSPLVCAINNAFSRYSISDNDLFRFNKKMFARRRILLKKNRHKRAGHGAKNKLKPISILTEKSERFRKKLIERWACEIADFFIKNKVGTVQMENLESMKRREDSYFSTRLRGFWPYAKMQNKIEFKLKQYGIEIRKVAPNNTSKTCSKCGHLNNYFNFEYRKKNKFPHFKCEKCNFKENADYNAALNISNPKLKSTKEEP

SEQ ID NO: 3208 - protein, 726 aa, synthetic construct
SEVEFSHEYWMRHALTLAKRARDEREVPVGAVLVLNNRVIGVGWNRAIGLHDPTAHAEIMALRQGGLVMQNYRLTDATLYVTFEPCVMCAGAMVHSRIGRVVFGVRNSKRGAAGSLMNVLNYPGMSHCVEITEGILVDECAALLCDFYRMPRQVLSAQKKAQSSISSGGSSGGSSGSETPGTSESVTPKSSVGSSAGSTKNTITKTLKLRIVRPYNSAEVEKIVADEKNNREKIALEKNKDKVEEACSKHLKVATYCTTQVERNACLFCKARKLDDKFYQKLRGQFPDAVFWQEIGEIFRQLQKQAAEIYNQSLVELYYEIFIKGKGIANASSVEHYLSDVCYTRAAELFKNAAIASGLRNKIKSNFRLKELRNMKSGLPTTKSDNFPIPLVRQKGGQYTGFEISNHNGDFIIKIPFGRWQVKKEICKHRPWEKFDFEQVRKSPKPISLLLSTQRRKRNRGWSKDEGTEAEIKKVMNGDYQTSYIEVKRGSKTGEKSAWMLNLSIDVPKIDKGVDPCIIGGIDVGVKSPLVCAINNALSRYSISDNDLFHFNKKMFARRRILLKKTRHKRAGHGAKNKLKPVSILTEKSERFRKKLIERWACEIADFFIKNKVGTVQMENLESMKRREDSYFNIRLRGFWPYAKMQNKIEFKLKQYGIEIRKVAPNNTSKTCSKCGHLNNYFDFEYRKKNKFPHFKCEKCNFKESADYNAALNISNPKLKSTKEEP

SEQ ID NO: 3209 - protein, 726 aa, synthetic construct
SEDEFSHEYWMRHALTLAKRARDEREVPVGAVLVLNNRVIGEGWNRAIGLHDPTAHAEIMALRQGGLVMQNYRLTDATLYATFEPCVMCAGAMVHSRIGRVVFGVRNSKRGAAGSLMNVLNYPGMDHRVEITGGILADECAALLCDFYRMPRRVFNAQKKAQSSINSGGSSGGSSGSVTPGTSESATPESSGGSFGGSAKNTITKTLKLRIVRPYNSAEVEKIVADEKNSREKIALEKNKDKVKEACSKHLKVASYCTTQVERNACLFCKARKLDDKFYQKLRGQFPDAVFWQELGEIFRQLQKQAAEIYNQSLIELYYEIFIKGKGLANASSVEHYLSDVCYTRAAELFKNAAIASGLRGKVKSNFKLKELKSMKSGLPSTKSDNFPIPLVKQRGGQYTGFEISSHNDDFIIKIPFGRWQAKKEIDKYRPWEKFDFEQVRKSPKPISLLLSTQRRKRNRGWSKDESTEAEIKRVMNGDYQTSYIEVKRGSKVGEKSAWMLNLSIDVPKIDKGVDPSIIGGIDVGVKSPLVCAINNALSRYSISDNDLYRFNKKMFARRRILLKKSKHKRAGHGAKNKLKPITILTEKSGRFRKKLIERWACEIADFFIKNKVGTVQMENLEGMKRKEDSYFNIRLRGFWPYAEMQNKIEFKLKQYGIEIRKVAPNNTSKTCSKCGHLNNYFNFEYRKKNKFPHFKCEKCNFKEDADYNAALNISNPKLKSTKEES

SEQ ID NO: 3210 - protein, 726 aa, synthetic construct
SEVEFSHEYWMRHALTLAKRARDEREVPVGAILVLNNRVIGEGWNHAIGLHDPTAHAEITALRQGGLVMQNYRLIDATLYVTFEPCVMCAGAMIHSRIGRVVFGVRNNKHGAAGSLVNVLDYPGMNHRVEITEGILADECAALLCDFYRMPRQVFNARKKAQSSINPGGSSGGSSGSETPGTSESATPESSGGSSGSSAKNTITKTLKLRIVRPYNSAEVEKVVADEKNNREKIALEKNKDKVKEACSKHLKVAAYCTTQVERNACLFCKARRLDDKFYQKLRGQFPDAVFWQEIGEIFRQLQKQAAEIYNQSLVELYYEILIKGRGIANASSVEHYLSDVCYTRAAGLFKNAAIASGLRNKIKSNFRLKELRNMKSGLPTTKSDNFPIPLVKQKGGQYTGFEISNHNSDFIIKIPFGRWQAKKEIDKYRPWEKFDFEQVRKSPKPISLLLSTQRRKKNRGWSKDEGTEAEIKKVMNGDYQTSYIEVKRGSKIGEKSAWMLNLSIDVPKIDKGVDPSIIGGIDVGVKSPLVCAINNALSRYSISDNDLFHFNKKMFARRRILLKRNGHRRAGHGARNKLKPITVLTEKSKRFRKKLIERWACEIADFFIKNKVGTVQMENLESMKRKEDSYFNIRLRGLWPYAEMQNKIEFKLKQYGIEVRKVAPNNTSKTCSKCGHLNNYFNFEYRKRNKFPHFKCEKCNFKENADYNAALNISNPELKSTKEEP

SEQ ID NO: 3211 - protein, 726 aa, synthetic construct
SEVEFSHEYWMRHALTLAKRARDEREVPVGAVLVLNNRVIGEGWNRAIGLYDPTAHAEIMALRQGGLVMQNYRLTDATLYVTFEPCVMCAGAMIHSRIGRVVFGVRNSKRGAAGSLMNVLNYPGMNHCVEITEGILVDECAALLCDFYRMPRQVLNAQKKAQPSISSGGSSGGSSGSETPGASESVTPKSSGGGSAGSTKNTITKTLKLRIVRPYNSAEVEKIVADEKNSRERIALEKNKDKVKEACSKHLKVAAYCTTQVERNACLFCKARRLDDKFYQKLRGQFPDAVFWQEIGEIFRQLQKQAAEVYNQSLVELYYEILIKGKGIANASSVEHYLSDVCYTRAAELFKNAAIASGLRNKIKSNFRLKELRNMKSGLPTTKSDNFPIPLVRQKGGQYTGFEISNHDGDFIIKIPFGRWQVKEEIDKYRPWEKFDFEQVRKSPKPISLLLSTQRRKRNKGWSKDEGTEAEIRKVMNGDYQTSYIEVKRGSKIGEKSAWMLSLSIDVPKVDKGVDPSIIGGIDVGVKSPLVCAINNAFSRYSISDNDLFRFNKKVFARRRILLKRNRHKRAGHGTKNKLKPITILTEKSGRFRKKLIERWACEIANFLIKNKVGTVQMENLESMKRKEDSYFNIRLRGFWPYAEMQSKIEFKLKQYGIKIRKVAPNNTSKTCSKCGHLNNYFNFEYRKKNKFPHFKCEKCNFEENADYNAALNISNPKLKSTKGEP

SEQ ID NO: 3212 - protein, 726 aa, synthetic construct
SEVEFSHEYWMRHALALAKRARDEREVPVGAILVLNNRVIGEGWNRAIGLHDPTAHAEIMALRQGGLVMQNYRLIDATLYVTFEPCVMCAGAMIHSRIGRVVFGVRNNKHGAAGSLVNVLNYPGMNHRVEITEGILADECAALLCDFYRMPCQVFNARKKAQSSISPGGPSGGSSGSETPGTSESATPESSGGSSGGSAKNTITKTLKLRIVRPYNSAEVEKIVADEKSNREKIALEKNKDKVKEACSEHLKVAAYCTTQVERSACLFCKARKLDDKFYQKLRGQFPDAVFWQEIGEIFRQLQKQAAEIYNQSLIELYYEIFIKGKGFANASSVEHYLSDVCYTRAAELFKNAAIASGLRGKVKSNFRLKELKNMKSGLPTTKSDNFPIPLVKQKGGQYTGFEVSSHNDDFIIKIPFGRWQVKKEIDKYRPWEKFDFEQVRKSPRPIRLLLSTQRRKRNKGWSKDEGTEAEIRKVMNGDYQTSYIEVKRGSKIGEKSTWMLNLSIDVPKIDKGVDPSIIGGIDVGVKSPLVCAINNAFSRYSISDNDLFHFNKKMFARRRILLKKTRHKRAGHGAKNKLKPISILTEKSERFRKKLIERWACEIANFFIKNKVGTVQMENLESMKRKEDSYFNIRLRGFWPYAEMQNKIEFKLKQYGIEIRKVAPNNTSKTCSKCGHLNNYFSFEYRKKNKFPHFKCEKCNFKEDADYNAALNISNPKLKSTKEEP

SEQ ID NO: 3213 - protein, 726 aa, synthetic construct
SEVEFSHEYWMRHALTLAKRARDEREVPVGAILVLNNRVIGVGWNRAIGLHDPTAHAEIMALRQGGLVMQNYRLIDATLYVTFEPCVMCAGAMIHSRIGRVVFGARNSKRGAAGSLMNVLSYPGMNHRVEITEGILADECAALLCDFYRMPRQVFNARKKAQSSINPGGSSGGSSGSETPGTSESATPESSGGSSGGSAKNTITKTLKLRIVRPYNSAEVEKIVADEKNNRERIALEKNKDKVKEACSKHLKVAAYCTAQVERNACLFCKARKLDDKFYQKLRDQFPDAVFWQEIGEIFRQLQKQAAEIYNQSLIELYYEIFIKGRGFANASSVEHYLSDVCYTRAAELFKNAAIASGLRGKVKSNFRLKELKNMKSGLPTTKSDNFPIPLVKQKGGQYTGFEISSHNDDFIIKIPFGRWQVKEETDKYRPWEKFDFEQVRKNPKPISLLLSTQRRKRNKGWSKDEGTEAEIRKVMNGDYQTSYVEVKRGSKIGEKSAWMLNLSIDVPKIDKGVDPSIIGGIDVGVKSPLVCAINNAFSRYSISDNDLFRFNKKVFARRRILLKKNRHKRAGHGTKNKLKPITILTEKSGRFRKKLIERWACEIANFFTKNKVGTVQMENLESMKRKEDSYFNIRLRGLWPYAEMQNKIEFKLKQYGIKIRKVAPNNTSKTCSKCGHLNNYFNFEYRKKNKFPHFKCEKCSFKENADYNAALNISNPKLKSTKEEP

SEQ ID NO: 3214 - protein, 726 aa, synthetic construct
SEVEFSHEYWMRHALTLAKRARDEREVPVGAVLVLNNRVIGEGWNRAIGLHDPTAHAEIMALRQGGLVMQNYRLVDATLYVTFEPCVLCAGAMVHSRIGRVVFGVRNSKRGAAGSLMNVLNYPGMNHRVEITEGILADECAALLCDFYRMPRQVFNAQKKARSKINSGGSSGGSSGSETPDTSESATPESPGGSSGGSAKSTITKTLKLRIVRPYNSAEVEKIVADEKNNREKIALEKNRDKVKEACSEHLKVAAYCTTQVERNACLFCKARKLDDKFYQKLRGQFPDAVFWQEIGEIFRQLQKQAAEIYNQSLIELYYEIFIKGKGFANASSVEHYLSDVCYTRAAGLFKNAAIASGLRSKVRSNFRLKELKNMKSGLPTTKSDNFPIPLVKQKGGQYTGFEISSHNSDFIIKIPFGRWQVKEEIDKYRPWEKFDFEQVRKNPKPISLLLSIQRRKRNKGWSRDEGTEAEIRKVMNGDYQTSYIEVKRGSKIGEKSAWMLNLSIDVPRIDKGVDPSIIGGIDVGVKSPLICAINNAFSRYGISDNDLFRFNKKVFARRRILLKKNRHKRAGHGTKNKLKPITILTEKSGRFRKKLIERWACEIANFFIKNKVGTVQMEDLESMKKREDSYFNIRLRGLWPYAEMQSKIEFKLKQYGIEIRKVAPNNTSKTCSKCGHLNNYFNFEFRKKNKFPHFKCEKCNFKENADYNAALNISNPKLKSTKERP

SEQ ID NO: 3215 - protein, 726 aa, synthetic construct
SEVEFSHEYWMRHALTLAKRARDEREVPVGAVLVLNNRVIGEGWNRAIGMHDPTAHAEIMALRQGGLVMQNYRLIDATLYVTFEPCVMCAGAMIHSRIGRVVFGVRNSKHGAAGSLVNVLNYPGMNHRVEITEGILADECAALLCDFYRMPRQVFNARKKAQSSINPSGLSGGSSGSVTPGTSESATPESSGGGFGGSAKNTITKTLQLRIVRPYNSAEVEKIVADEKDNREKTALEKNKDKVKEACSKHLKVASYCTTQVERNTCLFCKARKLDDKFYQKLRGQFPDAVFWQELGEIFRQLQKQAAEIYNQSLIELYYEIFIKGKGLANASSVEHYLSDVCYTRAAGLFKNAAIASGLRGKVKSNFKLKELKSMKSGLPSTKSDNFPIPLVKQRGGQYTGFEISSHNDDFIIKIPFGRWQAKKEIDKYRPWEKFDFEQVRKSPKPISLLLSTQRRKRNRGWSKDEGTEAEIRKVMNGDYQTSYIEVKRGSKIGEKSAWMLNLSIDVPKIDKGVDPSIIGGIDVGVKSPLVCAINNAFSRYSISDNDLFRFNKKMFARRRVLLKKNRHKRAGHGAKNKLKPISILTEKSKRFRKKLIERWACEIADFFIKNKVGTVQMENLESMKRKEDSYFNIRLRGFWPYAEMQNKIEFKLKQYGIEIRKVAPNNTSKTCSMCGHLNNYFNFEYRKRNKFPHFKCEKCNFKENADYNAALNISNPKLESTKEEP

SEQ ID NO: 3216 - protein, 726 aa, synthetic construct
SEVEFSHEYWMRHALILAKRARDEREVPVGAVLVLNNRVIGEGWNRAIGLHDPTAHAEIMALRQGGLVMQNYRLIDATLYVTFEPCVMCAGAMIHSRIGRVVFGVRNSKRGAAGSLMNVLNYPGMNHRVEITEGILTDECAALLCDFYRMPHQVLNAQKKAQSSINPSGSSGGSSGSVTPGTSESATPESSGGGFGGSAKNTITKTLQLRIVRPYNSAEVEKIVADEKNNREKIALEKNKDKVKEACSKHLKVASYCTTQVERNACLFCKARKLDDKFYQKLRGQFPDAVFWQELGEIFRQLQKQAAEIYNQSLIELYYVIFIKGKGLANASSVEHYLSDVCYTRAAELFKNAAIASGLRGKVKSNFKLKELKSMKSGLPSTKSDNFPIPLVKQKGGQYTGFEISSHNSDFIIKIPFGRWQMKEEIDKYRPWEKFDFEQVRKSPKPISLLLSTQRRKKNKGWSKDEGTEAEIRRVMNGDYQTSYIEVKRGSKIGEKSAWMLNLSIDVPKIDKGVDPSIIGGIDVGVKSPLVCAINNSSSRYSICDNDLFRFNKKMFARRRILLKKNRHKRAGHGAKNKLKPITILTKKSERFRKKLIERWVCEVADFFIKNKVGTVQMENLESMKRKEDSYFNIRLRGFWPYAEMQNRIELKLKQYGIEIRRVAPNNTSRTCSKCGHLNNYFNFEYRKKSKFPHFKCEKCNFREDADYNAALNISNPKLKSTKEEP

SEQ ID NO: 3217 - protein, 726 aa, synthetic construct
SEAEFSHEYWMRHALTLAKRARDEREVPVGAVLVLNNRVIGEGWNRAIGLHDPTAHAEIMALRQGGLVMQNYRLVDATLYVTFEPCVLCAGAMVHSRIGRVVFGVRNNKRGAAGSLMNILNYPGMNHRVEITEGILADECAALLCDFYRMPRQVFNAQKKARSNINSGGSSGGSSGSETPGTSESPTPENSGGSSGGSAKNTITKTLKLRIVRPYNSAEVEKIVADEKNNREKIALEKNKGKVKEACSKHLKVATYCTTQVERNACLFCKARKLDDKFYQKLRGQFPDAVFWQETGEIFRQLQRQAAEIYNQSLIELYYEIFIKGKGIANASSVEHYLSGVCYTRAAELFKNAAIASGLRNKVKSNFRLKELKSMKSGLPTTKSDNFPIPLVRQKGGQYTGFEISNHNSDFIIKIPFGRWQAKKEINKHRPWERFDFEQVRKSPKPISLLLSTQRRKRNKGWSKDEGTEAEIRKVMNGDYQTSYIEVKRGSKIGEKSAWMLNLSIDVPKIDKGVDPSIIGGIDVGVKSPLVCAINNAPSRYSISDNDLFHFNKKMFARRRILLRKNRHKRAGHGARNKLKPITVLTEKSERFRKKLIERWACEIANFFIKNKVGTVQMENLESMKRREDSYFNIRLRGFWPYAEMQNKIEFKLKQYGIEIRKVTPNNTSKTCSKCGHLNNYFNFEYRKKNKFPHFKCEKCNFKENADYNAALNISNPKLKGTKGEP

SEQ ID NO: 3218 - protein, 726 aa, synthetic construct
SEVEFSHEYWMRHALTLAKRARDEREVPVGAVLVLNNRVIGEGWNRAIGLHDPTAHAEIMALRQGGLVMQNYRLSDATLYVTFEPCVMCAGAMIHSRIGRVVFGVRNSKRGAAGSLMNVLNYPGMNHCVEITEGILVDECAALLCDFYRMPRQVLSAQKKAQSSVSSGGSSGGSSGSETPGTSESATPKSSGGSSGGSAKNTITKALKLRIVRPYNSAEVEKIVADEKNNRERIALEKNKDKVKEACSKHLKVAAYCTTQVERNACLFCKARKLDDKFYQKLRGQFPDAVFWQEIGEIFRQLQKQAAEIYNQSLIELYYEIFIKGKGFANASSVEHYLSDVCYARAAELFKNAAIASGLRNKIKSNFRLKELRNMKSGLPTTKSDNFPIPLVKQKGGQYTGFEISNHDGDFIIKIPFGRWQVKKEIDKHRPWEKFDFEQVRKSPKPISLLLSTQRRKRNEGWSKDEGTEAEIRKVMNGDYQASYIEVKRGSKIGEKSAWMLNLSIDVPKIDKGVDPSIIGGIDVGVKSPLVCAINNAFSRYSISDNDLFHFNKKVFARRRILLKKNRHRRAGHGAKNKLKPITILTEKSKRFRKKLIERWACEIADFFIKNKVGTVQMENLESMKRKEDSYFNIRLRGFWPYAEMQNKIEFKLKQYGIKIRKVAPNNTSRTCSKCGHLNNYFSFEYRKKNKFPHFKCEKCNFKEDADYNAALNISNPKLKGTKEEL

SEQ ID NO: 3219 - protein, 726 aa, synthetic construct
SEVEFSHEYWMRHALILAKRARDEREVPVGAVLVLNNRVIGVGWNRAIGLHDPTAHAEIMALRQGGLVMRNYRLIDATLYVTFEPCAMCAGAMIHSRIGRVVFGVRNSKRGAAGSLMNVLNYPGMNHRVEITEGILTDECAALLCDFYRMPHQVLNAQKKAQSSINSGGSSGGSSGSETPGTSGSATPEGSGGSSAGSTKDTITKTLKLRIVRPYNSAEVEKVVADEKNNREKIALEKNKDKVKEACSKHLKVASYCTTQVERNACLFCKARKLDDKFYQKLRGQFPDAVFWQELGGIFRQLQKQAAEIYNQSLIELYYEIFIKGKGITNASRVEHYLSDVCYTRAAELFKNAAIASGLRSKVRSNFRLKELKNMRSGLPTTKSDNFPIPLVRQKGGQYTGFEISNHDGDFIIKIPFGRWQVKKEINKHRPWEKFDFEQVRKSPKPISLLLSTQRRKRNKGWSKDEGTEAEIRKVMNGDYQTSYIEVKRGSRTGEKSAWMLSLSIDVPKIDRGVDPSIIGGIDVGVKSPLVCAINNAFCRYSISDNDLFHFNKKMFARRRILLKKSRHKRAGHGAKNKLKPISILTEKSKRFRKKLIERWACEIADFFIKNKVGTVQMENLESMKRREDSYFNIRLRGFWPYAEMQNKIEFKLKQYGIEIRKVAPNNTSKTCSKCGHLNNYFNFEYRKKNKFPHFKCEKCNFKENADYNAALNISNPKLKSTKEEP

SEQ ID NO: 3220 - protein, 726 aa, synthetic construct
SEDEFSHEYWMRHALTLAKRARDGREVPVGAVLVLNNRVIGEGWNRAIGLHDPTAHAEIMALRQGGLEMQNYRLIDATLYVTFEPCVMCAGAMVHSRIGRVVFGVRNSKRGAAGSLMNVLNHPGMGHRVEITEGILADECAALLCDFYCMPRQVFNAQKRAQSSISPGGSSGGSSGSETPGTSESATPESSGGSSSGSAKNAITKTLKLRIVRPYNSAEVEKIVADEKNNREKIALEKNKGKVKEACSKHLKVAAYCTTQVEGNACLFCKARRLDDKFYQKLRGQFPDAVFWQELGEIFRQLQKQATEIYNQSLIELYYEIFIKGKGFANASSVEHYLSDVCYTRAAELFKNAAIASGLRGKVKSNFRLKELKNMKSGLPTTKSDNFPIPLVKQKGGQYTGFEISSHNDDFIIKIPFGRWQVKKEIDKYRPWEKFDFEQVRKSPKPISLLLSTQRRKRDKGWSKDEGTEAEIRKVMNGDYQTSYIEVKRGSKIGEKSAWMLNLSIDVPKIDKGVDPSIIGGIDVGVKSPLVCAINNAFSRYSIGDNDLFHFNKKMFARRRILLKKNRHKRAGHGAKNKLKPISILTEKSERFRKKLIERWACEIADFFIRNKVGTVQMENLEGMKRKEDSYFNIRLRGFWPYAEMQNKIEFKLKQYGIEVRKVAPNNTSKTCSKCGHLNNYFNFEYRKKNKFPHFKCEKCNFKENADYNAALNISNPKLKSTKEEP

SEQ ID NO: 3221 - protein, 726 aa, synthetic construct
SEVEFSHEYWMRHALTLAKRARDEREVPVGAILVLNNRVIGEGWNRAIGLHDPTAHAEIMALRQGGLVMQNYRLIDATLYVTFEPCVMCAGAMIHSRIGRVVFGVRNSKHGAAGSLVNVLNYPGMNHRVEITEGILADECAALLCDFYRMPRQVFNARKKAQSSINPSGSSGGSSGSVTPGTSESATPESSGGGFGGSAKNTITKTLQLRIVRPYNSAEVEKIVADEKNNREKIALEKNKDKVKEACSKHLKVASYCTTQVERNACLFCKARKLDDKFYQKLRGQFPDAVFWQELGEIFRQLQKQAAEIYNQSLIELYYVIFIKGKGLANASSVEHYLSDVCYTRAAELFKNAAIASGLRGKVKSNFKLKELKSMKSGLPSTKSDNFPIPLVKQRGGQYTGFEISSHNDDFIIKIPFGRWQVKKEIDKYRPWEKFDFEQVRKSPKPISLLLSTQRRKRNKGWSKDEGTEAEIRKVMNGDYQTSYIEVKRGSKIGEKSAWMLNLSIDVPKIDKGVDPSIIGGIDVGVKSPLVCAINNAFSRYSIGDNDLFHYNKKMFARRRILLKKNRHKRAGHGAKNKLKPISILTGKSERFRKKLIERWACEIADFFIKNKVGTVQMENLESMKRKEDSYFNIRLRGFWPYAEMQNKIEFKLKQYGIEVRKVAPNNTSKTCSKCGHLNNYFNFEYRKKNKFPHFKCEECNFKENADYNAALNISNPRLKSTKEEP

SEQ ID NO: 3222 - protein, 726 aa, synthetic construct
SEVEFSHEYWMRHALTLAKRARDEREVPVGAILVLNNRVIGEGWNRAIGLHDPTAHAEIMALRQGGLVMQNYRLIDATLYVTFEPCVMCAGAMIHSRIGRVVFGVRNNKHGAAGSLVNVLNYPGMNHRVEITEGILADECAALLCDFYRMPRQVFNARKKAQSSINSGGSSGGGSGSDTPSTSESTTPESSGGSSGGPAKNTITKTLKLRIVRPYNSAEVEKIVADEKNNREKTALEKNKDKVKEACSKHLKVAAYCTTQVERNACLFCKARKLDDKFYQKLRGQFPDAVFWQEVGEIFRQLQKQAAEIYNQSLIELYYEIFIRGRGFANASSVEHYLSDVCYTRAAELFKNAAIASGLRGKVKGNFRLKELKNMKSGLPTTKSDNFPIPLVKQKGGQYTGFEISSHNSDFIIKIPFGRWQEKEEIDKYRPWEKFDFEQVRRSPKPISLLLSTQRRKKNKGWSKDEGTEAEIRRVMNGDYQTSYIEVKRGSKIGEKSAWMLNLSIDVPKIDKGVDPSIIGGIDVGVKSPLVCAINNAFSRYSISDNDLFHFNKKMFARRRILLKKNRRRRAGHGAKNKLKPITILTEKSARFRKKLIERWACEIADFFIKNKVGTVQMENLESMKRKEDSYFNIRLRGFWPYAEMQNKIEFKLKQYGIEIRRVAPNNTSRTCSKCGHLNNYFNFEYRRKYKFPHFKCEKCNFKEDADYNAALNISNPKLKSTKEEP

SEQ ID NO: 3223 - protein, 726 aa, synthetic construct
SEVEFSHEYWMRHALTLAKRARDEREVPVGAVLVLNNRVIGEGWNRAIGLHDPTAHAEIMALRQGGLVMQNYRLIGATLYVTFEPCAMCAGAMIHSRIGRVVFGVRNSKRGAAGSLMNVLNYPGMNHRVEIMEGILTDECAALLCDFYRMPHQVLNAQKKAQSSINSGGSSGGSSGSETPGTSGSATPEGSGGSSGGSTKNTITKTLKLRIVRPYNSAEVEKIVADEKNNREKIALEKNKGKVKEACSKHLKVATYCTTQVERNACLFCKARKLDDKFYQKLRGQFPDAVFWQEVGEIFRQLQKQAAEIYNQSLIELYYEIFIKGKGIANASSVGHYLSDVCYTRAAELFKNAAIASGLRSKVRSNFRLKELKNMRSGLPTTKSDNFPIPLVKQKGGQYTGFEISSHNDDFIIKIPFGRWQVKKEIDKYRPWVKFDFEQVRKSPKPISLLLSTRRRKRNKGWSKDEGTEAEIRKVMNGDYQTSYIEVKRGSKIGEKSAWMLNLSIDVPKIDKGADPSIIGGIDVGVKSPLVCAINNAFSRYSISDNDLFRFNKKMFARRRILLKKNRHQRAGHGAKNKLKPITILTEKSGRFRRKLIERWACEIADFFIKNKVGTVQMENLESMRRREDSYFNIRLRGFWPYAEMQNRIEFKLRQYGIKIRKVAPNNTSKTCSKCGHLNNYFSFEYRKKNKFPHFKCEKCNFKENADYNAALNISNPKLMSTKEEP

SEQ ID NO: 3224 - protein, 726 aa, synthetic construct
SEVEFSHEYWMRHALTLAKRARDEREVPVGAVLVLNNRVIGVGWNRAIGLHDPTAHAEIMALRQGGLVMQNYRLTDATLYVTFEPCVMCAGAMIHSRIGRVVFGVRNSKRGAAGSLMNVLNYPGMNHCVEITEGILADECAALLCDFYRMPRQVFNARKKAQPSINPGGLSGGSSGSKTPGTSESPTPESSGGSSGGSAKNTITKTLKLRIVRPYNSAEVEKIVADEKNNREKIALEKNKDKVKEACSKHLKVAAYCTTQVERNACLFCKARKLDDKFYQKLRGQFPDAVFWREISEIFRQLQKQAAEIYNQSLIELYYEIFIKGKGIANASRVEHYLSDVCYTRAAELFKNAAIASGLRSKIKSNFRLKELKSMKSGLPTTKSDNFPIPLVKQKGGQYTGFEISNHNSDFIIKIPFGRWQVKEEVDKYRPWEKFDFEQVRRSPKPISLLLSTQRRKRNKGWSKDEGTEAEIRRVMNGDYQTSYIEVKRGSKIGEKSAWMLNLSIGVPKIDKGVDPGTTGGIDVGVKSPLVCAINNAFSRYSISDNDLFRFNKKMFARRRILLMKNRHRRAGHGAKNKLKPITILTEKSGRFRRKLIERWACEIADFFIKNKVGTVQMENLESMKRKEDSYFNIRLRGFWPYAEMQNKIEFKLKQYGIEIRKVAPNNTSKTCSKCGHLNNYFNFEYRKKNKFPHFKCEKCNFKENADYNAALNISNPKLKSTKKEP

SEQ ID NO: 3225 - protein, 726 aa, synthetic construct
SEVEFSHEYWMRHALTLAKRARDEREVPVGAVLVLNNRVIGEGWNRAIGLHDPTAHAEIMALRQGGLVMQNYRLIDATLYVTFEPCVMCAGAMIHSRIGHVVFGVRNNKHGAAGSLVNVLDYPGMNHRVEITEGILADECAALLCDFYRMPRQVFNARKKAQSSISSGGSSGGSSCGETPGASESVTPKSSGGSSAGSTKNTITKTLKLRIVRPYNSAEVEKIVADEKNSREKIALEKNKDKVKEACSEHLKVAAYCTTQVERNACLFCKARKLDDRFYQKLRGQFPDAVFWQEIGEIFRQLQRQAAEIYNQSLIELYYGIFIKGKGFANASSVEHYLSDVCYTRAAELFKNAAIASGLRGKVKSNFRLKELRSMRSGLPTAKSDNFPIPLVKQKGGQYTGFEISSHNDDFIIKIPFGRWQVKKEIDKYRPWEKFDFEQVRKSPKPISLLLSTRRRKRNKGWSKDEGTEAEIRKVMNGDYQTSYIEVKRGSKIGEKSAWMLNLSIDVPKVDKGVDPSIIGGIDVGVKSPLVCAINNAFSRYSISDNELFHFNKKMFARRRILLKKNRHKRAGHGAKNKLKPISVLTGKSERFRKKLIERWACEIADFFIKNKVGTVQMESLESMKRKEDSYFNIRLRGFWPYAEMQNKIEFKLKQYGIKIRKVAPNNTSKTCSKCGHLNNYFSFEYRRKNKFPHFKCEKCNFKESADYNAALNISNPKLMSTKEEP

SEQ ID NO: 3226 - protein, 726 aa, synthetic construct
SEDEFSHEYWMRHALTLAKRARDGREVPVGAVLVLNNRVIGEGWNRAIGLHDPTAHAEIMALRQGGLVMQNYRLIDATLYVTFEPCVMCAGAMVHSRIGRVVFGVRNGKRGAAGSLMNVLDYPGMGHRVEITEGILADECAALLCDFYCMPRQVFNAQKRAQSSINSGGSSGGSSGSETPGTSESATPKSSGGSSGGSAKNTITKALKLRIVRPYNSAEVEKIVADEKNNRERIALEKNKDKVKEACSKHLKVAAYCTTQVERNACLFCKARKLDDKFYQKLRGQFPDAVFWQELGEILRQLQKQAAEIYNQSLIELYYEIFIKGRGFANASSVEHYLSDVCYTRAAELFKNAAIASGLRGKVKSNFKLKELKSMKSGLPSTKSDNFPIPLVKQKGGQYTGFEISSHNDDFIIKIPFGRWQLKKEIDKYRPWEKFDFEQVRKSPKPISLLLSTQRRKRNKGWGKDEGTEAEIRKVMNGDYQTSYIEVKRGSKIGEKSAWMLNLSIDVPKIDKGVDPSIIGGIDVGVKSPLVCAINNAFSRYSISDNDLFCFNKKVFARRRILLRKNRHKRAGHGARNKLKPITVLTEKSERFRKKLIERWACEIANFFIKNKVGTVQMENLESMKRREDSYFNIRLRGFWPYAEMQSKIEFKLKQYGIKIRKVAPNNTSRTCSKCGHLNNYFNFEFRKKNKFPHFKCEKCNFKEDADYNAALNISDPKLKSTKEEP

SEQ ID NO: 3227 - protein, 726 aa, synthetic construct
SEVEFSHEYWMRHALTLAKRARDEREVPVGAVLVLNNRVIGEGWNRAIGLHDPTAHAEIMALRQGGLVLQNYRLIDATLYVTFEPCVMCAGAMIHSRIGRVVFGVRNSKRGAAGSLMNVLNCPGMNHRVEVTEGILADECAALLCDFYRMPRQVFNAQKKARSNINSGGSSGGSSGSETPGTSESASPESSGGSSGGSAKDTITKTLKLRIVRPYNSAEVEKIVADEKNNREKIALEKNKDKVKEACSKHLKVAAYCTTQVERNACLFCKARRLDDKFYQKLRGQFPDAVFWQEIGEIFRQLQKQAAEVYNQSLVELYYEILIKGKGIANASSVEHYLSDVCYTRAAELFKNAAIASGLRNKIKSNFRLKELRNMKSGLPTTKSDNFPIPLVRQKGGQYTGFEISNHDGDFIIKIPFGRWQVKKEINKHRPWEKFDFEQVRKSPKPISLLLSTQRRKRNKGWSKDEGTEAEIRKVMNGDYQTSYIEVKRGSKIGEKSAWMLNLSIDVPKIDKGVDPSIIGGIDVGVKSPLVCAINNALSRYSISDNDLFHFNKKMFARRRILLKKNRRRRAGHGAKNKLKPITILTEKSVRFRKKLIERWACEIADFFIKNKVGTVQMENLESMKRKEDSYFNIRLRGFWPYAEMQNKIEFKLKQYGIEIRRVAPNNTSRTCSKCGHLNNYFNFEYRRKYKFPHFKCEKCSFKENADYNAALNISNPKLKSTKEEP

SEQ ID NO: 3228 - protein, 726 aa, synthetic construct
SEVEFSHEYWMRRALTLAKRARDEREVPVGAILVLNNRVIGEGWNRAIGLHDPTAHAEITALRQGGLVMQNYRLIDATLYVTFEPCVMCAGAMIHSRIGRVVFGVRNSKHGAAGSLVNVLNYPGMNHCVEITEGILVDECAALLCDFYRMPRQVLNAQKKAQSSISSGGSSGGSSGNETPGASGSVTPKSSGGSSAGSTKDTITKTLKLRIVRPYNSAEVEKIVADEKNSREKIALEKNKDKVKEACSEHLKVAAYCTTQVERNACLFCKARKLDDRFYQKLRGQFPDAAFWQEIGEIFRQLQKQAAEIYNQSLIELYYEIFIKGKGFANASSVEHYLSDVCYTRAAELFKNAAIASGLRGKVKSNFRLKELKNMKSGLPTTKSDNFPIPLVKQKGGQYTGFEISNHNSDFIIKIPFGRWQAKKEIDKYRPWEKFDFEQVRKSPKPISLLLSTQRRKKNRGWSKDEGTEAEIKKVMNGDYQTSYIEVKRGSKIGEKSAWMLNLSIDVPKIDKGVDPSIIGGIDVGVKSPLVCAISNAFSRYSISDNDLFHFNKKMFARRRILLKKSKHKRAGHGAKNKLKPITTLTEKSRRFRKKLIERWACEIADFFIKNKVGTVQMENLESMKRREDSYFNIKLRGFWPYAEMQNKIEFKLKQYGIEIRKVAPNNTSKTCSKCGHLNNYFNFEYRKKNKFPHFKCEKCNFKENADYNAALNISNPKLKGTKEEP

SEQ ID NO: 3229 - protein, 726 aa, synthetic construct
SEVEFSHEYWMRHALTLAKRARDGREVPVGAVLVLNNRVIGEGWNRAIGLHDPTAHAEIMALRQGGLVMQNYRLIDATLYVTFEPCVMCAGAMIHSRIGRVVFGVRNNKRGAAGSLMNVLNYPGMNHRVEITEGILADECAALLCDFYRMPPQVLNARKKAQSSISSGGSSGGSNGSKTPGASESATPKSSGGSSAGSTRNTITKTLKLRIVRPYNSAEVEKIVADEKNNREKIALEKNKGKVKEACSKHLKVAAYCTTQVERNACLFCKARKLDDKFYQKLRGQFPDAVFWQEIGEIFRQLQKQAAEIYNQSLIELYYEIFIKGRGFANASSVEHYLSDVCYTRAAELFKNAAIASGLRGKVKSNFRLKELKNMKSGLPTTKSDNFPIPLVRQKGGQYTGFEISSHNDDFIIKIPFGRWQVKKEIDKYRPWEKFDFEQVRKSPKPISLLLSTQRRKRNKGWSKDEGTEAEIRKVMNGDYQTSYIEVKRGSKIGEKSAWTLNLSVDVPKIDKGVDPSIIGGIDVGVKSPLVCAINNALSRYSISDNDLFHFNKKVFARRRILLKKNRHRRAGHGAKNKLKPITILTEKSKRFRKKLIERWACEIADFFIKNKVGTVQMENLESMKRREDSYFNIRLRGFWPYAKMQNKIEFKLKQYGIEIRKVAPNNTSKTCSKCGHLNNYFNFEYRKKNKFPHFKCEKCNFKESADYNAALNISNPKLKSTKEES

SEQ ID NO: 3230 - protein, 726 aa, synthetic construct
SEVGFSHEYWMRHALTLAKRARDEREVPVGAVLVLNNRVIGEGWNRAIGLHDPTAHAEIMALRQGGLVMQNYRLVEATLYVTFEPCIMCAGAMVHSRIGRVVFGVRNSKRGAAGSLMNILNYPGMNHRVEITEGVLADECAALLCDFYRMPRQVFNAQKKVQSSINSGGSSGGSSGSETPSTSESATPESSGGSSGGSAKNTITKTLQLRIVRSYNSAEVEKIVTDEKNNREKIALEKNKDKVKEACSKHLKVAAYCTTQVGRNACLFCKARRLDDKFYQKLRGQFPDAVFWQEIGEIFRQLQKQAAEVYNQSLVELYYEILIKGKGIANASSVEHYLSDVCYTRAAELFKNAAIASGLRNKIKSNFRLKELRNMKSGLPTTKSDNFPIPLVRQKGGQYTGFEISNHDGDFIIKIPFGRWQVKKEIDKYRPWEKFDFEQVRKSPKPISLLLSTQRRKRNKGWSKDEGTEAEIRKVMNGDYQTSYIEVKRGSRIGEKSAWMLNLSIDVPKIDKGVDPSIIGGIDVGVKSPLVCAINNAFSRYSISDNDLFHYNKKMFARRRILLKKNRHKRAGHGAKNKLKPISILTEKNKRFRKKLIERWACEIADFFIKNKVGTVQIENLESMKRKEDSYFNIRLRGFWPYAEMQNKIEFKLKQYGIEIRKVAPNNTSKTCSKCGHLNSYFNFEYRKKNKFPHFRCEKCNFRENADYNAALNISNPKLRSTKEEP

SEQ ID NO: 3231 - protein, 726 aa, synthetic construct
SEVEFSHEYWMRHALTLAKRARDEREVPVGAILVLNNRVIGEGWNRAIGLHDPTAHAEIMALRQGGLVMQNYRLIDATLYVTFEPCVMCAGAMIHSRIGRVVFGVRNNKHGAAGSLVNVLDYPGMGHRVEITEGILADECAALLCDFYRMPRQVFNARKKAQSSINSGGSSGGSSGSEAPGTSESATPESSGGSSGGSAKNTITKTLQLRIVRPYNSAEVEKFVADEKNNREKIALEKNKDKVKEACSQHLKMASYCTTQVERNACLFCKARKLDDKFYQKLRGQFPDAVFWQETGEIFRQLQRQAAEIYNQSLIELYYEIFIKGRGFANASSVEHYLSDVCYTRAAELFKNAAIASGLRGKVKGNFRLKELKNMKSGLPTTKSDNFPIPLVRQKGGQYTGFEISNHNGDFIIKIPFGRWQVKKEICKHRPWEKFDFEQVRKSPKPISLLLSTQRRKRNKGWGKDEGTEAEIRKVMNGDYQTSYIEVKRGSKIGEKSAWMLNLSIDVPKIDKGVDPSIIGGIDVGVKSPLVCAINNALSRYSISDNDLFHFNKKMFARRRILLRKNRHKRAGHGARNKLKPITVLTEKSERFRKKLIERWACEIANFFIKNKVGTVQMENLESMKRREDSYFNIRLRGFWPYAEMQSKIEFKLKQYGIKIRKVAPNNTSKTCSKCGHLNSYFNFEYRKKNKFPHFKCEKCNFKEDADYNAALNISNPKLKGTKEEP

SEQ ID NO: 3232 - protein, 726 aa, synthetic construct
SEVEYSHEYWMRHALTLAKRARDEREVPVGAILVLNNRVIGEGWNRAIGLHDPTAHAEIMALRQGGLVLQNYRLIDATLYVTFEPCVMCAGAMIHSRIGRVVFGVRNNKHGAAGSLVNVLNYPGMNHRVEITEGILANECAALLCDFYRMPRQVFNARKKAQSSINPGGSSGGSSGSETPGTSESTTPESSGGSSGGSAKNTITKALKLRIVRPYNSAEVEKIVADEKNNREKIALEKNKDKVKEACSKHLKVAAYCTTQVERNACLFCKARRLDDKFYQKLRGQFPDAVFWQETGEIFRQLQRQAAEIYNRSLIELYYEIFIKGKGFANASSVEHYLSDVCYTRAAELFKNAAIASGLRGKVKSNFRLKELKNMKSGLPTTKSDNFPIPLVKQKGGQYTGFEISSHNDDFIIKIPFGRWQVKKEIDKYRPWEKFDFEQVRKSPKPISLLLSTQRRKRNKGWSKDEGTEAEIRKVMNGDYQTSYIEVKRGSKIGEKSAWMLNLSIDVPKIDKGVDPGIIGGIDVGVKSPLVCAINNAFSRYSISDNDLFRFNKKMFARRRILLRKNRHRRAGHGAKNKLKPITILTEKSERFRKKLVEKWACEIADFFIKNKVGTVQMENLESMKRKEDSYFNIRLRGLWPYAEMQNKIEFKLKQYGIEIRKVAPNNTSKTCSKCGHLNNYFNFEYRKKNKFPHFKCEKCNFKENADYNAALNISNPKLKSTKEEP

SEQ ID NO: 3233 - protein, 726 aa, synthetic construct
SEVEFSYEYWMRRALTLAKRARDEREVPVGAVLVLNDRVIGEGWNRAVGLHDPTAHAEIMALRQGGLVMQNHRLIEATLYVTFEPCIMCAGAMIHSRIGRVVFGVRNSKRGAAGSLMNVLNYPGMNHRVEITEGILADECAALLCDYYRMPRQVFNARKKAQSSIDSGGSSDGGSGSGTPGTSESATPESSGGSSGGSAKNTITKTLKLRIVRPYNSAEVEKIVADEKNNREKIALEKNKDKVKEACSKHLKVAAYCTTQVERNACLFCKARKLDDKFYQKLRGQFPDAVFWQEISEIFRQLQKQAAVIYNQGLIELYYEIFIKGKGIANASRVEHYLSNVCYTRAAELFKNAAIASGLRSKIKSNFRLKELKNMKSGLPTTKSDNFPIPMVKQKGGRCTGFEISNHNGDFIIKIPFGRWQVKKGIDKYRPWEKFDFEQVRKSPKPISLLLSTQRRRRNKGWSKDEGTEAEIKRVMNGDYQASYIEVKRGSKIGEKSAWMLNLSIDVPKIDKGVDPSIIGGIDVGVKSPLVCAINNAFSRYSISDNDLFHFNKKVFARRRILLKKNRHKRAGHGAKNKLKPITILTGKSKRFRKKLIERWACEIADFFIKNKVGTVQMENLESMKRKEDSYFNIRLRGFWPYAEMQNKIEFKLEQYGIEIRKVAPNNTSRTCSKCGHLNNYFNFEYRKKNKFPHFKCEKCNFKENADYNAALNISNPKLKSTKEEP

SEQ ID NO: 3234 - protein, 726 aa, synthetic construct
SEVEFSHEYWMRHALTLAKRARDEREVPVGAVLVLNNRVIGEGWNRAIGLHDPTAHAEIMALRQGGLAMQNYRLVDATLYVTFEPCVLCAGAMVHSRIGRVVFGVRNSKRGAAGSLMNVLNHPGMNHRVEITGGILADECAALLCDFYRMPRQVFNAQKKARSNINSGGSSGGSSGSETLGTSESATPESSGGSSGGSAKDTITKTLKLRIVRPYNSAEVEKIVADEKNNREKVALEKNKDKVKEACSEHLKVAAYCTTQVERNACLFCKARKLDDRFYQKLRGQFPDAVFWQETGEIFRQLQRQAAEIYNQSLIELYYEIFIKGKGFANASSVEHYLSDVCYTRAAELFKNAAIASGLRGKVRSNFRLKELKNMKSGLPTTKSDNFPIPLVKQKGGQYTGFEISSHNSDFIIKIPFGRWQEKEEIDKYRPWEKFDFEQVRRSPKPISLLLSTQRRKKNKGWSKDEGTEAEIRRVMNGDYQTSYIEVKRGSKIGEKSAWMLNLSIDVPKIDKGVDPSIIGGIDVGVKSPLVCAINNAFSRYSISDNDLFHFNKKMFARRRILLKKNRRRRAGHGAKNKLKPITILTEKSVRFRKKLIERWACEIADFFIKNKVGTVQMENLESMKRKEDSYFNIRLRGFWPYAEMQNKIEFKLKQYGIKVRKVAPNNTSKTCSKCGHLNNYFSFEYRKKNKFPHFKCEKCNFKENADYNAALNISNPKLKSTKEEP

SEQ ID NO: 3235 - protein, 726 aa, synthetic construct
SEVEFSHEYWMRHALTLAKRARDEREVPVGAILVLNNRVIGVGWNRAIGLHDPTAHAEIMALRQGGLVTQNYRLIDATLYVTFEPCVMCAGAMIHSRIGRVVFGVRNSKHGAAGSLVNVLNYPGMNHRVEITEGILADECAALLCDFYRMPRQVFNARKKAQSSINSGGSSGGSSGSETPGTSESATPKSSGGSSGGSAKNTITKALKLRIVRPYNSAEVEKIVADEKNNRERIALEKSKDKVKEACSKHLKVAAYCTTQVERNACLFCKARKLDDKFYQKLRGQFPDAVFWQEIGEIFRQLQKQAAEIYNQSLIELYYEIFIKGKGFANASSVEHYLSDVCYTRAAELFKNAAIASGLRGKVKSNFRLKELKNMRSGLPTTKSDNFPIPLVKQKGGQYAGFEISSHNDDFIIKIPFGRWQAKKEIDKYRPWEKFDFEQVRKSPKPISLLLSTQRRKRNRGWSKDEGTEAEIRKVMNGDYQTSYIEVKRGSKTGEKSAWMLNLSIDVPKIDKGVDPSIIGGIDVGVKSPLVCAINNAFSRYSISDNDLFRFNKKMFARRRILLKKNRHKRAGHGAKNKLKPISILTGKGERFRKKLIERWACEIADFFIKNKVGTVQMENLESMKRKEDSYFNIRLRGFWPYAEMQNKIEFKLKQYGIEIRKVAPNNTSKTCSKCGHLNNYFNFEYRKKNKFPHFKCEKCNFKESADYNAALNISNPKLMSTKEEP

SEQ ID NO: 3236 - protein, 726 aa, synthetic construct
SEVEFSHEYWMRHALALAKRARDEREVPVGAVLVLNNRAIGEGWNRAIGLHDPTAHAEIMALRQGGLVTQNYRLIDATLYVTFEPCVMCAGAMIHSRIGRVVFGVRNSKHGAAGSLVNVLNYPGMNHRVEITEGILADECAALLCDFYRMPRQVFNARKKAQSSVNSGGSSGGSSGSETPGTSESATPKSSGGSSGGSAKNTITKALKLRIVRPYNSAEVEKIVADEKNNREKIALEKNKDKVKEACSKHLKVAAYCTTQVERNACLFCKARKLDDKFYQKLRGQFPDAVFWQEIGEIFRQLQRQAAEIYNQSLIELYYEIFIKGKGSANASSVEHYLSDVCYTRAAELFKNAAIASGLRGKVKSNFRLKELKNMKSGLPTTKSDNFPIPLVKQKGGQYTGFEISSHNDDFIIKIPFGRWQVKEEIDKYRPWEKFDFEQVRKSPKPISLLLSTQRRKKNKGWSKDEGTEAEIRRVMNGDYQTSYIEVKRGSKIGEKSAWMLNLSIDVPKIDKGVDPSIIGGIDVGVKSPLVCAINNSSSRYSICDNDLFRFNKKMFARRRILLKKNRHKRAGHGAKNKLKPITILTKKSERFRKKLIERWVCEVADFFIKNKVGTVQMENLESMKRKEDSYFNIRLRGFWPYAEMQNRIELKLKQYGIEIRRVAPNNTSRTCSKCGHLNNYFNFEYRKKSKFPHFKCEKCNFREDADYNAALNISNPKLKSTKEEP

SEQ ID NO: 3237 - protein, 726 aa, synthetic construct
SEVEFSHEYWMRHALTLAKRARDEREVPVGAILVLNNRVIGEGWNRTIGLHDPTAHAEIVALRQGGLVMQNYRLIDATLYVTFEPCVMCAGAMIHSRIGRVVFGVRNSKHGAAGSLVNVLNYPGMNHRVEITEGILADECAALLCDFYRMPRQVFNARKKAQSSINPSGSSGGSSGSVTPGTSESATPESSGGGFGGSAKNTITKTLQLRIVRPYNSAEVEKIVADEKNNREKIALEKNKDKVKEACSKHLKVASYCTTQVERNACLFCKARKLDDKFYQKLRGQFPDAVFWQELGEIFRQLQKQAAEIYNQSLIELYYEIFIKGKGLANASSVEHYLSDVCYTRAAELFKNAAIASGLRGKVKSNFKLKELKSMKSGLPSTKSDNFPIPLVKQRGGQYTGFEISNHNSDFIIKIPFGRWQVKREIDKYRPWEKFDFEQVRKSPKPISLLLSTQRRKRSRGWSKDEGTEAEIKKVMNGDYQTSYIEVKRGSKTGEKSAWMLNLSIDVPRIDKGVDPSIIGGIDVGVKSPLVCAINNAFSRYSISDNDLFHFNKKMFARRRILLKKNRHKRAGHGAKNKLKPFTILTEKSGRFRKKLIERWVCEIADFFVKNKVGTVQMENLESMKRKEDSYFNIRLRGFWPYAEMQNRIEFKLKQYGIKVRKVAPNNTSKTCSKCGHLNSYFSFEYRKKNKFPHFKCEKCNFKENADYNAALNISNPKLKSTKEEP

SEQ ID NO: 3238 - protein, 726 aa, synthetic construct
SEVEFSHEYWMRHALTLAKRARDEREVPVGAVLVLNNSVIGEGWNRAIGLHDPTAHAEIMALRQGGLVMQNYRLTDATLYVTFEPCVMCAGAMIHSRIGRVVFGVRNSKRGAAGSLMNVLNYPGMNHRVEITEGILVDECAALLCDFYRMPCQVLNAQKKAQSSISSGGSSGGSSGGDTLGASESVTPKSSVGSSASSTKNTITKTLKLRIVRPYNSAEVEKIVADEKNNREKIALEKNKDKVKEACSEHLKVAAYCTTQVERNACLFCKARKLDDKFYQKLRGQFPDAMFWQEVGEIFRQLQKQAAEIYNQSLVELYHEIFIKGKGFANASSVEHYLSDVCYTRAAELFKNAAIASGLRGKVKSNFRLKELKNMKSGLPTTKSDNFPIPLVKQKGGQYTGFEISSHNDDFIIKIPFGRWQVRKEVDKYRPWVKFDFEQVRKSPKPISLLLSTQRRKRNKGWGKDEGTEAEIKKVMNGDYQTSYIEVKRGSRIGEKSAWMLSLSIDVPKIDRGVDPSIIGGIDVGVKSPLVCAISNAFSRYSISDNDLFHFNKKMFARRRILLKKSKHKRAGHGAKNKLKPITILTEKSRRFRKKLIERWACEIADFFIKNKVGTVQMENLECMKRKEDSYFNIRLRGFWPYAEMQNKIEFKLKQYGIEIRKVAPNNTSKTCSRCGHLNNYFNFEYRKKNKFPHFKCEKCNFKENADYNAALNISNPKLKSTKEEP

SEQ ID NO: 3239 - protein, 726 aa, synthetic construct
SEDEFSHEYWMRHALTLAKRARDGREVPVGAVLVLNNRVIGEGWNRAIGLHDPTAHAEIMALRQGGLVMQNYRLTDATLYVTFEPCVMCAGAMIHSRIGRVVFGVRNSKRGAAGSLMNVLNYPGMNHRVEITEGILADECAALLCDFYRMPRQVFNARKKAQSSINPGGSSGGSSGSETPGTSESATPESSGGSSGSSAKNTITKTLKLRIVRPYNSAEVEKIVADEKNNREKIALEKNEDKVKEACSKHLKVAAYCTTQVGRNACLFCKARRLDDKFYQKLRGQFPDAVFWQEIGEIFRQLQKQAAEVYNQSLVELYYEILIKGKGIANASSVEHYLSDVCYTRAAELFKNAAIASGLRNKIKSNFRLKELRNMKSGLPTTKSDNFPIPLVRQKGGQYTGFEISSHNSDFIIKIPFGRWQVKEEIDKFRPWEKFDFEQVRKSPKPISLLLSTQRRKKNKGWSKDEGTEAEIRRVMNGDYQTSYIEVKRGSKIGEKSAWMLNLSIDVPKIDKGVDPSIIGGIDVGVKSPLVCAINNALSRYSIGDNDLFHFNKKMFARRRILLKKNRRKRAGHGAKNKLKPISILTEKSERFRKKLIERWACEIADFFIKNKVGTVQMENLESMKRREDSYFNIRLRGFWPYAKMLNKIEFKLKQYGIKIRKVAPNNTSKTCSKCGHLNNYFNFEYRKKNKFPHFKCEKCNFKENADYNAALNISNPKLKSTKGEP

SEQ ID NO: 3240 - protein, 726 aa, synthetic construct
SEVEFSHEYWMRHALTLAKRARVEREVPVGAVLVLNNRVIGEGWNRAIGLHDPTAHAEIVALRQGGLVMQNYRLTDATLYVTFEPCVMCAGAMIHSRIGRVVFGVRNSKRGAAGSLMNVLNYPGMNHCVEITEGILVDECAALLCDFYRMPRQVLNAQKKAQSSISSGGSSGGSGGSEPPGASESVTPKSSAGSSAGSTKNTITKTLKLRVVRPYNSAEVEKIVADEKNNREKIALEKNKDKVKEACSKHLKVAAYCTTQVERNACLFCKARRLDDKFYQKLRGQFPDAVFWQELGEIFRQLQKQAAEIYNQSLIELYYEIFIKGKGFANASSVEHYLSDVCYTRAAELFKNAAIASGLRGKVKSNFRLKELRNMKSGLPTTKSDNFPIPLVRQKGGQYTGFEISSRNDDFIIKIPFGRWQVKEEIDKYRPWEKFDFEQVRKSPKPISLLLSTQRRKRNKGWSKDEGTEAEIRKVMNGDYQTSYIEVKRGSKTGEKSAWVLNLSIDVPKIDKGVDPSIIGGIDVGVKSPLVCAINNAFSRYSISDNDLFRFNKKMFARRRILLGKNRHKRAGHGVKNKLKPITILTEKSGRFRKKLIEKWACEIADFFIRNKVGTVQMENLESMKRKEDSYFNIRLRGFWPYAEMQNKIEFKLEQYGIEIRKVAPNNTSKTCSKCGHLNNYFNFEYRKKNKFPHFKCEKCNFKENADYNAALNISNPKLKSTKEVP

SEQ ID NO: 3241 - protein, 726 aa, synthetic construct
SEVEFSHEYWMRHALTLAKRARDEREVPVGAVLVLNNRVIGVGWNRAVGLHDPTAHAEIMALRQGGLVMQNYRLTDATLYVTFEPCVMCAGAMIHSRIGRVVFGVRNSKRGAAGSLMNVLNYPGMNHCVEITEGILVDECAALLCDFYRMPRQVLNAQKKAQSSISSGGSSGGSSCSETPGASESVTPKSSGGSSAGSTKNTITKTLKLRIVRPYNSAEVEKIVADEKNSREKIALEKNKDKVKEACSEHLKVAAYCTTQVERNACLFCKARKLDDRFYQKLRGQFPDAVFWQEIGEIFRQLQKQAAEIYNQSLIELYYEIFIKGKGFANASSVEHYLSDVCYTRAAELFKNAAIASGLRGKVKSNFRLKELKNMKSGLPTTKSDNFPIPLVKQKGGQYTGFEVSSHNDDFIIKIPFGRWQVKEEIDKYRPWEKFDFEQVRKNPKPISLLLSTQRRKRNKGWSKDEGTEAEIRRVMNGDYQTSYIEVKRGSKIGEKSTWMLNLSIDVPKIDKGVDPSIIGGIDVGVKSPLVCAINNAFSRYSISDNDLFRFNKKVFARRRILLKKNRHKRAGHGAKNKLKPITILTERSKRFRKKLIERWACEIANFFIKNKVGTVQMENLESMKRKEDSYFNIRLRGLWPYAEMQNKIEFKLKQYGIKIRKVAPNNTSKTCSKCGHLNNYFSFEYRKKNKFPHFKCEKCNFKEDADYNAALNISNPKLKSTKEEP

SEQ ID NO: 3242 - protein, 726 aa, synthetic construct
SEVEFSHEYWMRHALTLAKRARDEREVPVGAVLVLNNRVIGEGWNRTTGLHDPTAHAEIMALRQGGLVMRNHRLVDATLYVTFEPCVMCAGAMIHSRIGRVVFGVRNSKRGAAGSLTNVLNYPGMNHRVEITEGILVDECAALLCDFYRMPRQVFNAQKKAQSTINSGGSSGGSSGSETPGTSESPTPESSGGSPGGSTKNTITKTLKLRIVRPYNSAEVEKIVADEKNNRERIALEKNKDKVKEACSKHLKVAAYCTTQVERNACLFCKARKLDDKFYQKLRGQFPDAVFWQEIGEIFRQLQKQAAEIYNQSLIELYYEIFIKGKGFANASSVEHYLSDVCYTRAAGLFKNAAIASGLRGKVKSNFRLKELKNTKSGLPTTKSDNFPIPLVKQKGGQYTGFEISSHNDDFIIKIPFGRWQAKEEIDKYRPWEKFDFEQVRKSPKPISLLLSTQGRKKNKGWSKDEGTEAEIRKVMNGDYQTSYIEVKRGSKIGEKSAWMLNLSIDVPKIDKGVDPSIIGGIDVGVKSPLVCAINNASSRYSISDNDLFRFNKKMFARRRILLKKNRHKRAGHGAKNKLKPITIMTEKSKRFRKKLIERWACEIADFFIKNKVGTVQMENLESMKKKEDSYFNIRLRGLWPYAEMQNRIELKLKQYGIEIRRVAPNNTSRTCSKCGHLNNYFNFEYRKKSKFPHFKCEKCNFREDADYNAALNISNPKLRSTKEEP

SEQ ID NO: 3243 - protein, 726 aa, synthetic construct
SEVEFSHEYWMRHALTLAKRARDEREVPVGAILVLNNRVIGVGWNRAIGLHDPTAHAEIMALRQGGLVMQNYRLIDATLYVTFEPCVMCAGAMIHSRIGRVVFGVRNSKHGAAGSLVNVLNYPGMNHRVEVTEGILADECAALLCDFYRMPRQVFNARKKAQSSINPGGSSGGSSGSGTPGTSESATPESSGGSSSGSAKNTITKTLKLRIVRPYNSAEVEKIVADEKNNREKIALEKNKDKVKEACSEHLRVAAYCTTQVERNACLFCKARKLDDGFYQKLRGQFPDAVFWQEVGEIFRQLQRQAAEIYNQSLIELYYEVLIKGKGIANASRVEHYLSDVCYTRAAELFKNAAIASGLRSKIKSNFRLKELRNMKSGLPTTRSDNFPIPLVKQKGGRCTGFEISNHNSNFIIKIPFGRWQVKKEIDKYRPWEKFDFEQVRKSPKPISLLLSTQRRKRNKGWSTDEGTEAEIRKVMNGGYQTSYIEVKRGSKVGEKSAWMVNLSIDVPKIDKGVDPSIIGGIDVGVKSPLVCAVNNALSRYSIDDNDLFHFNKKMFARRRILLKKSRHKRAGHGAKNKLKPISILSGKSERFRKKLIERWACEIASFFIKNKVGTVQMENLESMKRREDSYFNIRLRGFWPYAEMQSKIEFKLKQYGIKIRKVAPNNTSKTCSKCGHLNNYFNFEFRKKNKFPHFKCEKCNFKEDADYNAALNISNPKLKGTKEEP

SEQ ID NO: 3244 - protein, 725 aa, synthetic construct
SEVEFSHEYWMRHALTLAKRARDEREVPVGAILVLNNRVIGEGWNRAIGLHDPTAHAEIMALRQGGLVMQNYRLIDATLYVTFEPCVMCAGAMIHSRIGRVVFGVRNNKHGAAGSLVNVLNYPGMNHRVEITEGILADECAALLCDFYRMPRQVFNARKKARSNINSGGSSGGSSGSETPGTSESATPESSGGSSGGSTRNTITKTLKLRIVRPYNSAEVEKIVADEKNNREIALEKNKDKVKEACSKHLKVAAYCTTQVERNACLFCRARRLDDKFYQKLRGQFPDAVFWQEIGEIFRQLQKQAAEIYNQSLVELYYEIFIKGKGIANASSVEHYLSDVCYTRAAELFKNAAIASGLRNKVKSNFRLKELRNMKSGLPTTKSDNFPIPLVRQKGGQYTGFEISNHNSDFIIKIPFGRWQVKKEIDKYRPWEKLDFEQVRKSPKPISLLLSTQRRKRNKGWSKDEGTEAEIRKVMNGDYQTSYIEVKRGSKIGEKSAWMLNLSIDVPKIDKGVDPSIVGGIDVGVRSPLVCAIDNVLSRYSICDNDLFRFNKKMFARRRILLKKNRHKRAGHGAKNKLKPISILTERSERFRKKLIERWACEIADFFIKNKVGTVQMENLESMKRKEDSYFNIRLRGFWPYAEMQNKIEFKLKQYGIEIRKVAPNNTSKTCSKCGHLNNYFNFEYRKRNKFPHFKCEKCNFKENADYNAALNISNPKLKSTKEEP

SEQ ID NO: 3245 - protein, 726 aa, synthetic construct
SEVEFSHEYWMRRALTLAKRARDEREVPVGAVLVLNNRVIGVGWNRAAGLHDPTAHAEIMALRQGGLVMQNYRLIEATLYVTFEPCIMCAGAMIHSRIGRVVFGVRNSKRGAAGSLMNVLNYPGMNHRVEITEGILADECAALLCDYYRMPRQVFNARKKVQSSINSGGSSDGGSSSETPGTIESATPESSGGSSGGSAKNTITKTLKLRIVRPYNSAEVEKIVADEKNNREKIALEKNKDRVKEACSEHLKVAAYCTTQVERNACLFCKARKLDDKFYQRLRGQFPDAVFWQELGEIFRQLQKQAAEIYNQSLIELYYEIFIKGKGFANASSVEHYLSDVCYTRAAELFKNAAIASGLRGKVKSNFRLKELKNMKSGLPTTKSDNFPIPLVRQKGGQYTGFEISSHNDDFIIKIPFGRWQVKKEIDKYRPWEKFDFEQVRKSPKPISLLLSTQRRKRNKGWSKDEGTEAEIRKVMNGDYQTSYIEVKRGSKTGGKSAWMLNLSIDVPKIDKGVDPCIIGGIDVGVKSPLVCAINDAFSRYSISDNDLFHFNKKMFARRRILLKKNGHKRAGHGAKNKLRPITIMTEKSKRFRKKLIERWACEIADFFIENKVGTVQMENLESMKRKEDSYFNIRLRGFWPYAEMQNKVEFKLKQYGIKVRKVAPNNTSKTCSKCGHLNNYFSFEYRKTNKFPHFKCEKCNFKENADYNAALNISNPKLMSTKEEP

SEQ ID NO: 3246 - protein, 726 aa, synthetic construct
SEVEFSHEYWMRHALTLAKRARDEREVPVGAVLVLNNRVIGEGWNRAIGLHDPTAHAEIMALRQGGLAMQNYRLVDATLYVTFEPCVLCAGAMVHSRIGRVVFGVRNSKRGAAGSLMNVLNHPGMNHRVEITGGILADECAALLCDFYRMPRQVFNAQKKARSNINPGGSSGGSSGSETPGTSESATPESSGGSSGGSAKNTITKTLKLRIVRPYNSAEVEKIVADEKNNREKIALEKNKDKVKEACSKHLKVAAYCTTQVERNACLFCKARRLDDKFYQKLRGQFPDAVFWQEIGEIFRQLQKQAAEIYNRSLIELYYEIFIKGKGIANASRVEHYLSDVCYTRAAELFKNAAIASGLRNRIKSNFRLKELKNMKSGLPTTKSDNFPIPLVKQKGGQYTGFEISSHNSDFIIKIPFGRWQAKKEIDKYRPWEKFDFEQVRKSPKPISLLLSTRRRKRNKGWSKDEGTEAEIRKVMNGDYQTSYIEVKRGSKIGEKSAWMLNLSIDVPKIDKGVNPSIIGGIDVGVKSPLVCAINNAFSRYSISDNDLFRFNKKMFARRRILLGKNRHKRAGHGVKNKLKPITILTEKSGRFRKKLIERWACEIANFFIKNKVGTVQMENLESMKGKEDSYFNIRLRGFWPYAEMQNKIEFKLKQYGIEIRKVAPNNTSKTCSKCGHLNNYFNFEYRKKSKFPHFKCEKCNFREDADYNAALNISNPKLKSTKEEP

SEQ ID NO: 3247 - protein, 726 aa, synthetic construct
SEVEFSHEYWMRHALTLAKRARDEREVPVGAVLVLNNRVIGEGWNRAIGLHDPTAHAEIMALRQGGLVMQNYRLTDATLYVTFEPCVMCAGAMIHSRIGRVVFGVRNSKRGAAGSQMNVLNYPGMNHCVEITEGILVDECAALLCDFYRMPRQVLNAQKKAQSSINSGGSAGGSSGSETPGTSGSTTPVSSGGSSGGSAKNTITKALKLRIVRPYNSAEVEKIVADEKNNREKIALEKNKDKVKEACSKHLKVAAYCTTQVERNACLFCKARKLDDKFYQKLRGQFPDAVFWQEIGEIFRQLQRQAAEIYNQSLIVLYYEIFIKGKGFANASSVEHYLSDVCYTRAAELFKNAAIASGLRGKVKSNFRLKELKNMKSGLPTTKSDNFPIPLVKQKGGQYTGFEISNHNSDFIIKIPFGRWQVKEEIDKYRPWEKFDFEQVRKSPKPISLLLSTQRRKKNKGWSKDEGTEAEIRRVMNGDYQTSYIEVKRGSKIGEKSAWMLNLSIDVPRIDKGVDPSIIGGIDVGVKSPLVCAVNNSFSRYSICDNDLFRFNKKMFARRRILLKKNSHKRAGHGAKNKLKPISILTEKSERFRKKLIERWACEIADFFIKNKVGTVQMENLESMKRKEDSYFNIRLRGFWPYAEMQNKIEFKLKQYGIEIRKVAPNNTSKTCSKCGHLNNYFNFEYRKKNKFPHFKCEKCNFKENADYNAALNISNPKLKSTKEEP

SEQ ID NO: 3248 - protein, 726 aa, synthetic construct
SEVEFSHEYWMRHALTLARRARDEREVPVGAVLVLNNRVIGEGWNRAVGLHDPTAHAEIMALRQGGLVVQNYRLIEATLYVTFEPCIMCAGAMIHSRIGRVVFGARNSKRGAAGSLMNVLNYPGMNHHVEITEGILADECAALLCDYYRMPRQVFNARKKVQSSINSGGSSDGGSSSETPGTSESATPESSGGSSGGSAKNTITKTLKLRIVRPYNSAEVEKIVADEKNNREKIALEKNKGKVKEACSRHLKVAAYCTTQVERNACLFCKARRLDDKFYQKLRGQFPDAVFWQEIGEIFRQLQKQAAEVYNQSLVELYYEILIKGKGIANASSVEHYLSDVCYTRAAELFKNAAIASGLRNKIKSNFRLKELRNMKSGLPTTKSDNFPIPLVRQKGGQYTGFEISNHDGDFIIKIPFGRWQVKKEINKHRPWEKFDFEQVRKSPKPISLLLSTQRRKRNKGWSKDEGTEAEIRKVMSGDYQTSYIEVKRGSKTGEKSAWMLNLSVDVPKIDKGVDPSIIGGIDVGVKSPLVCAINNAFSRYSISDNDLFHFNKKMFARRRILLKKNGHKRAGHGAKNKLKPITIMTEKSKRFRKKLIERWACEIADFFIKNKVGTVQMENLESMKRREDSYFNIRLRGFWPYAEMQDKIEFKLKQYGIVVRKVTPNNTSKTCSKCGHLNNYFNFEYRKKNKFPHFKCEKCNFKENADYNAALNISNPKLKSTKGEP

SEQ ID NO: 3249 - protein, 726 aa, synthetic construct
SEVEFSHEYWMRHALTLAKRARDEREVPVGAILVLNNRVIGVGWNRAIGLHDPTAHAEIMALRQGGLVTQNYRLIDATLYVTFEPCVMCAGAMIHSRIGRVVFGVRNSKHGAAGSLVNVLNCPGMNHCVEITEGILVDECAALLCDFYRMPRQVLSAQKKAQSSISPGGSSGGSSGSETPGASGSVTPKSSGGSSAGSTKDTITKTLKLRIVRPYNSAEVEKIVADEKNSREKIALEKNKDKVKEACSKHLKVASYCTTQVERNACPFCKARKLDDKFYQKLRSQFPDAVFWQELGEILRQLQKQAAEIYNQSLIELYYEIFIKGRGFANASSVEHYLSDVCYTRAAELFKNAAIASGLRGKVKSNFRLKELKNMKSGLPTTKSDNFPIPLVKQKGGQYTGFEISSHNSDLIIKIPFGRWQVKEEIDKYRPWEKFDFEQVRKSPKPISLLLSTQRRKKNKGWSKDEGTEAEIRRVMNGDYQTSYIEVRRGNKIGEKSAWMLSLSIDVPKIDKGVDPSIIGGIDVGVKSPLVCAINNSFSRYSICDNDLFRFNKKMFARRRILLKKNRHKRAGHGAKNKLKPITILTKKSERFRKKLIERWVCEVADFFIKNKVGTVQMENLESMKRKEDSYFNIRLRGFWPYAEMQNRIELKLKQYGIEIRRVAPNNTSRTCSKCGHLNNYFNFEYRKKNKFPHFKCEKCNFREDADYNAALNISNPKLKSTKEEP

SEQ ID NO: 3250 - protein, 726 aa, synthetic construct
SEVEFSHEYWMRHALTLAKRARDEREVPVGAVLVLNNRVIGEGWNRAIGLHDPTAHAEIMALRQGGLVLQNYRLIDATLYVTFEPCVMCAGAMIHSRIGRVVFGVRNNKHGAAGSLVNVLNYPGMNHRVEITEGILANECAALLCDFYRMPRQVFNARKKAQSSINPGGSSGGSSGSETPGTSESATPESSGGSSGSSAKNTITKTLKLRIVRPYNSAEVEKIVADEKNNREKIALEKNKDKVKEACSEHLKVAAYCTTQVERSACLFCKARKLDDKFYQKLRGQFPDAVFWQEISEIFRQLQKQAAEIYNQSLIELYYEVFIKGKGIANAGSVEHYLSDVCYTRAAGLFKNAAIASGLRNKIKSNFRPKELKNMKSGLPTTKSDNFPIPLVKQKGGQYTGFEISNHNSDFIIKIPFGRWQAKKEIDKYRPWERFDFEQVRKSPKPISLLLSTQRRKRNRGWSKDEGTEAEIRKVMNGDYQTSYIEVKRGSKIGEKSAWMLNLSIDVPKIDKGVDPSIIGGIDVGVKSPLVCAINNAFSRYSISDNDLFRFNKKMFARRRILLEKNRHKRAGHGVKNKLKPITILTEKSGRFRKKLIERWACEIADFFIKNKVGTVQMENLEGMKRKEDSYFNVRLKGFWPYAEMQNKIEFKLKQYGIEIRRVAPNNTSRTCSKCGHLNNYFNFEYRRKNKFPRFKCEKCNFKEDADYNAALNISNPKLKSTKEEP

SEQ ID NO: 3251 - protein, 726 aa, synthetic construct
SEVEFSHEYWMRHALTLAKRARDEREVPVGAVLVLNNRVIGEGWNRAIGLHDPTAHAEIMALRQGGLVMQNYRLIDATLYVTFEPCVMCAGAMIHSRIGRVVFGVRNSKHGAAGSLVNVLNYPGMNHRVEITEGILADECAALLCDFYRMPRQVFNARKKAQSSINPSGSSGGSSGSVTPGTSESATPESSGGGFGGSAKNTITKTLQLRIVRPYNSAEVEKIVADEKNNREKIALEKNKDKVKEACSKHLKVASYCTTQVERNACLFCKARKLDDRFYQKLRGQFPDAVFWQEIGEIFRQLQKQAAEIYNQSLIELYYEIFIKGKGVANANNVEHYLSDVCYTRAAELFKNAAIASGLRGKVKSNFRLKELKNMKSGLPTTKSDNFPIPLVRQKGGQYTGFEISDHNGDFVIKIPFGRWQVKKEIDKYRPWEKFDFAQVRKSPKPISLLLSTQRRKRNRGWSKDEGTEAEIKKVMNGDYQASYIEVKRGSRIGEKSAWMLNLSIDVPKIDKGVDPSIIGGIDVGVKSPLVCAINNAISRYSISDNDLFHFNKKVFARRRILLKKNRHRRAGHGTKNKLKPITILTEKSKRFRKKLIERWACEIADFFIKNKVGTVQMENLESMKRKEDSYFNIRLRGFWPYAEMQNKIEFKLKQYGIKIRKVAPNNTSRTCSKCGHLNNYFSFEYRKKNKFPHFKCEKCNFKEDADYNAALNISNPKLKGTKEEL

SEQ ID NO: 3252 - protein, 726 aa, synthetic construct
SEVEFSHEYWMRHALTLAKRARDEREVPVGAVLVLNNRVIGGGWNRAIGLHDPTAHAEIMALRQGGLVMQNCRLVDATLYVTFEPCVMCAGAMVHSRIGRVVFGVRNSKRGAAGSLMNVLDYPGMGHRVEITEGILTDECAALLCDFYRMPHQVLNAQKKAQSSINSGGSAGGSSGSETPGTSGSTTPVSSGGSSGGSAKNTITKALKLRIVRPYNSAEVEKIVADEKNNREKIALEKNKDKVKEACSKHLKVAAYCTTQVERNACLFCKARKLDDKFYQKLRGQFPDAVFWQEIGEIFRQLQRQAAEIYNQSLIELYYEIFIKGKGFANASSVEHYLSDVCYTRAAELFKNAAIASGLRGKVKSNFRLKELKNMRSGLPTTKSDNFPIPLVKQKGGQYAGFEISSHNDDFIIKIPFGRWQVKKEIDKYRPWEKFDFGQVRKSPKPISLLLSTRRRKRNKGWSKDEGTEAEIRKVMNGDYQTSYIEVKRGSKIGEKSAWMLSLSIDVPKIDKGVDPSIIGGIDVGVKSPLVCAINNAFGRYSISDNDLFHFNKKMFAMRRILLKKNRHKRAGHGAKNKLKPITILTEKSKRFRKKLIERWACEIADFFIKNKVGTVQMENLESMKRKEDSYFNIRLRGFWPYAEMQDKIEFKLKQYGIEIRKVAPNNTSKTCSRCGHLNNYFNFEYRRKNKFPHFKCEKCNFKENADYNAALNISNPKLKSTKEEP

SEQ ID NO: 3253 - protein, 726 aa, synthetic construct
SEVEFSHEYWMRHALTLAKRARDEREVPVGAVLVLNNRVIGEGWNRTTGLHDPTAHAEIMALRQGGLVMQNHRLVDATLYVTFEPCVMCAGAMIHSRIGRVVFGVRNSKRGAAGSLTNVLNYPGMNHRVEITEGVLVDECAALLCDFYRMPRQVFNAQKKAQSTINSGGSSGGSSGSETPGTSESPTPESSGGSPGGSAKNTITKTLKLRIVRPYNSAEVEKIVADEKNNREKIALEKNKDKVKEACSKHLKVAAYCTTQVERNACLFCKARRLDDKFYQKLRGQFPDAVFWQEIGEIFRQLQKQAAEVYNQSLVELYYEILIKGKGIANASSVEHYLSDVCYTRAAELFKNAAIASGLRNKIKSNFRLKELRSMKSGLPTTKSDNFPIPLVRQKGGQYTGFEISNHNSDFIIKIPFGRWQAKKEIDKYRPWEKFDFEQVRKSPKPISLLLSTQRRKRNRGWSKDESTEAEIKKAMNGDYQTSYIEVKRGSKVGEKSAWMLNLSIDVPKIDKGVDPSIIGGIDVGVKSPLVCAINDAFSRYSISDNDLFRFNKKVFARRRILLKKNRHKRAGHGAKNKLKPITILTKKSERFRKKLIERWACEIADFFIKNKVGTVQMENLESMKRKEDSYFNIRLRGFWPYAEMQDKIEFKLKQYGIEIRKVAPNNTSRTCSRCGHLNNYFNFEYRRKNKFPHFKCEKCYFKEDADYNAALNISNPRLKSTKEEP

SEQ ID NO: 3254 - protein, 726 aa, synthetic construct
SEVEFSHEYWMRHALTLAKRARDEREVPVGAILVLNNRVIGVGWNRAIGLHDPTAHAEIMALRQGGLVMQNYRLVNATLYVTFEPCVMCAGAMIHSRIGRVVIGVRNSKRGAAGSLMNVLNYPGMNHRVEITEGILTGECAALLCDFYRMPHQVLNAQKKAQSSINSGGSSGGSSGSETPGTSGSATPEGSGGSSGGFAKNTITKTLKLRIVRPYNSAEVEKIVADEKNNREKVALEKNKDKVKEACSKHLKMASYCTTQVERNACLFCKARKLDDKFYQKLRGQFPGAVFWQEIGEIFRQLQKQAAEVYNQSLIELYYEIFVKGKGFANASSVEHYLSDVCYTRAAELFKNAAIASGLRGKVKSNFRLKELKSMRSGLPTTKSDNFPIPLVKQKGGQYTGFEISSHNDDFIIKIPFGRWQVKKEIDKYRPWEKFDFEQVRKSPKPISLLLSTQRRKRNKGWSKDEGTEAEIRKVMNGDYQTSYIEVKRGSKIGEKSAWMLNLSIDVPKIDKGVNPSIIGGIDVGVKSPLVCAINNALSRYSVSDNDLFRFNKKMFARRRILLKRSKHKRAGHGAKNKLKPITILTEKSGRFRKKLIERWACEIADFFIKNKVGTVQMENLESMKRKEDSYFNIRLRGFWPYAEMQNKIEFKLKQYGIEIRKVAPSNTSKTCSKCGHLNNYFNFEYRKKNKFPHFRCEKCNFKENADYNAALNISNPKLKSTKEEP

SEQ ID NO: 3255 - protein, 726 aa, synthetic construct
SEVEFSHEYWMRHALTLAKRARDEREVPVGAVLVLNNRVIGEGWNRAIGLHDPTAHAEIMALRQGGLVMQNYRLTDATLYVTFEPCVMCAGAMVHSRIGRVVFGVRNSKRGAAGSLMNVLNYPGVNHCVEITEGILVDECAALLCDFYRMPRQVLNAQKKAQSSISSGGSSGGCSGSETPGTSESATLENSGGSSGGSAKNTITKTLKLRIVRPYNSAEVERIVADEKNNRERIALEKNKDKVKEACSKHLKVAAYCTTQVERNACPFCKARRLDDKFYQKLRGQFPDAVFWEELGEIFRQLQKQAAEIYNQSLIELYYEIFIKGKGFANASSVEHYLSDVCYTRAAELFKNAAIASGLRGKVKGNFRLKELKNMKSGLPTTKSDNFPIPLVKQKGGQYTGFEISSHNDDFIIKIPFGRWQVKKEIDKYRPWEKFDFEQVRKSPKPISLLLSTQRRKRNKGWSKDEGTEAEIRKVMNGDYQTSYIEVERGSKIGEKSAWMLNLSIDVPKIDKGVDPSIIGGIDVGVKSPLVCAINNAFSRYSIGDNDLFHYNKKMFARRRILLKKNRHKRAGHGAKNKLKPISILTEKSKRFRKKLIERWACEIADFFIKNKVGIVQIENLESMKRREDSYFNIRLRGFWPYAEMQNKIEFKLKQYGIEIRKVAPNNTSKTCSKCGHLNSYFNFEYRKKNKFPHFKCEKCNFKENADYNAALNISNPKLKSTKEEP

SEQ ID NO: 3256 - protein, 726 aa, synthetic construct
SEVEFSHEYWMRHALTLAKRARDGREVPVGAVLVLNNRVIGEGWNRAIGLHDPTAHAEIMALRQGGLVMQNYRLIGATLYVTFEPCVMCAGAMVHSRIGRVVFGVRNSKRGAAGSLMNVLDYPGMGHRVEITEGILADECAALLCDFYCMPCQVFNAQKRAQSSINSGGSSGSSSGSETLGTSESATPESSGGSSAGSAKNTITKTLKLRIVRPYNSAEVEKIVADEKNNREKIALEKNKDKVKEACSEHLKVAAYCTTQVERNACLFCRARKLDDKFYQKLRGQFPDAVFWQEIGEIFRQLQKQAAEIYNQSLIELYYEIFIKGKGFANASSVEHYLSDVCYTRAAELFKNAAIASGLRGKVKSNLRLKELKNMKSGLPTTKSDNFPIPLVKQKGGQYTGFEISSHNDDFIIKIPFGRWQVKKEIDKYRPWEKFDFEQVRKSPKPISLLLSTQRRKRNKGWGKDEGTEAEIRKVMNGDYRTSYIEVKRGSKIGEKSAWMLSLSIDVPKIDKGVDPRIIGGIDVGVRSPLVCAINNALNRYSISDNDLFHFNKKMFARRRILLRNNRHKRAGHGAKSKLKPITVLTERGERFRKKLIERWACEIANFFIKNKVGTVQMENLESMKRREDSYFNVRLRGFWPYAEMQNKIEFKLKQYGIKIRKVAPNNTSKTCSKCGHLNNYFSFEYRKKNKFPHFKCEKCNFKEDADYNAALNISNPKLKSTKEEP

SEQ ID NO: 3257 - protein, 726 aa, synthetic construct
GEVEFSHEYWMRRALTLAKRARDEREVPVGAILVLNNRVIGEGWNRAIGLHDPTAHAEITALRQGGLVMQNYRLIDATLYVTFEPCVMCAGAMIHSRIGRVVFGVRNSKHGAAGSLVNVLNYPGMNHRVEITEGILADECAALLCDYYRMPRQVFNARKKAQSSINSGGSSDGGSGSETPGTSESATPESSGGSSGGSAKNTITKTLKLRIVRPYNSAEVEKIVADEKNNREKIALEKNKDKVKEACSEHLKVAAYCTTQVERNACLFCKARKLDDKFYQKLRGQFPDAVFWQEVGEIFRQLQKQAAEIYNQSLIELYYEIFIKGKGIANASSVGHYLSDVCYTRAAELFKNAAIASGLRGKIKSNFRLKELKNMKSGLPTTKSDNFPIPLVKQKGGQYTGFEISNHNGDFIIKIPFGRWQVKKEIDRYRPWEKFDFEQVRKSPKPISLLLSTQRRKGNKGWSKDEGTEAEIRKVMNGDYQTSYIEVKRGSKIGEKSAWMLNLSIDVPKIDKGVDPSIIGGIDVGVKSPLVCAVNNAFSRYSISDNELFHFNKKMFARRRILLKKNRHKRAGHGAKNKLKPISILTEKSERFRKKLIEKWACEIADFFIKNKVGTVQMENLESMKRKEDSYFNIRLRGFWPYAEMQNKIEFKLKQYGIEIRKVAPNNTSKTCSKCGHLNSYFNFEYRKKNKFPHFRCEKCNFRENADYNAALNISNPKLRSTKEEP

SEQ ID NO: 3258 - protein, 726 aa, synthetic construct
SEVEFSHEYWMRHALTLAKRARDEREVPVGAVLVLNNRVIGEGWNRAIGLHDPTAHAEIMALRQGGLVLQNYRLIDATLYVTFEPCVMCAGAMIHSRIGRVVFGVRNNKHGAAGSLVNVLNYPGMNHRVEITEGILANECAALLCDFYRMPRQVFNARKKAQSSINPGGSSGGSSGSETPGTSESATPESSGGSSGGSAKNTITKALKLRIVRPYNSAEVEKIVADEKNNREKIALEKNKDKVKEACSKHLKVASYCTTQVERSACPFCKARKLDDKFYQKLRGQYPDAVFWQELGEILRQLQKQTAEIYNQSLIELYYEILIKGKGFANASSVEHYLSDVCYTRAAELFKNAAIASGLRGKVKSNFRLKELKNMRSGLPTTKSDNFPIPLVKQKGGQYTGFEISSHNDDFIIKIPFGRWQVKKEIDKYRPWERFDFEQVRKSPKPISLLLSTQRRKRNKGWSKDEGTEAEIRKVMNGDYQTSYIEVKRGSKIGEKSAWMLNLSIGVPKIDKGVDPSIIGGIDVGVKSPLVCAINNAFSRYSISDNDLFHFNKKMFARRRILLKKNRHKRAGHGAKNKLKPISILTEKSKRFRKKLIERWACEIADFFIKNKVGTVQMENLESMKRKEDSYFNIRLRGFWPYAEMQNRIEFKLKQYGIEVRRVAPNNTSKTCSKCGHLNNYFNFEYRKKNKYPYFKCEKCNFKENADYNAALNISNPKLRSTKEEP

SEQ ID NO: 3259 - protein, 726 aa, synthetic construct
SEVEFSHEYWMRHALTLAKRARDEREVPVGAVLVLNNRVIGEGWNRTTGLHDPTAHAEIMTLRQGGLVMQNHRLVDATLYVTFEPCVMCAGAMIHSRIGRVVFGVRNSKRGAAGSLTNVLNYPGMNHRVEITEGILVDECAALLCDFYRMPRQVFNAQKKAQSSINPGGSSGGSSGSETPGTSESAIPESSGGSSGGSAKNTITKTLQLRIVRPYNSAEVEKIVADEKNNREKIALEKNKDKVKEACSRHLKVASYCTTQVERNACPFCKARKLDDRFYQKLRGQFPDAVFWQELGGIFRQLQKQAAEIYNQSLIELYYEIFIKGKGITNASRVEHYLSDVCYARAAELFKNAAIASGLRSKVRSNFRLKELKNMKSGLPTTKSDNFPIPLVKQKGGQYTGFEISSHNSDFIIKIPFGRWQEKEEIDKYRPWEKFDFEQVRKSPKPISLLLSTQRRKKNKGWSKDEGTEAEIRRVMNGDYQTSYIEVKRGSKIGEKSAWMLNLSIDVPKIDKGVDPSIIGGIDVGVKSPLVCAINNAFSRYSISDNDLFHFNKKMFARRRILLKKNRHRRAGHGAKNKLKPITILTEKSVRFRKKLIERWACEIADFFIKNKVGTVQMENLESMKRKEDSYFNIRLRGFWPYAEMQNKIEFKLKQYGVEIRRVAPNNTSRTCSKCGHLNNYFNFEYRRKNKFPHFKCEKCNFKENADYNAALNISNPKLKSTKEEP

SEQ ID NO: 3260 - protein, 726 aa, synthetic construct
SEDEFSHEYWMRHALTLAKRARDEREVPVGAILVLNNRVIGEGWNRAIGLHDPTAHAEIMALRQGGLVMQNYRLIDATLYVTFEPCVMCAGAMIHSRIGRVVFGVRNSKHGAAGSLMNVLNYPGMNHRVEITEGILADECAALLCDFYRMPHQVFSARKKAQSSINPGGSSGGSSGSKTPGTSESATPESSGGSSGGSAKNSTTKTLKLRIVRPYNSAEVEKIVADEKNNREKIALEKNKGKVKEACSKHLKVATYCTTQVERNACLFCKARKLDDKFYQKLRGQFPDAVFWQEIGEIFRQLQKQAAEIYNQSLIELYYEIFIEGKGFANASSVEHYLSDVCYTRAAELFKNAAIASGLRGKVKGNFRLKELKNMKSGLPTTKSDNFPVPLVKQKGGQYTGFEISSHNDDFIIKIPFGRWQVKKEIDKYRPWEKFDFEQVRKSPKPISLLLSTQRRKRNKGWSKDEGTEAEIRKVMNGDYQTSYIEVKRGSKAGEKSAWVLSLSIDVPKIDKGVDPSIIGGIDVGVKSPLVCAINNAFSRYSISDNDLFHFNKKVFARRRILLKKNRHRRAGHGTKNKLKPITILTEKSGRFRKKLIERWACEIANFFIKNKVGTVQMENLESMKRRGDSYFNIRLRGFWPYAEMQNKIEFKLKQYGIKIRKVAPNNTSKTCSKCGHLNNYFSFEYRKKNKFPHFKCEKCNFKEDADYNAALNISNPKLKSTKEEP

SEQ ID NO: 3261 - protein, 726 aa, synthetic construct
SEVEFSHEYWMRHALTLAKRARDEREVPVGAILVLNNRVIGEGWNRTTGLHDPTAHAEIMALRQGGLVMQNHRLVDATLYATFEPCVMCAGAMIHSRIGRVVFGVRNSKRGAAGSLTNVLNYPGMNHRVEITEGILVDECAALLCDFYRMPRQVLNAQKKAQSSISSGGSSGGSGGGETPGASESVTPKNSGGSSASSTKNTITKTLKLRIVRPYNSAEVEKIVADEKNSREKIALEKNKDKVKEACREHLKVAAYCTTQVERSACLFCKARKLDDKFYQKLRGQFPDAVFWQELGGIFRQLQKQAAEIYNQSLIELYYEIFIKGKGITNASRVEHYLSDVCYTRAAELFKNAAIASGLRSKVRSNFRLKELKNMKSGLPTTKSDNFPIPLVKQKGGQYTGFEISSHNSDFIIKIPFGRWQVKEEIDKYRPWEKFDFEQVRKSPKPISLLLSTQRRKKNKGWSEDEGTEAEIRRVMNGDYQTSYIEVKRGSKIGEKSAWMLNLSIDVPKIDKGVDPSIIGGIDVGVKSPLVCAINNAFSRYSISDNDLFHFNKKMFARRRILLKKSRHKRAGHGAKNKLKPISILTEKSERFRKKLIERWACEIANFFIKNKVGTVQMENLEGMKRKEDSYFNIRLRGFWPYAEMQNKIEFKLKQYGIEIRKVAPNNTSKTCSKCGHLNNYFNFEYRKKNKFPHFKCEKCNFKENADYNAALNISNPKLKSAKEEP

SEQ ID NO: 3262 - protein, 726 aa, synthetic construct
SEVEFSHEYWMRHALTLAKRARDEREVPVGAVLVLNNRVIGEGWNRAIGLHDPTAHAEIMALRQGGLVMQNYRLTDATLYVTFEPCVMCAGAMIHSRIGRVVFGVRNSKRGAAGSLMNVLNYPGMNHRVEITEGILMDECAALLCDFYRMPCQVLNAQKKARSNINSSGSSGSSSGSETPGTSESATPESSGGSSGGSAKNTITKTLKLRIVRPYNSAEVEKIVADEKNNREKIALEKNKDKVKEACSKHLKVAAYCTTQVERNACLFCKARRLDDKFYQKLRGQFPDAVFWQEIGEIFRQLQKQAAEIYNQSLIELYYEIFIKGKGFAIASSVEHYLSCVCYTRAAELFKNAAIASGLRGKVKSNFRLKELKNMKSGLPTTKSDNFPIPLVKQKGGQYTGFEISNHDSDFIIKIPFGRWQVKKEIDKYRPWEKFDFEQVRKSPKPISLLLSTQRRKRNKGWSKDEGTEAEIKRVMNGDYQISYIEVKRGSKIGEKSAWMLSLSVDVPKIDKGVDPSIIGGIDVGVKSPLVCAINNALSRYSISDNDLFHFNKKMFARRRILLRNNRHKRAGHGAESKLKPITILTEKGERFRKKLIERWVCEVADFFIKNKVGTVQMENLESMKRKEDSYFNIRLRGFWPYAEMQNKIEFKLKQYGIEIRKVAPNNTSKTCSKCGHLNNYFNFEYRKKNKFPHFKCEKCNFKENADYNAALNICNPKLKSTKEEP

SEQ ID NO: 3263 - protein, 726 aa, synthetic construct; identical to SEQ ID NO: 3199

SEQ ID NO: 3264 - protein, 726 aa, synthetic construct
SEAEFSHEYWMRHALTLAKRARDEREVPVGAVLVLNNRVIGEGWNRAIGLHDPTAHAEIMALRQGGLVMQNYRLVDATLYVTFEPCVLCAGAMVHSRIGRVVFGVRNNKRGAAGSLMNILNYPGMNHRVEITEGILADECAALLCDFYRMPRQVFNARKKARSNINSGGSSGGSSGSETLGTREGATPESTGGSSGGSAKNTITKTLKLRIVRPYNSAEVEKIVVDEKNNREKIAMEKNKDKVKEACSEHLKVAAYCTTQVERNACLFCKARKLDDKFYQKLRGQFPDAVFWQEIGEIFRQLQKQAAEIYNQSLIELYYEIFIKGKGFANASSVEHYLSDVCYTRAAELFKNAAIASGLRGKVRSNFRLKELKNMKSGLPTTKSDNFPIPLVKQKGGQHTGFEISSHNSDFIIKIPFGRWQVKEEIDKYRPWEKFDFEQVRKNPKPISLLLSTQRRKGNRGWSKDEGTEAEIRRVMNGDYQTSYIEVKRGSKIGEKSAWMLNLSIDVPKIDKGVDPSIIGGIDVGVKSPLVCAINNSSCRYSISDNELFHFNKKMFARRRILLKKNGHKRAGHGAKNKLKPISTLTERSKRFRKKLIERWACEIADFFIKNKVGTVQMENLESMKRKEDSYFNIRLRGFWPYAEMQNKIEFKLKQYGIEIRKVAPNNTSKTCSKCGHLNNYFNFEYRKKNKFPHFKCEKCNFKENADYNAALNISNPKLKSTKKEP

SEQ ID NO: 3265 - protein, 726 aa, synthetic construct
SEVEFSHEYWMRHALTLAKRARDEREVPVGAILVLNNRVIGVGWNRAIGLHDPTAHAEIMALRQGGLVMQNYRLTDATLYATFEPCVMCAGAMIHSRIGRVVFGVRNGKHGAAGSLMNVLNYPGMNHRVEITEGILADECAGLLCDFYRMPRQVFSARKKAQSSINPGGSSGGSSGSETPGASGSVIPKSSGGSSAGSTKDTITKTLKLRIVRPYNSAEVEKIVADEKNNREKIALEKNKDKVKEACSKHLKVAAYCTTQVERNACLFCKARRLDDKFYQKLRGQFPDAVFWQEIGEIFRQLQKQAAEVYNQSLVELYYEILIKGKGIANASSVEHYLSDVCYTRAAELFKNAAIASGLRNKIKSNFRLKELRNMKSGLPTTKSDNFPIPLVRQKGGQYTGFEISNHDGDFIIKIPFGRWQVKKEINKHRPWEKFDFEQVRKSPKPISLLLSTQRRKRNKGWGKDEGTEAEIRKVMNGDYQTSYIEVKRGNKTGEKSAWMLNLSIDVPKIDKGVDPSIIGGIDVGVKSPLVCAINNAFSRHSISDNDLFRFNKKMFARRRILLKRNRHKRAGHGAKNKLKPISILTEKSKRFRKKLIERWACEIADFFIKNKVGTVQMENLESMKRREDSYFNIRLRGLWPYAEMQNKIEFKLKQYGIEVRKVAPNNTSKTCSKCGHLNNYFNFEYRKKNKFPHFKCEKCNFKEDADYNAALNISNPKLKSTKEEP

SEQ ID NO: 3266 - protein, 726 aa, synthetic construct
SEVEFSHEYWMRHALTLAKRARDEREVPVGAILVLNNRVIGEGWNRAIGLHDPTAHAEIMALRQGGLVMQNYRLIDATLYVTFEPCVMCAGAMIHSRIGRVVFGVRNNKHGAAGSLVNVLNYPGMNHRVEITEGILADECAALLCDFYRMPHQVFNAWKKAQSSINPGGSSGGSSGSETPGTSESATPESSGGSSGSSAKNTITKTLKLRIVRPYNSAEVEKIVADEKNNREKIALEKNKDKVKGACSKHLKVAAYCTTQVGRNACLFCKARRLDDKFYQKLRGQFPDAVFWQEIGEIFRQLQKQAAEIYNQSLIELYYEIFIKGKGFANASSVEHYLSDVCYTRAAEQFKNAAIASGLRGKVKSNFRLKELKNMKSGLPTTKSDNFPIPLVKQKGGQYTGFEISSHNDDFIIKIPFGRWQVKKEIDKYRPWEKFDFEQVRKSPKPISLLLSTQRRKRNKGWSKDEGTEAEIRKVMYGDYQTSYIEVKRGSKTGEKSAWMLNLSIDVPKIDKGVDPSIIGGIDVGVKSPLVCAINNAFSRYSISDNDLFRFNKKMFARRRILLKKNRHKRAGHGAKNKLKPISILTGKSERFRKKLIERWACEIADFFTKNKVGTVQMENLESMKRKEDSYFNIRLRGFWPYAEMQNKIEFKLKQYGIEIRKVAPNNTSKTCSKCGHLNNYFNFEYRKKNKFPHFRCEKCNFKENADYNAALNISNPKLKSTKEEP

SEQ ID NO: 3267 - protein, 726 aa, synthetic construct
SEVEFSHEYWMRHALTLAKRARDEREVPVGAVLVLNNRVIGEGWNRTTGLHDPTAHAEIMALRQGGLAMQNHRLVDATLYVTFEPCVMCAGAMIHSRIGRVVFGVRNSKRGAAGSLTNVLNYPGMNHRVEITEGILVDECAALLCDFYRMPRQVFNAQKKAQSTINSGGSSGGSSGSETPGTSESATPESSGGGSSGSAKNTLTKTLQLRIVRPYNSAEVEKIVADEKNNREKIALEKNKDKVREACSKHLKVAAYCTTQVGRNACLFCKARRLDDKFYQKLRGQFPDAAFWQEIGEIFRQLQKQAAEVYNQSLVELYYEILIKGRGIANASSVEHYLSDVCYTRAAELFKNAAIASGLRNKIKSNFRLKELKNMKSGLPTTKSDNFPIPLVKQKGGQYTGFEISSHDDDFIIKIPFGRWQVKEEIDKYRPWEKFDFEQVRKNPKPISLLLSTQRRKGNKGWSKDEGTEAEIRKVMNGDYQTSYIEVKRGSKIGEKGAWMLNLSIDVPKIDKGVDPSIIGGIDVGVKSPLVCAINNAFSRYSISDNDLFRFNKKVFARRRILLKKNRHKRAGHGTKNKLKPITILTEKSGRFRKKLIERWACEIANFFIKNKVGTVQMENLESMKRKEDSYFNIRLRGFWPYAEMQNKIEFKLKQYGIKIRKVAPNNTSKTCSKCGHLNNYFSFEYRKKNKFPHFKCEKCNFKENADYNAALNISNPKLKSTKEEP

SEQ ID NO: 3268 - protein, 725 aa, synthetic construct
SEGEFSHEYWMRHALTLAKRARDGREVPVGAVLVLNNRVIGEGWNRAIGLHDPTAHAEIMALRQGGLVMQNYRLIDATLYVTFEPCVMCAGAMVHSRIGRVVFGVRNSKRGAAGSLMNVLDYPGMGHRVEITEGVLADECAALLCDFYCMPRQVFSAQKRAQSSINSGGSSGGSSGSETPGTSESATPESSGGGSSGSAKNTITKTLQLRIVRPYNSAEVEKIVADEKNNREKIALEKNKDKVKEACSKHLKVAAYCTTQVERNACLFCKARKLDDRFYQKLRGQFPDAVFWQEIGEIFRQLQKQAAEVYNQSLVELYYEIFIKGKGFASASSVEHYLSDVCYTRAAELFKNAAIASGLRGKVKGNFRLKELKNMKSGLPTTKSDNFPIPLVKQKGGQYTGFEISSHNDDFIIKIPFGRWVKKEIDKYRPWEKFDFEQVRKSPKPISLLLSTQRRKRNKGWSKDEGTEAEIRKVMNGDYQTSYIEVKRGSKIGEKSAWTLNLSIGVPKIDKGVDPSIIGGIDVGVKSPLVCAINNAFSRYSISDNDLFHFNKKMFARRRILLKKNRHKRAGHGAKNKLKPISILTEKSKRFRKKLIERWACEIADFFIKNKVGTVQMENLESMKRKEDSYFNIRLRGFWPYAEMQNRIEFKLKQYGIEIRKVAPNNTSKTCSKCGHLNNYFNFEYRKKNKFPHFKCEKCNFKENADYNAALNISNPKLKSTKEES

SEQ ID NO: 3269 - protein, 726 aa, synthetic construct
SEVEFSHEYWMRHALTLAKRARDEREVPVGAVLVLNNRVIGEGWNRAIGLHDPTAHAEIMALRQGGLVMQDYRLVNATLYVTFEPCVMCAGAMIHSRIGRVVFGVRNSKRGAAGSQMNVLNYPGMNHRVEITEGILADECAALLCDFYRMPRQVFNAQKKAQSYINSSGSSGGSSGSETPGTSESATPGSSGGSSGSSAKNTITKTLRLRIVRPYNSAEVEKIVADEKNNREKIALEKNKDKVKEACSKHLKVAAYCTTQVERNACLFCKARRLDDKFYQKLRGQFPDAVFWQEIGEIFRQLQKQAAEVYNQSLVELYYEILIKGKGIANASSVEHYLSDVCYTRAAELFKNAAIASGLRNKIKSNFRLKELRNMRSGLPTTKSDNFPIPLVRQKGGQYTGFEISNHDGDFIIKIPFGRWQVKEEINKHRPWEKFDFEQVRKSPKPISLLLSTQRRKRNRGWSKDEGTEAEIRKVMNGDYQTSYIEVKRGSKIGEKSAWMLNLSIDVPKIDKGVDPSIIGGIDVGVKSPLVCAINNAFSRYSISDNDLFRFNKKMFARRRILLKKNRHKRAGHGAKNKLKPITILTKKSERFRKKLIERWVCEVADFFIKNKVGTVQMENLESMKRKEDSYFNIRLRGFWPYAEMQNRIELKLKQYGIEIRRVAPNNTSRTCSKCGHLNNYFNFEYRKKNKFPHFKCEKCNFREDADYNAALNISNPKLKSTKEEP

SEQ ID NO: 3270 - protein, 726 aa, synthetic construct
SEVEFSHEYWMRRALTLAKRARDEREVPVGAVLVLNNRVIGVGWNRAIGLHDPTAHAEITALRQGGLVMQNYRLIDATLYVTFEPCVMCAGAMIHSRIGRVVFGVRNSKHGAAGSLVNVLNYPGMNHRVEITEGILADECAALLCDFYRMPRQVFNARKKAQPSINPGGSSGGSSGSETPGTSESATPESSGGSSGGSAKNTITKTLKLRIVRPYNSAEVEKIMADEKNNREKIALEKNKDKVKEACSKHLKVASYCTTQVERNACLFCKARKLDDKFYQKLRGQFPDAVFWQELGGIFRQLQKQAAEIYNQSLIELYYEIFIKGKGITNASRVEHYLSDVCYTRAAELFKNAAIASGLRSKVRSNFRLKELKNMKSGLPTTKSDNFPIPLVKQKGGQYTGFEISSHNSDFIIKIPFGRWQEKEEIDKYRPWEKFDFEQVRRSPKPISLLLSTQRRKKNKGWSKDEGTEAEIRRVMNGDYQTSYIEVKRGSKIGEKSAWMLNLSIDVPKIDKGVDPSIIGGIDVGVKSPLVCAINNAFSRYSISDNDLFHFNKKMFARRRILLKKNRRRRAGHGAKNKLKPITILTEKSVRFRKKLIERWACEIADFFIKNKVGTVQMENLESMKRKEDSYFNIRLRGFWPYAEMQNKIEFKLKQYGIEIRRVAPNNTSRTCSKCGHLNNYFNFEYRRKYKFPHFKCEKCNFKENADYNAALNISNPKLMSTKEGP

SEQ ID NO: 3271 - protein, 726 aa, synthetic construct
SEVEFSHEYWMRRALTLAKRARDEREVPVGAVLVLNNRVIGVGWNRAVGLHDPTAHAEIMALRQGGLVMQNYRLIEATLYVTFEPCIMCAGAMIHSRIGRVVFGVRNSKRGAAGSLMNVLNYPGMNHRVEITEGILVDECAALLCDFYRMPRQVLNAQKKAQSSISPGGSSGGSSGSETPGASESVTPKSSGGSSGGSAKNTITKTLKLRIVRPYNSAEVEKIVADEKNNREKIALEKNKGKVREACSKHLKVAAYCTTQVERSACLFCKARKLDDKFYQKLRGQFPDAVFWQEIGEIFRQLQKQAAEIYNQSLIELYYEIFIKGKGFANASSVEHYLSDVCYTRAAELFKNAAIASGLRGKVKSSFRLKELRNMKSGLPTTKSDNFPIPLVKQKGGQYTGFEISSHSDDFIIKIPFGRWQAKKEIDKHRPWEKFDFEQVRKSPKPISLLLSTQRRKRNKGWSKDEGTEAEIRKVMNGDYQISYIEVKRGSKTGEKSAWMLNLSIDVPKIDKGVDPSIIGGIDVGVKSPLVCAINNSSSRYSIRDNDLFRFNKKMFARRRILLKKNRRRRAGHGAKNKLKPITILTEKSVRFRKKLIERWACEIADFFIKNKVGTVQMENLESMKRKEDSYFNIRLRGFWPYAEMQNKIEYKLKQYGIKIRKVAPNNTSKTCSKCGHLNNHFSFEYRKKNKFPHFKCEKCNLKEDADYNAALNISNPKLKSTKEEP

SEQ ID NO: 3272 - protein, 726 aa, synthetic construct
SEVEFSHEYWMRHALTLAKRARDEREVPVGAILVLNNRVIGVGWNRAIGLHDPTAHAEIMALRQGGLVMQNYRLIDATLYVTFEPCVMCAGAMVHSRIGRVVFGVRNSKRGAAGSLMNVLNYPGVNHCVEITEGILVDECAALLCDFYRMPRQVFNAQKKAQSSINSGGSSGGSSGSETPGTSESATPESSGGSSGGSARNTITKTLQLRIVRPYNSAEVEKIVADEKNNREKIALEKNKDKVKEACSKHLKVAAYCTTQVERNACLFCKARRLDDKFYQKLRGQFPDAVFWQEISEIFRQLQKQAAEIYNQSLIELYYEIFIKGKGITNASRVEHYLSDVCYTRAAELFKNAAIASGLRSKVRGNFRLKELKNMKSGLPTTKSDNFPIPLVKQKGGQYTGFEISSHNSDFIIKIPFGRWQEKEEIDKYRPWEKFDFEQVRRSPKPISLLLSTQRRKKNKGWSKDEGTEAEIRRVMNGDYQTSYIEVKRGSKIGEKSAWMLNLSIDVPKIDKGVDPSIIGGIDVGVKSPLVCAINNAFSRYSISDNDLFHFNKKMFARRRILLKKNRRRRAGHGAKNKLKPITILTEKSVRFRKKLIERWACEIADFFIKNKVGTAQMENLESMKRREDSYFNIRLRGFWPYAEMQNKIEFKLKQYGIEIRKVAPNNTSKTCSKCGHLNNYFNFEYRKKNKFPHFKCEKCNFKENADYNAALNISNPKLKSTKEEP

SEQ ID NO: 3273 - protein, 726 aa, synthetic construct
SEVEFSHEYWMRHALTLAKRARDEREVPVGAVLVLNNRVIGEGWNRTTGLHDPTAHAEIMALRQGGLVMQNHRLVDATLYVTFEPCVMCAGAMIHSRIGRVVFGVRNGKRGAAGSLTNVLNYPSMNHRVEITEGILVDECAALLCDFYRMPRQVFNAQKKAQSTINSGGSSGGSSGSETPGTSESPTPESSGGSPGGSAKDTITKTLKLRIVRPYNSAEVEKIVADEKNNREKIALEKNKDKVKEACSKHLKVAAYCTTQVERNACLFCKARKLDDKFYQKLRGQFPDAVFWQEIGEIFRQLQKQAAEVYNQSLIELYYEIFIKGKGFANASSVEHYLSDVCYTRAAELFKNAAIASGLRGKVKSNFRLKELKNMKSGLPTTKSDNFPIPLVKQKGGQYTGFEISSHNDDFIIKIPFGRWQVKKEINKYRPWEKFDFEQVRKSPKPISLLLSTQRRKRNKGWSKDEGTEAEIRKVMNGDYQTSHIEVKRGSKTGEKSAWMLNLSIDVPKIDKGVDPSIIGGIDVGVKSPLVCAINNALSRYSIRDNDLFRFNKKMFARRRILLKKNRHKRAGHGAKNKLKPITILTEKSRRFRKKLIERWACEIADFFIKNKVGTVQMENLEGMKRKEDSYFNIRLRGFWPYAEMQNKIEFKLKQYGIEIRKVAPNNTSKTCSKCGHLNNYFNFEYRKKNKFPHFKCEKCSFKENADYNAALNISNPKLKSTKEEP

SEQ ID NO: 3274 - protein, 726 aa, synthetic construct
GEVEFSHEYWMRHALILAKRARDEREVPVGAVLVLNNRVIGVGWNRAIGLHDPTAHAEIMALRQGGLVMQNYRLIGATLYVTFEPCAMCAGAMIHSRIGRVVFGVRNSKRGAAGSLMNVLNHPGMNHRVEIMEGILTDECAALLCDFYRMPHQVLNAQKKAQSSINSGGSSGGSSGSETPGTSGSATPEGSGGSSGGSTKNTITKTLKLRIVRPYNSAEVEKIVADEKNNREKIALEKNKGKVKEACSKHLKVATYCTTQVERNACLFCKARKLDDKFYQKLRGQFPDAVFWQEVGEIFRQLQKQAAEIYNQSLIELYYEIFIKGKGIANASSVGHYLSDVCYTRAAELFKNAAIASGLRGKVKSNFRLKELRNMKSSLPTTKSDNFPIPLVRQKGGQYTGFEISNHNGDFIIKIPFGRWQVKKEICKHRPWEKFDFEQVRKSPKPISLLLSTQRRKRNKGWGKDEGTEAEIRKVMNGDYQTSYIEVKRGSKIGEKSAWMLNLSIDVPKIDKGVDPSIIGGIDVGVKSPLVCAINNAFSRYSISDNDLFRFNKKMFARRRILLGKNRHKRAGHGVKNKLKPITILTEKSGRFRKKLIERWACEIADFFIKNKVGTVQMENLESMKRKEDSYFNIRLRGFWPYAEMQNKIEFKLKQYGIKIRKVAPNNTSKTCGKCGHLNNYFSFEYRKKNKFPHFKCEKCNFKEDADYNAALNISNPKLKSTKEEP

SEQ ID NO: 3275 - protein, 726 aa, synthetic construct
SEVEFSHEYWMRHALTLAKRARDEREVPVGAILVLNNRVIGEGWNRAIGLHDPTAHAEIMALRQGGLVMQNYRLIDATLYVTFEPCVMCAGAMIHSRIGRVVFGVRNNKHGAAGSLVNVLNYPGMNHRVEITEGILADECAALLCDFYRMPRQVFNARKKAQSSINPGGSSGGSGGSETPGTSESATPESSGGSSGSSAKNTITKTLKLRIVRPYNSAEVEKIVADEKNNREKIALEKNKDKVKEACSKHLKVAAYCTTQVERNACLFCKARKLDDRFYQKLRGQFPDAVFWQEIGEIFRQLQKQAAEIYNQSLIELYYEIFIKGRGFANASSVEHYLSDVCYTRAAELFKNAAIASGLRGKVKSNFRLKELKNMKSGLPTTKSDNFPIPLVKQKGGQYTGFEISSHNDDFIIKIPFGRWQVKKEIDKYRPWEKFDFEQVRKSPKPISLLLSTQRRKRNKGWGKDEGTEAEIRKVMNGDYRTSYIEVKRGSKTGEKSAWMLNLSIDVPKIDKGVDPSIIGGIDVGVKSPLVCAINNAFSRYSISDNDLFRFNKKMFARRRILLKKNRHKRAGHGAKNKLKPITILTKKSERFRKKLIERWVCEVADFFIKNRVGTVQMENLESMKRKEDSYFNIRLRGFWPYAEMQNRIELKLKQYGIEIRRVAPNNTSRTCSKCGHLNNYFNFEYRKKNKFPHFKCEKCNFKENADYNAALNISNPKLKSTKKEP

SEQ ID NO: 3276 - protein, 725 aa, synthetic construct
SEVEFSHEYWMRHALTLAKRARDEREVPVGAILVLNNRVIGEGWNRAIGLHDPTAHAEIMALRQGGLVMQNYRLIDATLYVTFEPCVMCAGAMIHSRIGRVVFGVRNSKHGAAGSLVNVLNYPGMNHRVEITEGILADECAALLCDFYRMPRQVFSVRRKAQSSISPGGSSGGSSGSETPGTGKSPTPESPGGSSGGSAKNTITKTLKLRIVRPYNSAEVEKIVADEKNNREKIALEKNKDKVKEACSEHLKVAAYCTTQVERSACLFCKARKLDDKFYQKLRGFPDAVFWQEIGEIFRQLQKQAAEIYNQSLIELYYEIFIKGKGFANASSVEHYLSDVCYTRAAELFKNAAIASGLRGKVKSNFRPKELKNMKSGLPTTKSDNFPIPLVKQKGGQYTGFEISSHNDDFIIKIPFGRWQVKEEIDKYRPWEKFDFEQVRKNPKPISLLLSTQRRKGNKGWSKDEGTEAEIRKVMNGDYQTSYIEVKRGSKIGEKSAWMLNLSIDVPKIDKGVDPSIIGGIDVGVKSPLVCAINNALSRYSISDNDLFHFNKKMFARRRILLRKNRHKRAGHGARNKLKPITVLTEKSERFRKKLIERWACEIANFFIKNKVGTVQMENLESMKRKEDSYFNIRLRGFWPYAEMQNKIEFKLKQYGIEIRKVAPNNTSKTCSKCGHLNNYFNFEYRKKNKFPHFKCEKCNFKENADYNAALNISNPKLKSPKEEP

SEQ ID NO: 3277 - protein, 725 aa, synthetic construct
SEDEFSHEYWMRHALTLAKRARDRREVPVGAVLVLNNRVIGEGWNRAIGLHDPTAHAEIMALRQGGLVMQNYRLIDATLYVTFEPCVMCAGAMVHSRIGRVVFGVRNSKRGAAGSLMNVLDYPGMGHRVEITEGILADECAALLCDFYCMPRQVFNAQKRAQSGISSGGSSGGSSGSETPGASGSVTPKSSVGSSAGSTRNTITKTLKLRIVRPYNSAEVERIVADEKNNREKIALEKNKDKVKEACSKHLKVAAYCTTQVERNACLFCKARKLDDKFYQKLRGQFPDAVFWQEISEILRQLQKQAAEIYNQSLIELYYEIFIKGKGFANASSVEHYLSDVCYTRAAELFKNAAIASGLRGKVKSNFRLKELKNMKSGLPTTKSDNFPIPLVKQKGGQYTGFEISSHNDDFIIKIPFGRWQVRKEIDKYRPWEKFNFEQVRKSPKPISLLLSTQRRKRNKGWSKDEGTEAEIRKVMNGDYQTSYIEVKRGSKIGEKSSWMLSLSIDVPKIDKGVDPSIIGGIDVGVKSPLVCAINNAFDRYSISDNSLFHFNKKMFARRRILLKKNRHRAGHGAKNKLKPITILTEKSVRFRKKLIERWACEIADFFIKNKVGTVQMENLESMKRKEDSYFNIRLRGFWPYAEMQNKIEFKLKQYGIEIRKVAPNNTSKTCSKCGHLNNYFNFEYRKKNKFPHFKCEKCNFKENADYNAALNISNPKLKGTKEEP

SEQ ID NO: 3278 - protein, 726 aa, synthetic construct
SEVEFSHEYWMRHALALAKRARDEREVPVGAVLVLNNRAIGEGWNRAIGLHDPTAHAEIMALRQGGLVMQNYRLTDATLYVTFEPCVMCAGAMIHSRIGRVVFGVRNSKRGAAGSLMNVLNYPGMNHCVEITEGILVDECAALLCDFYRMPRQVLNAQKKAQSSISSGGSSGGSSGSETPGASGSVIPRSSGGSSAGSTKDTITKTLKLRIVRPYNSAEVEKVVADEKNNREKIAMEKNKDKVKEACSKHLKVASYCTTQVERNACLFCKARKLDDKFYQKLRGQFPDAVFWQETGEIFRQLQRQAAEIYNQSLIELYYEIFIKGKGFANASSVEHYLSDVCYTRAAELFKNAAIASGLRGKVKSNFRLKELKNMKSGLPTTKSDNFPIPLVKQKGGQYTGFEISSHNDDFIIKIPFGRWQVKKEIDKYRPWEKFDFEQVRKSPKPISLLLSTQRRKRNKGWSKDEGTEAEIRKVMNGDYQTSYIEVKRGSKIGEKSAWMLNLSIDVPKIDKGVDPSIIGGIDVGVKSPLVCAINNAFSRYSISDNDLFRFNKKMFARRRILLGKNRHKRAGHGVKNKLKPITILTGKSGRFRKKLIERWACEIADFFIKNKVGTVQMENLESMKRKEDSYFNIRLRGFWPYAEMQNKIEFKLKQYGIEIRKVAPNNTSKTCSKCGHLNYYFNFEYRKKNKFPHFKCEKCNFKEDADYNAALNISNPKLKSTKEEP

SEQ ID NO: 3279 - protein, 726 aa, synthetic construct
SEVEFSHEYWMCHALTLAKRARDEREVPVGAVLVLNNRVIGVGWNRAVGLHDPTAHAEIMALRQGGLVMQNYRLIEATLYVTFEPCIMCAGAMVHSRIGRVVFGVRNSKRGAAGSLMNVLNYPGMNHRVEITEGILADECAALLCDYYRMPRQVFNARKKVQSSINSGGSSGGGSGSETPSTSESATPESSGGSSGGSAKNTITKTLKLRIVRPYNSAEVEKIVADEKNNREKIALEKNKDKVKEACSKHLKVAAYCTTQVERNACLFCKARRLDDKFYQKLRGQFPDAVFWQEIGEIFRQLQKQAAEIYNQSLIELYYEIFIKGRGFANASSVEHYLSDVCYTRAAELFKNAAIASGLRGKVKSNFRLKELKNMKSGLPTTKSDNFPIPLVKQKGGQYTGFEISSHNDDFIIKIPFGRWQVKKEIVKYRPWEKFDFEQVRKSPKPISLLLSTQRRKRNKGWSKDEGTEAEIKRVMNGDYQTSYIEVKRGSKIGEKSAWLLNLSIDVPKIDKGVDPSIIGGIDVGVKSPLVCAINNAYSRYSISDNDLFRFNKKVFARRRILLKKNRHKRAGHGTKNKLKPITILTEKSGRFRKKLIERWACEIANFFIKNKVGTVQMENLESMKRKEDSYFNIRLRGFWPYAEMQNRIELKLKQYGIEIRRVAPNNTSRTCSKCGHLNNYFNFEYRKKNKFPHFKCEKCNFREDADYNAALNISNPKLKSTKEEP

SEQ ID NO: 3280 - protein, 726 aa, synthetic construct
SEVEFSHEYWMRHALTLAERARDEREVPVGAVLVLNNRVIGVGWNRAIGLHDPTAHAEIMALRQGGLVMQNYRLIDATLYVTFEPCAMCAGAMVHSRIGRVVFGVRNSKRGAAGSLMNVLNYPGMDHRVEITGGILADECAALLCDFYRMPRRVFNAQKKAHSSINSGGSSGGSSGSVTPGTSESATPESSGGGFGGSAKNTITKTLQLRIVRPYNSAEVEKIVADEKNNRERIALEKNKDKVKEACSKHLKVAAYCTTQVERNACLFCKARKLDDKFYQKLRGQFPDAVFWRETGEIFRQLQRQAAEIYNQSLIELYYEIFIKGKGLANASSVEHYLSDVCYTRAAELFKNAAIASGLRGKVKSNFKLKELKSMKSGLPSTKSDNFPIPLVKQRGGQYTGFEISSHNDDFIIKIPFGRWQMKKEIDRYRPWEKFDFEQVRKSPKPISLLLSTQRRKRNKGWSKDEGTEAEIRKVMNGDYQTSYIEVKRGSKIGEKSAWMLSLSIDVPKIDKGVDPSIIGGIDVGVKSPLVCAINNAFRRYSISDNDLFHFNKKMFARRRILLKKSRHKRAGHGAKNKLKPISILTEKSKRFRKKLIERWACEIADFFIKNKVGTVQMENLESMKRKEDSYFNIRLRGFWPYAEMQNKIEFKLKQYGIEIRKVAPNNTSKTCSKCGHLNNYFNFEYRKKNKFPHFKCEKCNFKENADYNAALNISNPMLKSTKEEP

SEQ ID NO: 3281 - protein, 726 aa, synthetic construct
SEVEFSHEYWMRRALTLAKRARDEREVPVGAVLVLNNRVIGVGWNRAVGLHDPTAHAEIMALRQGGLVMQNYRLIDATLYVTFEPCIMCAGAMIHSRIGRVVFGVRNSKRGAAGSLMNVLNYPGMNHRVEITEGILADECAALLCDFYRMPRQVFNARKKAQSSINPGGSSGGSSSSETPGTSESPTPESSGGSSGGSAKSTITKTLRLRIVRPYNSAEVEKIVADEKNNREKIALEKNKDKVKEACSEHLKVAAYCTTQVERNACPFCKARKLDDKFYQKLRGQFPDAVFWQEIGEIFRQLQKQAAEVYNQSLIELYYEIFIKGKGFANASSAEHYLSDVCYTRAAELFKNAAIASGLRGKVKSNFRLKELKNMKSGLPTTKSDNFPIPLVKQKGGQYTGFEISNHNDDFIIKIPFGRWQVKKEIDKYRPWEKFDFEQVRKSPKPISLLLSTQRRKKNKGWSKDEGTEAEIRRVMNGDYQTSYIEVKRGSKTGERSAWMLNLSIDVPKIDKGVDPSIIGGIDVGVKSPLVCAINNAFSRYIISDNDLFRFNKKMFARRRILLKKNRHKRAGHGAKNKLKPISILTGKSERFRKKLIERWACEIADFFIKNKVGTVQMENLEGMKRKEDSYFNIRLRGFWPYAEMQNKIEFKLKQYGIEIRKVAPNNTSKTCSKCGHLNNYFNFEYRKKNKFPHFKCEKCNFKENADYNAALNISNPKLKSTKEEP

SEQ ID NO: 3282 - protein, 726 aa, synthetic construct
SEVEFSHEYWMRHALTLAKRARDEREVPVGAVLVLNNRVIGEGWNRTTGLHDPTAHAEIMALRQGGLVMQNHRLVDATLYVTFEPCVMCAGAMIHGRIGRVVFGVRNSKRGAAGSLMNVLNYPGMNHCVEITEGILVDECAALLCDFYRMPRQVLNAQKKAQPSISSGGLSGGSSGSETPGASGSVIPKSSGGSSAGPTKDTITKTLKLRIVRPYNSAVVEKIVADEKNSREKIALEKNKDKVKEACSRHLKVAAYCTTQVERNACLFCKARRLDDKFYQKLRGQFPDAVFWQEIGEIFRQLQKQAAEVYNQSLVELYYEILIKGKGIANASSVEHYLSDVCYTRAAELFKNAAIASGLRNKIKSNFRLKELRNMKSGLPTTKSDNFPIPLVRQKGGQYTGFEISNHDGDFIIKIPFGRWQVKKEINKHRPWEKFDFEQVRKSPKPISLLLSTQRRKRNRGWGKDEGTEAEIRKVMNGDYQTSYIEVKRGSKIGEKSAWMLSLSIDVPKIDKGVDPRIIGGIDVGVKSPLVCAINNAFSRYSISDNDLFHFNKKMFARRRILLKKNRHKRAGHGAKNKLKPITILTEKSVRFRKKLIERWACEIADFFIKNKVGTVQMENLESMKGKEDSYFNIRLRGFWPYAEMQNKIEFKLKQYGVEIRKVAPNNTSKTCSKCGHLNNYFNFEYRKKNKFPHFKCEKCYFKEDADYNAALNISNPRLKSTKEEP

SEQ ID NO: 3283 - protein, 726 aa, synthetic construct
SEVEFSHEYWMRHALTLAKRARDEREVPVGAVLVLNNRVIGEGWNRAIGLHDPTAHAEIMALRQGGLVMQNHRLVDATLYVTFEPCVLCAGAMVHSRIGRVVFGVRNSKRGAAGSLMNVLNYPGMNHRVEITEGILADECAALLCDFYHMPRQVFNGRKKARSSINSGGSSGGSSGSETPGTSESATPESSGGSSSGSTKNTITKTLKLRIVRPYNSAEVEKIVADEKNNREKIALEKNKDKVKEACSKHLKVASYCTTQVERNACLFCKARKLDDKFYQKLRGQFPDAVFWREISEIFRQLQKQAAVIYNQSLIELYYEILIKGKGIANASRVEHYLSDVCYTRAAELFKNAAIASGLRSKVRSNFRLKELKSMKSGLPTTKSDNFPIPLVKQKGGQYTGFEISSHNSDFIIKIPFGRWQVKKEIDKYRPWEKFDFGQVRKSPKPISLLLSTQRRKGNKGWSKDEGTEAEIRKVMNGDYQTSYIEVKRGSKTGEKSAWMLNLSIDVPKIDKGVDPSIIGGIDVGVKSPLVCAINNGLSRYSISDNDLFHFNKKMFARRRILLKKNRHRRAGHGARNKLKPITVLTEKSKRFRKKLIERWACEIANFFARNKVGTVQMENLESMKRKEDSYFNIRLRGLWPYAEMQNKIEFKLKQYGIEVRKVAPNNTSKTCSKCGHLNNYFNFEYRKRNKFPHFKCEKCNFKENADYNAALNISNPKLKSTKEEP

SEQ ID NO: 3284 - protein, 726 aa, synthetic construct
SEVEFSHEYWMRHALTLAKRARDEREVPVGAILVLNNRVIGEGWNRAIGLHDPTAHAEIMALRQGGLVMQNYRLIDATLYVTFEPCVMCAGAMVHSRIGRVVFGVRNSKRGAAGSLMNVLNHPGMNHRVEITGGILADECAALLCDFYRMPRQVFNAQKKARSNINSGGSSGGSSGSETLGTSESATPESSGGSSGGSAKNTITKTLKLRIVRPYNSAEVEKIVADEKNNREKIALEKNKDKVKEACSEHLKVAAYCTTQVERNACLFCKARKLDDKFYQKLRGQFPDAVFWQELGEILRQLQKQAAEIYNQSLVELYYEIFIKGRGFANASSVEHYLSDVCYTRAAELFKNAAIASGLRGKVKSNFRLKELKNMKSGLPTTKSDNFPIPLVKQKGGQYTGFEISSHNDDFIIKIPFGKWQVKKEIDKYRPWEKFDFEQVRKSPKPISLLLSTQRRKRNKGWSKDEGTEAEIRKVMNGDYQTSYIEVKRGSKIGEKSAWMLSLSIDVPKIDKGVDPSIIGGIDVGVKSPLVCGINNALSRYSISDNDLFHFNKKMFARRRILLKKNRHRRAGHGAKNKLKPITILTEKSKRFRKKLIERWACEIADFFIKNKVGTVQMENLESMKRREDSYFNIRLRGFWPYAKMQNKIEFKLKQYGIEIRKVAPNNTSKTCSKCGHLNNYFNFEYRKKNKFPHFKCEKCNFKESADYNAALNISNPKLKSTKEEP

SEQ ID NO: 3285 - protein, 726 aa, synthetic construct
SEVEFSHEYWMRHALTLAKRARDDREVPVGAVLVLNNRVIGEGWNRAIGLHDPTAHAEIMALRQGGLVMQNYRLVDATLYVTFEPCVLCAGAMVHSRIGRVVFGVRNSKRGAAGSLMNVLNYPGMNHRVEITEGILADECAALLCDFYRMPRQVFNARKKARSNINSGGSSGGSSGSETPGTSESATPESSGGSSGGSAKNTITKTLTLRIVRPYNSAEVEKIVADEKNNREKIALEKNKDKVKEACSEHLKVATYCTTQVERNACLFCKARKLDDKFYQKLRGQFPDAVFWQELGEIFRQLQKQAAEIYNQSLIELYYEIFIKGKGFANASSVEHYLSDVCYTRAAELFKNAAIASGLRGKVKSNFRLKELRNMKSGLPTTKSDNFPIPLVRQKGGQYTGFEISSRNDDFIIKVPFGRWQVKKEIDKYRPWEKFDFEQVRKSPKPISLLLSTQRRKRNKGWCKDEGTEAEIKKVMNGDYQTSYIEVKRGSKVGEKSVWMLSLSIDVPKIDKGVDPSIIGGIDVGVKSPLVCAISNAFSRYSISDNDLFHFNKKMFARRRILLKKSKHKRAGHGAKNKLKPITILTEKSRRFRKKLIERWACEIADFFIKNKVGTVQMENLESMKRKEDSYFNIRLRGFWPYAEMQNKIEFKLKQYGIEIRKVAPNNTSKTCSKCGHLNNYFNFEYRKKNKFPHFKCEKCNFKENADYNAALNISNPKLKSTKEEP

SEQ ID NO: 3286 - protein, 726 aa, synthetic construct
SEVEFSHEYWMRHALTLAKRARDEREVPVGAILVLNNRVVGEGWNRAIGLHDPTAHAEIMALRQGGLVMQNYRLTDATLYVTFEPCVMCAGAMIHSRIGRVVFGVRNSKHGAAGSLVNVLNYPGMNHRVEITEGILADECAALLCDFYRMPRQVFNARKKAQSSINPGGSSGGSSGSETPGTSESATLENSGGSSAGSTKDTITKTLKLRIVRPYNSAEVEKIVTDEKNSREKIALERNKDKVKEACSEHLKVAAYCTTQVERNACLFCKARKLDDRFYQKLRGQFPDAVFWQETGEIFRQLQRQAAEIYNQSLIELYYEIFIKGKGFANASSVEHYLSDVCYTRAAELFKNAAIASGLRGKVKSNFRLKELKNMKSGLPTTKSDNFPIPLVKQKGGQYAGFEISSHDGDFIIKIPFGRWQAKEEIDKYRPWEKFDFEQVRKSPKPISLLLSTQRRKRNKGWSKDEGTEAEIKKVMNGDYQTSYIEVKRGRKIGEKSVWMLNLSIDVPKIDKGVDPSTIGGIDVGVKSPLVCAINNAFSRYSISDNDLFRFNKKMFARRRILLKKSKHKRAGHGAKNKLKPITILTEKSGRFRKKLIERWACEIADFFIKNKVGTVQMENLEGMKRKEDSYFNIRLRGFWPYAEMQNKIEFKLKQYGIKIRKVAPNNTSKTCSKCGHLNNYFSFEYRKKSKFPHFKCEKCNFKEDADYNAALNISNPKLKSTKEEP

SEQ ID NO: 3287 - protein, 726 aa, synthetic construct
SEVEFSHEYWMRHALTLAKRARDEREVPVGAVLVLNNRVIGEGWNRTTGLHDPTAHAEIMALRQGGLVMQNHRLVDATLYVTFEPCVMCAGAMIHSRIGRVVFGIRNSKRGAAGSLTNVLNYPGMNHRVEITGGILADECAALLCDFYRMPRQVFNAQKKARSNINPGGSSGGSSGSETLGTSESATPESSGGSSGGSAKNTITKTLKLRIVRPYNSAEVEKIVADEKNNREKIALEKNKDKVKEACSEHLKVAAYCTTQVGRNACLFCKARKLDDKFYQKLRGQFPDAVFWQEISEIFRQLQKQAAEIYNQSLIELYYEIFIKGRGFANASSVEHYLSDVCYTRAAELFKNAAIASGLRGKVKSNFRLKELKNMKSGLPTTKSDNFPIPLVKQKGGQYTGFEISSHNDDFIIKIPFGRWQVKKEIDKYRPWEKFDFEQVRKSPKPISLLLSTQRRKRNKGWSKDEGTEAEIRKVMNGDYQTSYIEVRRGSKTGERSAWMLNLSIDVPKIDKGVDPSIIGGIDVGVKSPLVCAINNAFSRYSISDNDLFRFNKKMFARRRILLKKNRHKRAGHGAKNKLKPISILTGKSVRFRKKLIERWACEIADFFIRNKVGTVQMENLESMKRKEDSYFNIRLRGLWPYAEMQNKIEFKLKQYGIEVRKVAPNNTSKTCSKCGHLNNYFNFEYRKKNKFPPFKCEKCNFKEDADYNAALNISNPKLKGTKEEP

SEQ ID NO: 3288 - protein, 726 aa, synthetic construct
SEVEFSHEYWMRHALTLAKRARDEREVPVGAVLVLNNRAIGEGWNRAIDLHDPTAHAEIMALRQGGLVMQNYRLTDATLYVTFEPCVMCAGAMIHSRIGRVVFGVRNSKRGAAGSLMNVLNYPGMNHCVEITEGILVDECAALLCDFYRMPRQVLNAQKKAQSSISSGGSSGGSSGSETPGASGSVIPKSSGGSSAGSTKDTITKTLKLRIVRPYNSAEVEKVVADEKNNREKIAMEKNKDKVKEACSKHLKVASYCTTQVERNACLFCKARRLDDKFYQKLRGQFPDAVFWQEIGEIFRQLQKQAAEIYNQSLIELYYEIFIKGKGFANASSVEHYLSDVCYTRAAELFKNAAVASGLRGKVKSNFRLKELKNMKSGLPTTKSDNFPIPLVRQKGGQYTGFEISSHNDDFIIKIPFGRWQVKKEIDKYRPWEKFDFEQVRKSPKPISLLLSTRRRKRNKGWSKDEGTEAEIRKVMNGDYQTSYIEVKRGSKTGEKSAWMLNLSIDVPKIDKGVDPSIIGGIDVGVKSPLVCAINNAFSRYGISDNDLFRFNKKMFARRRILLKKNRHQRAGHGAKNKLKPITILTEKSGRFRKKLIERWACEIADFFIKNKVGTVQMENLESMKRKEDSYFNIRLRGFWPYAEMQSKIEFKLKQYGIKIRKVAPNNTSKTCSKCGHLNNYFSFEYRKKNKFPHFKCEKCNFKENADYNAALNISNPKLKSTKEEP

SEQ ID NO: 3289 - protein, 726 aa, synthetic construct
SEVEFSHEYWMRHALTLAKRARDEREVPVGAILVLNNRVIGEGWNRAIGLHDPTAHAEIMALRQGGLVMQNYRLIDATLYVTFEPCVMCAGAMIHSRIGRVVFGVRNSKHGAAGSLVNVLNYPGMNHRVEITEGILADECAALLCDFYRMPRQVFGARRKAQSSINPGGSSGGSSGSETTGTSESATPESSGGSSGGSAKNTITKTLKLRIVRPYNSAEVEKIVADEKNNREKIALEKNKDKVKEACGKHLKVASYCTTQVERNACLFCKARKLDDKFYQKLRGQFPDAVFWQELGEIFRQLQKQAAEIYNQSLIELYYEIFIKGKGLANASSVEHYLSDVCYTRAAELFKNAAIASGLRGKVKSNFKLKELKSMKSGLPSTKSDNFPIPLVKQKGGQYTGFEISSYNDDLIIKIPFGRWQVKKEIDKYRPWEKFDFEQVRKSPKPISLLLSTQRRKRNKGWSKDEGTEAEIRKVMNGDYQTSYIEVKRGNKIGEKSAWMLNLSIDVPKIDKGVDPSIIGGIDVGVKAPLVCAINNAFSRYSISDNDLFRFNKKVFARRRILLKKSKHKRAGHGAKNKLKPITILTEKSGRFRKKLIERWACEIANFFIKNKVGTVQMENLESMKRKEDSYFNIRLRGFWPYAEMQNKIEFKLKQYGIEIRKVAPNNTSKTCSKCGHLNNYFNFEYRKKNKFPHFKCEKCNFKENADYNAALNISNPKLKSTKEEP

SEQ ID NO: 3290 - protein, 726 aa, synthetic construct
SEVEFSHEYWMRHALTLAERARDEREVPVGAVLVLDNRVIGEGWNRAIGLHDPTAHAEIMALRQGGLVMQNYRLVDATLYVTFEPCVLCAGAMVHSRIGRVVFGVRNSKRGAAGSLMNVLNYPGMNHRVEITEGILADECAALLCDFYRMPRQVFNAQKKAQSNINSGGSPGGSSGCETPGTSESPTPESSGGCSGGSAKNTITKTLKLRIVRPYNSAEVEKIVADEKNNREKIALEKNKGKVKEACSKHLEVAAYCTTQVERNACLFCRARKLDDKFYQKLRGQFPDAVFWQELGEIFRQLQKQAAEIYNQSLIELYYEIFIKGKGIANASSVEHYLSDVCYTRAAELFKNAAIASGLRNKIKSNFRLKELRNMKSGLPTTKSDNFPIPLVRQKGGQYTGFEISNHNGDFIIKIPFGRWQVKKEISKHRPWEKFDFEQVRKSPKPISLLLSTQRRKRNKGWGKDEGTEAEIRKVMNGDYQTSYIEVKRGSKIGEKSAWVLNLSIDVPKIDKGVDPSVIGGIDVGVKSPLVCAISNAFSRYSISDNDLFHFNKKMFARRRILLKKSKHKRAGHGAKNKLKPITILTEKSGRFRKKLIERWACEIANFFIKNKVGTVQMENLESMKRKEDSYFNIRLRGFWPYAEMQNKIEFKLKQYGIEIRKVAPNNTSRTCSKCGHLNNYFNFEYRKKNKFPHFKCEKCNFREDADYNAALNISNPKLKSTKEEL

SEQ ID NO: 3291 - protein, 726 aa, synthetic construct
SEVEFSHEYWMRHALTLAKRARDEREVPVGAVLVLNNRVIGEGWNRAIGLHDPTAHAEIMALRQGGLVMQNYRLTDATLYVTFEPCVMCAGAMIHSRIGRVVFGVRNSKRGAAGSLMNVLNYPGMNHCVEITEGILMDECAALLCDFYRMPRQVLNAQRKAQSSISSGGSSGGSSGSETPGASGSVTPKSSGGSSAGSTRDTITKTLKLRIVRPYNSAEVEKIVADEKNSREKIALEKNKDKVKEACSEHLKVAAYCTTQVERNACLFCKARKLDDGFYQKLRGQFPDAVFWQEIGEIFRQLQKQAAEIYNQSLIELYYEIFIKGKGIANASSVGHYLSDVCYTRAAELFKNAAIASGLRSKIKSNFRLKELRNMRGGLPTTKSDNFPIPLVKQKGGQYTGFEISSHNDDFIIKIPFGRWQVKKEIDKYRPWEKFDFEQVRKSPKPISLLLSTQRRKRNKGWSKDEGTEAEIRKVMNGDYQTSYIEVKRGSKIGEKSAWTLSLSIDVPKIDKGVDPSIIGGIDVGVKSPLVCAINNAFCRYSISDNDLFHFNEKMFARRRILLKKSRHKRAGHGAKNKLKPISILTEKSKRFRKKLIERWACEIADFFIKNKVGTVQMENLESMKRKEDSYFNIRLRGFWPYAEMQNKIEFKLKQYGIEIRKVAPNNTSKTCSKCGHLNNYFNFEYRKKNKFPHFKCEKCSFKEDADYNAALNISNPKLKSTKEEP

SEQ ID NO: 3292 - protein, 726 aa, synthetic construct
SEVEFSHEYWMRHALTLAKRARDGREVPVGAVLVLNNRVIGEGWNRAIGQHDPTAHAEIMALRQGGLVMQNYRLIDATLYVTFEPCVMCAGAMIHSRIGRVVFGVRNSKHGAAGSLMNVLNYPGMNHRVETTEGILAEECAALLCDFYRMPRQVFNAQKKAQSTINSGSSSGGSSGSETPGTSESATPENSGGSSGSSAKNTITKTLKLRIVRPYNSAEVEKIVADEKNNREKIALEKNKDKVKEACSKHLEVAAYCTTQVERNACLFCKARKLDDKFYQKLRGQFPDAVFWQELGEIFRQLQKQAAEIYNQSLIELYYEIFIKGKGFANASSVEHYLSDVCYTRAAELFKNAAIASGLRGKVKSNFRLKELKNMKSGLPTTKSNNFPIPLVKQKGGQYTGFEISNHNGDFIIKIPFGRWQVKKEIDKYRPWEKFDFEQVRKSPKPISLLLSTQRRKRNKGWSKDEGTEAEIRRVMNGDYQTSYIEVKRGSKTGEKSAWMLNLSIDVPKIDKGVDPSIIGGIDVGVKSPLVCAINNALSRYSISDNDLFHFNKKMFARRRILLKKNRHRRAGHGARNKLKPITVLTEKSKRFRKKLIERWACEIVNFFIKNKVGTVQMENLEGMKRKEDSYFNIRLRGLWPYAEMQNKIEFKLKQYGIEIRKVAPNNTSKTCSKCGHLNNYFSFEYRKRNKFPHFKCEKCNFKENADYNAALNISNPKLKGTKEEP

SEQ ID NO: 3293 - protein, 726 aa, synthetic construct
SEVEFSHEYWMRHALTLAKRARDEREVPVGAVLVLNNRVIGEGWNRTTGLHDPTAHAEIMALRQGGLVMQNHRLVDATLYVTFEPCVMCAGAMIHSRIGRVVFGVRNSKRGAAGSLTNVLNYPGMNHRVEITEGILVDECAALLCDFYRMPRQVFNAQKKAQSTINSDGLSGGSSGSETPGTSESPTPESSGGSPGGSAKNTITKTLQLRIVRPYNSAEVEKIVADEKNNREKIALEKNKDKVKEACSKHLKVATYCTTQVERSACLFCKARKLDDKFYQKLRGQFPDAVFWQEISEIFRQLQKQAAEIYNRSLIELYYEIFIKGKGFANASSVEHYLSDVCYTRAGELFKNAAIASGLRGKVKSNFRLKELKNMKSGLPTTKSGNFPIPLVKQKGSQYTGFEISSHNDDFIIKIPFGRWQVKKEIDKYRPWEKFDFEQVRKSPKPISLLLSTQRRKRNKGWSKDEGTEAEIRRVMNGDYRTSYIEVKRGSKTGEKSAWMLNLSIDVPKIDKGVDPSIIGGIDVGVKSPLVCAINNSSSRYSICDNDLFRFNKKMFARRRILLKKNRHKRAGHGAKNKLKPITILTKKSERFRKKLIERWVCEVADFFIKNKVGTVQMENLESMKRKEDSYFNIRLRGFWPYAEMQNRIEFKLKQYGIEIRKVAPNNTSKTCSRCGHLNNYFNFEYRKKNKFPHFKCEKCSFKENADYNAALNISNPKLKSTKEEP

SEQ ID NO: 3294 - protein, 726 aa, synthetic construct
SEVEFSHEYWMRHALTLAKRARDEREVPVGAILVLNNRVIGEGWNRAIGLHDPTAHAEIMALRQGGLVMQNYRLIDATLYVTFEPCVMCAGAMIHSRIGRVVFGVRNSKHGAAGSLVNVLNYPGMNHRVEITEGILADECAALLCNFYRMPRQVFNVRKKAQSSINPGGSSGGSSGSETPGTSESATPESSGGSSGGSAKNTITKTLKLRIVRPYNSAEVEKIVADEKNNREKIALEKNKDKVKEACSKHLKVAAYCTTQVERNACLFCKARRLDDKFYQKLRGQFPDAVFWQEIGEIFRQLQKQAAEIYNRSLIELYYEIFIKGKGIANASRVGHYLSDVCYTRAAELFKNAAIASGLRNKIKSNFRLKELKNMKSGLPTTKSDNFPIPLVKQKGGQYTGFGISSHNSDFVIKIPFGRWQVKEEIDKYRPWEKFDFEQVRKSPKPISLLLSTQRRKKNKGWSKDEGTEAEIRRVMNGDYQTSYIEVKRGSKIGEKSAWMLNLSIDVPKIDKGVDPSIIGGIDVGVKSPLVCAINNALSRYSISDNDLFHFNKKMFARRRILLRKNRHKRAGHGAKNKLKPISILTEKSERFRKKLIERWACEVADFFIKNKVGTVQIENLESMKRKEDSYFNIRLRGFWPYAEMQNKIEFKLKQYGVEIRKVAPNNTSKTCSKCGHLNGYFNFEYRKKNKFPHFKCEKCNFKEDADYNAALNISNPKLKSTKEEP

SEQ ID NO: 3295 - protein, 726 aa, synthetic construct
SEDEFCHEYWMRHALTLAKRARDEREVPVGAVLVLNNRVIGEGWNRAIGLHDPTAHAEIMALRQGGLVLQNCRLIDATLYVTFEPCVMCAGAMVHSRIGRVVFGVRNSKRGAAGSLMNVLDYPGMGHRVEITEGILADECAALLCDFYCMPRQVFNAQKRAQSSIDSGGSSGGSSGSETPGTSESATPESSGGGSSGSAKNTITKTLQLRIVRPYNSAEVEKIVADEKNNREEIALEKNKDKVKEACSKHLEVAAYCTTQVERNACLFCKARKLDDKFYQKLRGQFPDAVFWQEIGEIFRQLQKQTAEIYNQSLIELYYEIFIKGKGFANASSVEHYLSDVCYTRAAELFKNAAIASGLRGKVKSNFRLKELKSMKSGLPTTKSDNFPIPLVKQKGGQYTGFEISSHNDDFIIKIPFGRWQVKKEIDRYRPWEKFDFEQVRKSPKPISLLLSTQRRKRNKGWSKDEGTEAEIRRVMNGDYQTSYIEVKRGSKIGEKSAWMLNLSIDVPKIDKGVDPSIIGGIDVGVKSPLVCAINNSSSRYSICDNDLFRFNKKMFARRRILLKKNRHKRAGHGAKNKLKPITILTKKSERFRKKLIERWVCEVADFFIKNKVGTVQMENLESMKRKEDSYFNIRLRGFWPYAEMQNRIELKLKQYGIEIRRVAPNNTSRTCSKCGHLNNYFNFEYRKRNKFPHFKCEKCNFKENADYNAALNISNPKLKGTKEEP

SEQ ID NO: 3296 - protein, 725 aa, synthetic construct
SEVEFSHEYWMRHALTLAKRARDEREVPVGAILVLNNRVIGEGWNRAIGLHDPTAHAEIMALRQGGLVMQNYRLIDATLYVTFEPCVMCAGAMIHSRIGRVVFGVRNNKHGAAGSLVNVLNYPGMNHRVEITEGILADECAALLCDFYRMPRQIFNARKKARSNINSGGSSGGSSGSETLGTSESATPESSGGGSGGSAKNTITKTLKLRIVRPYNSAEVEKIVADEKNNREKIALEKNKDKVKEACSEHLKVAAYCTTQVERNACLFCKARKLDDKFYQKLRGQFPDAVFWQEISEIFRQLQKQAAEIYNQSLIELYYEIFIKGKGFANASSVEHYLSDVCYTRAAELFKNAAIASGLRGKVKSNFRLKELKSMKSGLPTTKSDNFPIPLVKQKGGQCTGFEISNHNSDFIIKIPFGRWVKKEIDKYRPWEKFDFEQVRKSPKPISLLLSTQRRRRNKGWSKDEGTEAEIRRVMNGDYQTSYIEVKRGSKIGEKSAWMLNLSIDVPKIDKGVDPSIIGGIDVGVKSPLVCAIDNAFSRYSISDNDLYRFNKKMFARRRILLKKNRHKRAGHGVKNKLKPITILTEKSGRFRKKLIERWACEIADFFVKNKVGTVQMENLESMKRKEDSYFNIRLRGFWPYAEMQDKIEFKLKQYGIEIRKVAPNNTSKTCSRCGHLNNYFNFEYRRKNKFPHFKCEKCNFKENADYNAALNISNPKLKSTKEEP

SEQ ID NO: 3297 - protein, 726 aa, synthetic construct
SEVEFSHEYWMRHALTLAKRARDEREVPVGAVLVLNNRVIGEGWNRAIGLHDPTAHAEIMALRQGGLVMQNYRLIDATLYVTFEPCVMCAGAMIHSRIGRVVFGVRNNKHGAAGSLVNVLNYPGMNHRVEITEGILADECAALLCDFYRMPRQVFNARKKAQSSTNPGGSSGGSSGSETPGTSESATPESPGGSSTGSTKNTITKTLKLRIVRPYNSAEVEKIVADEKNNRERIALEKNKDKVKEACSKHLKVAVYCTTQVERNACLFCKARKLDDKFYQKLRGQFPDAVFWQELGEIFRQLQKQAAEIYNQSLIELYYEIFIKGKGFANASSAEHYLSDVCYTRAAELFKNAAIASGLRGKVKSNFRLKELKNMKSGLPTTKSDNFPIPLVKQKGGQYTGFEISSHNDDFIIKIPFGRWQAKKEIDKYRPWEKFDFGQVRKNPKPISLLLSTQRRKGNKGWSKDEGTEAEIRKVMNGDYQTSYIEVKRGSKIGEKSAWMLNLSIDVPKIDKGVDPSIIGGIDVGVKSPLVCAINNAFSRYSISDNDLFRFNKKVFARRRILLKKNRHKRAGHGTKNKLKPITILTEKSGRFRKKLIERWACEIANFFVKNKVGTVQMENLESMKRKEDSYFNIRLRGFWPYAEMQNKIEFKLKQYGIKIRKVAPNNTSKTCSKCGHLNNYFSFEYRKKNKFPHFKCEKCNFKEDADYNAALNVSNPKLKSTKEEP

SEQ ID NO: 3298 - protein, 726 aa, synthetic construct
SEVEFSHEYWMRHALTLAKRARDEREVPVGAILVLNNRVIGEGWNRAIGLHDPTAHAEIMALRQGGLVMQNYRLVDATLYVTFEPCVLCAGAMVHSRIGRVVFGVRNSKRGAAGSLMNVLNHPGMNHRVEITGGILADECAALLCDFYRVPRQVFNAQKKARSNINSGGSSGGSSGSETLGTSESATPESSSGSSGGSAKNTITKTLKLRIVRPYNSAEVEKIVADEKNNREKIALEKNKDKVKEACSEHLKVAAYCTTQVERNACLFCRARKLDDKFYQKLRGQFPDAVFWQEISEIFRQLQKQAAEIYNQSLIELYYEIFIKGRGFANASSVEHYLSDVCYTRAAELFKNAAIASGLRGKVKSNFRLKELKSMKSGLPSTKSDNFPIPLVKQRGGQYTGFEISSHNDDFIIKIPFGRWQAKKEIDKYRPWEKFDFEQVRKSPKPISLLLSTQRRKRNRGWSKDEGTEAEIRKVMNGDYQTSYIEVKRGSKIGEKSAWMLNLSIDVPKIDKGVDPSIIGGIDVGVKSPLVCAINNTFSRYSISDNDLFRFNKKMFARRRILLGKNRHKRAGHGVKNKLKPITILTEKSGRFRKKLIERWACEIADFFVKNKVGTVQMENLESMKRKEDSYFNIRLRGFWPYAEMQNKIEFKLKQYGIKVRKVAPNNTSKTCSKCGHLNNYFSFEYRKKNKFPHFKCEKCNFKENADYNAALNISNPKLKSTKEEP

SEQ ID NO: 3299 - protein, 726 aa, synthetic construct
SEVEFSHEYWMRHALTLAKRARDEREVPVGAVLVLNNRVIGEGWNRAIGLHDPTAHAEIMALRQGGLVMQNYRLTDATLYVTFEPCVMCAGAMIHSRIGRVVFGVRNSKRGAAGSQMNVLNYPGMNHCVEITEGILVDECAALLCDFYRMPRQVLNAQKKAQSSISPGGSSGGSSGSETPGASGSVTPKSSGGSSAGSTKDTITKTLKLRIVRPYNSAEVEKIVADEKNSREKIALEKNKDKVKEACSEHLKVAAYCTTQVERNACLFCKARKLDDRFYQKLRGQFPDAVFWQEIGEIFRQLQKQAAEIYNQSLIELYYEIFIKGKGFANASSVEHYLSDVCYTRAAELFKNAAIASGLRGKVKSNFRLKELKNMKSGLPTTKSNNFPIPLVKQKGGQYTGFEISNHNSDFIIKIPFGRWQAKKEIDKYRPWEKFDFEQVRKSPKPISLLLSTQRRKKNRGWSKDEGTEAEIKKVMNGDYQTSYIEVKRGSKIGEKSAWMLNLSIDVPKIDKGVDPSIIGGIDVGVKSPLVCAISNAFSRYSISDNDLFHFNKKMFARRRILLKKSKHKRAGHGAKNKLKPITILTEKSRRFRKKLIERWACEIADFFIKNKVGTVQMENLESMKRREDSYFNIRLRGFWPYAKMQNKIEFKLKQYGVEIRKVAPNNTSKTCSKCGHLNSYFNFEYRKRNKFPHFKCEKCKFKENADYNAALNISNPKLKSTKEEP

SEQ ID NO: 3300 - protein, 726 aa, synthetic construct
SEVESSHEYWMRHALTLAKRARDEREVPVGAVLVLNNRVIGEGWNRAIGLHDPTAHAEIMALRQGGLVMQNYRLIDATLYVTFEPCAMCAGAMIHSRIGRVVFGVRNSKRGAAGSLMNVLDHPGMNHRVEITEGILTDECAALLCDFYRMPHQVLNAQKKTQSSINSGGSSGGSSGRETPGTSGSATPEGSGGSSGGSAKNTITKTLKLRIVRPYNSAEVEKIVADEKNNREKIALEKNKGKVKEACSKHLKVATYCTTQVERNACLFCKARKLDDKFYQKLRGQFPDAVFWQEIGEIFRQLQKQAAEIYNQSLIELYYEIFIKGKGIANASRVEHYLSDVCYTRAAELFKNAAIASGLRNKIKSNFRLKELKNMKGGLPTTKSDNFPIPLVKQKGGQYTGFEISNHNGDFVIKIPFGRWQAKKEIGKYRPWEKFDFEQVRKSPKPISLLLSTQRRKRNRDWSKDEGTEAEIKKVMNGDYQTSYIEVKRGSKIGEKSAWVLSLSIDVPKTDKGVDPSIIGGIDVGVKSPLVCAINNAFSRYSISDNDLFHFNKKMFARRRILLKKNRHRRAGHGAKNKLKPITILTEKSVRFRKKLIERWACEIADFFIKNKVGTVQMENLGSMKRKEDSYFNIRLRGFWPYAEMQNKIEFKLKQYGIEIRKVAPYNTSKTCSKCGHLNNYFNFEYRRKNKFPHFKCEKCSFKENADYNAALNISNPKLKSTKEKP

SEQ ID NO: 3301 - protein, 726 aa, synthetic construct
SEVEFSHEYWMRHALTLARRARDEREVPVGAILVLNNRVIGEGWNRAIGLHDPTAHAEIMALRQGGLVMQNYRLTDATLYVTFEPCVMCAGAMIHSRIGRVVFGVRNSKHGAAGSLVNVLNYPGMNHRVEITEGILADECAALLCDFYRMPRQVFNARKKAQSSINPGGSSGGSSGSETPGTSESATLENSGGSSGGSAKNTITKTLKLRIVRPYNSAEVEKIVADEKNNREKIALEKNKGKVKEACSKHLEVAAYCTTQVERNACLFCKARKLDDKFYQKLRGQFPDAVFWQELGEIFRQLQRQAAEIYNQSLIELYYEIFIKGKGFANASSVEHYLSDVCYTRAAELFKNAAIASGLRGKVKSNFRLKELKNMKSGLPTTKSDNFPIPLVKQKGGQYTGFEISSHNDDFIIKIPFGRWQVRKEIDKYRPWEKFNFEQVRKSPKPISLLLSTQRRKRNKGWSKDEGTEAEIRKVMNGDYQTSYIEVKRGSKIGEKSAWMLSLSIDVPKIDKGVDPSIIGGIDVGVKSPLVCAINNAFNRYSISDNNLFHFNKKMFARRRILLKKNGHKRAGHGAKNKLKPISVLTEKSGRFRKKLIERWACEIADFFIKNKVGTVQMENLGSMKRKEDSYFNIRLRGFWPYAEMQNEIEFKLKQYGIEIRKVAPDNTSKTCSKCGHLNNYFNFEYRKKNKFPHFKCEKCNFKEDADYNAALNISNPKLKSTKEEP

SEQ ID NO: 3302 - protein, 726 aa, synthetic construct
SEVEFSHEYWMRHALTLAKRARDEREVPVGAVLVLNNRVIGEGWNRAIGLHDPTAHAEIMALRQGGLVMQNYRLVDATLYVTFEPCVLCAGAMVHSRIGRVVFGVRNNKRGAAGSLMNVLNYPGMNHCVEITEGILADECAALICDYYRMPRQVFNARKKAQSSISPGGPSGGSSGSETPGTSESATPKSSGGSSGGSAKNTITKALKLRIVRPYNSAEVEKIVADEKNNRERIALEKNKGKVKEACSKHLKVAAYCTTQVERNACLFCKARKLDDKFYQKLRGQFPDAVFWQEIGEIFRQLQKQAAEIYNQSLVELYYEILIKGKGIANASSVEHYLSDVCYTRAAELFKNAAIASGLRNKIKSNFRLKELRNMKSGLPTTKSDNFPIPLVRQKGGQYTGFEISNHDGDFIIKIPFGRWQVKKEINKHRPWEKFDFEQVRKSPKPISLLLSTQRRKRNKGWSKDEGTEAEIRKVTNGDYQTSYIEVKRGSKIGEKSAWMLNLSIDVPKIDKGVDPGIIGGIDVGVKSPLVCAINNAFSRYSISDNDLFHFNKKMFARRRILLKKNRRRRAGHGAKNKLKPITILTEKSVRFRKKLIERWACEIADFFIKNKVGTVQMENLESMKRREDSYFNIRLRGFWPYAEMQSKIEFKLKQYGIKIRKVAPNNTSKTCSKCGHLNNYFNFEFRKKNKFPHFKCEKCNFKEDADYNAALNISNPKLKSTKEEP

SEQ ID NO: 3303 - protein, 726 aa, synthetic construct
GEVEFSHEYWMRHALTLAKRARDEREVPVGAILVLNNRVIGEGWNRAIGLHDPTAHAEIMALRQGGLVMQNYRLTDATLYATFEPCVMCAGAMIHSRIGRVVFGVRNSKHGAAGSLMNVLNYPGMNHRVEITEGILVDECAALLSDFYRMPRQVLSAQKKAQSSVSSGGSSGGSSGSETPGASGSVTPKSFVGSSAGSTKNTITKTLKLRIVRPYNSAEVEKIVADEKNNREKIALEKNRDKVKEACSKHLKVAAYCTTQVERNACLFCKARKLDDKFYQKLRGQFPDAVFWQEISEIFRQLQKQAAEIYNQSLIELYYEIFIKGKGFANASSVEHYLSDVCYTRAAELFKNAAIASGLRGKVKSNFRLKELKSMKSGLPTTKSDNFPIPLVKQKGGQYAGFEISSHNDDFIIKIPFGRWQVKKEIDKYRPWEKFDFEQVRKSPKPISLLLSTQRRKRNKGWSKDEGTEAEIRKVMSGDYQTSYIEVKRGSKTGEKSAWMLNLSIDVPKIDKGVDPSIIGGIDVGVKSPLVCAINNAFSRYSISDNDLFRFNKKMFARRRILLEKNRHKRAGHGVKNKLKPITILTEKSGRFRKKLIERWACEIANFFIKNKVGTVQMENLESMKRREDSYFNIRLRGFWPYAEMQSKIEFKLKQYGIKIRKVAPNNTSKTCSKCGHLNNYFNFEYRRKNKFPHFKCEKCNFKENADYNAALNISNPKLKSTKEEP

SEQ ID NO: 3304 - protein, 726 aa, synthetic construct
SEVEFSHEYWMRHALTLAKRARDEREVPVGAILVLNNRVIGEGWNRTTGLHDPTAHAEIMALRQGGLVLQNYRLIDATLYVTFEPCVMCAGAMIHSRIGRVVFGVRNNKHGAAGSLVNVLNYPGMNHRVEITEGILAGECAALLCDFYRMPRQVFNAQKKAQSTINSGGSSGGSSSSETPGTSGSATPEGSGGSSGGSAKNTITKTLKLRIVRPYNSAEVEKIVADEKNNREKIALEKNKDKVKEACSKHLKVASYCTTQVERNACLFCKARKLDDKFYQKLRGQFPDAVFWQELGGIFRQLQKQAAEIYNQSLIELYYEIFIKGKGFANASSVEHYLSDVCYTRAAELFKNAAIASGLRGKVKSNFRLKELKNMKSGLPTTKSDNFPIPLVKQKGGQYTGFEISSHNDDFIIKIPFGRWQVKEEIDKYRPWEKFDFEQVRKNPKPISLLLSTQRRKRSKGWSKDEGTEAEIRKVMNGDYQTSYIEVKRGSKIGEKSAWMLNLSIDVPKIDKGVDPSIIGGIDVGVKSPLVCAINNAFSRYSISDNDLFRFNKKVFARRRILLKRNGHKRAGHGTKNKLKPISILTGKSERFRKKLIERWACEIADFFIKNKVGTVQMENLESMKRKEDGYFNIRLRGFWPYAEMQNKIEFKLKQYGIKIRKVAPNNTSKTCSKCGHLNNYFNFEYRKKNKFPHFKCEKCNFKENADYNAALNISNPKLKNTKEEP

SEQ ID NO: 3305 - protein, 726 aa, synthetic construct
SEVEFSHEYWMRHALTLAKRARDEREVPVGAVLVLNNRVIGEGWNRAIGLHDPTAHAEVMALRQGGLVMQNYRLTDATLYATFEPCVMCAGAMIHSRIGRVVFGVRNSKRGAAGSLMNVLNHPGMNHRVEITGGILADECAALLCDFYRMPRQVFNAQKKARSNINSGGSSGGSSGSETLGTSESATPESSVGSSASSTKNTITKTLQLRIVRPYNSAEVEKIVADEKNNREKIALEKNKDKVKEACSKHLKVVAYCTTQVERNACLFCKARRLDDKFYQKLRGQFPDAVFWQEIGEIFRQLQKQAAEVYNQSLVELYYEILIKAKGIANASSVEHYLSDVCYTRAAELFKNAAIASGLRNKIKSNFRLKELRNMRSGLPTTKSENFPIPLVRQKGGQYTGFEISNHDGDFIIKIPFGRWQVRKEINKHRPWEKFDFEQVRKSPKPISLLLSTQRRKRNKGWSKDEGTEAEIRRVMNGDYQTSYIEVKRGSKIGEKSAWMLNLSIDVPKIDKGVDPSIIGGIDVGVKSPLVCAINNAFSRYSISDNDLFHFNKKMFARRRILLKKTRHKRAGHGTKNKLKPISILTEKSERFRKKLIERWACEIADFFIKNKVGTVQMENLESMKRREDSYFNIRLRGFWPYAKMQNKIEFKLKQYGIEIRKVAPNNTSKTCSKCGHLNNYFNFEYRKKNKFPHFKCEKCNFKENADYNAALNISNPKLKSTKEEP

SEQ ID NO: 3306 - protein, 726 aa, synthetic construct
SEVEFSHEYWMRHALTLAKRARDEREVPVGAVLVLNNRVIGEGWNRAIGLQDPTAHAEIMALRQGGLVMQNYRLSDATLYVTFEPCVMCAGAMIHSRIGRVVFGVRNSKRGAAGSLMNVLNYPGMNHCVEITEGILVDECAALLCDFYRMPRQVLSAQKKAQSSVSSGGSSGGSSGSETPGTSESVAPKSSGGSSAGSTKNTITKTLRLRIVRPYNSAEVEKIVADEKNSRERIALEKNKDKVKEACSEHLKVAAYCTTQVERNTCLFCKARKLDDRFYQKLRGQFPDAVFWQEIGEIFRQLQKQAAEIYNQSLIELYYEIFIKGKGFANASSVEHYLSDVCYTRAAELFKNAAIASGLRGKVKSNFRLKELKNMKSGLPTTKSDNFPIPLVKQKGGQYTGFEVSSHNDDFIIKIPFGRWQVKKEISKHRPWEKFDFEQVRKSPKPISLLLSTQRRKRNKGWSKDEGTEAEIRKAMNGDYQTSYIEVKRGSKIGEKSAWMLNLSIDVPKIDKGVDPSITGGIDVGVKSPLVCAINNAFSRYSISDNDLFRFNKKVFARRRILLKKNRHKRAGHGTKNKLKPITILTKKSERFRKKLIERWACEIADFFIKNKVGTVQMENLESMKRKEDSYFNIRLRGFWPYAEMQNKIEFKLKQYGIEIRKVAPNNTSKTCSKCGHLNNYFSFEYRKKNKFPHFKCEKCNFKENADYNAALNISNPKLKSTKEEP

SEQ ID NO: 3307 - protein, 726 aa, synthetic construct
SEVEFSHEYWMRHALTLAKRARDEREVPVGAILVLNNRVIGEGWNRAIGLHDPTAHAEIMALRQGGLVMQNYRLIDATLYVTFEPCVMCAGAMIHSRIGRVVFGVRNSKHGAAGSLMNVLNYPGMNHRVEITEGILADECAALLCDFYRMPHQVFSARKKAQSSINPGGSSGGSSGSKTPGTSESATPESSGGSSGGSAKNSITKTLKLRIVRPYNSAEVEKIVADEKNNREKIALEKNKGKVKEACSRHLEVAAYCTTQVERNACLFCKARKLDDKFYQKLRGQFPDAVFWQELGEILRQLQKQAAEIYNQSLIELYYEIFIKGRGFANASSVEHYLSGVCYTRAAELFRNAAIASGLRGKVKSNFRLKELKNMKSGLPTTKSDNFPIPLVKQKGGQYTGFEISSHNDDFIIKIPFGRWQVKKEIDKYRPWEKFDFEQVRKSPKPISLLLSTRRRKRNKGWSKDVGTEAEIRKVMNGDYQTSYIEVKRGSKIGEKSAWMLNLSIDVPKIDKGVDPSIIGGIDVGVKSPLVCAINNSSSRYSICDNDLFRFNKKMFARRRILLKKNRHKRAGHGAKNKLKPITILTKKSERFRKKLIEKWACGIADFFIKNKVGTVQMENLESMKRKEDSYFNIRLRGFWPYAEMQNKIEFKLKQYGIEIRKVAPNNTSKTCSKCGHLNNYFNFEYRKKNKFPHFKCEKCNFKENADYNAALNISNPKLKSTKGEP

SEQ ID NO: 3308 - protein, 726 aa, synthetic construct
SEVEFSHEYWMRHALTLAKRARDEREVPVGAVLVLNNRVIGVGWNRAVGLHDPTAHAEIMALRQGGLVMQNYRLIEATLYVTFEPCIMCAGAMIHSRIGRVVFGVRNSKRGAAGSLMNVLNYPGMNHRVEITEGILADECAALLCDYYRMPRQVFNARKKAQPSTNSGGPSDGGSGSETPGTSESATPESSGGSSGGSAKNTIAKTLKLRIVRPYNSAEVEKIVADEKSNREKIALEKNKDKVKEACSEHLKVAAYCTTQVERSACLFCKARKLDDKFYQKLRGQFPDAVFWQELGEIFRQLQKQAAEIYNQSLIELYYEIFIKGKGFANASSVEHYLSDVCYTRAAELFKNAAIASGLRGKVKSNFRLKELKNMRSGLPTTKSDNFPIPLVKQKGGQYTGFEISSHNDDFIIKIPFGRWQVKKEIDKYRPWEKFDFEQVRRSPKPISLLLSTQRRKRSKGWSKDEGTEAEIRKVMNGDYQTSYVEVKRGSKIGEKSAWMLNLSIGVPKIDKGVDPSIIGGIDVGVKSPLVCAINNAFCRYSISDNDLFHFNKKMFARRRILLKKNRHKRAGHGAKNKLKPITILTKKSERFRKKLIERWVCEVADFFIKNKVGTVQMENLESMKRKEDSYFNIRLRGFWPYAEMQNRIELKLKQYGIEIRRVAPNNTSRTCSKCGHLNNYFNFEYRKKNKFPHFKCEKCNFREDADYNAALNISNPKLKSTKEEP

SEQ ID NO: 3309 - protein, 726 aa, synthetic construct
SEVEFSHEYWMRRALTLAKRARDEREVPVGAVLVLNNRVIGVGWNRAVGLHDPTAHAEIMALRQGGLVMQNYRLVEATLYVTFEPCIMCAGAMIHSRIGRVVFGVRNSKRGAAGSLMNVLNYPGMNHRVEITEGILADECAALLCDYYRMPHQVFNARKKAQSSINSGGSSGGSSGSETPGTSESPTPESSGGSSGGSAKNTITKTLKLRIVRPYNSAEVEKIVADEKNNREKIALEKNKDKVKEACSEHLKVAAYCTTQVERNACLFCKARKLDDKFYQKLRGQFPGAVFWQEIGEIFRQLQKQAAEVYNQSLIELYYEIFVKGKGFANASSVEHYLSDVCYTRAAELFKNAAIASGLRGKVKSNFRLRELKSMRSGLPTTKSDNFPIPLVKQKGGQYTGFEISSHNDDFIIKIPFGRWQVKKEIDKYRPWEKFDFEQVRKSPKPISLLLSTQRRKRNKGWSKDEGTEAEIRKVMNGDYQTSYIEVKRGSKIGEKSAWMLSLSIDVPKIDKGVDPSIIGGIDVGVKSPLVCAINNAFSRYSISDNDLFHFNKKMFARRRILLKKNRRKRAGHGAKNKLKPITIMTEKSKRFRKKLIERWACEIADFFIKNKVGAVQMENLESMKRKEDSYFNIRLRGLWPYAEMQNRIELKLKQYGIEIRRVAPNNTSRTCSKCGHLNNYFNFEYRKKNKFPHFKCEKCNFREDADYNAALNISNPKLKSTKEEP

SEQ ID NO: 3310 - protein, 726 aa, synthetic construct
SEVEFSHEYWMRHALTLAKRARDEREVPVGAILVLNNRVIGVGWNRAVGLHDPTAHAEIMALRQGGLVMQNYRLIDATLYVTFEPCIMCAGAMIHSRIGRVVFGVRNSKRGAAGSLMNVLNYPGMDHRVEITEGILADECAALLCDYYRMPRQVFNARKKAQSSINSGGSSGGSSGSVTPGTSESATPESSGGGFGGSAKNTITKTLQLRIVRPYNSAEVEKIVADEKNNREKIALEKNKDKVKEACSEHLKVAAYCTTQVERNACLFCKARKLDDKFYQKLRGQFPDAVFWQEVSEIFRQLQKQAAVIYNQSLIELYYEIFIKGKGFANASSVEHYLSDVCYTRAAELFRNAAIASGLRGKVKSNFRLKELKNMKSGLPTTKSDNFPIPLVKQKGGQYTGFEISSHNDDLIIKIPFGRWQVKKEIDKYRPWEKFDFEQVRKSPKPISLLLSTQRRKRNKGWSKDEGTEAEIRKVMNGDYQTSYIEVKRGSKIGEKSAWMLNLSIDVPKIDKGVDPSIIGGIDVGVKSPLVCAVNNAFSRYSISDNDLFRFNKKMFARRRILLKKNRHQRAGHGAKNKLKPITTMTEKSKRFRKKLIERWACEIADFFIKNKVGTVQMENLESMKRKEDSYFNIRLRGFWPYAEMQNKIEFKLKQYGIEIRKVAPNNTSKTCSRCGHLNNYFNFEYRRKNKFPHFKCEECSFKENADYNAALNISNPKLKSTKGEP

SEQ ID NO: 3311 - protein, 726 aa, synthetic construct
SEVEFSHEYWMRHALTLAKRARDEREVPVGAILVLNNRVIGEGWNRAIGLHDPTAHAEIMALRQGGLVMQNYRLIDATLYVTFEPCVMCAGAMIHSRIGRVVFGVRNNKHGAAGSLVNVLNYPGMNHRVEITEGILADECAALLCDFYRMPRRVFNAQKKAQSSISSGGSSGGCSGSEMPGASESVTPKSSGDSSAGSTKNTITKTLKLRIVRPYNSAEVEKIVADEKNNREKIALEKNKGRVKEACSKHLEVAAYCTTQVERNACLFCKARKLDDKFYQKLRGQFPDAVLWQELGEIFRQLQKQAAEIYNQSLIELYYEIFIKGKGFANASNVEHYLSDVCYTRAAELFRNAAIASGLRGKVKSNFRPKELKNMKSGLPTTKSDNFPIPLVKQKGGQYTGFEISSHNDDFIIKIPFGRWQAKEEIDKYRPWEKFDFEQVRKSPKPISLLLSTQRRKRNKGWSKDEGTEAEIRKVMNGDYQTSYIEVKRGSKIGEKSAWMLNLSIDVPKIDKGVDPSIIGGIDVGVKSPLVCAINNAFSRYSISDNDLFRFNKKMFARRRILLKKTRHKRAGHGAKNKLKPISILTEKSERFRKKLIERWACEIADFFVKNKVGTVQMENLESMKRKEDSYFNIRLRGFWPYAEMQNKIEFKLKQYGIKVRKVAPNNTSKTCSKCGHLNNYFSFEYRKKNKFPHFKCEKCNFKENADYNAALNISSPKLKSTKEEP

SEQ ID NO: 3312 - protein, 726 aa, synthetic construct
SEVEFSHEYWMRHALTLAKRARDEREVPVGAVLVLNNRVIGEGWNRAIGLHDPTAHAEIMALRQGGLVMQNYRLVDATLYVTFEPCVLCAGAMVHSRIGRVVFGVRNSKRGAAGSLMNVLNYPGMNHRVEITEGILADECAALLCDFYRMPRQVFNARKKARSNINSSGSSGGSSGSETPGTSKSATPESSGGSSGGSAKNTITKTLKLRIVRPYNSAEVEKIVADEKNNREKIALEKNKDKVKEACSEHLKVAAYCTTQVERNACLFCRARKLDDKFYQKLRGQFPDAVFWQEIGEIFRQLQKQAAEIYNQSLIELYYEIFIKGKGFANANSVEHYLSDVCYTRAAELFKNAAIASGLRGKVKSNLRLKELKNMKSGLPTTKSDNFPIPLVKQKGGQYTGFEISSHNDDFIIKIPFGRWQVRKEIDKYRPWEKFNFEQVRKSPKPISLLLSTQRRKRNKGWSKDEGTEAEIRKVMNGDYQTSYIEVKRGSKIGEKSAWMLSLSIDVPKIDKGVDPSIIGGIDVGVKSPLVCAINNAFNRYSISDNNLFHFNKKMFARRRILLKKNRHKRAGHGAKNKLKPISILTEKSKRFRKKLIERWACEIADFFVKNKVGTVQMENLESMKRKEDSYFNIRLRGLWPYAEMQNKIEFKLKQYGIEIRKVAPNNTSKTCSKCGHLNNYFNFEYRKKNKFPHFKCEKCNFKENADYNAALNISNPKLKSTKEEL

SEQ ID NO: 3313 - protein, 726 aa, synthetic construct
SEVEFSHEYWMRHALTLAKRARDEREVPVGAILVLNNRVIGEGWNRAIGLHDPTAHAEIMALRQGGLVMQNYRLTDATLYVTFEPCVMCAGAMIHSRIGRVVFGVRNSKRGAAGSLMNVLNYPGMNHCVEITEGILVDECAALLCDFYRMPRQVLNAQKKAQSSISSGGSSGGSSCSETPGASESVTPKSSGGGSAGSTKNTITKTLKLRIVRPYNSAEVEKIVADEKNNREKIALEKNKDKVKEACSEHLKVAAYCTTQVERNACLFCKARKLDDKFYQKLRGQFPDAVFWQEIGEIFRQLQRRAAEIYNQSLIELYYEIFIKGKGFANASSVEHYLSDVCYTRAAELFKNAAIASGLRGKVKSNFRLKELKNMKSGLPTTKSDNFPIPLVRQKGGQYTGFEISNHNGDFIIKIPFGRWQVKKEICKHRPWEKFDFEQVRKSPKPISLLLSTQRRKRNKGWGKDEGTEAEIRKVMNGDYQTSYIEVKRGSRIGEKSAWMLSLSIDVPKIDKGVDPSIIGGIDVGVKSPLVCAINNALSRYSISDNDLFHFNKKMFARRRILLKKNRHKRAGHGAKNKLRPFTVLTEKSERFRKKLIERWACEIADFFIKNKVGTVQMENLESMKGKEDSYFNIRLRGFWPYAEMQNKIEFKLKQYGIEIRKVAPNNTSKTCSKCGHLNNYFNFEYRKKNKFPHFKCEKCNFKENADYNAALNISNPKLKSTKEEP

SEQ ID NO: 3314 - protein, 726 aa, synthetic construct
SEDEFSHEYWMRHALTLAKRARDGREVPVGAVLVLNNRVIGEGWNRAIGLHDPTAHAEIMALRQGGLVMQNYRLIDATLYVTFEPCVMCAGAMVHSRIGRVVFGVRNSKRGAAGSLVNVLNYPGMNNRVEITEGILADECAALLCDFYRMPRQVFNARKKAQSSINPSGSSGGSSGSLTPGTSESATPESSGGGFGGSAKNTITKTLQLRIVRPYNSAEVEKIVADEKNNREKIALEKNKDKVKEACSKHLKVAAYCTTQVERNACLFCKARKLDDRFYQKLRGQFPDAVFWQEISEIFRQLQKQAAVIYNQGLIELYYEIFIKGKGIANASRVEHYLSNVCYTRAAELFKNAAIASGLRNKIKSNFRLKELRNMKSGLPTTKSDNFPIPLVRQKGGQYTGFEISSHNDDFIIKIPFGRWQAKKEIDKYRPWEKFDFEQVRKSPKPISLLLSTRRRKRNKGWSKDEGTEAEIRRVMNGDYQTSYIEVKRGSKIGEKSAWMLNLSIDVPKIDKGVDPSIIGGIDVGVKSPLVCAINNAFSRYSISDNELFHFNKKMFARRRILLKKNRHKRAGHGAKNKLKPISVLTEKSGRFRKKLIERWACEIADFFIKNKVGTVQMENLGSMKRKEDSYFNIRLRGFWPYAEMQNKIEFKLKQYGIEIRKVAPDNTSKTCSKCGHLNNYFNFEYRKKSKFPHFKCEKCNFREDADYNAALNISNPKLKSTKEEP

SEQ ID NO: 3315 - protein, 726 aa, synthetic construct
SEVEFSHEHWMRHALTLAKRARDEREVPVGAVLVLNNRVIGEGWNRAIGLHDPTAHAEIMALRQGGLVMQNYRLIDATLYVTFEPCVMCAGAMIHSRIGRVVFGVRNSKHGAAGSLVNVLNYPGMNHRVEITEGILADECAALLCDFYRMPRQVFNAQKKAQSTINSGGSSGGSSGSETPGTSESATPESSGGSSGSSAKNTITKTLQLRIVRPYNSAEVEKIVADEKNNREKIALEKNKDKVKEACSKHLKVASYCTTQVERNACLFCKARKLDDKFYQRLRGQFPDAVFWQELGEIFRQLQKQAAEIYNQSLIELYYEIFIKGKGFANANSVEHYLSDVCYTRAAELFKNAAIASGLRGKVKSNFRLKELKNMRSGLPTTKSDNFPIPLVRQKGGQYTGFEISSHNDDFIIKIPFGRWQVRKEIDKYRPWEKFDFEQVRKSPKPISLLLSTQRRKKSKGWSKDEGTEAEIRRVMNGDYQTSYVEVKRGSKIGEKSAWMLNLSIDVPKIDKGVDPSIIGGIDVGVRSPLVCAINNAFSRYSISDNDLFRFNKKVFARRRILLKKTRHKRAGHGAKNKLKPISILTEKGERFRKKLIERWACEIADFFIKNKVGTVQMENLESMKRREDSYFNIRLRGFWPYAEMQNKIEFKLRQYGIEIRKVAPNNTSKTCSKCGHLNNYFDFEYRKKNKFPHFKCEKCNFKENADYNAALNISNPKLRSTKEEP

SEQ ID NO: 3316 - protein, 725 aa, synthetic construct
SEVEFSHEYWMRHALTLAKRARDEREVPVGAVLVLNNRVIGEGWNRAIGLHDPTAHAEIMALRQGGLVMQNYRLTDATLYVTFEPCVMCAGAMIHSRIGRVVFGVRNNKHGAAGSLVNVLNYPGMNHRVEITEGILADECAALLCDFYRMPRRVFNAQKKAQSSINSGGSSGGSSGSVMPGTSESATPESSGGSFGGSAKNTITKTLQLRIVRPYNSAEVEEIVTDEKNNREKIALEKNKGKVKEACSKHLKMASYCTTQVERNACLFCKARKLDDKFYQKLRGQFPDAVFWQELGGIFRQLQKAAEIYNQSLIELYYEIFIKGKGITNASRVEHYLSDVCYTRAAELFKNAAIASGLRSKVRSNFRLKELKNMKSGLPTTKSDNFPIPLVKQKGGQYTGFEISSHNSDFIIKIPFGRWRVKREIDKYRPWEKFDFEQVRRSPKPISLLLSTQRRKKNKGWSKDEGTEAEIRKVMNGDYQTSYIEVKRGSKIGEKSAWTLSLSIDVPKIDKGVDPSIIGGIDVGVKSPLVCAINNAFCRYSISDNDLFHFNKKMFARRRILLKKSRHKRAGHGAKNKLKPISILTEKSKRFRKKLIERWACEIADFFIKNKVGTVQMENLESMKRKEDSYFNIRLRGFWPYAEMQNKIEFKLKQYGIEIRKVAPNNTSKTCSKCGHLNNYFNFEYRKKNKFPHFKCEKCSFKENADYNAALNISNPKLKSTREEP

SEQ ID NO: 3317 - protein, 726 aa, synthetic construct
SEVEFSHEYWMRHALTLAKRARDEREVPVGAILVLNNRVIGEGWNRAIGLHDPTAHAEIMALRQGGLVTQNYRLIGATLYVTFEPCVMCAGAMIHSRVGRVVFGVRNNKHGAAGSLVNVLNYPGMNHRVEITEGILADECAALLCDFYRMPRQVFNARKKAQSGINPGGSSGGSSGSETPGTSESATPESSGGSSGGSAKNTITKTLKLRIVRPYNSAEVEKIVADEKNNREKIALEKNKDKVKEACSKHLKVAAYCTTQVERDACLFCKARRLDDKFYQKLRGQFPDAVFWQEVGEIFRQLQKQAAEIYNQSLIELYYEILIKGKGIANASSVEHYLSDVCYTRAAELFKNAAIASGLRNKIKSNFRLKELRSMKSGLPTTKSDNFPIPLVRQKGGQYTGFEISDHNGDFIIKIPFGRWQVKKEINKHRPWEKFDFEQVRKSPKPISLLLSTQRRKKNKGWSKDEGTEAEIRRVMNGDYQTSYIEVRRGSKIGEKSAWMLSLSIDVPKIDKGVDPSIIGGIDVGVKSPLVCAINNSFSRYSICDNDLFRFNKKMFARRRILLKKNRHKRAGHGAKNKLKPITILTKKSERFRKKLIERWVCEVADFFIKNKVGTVQMENLESMKRKEDSYFNIRLRGFWPYAEMQNRIELKLKQYGIEIRRVAPNNTSRTCSKCGHLNNYFNFEYRKKNKFPHFKCEKCNFREDADYNAALNISNPKLKSTKEEP

SEQ ID NO: 3318 - protein, 726 aa, synthetic construct
SEVEFSHEYWMRHALTLAKRARDEREVPVGAVLVLNNRVIGEGWNRTTGLHDPTAHAEIVALRQGGLVMRNYRLTDATLYVTFEPCVMCAGAMIHSRIGRVVFGVRNSKRGAAGSLMNVLNYPGMNHCVEITEGILVDECAALLCDFYRMPRQVLNAQKKAQSSISPGGSSGGSSGSETPGASESVTPKSSGGSSGGSAKNTITKTLKLRIVRPYNSAEVEKIVADEKNNREKIALEKNKGKVKEACSKHLEVAAYCTTQMERNACLFCKARKLDDKFYQKLRGQFPDAVFWQELGEIFRQLQKQAAEIYNQSLIELYYEIFIKGKGFANASSVEHYLSDVCYTRAAELFKNAAIASGLRGKVKSNFRLKELKNMKSGLPTTKSDNFPIPLVKQKGGQYTGFEISSHNDDFIIKIPFGRWQVKKEIDKYRPWEKFDFEQVRKSPKPISLLLSTQRRKRNKGWSKDEGTEAEIRKVMNGDYQTSYIEVKRGSKIGEKSAWMLNLSIDVPKIDKGVDPSIIGGIDVGVKSPLVCAIDNAFSRYSISDNDLFHFNKKMFARRRILLKKNRHKRAGHGAKNKLKPISILTEKSKRFRKKLIERWACEIADFFIKNKVGTVQMENLESMKRKEDSYFNIRLRGLWPYAEMQNKIEFKLKQYGIKIRKVAPNNTSKTCSKCGHLNNYFNFEYRKKNKFPYFKCEKCNFKENADYNAALNISNPQLKSTKGEP

SEQ ID NO: 3319 - protein, 726 aa, synthetic construct
SEVEFSHEYWMCHALTLAKRARDEREVPVGAVLVLNDRVIGVGWNRAIGLHDPTAHAEIMALRQGGLVLQNYRLIDATLYVTFEPCVLCAGAMVHSRIGRVVFGVRNSKRGAAGSLMNVLNYPGMNHRVEITEGVLADECAALLCDFYRMSRQVFNTQKKAQSNINSGGSSGGSSGSETPGTSESPTPESSGGSSGGSTKNTITKTLKLRIVRPYNSAEVEKIVADEKNNREKIALEKNKDKVKEACSKHLKVAAYCTTQVERNACLFCKARKLDDRFYQKLRGQFPDAVFWQETGEIFRQLQRQAAEIYNQSLIELYYEIFIKGKGFANASSVEHYLSDVCYTRAAELFKNAAIASGLRGKVKSNFRLKELKNMKSGLPTTKSDNFPIPLVKQKGGQYTGFEISNHNSDFIIKIPFGKWQVKKEIDKYRPWEKFDFEQVRKSPKPISLLLSTQRRKRNKGWSKDEGTEAEIKRVMNGDYQISYIEVKRGSKIGEKSAWMLSLSVDVPKIDKGVDPSIIGGIDVGVKSPLVCAINNAFSRYSISDNDLFHFNKKMFARRRILLKKNGRKRAGHGVKNKLKPITILTEKSGRFRKKLIERWACEIADFFVKNKVGTVQMENLESMKRKEDSYFNIRLRGFWPYAEMQNKIEFKLKQYGIKVRKVAPNNTSKTCSRCGHLNNYFNFEYRRKNKFPHFKCEKCNFKEDADYNAALNISNPKLKSTKEEP

SEQ ID NO: 3320 - protein, 726 aa, synthetic construct
SEVEFSHEYWMRHALTLAKRARDEREVPVGAILVLNNRVIGEGWNRAIGLHDPAAHAEIMALRQGGLVMQNYRLIDATLYVTFEPCVMCAGAMIHSRIGRVVFGVRNSKHGAAGSLVNVLNYPGMNHRVEITEGILADECAALLCDFYRMPRQVFNAQKRAQSSINSGGSSGGSSGSETPGTSESATPESSGGSSAGSTKDTITKTLKLRIVRPYNSAEVEKVVADEKNNREKIAMEKNKDKVKEACSKHLKVASYCTTQVERNACLFCKARKLDDKFYQKLRGQFPDAVFWQEIGEIFRQLQKQAAEIYNQSLVELYYEILIKGKGIANASSVEHYLSDVCYTRAAKLFKNAAIASGLRNKIKSNFRLKELRNMKSGLPTTKSDNFPIPLVKQKGGQYTGFEISSHNDDFIIKIPFGRWQVKKEIDKYRPWEKFDFEQVRKSPKPISLLLSTQRRKRNKGWSKDEGTEAEIRKVMNGDYQTSYIEVKRGSKIGEKSAWMLNLSIDVPKIDKGVDPSIIGGIDVGVKSPLVCAINNAFSRYIIGDNDLFHYNKKMFARRRILLKKNRLKRAGHGAKNKLKPISILTERSKRFRKKLIERWACEIADFFIKNKVGTVQIENLESMKRKEDSYFNIRLRGFWPYAEMQNKIEFKLKQYGIEIRKVAPNNTSKTCSKCGHLNNYFNFEYRKKNKFPHFKCEKCNFKENADYNAALNISNPKLKSTKEGP

SEQ ID NO: 3321 - protein, 726 aa, synthetic construct
SEVEFSHEYWMRHALTLAKRARDEREVPVGAVLVLNNRVIGEGWNRAIGLHDPTAHAEVMALRQGGLVMQNYRLTDATLYVTFEPCVMCAGAMIHSRIGRVVFGVRNSKRGAAGSLMNVLNYPGMNHCVEITEGILVDECAALLCDFYRMPRQVLNAQKKAQSSISPGDSSGGSSGSEAPGASGSVTPKSSGGSSAGSTKDTITKTLRLRIVRPYNSAEVEKIVADEKNSREKIALEKNKDRVKEACSEHLKVAAYCTTQVERNACLFCRARKLDDKFYQKLRGQFPDAVFWQELGGIFRQLQRQAAEIYNQSLIELYYEIFIKGKGFANASSVEHYLSDVCYTRAAELFKNAAIASGLRGKVKSNFRLKELKNMKSGLPTTKSDNFPVPLVRQKGGQYTGFEISSHNSDFIIKIPFGRWQVKEEIDKFRPWEKFDFEQVRKSPKPISLLLSTQRRKRNKGWSKDEGTEAEIRKVMNGDYQTSYIEVKRGSKIGEKSAWMLNLSIDVPKIDKGVDPSIIGGIDVGVKSPLVCAINNAFSRYSVSDNDLFRFNKKMFARRRILLKKNRHKRAGHGAKNRLKPITILTGKSRRFRKKLIERWACEIADFFIKNKVGTVQMENLEGMKRKEDSYFNIRLRGFWPYAEMQNKIEFKLKQYGIEIRKVAPNNTSKTCSKCGHLNDYFDFEYRRKNKFPHFKCERCSFKENADYNAALNISSPKLKSTKEEP

SEQ ID NO: 3322 - protein, 726 aa, synthetic construct
SEVEFSHEHWMRHALTLAKRARDAREVPVGAILVLNNRVIGEGWNRAIGQHDPTAHAEIMALRQGGLVMQNYRLIDATLYVTFEPCVMCAGAMIHSRIGRVVFGVRNSKHGAAGSLVNVLNYPGMNHRVEITEGILADECAALLCDFYRMPRQVFGARRKAQSSISSGGSSGGSNGSETPGASESATPKSSGGSSAGSTKNTITKTLKLRIVRPYNSAEVEKIVADEKNSREKTALEKNKDKVKEACSEHLKVAAYCTTQVERSACLFCKARKLDDKFYQKLRGQFPDAVFWQEIGEIFRQLQKQAAEIYNQSLIELYYEIFIKGKGFANASSVEHYLSDVCYTRAAELFKNAAIASGLRGKVKSNFRLKELKNMRSGLPTTKSDNFPIPLVKQKGGQYAGFEISSHNDDFIIKIPFGRWQVKKEIDKYRPWEKFDFEQVRKSPKPISLLLSTRRRKRNKGWSKDEGTEAEIRKVMNGDYQTSYIEVKRGSKIGEKSAWMLNLSIDVPRIDKGVDPSIIGGIDVGVKSPLVCAINNAFSRYSISDNDLFRFNKKMFARRRVLLKKSKHKRAGHGARNKLKPITVLTEKNERFRKKLIERWACEIANFFIKNKVGTVQMENLESMKRREDSYFNIRLRGFWPYAEMQSKIEFKLKQYGIEVRKVAPNNTSKTCSKCGHLNNYFNFEFRKKSKFPHFKCEKCNFKEDADYNAALNISNPKLKSTKEEP

SEQ ID NO: 3323 - protein, 726 aa, synthetic construct
SEVEFSHEYWMRHALTLAKRARDEREVPVGAVLVLNNRVIGEGWNRAIGLHDPTAHAEIMALRQGGLVLQNYRLIDATLYVTFEPCVMCAGAMIHSRIGRVVFGVRNNKHGAAGSLVNVLNYPGMNHRVEITEGILVNECAALLCDFYRMPRQVFNARKKAQSSINSGGSSDGGSGSETPGTCESVTPESSGGSSGGSAKNTITKTLKLRIVRPYNSAEVEKIVADEKNNREKIALEKNEDKVKEACSEHLKVAAYCTTQVERSACLFCKARKLDDKFYQKLRGQFPDAVFWQEIGEILRQLQKQAAEIYNQSLIELYYEIFIKGKGFANASSAEHYLSDVCYTRAAELFKNAAIASGLRGKVKSNFRLKELKNMKSGLPTTKSDNFPIPLVKQKGGKYTGFEISCHNDDFIIKIPFGRWQVKKEIDKYRPWEKFDFEQVRKSPKPISLLLSTQRRKRNKGWSKDEGTEAEIRKVMNGDYQTSYIEVKRGSKIGEKSAWMLNLSIDVPKIDKGVDPSIIGGIDVGVKSPLVCAINNAFSRYSISDNDLFHFNKKMFARRRILLKKTRHKRAGHGAKNKLKPISILTEKSGRFRKKLIERWACEIADFFIKNKVGTVQMENLESMKRKEDSYFNIRLRGFWPYAEMQNKIEFKLKQYGIVVRKVAPNNTSKTCSKCGHLNNYFNFEYRKKNKFPHFKCEKCNFKEDADYNAALNISNPKLKSTKEEP

SEQ ID NO: 3324 - protein, 726 aa, synthetic construct
SEVEFSHEYWMHHALTLAKRARDEREVPVGAILVLNNRVIGEGWNRAIGLHDPTAHAEIMALRQGGLVMQNYRLIDATLYVTFEPCVMCAGAMIHSRVGRVVFGVRNSKHGAAGSLINVLNYPGMNHRVEITEGILADECAALLCDFYRMPRRVFNAQKKAQSSISSGGSSGGCSGSEMPGASESVTPKSSGGGSAGSTKNTITKTLKLRIVRPYNSAEVEKIVADEKNSREKIALERNKDKVKEACSEHLKVAAYCTTQVERNACLFCKARRLDDKFYQKLRGQFPDAVFWQEIGEIFRQLQKQAAEIYNQSLIELYYEIFIKGKGFANASSVEHYLSDVCYSRAAELFKNAAIASGLRGKVKSNFRLKELKNMKSGLPTTKSDNFPIPLVKQKGGQYTGFEISSHSDDFIIKIPFGRWQVRKEIDKYRPWEKFDFEQVRKSPKPISLLLSTQRRKRNKGWSKDEGTEAEIRKVMNGDYQTSYIEVKRGGKIGEKSAWMLSLSIDVPKIDKGVDPRIIGGIDVGVKSPLVCAINDAFSRYSISDNDLFHFNKKVFARRRILLKKSKHKRAGHGAKNKLRPITILTEKSRRFRKKLIERWACEIADFFIKNKVGTVQMENLESMKRREDSYFNIRLRGFWPYAEMQNKIEFKLKQYGIEIRKVAPNNTSKTCSKCGHLNNHFNFEYRRKNKFPHFKCEKCNFKENADYNAALNISNPKLKGTKEEP

SEQ ID NO: 3325 - protein, 726 aa, synthetic construct
SEVEFSHEYWMRHALTLAKCARDEREVPVGAILVLNNRVIGEGWNRAIGLHDPTAHAEIMALRQGGLVMQNYRLTDATLYVTFEPCVMCAGAMVHSRIGRVVFGVRNSKRGAAGSLMNVLDYPGMGHRVEITEGILADECAALLCDFYCMPRQVFNAQKRAQSSINSGGSSGGSSGSDTPGTSESATPESSGGGSSGSAKNTITKTLQLRIVRPYNSAEVEKIVADEKNNREKIALEKNKDKVREACSKHLKVASYCTTQVERNACPFCKARKLDDKFYQKLRGQFPDAVFWQELGEILRQLQKQAAEIYNQSLIELYYEIFIKGRGFANASGVEHYLSDVCYTRAAELFKNAAIASGLRGKVKSNFRLKELKNMRSGLPTTKSDNFPIPLVKQKGGQYTGFEINSHNDDFIIKIPFGRWQAKKEINKYRPWEKFDFEQVRRSPKPISLLLSTQRRKRNKGWSKDEGTEAEIKKVMNGDYQTSYIEVKRGSKIGEKSAWMLNLSIDVPKIDKGVDPRIIGGIDVGVRSPLVCAINNAFSRYSISDNDLFHFNKKMFARRRILLKKNRHKRAGHGATNKLKPITIPTEKSERFRKKLIERWACEIADFFVKNKVGTVQMENLGSMKGKEDSYFNIRLRGFWPYAEMQNKIEFKLKQYGIVVRKVAPNNTSKTCSECGHLNNYFNFEYRKKNKFPHFKCEKCNFKENADYNAALNISNPKLKSTKGEP

SEQ ID NO: 3326 - protein, 726 aa, synthetic construct
SEVEFSHEYWMRHALTLAKRARDEREVPVGAVLVLNNRVIGEGWNRAIGLHDPTAHAEIMALRQGGLVMQNYRLTDATLYVTFEPCVMCAGAMIHSRIGRVVFGVRNSKRGAAGSLMNVLNYPGMNHCVEITEGILMDECAALLCDFYRMPRQVLNAQKKAQSSISSGGPSGSSSCSETPGASESVTPKSSGGSSTGSTKDTITKTLKLRIVRPYNSAEVEEIVADEKNSREKIALEKNKDKVKEACSKHLKVAAYCTTQVERNACLFCKARKLDDKFYQKLRGQFPDAVFWQEIGEIFRQLQKQAAEIYNQSLIELYYEIFIKGEGFANASSVEHYLSDVCYTRAAELFKNAAIASGLRGKVKSNFRLKELKNMRSGLPTTKSDNFPIPLVKQRGGQYTGFEISSHNDDFIIKIPFGRWQAKKEIDKYRPWEKFDFEQVRKNPKPISLLLSTQRRKRNKGWSKDEGTEAEIRKVMNGDYQTSYIEVKRSSKIGEKSAWMLNLSIDVPKIDKGVDPSIIGGIDVGVKSPLVCAINNAFSRYSISDNDLFRFNKKVFARRRILLKKNRHKRAGHGTKNKLKPITILTEKSGRFRKKLIERWACEIANFFIKNKVGTVQMENLESMKRKGDSYFNIRLRGFWPYAEMQNKIEFKLKQYGIEIRKVAPNNTSKTCSKCGHLNNYFSFEYRKKNKFPHFKCEKCNFKENADYNAALNISNPKLKSAKEEP

SEQ ID NO: 3327 - protein, 726 aa, synthetic construct
SEVEFSHEYWMRHALTLAKRARDEREVPVGAILVLNNRVIGEGWNRAIGLRDPTAHAEIMALRQGGLEMQNYRLIDATLYVTFEPCVMCAGAMIHSRIGRVVFGVRNNKHGAAGSLVNVLNYPGMNHRVEITEGILADECAALLCDFYRMPRQVFNARKKAQSSINPGGSSGGSSGSETPGNSESATPESSGGSSGGSAKNTITKTLKLRIVRPFNSAEVERIVADEKNNREKIALEKNKDKVKEACSEHLKVAAYCTTQVERSACLFCKARKLDDKFYQKLRGQFPDAVFWQEIGEIFRQLQKQAAEIYNQSLIELYYEIFIKGKGFANASSVEHYLSDVCYTRAAELFKNAAIASGLRGKVKSNFRLKELKNMKSGLPTTKSDNFPIPLVKQKGGQYTGFEISSHNDDFIIKIPFGRWQVKKEIDKYRPWEKFDFEQVRKSPKPISLLLSTQRRKRNKGWSKDEGTEAEIRKVMNGDYQTSYIEVKRGSKIGEKSAWMLNLSIDVPKIDKGVDPSIIGGIDVGVRSPLVCAINNAFSRYSISDNDLFRFNKKMFARRRILLKKNRHKRAGHGAKNKLKPITILTEKSRRFRKKLIERWACEIADFFIKNKVGTVQIESLESMKRKEDSYFNVRLRGFWPYAEMQNKIEFKLKQYGIKIRKVAPNNTNKTCSMCGHLNNYFSFEYRKKNKFPHFKCEKCNFKENADYNAALNISNPKLMSTKEGP

SEQ ID NO: 3328 - protein, 726 aa, synthetic construct
SEVEFSHEYWMRHALTLAKRARDEREVPVGAVLVLNNRVIGEGWNRAIGLHDPTAHAEIMALRQGGLVMQNYRLTDATLYVTFEPCVMCAGAMIHSRIGRVVFGVRNSKRGAAGSLMNVLNYPGMNHCVEITEGILADECAALLCDFYRMPRQVFNARKKAQSSINPGGSSGGSSSSETPGTSESATLENSGGSSGGSVKNTITKTLKLRIVRPYNSAEVEKIVADEKNNREKIALEKNKDKVKEACSKHLKVASYCTTQVERSACPFCKARKLDDKFYQKLGGQFPDAVFWQELGEIFRQLQKQAAEIYNQSLIELYYEIFIKGKGIANASSVEHYLSDVCYTRAAELFKNAAIASGLRGKVKSNFRLKELRNMKSGLPTTKSDNFPIPLVRQKGGQYTGFEISNRNSDFIIKIPFGRWQVKKEINRYRPWEKLDFEQVRKSPKPISLLLSTQRRKRNKGWSKDEGTEAEIRKVMNGDYQTSYIEVKRGSKIGEKSAWMLNLSIDVPKIDKGVDPSIVGGIDVGVKSPLVCAINNASSRYSISDNDLFRFNKKMFARRRILLKKNKHKRAGHGAKNKLKPITILTKKSERFRKKLIERWVCEVADFFIKNKVGTVQMENLESMKRKEDSYFNIRLRGFWPYAEMQNRIELKLKQYGIEIRRVAPNNTSRTCSKCGHLNNYFNFEYRKKSKFPHFKCEKCNFREDADYNAALNISNPKLKSTKEEP

SEQ ID NO: 3329 - protein, 726 aa, synthetic construct
SEVEFSHEYWMRRALTLAKRARDEREVPVGAVLVLNNRVIGEGWNRAIGLHDPTAHAEIMALRQGGLVMQNYRLIDATLYVTFEPCVMCAGAMVHSRIGRVVFGVRNSKRGAAGSLMNVLDHPGMGHRVEITEGILADECAALLCGFYCMPRQVFNAQKRAQSSINSGGSSGGSSGSETPGTSESATPKSSGGSSGGSAKNTITKTLQLRIVRPYNSAEVEKIVADEKNNREKIALEKNKDKVKEACSKHLKVASYCTTQVERNACPFCKARKLDDKFYQKLRGQFPDAVFWQELGEILRQLQKQAAEIYNQSLIELYYEIFIKGRGFANASSVEHYLSDVCYTRAAGLFKNAAIASGLRGKVKSNFRLKELKNMKSGLPTTKSDNFPIPLVKQKGGQYTGFEISSHNDDFIIKIPFGRWQAKKEIDKYRPWEKFDFEQVRKSPKPISLLLSTRRRKRNKGWSKDEGTEAEIRKVMNGDYQTSYIEVKRGSKIGEKSAWMLNLSIGVPKIDKGVDPSIIGGIDVGVKSPLVCAINNAFSRHSISDNDLFHFNKKMFARRRILLKKTRHKRAGHGAKNKLKPISILTEKSERFRKKLIERWACEIADFFIKNKVGTVQMENLESMKRREDSYFNIRLRGFWPYAKMQNKIEFKLKQYGIEIRRVAPNNTSKTCSKCGHLNNYFNFEYRKKNKFPHFKCEKCNFKESADYNAALNISNPKLKSTKEEP

SEQ ID NO: 3330 - protein, 726 aa, synthetic construct
SEVEFSHEYWMRHALTLAKRARDEREVPVGAILVLNNHVIGEGWNRAIGRHDPTAHAEIMALRQGGLVMQNYRLIDATLYVTFEPCVMCAGAMIHSRIGRVVFGVRNSKHGAAGSLVNVLNHPGMNHRVEITEGILADECAALLCDFYRMPRQVFNARKKAQSSINPGCSSGGSRGSETPGTSESPTPESPGGSSGGSAKNTITKTLKLRIVRPYNSAEVEKIVADEKNNREKIALEKNKDKVKEACSKHLKVAAYCTTQVERNACLFCKARRLDDKFYQKLRGQFPDAVFWQEIGEIFRQLQKQAAEIYNQSLIELYYEIFIKGRGFANASSVEHYLSDVCYTRAAELFKNAAIASGLRGKVKSNFRLKELKNMKSGLPTTKSDNFPIPLVKQKGGQYTGFEISDHNSDFIIKIPFGRWQVKKEIDKFRPWEKFDFEQVRKSPKPISLLLSTQRRKRNKGWGKDEGTEAEIRKVMNGDYQTSYIEVKRGSKIGEKSAWMLNLSIDVPKIDKGVDPSIIGGIDVGVKSPLVCAINNAFSRYGISDNDLFHFNKKMFARRRILLKKNRHRRAGHGAKNKLKPITILTEKSKRFRKKLIERWACEIADFFIKNKVGTVQMENLESMKRKEDSYFNIRLRGFWPYAEMQNKIEFKLKQYGIKIRKVAPNNTSKTCSKCGHLNNYFSFEYRKKNKFPHFKCEKCNFKENSDYNAALNISNPKLMGTKEEP

SEQ ID NO: 3331 - protein, 725 aa, synthetic construct
SEVEFSHEYWMRHALTLAKRARDEREVPVGAVLVLNNRVIGEGWNRAIGQHDPTAHAEIMALRQGGLVMQNYRLVGATLYVTFEPCVMCAGAMIHSRIGRVVYGVRNGKRGAAGSLMNVLNYPGMNHRVEITEGILADECAALLCDFYRMPRRVLNAQKRAQSSINSGGPSGGSSGSETPGTSKSATPESSGGSSGGSAKNTITKTLKLRIVRPYNSAEVEKIVADEKNNREKIALEKNEDKVKEACSEHLKVAAYCTTQVERNACLFCKARKLDDKFYQKLRGQFPDAVFWQEIGEVFRLQKQAAEIYNQSLIELYYEIFIKGKGFANASSVEHYLSDVCYTRAAELFKNAAIASGLRGKVKSNFRLRELKNMKSGLPTTKSDNFPIPLVKQKGGQYTGFEISNHNSDFIIKIPFGRWQVKKEINKYRPWEKFDFEQVRKSPKPISLLLSTQRRKRNKGWSKDEGTEAEIRKVMNGDYQTSYIEVKRGSRIGEKSAWMLSLSIDVPKIDRGVDPSIIGGIDVGVKSPLVCAINNALSRYSISDNDLFHFNKKMFARRRILLKKNRHRRAGHGARNKLKPITVLTEKSKRFRKKLIERWACEIANFFVKNKVGTVQMENLESMKRKEDSYFNIRLRGLWPYAEMQNKIEFKLKQYGIEVRKVAPNNTSKTCSRCGHLNNYFNFEYRKRNKFPHFKCEKCNFKETADYNAALNISNPKLKGTKEEP

SEQ ID NO: 3332 - protein, 726 aa, synthetic construct
SEVEFSHEYWMRHALTLAKRARDEREVPVGAVLVLNNRVIGEGWNRAIGLYDPTAHAEIMALRQGGLVMQNYRLTDATLYVTFEPCVMCAGAMIHSRIGRVVFGVRNSRRGAAGSLMNVLNYPGMNHCVEITEGILVDECAALLCDFYRMPRQVLNAQKKAQSSISSGGSSGGSSGSETPGTSESPTPESSGGGSGGSAKNTITKTLKLRIVRPYNSAEVEKIVADEKSNREKIALEKNKGKVKEACSKHLEVAAYCTTQVERNACLFCKARKLDDKFYQKLRGQFPDAVFWQELGEIFRQLQKQAAEIYNQSLIELYFEIFIKGKGFANASSVEHYLSDVCYTRAAELFKNAAIASGLRGKVKSNFRLKELKNMKSGLPTTKSDNFPIPLVKQKGGQYTGFEISNHDGDFIIKIPFGRWQVKEEINKHRPWEKFDFEQVRKSPKPISLLLSTQRRKRNKGWSKDEGTEAEIRKVMKGDYQTSYIEVKRGSKIGEKSAWMLNLSIDVPKIDKGVDPSIIGGIDVGVKSPLVCAINNALSRYSISDNDLFRFNKKMFARRRILLKKNRHRRAGHGAKNKLKPIAVLAEKSVGFRKKLIERWACEVADFFIKNKVGTVQMENLEGMKRREDSYFNIRLRGFWPYAEMQNKIEFKLKQYGIKVRRVAPNNTSKTCSKCGHLNNYFNFEYRKKSKFPHFKCEKCNFREDADYNAALNISNPKLKSTKEEP

SEQ ID NO: 3333 - protein, 726 aa, synthetic construct
SEVEFGHEYWMRRALTLAKRARDEREVPVGAVLVLNNRVIGVGWNRAVGLHDPTAHAEIMALRQGGLVMQNYRLIDATLYVTFEPCVMCAGAMIHSRIGRVVFGVRNNKHGAAGSLVNVLNYPGMNHRVEVTEGILADECAALLCDFYRMPRRVFNARKKAQSSTNPGGSSGGSSGSETPGTSESATPESSGGSSGGSAKNTITKTLKLRIVRPYNSAEVEKIVADEKNNREKIALEKNKDKVKEACSKHLKVAAYCTTQVERNACLFCKARRLDDKFYQKLRGQFPDAVFWQEIGEIFRQLQKQAAEIYNQSLIELYYEIFIKGKGFANASSVEHYLSDVCYTRAAELFKNAAIASGLRGKVKSNFRLKELKNMKSGLPTTKSDNFPIPLVKQKGGQYTGFEISSHNSDFIIKIPFGRWQEKEEIDKYRPWEKFDFEQVRRSPKPISLLLSTQRRKKNKGWSKDEGTEAEIRRVMNGDYQTSYIEVKRGSKIGEKSAWMLNLSIDVPKIDKGVDPSIIGGIDVGVKSPLVCAINNAFSRYSISDNDLFHFNKKMFARRRILLKKNRRRRAGHGAKNKLKSISILTGKSERFRKKLIERWACEIADFFIKNKVGTVQMENLESMKRKEDSYFNIRLRGFWPYAEMQNKIEFKLKQYGIVVRKVAPNNTSKTCSKCGHLNNYFNFEYRKKNKFPHFKCEKCNFKEVADYNAALNISNPKLKSTKEVP

SEQ ID NO: 3334 - protein, 726 aa, synthetic construct
SEVEFSHEYWMRHALTLAKRARDEREVPVGAVLVLNNRVIGEGWNRAIGLHDPTAHAEIMALRQGGLVMQNYRLIDATLYVTFEPCVMCAGAMVHSRIGRVVFGVRNSKRGAAGSLMNVLDYPGMGHRVEITEGILADKCAALLCDFYCMPRQVFNAQKRAQSCISSGGSSGGSSGSDTPGTSESATPESSGGGSSGSAKNTITKTLQLRIVRPYNSAEVEKIVADEKNNREKIALEKNKDKVREACSKHLKVASYCTTQVERNACPFCKARKLDDKFYQKLRGQFPDAVFWQELGEILRQLQKQAAEIYNQSLIELYYEIFIKGRGFANASSVEHYLSDVCYTRAADLFKNAAIASGLRGKVKGNFRLKELKNMKSGLPTTKSDNFPIPLVKQKGGQYTGFEISSHNDDLIIKIPFGRWQVKKEIDKHRPWEKFDFEQVRKGPKPISLLLSTQRRKRNKGWSKDEGTEAEIRKVMNGDYQTSYIEVKRGGKIGEKSAWMLNLSIDVPKIDKGVDPSIIGGIDVGVKSPLVCAINNAFSRYSISDNDLFHFNKKMFARRRILLKKNRRKRAGHGAKNKLKPISILTEKSERFRKKLIERWACEIANFFIKNKVGTVQMENLESMKRKEDSYFNIRLRGFWPYAEMQDKIEFKLKQYGIEIRRVAPNNTSKTCSRCGHLNNYFNFEYRRKNKFPHFKCEKCNFKENADYNAALNISNPKLKSTKEEP

SEQ ID NO: 3335 - protein, 726 aa, synthetic construct
SEVEFSHEYWMRHALTLAKRARDEREVPVGAVLVLNNRVIGEGWNRAIGLHDPTAHAEIMALRQGGLVMQNYRLVDATLYVTFEPCVLCAGAMIHSRIGRVVFGVRNSKRGAAGSLMNVLNYPGMNHCVEITEGILVDECAALLCDFYRMPRQVLNAQKKAQSSISPGGSSGGSSGSETPGTREGATPESSGGSSGGSAKNTITKTLKLRIVRPYNSAEVEKIVVDEKNNREKVALEKNKDKVKEACSEHLKVAAYCTTQVERSACLFCKARKLDDKFYQKLRGQFPDAVFWQEIGEIFRQLQKQAAEIYNQSLIELYYEIFIKGKGFANASSVEHYLSDVCYTRAAELFKNAAIASGLRGKVKSNFRLKELKNMKSGLPTTKSDNFPIPLVKQKGGQYTGFEISSHNDDFIIKIPFGRWQVKKEIDKYRPWEKFDFEQVRKSPKPISLLLSTRRRKRNKGWSKDEGTEAEIRKVMNSDYQTSYIEVKRGSKIGEKSAWMLNLSIDVPKIDKGVDPSIIGGIDVGVKSPLVCAINNAFGRYSISDNDLFRFNKKVFARRRILLKKNRHKRAGHGTKNKLKPITILTEKSGRFRKKLIERWACEIANFFIKNKVGTVQMENLESMKRKEDSYFNIRLRGFWPYAEMQNKIEFKLKQYGIKIRKVAPNNTSKTCSKCGHLNNYFGFEYRKKNKFPHFKCEKCNFKEDADYNAALNISNPKLKSTKEEP

SEQ ID NO: 3336 - protein, 726 aa, synthetic construct
SEVEFSHEYWMRHALALAKRARDEREVPVGAVLVLNNRVIGEGWNRTTGLHDPTAHAEIMALRQGGLVMQNHRLVDATLYVTFEPCVMCAGAMIHSRIGRVVFGVRNSKRGAAGSLMNVLNYPGMNHRVEITEGILADECAAPLCDFYRMPRQVFNAQKKAQSAINSGGSSGGSSGSETPGTSESPTPESSGGSPGGSAKNTITKTLKLRIVRPYNSAEVEKIVADEKNNREKIALEKNKDKVKEACSKHLKVAAYCTTQVERNACLFCKARRLDDKFYQKLRGQFPDAVFWQEIGEIFRQLQKQAAEVYNQSLVELYYEILIKGKGIANASSVEHYLSDVCYTRAAELFKNAAIASGLRNKIKSNFRLKELRNMKSGLPTTKSDNFPIPLVRQKGGQYTGFEISNHDGDFIIKIPFGRRQVKKEINKHRPWEKFDFEQVRKSPKPISLLLSTQRRKRNKGWSKDEGTEAEIRKVMNGDYQTSYIEVKRGSKIGEKSAWMLNLSIDVPKIDKGVDPSIIGGIDVGVKSPLVCAISNAFSRYSISDNDLFHFNKKMFARRRILLKKSKHKRAGHGAKNKLKPITILTEKSRRFRKKLIERWACEIADFFIKNKVGTVQMENLESMKRREDSYFNIRLRGFWPYAEMQNKIEFKLKQYGIEIRKVAPNNTSRTCSKCGHLNNYFSYEYRKKNKFPHFKCEKCNFKEDADYNAALNISNPKLKGTKEEL

SEQ ID NO: 3337 - protein, 726 aa, synthetic construct
SEVEFSHEYWMRHALTLAKRARDEREVPVGAVLVLNNRVIGEGWNRAIGLHDPTAHAEVMALRQGGLVMQNYRLTDATLYVTFEPCVMCAGAMVHSRIGRVVFGVRNSKRGAAGSLMNVLDYPGMNHCVEITEGILVDECAALLCDFYRMPRQVLNAQKKAQSSISPGGSSGGSSGSETPGASGSVTPKSSGGSSAGSTKDTITKTLKLRIVRPYNSAEVEKIVADEKNSREKIALEKYKDKVKEACSEHLKVAAYCTTQVERNACLFCKARKLDDRFYQKLRGQFPGAVFWQEIGEVFRQLQKQAAEIYNQSLIELYYEIFIKGKGFANASSVEHYLSDVCYTRAAELFKNAAIASGLRGKVKSNFRLKELKNMKSGLPTTKSDNFPIPLVKQKGGQCTGFEINNHNSDFIIKIPFGRWQVKKEIDKYRPWEKFNFEQVRKSPKPISLLLSTQRRKRNKGWSKDEGTEAEIRKVMNGDYQTSYIEVKRGSKIGEKSAWMLSLSIDVPKIDKGVDPSIIGGIDVGVKSPLVCAINNAFNRYSISDNNLFHFNKKMFARRRILLKKNRHKRAGHGAKNKLKPISILTEKSKRFRKKLIERWACEIADFFIKNKVGTVQMENLESMKRKEDSYFNIRLRGFWPYAEMQNKIEFKLKQYGIEIRKVAPNNTSKTCSKCGHLNNYFSFEYRKKNKFPHFKCEKCNFKENADYNAALNISNPKLKSTKEGP

SEQ ID NO: 3338 - protein, 726 aa, synthetic construct
SEVEFSHEYWMRHALTLAKRARDEREVPVGAVLVLNNRVIGEGWNRTTGLHDPTAHAEIMALRQGGLVMQNHRLVDATLYVTFEPCVMCAGAMIHSRIGRVVFGVRNSKRGAAGSLTNVLNYPGMNHHVEITEGILVDECAALLCDFYRMPRQVFNAQKKAQSTINSGGSSGGSSGSETPGTSESPTPESSGGSPGGSAKNTITKTLKLRIVRPYNSAEVEKIVADEKNNREKIALEKNKDKVKEACSKHLKVAAYCTTQVERDACLFCRARKLDDKFYQKLRGQFPDAVFWQEIGEIFRQLQKQAAEIYNQSLIELYYEILIKGKGIANASSVEHYLSDVCYTRAAELFKNAAIASGLRGKVKSNFRLKELKSMKSGLPSTKSDNFPIPLVKQRGGQYTGFEIGSHNDDFIIKIPFGRWQAKKEIDKYRPWEKFDFEQVRKSPKPISLLLSTQRRKRNRGWSKDEGTEAEIRKVLNGDYQTSYIEVKRGSKTGEKSAWMLNLSIDVPKIDKGVDPSIIGGIDVGVKSPLVCAINNAFSRYSISDNDLFRFNKKMFARRRILLKKNRHKRAGHGAKNKLKPISILTGKSERFRKKLIERWACEIADFFVKNKVGTVQMENLESMKRKEDSYFNIRLRGFWPYAEMQNKIEFKLKQYGIRVRKVAPNNTSKTCSKCGHLNNYFSFEYRKKNKFPHFKCEKCNFKENADYNAALNISNPKLKSTKEEP

SEQ ID NO: 3339 - protein, 726 aa, synthetic construct
SEVEFSHEYWMRHALTLAKRARDEREVPVGAVLVLNNSVIGEGWNRAIGLHDPTAHAEIMALRQGGLVMQNYRLIDATLYVTFEPCVMCAGAMIHSRIGRVVFGVRNSKHGAAGSLMNVLNYPGMNHRVEITEGILADECAALLCDFYRMPRQVLNAQKKAQSGISSGGSSGGSSGGETPGASESVTPKSSAGSSAGSTKNTITKTLKLRIVRPYNSAEVEKIVADEKNNREKIALEKNKNKVKEACSKHLKVAAYCTTQVERSACLFCKARKLDDKFYQKLRGQFPDAVFWQELGGIFRQLQKQAAEIYNQSLIELYYEIFIKGRGFANASSVEHYLSDVCYTRAAELFKNAAIASGLRGKVKSNFRLKELKNMKSGLPTTKSDNFPIPLVKQKGGQYTGFEISSHNDDFIIKIPFGRWQMKKEIDRYRPWEKFDFEQVRKSPKPISLLLSTQRRKRNKGWSKDEGTEAEIRRVMNGDYQTSYIEVKRGSKAGEKSAWVLSLSIDVPRIDKGVDPSIIGGIDVGVKSPLVCAINNAFSRYSISDNDLFRFNKKMFARRRILLKKNRHKRAGHGARNKLKPITILTKKSERFRKKLIERWVCEVADFFIKSKVGTVQMENLESMKRREDSYFNTRLRGFWPYAEMQNKIEFKLKQYGIEIRKVAPNNTSKTCSKCGHLNNYFNFEYRKKNKFPHFKCEKCYFKEDADYNAALNISNPKLRSTKEEP

SEQ ID NO: 3340 - protein, 726 aa, synthetic construct
SEVEFSHEYWMRHALTLAKRARDEREVPVGAILVLNNRVIGEGWNRAIGLHDPTAHAEIMALRQGGLVMQNYRLIDATLYVTFEPCVMCAGAMIHSRIGRVVYGVRNNKHGAAGSLVNVLNYPGMNHCVEITEGILVDECAALLCDFYCMPRQVFNAQKRAQSSINSGGSSGGSSGSETLGTSESATPGSSGGGSSGSAKNTITKTLQLRIVRPYNSAEVEKIVADEKNNREKIALEKNKDKVKEACSKHLKVAAYCTTQVERNACLFCKARKLDDKFYQKLRGQFPDAVFWQEIGEIFRQLQKQAAEIYNQSLIELYYEIFIKGKGFANASSVEHYLSDVCYTRAAELFKNAAIASGLRGKVKSNFRLKELKNMKSGLPTTKSDNFPIPLVKQKGGQYTGFEISSHNDDFIIKIPFGRWQVKKEINKHRPWEKFDFEQVRKSPKPISLLLSTQRRKRNKGWSKDEGTEAEIRKVMNGDYQTSYIEVRRGSKIGERSAWMLNLSIDVPKIDKGVNPSIIGGIDVGVKSPLVCAINNAFSRYSISDNDLFRFNKKMFARRRILLGKNRHKRAGHGVKNKLKPITILTEKSKRFRKKLIERWACEIADFFIKNKVGTVQMENLESMKRKEDSYFNIRLRGFWPYAEMQNKIEFKLKQYGIKIRKVAPNNTSKTCSKCGHLNNYFNFEYRKKNKFPHFKCEKCNFKEDADYNAGLNISNPKLKSTKEEP

SEQ ID NO: 3341 - protein, 726 aa, synthetic construct
SEVEFSHEYWMRHALTLAKRARDEREVPVGAVLVLNNRVIGEGWNRAIGLHDPTAHAEIMALRQGGLVMQNYRLTDATLYVTFEPCVMCAGAMVHSRIGRVVFGVRNSKHGAAGSLMNVLNYPGMNHRVEITEGILADECAALLCDFYRMPRQVFNARKKTQSSINSGGPSGGSSGSETPDTSESATPESSSGSSGGSAKNTITKTLKLRIVRPYNSAEVEKIVADEKNNREKIALEKNKDKVKEACSKHLKVAAYCTTQVERNACLFCKARRLDDKFYQKLRGQFPDAVFWQEIGEIFRQLQKQAAEVYNQSLVELYYEILIKGKGIANASSVEHYLSDVCYTRAAELFKNAAIASGLRNRIKSNFRLKELRNMKSGLPTTKSDNFPIPLVRQKGGQYTGFEISSHNDDFIIKIPFGRWQVKKEINKHRPWEKFDFEQVRRSPKPISLLLSTQRRKRNKGWSKDEGTEAEIRKVMNGDYQTSYIEVKRGSKIGEKSAWMLNLSIDVPKIDKGVDPSIIGGIDVGVKSPLVCAINNAFSRYSIIDNDLFRFNKKMFARRRILLKKSRHKRAGHGAKNKLKPITILTEKSRRFRKKLIEKWACEIADFFIKNKVGTVQMENLESMKRKEDSYFNIRLRGFWPYAEMQNKIEFKLKQYGIVVRKVAPNNTSKTCSKCGHLNNYFNFEYRKKNKFPHFKCERCNFKEDADYNAALNISNPKLKGTKGEP

SEQ ID NO: 3342 - protein, 726 aa, synthetic construct
SEVEFSHEYWMRRALTLAKRARDEREVPVGAVLVLNNRVIGVGWNRAVGLHDPTAHAEIMALRQGGLVMQNYRLIEATLYVTFEPCIMCAGAMIHSRIGRVVFGVRNSKRGAAGSLMNVLNYPGMNHCVEITEGILVDECAALLCDFYRMPRQVLNAQKKAQPSISPGGSSGGSSGSETPGASGSVTPKSSGGSSAGSTKDTITKTLKLRIVRPYNSAEVEKIVADERNSREKIALEKNKDKVKEACSEHLKVAAYCTTQVERNACLFCKARRLDDKFYQKLRGQFPDAVFWQEIGEIFRQLQKQAAEIYNQSLIELYYEIFIKGKGFANASSVEHYLSDVCYTRAAELFKNAAIASGLRGKVKSNFRLKELKNMKSGLPTTKSDNFPIPLVKQKGGQYTGFEISSHNDDFIIKIPFGRWQVKKEIDKYRPWEKFDFEQVRKSPKPISLLLSTQRRKRNKGWSKDEGTEAEIRKVMNGDYQTSYIEVKRGSKTGEKSAWMLNLSIDVPKIDKGVDPSIIGGIDVGVKSPLVCAINNSSSRYSICDNDLFRFNKKMFARRRILLKKNRHKRAGHGAKNKLKPITILTKKSERFRKKLIERWVCEVADFFIKNKVGTVQMENLESMKRKEDSYFNIRLRGFWPYAEMQNKIEFKLKQYGIEIRKVAPNNTSKTCSKCGHLNNYFNFEYRKKNKFPHFKCEKCNFKENADYNAALNISNPKLKSTKEEP

SEQ ID NO: 3343 - protein, 725 aa, synthetic construct
SEVEFSHEYWMRHALTLAKRARDEREVPVGAVLVLNNRVIGEGWNRAIGLHDPTAHAEIMALRQGGLVMQNYRLVDATLYVTFEPCVLCAGAMVHSRIGRVVFGVRNSKRGAAGSLMNVLNYPGMNHRVEITEGILADECAALLCDFYCMPRQVFNAQKRAQSSINSGGSSGGSSGSETPGTSESATPESSGGGPSGSAKNTITKTLQLRIVRPYNSAEVEKIVTDEKNNREKIALEKNKDKVKEACSKHLKMASYCTTQVERNACLFCKARKLDDKFYQRLRGQFPDAVFWQELGEIFRQLQKQAAEVYNQSLIELYYEIFIKGKGFANAGSVEHYLSDVCYTRAAELFKNAAIASGLRGKVKSNFRLKELKNMKSGLPTTKSDNFPIPLVRQKGGQYTGFEISSHNDDFIIKIPFGRWAKKEIDKYRPWEKFDFEQVRKSPRPISLLLSTQRRKRNRGWSKDEGTEAEIRKVMNGEYQTSYIEVKRGSKIGEKSAWMLNLSIDVPKIDKGVDPSIVGGIDVGVKSPLVCAIDNALSRYSISDNDLFHFNKKMFARRRVLLKKNRHRRAGHGAKNKLKPLTIMTEKSKRFRKKLIERWACEIADFFIKNKVGTVQMENLESMKRKEDSYFNIRLRGFWPYAEMQNKIEFKLKQYGIEIRRVAPNNTSKTCSKCGHLNNYFNFEYRKKNKFPHFKCEKCNFKENADYNAALNISNPRLKSTKEEP

SEQ ID NO: 3344 - protein, 726 aa, synthetic construct
GEVEFSHEYWMRHALTLAKCARDEREVPVGAILVLNNRVIGEGWNRAIGLHDPTAHAEIMALRQGGLVMQNYRLIDATLYVTFEPCVMCAGAMIHSRIGRVVFGVRNNKHGAAGSLVNVLNYPGMNHRVEITEGILANECAALLCDFYRMPRQVFNARKKAQSSINPGGSSGDSSGSETPGTSESATPESSGGSSGGSAKNTITKTLKLRIVRPYNSAEVEKIVADEKNNREKIALEKNKDKVKEACSKHLKVAAYCTTQVERNACLFCKARRLDDKFYQKLRGQFPDAVFWQEIGEIFRQLQKQAAEIYNQSLVELYYEILIKGKGIANASSVEHYLSDVCYTRAAELFKNAAIASGLRNKIKSNFRLKELRNMKSGLPTTKSDNFPIPLVRQKGGRYTGFEISNHNGDFIIKIPFGRWQVKKEINKHRPWEKFDFEQVRKSPKPISLLLSTQRRKRNRGWSKDESTEAEIKKVMNGDYQTSYIEVKRGSKIGEKSAWMLNLSIDVPKIDKGVDPSIVGGIDVGVKSPLVCAIDNALSRYSISDNDLFHFNKKMFARRRVLLKRNRHRRAGHGAKNKLKPISILTEKSKRFRKKLIERWACEIADFFIKNKVGTVQMENLESMKRKEDSYFNIRLRGFWPYAEMQNKVEFKLKQYGIEVRKVAPNNTSKTCSRCGHLNNYFNFEYRRKNKFPHFKCEKCNFKENADYNAALNISNPKLKSTKEEP

SEQ ID NO: 3345 - protein, 726 aa, synthetic construct
SEVEFSHEYWMRHALTLAKRARDEREVPVGAVLVLNNRVIGEGWNRAIGLHDPTAHAEIMALRQGGLVMQNYRLIDATLYVTFEPCVMCAGAMIHSRIGRVVFGVRNSKRGAAGSLMNVLNYPGMNHRVEITEGILADECAALLCDFYRMPRQVFNAQKKAQSSINSGGSSGGSSGSETPGTSESATPESSGGSSGGSAKNTITKTLKLRIVRPYNSAEVEKIVADEKNNREKIALEKNKDKVKEACSKHLKVAAYCTTQVERNACLFCKARKLDDKFYQKLRGQFPDAVFWQEISEIFRQLQKQAAEIYNQSLIELYYEIFIKGKGIANASSVEHYLSDVCYTRAAELFKNAAIASGLRSKIKSNFRLKELKNMKSGLPTTKSDNFPIPLVKQKGGQYTGFEISNHNSDFIIKIPFGRWQVKKEIDKYRPSEKFDFEQVQKSPKPISLLLSTQRRKRNKGWSKDEGTEAEIKKVMNGDYQTSYIEVKRGSKIGEKSAWMLNLSIDVPKIDKGVDPSIIGGIDVGVKSPLVCAINNAFSRYSISDNDLFHFNKKMFARRRILLKKNRHKRAGHGAKNKLKPITILTEKSERFRKKLIERWACEIADFFIKNKVGTVQMENLESMKRKEDSYFNIRLRGFWPYAEMQNKIEFKLKQYGIEIRKVAPNNTSKTCSKCGHLNNYFNFEYRKKNKFPHFKCEKCNFKENADYNAALNISNPKLKSTKEEP

SEQ ID NO: 3346 - protein, 726 aa, synthetic construct
GEVEFSHEYWMRRALTLAKRARDEREVPVGAILVLNNRVIGEGWNRAIGLHDPTAHAEITALRQGGLVMQNYRLIDATLYVTFEPCVMCAGAMIHSRIGRVVFGVRNSKHGAAGSLVNVLNYPGMNHRVEITEGILADECAALLCDFYRMPRQVFNARKKAQPSINPGGSSGGSSDSETPGTSESATPESSGSSSGGSAKNTITKTLKLRIVRPYNSAEVEKIVADEKNNREKIALEKNKDKVKEACSKHLKVAAYCTTQVERNACLFCKARRLDDKFYQKLRGQFPDAVFWQEIGEIFRQLQKQAAEIYNQSLIELYYEIFIKGKGIANASSVEHYLSDVCYTRAAELFKNAAIASGLRNKVKSNFRLKELRNMRGGLPTTKSDNFPIPLVKQKGGQYTGFEISNHNDDFIIKIPFGRWQMKKEIDKYRPWEKFDFEQVRKSPKPISLLLSTQRRKRNKGWSKDEGTEAEIRKVMNSDYQTSYIEVKRGSKIGEKSAWMLNLSIDVPKIDKGVDPSIVGGIDVGVKSPLVCAIDSALSRYSISDNDLFHFNKKLFARRRILLKKNRHRRAGHGAKNKLKPISILTEKSKRFRKKLIERWACEVADFFIKNKVGTVQMENLESMKRKEDSYFNIRLRGFWPYAEMQNKIEFKLKQYGIEIRKVAPNNTSKTCSKCGHLNNYFNFEYRKKNKFPHFKCEKCNFKENADYNAALNISNPMLKSTMEEP

SEQ ID NO: 3347 - protein, 726 aa, synthetic construct
SEVEFSHEYWMRHALTLAKRARDEREVPVGAVLVLNNRVIGEGWNRAIGLHDPTAHAEIMALRQGGLVMQNYRLVDATLYVTFEPCVLCAGAMVHSRIGRVVFGVRNNKRGAAGSLMNILNYPGMGHRVEITEGVLADECAALLCDFYCMPRQVFSAQKRAQSSINSGGSSGGSSGSETPGTSESATPESSGGGSSGSAKNTITKTLQLRIVRPYNSAEVEKIVADEKNNREKIALEKNKDKVKEACSKHLKVASYCTTQVGRNACLFCKARRLDDKFYQKLRGQFPDAVFWQEIGEIFRQLQKQAAEIYNQSLVELYYEILIKGKGIANASSVEHYLSDVCYTRAAELFKNAAIASGLRSKIKSNFRLKELKNMKSGLPTTKSDNFPIPLVKQKGGQYTGFEISSHNDDFIIKIPFGRWQVKKEIDKYRPWEKFDFEQVRKSPKPISLLLSTQGRKKNKGWSRDEGTEAEIRKVMNGDYQTSYIEVKRGSKIGEKSAWTLNLSIDVPKIDKGVDPSIIGGIDVGVKSPLVCAINNASSRYSISDNDLFRFNKKMFARRRILLKKNRHKRAGHGAKNKLKPISILTEKSERFRKKLIERWACEIADFFVKNKVGTVQMENLESMKGKEDSYFNIRLRGFWPYAGMQNKIEFKLKQYGIEIRKVAPNNTSKTCSKCGHLNNYFDFEYRKKNKFPHFKCEKCNFKENADYNAALNISNPKLMSTKEEP

SEQ ID NO: 3348 - protein, 726 aa, synthetic construct
SEDEFSHEYWMRHALTLAKRARDGREVPVGAVLVLNNRVIGEGWNRAIGLHDPTAHAEIMALRQGGLVLQNYRLVDATLYVTFEPCVLCAGAMVHSRIGRVVFGARNSKRGAAGSLMNILNYPGMNHRVEITEGILADECAALLCDFYRMPRQVFNARKKAQSSINSGGSSGGSSGSETPGTSESATPKSSGGSSGGSAKNTVTKALKLRIVRPYNSAEVEKIVADEKNNRERIALEKNKDKVKEACSKHLKVAAYCTTQVERNACLFCKARKLDDKFYQKLRGQFPDAVFWQEIGEIFRQLQKQAAEIYNQSLIELYYEIFIKGKGFANASSVEHYLSDVCYTRAAELFKNAAIASGLRGKVKSNFRLKELKNMKSGLPTTKSDNFPIPLVKQKGGQYTGFEISSHNDDFIIKIPFGRWQVKKEIDKYRPWEKFDFEQVRKSPKPISLLLSTQRRKRNRGWSKDEGTEAEIRKVMNGDYQTSYIEVKRGSKIGEKSAWMLNLSIDVPKIDKGVDPSIIGGIDVGVKSPLVCAINNAFSRYSVSDNDLFHYNKKMFARRRILQKKNRYKRAGHGAKNKLKPISILTEKSKRFRKKLIERWACEIADFFIKNKVGTVQVENLESMKRREDSYFNVRLRGFWPYAEMQNKIEFKLRQYGIEIRKVAPNNTSKTCSKCGHLNNYFSFEYRKKNKFPHFKCEKCNFKENADYNAALNISNPKLKSTKEEP

SEQ ID NO: 3349 - protein, 726 aa, synthetic construct
SEVEFSHEYWMRHALTLAKRARDEREVPVGAVLVLNNRVIGEGWNRAIGLHDPTAHAEIMALRQGGLAMQNYRLVDATLYVTFEPCVLCAGAMVHSRIGRVVFGVRNSKRGAAGSLMNVLNHPGMNHRVEITGGILADECAALLCDFYRMPRQVFNAQKKARSNINSGGSSGCSSGNETPGASESTTPESSGGSSGGSAKNTITKTLKLRIVRPYNSAEVEKIVADEKNNREKIALEKNKDKVKEACSKHLKVAAYCTTQVERNACQFCRARKLDDKFYQKLRGQFPDAVFWQEIGEIFRQLQKQAAEIYNQSLIELYYEIFIKGKGFANASSVEHYLSDVCYTRAAELFKNAAIASGLRGKVKSNFRLKELKNMKSGLPTTKSDNFPIPLVKQKGGQYTGFEISSHNDDFIIKIPFGRWQVKKEIDKYRPWEKFDFEQVRKSPKPISLLLSTQRRKRNRGWSKDVGTEAEIRKVMNGDYQTSYIEVKRGSKIGEKSAWMLNLSIDVPKIDKGVDPSITGGIDVGVKSPLVCAINNAFSRYSISDNDLFRFNKKVFARRRILLKKNRHRRAGHGAKNKLKPIAVLAEKSEGFRKKLIERWACEVADFFIKNKVGTVQLENLESMKRREDSYFNIRLRGFWPYAEMQNKIEFKLRQYGIEIRKVAPNNTSKTCSKCGHLNNYFDFEYRKKNKFPHFKCEKCNFKENADYNAALNISNPKLRSTKEEP

SEQ ID NO: 3350 - protein, 726 aa, synthetic construct
SEVEFSHEYWMRHALTLAKRARDEREVPVGAILVLNNRVIGEGWNRAIGLHDPTAHAEIMALRQGGLVMQNYRLIDATLYVTFEPCVMCAGAMIHSRIGRVVFGVRNSKHGAAGSLVNVLNYPGMNHRVEITEGILADECAALLCDFYRMPRQVFNARKKAQSSINPSGSSGGSSGSVTPGTSESATPESSGGGFGGSAKNTITKTLQLRIVRPYNSAEVEKIVADEKNNREKIALEKYKDKVKEACSKHLKVASYCTTQVERNACLFCKARKLDDKFYQKLRGQFPDAVFWQEIGEIFRQLQKQAAEIYNQSLVELYYEILIKGKGIANASSVEHYLSDVCYTRAAELFKNAAIASGLRNKIKSNFRLKELRNMKSGLPTTKSDNFPIPLVRQKGGQYTGFEVSSHNDDFIIKIPFGRWQVKKEIDKYRPWEKFDFEQVRKSPRPISLLLSTQRRKRNKGWSKDEGTEAEIRKVMNGDYQTSYIEVKRGSKIGEKSAWMLNLSIDVPKIDKGVDPSIIGGIDVGVKSPLVCAIDNAFSRYSISDNDLYHFNKKMFARRRILLKKNRHRRAGHGAKNKLKPITILTEKSGRFRKKLIERWACEIANFFIKNKVGTVQVENLESMKRREDSYFNIRLRGFWPYAEMQNKIEFKLKQYGIEIRKVAPNNTSKTCSKCGHLNNYFNFEYRKKNKFPHFKCEKCNFKENADYNAALNISNPKLKSTKEEP

SEQ ID NO: 3351 - protein, 726 aa, synthetic construct
SEVEFSHEYWMRHALILAKRARDEREVPVGAVLVLNNRAIGEGWNRAIGLHDPTAHAEIMALRQGGLVMQNYRLTDATLYVTFEPCVMCAGAMIHSRIGRVVFGVRNSKRGAAGSLMNVLNYPGMNHCVEITEGILVDECAALLCDFYRMPRQVLNAQKKAQSSISSGGSSGGSSGSETPGASGSVTPKSSGGSSAGSTKDTITKTLKLRIVRPYNSAEVEKIVADEKSNREKIALEKNKDKVEEACSEHLKVAAYCTTQVERSACLFCKARKLDDKFYQKLRGQFPDAVFWQEVGEIFRQLQKQAAEIYNQSLIELYYEIFIKGKGFANASSVEHYLSDVCYTRAAELFKNAAIASGLRGKVKSNFRLRELKNMKSGLPTTKSDNFPIPLVKQKGGQYTGFEISNHNDDFIIKIPFGRWQVKKEIDKYRPWVKFDFEQVRKSPKPISLLLSTQRRKRNKGWGKDEGTEAEIRKVMNGDYQTSYIEVKRGSKTGEKSAWMLNLSIDVPKIDKGVDPSIIGGIDVGVKSPLVCAINNALSRYSISDNDLFHFNKKMFARRRILLRKNRHKRAGHGAKNKLKPITILTEKSRRFRKKLIERWACEIADFFIKNKVGTVQMENLEGMKRKEDSYFNIRLRGFWPYAEMQNKIEFKLKQYGIEIRKVAPNNTSKTCSRCGHLNNYFSFEYRKKNKFPHFKCEKCNFKENADYNAALNISNPKLKSTKEEP

SEQ ID NO: 3352 - protein, 726 aa, synthetic construct
SEVEFSHEYWMRHALTLAKRARDEREVPVGAVLVLNNRVIGEGWNRAIGLHDPTAHAEIMALRQGGLVMQNYRLIDATLYVTFEPCVMCAGAMIHSRIGRAVFGVRNSKHGAAGSLMNVLDYPGMDHRVEITEGILADECAALLCDFYRMPRQVFNAQKKAQSNTNSGGSSGGSSGSETPGTSESPTPESSGGSSGGSAKSTITKTLRLRIVRPYNSAEVEKIVADEKNNREKIALEKNKDKVKEACSKHLKVAAYCTTQVERNACLFCKARKLDDKFYQKLRGQFSDAVFWQEIGEIFRQLQKQAAEIYNQSLIELYYEIFIKGKGITNASRVEHYLSDVCYTRAAELFKNAAIASGLRNKIKSNFRLKELKNMKSGLPTTKSDNFPIPLVKQKGGQYTGFEISNHNGDFIIKVPFGRWQAKKEIDKYRPWEKFDFEQVRKSPKPISLLLSTQRRKRNRGWSKDEGTEAEIRKVMNGDYQTSYIEVKRGSRIGEKSAWMLNLSIDVPKIDKGVDPSIIGGIDVGVKSPLVCAINNAFSRYSISDNDLFHFNKKMFARRRILLKKNGHKRAGHGAKNKLKPITIMTEKSKRFRKKLIERWACEIADFFIKNKVGTVQMENLESMKRKEDSYFNIRLRGFWPYAEMQNKIEFKLKQYGIEIRKVAPNNTSKTCSKCGHLNNYFNFEYRKKNKFPHFKCEKCNFKENADYNAALNISNPKLESTKEEP

SEQ ID NO: 3353 - protein, 726 aa, synthetic construct
SEVEFSHEYWMRHALTLAKRARDEREVPVGAVLVLNNRVIGEGWNRAIGLHDPTAHAEIMALRQGGLVMQNYRLVDATLYVTFEPCVLCAGAMVHSRIGRVVFGVRNSKRGAAGSLMNVLNYPGMNHRVEITEGILADECAALLCDFYRMPRQVFNAQKKARSNINPGGSSGGSSGSETPGTSESATPESSGGSSAGSTKDTITKTLKLRIVRPYNSAEVEKIVADEKNSREKIALEKNKDKVKEACSEHLKVAAYCTTQVERNACLFCKARKLDDGFYQKLRGQFPDAVFWQEIGEIFRQLQKQAAEIYNQSLIELYYEIFIKGKGFANASSVEHYLSDVCYTRAAELFKNAAIASGLRNKTKSNFRLKELRSMKSGLPTTKSDNFPIPLVKQKGGQYTGFEISNHNSDFIIKIPFGRWQVKKEINRYRPWEMFDFEQVRKSPKPISLLLSTQRRKRNKGWSKDEGTEAEIRKVMNGDYQTSYIEVKRGSKTGERSAWMLNLSIDVPKIDKGVDPSIIGGIDVGVKSPLVCAINNAFSRYSISDNDLFRFNKKMFARRRILLKKNRHKRAGHGAKNKLKPISILTGKSERFRKKLIERWACEIADFFIKNKVGTVQMENLESMKRKEDSYFNIRLRGFWPYAEMQNKIEFKLKQYGIEIRKVAPNNTSKTCSKCGHLNNYFNFEYRKKNKFPHFKCEKCNFKEDADYNAALNISNPKLKSTKEEP

SEQ ID NO: 3354 - protein, 726 aa, synthetic construct
SEVEFSHEYWMRHALTLAKRARDEREVPVGAVLVLNNRVIGVGWNRAIGLHDPTAHAEIMAMRQGGLVLQNYRLIDATLYVTFEPCVMCAGAMIHSRIGRVVFGVRNNKHGAAGSLVNVLNYPGMNHRVEITEGILADECAALLCDFYRMPRQVFNARKKAQSSINPGGSSGGSSGSETPGTSGSTTPVSSGGSSGGSAKNTITKALKLRIVRPYNSAEVEKIVADEKNNREKIALEKNKDKVKEACSKHLKMASYCTTQVERNACLFCKARKLDDKFYQKLRGQFPDAVFWQELGGIFRQLQKQAAEIYNQSLIELYYEIFIKGKGITNASRVEHYLSDVCYTRAAELFKNAAVASGLRGKVKSNFRLKELKNMKSGLPSTKSDNFPIPLVKQRGGQYTGFEISSHNDDFIIKIPFGRWQAKKEIDKYRPWEKFDFEQVRKNPKPISLLLSTQRRKRNKGWSKDEGTEAEIRKVMNGDYQTSYIEVKRGSKIGEKSAWMLNLSIDVPKIDKGVDPSIIGGIDVGVKSPLVCAVNNAFSRYSISDNDLFRFNKKVFARRRILLKKNRHKRAGHGAKNKLKPISILTEKSERFRKKLIERWACEIADFFIKNRVGTVQMENLESMKRREDSYFNIRLRGFWPYAKMLNRIEFKLKQYGIKIRKVAPNNTSKTCSKCGHLNNYFNFEYRKKNKFPHFKCEKCNFKENADYNAALNISNPKLKSTKGEP

SEQ ID NO: 3355 - protein, 726 aa, synthetic construct
SEVEFSHEHWMRHALTLAKRARDEREVPVGAVLVLNNRVIGEGWNRAIGLHDPTAHAEIMALRQGGQVMQNYRLTDATLYVTFEPCVMCAGAMIHSRIGRVVFGVRNSKRGAAGSLMNVLNYPGMNHCVEITEGILVDECAALLCDFYRMPRQVLNAQKKAQSSISSGGSSGGSSGSETPGASGSVTPKSSGGSSAGSTKDAITKTLKLRIVRPYNSAEVEKIVADEKNNREKIALEKNKDKVKEACSKHLKVAAYCTTQVERNACLFCKARKLDDKFYQKLRGQFPDAVFWQEIGEIFRQLQKQAAEIYNQSLIELYYEIFIKGKGFANASSVEHYLSDVCYTRAAELFKNAAIASGLRGKVKSNFRLKELKNMKSGLPTTKSDNFPIPLVKQKGGQYTGFEISSHNDDIIIKIPFGRWQVKKEIDKYRPWEKFDFEQVRKCPKPISLLLSTQRRKRNKGWSKDEGTEAEIRKVMNGDYQTSYIEVKRGSKIGEKSAWMLSLSIDVPKIDKGVDPSIIGGIDVGVKSPLVCAINNAFNRYSISDNNLFHFNKKMFARRRILLKKTRHKRAGHGAKNKLKPISTLTEKSERFRKKLIERWACEIADFFIKNKVGTVQMENLESMKRREDSYFNIRLRGFWPYAKMQNKIEFKLKQYGIEIRKVAPNNTSKTCSKCGHLNNYFNFEYRKKNKFPHFKCEKCNFKESADYNAALNISNPKLKSTKEEP

SEQ ID NO: 3356 - protein, 726 aa, synthetic construct
SEVEFSHEYWMRHALTLAKRARDEREVPVGAVLVLNNRVIGEGWNRAIGLHDPTAHAEIMALRQGGLVMQNYRLIDATLYVTFEPCVMCAGAMVHSRIGRVVFGVRNSKRGAAGSLMNVLNYPGMSHCVGITEGILVDECAALLCDFYRMPRQVLDAQKKAQSSISSGGSSGGSGGGETPGASESVTPKNSGGSPAGSTKNTITKTLKLRIVRPYNSAEVEKIVADEKNNREKIALKKNKDKVKEACREHLKVASYCTTQVERNACLFCKARKLDDKFYQKLRGQFPDAVFWQELGGIFRQLQKQAAEIYNQSLIGLYYEIFIKGKGITNASRVEHYLSDVCYTRAAELFKNAAIASGLRSKVRSNFRLKELKNMKSGLPTTKSDNFPIPLVKQKGGQYTGFEISSHNSDFIIKIPFGRWQVKEGIDKYRPWEKFDFEQVRKSPKPISLLLSTQRRKKNKGWSKDEGTEAEIRRVMNGDYQTSYIEVKRGSKIGEKSAWMLNLSIDVPKIDKGVDPSIIGGIDVGVKSPLVCAINNAFSRYSICDNDLFRFNKKMFARRRILLKKNRHKRAGHGAKNKLKPITILTKKSERFRKKLIERWACEVADFFIKNKVGTVQMENLESMKRKEDSYFNIRLRGFWPYAEMQNRIEFKLKQYGIEIRRVAPNNTSRTCSKCGHLNNYFNFEYRKKNKFPHFKCEKCNFKENADYNAALNISNPRLKSTKEEP

SEQ ID NO: 3357 - protein, 726 aa, synthetic construct
SEDEFSHEYWMRHALTLAKRARDGREVPVGAVLVLNNRVIGEGWNRTTGLHDPTAHAEIMALRQGGLVMQNYRLIDATLYVTFEPCVMCAGAMIHSRIGRVVFGVRNNKHGAAGSLVNVLNYPGMNHRVEITEGILANECAALLCDFYRMPRQVFNARKKAQSSINPGGPSGGSSGSETPDTSESATLESPGGSSGDSAKNSITKTLKLRIVRPYNSAEVEKIVADEKNNREKIALEKNKGKVKEACSKHLKVATYCTTQVERNACLFCKARKLDDKFYQKLRGQFPDAVFWQEIGEIFRQLQKQAAEIYNQSLIELYYEIFIEGKGSANARSVEHYLSDVCYTRAAELFKNAAIASGLRGKVKSNFRLKELKSMKSGLPTTKSDNFPIPLVKQKGGQYTGFEISSHNDDFIIKIPFGRWQEKKEINKYRPWEKFDFEQVRKSPKPISLLLSTQRRKRNKGWSKDEGTEAEIRKVMNGNYQTSYIEVKRGSKIGEKNAWMLSLSIDVPKVDKGVDPSIIGGIDVGVKSPLVCAINNALSRYSISDNDLFHFNKKMFARRRILLKKNRHKRAGHGARNKLRPITVLTEKSERFRKKLIERWACEIANFFIKNKVGTVQMEDLESMKRKEDSYFNIRLRGFWPYAEMQNKIEFKLKQHGIEIRKVAPNNTSKTCSVCGHLNNYFNFEYRKKNKFPHFKCEKCNFKENADYNAALNISNPKLKSTKEEP

SEQ ID NO: 3358 - protein, 726 aa, synthetic construct
SEVEFSHEYWMRHALTLAKRARDEREVPVGAILVLNNRVIGEGWNRAIGLHDPTAHAEIMALRQGGLVMQNYRLIDATLYVTFEPCVMCAGAMIHSRIGRVVFGVRNSKHGAAGSLVNVLNYPGMNHRVEITEGILADECAALLCDFYRMPRQVFNAQKKAQSSINSGGSSGGCSGSETPGTSESATPESSGGSSGGSTKNTITKTLKLRIVRPYNSAEVEKIVADEKSNREKIALEKNKDKVKEACSEHLKVAAYCTTQVERSACLFCKARKLDDKFYQKLRGQFPDAVFWQEIGEIFRQLQKQAAEIYNQSLIELYYEIFIKGKGFANTSSVEHYLSDVCYTRAAELFKNAAIASGLRGKVKSNFRLKELRNMRSGLPTAKSDNFPIPLVKQKGGQYTGFEISSHNDDFIIKIPFGRWQVKKEIDKYRPWEKFDFEQVRKSPKPISLLLSTQRRKRNKGWSKDEGTEAEIRKVMNGDYQTSYIEVKRGSKIGEKSAWMLNLSIDVPKIDKGVDPSIIGGIDVGVKSPLVCAINNAFSRYSISDNDLFRFNKKMFARRRILLGKNRHKRAGHGAKNKLKPITILTKKSERFRKKLIERWVCEVADFFIKNKVGTVQMENLESMKRKEDSYFNIRLRGFWPYAEMQNKIEFKLKQYGIEIRKVAPNNTSKTCSKCGHLNNYFNFEYRKKNKFPHFKCEKCNFKENADYNAALNISNPKLKSTKEEP

SEQ ID NO: 3359 - protein, 726 aa, synthetic construct
SEVEFSHEYWMRHALTLAKRARDEREVPVGAVLVLNNRVIGEGWNRAIGLHDPTAHAEIMALHQGGLVMQNYRLIDATLYVTFEPCVMCAGAMIHSRIGRVVFGARNSKRGAAGSLMNVLSYPGMNHRVEITEGILADECAALLRDFYRMPRRVFNAQKKAQSSINSGGSSGGSGGSETPGASESATPKSSVGSSAGSTKSTITKTLKLRIVRPYNSAEVEKIVADEKNNREKIALEKNKDKVKEACSKHLKVAAYCTTQVERNACLFCKARKLDDKFYQKLRGQFPDAVFWQETGEIFRQLQRQAAEIYNQSLIELYYEIFIKGKGFANASSVEHYLSDVCYTRAAELFKNAAIASGLRGKVKGNFRLKELKNMKSGLPTTMSGNFPIPLVKQKGGQYTGFEISSHNDDFIIKIPFGRWQVKKEIDKYRPWEKFDFEQVRKSPKPISLLLSTQRRKRNKGWSKDEGTEAEIRKVMNGDYQTSYIEVKRGSKIGEKSAWMLNLSIGVPKIDKGVNPSIIGGIDVGVKSPLVCAINNAFSRYSISDNDLFHFNKKMFARRRILLKKNRHKRAGHGAKNKLKPISILTEKSKRFRKKLIERWACEIADFFIKNKVGTVQMENLESMKRKEDSYFNIRLRGFWPYAEMQNRIEFKLKQYGIEIRKVAPNNTSKTCSKCGHLNNYFNFEYRKKNKFPHFKCERCNFKENADYNAALNISNPKLKSTKEES

SEQ ID NO: 3360 - protein, 726 aa, synthetic construct
SEVEFSHEYWMRHALTLAKRARDEREVPVGAVLVLNNRVIGEGWNRAIGLHDPTAHAEIMALRQGGLVMRNYRLTDATLYVTFEPCVMCAGAMIHSRIGRVVFGVRNSKRGAAGSLMNVLNYPGMNHCVEITEGILVDECAALLCDFYRMPRQVLNAQKKAQSSISPGGSSGGSSGSETPGASESVTPKSSGGSSGGSAKNTITKTLKLRIVRPYNCAEVEKIVADEKNNREKTALEKNKDKVKEACSKHLKVAAYCTTQVERNACLFCKARKLDDKFYQKLRGQFPDAVFWQEVGEIFRQLQKQAAEIYNQSLIELYYEIFIKGKGFANASSVEHYLSDVCYTRAAELFKNAAIASGLRGKVKSNFRLKELKNMKSGLPTTKSDNFPIPLVRQKGGQYTGFEISSHNSDFIIKIPFGRWQEKEEIGKYRPWEKFDFEQVRRSPKPISLLLSTQRRKKNKGWSKDEGTEAEIRRVMNGDYQTSYIEVKRGSKIGEKGAWMLNLSIDVPKIDKGVDPSIIGGIDVGVKSPLVCAINNALSRYSISDNDLFHFNKKMFARRRILLKKNGHKRAGHGARNKLKPIAVLTEKSKRFRKKLIERWACEIANFFIKNKVGTVQMENLESMKRKEDSYFNIRLRGLWPYAEMQNRIEFKLKQYGIEIRKVAPNNTSKTCSKCGHLNNYFNFEYRKRNKFPHFKCEECNFKENADYNAALNISNPKLKGTKEEP

SEQ ID NO: 3361 - protein, 726 aa, synthetic construct
SEVEFSHEYWMRHALTLAKRARDEREVPVGAILVLNNRVIGEGWNRAIGLHDPTAHAEIMALRQGGLVMQNYRLIDATLYVTFEPCVMCAGAMIHSRIGRVVFGVRNSKHGAAGSLVNVLNYPGMNHRVEITEGILADECAALLCDFYRMPRQVFNARKKARSSINPSGSSGGSSGSVTPGTSESATPESSGGGFGGSAKNTITKTLQLRIVRPYNSAEVEKIVADEKNNREKIALEKNKDKVKEACSKHLKVASYCTTQVERNACLFCKARKLDDKFYQKLRGQFPDAVFWQELGEIFRQLQKQAAEIYNQSLIELYYVIFIKGKGLANASSVEHYLSDVCYTRAAELFKNAAIASGLRGKVKSNFKLKELKSMKSGLPSTKSDNFPIPLVKQRGGQYTGFEISNHDGDFIIKIPFGRWQVKKEINKHRPWEKFDFEQVRKSPKPISLLLSTQRRKRNKGWSKDEGTEAEIRKVMNGDYQTSYIEVKRGGKIGEKSAWMLNLSIDVPKIDKGVDPRIIGGIDVGVKSPLVCAINNAFSRYSISDNDLFHFNKKMFARRRILLKKNSHKRAGHGAKNKLKPISILTEKSKRFRKKLIERWACEIADFFIKNKVGTVQMENLESMKRKEDSYFNIRLRGFWPYAEMQNKIEFKLRQYGIKIRKVAPNNTSKTCSKCGHLNNYFNFEYRKKNKFPHFKCEKCNFKEDADYNAALNISNPKLKSTKEEP

SEQ ID NO: 3362 - protein, 726 aa, synthetic construct
SEVEFSHEYWMRHALTLAKRARDEREVPVGAILVLNNRVIGEGWNRAIGLNDPTAHAEIMALRQGGLVMQNYRLIDATLYVTFEPCVMCAGAMIHSRIGRVVFGVRNNKHGAAGSLVNVLNYPGMNHRVEITEGILVDECAALLCDFYRMPRQVLNAQKKAQSSISSGGSSGGSSSSETPGASESATPKSSVGSSAGSTKNTITKTLKLRIVRPYNSAEVEKIVVDEKNNREKVALEKNKDKVKEACSEHLKVAAYCTTQVERSACLFCKARRLDDKFYQKLRGQFPDALFWQEIGEIFRQLQKQAAEIYNQSLIELYYEIFIKGKGITNASRVEHYLSDVCYTRAAELFKNAAIASGLRSKVRSNFRLKELKNMKSGLSTTKSDNFPIPLVKQKGGQYTGFEISSHNDDFIIKIPFGRWQAKKEIGKYRPWEKFDFEQVRKSPKPISLLLSTQRRKRNKGWSKDEGTEAEIRKVMNGDYQTSYIEVKRGSKIGEKSAWMLNLSIDVPKIDKGVDPSIIGGIDVGVKSPLVCAINNTIGRYSISDNDLFRFNKKMFARRRILLKKNRHKRAGHGAKNKLKPISILTEKSGRFRKKLIERWACEIADFFIKNKVGTVQMENLEGMKRKEDSYFNIRLRGFWPYAEMQNKIEFKLKQYGIKVRKVAPNNTSKTCSKCGHLNNYFSFEYRKKNKFPHFKCKKCNFKENADYNAALNISNPKLKSTKEEP

SEQ ID NO: 3363 - protein, 726 aa, synthetic construct
GEVEFSHEYWMRRALTLAKRARDEREVPVGAILVLNNRVIGEGWNRAIGLHDPTAHAEITALRQGGLVMQNYRLIDATLYVTFEPCVMCAGAMIHSRIGRVVFGVRNSKHGAAGSLVNVLNYPGMNHCVEITEGILVDECAALLCDFYRMPRQVLNAQKKAQSSISSGGSSGGSSGSETPGASGSVTPKSSGGSSAGSTKDTITKTLKLRIVRPYNSAEVEKVVADEKNNREKIAIEKNKDMVKEACSKHLKVASYCTTQVERNACLFCKARKLDDKFYQKLRGQFPDAVFWQELGGIFRQLQKQAAEIYNQSLIELYYEIFIKGKGITNASRVEHYLSDVCYTRAAELFKNAAIASGLRSKVRSNFRLKELKNMKSGLPTTKSDNFPIPLVKQKGGQYTGFEISSHNDDFIIKIPFGRWQVKKEIDKYRPWEKFDFEQVRKSPKPISLLLSTQRRKRNKGWSKDEGTEAEIRKVMNGDYQTSYIEVKRGRKIGEKSVWMLNLSIDVPKVDKGVDPSTTGGIDVGVKSPLVCAINNAFSRYSISDNDLFRFNKKMFARRRILLKKNRHKRAGHGAKNKLRPITILTEKSGRFRKKLIERWACEIADFFIKNKVGTVQMENLEGMKRKEDSYFNIRLRGFWPYAKMQSKIEFKLKQYGIEIRKVAPNNTSKTCSKCGHLNNYFSFEYRKKNKFPHFKCEKCNFKENADYNAALNISNPKLKSTKEEP

SEQ ID NO: 3364 - protein, 726 aa, synthetic construct
SEVEFSHEYWMRHALSLAKRARDEREVPVGAVLVLNNRVIGEGWNRAIGLHDPTAHAEIVALRQGGLVMQNYRLIDATLYVTFEPCVMCAGALVHSRIGRVVFGVRNSKRGAAGSLMNVLDYPGMGHRVEITEGILADECAALLCDFYCMPRQVFNAQKRAQSSTNPGGSSGGSSGSETPGTSESAAPESPGGSSGGSAKNTITKTLKLRIVRPYNSAEVEKIVADEKNNREKIAMEKNKDKVKEACSEHLKVAAYCTTQVERNACLFCKARKLDDKFYQKLRGQFPDAVFWQEIGEIFRQLQKQAAEIYNQSLVELYYEILIKGKGFANASSVEHYLSDVCYTRAAELFKNAAIASGLRGKVKSNFRLKELKNMKSGLPTTKSDNFPIPLVKQKGGQYTGFEISSHHDDLIIKIPFGRWQVKEEIDKYRPWEKFDFEQVRKSPKPISLLLSTQRRKKNKGWSKDEGTEAEIRRVMNGDYQTSYIEVKRGSKIGEKSAWMLNLSIDVPKIDKGVNPSIIGGIDVGVKSPLVCAINNSSSRYSICDNDLFRFNKKMFARRRILLKKNRHKRAGHGAKNKLKPITILTKKSERFRKKLIERWVCEVADFFIKNKVGTVQMENLESMKRKEDSYFNIRLRGFWPYAEMQNRIELKLKQYGIEIRRVAPNNTSRTCSKCGHLNNYFNFEFRKKNKFPHFKCEKCNFKEDADYNAALNISNPKLKSTKEEP

SEQ ID NO: 3365 - protein, 726 aa, synthetic construct
SEVEFSHEYWMRHALTLAKRARDEREVPVGAVLVLNNRVIGEGWNRAIGLHDPTAHAEIMALRQGGLVMQNYRLTDATLYVTFEPCVMCAGAMVHSRIGRVVFGVRNSKRGAAGSLMNVLNYPDMNHCVEITEGILVDECAALLCDFYRMPRQVLNAQKKAQSSISSGGSSGGSSGSETRGASESTTPESSGGSSGGPAKNTITKTLKLRIVRPYNSAEVEKIVADEKNNREKTALEKNKDKVKEACSKHLKMASYCTTQVERNACLFCKARKLDDKFYQKLRGQFPDAVFWQEIGEIFRQLQKQAAEIYNQSLIELYYEIFIKGKGFANASSVEHYLSGVCYTRAAELFKNAAIASGLRGKVRSNFRLKELKNMKSGLPTTKSDNFPIPLVKQKGGQYTGFEISSHNSDFIIKIPFGRWQMKEEIDKYRPWEKFDFEQVRKSPKPISLLLSTQRRKKNKGWSKDEGTEAEIRRVMNGDYQTSYIEVKRGSKIGEKSAWMLNLSIDVPKIDKGVDPSIIGGIDVGVKSPLVCAINNSSSRYSICDNDLFRFNKKMFARRRILLKKNRHKRAGHGAKNKLKPITILTKKSERFRKKLIERWVCEVADFFIKNKVGTVQMENLESMKRREDSYFNIRLRGFWPYAEMQNRIELKLKQYGIEIRRVAPNNTSRTCSKCGHLNNYFNFEYRKKSKFPHFKCEKCNFREDADYNAALNISNPKLKSTKEEP

SEQ ID NO: 3366 - protein, 726 aa, synthetic construct
SEVEFSHEYWMRHALTLAKRARDEREVPVGAILVLNNRVIGVGWNRAIGLHDPTAHAEIMALRQGGLVMQNYRLIDATLYVTFEPCVMCAGAMIHSRIGRVVFGVSNSKHGAAGSLVNVLNYPGMNHRVEVTEGILADECAALLCDFYRMPRQVFNARKKAQSSINSGGSSGGSSGSETPGTSESATPKSSGGSSGGSAKNTITKALKLRIVRPYNSAEVEKIVADEKDNRERIALEKNKDKVKEACSKHLKVASYCTTQVEGNACLFCKARKLDDKFYQKLRGQFPDAVFWQEIGEIFRQLQKQAAEIYNQGLIELYYEIFIKGKGTANASSVEHYLSDVCYTRAAELFKNAAIASGLRNKIKSNFRLKELKNMKSGLPTTKSDNFPIPLVKQKGGQYTGFEISDHNSDFIIKIPFGGWQVKKEINKYRPWEKFDFEQVRKSPKPISLLLSTQRRRRNKGWSKDEGTEAEIRKVMNGGYQTSYIEVKRGSKVGEKSAWMVNLSIDVPKIDKGVDPSIIGGIDVGVKSPLVCAVNNALSRYSIDDNDLFHFNKKMFARRRILLKKSRHKRAGHGAKNKLKPITILTEKSRRFRKKLIERWACEIADFFIKNKVGTVQMENLESMKRKEDSYFNIRLRGFWPYAEMQNKIEFKLKQYGIVVRKVAPNNTSKTCSKCGHLNNYFNFEYRKKNKFPHFKCEKCNFKEDADYNAALNISNPKLKSTKEEP

SEQ ID NO: 3367 - protein, 726 aa, synthetic construct
SEVEFSHEYWMRHALTLAKRARDEREVPVGAILVLNNRVIGVGWNRAIGLHDPTAHAEIMALRQGGLVMQNYRLIDATLYVTFEPCVMCAGAMIHSRIGRVVFGVRNSKHGAAGSLVNVLNYPGMNHRVEITEGILADECAALLCDFYRMPRQVFNARKKAQSSINSGGSSGGSSGSETPGTSESATPKSSGGSSGGSAKNTITKALKLRIVRPYNSAEVEKIVADEKNNRERIALEKNKDKVKEACSKHLKVAAYCTTQVERNACLFCKARKLDDMFYQKLRGQFPDAVFWQEIGEIFRQLQKQAAEIYNQSLIELYYEIFIKGKGFANASSVEHYLSDVCYTRAAELFKNAAIASGLRGKVKSNFRLKELKNMRSGLPTTKSDNFPIPLVKQKGGQYAGFEISSHNDDFIIKIPFGRWQVKKEIDKYRPWEKFDFEQVRKSPKPISLLLSTRRRKRNKGWSKDEGTEAEIRKVMNGDYQTSYIEVKRGSKIGEKSAWMLNLSIDVPKIDKGVDPSTIGGIDVGVKSPLVCAIDNAFSRYSISDNDLYHFNKKMFAKRRILLRKNRHKRAGHGAKNKLKPISILTEKSERFRKKLIERWACEIADFFIKNKVGTVQMENLESMKRKEDSYFNIRLRGFWPYAEMQNKIEFKLKQYGIEIRKVAPNNTSKTCSKCGHLNDYFNFEYRKRNKFPHFKCEKCNFKEDADYNAALNISNPKLKSTKEEP

SEQ ID NO: 3368 - protein, 726 aa, synthetic construct
SEVEFSHEYWMRHALTLAKRARDEREVPVGAVLVLNNRVIGEGWNRAIGLHDPTAHAEIMALRQGGLVMQNYRLIDATLYVTFEPCVMCAGAMVHSRIGRVVFGVRNSKRGAAGSLMNVLNHPGMNHRVEITGGILADECAALLCDFYRMPRQVFNAQKKARSNINSGGSSGGSSGSETLGTSESVTPESSGGSSGGSAKNTITKTLKLRIVRPYNSTEVEKIVVDEKNNREKVALEKNKDKVKEACSEHLKVAAYCTTQVERSACLFCKARKLDDKFYQKLRGQFPDAVFWQEISEIFRQLQKQAAEIYNQSLIELYYEIFIKGKGFANASSVEHYLSDVCYTRAAELFKNAAIASGLRGKVKGNFRLKELKNMKSGLPTTKSDNFPIPLVKQKGGQYTGFEISSHNDDFIIKIPFGRWQAKKEIDKYRPWEKFDFEQVRKSPKPISLLLSTQRRKRNRGWSEDEGTEAEIRKVMNGDYQTSYIEVKRGSKIGEKSAWMLNLSIDVPKIDKGVDPSIIGGIDVGVKSPLVCAINNAFSRYSVSDNDLFRFNKKMFARRRILLKKNRRRRVGHGAKNKLKPITILTEKSVRFRKKLIERWACEIADFFIKNKVGTVQMENLESMKRKEDSYFNIRLRGFWPYAEMQNKIEFKLKQYGIKIRKVAPNNTSKTCSKCGHLNNYFNFEYRKKNKFPHFKCEKCNFREDADYNAALNISNPKLKSTEEEP

SEQ ID NO: 3369 - protein, 726 aa, synthetic construct
SEVEFSHEYWMRHALTLAKRARDEREVPVGAVLVLNNRVIGEGWNRAIGLRDPTAHAEIMALRQGGLVMQNYRLIDATLYVTFEPCVMCAGAMIHSRIGRVVFGVRNNKHGAAGSLVNVLNYPGMNHRVEITEGILANECAALLCDFYRMPRQVFNARKKAQSSINPGGSSGGSSGSETPGTSESTTPESSGGSSGGSAKNTITKTLKLRIVRPYNSAEVEKIVADEKNNRERIALEKNKDKVKEACSKHLKVAAYCTTQVERNACLFCKARKLDDKFYQKLRGQFPDAVFWQETGEIFRQLQKQAAEIYNQSLIELYYEIFIKGKGFANASSVEHYLSDVCYTRVAELFKNAAIASGLRGKVKSNFRLKELKNMKSGLPTTKSDNFPIPLVKQKGGQYTGFEISSHNDDFIIKIPFGRWQAKKEIDKYRPWEKFDFEQVRKSPKPISLLLSTQRRKRNRGWSKDEGTEAEIRKVMNGDYQTSYIEVKRGSKIGEKSAWMLNLSIDVPKIDKGVDPSIIGGIDVGVKSPLVCAINNAFSRYSISDNDLFRFNKKMFARRRILLGKNRHKRAGHGVKNKLKPITILTEKSGRFRKKLIERWACEIADFFVKNKVGTVQMENLESMKRKEDSYFNIRLRGFWPYAEMQNRIEFKLKQYGIEIRKVAPNNTSKTCSKCGHLNNYFNFEYRKKNKFPHFKCEKCNFKENADYNAALNISNPKLKSTKEEP

SEQ ID NO: 3370 - protein, 726 aa, synthetic construct
SEVEFSHEYWMRRALTLAKRARDEREVPVGAVLVLNNRVIGVGWNRAAGLHDPTAHAEIMALRQGGLVMQNYRLVEATLYVTFEPCIMCAGAMIHSRIGRVVFGVRNSKRGAAGSLMNVLNYPGMNHRVEITEGILADECAALLCDYYRMPRQVFNARKKAQSSINSGGSSDGGSGSETPGTSESATPESSGGSSGGSAKNTITKTLKLRIVRPYNSAEVEKIVADEKNDREKIALEKNKDKVKEACSEHLKVAAYCTTQVERSACLFCKARKLDDKFYQKLRGQFPDAVFWQEIGEIFRQLQKQAAEIYNQSLIELYYEIFIKGKGFANASSVEHYLSDVCYTRAAELFKNAAIASGLRGKVKSNFRLKELKNMKSGLPTTKSDNFPIPLVKQKGGQYTGFGISSHNSDFVIKIPFGRWQVKEEIDKYRPWEKFDFEQVRKSPKPISLLLSTQRRKKNKGWSKDEGTEAEIRKVMNGDYQTSYIEVKRGSKIGEKSAWVLNLSIDVPKIDRGVDPSIIGGIDVGVKSPLVCAINNSFSRYSICDNDLFRFNKKMFARRRILLKKNRHKRAGHGAKNKLKPITILTKKSERFRKKLIERWVCEVADFFVKNKVGTVQMENLESMKRKEDSYFNIRLRGFWPYAEMQDKIEFKLKQYGIKVRKVAPNNTSKTCSKCGHLNNYFSFEHRKKNKFPHFKCEKCNFKENADYNAALNISNPKLKSTKEEP

SEQ ID NO: 3371 - protein, 726 aa, synthetic construct
SEDEFSHEYWMRHALTLAKRARDGREVPVGAVLVLNNRVIGEGWNRAIGLHDPTAHAEIMALRQGGLVMQNYRLIDATLYVTFEPCVMCAGAMVHSRIGRVVFGVRNSKRGAAGSLMNVLDYPGMGHRVEITEGILADECAALLCDFYRMPRQVLNAQKKAQSSISSGGSSGGSSCSETPGASESVTPKSSVGSSAGSTKNTITKTLKLRIVRPYNSAEVEKIVADEKNNREKIALEKNKDKVKEACSKHLKVASYCTTQVERNACLFCKARKLDDKFYQKLRGQFPDAVFWQELGGIFRQLQKQAAEIYNQSLIELYYEIFIKGRGFANASNVEHYLSDVCYTRAAELFKNAAIASGLRGKVKGNFRLKELKSMKSGLPTTKSDNFSIPLVKQKGGQYTGFEISSHNDDFIIKIPFGRWQAKKEIDKYRPWEKFDFEQVRKSPKPISLLLSTQRRRRNKGWSEDEGTEAEIRKVMNGDYQTSYIEVKRGSKIGEKSAWMLNLSIDVPKIDKGVDPSIIGGIDVGVKSPLVCAINNALSRYSISDNDLFHFNKKMFARRRILLKKNRHRRAGHGARNKLKPIIVLTEKSERFRKKLIERWACEIANFFIKNKVGTVQMENLESMKRREDSYFNIRLRGLWPYAEMQNKIEFKLKQYGIEIRKVAPYNTSKTCSKCGHLNNYFNFEYRKKNKFPYFKCEKCNFKENADYNAALNISNPKLKSTKEEP

SEQ ID NO: 3372 - protein, 726 aa, synthetic construct
SEVEFSHEYWMRHALTLARRARDGREVPVGAVLVLNNRVIGEGWNRAIGLHDPTAHAEIMALRQGGLVMQNYRLIDATLYVTFEPCVMCAGAMVHSRIGRVVFGVRNSKRGAAGSLMNVLDYPGMDHRVEITEGILADECAALLCDFYRMPRQVFNAQKKAQSSINSGGSSGGSSGSETPSTSESATPESSGGSSGGSAKNTITKTLQLRIVRPYNSAEVEKIVTDEKNNREKIALEKNKDKVKEACSKHLKMASYCTTQVERNACLFCKARKLDDKFYQKLRGQFPDAVFWQELGEIFRQLQKQAAEIYNQSLIELYYKIFIKGKGLANASNVEHYLSDVCYTRAAELFKNAAIASGLRGKVKSNFRLKELKNMKSGLPTTKSDNFPIPLVRQKGGQYTGFEISNHDGDFIIKIPFGRWRVKKEINKHRPWEKFDFEQVRKSPKPISLLLSTQRRKRNKGWSKDEGTEAEIRKVMNGDYQTSYIEVKRGSKIGEKSAWMLNLSIDVPKIDKGVDPGIIGGIDVGVKSPLVCAINSASSRYSISDNDLFHFNKKMFARRRILLKKNGHKRAGHGAKNKLKPITIMTEKSKRFRKKLIERWACEIADFFIKNKVGTVQMENLESMKRREDSYFNIRLRGFWPYAEMQNKIEFKLKQYGIEIRKVAPNNTSKTCSKCGHLNNYFNFEYRKKNKFPHFKCEKCSFKENADYNAALNISNPKLKNTKEEP

SEQ ID NO: 3373 - protein, 726 aa, synthetic construct
SEDEFSHEYWMRHALTLAKRARDEREVPVGAVLVLNNRVIGEGWNRTTGLHDPTAHAEIMALRQGGLVMRNYRLTDATLYVTFEPCVMCAGAMIHSRIGRVVFGVRNSKRGAAGSLMNVLNYPGMNHCVEITEGILVDECAALLCDFYRMPRQVLNAQKKAQSSISPGGSSGGSSGSETPGASESVTPKSSGGSSGGSAKNTITKTLKLRIVRPYNSAEVERIVADEKNNREKIALEKNKDKVKEACSKHLKVAAYCTTQVERNACLFCKARRLDDKFYQKLRGQFPDAVFWQEIGEIFRQLQKQAAEVYNQSLVELYYEILIKGKGIANASSVEHYLSDVCYTRAAELFKNAAIASGLRNKIKSNFRLKELRNMKSGLPTTKSDNFPIPLVRQKGGQYTGFEISSHNDDFIIKIPFGRWQVKKEIDKYRPWERFNFEQVRKSPKPISLLLSTQRRKRNKGWSKDEGTEAEIRKVMNGDYQTSYVEVKKGSKIGEKSAWMLSLSIDVPKIDRGVDPCIIGGIDVGVKSPLVCAINNAFSRYSISDNDLFRFNKKMFARRRILLKKNRHKRAGHGARNKLKPITILTEKSGRFRKKLIERWACEIADFFIKNKVGTVQMENLEGMKRKEDSYFNIRLRGFWPYAEMQNKIEFKLKQYGIGIRRVAPNNTSRTCSKCGHLNNYFNFEYRKRSKFPHFKCEKCNFREDADYNAALNISNPKLKSTKEEP

SEQ ID NO: 3374 - protein, 726 aa, synthetic construct
SEVEFSHEYWMRRALTLAKRARDEREVPVGAVLVLNNRVIGVGWNRAVGLHDPTAHAEIMALRQGGLVMQNYRLIEATLYVTFEPCIMCAGAMIHSRIGRVVFGVRNSKRGAAGSLMNVLNYPGMNHRVEITEGILANECAALLCDFYRMPRQVFNARKKAQSSINPGGSSGGSSGSETPGTSESATPESSGGSSGGSAKNTITKALKLRIVRPYNSAEVEKIVADEKSNREKIALEKNKDKVKEACSKHLKMASYCTTQVERNACLFCKARKLDDKFYQKLRGQFPDAVFWQEIGEIFRQLQKQAAEIYNRSLIELYYEIFIKGKGFANASSVEHYLSDVCYTRAAELFKNAAIASGLRGKVKSNFRLKELKNMKSGLPTTKSDNFSIPLVKQKGGQYTGFEISSHNDDFIIKIPFGRWQVKKEIDKYRPWEKFDFEQVRKSPKPISLLLSTQRRKRNKGWSKDEGTEAEIRKVMNGDYQTSYIEVKRGSKIGEKSAWVLNLSIDVPKIDKGVDPSIIGGIDVGVKSPLVCAINNAFSRYSISDNDLFHFNKKMFARRRILLKKNRHKRAGHGAKNKLKPISILTERSKRFRKKLIERWACEIADFFIKNKVGTVQMENLESMKRKEDSYFNIRLRGFWPYAEMQNKIVFKLKQYGIEIRKVAPNNTSKTCSKCGHLNNYFNFEYRKMNKFPHFKCEWCNFKENADYNAALNISNPKLKSTKEEP

SEQ ID NO: 3375 - protein, 726 aa, synthetic construct
SEVEFSHEYWMRHALTLAKRARDEREVPVGAVLVLNNRVIGEGWNRAIGLHDPTAHAEIMALRQGGLVLQNYRLVDATLYVTFEPCVLCAGAMVHSRIGRVVFGVRNSKRGAAGSLMNVLDYPGMGHRVEITEGILADECAALLCDFYCMPRQVFNAQKRAQSSINSGGSSGGSSGSETPGTSESATPESSGGGSSGSAKNTITKTLQLRIVRPYNSAEVEKIVADEKNYREKIALEENKDKVKEACSEHLKVAAYCTTQVERSACLFCKARKLDDRFYQKLRGQFPDAVFWQEISEIFRQLQKQAAEIYNQSLIELYYEILIKGKGIANASRVEHYLSDVCYTRAAELFKNAAIASGLRGKVKGNFRPKELKNMKSGLPTTKSDNFPIPLVKQKGGQYTGFEISSHNDDFIIKIPFGRWQVKKEIDRYRPWEKFDFEQVRKSPKPISLLLSTQRRKRNKGWSKDEGTEAEIRKVMNGDYQTSYIEVKRGSKTGEKSAWMLNLSIDVPKIDKGVDPSIIGGIDVGVKSPLVCAINNAFSRYSISDNDLFRFNKKMFARRRILLKKNRRRRAGHGAKNKLKPITILTEKSVRFRKKLIERWACEIADFFIKNKVGTVQMENLESMKRKEDSYFNIRLRGFWPYAEMQNKIEFKLKQYGIEIRRVAPNNTSRTCSKCGHLNNYFNFEYRRKYKFPHFKCEKCNFKEDADYNAALNISNPKLKSTKEEP

SEQ ID NO: 3376 - protein, 726 aa, synthetic construct
SEVEFSHEYWMRHALTLAKRARDEREVPVGAVLVLNNRVIGEGWNRAIGLHDPTAHAEIMALRQGGLVMQNYRLIDATLYVTFEPCVMCAGAMVHSRIGRVVFGVRNSKRGAAGSLMNVLDYPGMDHRVEITEGILADECAALLCDFYRMPRQVLNAQKKAQSSISSGGSSGGSSCSETPGASESVTPKSSGGSSGGSAKNTITKTLQLRIVRPYNSAEVEKIVADEKNNREKIALEKNKDKVKEACSKHLKVASYCTTQVERNACPFCKARKLDDKFYQKLRGQFPDAVFWQELGEILRQLQKQAAEIYNQSLIELYYEIFIKGRGFANASSVEHYLSDVCYTRAAELFKNAAIASGLRGKVKSNFRLKELKNMKSGLPTTKSDNFPIPLVKQKGGQYTGFEISSHNDDFIIKIPFGRWQVKKEIDKYRPWEKFDFEQVRKSPKPISLLLSTQRRKRNKGWSKDEGTEAEIRKVMNGDYQTSYIEVKRGSKIGEKSAWMLNLSIDVPKIDKGVDPSIIGGIDVGVKSPLVCAINNAFSRYSISDNDLYRFNKKMFARRRILLKKNRHKRADHGAKNKLKPISILTERSRRFRKKLIERWACEIADFFIRNKVGTVQMENLESMKRKEDSYFNIRLRGFWPYAEMQNKIEFKLKQYGIEIRKVAPNNTSKTCSKCGHLNNYFNFEYRKRNKFPHFKCEKCNFKEDADYNAALNISNPKLKGTKKEP

SEQ ID NO: 3377 - protein, 726 aa, synthetic construct
SEVEFSHEYWMRHALTLAKRARDEREVPVGAILVLNNRVIGEGWNRAIGLHDPTAHAEIMALRQGGLVMQNYRLIDATLYVTFEPCVMCAGAMIHSRIGRVVFGVRNNKHGAAGSLVNVLNYPGMNHCVGITEGILVDECAALLCDFYHMPPQVLNARKKAQSSISSGGSSGGSNGSETPGASESATPESSGGSSGGSAKNTITKTLKLRIVRPYNNAEVEKIVADEKNNREKVALEKNKDKVKEACSKHLKVAAYCTTQVERNACLFCKARRLDDKFYQKLRGQFPDAVFWQEIGEIFRQLQKQAAETYNQSLIELYYEIFIKGKGIANASNVEHYLSDVCYTRAAELFKNAAIASGLRNKIKSNFRLKELRNMKSGLPTTKSDNFPIPLVKQKGGQYTGFEISNHNNDFIIKIPFGRWQAKKEVDRYRPWEKFDFEQVRKSPKPISLLLSTQRRKRNRGWSKDEGTEAEIKKVMNGDYQTSYIEVKRGSKIGEKSAWMLNLSIDVPKIDKGVDPSIIGGIDVGVKSPLVCAINNAFSRYSISDNDLFRFNKKMFARRRILLKKSKHKRAGHGTKNKLKPITTLTEKSERFRKKLIERWACEIADFFIKNKVGTVQMEDLESMKRREDSYFNIRLRGFWPYAKMQNKIEFKLKQYGIEIRKVAPNNTSKTCSKCGHLNNYFNFEYRKKNKFPHFKCEKCNFKESADYNAALNISNPKLKSTKEEP

SEQ ID NO: 3378 - protein, 726 aa, synthetic construct
SEVEFSHEYWMRHALTLAKRARDEREVPVGAILVLNNRVIGEGWNRAIGLHDPTAHAEIMALRQGGLVMQNYRLIDATLYVTFEPCVMCAGAMIHSRIGRVVFGVRNNKHGAAGSLVNVLNYPGMNHRVEITEGILVDECAALLCDFYRMPRQVLSAQKKAQSSVSSGGSSGGSSGSETPGASGSVTPKSSVGGSAGSTKNTITKALQLRIVRPYNSAEVEKIVADEKNNREKIALEKNKDKVREACSKHLKVASYCTTQVERNACPFCKARKLDDKFYQKLRGQFPDAVFWQELGEILRQLQKQAAEIYNQSLIELYYEIFIKGRGFANASSVEHYLSDVCYTRAAELFKNAAIASGLRGKVKSNFRLKELKNMKSGLPTTKSDNFPIPLVKQKGGQYTGFEISSHNDDFIIKIPFGRWQVKKEIDKYRPWEKFDFEQVRKSPKPISLLLSTQRRKRNKGWSKDEGTEAEVRKVMNGDYRTSYIEVRRGSKTGEKSAWMLNLSIDVPKIDKGVDPSIIGGIDVGVKSPLVCAINNAFSRYSISDNDLFRFNKKMFARRRILLKKNRHKRAGHGAKNKLKPISILTEKSKRFRKKLIERWACEIADFFIKNKVGTVQMENLESMKRKEDGYFNIRLRGFWPYAEMQNKIEFKLKQYGIETRKVAPNNTSKTCSKCGHLNNYFNFEYRKTNKFPHFKCEKCNFKEDADYNAALNIGNPKLKSTKEEP

SEQ ID NO: 3379 - protein, 726 aa, synthetic construct
SEVEFSHEYWMRHALTLAKRARDEREVPVGAVLVLNNRVIGEGWNRAIGLHDPTAHAEIMALRQGGLVLQNYRLVDATLYVTFEPCVLCAGAMVHSRIGRVVFGARNSKRGAAGSLMNILNYPGMNHRVEITEGILADECAALLCDFYRMPRQVFNAQKRAQSSINSGGSSGGSSGSETPGASESVTPKSSGGSSGGSAKNTITKTLKLRIVRPYNSAEVEKIVADEKNNREKIALEKNKGKVKEACSKHLEVAAYCTTQVERNACLFCKARKLDDKFYQKLRGQFPDAVFWQELGEIFRQLQKQAAEIYNQSLIELYYEIFIKGKGFANASSVEHYLSDVCYTRAAELFKNAAIASGLRGKVKSNFRLKELKNMKSGLPTTKSDNFPIPLVKQKGGQYTGFEISSHNDNFIIKIPFGRWQVRKEIDKYRPWEKFNFEQVRKSPKPISLLLSTQRRKRNKGWSEDEGTEAEIRKVMNGDYQTSYIEVKRGSKIGEKSAWMLSLSIDVPKIDKGVDPSIIGGIDVGVKSPLVCAINNAFNRYSISDNNLFRFNKKMFARRRILLKKNRHKRAGHGAKNKLKPISILTGKSERFRKKLIERWACEIADFFIKNKVGTVQMENLESMKRKEDSYFNIRLRGFWPYAEMQNKIEFKLKQYGIEIRKVAPNNTSKTCSKCGHLNNYFNFEYRKKNKFPHFKCERCNFKENADYNAALNISNPKLKSTKEEP

SEQ ID NO: 3380 - protein, 725 aa, synthetic construct
SEVEFSHEYWMRHALTLAKRARDEREVPVGAILVLNNRVIGEGWNRAIGLHDPTAHAEIMALRQGGLVMQNYRLIDATLYVTFEPCVMCAGAMIHSRIGRVVFGVRNNKHGAAGSLVNVLNYPGMNHRVEITEGILADECAALLCDFYRMPRQVFNARKKARSNINSGGSSGGSSGSETPGTSESAAPESSGGSSGGSTRNTITKTLKLRIVRPYNSAEVEKIVADEKNNREIALEKNKDKVKEACSKHLKVAAYCTTQVERNACLFCRARRLDDKFYQKLRGQFPDAVFWQEIGEIFRQLQKQAAEIYNQSLVELYYEIFIKGKGIANASSVEHYLSDVCYTRAAELFKNAAIASGLRNKVKSNFRLKELRNMKSGLPTTKSDNFPIPLVKQKGGQYTGFEVSSHNDDFIIKIPFGRWQVKKEIDKYRPWEKFDFEQVRKSPRPTSLLLSTQRRKRNKGWSKDEGTEAEIRKVMNGDYQTSYIEVKRGSKIGEKSAWMLNLSIDVPKIDKGVDPSIIGGIDVGVKSPLVCAIDNAFSRYSISDNDLFHFNKKMFAKRRILLKKNRHKRAGHGAKNKLKPISILTEKSERFRKKLIERWACEIADFFIKNKVGTVQMENLESMRRREDSYFNTRLRGFWPYAEMQNKIEFKLKQYGIEIRKVAPNNTSKTCSKCGHLNNYFNFEYRRKNKFPHFKCEKCNFKENADYNAALNISNPKLKSTKGEP

SEQ ID NO: 3381 - protein, 726 aa, synthetic construct
SEVEFSHEYWMRHALTLAKRARDEREVPVGAILVLNNRVIGEGWNRAIGLHDPTAHAEIMALRQGGLVMQNYRLTDATLYVTFEPCVMCAGAMVHSRIGRVVFGVRNSKRGAAGSLMNVLNYPGMNHRVEITEGILVDECAALLCDFYRMPRQVFNAQKKAQSTINSGGSSGSSSGSETPGTSESPTPESSGGSPGGSAKNTITKTLKLRIVRPYNSAEVEKIVADEKNNREKIALEKNKDKVKEACSKHLKVAAYCTTQVERNACLFCKARKLDDKFYQKLRGQFPDAVFWQETGEIFRQLQRQAAEIYNQSLIELYYEVFIKGKGFANASSVEHYLSDVCYTRAAELFKNAAIASGLRSKIKSNFRLKELKNMKSGLPTTKSDNFPIPLVKQKGGQCTGFEISNHNSDFIIKIPFGRWQVKKEIDKYRPWEKFDFEQVRKSPKPISLLLSTQRRRRNKGWSKDEGTEAEIRKVMNGDYQASYIEVKRGSKIGEKSAWMLNLSIDVPKIDKGVDPNIIGGIDVGVKSPLVCAINNAFSRYSISDNDLFRFNKKMFARRRILLRKNRHKRAGHGAKNKLKPISILTGKSERFRKKLIERWACEIADFFIKNKVGTVQMENLESMKRKEDSYFNIRLRGFWPYAEMQNKIEFKLKQYGIEIRKVAPNNTSKTCSKCGHLNNYFNFEYRKKNKFPHFKCEKCNFKENADYNAALNISNPKLKSTKEEP

SEQ ID NO: 3382 - protein, 726 aa, synthetic construct
SGVEFSHEYWMRHALTLAKRARDEREVPVGAVLVLNNRVIGEGWNRAVGLHDPTAHAEIMALRQGGLVMQNYRLIDATLYVTFEPCVMCAGAMIHSRIGRVVFGVRNNKHGAAGSLVNVLNYPGMNHRVEITEGILADECAALLCDFYRMPRRVFNAQKKAQSSINSGGSSGGSSGSETPGASGSVIPKSSGGSSAGSTKDTITKTLKLRIVRPYNSAEVEKVVADEKNNREKIAMEKNKDKVKEACSKHLKVASYCTTQVERNACLFCKARKLDDKFYQKLRGQFPDAVFWQELGGIFRQLQKQAAEIYNQSLIELYYEIFIKGKGITNASRVEHYLSDVCYTRAAELFKNAAIASGLRSKIKSNFRLKELKSMKSGLPTTKSDNFPIPLVKQKGGQYTGFEISSHNSDFIIKIPFGRWQEKEEIDKYRPWEKFDFEQVRRSPKPISLLLSTQRRKKNKGWSKDEGTEAEIRRVMNGDYQTSYIEVKRGSKIGGKSAWMLNLSIDVPKIDKGVDPSIIGSIDVGVKSPLVCAINNSFSRYSICDNDLFRFNKKMFARRRIMLKKNRHKRAGHGAKSKLKPITILTKKSERFRKKLIERWACEVADFFTKNKVGAVQMENLESMKRKEDSYFNIRLRGFWPYAEMQDRIEFKLKQYGIEIRRVAPNNTSRTCSKCGHLNNYFNFEYRKKNKFPHFKCEKCNFREDADYNAALNISNPKLKSTKEEP

SEQ ID NO: 3383 - protein, 726 aa, synthetic construct
SEVEFSHEYWMRHALTLAKRARDEREVPVGAVLVLNNRVIGGGWNRAIGLHDPTAHAEIMALRQGGLVMQSCRLVDATLYVTFEPCVMCAGAMIHGRIGRVVFGVRNSKRGAAGSLMNVLNYPGMNHRVEITEGILAGECAALLCDFYRMPRQVFNAQKKAQSTINSGGSSGGSSSSETPGTSGSATPESSGGSSGGSAKNTITKTLKLRIVRPYNSAEVEKIVADEKNNREKIALEKNKDKVKEACSEHLKVAAYCTTQVGRNACLFCKARKLDDKFYQKLRGQFPDAVFWQEIGEIFRQLQKQAAKIYNQSLVELYYEILIKGKGIANASSVEHYLSDVCYTRAAELFKNAAIASGLRNKVKSNFRLKELRNMKSGLPTTKSDNFPIPLVRQKGGQYTGFEISNHNGDFIIKIPFGRWQVKKEINKHRPWEKFDFEQVRKSPKPISLLLSTQRRKGNKGWSKDEGTEAEIRRVMNGDYQTSYIEVKRGSKTGEKSAWMLNLSIDVPKIDKGVDPSVIGGIDVGVKSPLVCAINNAFSRFSISDNDLFHFNKKMFARRRILLKKNGRKRAGHGAKNKLKPITILTEKSKRFRKKLIERWACEIAGFFIKNKVGTVQMENLESMKRKEDSYFNIRLRGFWPYAEMQNKIEFKLKQYGIEIRKVAPNNTSKTCSKCGHLNNYFNFEYRKKNKFPHFKCEKCNFKENADYNAALNICNPKLKSTREEP

SEQ ID NO: 3384 - protein, 726 aa, synthetic construct
SEVEFSHEYWMRHALTLAKRARDEREVPVGAILVLNNRVIGEGWNRAIGLHDPTAHAEIMALRQGGLVMQNYRLIDATLYVTFEPCVMCAGAMVHSRIGRVVFGVRNSKRGAAGSLMNVLDYPGMGHRVEITEGILADECAGLLCDFYCMPRQVFNAQKRAQSSINSGGSSGGSSGGDTPGTSESATPESSGGGSSGSAKNTTTKTLQLRIVRPYNSAEVEKIVADEKNNREKIALEKNKDKVREACSKHLKVASYCTTQVERNACPFCKARKLDDKFYQKLRGQFPDAVFWQELGEILRQLQKQAAEIYNRSLIELYYEIFIKGRCFANASSVEHYLSDVCYTRAAELFKNAAIASGLRNKVKSNFRLKELKNMKSGLPTTKSDNFPIPLVKQKGGKYTGFEISSHNDDFIIKIPFGRWQVKKEIDKYRPWEKFDFEQVRKSPKPISLLLSTQRRKRNKGWSKDEGTEAEIRKVMNGDYQTSYIEVKRGSKIGEKSAWMLNLSIDVPKIDKGVDPNIIGGIDVGVKSPLVCAINNAFSRYSISDNDLFHFNKKMFARRRILLKKNRHKRAGHGAKNKLKPISILTGKSKRFRKKLIEKWACEIADFFIKNKVGTVQMENLESMKRKEDSYFNIRLRGFWPYAEMQNKIEFKLKQYGIEIRKVAPNNTSKTCSKCGHLNNYFNFEYRKKNKFPHFKCEKCSFKENADYNAALNISNPKLKSTKEEP

SEQ ID NO: 3385 - protein, 726 aa, synthetic construct
SEVEFSHEYWMRHALILAKRARDEREVPVGAVLVLNNRVIGVGWNRAVGLHDPTAHAEIMALRQGGLVMQNYRLIEATLYVTFEPCIMCAGAMIHSRIGRVVFGVRNSKRGAAGSLMNVLNYPGMDHCVEITEGILVDECAALLCDFYRMPPQVLNAQKKAQSSISSGGSSGGSSGSETPGASGSVTPKSSGGSSAGSTKDAITKTLKLRIVRPYNSAEVEKIVADEKNNREKIALEKNKGKVKEACSKHLEVAAYCTTQVERNACLFCKARKLDDKFYQKLRGQFPDAVFWQELGEIFRQLQKQAAEIYNQSLIELYYEIFIKGKGFANASSVEHYLSDVCYTRAAELFKNAAIASGLRGKVKSNFKLKELKSMKSGLPSTKSDNFPIPLVRQKGGQYTGFEISNHNGDFIIKIPFGRWQVKKEINKHRPWEKFDFEQVRKSPKPISLLLSTQRRRRNKGWSKDEGTEAEIRKVMNGDYQTSYIEVKRGNKIGEKSAWMLNLSIDVPKIDKGVDPSIIGGIDVGVKSPLVCAINNAFSRYSISDNDLFHFNKKMFARRRILLKKNRHRRAGHGAKNKLKPIAVLAEKSEGFRKKLIERWACEVADFFIKNKVGTVQMENLESMKRREDSYFNIRLRGFWPYAEMQNKIEFKLKQYGIKIRKVAPNNTSRTCSKCGHLNNYFSFEYRKKNKFPHFKCEKCNFKEDADYNAALNISNPKLKSTKEEP

SEQ ID NO: 3386 - protein, 726 aa, synthetic construct
SEVEFSHEYWMRHALTLAKRARDEREVPVGAVLVLNNRVIGEGWNRAIGLHDPTAHAEIMALRQGGLVMQNYRLVDATLYVTFEPCVLCAGAMVHSRIGRVVFGVRNSKRGAAGSLMNVLNYPGMNHRVEITEGILVDECAALLCDFYRMPRQVLNAQKKAQSSISSGGSSGGSSGSETPGASGSVIPKSSGGSSAGSTKDTITKTLKLRIVRPYNSAEVEKVVADEKNNREKIAMEKNKDKVKEACSKHLKVAAYCTTQVERSACLFCKARKLDDKFYQKLRGQFPDAVFWQEIGEIFRQLQKQAAEIYNQSLIELYYEVFIKGRGFANASSVEHYLSDVCYTRAAELFKNAAIASGLRGKVKSNFRLKELKNMKSGLPTTKSDNFPIPLVKQKGGQYTGFEISSHNDDFIIKIPFGRWQVKKEIDKYRPWEKFDFEQVRKSPKPISLLLSTQRRKRNKGWSKDEGTEAEIRKVMNGDYQTSYIEVKRGSKTGEKSAWMLNLSIDVPKIDKGVDPSIIGGVDVGVKSPLVCAINNAFSRYSISDNDLFHFNKKMFARRRILLKKTRHKRAGHGAKNKLKPISILTEKSERFRKKLIERWACEIADFFIKNKVGTVQMENLESMKRREDSYFNIRLRGFWPYAEMQNKIEFRLKQYGIEIRKVAPNNTSKTCSKCGHLNNYFNFEYRRMNKFPHFKCEKCNFKENADYNAALNISNPKLKSTKGEP

SEQ ID NO: 3387 - protein, 726 aa, synthetic construct
SEVEFSHEYWMRHALILAKRARDEREVPVGAVLVLNNRVIGVGWNRAIGLHDPTAHAEIMALRQGGLVMRNYRLIDATLYVTFEPCVMCAGAMVHSRIGRVVFGVRNSKRGAAGSLMNVLDYPGMGHRVEITEGILADECAALLCDFYCMPRQVFNARKKAQSSINSGGSSGGSSGSETPGTSESATPESSGGGSSGSAKNTITKTLKLRIVRPYNSAEVEKIVADEKNNREKIALEKNKDKVREACSEHLKVAAYCTTQVERNACLFCKARKLDDKFYQKLRGQFPDAMFWQEIGEIFRQLQKQAAEIYNQSLIELYYEIFIKGKGFANASSAEHYLSDVCYTRAAELFKNAAIASGLRGKVKSNFRLKELKNMKSGLPTTKSDNFPIPLVKQKGGKYTGFEISSHNDDFIIKIPFGRWQVKKEIDKYKPWEKFDFEQVRKSPKPISLLLSTQRRKRNKGWSKDEGTEAEIRKVMNGDYQTSYIEVKRGSKIGEKSAWMLNLSIDVPKIDKGVDPSIIGGIDVGVKSPLVCAINNAFSRYSISDNDLFHFNKKMFARRRILLKKNRHKRAGHGAKNKLKPITILTKKSERFRKKLIERWVCEVADFFIKNKVGTVQMENLESMKRKEDSYFNIRLRGFWPYAEMQNRIELKLKQYGIEIRRVAPNNTSRTCSKCGHLNNYFNFEYRKKNKFPPFKCEKCNFREDADYNAALNISNPKLKSTKKEP

SEQ ID NO: 3388 - protein, 726 aa, synthetic construct
SEVESSHEYWMRHALTLAKRARDEREVPVGAVLVLNNRVIGEGWNRAIGLHDPTAHAEIMALRQGGLVMQNYRLVDATLYVTFEPCVLCAGAMVHSRIGRVVFGVRNSKRGAAGSLMNVLNYPGMNHRVEITEGILADECAALMCDFYRMPRQVFNARKKAQSSTNPGGSSGGSSGSETPGTSESATPESPGGSSGGSAKNTITKTLKLRIVRPYNSAEVEKIVADEKNNREKIALEKNKDKVKEACSKHLKVAAYCTTQVERNACLFCKARRLDDKFYQKLRGQFPDAVFWQEIGEIFRQLQKQAAEVYNQSLVELYYEILIKGKGIANASSVEHYLSDVCYTRAAELFKNAAIASGLRNKIKSNFRLRELRNMKSGLPTTKSDNFPIPLVRQKGGQYTGFEISNHDGDFIIKIPFGRWQVKKEINKHRPWEKFDFEQVRKSPKPISLLLSTQRRKRNKGWSKDEGTEAEIRKVMNGDYQTSYIEVKRGSKVGEKSAWMLNLSIDVPKIDKGVDPSIIGGIDVGVKSPLVCAINNAFSRYSISDNDLFHFNKKMFARRRILLKKTRHKRAGHGAKNKLKPISILTEKSVRFRKKLIERWACEIADFFIKNKVGTVQMENLESMKRKEDSYFNIRLRGFWPYAEMQNKIEFKLKQYGIEIRKVAPNNTSKTCSKCGHLNNYFNFEYRKKNKFPHFKCEKCSFKENADYNAALNISNPKLKSTKEEP

SEQ ID NO: 3389 - protein, 725 aa, synthetic construct
SEVEFSHEYWMRHALTLAKRARDEREVPVGAVLVLNNRVIGEGWNRAIGLHDPTAHAEIMALRQGGLVMQNYRLTDAILYVTFEPCVMCAGAMVHSRIGRVVFGVRNSKRGAAGSLMNVLNYPDMNHYVEITEGILVDECAALLCDFYRMPRQVFNARKKAQSSINPSGSSGGSSGSVTPGTSESATPESSGGGFGGSAKNTITKTLQLRIVRPYNSAEVEKIVADEKNNREKIALERNKDKVKEACSKHLKVASYCTTQVERSACLFCKARKLDDKFYQKLRGQFPDAVFWQELGEIFRQLQKQAAEIYNQSLIELYYEIFIKGKGLANASSVEHYLSDVCYTRAAELFKNAAIASGLRGKVKSNFKLKELKSMKSGLPSTKSDNFPIPLVKQRGGQYTGFEISSHNSDFIIKIPFGRWQEKEEIDKYRPWEKFDFEQVRRSPKPISLLLSTQRRKKNKGWSKDEGTEAEIRRVMNGDYQTSYIEVKRGSKIGEKSAWMLNLSIDVPKIDKGVDPRIIGGIDVGVKSPLVCAINNAFSRYSVGDNDLFHFNKKMFARRRILLKKNRHKRAGHGAKNKLKPITILTEKSVRFRKKLIERWACEIADFFIKNKVGTVQMENLEGMKRKEDSYFNIRLRGFWPYAEMQNIEFKLKQYGIEIRKVAPNNTSKTCSKCGHLNNYFNFEYRRRNKFPLFKCEKCNFKEDADYNAALNISNPKLKSTKEEP

SEQ ID NO: 3390 - protein, 726 aa, synthetic construct
SEVEFSHEYWMRHALTLAKRARDEREVPVGAILVLNNRVIGEGWNRAIGQHDPTAHAEIMALRQGGLVMQNYRLIDATLYVTFEPCVMCAGAMIHSRIGRVVFGVRNSKHGAAGSLMNVLNYPGMNHRVEITEGILADECAALLCDFYRMPRQVFNARKKAQSSINPGGSSGGSSGSETPDTSESATPESSGGNSGGSAKNTITKTLKLRIVRPYNSAEVEKIVADEKNNREKIALEKNKDKVKEACSEHLKVAAYCTTQVERNACLFCKARKLDDKFYQKLRGQFPDAVFWQELGEIFRQLQKQTAEIYNQSLIELYYEIFIKGKGFANASSVEHYLSDVCYTRAAELFKNAAIASGLRGKVKSNLRLKELKNMRSGLPTTKSDNFPIPLVKQKGGQYTGFEISSHNDDLIVKIPFGRWQAKKEIDKYRPWEKFDFEQVRKSPKPISLLLSTQRRKKNRGWSKDEGTEAEIKKVMNGDYQTSYIEVKRGSKIGEKSAWMLNLSIDVPKIDKGVDPSIIGGIDVGVKSPLVCAINNAFSRYSISDNDLFHFNKKMFARRRILLKKSRHKRAGHGAKNKLKPISILTGKSKRFRKKLIERWACEIADFFIKNKVGTVQMENLESMKRKEDSYFNIRLRGFWPYAEMQNKIEFKLKQYGIEIRKVAPNNTSKTCSKCGHLNNYFNFEYRKKNKFPHFKCERCNFKENADYNAALNISNPKLKSTKEEP

SEQ ID NO: 3391 - protein, 725 aa, synthetic construct
SEVEFSHEYWMRRALTLAKRARDEREVPVGAVLVLSNRVIGVGWNRAVGLHDPTAHAEIMALRQGGLVMQNYRLIEATLYVTFEPCIMCAGAMIHSRIGRVVFGVRNSKRGAAGSLMNVLNYPGMNHRVEITEGILADECAALLCDFYRMPRRVFNAKKAQSSTNSGGSFDGSSGSGTLGTSGSPTRESSVGSSASSTKNTITKTLKLRIVRPHNSAEVEKIVADEKDNREKIALEKNKDKVKGACSKHLKVASYCTTQVERNACPFCKARKLDDKFYQKLRGQFPDAVFWQELGEILRQLQKQAAEIYNQSLIELYYEIFIKGKGIASASRVGHYLSDVCYTRAAEQFKNAAIASGLRGKVKSNFRLKELKNMRSGLPTTKSDNFPIPLVKQKGGQYTGFEINSHNDDFIIKIPFGRWQVKKEIDKYRPWEKFDFEQVRKSPKPISLLLSTQRRKRNKGWSKDEGTEAEIRKVMNGDYQTSYIEVKRGSKTGEKSAWMLNLSIDVPEIDKGVDPSIIGGIDVGVKSPLVCAINNAFSRYSISDNDLFRFNKKMFARRRILLKKNRHKRAGHGAKNKLKPISILTGKSERFRKKLIERWACEIADFFIKNKVGTVQMENLESMKRKEDSYFNIRLRGFWPYAEMQNKIEFKLKQYGIEIRKVAPNNTSKTCSKCGHLNNYFNFEYRKKNKFPHFKCEKCNFKEDADYNAALNISNPKLKSTKGEP

SEQ ID NO: 3392 - protein, 725 aa, synthetic construct
SEVEFSHEYWMRHALTLAKRARDEREVPVGAILVLNNRVIGEGWNRAIGQHDPTAHAEIMALRQGGLVMQNYRLIDATLYVTFEPCVMCAGAMIHGRIGRVVFGVRNSKHGAAGSLMNVLNYPGMNHRVEITEGILADECAALLCDFYCMPRQVFNAQKRAQSSINSGGSSGGSSGSETPGTSESATPGSSGGGSSSSAKNTITKTLQLRIVRPYNSAEVEKIVADEKDNREKIALEKNKDKVKEACSKHLKVASYCTTQVERNACPFCKARKLDDKFYQKLRGQFPDAVFWQEVGEIFRQLQKQAAEIYNQSLIELYYEIFIKGKGFANASSVEHYLSDVCYTRAAELFKNAAIASGLRGKVKSNFRLKELKNMKSGLPTTKSDNFPIPLVKQKGGQYTGFEISSHNDDFIIKIPFGRWQVKEEIDKYRPWEKFDFEQVRKNPKPISLLLSTRRRKRNKGWSKDEGTEAEIRKVMNGDYQTSYIEVKRGSKIGEKSAWMLNLSIDVPKIDKGVDPSIIGGIDVGVKSPLVCAINNAFSRYSISDNDLFRFNKKVFARRRILLKKNRHKRAGHGTKNKLKPITILTEKSGRFRKKLIERWACEIANFFIKNKVGTVQMENLESMKRKEDSYFNIRLRGFWPYAEMSKIEFKLKQYGIKIRKVAPNNTSKACSKCGHLNNYFNFEYRKKNKFPHFKCEKCSFKENADYNAALNISNPKLKSTKEEP

SEQ ID NO: 3393 - protein, 726 aa, synthetic construct
SEVEFSHEYWMRHALTLARRARDEREVPVGAVLVLNNRVIGEGWNRAIGLHDPTAHAEIMALRQGGLVMRNYRLTDATLYVTFEPCVMCAGAMIHSRIGRVVFGVRNSKRGAAGSLMNVLNYPGMNHCVEITEGILVDECAALLCDFYRMPRQVLNAQKKAQSSISPGGSSGGSSGSETPGASESVTPKSSGGSSGGSAKNTITKTLKLRIVRPYNSAEVEKIVADEKNNREKIALEKNKGKVREACSKHLEVAAYCITQVERNACLFCKARKLDDKFYQKLRGQFPDAVFWQELGEIFRQLQKQAAEIYNQSLIELYYEIFIKGKGITNASSVGHYLSDVCYTRAAELFKNAAIASGLRGKIKSNFRLKELKNMKSGLPTTKSDNFPIPLVKQKGGQYTGFEISSHNDDFIIKIPFGRWQVKKEIDKYRPWEKFDFEQVRKSPKPISLLLSTQRRKRNKGWSKDEGTEAEIRKVMNGDYQTSYIEVKRGSKTGEKSAWMLNLSIDVPKIDKGVDPSIIGGIDVGVKSPLVCAINNAFSRYSISDNDLFRFNKKMFARRRILLKKSKHRRAGHGAKNKLKPITILTEKSRRFRKKLIERWACEIADFFIKNKVGTVQMENLEGMKRKEDSYFNIRLRGFWPYAEMQNKIEFKLKQYGIEVRKVAPNNTSKTCSKCGHLNNYFNFEYRKKNKFPHFKCEKCSFKENADYNAALNISNPKLKSTKEKP

SEQ ID NO: 3394 - protein, 726 aa, synthetic construct
SEVEFSHEYWMRHALTLAKRARDEREVPVGAVLVLNNRVIGVGWNRAIGLHDPTAHAEIMALRQGGLVMQNYRLTDATLYVTFEPCVMCAGAMIHSRIGRVVFGVRNSKRGAAGSLMNVLNYPGMNHCVEITEGILVDECAALLCDFYRMPRQVLNAQKKAQSSISSGGSSGGSSGSETPGASGSVTPKSSGGSSAGSTKDTITKTLQLRIVRPYNSAEVEKIVADEKNNREKIALEKNKDKVKEACGKHLKVASYCTTQVERNACLFCKARKLDDKFYQKLRGQFPDAVFWQELGEIFRQLQKQAAEIYNQSLIELYYEIFIKGKGLANASSVEHYLSDVCYTRAAELFKNAAIASGLRGKVKSNFKLKELKSMKSGLPSTKSDNFPIPLVKQRGGQYTGFEISSHNSDFIIKIPFGRWQEKEEIGKYRPWEKFDFEQVRRSPKPISLLLSTQRRKKNKGWSKDEGTEAEIRRVMNGDYQTSYIEVKRGSKIGEKSAWMLNLSIDVPKIDKGVDPSIIGGIDVGVKSPLVCAINNSFSRYSICDNDLFRFNKKMFARRRILLKKNRHKRAGHGAKNKLKPITILTKKSERFRKKLIERWVCEVADFFIKNKVGTVQMENLESMKRKEDSYFNIRLRGFWPYAEMQNKIEYKLKQYGIEVRKVAPNNTSKTCSKCGHLNNYFNFEYRRKYKFPHFKCEKCNFKEDADYNAALNISNPKLKSTKEEP

SEQ ID NO: 3395 - protein, 726 aa, synthetic construct
SEVEFSHEYWMRHALTLAKRARDKREVPVGAILVLNNRVIGEGWNRAIGLHDPTAHAEIMALRQGGLVMQNYRLTDATLYVTFEPCVMCAGAMIHSRIGRVVFGVRNNKHGAAGSLVNVLNYPGMNHRVEITEGILADECAALLCDFYRMPRQVFNARKKAQSSINPGGSSGGNSGSETPGTSESATPESSGGSSGSSAKNTITKTLKLRIVRPYNSAEVEKIVADEKNNREKIALEKNKDKVKEACSEHLKVAAYCTTQVERNACLFCKARKLDDKFYQKLRGQFPDAVFWQEIGEIFRQLQKQAAEIYNQSLIELYYEIFIKGKGFADASSVEHYLSDVCYARAAELFKNAAIASGLRGKVKSNFRLKELKNMKSGLPTTKSDNFPIPLVRQKGGQYTGFEISSRNDDFIIKIPFGRWQVKKEIDKYRPWEKFDFEQVRKSPKPISLLLSTQRRKRNKGWSKDEGTEAEIRKVMNGDYQTSYIEVKRGSKIGEKSAWMLSLSIDVPKIDRGVDPSIIGGIDVGVKSPLVCAINNASSRLSISDNDLFRFNKKMFARRRILLKENGHKRAGHGAKNKLKPIAIMTEKSKRFRKKLIERWACEIADFFIKNKVGTVQMENLESMKRKEDSYFNIRLRGFWPYAEMQNKIEFKLKQYGIEIRKVAPNNTSKTCSKCGHLNNYFNFEYRKTNKFPHFKCEKCNFKENADYNAALNISNPKLKSTKEEP

SEQ ID NO: 3396 - protein, 726 aa, synthetic construct
SEVEFSHEYWMRHALTLAKRARDEREVPVGAVLVLNNRVIGEGWNRAIGLHDPTAHAEIMALRQGGLVMQNYRLIDATLYVTFEPCVMCAGAMIHSRIGRVVFGVRNSKRGAAGSLMNVLNYQGMNHRVEITEGILADECAALLCDFYRMPRQVFNAQKKAQSSINSGGSSGGSSGSETPGTSESATPESSGGSSGGSAKNTITKTLKLRIVRPYNSAEVEKIVADEKNNREKIALEKNKDKVKEACSKHLKVAAYCTTQVERNACLFCKARKLDDKFYQKLRGQFPDAVFWQEISEIFRQLQKQAAEIYNQSLIELYYEIFIKGKGIANASSVEHYLSDVCYTRAAELFKNAAIASGLRSKIKSNFRLKELKNMKSGLPTTKSDNFPIPLVKQKGGQYTGFEISNHNSDFIIKIPFGRWQVKKEIDKYRPWEKFDFEQVQKSPKPISLLLSTQRRKRNKGWSKDEGTEAEIKKVMNGDYQTSYIEVKRGSKIGEKSAWMLNLSIDVPKIDKGVDPSIIGGIDVGVKSPLVCAINNAFSRYSISDNDLFHFNKKMFARRRILLKKNRHKRAGHGAKNKLKPITILTEKSERFRKKLIERWACEIADFFIKNKVGTVQMENLESMKRKEDSYFNIRLRGFWPYAEMQNKIEFKLKQYGIEIRKVAPNNTSKTCSKCGHLNNYFNFEYRKKNKFPHFKCEKCNFKENADYNAALNISNPKLKSTKEEP

SEQ ID NO: 3397 - protein, 725 aa, synthetic construct
SDVEFSHEYWMRHALTLAERARDEREVPVGAILVLNNRVIGEGWNRAIGLHDPTAHAEIMALRQGGLVTQNYRLIDATLYVTFEPCVMCAGAMIHSRIGRVVFGVRNSKHGAAGSLVNVLNYPGMNHRVEITEGVLADECAALLCDFYRMPRQVFNARKKAQSNINPGGSSGGSSGSETPGTSDSATPGSSGGSSGGSAKNTITKTLKLRIVRPYNSAEVEKIVADEKNNREKTALEKNKDKVKEACSEHLKVATYCTTQVERNACLFCKARKLDDKFYQKLRGQFPDAVFWQELGEIFRQLQKQAAEIYNQSLIELYYEIFVKGKGFANASSVEHYLSDVCYTRAAELFKNAAIASGLRGKVKSNFRLKELKNMRSGLPTTKSDNFPIPLVKQKGGQYAGFEISSHNDDFIIKIPFGRWQVKKEIDKYRPWEKFDFEQVRKSPKPISLLLSTQRRKRNKGWGKDEGTEAEIRKVMNGDYRTSYIEVKRGSKIGEKSAWMLSLSIDVPKIDKGVDPRIIGGIDVGVKSPLVCAINNAFSRYSISDNDLFHFNKKMFARRRILLKKNRHKRAGHGAKNKLKPISILTGKSERFRKKLIERWACEIADFFIKNKVGTVQMENLESMKRREDSYFNIRLRGFWPYAKMNKIEFKLKQYGIEIRKVAPNNTSKTCSKCGHLNNYFNFEYRKKNKFPHFKCEKCNFKESADYNAALNISNPKLKSPKEEP

SEQ ID NO: 3398 - protein, 726 aa, synthetic construct
SEVEFSDEYWMRHALTLAKRARDEREVPVGAVLVLNNRVIGEGWNRAIGLYDPTAHAEIMALRQGGLVMRNYRLTDATLYVTFEPCVMCAGAMIHSRIGRVVFGVRNSKRGAAGSLMNVLNYPGMNHCVEITEGILTDECAALLCDFYRMPHQVLNAQRKAQSNINSGGPSGGSSCSETPGASESVTPKSFGGSSAGSTKNTITKTLKLRIVRPYNSAEVEKIVTDEKNSREKIALEKNKDKVKEACSEHLKVAAYCTTQVERSACLFCKARKLDDRFYQKLRGQFPDAVFWQETGEIFRQLQRQAAEIYNQSLIELYYEIFIKGKGFANASSVEHYLSDVCYTRAAELFKNAAIASGLRGKVKSNFRLKELKNMKSGLPTTKSDNFPIPLVKQKGGQYTGFEISSHNDDFIIKIPFGRWQAKKEIDKYRPWEKFDFEQVRKSPKPISLLLSTQRRKRNKGWSKDEGTEAEIKKVMNGDYQTSYIEVKRGSKIGEKSAWMLSLSIDVPKIDKGVDPSIIGGIDVGVKSPLVCAINNALSRYSISDNDLFRFNKKMFARRRILLKKNRHRRAGHGAKNKLKPIAVLAEKSVGFRKKLIERWACEVADFFIKNKVGSVQMENLESMKRKEDSYFNIRLRGFWPYAEMQDKIEFKLKQYGIKIRKVAPNNTSKTCSKCGHLNNYFNFEYRKMNKFPHFKCEKCNFKENADYNAALNISNPKLKSTKEEP

SEQ ID NO: 3399 - protein, 726 aa, synthetic construct
SEVEFSHEYWMRHALTLAKRARDEREVPVGAILVLNNRVIGEGWNRAIGLHDPTAHAEIMALRQGGLVMQNYRLIDATLYVTFEPCVMCAGAMIHSRIGRVVFGVRNNKHGAAGSLMNVLNYPGMNHRVEITEGILADECAALLCDFYRMPRQVFNARKKAQSSINPGGSSGGSGGSETPGTSESATPENSGGSSGSSAKNTITKTLKLRIVRPYNSAEVEKIVADEKNNREKNALEENKDKVKEACSEHLKVAAYCTTQVERSACLFCKARKLDDKFYQKLRGQFPDAVFWQEIGEIFRQLQRQAAEIYNQSLIELYYEIFIKGKGFANASSVEHYLSDVCYARAAELFKNAAIASGLRGKVKSNFRLKELKNMKSGLPTTKSDNFPIPLVKQKGGQYTGFEISNHNDDFIIKIPFGRWQVKEEIDKYRPWEKFDFEQVRKNPKPISLLLSTQRRKGNKGWSKDEGTEAEIRKVMNGDYQTSYIEVKRGSKTGEKSAWMLNLSIDVPKIDKGVDPSIIGGIDVGVKSPLVCAINNAFSRYSISDNDLFHFNKKVFARRRILLKKTRHKRAGHGAKNKLKPISILTEKSKRFRKKLIERWACEIANFFIKNRVGTVQMENLESMKRKEDSYFNIRLRGFWPYAEMQNRIEFKLKQYGIEIRKVAPSNTSKTCSKCGHLNNYFSFEYRKRNKFPHFKCEKCNFKENADYNAALNISNPKLKSTKEEP

SEQ ID NO: 3400 - protein, 726 aa, synthetic construct
SEVEFSHEYWMRHALTLAKRARDEREVPVGAVLVLNNRVIGEGWNRTTGLHDPTAHAEIMALRQGGLVMRNYRLTDATLYVTFEPCVMCAGAMIHSRIGRVVFGVRNSKHGAAGSLMNVLNYPGMNHRVEITEGILADECAALLCDFYRMPRQVFNARKKVQSSINPGGSSGGSSGSETPGTSESATPESSGGSSGGSAKNTITKALKLRIVRPYNSAEVEKIVADEKNIREKIALEKNKDKVKEACSKHLKVAAYCTTQVERNACLFCKARRLDDKFYQKLRGQFPDAVFWQEIGEIFRQLQKQAAEIYNQSLIELYYEIFIKGRGLANASSVEHYLSDVCYTRAAELFKNAAIASGLRGKVKSNFRLKELKSMKSGLPTTKSDNFPIPLVKQKGGQYTGFEVSSHNDDFIIKIPFGRWQVKKEIDKYRPWEKFDFEQVRKSPRPISLLLSTQRRKRNKGWSKDEGTEAEIRKVMNGDYQTSYIEVRRGSKIGEKSAWMLNLTIDVPKIDKGVDPSIIGGIDVGVKSPLVCAIDNAFSRYSISDNDLYHFNKKMFAKRRILLKKNRHKRAGHGAKNKLKPISILTEKSERFRKKLIERWACEIADFFIKNKVGTVQMENLESMKRREDSYFNTRLRGFWPYAEMQNRIEFKLKQYGIEIRKVAPNNTSKTCSKCGHLNNYFNFEYRKKNKFPHFKCEKCNFKENADYNAALNISNPRLKSTKEEP

SEQ ID NO: 3401 - protein, 726 aa, synthetic construct
SEVEFSHEYWMRHALTLAKRARDGREVPVGAVLVLNNRVIGEGWNRAIGLHDPTAHAEIMALRQGGLVMQNYRLIDATLYVTFEPCVMCAGAMIHSRIGRVVFGVRNSKRGAAGSLMNVLNYPGMNHCVEITEGILVDECAALLCDFYRMPRQVLNAQKKAQSSISSGGSSGGSSGSETPGASESATPKSSVGSSAGSTKNTITKTLKLRIVRPYNSAEVEKIVADEKNNREKIALEKNKDKVKEACSEHLKVAAYCTTQVERNACPFCKARKLDDKFYQKLRGQFPDAVFWQEISEIFRQLQKQAAEIYNQSLIELYYEIFIKGKGFANASSVEHYLSDVCYTRAAELFKNAAIASGLRGKVKSNFRLKELKNMKSGLPTTKSDNFPIPLVKQKGGQYTGFEISSHNDDFIIKIPFGRWQEKKEINKYRPWEKFDFEQVRKGPKPISLLLSTQRRKRNKGWSKDEGTEAEIRKVMNGNYQTSYIEVKRGSKIGEKNAWMLSLSIDVPKIDKGVDPSIIGGIDVGVKSPLVCAINNALSRYSISDNDLFHFNKKMFARRRILLKKNRHKRAGHGAKNKLKPITILTKKSERFRKKLIERWVCEVADFFIKNKVGTVQMENLESMKRKEDSYFNIRLRGFWPYAEMQNRIELKLKQYGIEIRRVAPNNTSRTCSKCGHLNNYFNFEYRKKSKFPHFKCEKCNFREDADYNAALNISNPKLKSTKEEP

SEQ ID NO: 3402 - protein, 726 aa, synthetic construct
SEVEFSHEYWMRHALTLAERARDGREVPVGAVLVLNNRVIGEGWNRAIGLHDPTAHAEIMALRQGGLVMQNYRLIDATLYVTFEPCVMCAGAMVHSRIGRVVFGIRNSKRGAAGSLTNVLNYPGMNHRVEITEGILVDECAALLCDFYRMPRQVFNAQKKAQSNINPGGSSGGSSDSETPGTSENATPGSSGGSSGGSAKNTITKTLKLRIVRPYNSAEVEKIVADEKNNREKIALEKNKDKVKEACSEHLKVAAYCTTQVERNACLFCKARKLDDKFYLKLRGQFPDAVFWQEIGEIFRQLQKQAAEIYNQSLIELYYEIFIKGKGITNASRVEHYLSDVCYTRAAELFKNAAIASGLRGKVKGNFRLKELKNMKSGLPTTKSDNFPIPLVKQKGGQYTGFEISSHNDDLIVKIPFGRWQVKKEIDRYRPWEKFDFEQVRKSPKPISLLLSTQRRKRNKGWSKDEGTEAEIRKVMNGDYQTSYIEVKRGSKIGEKSAWMLNLSIDVPKIDKGVDPSIIGGIDVGVKSPLVCAINNAFSRYSISDNDLFHFNKKMFARRRILLKKNRHKRAGHGAKNKLKPISILTEKSKRFRKKLIERWACGIADFFIKNKVGTVQMENLESMKRKEDSYFNIRLRGFWPYAEMQNKIEFKLKQYGIEIRKVAPNNTSKTCSRCGHLNNYFNFEYRRKNKFPHFKCEKCNFKEDADYNAALNISNPKLKSTKEEP

SEQ ID NO: 3403 - protein, 726 aa, synthetic construct
SEVEFSHEYWMRHALTLAKRARDEREVPVGAVLVLNNRVIGEGWNRAIGLHDPTAHAEIMALRQGGLVMQNHRLIDATLYVTFEPCVLCAGAMVHSRIGRVVFGVRNSKRGAAGSLMNVLNHPSMNHRIEITEGILADECAALLCDFYRMPRQVFNARKKAQSSINSGGSSGGSSGSETPGTSESATPESSGGSSGGSAKNTITKTLKLRIVRPYNSAEVEKIVADEKDNREKIALEKNKDKVKEACSEHLKVAAYCTTQVERNACLFCRARKLDDKFYQKLRGQFPDAVFWQEIGEIFRQLQKQAAEIYNQSLIELYYEIFIKGKGFANASSVEHYLSDVCYTRAAELFKNAAIASGLRGKVKSNLRLKELKNMKSGLPTTKSDNFPIPLVKQKGGQYAGFEISSHNDDFIIKIPFGRWQVKKEIDKYRPWEKFDFEQVRKSPKPISLLLSTQRRKRNKGWGKDEGTEAEIRKVMNGDYQTSYIEVKRGSKIGEKGAWMLSLSIDVPKIDKGVDPSIIGGIDVGVKSPLVCAINNAFSRYSISDNDLFRFNKKMFARRRILLKKNRHKRAGHGAKNKLKPISILTGKSVRFRKKLIERWACEIADFFIKNKVGTVQMENLESMKRKEDNYFNIRLRGFWPYAEMQNRIEFKLKQYGIEIRKVAPNNTSKTCSKCGHLNNYFNFEYRKMNKFPHFKCEKCNFKENADYNAALNISNPKLKSTKEEP

SEQ ID NO: 3404 - protein, 726 aa, synthetic construct
GEVEFSHEYWMRHALTLAKRARDEREVPVGAILVLNNRVIGEGWNRAIGLHDPTAHAEIMALRQGGLVMQNYRLTDATLYVTFEPCVMCAGAMIHSRIGRVVFGVRNSKRGAAGSLMNVLNYPGMNHCVEITEGILVDECAALLCDFYRMPRQVLNAQKKAQSSISSGGSSGGSSGSETPGASGSVTPKSSGGSSAGSTKDAITKTLKLRIVRPYNSAEVEKIVADEKNNREKIAMEKNKDKVKEACSKHLKVATYCTTQVERNACLFCKARKLDDKFYQKLRGQFPDAVFWQELGGIFRQLQKQAAEIYNQSLIELYYEIFIKGKGFANASSVEHYLSDVCYTRAAELFKNAAIASGLRGKVKSNFRLKELKNMKSGLPTTKSDNFPIPLVKQKGGQYTGFEISSHNDDFIIKIPFGRWQVKKEIDKYRPWEKFDFEQVRKSPKPISLLLSTQRRKRNKGWSKDEGTEAEIRKVMNGDYQTSYIEVKRGSKIGEKSAWMLNLSIDVPKIDKGVDPCIIGGIDVGVKSPLVCAINNAFSRYSISDNDLFRFNKKVFARRRILLKKNRHKRAGHGTKNKLKPISILTEKSERFRKKLIERWVCEVADFFIKNKVGTVQMENLESMKRKEDSYFNIRLRGFWPYAEMQNRIELKLKQYGIEIRRVAPNNTSRTCSKCGHLNNYFNFEYRKKSKFPHFKCEKCNFREDADYNAALNISNPKLKSTKEEP

SEQ ID NO: 3405 - protein, 726 aa, synthetic construct
SEVEFSHEYWMRHALTLAKRARDEREVPVGAILVLNNRVIGEGWNRAIGLHDPTAHAEIMALRQGGLVMQNYRLTDATLYATFEPCVMCAGAMIHSRIGRVVFGVRNSKHGAAGSLMNVLNYPGMNHRVEITEGILADECAGLLCDFYRMPRQVFSARKKAQSSINPGGSSGGSSGGKAPGTSESATLESSGGSSGDSAKNSITKTLKLRIVRPYNSAEVEKIVADEKNNREKIALEKNKGKVEEACSKHLKVATYCTTQVERNACLFCKARKLDDKFYQKLRGQFPDAVFWQEIGEIFRQLQKQAAEIYNQSLIELYYEIFIEGKGFANASSVEHYLSDVCYTRAAELFKNAAIASGLRGKVKGNFRLKELKSMKSGLPTTKSDNFPIPLVKQKGGQYTGFEISSHNDDFIIKIPFGRWQVKKEIDRYRPWEKFDFEQVRKSPKPISLLLSTQRRKRNKGWSKDEGTEAEIRKVMNGDYQTSYIEVKRGSRTGEKSAWMLSLSIDVPKIDKGVDPSIIGGIDVGVKSPLVCAINNALSRYSISDNDLFRFNKKMFARRRILLKKNRHRRAGHGAKNKLKPIAVLAEKSVGFRKKLIERWACEVADFFIKNKVGTVQMENLESMKRREDSYFNIRLRGFWPYAEMQNKIEFKLRQYGIEIRKVAPNNTSKTCSKCGHLNNYFNFEFRKKNKFPHFKCEKCNFKEDADYNAALNISNPKLKSTKEEP

SEQ ID NO: 3406 - protein, 726 aa, synthetic construct
SEVEFSHEYWMRHALTLAKRARDEREVPVGAVLVLNNRVIGEGWNRAIGLHDPTAHAEIMALRQGGLVMQNYRLTDATLYVTFEPCVMCAGAMIHSRIGRVVFGVRNGKRGAAGSLMNVLNYPGMNHCVEITEGILVDECAALLCDFYRMPRQVLNAQKKAQSSISSGGSSGGSNGSETPGASESATPKSSGGSSAGSTKNTITKTLKLRIVRPYNSAEVEKIVADEKNSREKTALEKNKDKVKEACSKHLKVASYCTTQVERNACLFCKARKLDDKFYQKLRGQFPDAVFWQEIGEIFRQLQKQAAEIYNQSLIELYYEIFIKGKGFANASSVEHYLSDVCYTRAAELFKNAAIASGLRGKVKGNFRPRELKNMKSGLPTTKSDNFPIPLVKQKGGQYTGFEISSHNDDFIIKVPFGRWQAKKEIDKYRPWEKFDFEQVRKSPKPISLLLSTQRRKRNKGWSKDEGTEAEIKKVMSGDYQTSYIEVKRGSKTGEKSAWMLNLSIDVPKIDKGVDPSIIGGIDVGVKSPLVCAINNAFSRYSISDNDLFRFNKKMFARRRILLGKNRHKRAGHGVKNKLKPITILTKKSERFRKKLIERWVCEVADFFIKNKVGTVQMENLESMKRKEDSYFNIRLRGFWPYAEMQNRIELKLKQYGIEVRRVAPNNTSRTCSKCGHLNNYFNFEYRKKNKFPHFKCEKCNFREDADYNAALNISNPKLKSTKEEP

SEQ ID NO: 3407 - protein, 726 aa, synthetic construct
SEVEFSHEYWMRHALTLAKRARDEREVPVGAVLVLNNRVIGEGWNRAIGLHDPTAHAEIMALRQGGLVLQNYRLADATLYVTFEPCVMCAGAMIHSRIGRVVFGVRNGKRGAAGSLMNVLNYPGMNHCVEITEGILMDECAALLCDFYRMPRQVLNAQKKAQSSINSGGSSGGSSGSETPGASESVTPKSSGGSSAGSTKNTITKTLKLRIVRPYNSAEVEKIVSDEKNNREKIALEKNKDKVKEACSKHLKVASYCTTQVERNACPFCKARKLDDKFYQKLRGQFPDAVFWQELGEILRQLQKQAAEIYNQSLIELYYEIFIRGRGFANASSAEHYLSDVCYTRAAELFKNAAIASGLRGKVKSNFRLKELKSMKSGLPSTKSDNFPIPLVKQKGGQYTGFEISSHNDDFIIKVPFGRWQVKKEIDKYRPWEKFDFEQVRKSPKPISLLLSTQRRKRNKGWSKDVGTEAEIRKVMNGDYQTSYIEVKRGSKIGEKSAWMLNLSIDVPKIDKGVDPSIIGGIDVGVKSPLVCAINNAFSRYSISDNDLFRFNKKMFARRRILLRKNRHKRAGHGAKNKLKPITMMTEKSKRFRKKLIERWACEIADFFIKNKVGTVQMENLESMKRKEDSYFNIRLRGFWPYAEMQNKIEFKLKQYGIVVRKVAPNNTSKTCSKCGHLNNYFNFEYRKKNKFPHFKCEKCNFKENADYNAALNISNPQLKSTKGEP

SEQ ID NO: 3408 - protein, 726 aa, synthetic construct
SEVEFSHEYWMRHALTLAKRARDEREVPVGAVLVLNNRAIGEGWNRAIGLHDPTAHAEIMALRQGGLVMQNYRLTDATLYVTFEPCVMCAGAMIYSRIGRVVFGVRNSKRGAAGSLMNVLNYPGMNHCVEITEGILVDECAALLCDFYRMPRQVLNAQKKAQSSISSGGSSGGSSGSETPGASGSVIPRSSGGSSAGSTKDTITKTLKLRIVRPYNSAEVEKVVADEKNNREKIAMEKNKDKVKEACSKHLKVASYCTTQVERNACLFCKARKLDDKFYQKLRGQFPDAVFWQEVGEIFRQLQKQAAEIYNQSLIELYYEIFIKGKGFANASSVEHYLSDVCYTRAAELLKNAAIASGLRGKVKSNFRLKELKNMKSGLPTTKSDNFPIPLVKQKGGQYTGFEISNHNDDFIIKIPFGRWQVKEEIDKYRPWEKFDFEQVRKNPKPISLLLSTQRRKRNKGWSKDEGTEAEIRKVMNGDYQTSYIEVKRGSKIGEKSAWMLNLSIDVPKIDRGVDPSIIGGIDVGVKSPLVCAINSAFSRYSISDNDLFRFNKKVFARRRILLKKNRHKRAGHGTKNKLKPITILTEKSGRFRKKLIERWACEIADFFIKNKVGTVQMENLESMKRKEDSYFNLRLRGFWPYAEMQNKIEFKLKQYGIEIRRVAPNNTSKTCSKCGHLNNYFNFEYRKKNKFPHFKCEKCNFKENADYNAALNISNPKLKSTKEEP

SEQ ID NO: 3409 - protein, 726 aa, synthetic construct
SEVEFSHEYWMRHALTLAKRARDEREVPVGAVLVLNNRVIGEGWNRTIGLHDPTAHAEIMALRQGGLVMQNHRLVDATLYVTFEPCVMCAGAMIHSRIGRVVFGVRNSKRGAAGSLTNVLNYPGTNHRVEITEGILADECAALLCDFYRMPRQVFIAQKKAQSSINSGGSSGGGSGSDTPSTSESTTPESSGGSSGGSAKNTITKTLKLRIVRPYNSAEVEKIVADEKNNREKIALEKNTDKVKEACSKHLKVAAYCTTLVERSACLFCKARRLDDKFYQKLRGQFPDAVFWQEIGEIFRQLQKQAAEIYNQSLVELYYEIFIKGKGFANASSAEHYLSDVCYTRAAELFKNAAIASGLRGKVKSNFRLKELKNMKSGLPTTKSDNFPIPLVKQKGGQYTGFEISSHNDDFIIKIPFGRWQVKKEIDKYRPWEKFDFEQVRKSPKPISLLLSTQRRKRNKGWSKDEGTEAEIRKVMNGDYQTSYIEVKRGRKTGEKSAWMLNLSIDVPKIDRGVDPSIIGGIDVGVKSPLVCAINNAFSRYSISDNDLFRYNKKMFARRRILLKKNRHKRAGHGAKNKLKPISILTEKSKRFRKKLIERWACEIADFFIKNKVGTVQMENLESMKRKEDSYFNIRLRGFWPYAEMQNKIEFKLKQYGIEIRKVAPNNTSRTCSKCGHLNNYFNFEYRKKNKFPHFKCEKCNFKEDADYNAALNISNPKLKSTKEEH

SEQ ID NO: 3410 - protein, 726 aa, synthetic construct
SEVEFSHEYWMRHALTLAKRARDEREVPVGAILVLNNRVIGEGWNRAIGLHDPTAHAEIMALRQGGLVMQNYRLIDATLYVTFEPCVMCAGAMIHSRIGRVVFGVRNNKHGAAGSLVNVLNYPGMNHRVEITEGILADECAALLCDFYCMPRQVFNAQKRPQSSINSGGSSGGSSGSETPGTSESATPESSDGGSSGSAKNTITKTLQLRIVRPYNSAEVEKIVADEKNNREKIALEKNKDKVKEACSKHLKVASYCTTQVERNACPFCKARKLDDKFYQKLRGQFPDAVFWQELGEILRQLQKQAAEIYNQSLIELYYEIFIKGRGFANASSVEHYLSDVCYTRAAELFKNAAIASGLRSKVRSNFRLKELKNMKSGLPTTKSDNFPIPLVKQKGGQYTGFEISSHNSDFIIKIPFGRWQVKEEIDKYRPWEKFDFEQVRKSPKPISLLLSTQRRKKNKGWSKDEGTEAEIRRVMNGDYQTSYIEVKRGSKIGEKSAWMLSLSIDVPKIDKGVDPRTIGGIDVGVKSPLVCAINNAFGRYSISDNDLFHFNKKMFARRRILLKKNRHKRAGHGAKNKLKPITILTEKSGRFRKKLIERWACEIADFFIKNKVGTVQMENLEGMKRKEDSYFNIRLRGFWPYAEMQNKIEFKLKQYGIEIRKVAPNNTSKTCSVCGHLNNYFNFEYRKKNKFPHFKCEKCNFKENADYNAALNISNPKLKSTKGEP

SEQ ID NO: 3411 - protein, 726 aa, synthetic construct
SEVEFSHEYWMRHALTLAKRARDEREVPVGAVLVLNNRLIGEGWNRAIGLHDPTAHAEIMALRQGGLVMQNHRLVDATLYVTFEPCVMCAGAMIHSRIGRVVFGVRNSKRGAAGSLTNVLNYPGMNHRVEITEGILVDECAALLCDFYRMPRQVFSAQKKAQSTINSGGSSGGSSGSETPGTSESPTPESSGGSPGGSAKNTITKTLKLRIVRPYNSAEVEKIVADEKDNREKIALEKNKDKVKEACSKHLKVAAYCTTQVERNACQFCKARKLDDKFYQKLRGQFPDAVFWQEIGEIFRQLQKQAAEIYNQSLVELYYEIFIRGKGIANASSVEHYLSDVCYTRAAGLFKNAAIASGLRNKIKSNFRLKELRNMKSGLPTTKSDNFPIPLVRQKGGQYTGFEISSHNDDFIIKIPFGRWQVKKEIDKYRPWEKFDFEQVRKSPKPISLLLSTQRRRRNKGWSKDEGTEAEIRKVMNGDYQTSYIEVKRGSKIGEKSAWMLNLSIDVPKIDKGVDPSIIGGIDVGVKSPLVCAIDNAFSRYSISDNDLYRFNKKMFARRRILLKKNRHKRAGHGAMNKLKPITILTEKSGRFRKKLIERWACEIANFFIKNKVGTVQMENLESMKRKEDSYFNIRLRGFWPYAEMQNKIEFKLKQYGIEIRKVAPNNTSKICSKCGHLNSYFNFEYRRKNKFPHFKCEKCNFKENADHNAALNISNPKLKSTKEEP

SEQ ID NO: 3412 - protein, 726 aa, synthetic construct
SEVEFSHEYWMRHALTLAKRARDEREVPVGAVLVLNNRVIGEGWNRAIGLHDPTAHAEIMALRQGGLVMRNYRLTDATLYVTFEPCVMCAGAMIHSRIGRVVFGVRNSKRGAAGSLMNVLNYPGMNHCVEITEGILVDECAALLCDFYRMPRQVLNAQKKAQSSISPGGSSGGSSGSETPGTSESATPESSGGSSAGSTKNAITKTLKLRIVRPYNSAEVEKIVANEKNNRERIALEKNKDKVKEACSKHLKVAAYCTTQVERNACLFCKARKLDDKFYQKLRGQFPDAVFWQETGEIFRQLQRQAAEIYNQSLIELYYEIFIKGKGFANASRVEHYLSDVCYTRAAELFKNAAIASGLRGKVKGNFRLKELKNMKSGLPTTKSDNFPISLVKQKGGQYTGFEISSHNDDFIIKIPFGRWQAKKEIDKYRPWEKFDFEQVRKSPKPISLLLSTQRRKRNKGWSKDEGTEAEIRKVMNGDYRTSYIEVKRGGKTGEKSAWMLNLSIDVPKIDKGVDPSIIGGIDVGVKSPLVCAINNAFGRYSISDNDLFHFNKKMFARRRVLLKKNRHQRAGHGAKNKLKPITILTEKSGRFRKKLIERWACEIADFFIKNKVGTVQMENLESMKRKEDSYFNIRLRGFWPYAEMQNKIEFKLKQYGIKIRKVAPNNTSKTCSKCGHLNNYFSFEYRKKNKFPHFKCEKCNFKENADYNAALNISNPKLMSTKEEP

SEQ ID NO: 3413 - protein, 726 aa, synthetic construct
SEIEFSHEYWMRHALTLAKRARDEREVPVGAILVLNNRVIGEGWNRAIGLHDPTAHAEIMALRQGGLVMQNYRLIDATLYVTFEPCVMCAGAMIHSRIGRVVFGVRNNKHGAAGSLVNVLNYPGMNHRVEITEGILADECAALLCDFYRMPRQVFNARKKAQSSISSGGTSGGCSGSEMPGASESVTPKCSGGSSAGSTKNTITKTLKLRIVRPYNSAEVEKIVADEKNNRERIALEKNKDKVKEACSKHLKVAAYCTTQVERNACLFCKARKLDDKFYQKLRGQFPDAVFWQETGEIFRQLQRQAAEIYNQSLIELYYEIFIKGRGFANASSVEHYLSDVCYTRAAELFKNAAIASGLRGKVKGNFRLKELKNMKSGLPTTKSDNFPIPLVKQKGGQYTGFEISSHNDDFIIKIPFGRWQAKKEIDKYRPWEKFDFEQVRKSPKPISLLLSTQRRKRNKGWSKDEGTEAEIRKVMNGDHQTSYIEVKRGSKTGEKSAWMLNLSIDVPKINKGVDPSIIGGIDVGVKSPLVCAINNAFSRYSISDNDLFRFNKKMFARRRILLKKNRHKRAGHGAKNKLKPISILTGKSERFRKKLIERWACEIADFFIKNKVGTVQMENLESMKRKEDSYFNIRLRGFWPYAEMQNRIELKLKQYGIEIRRVAPNNTSRTCSKCGHLNNYFNFEYRKKNKFPYFKCEKCNFKENADYNAALNISNPQLKSTKGEP

SEQ ID NO: 3414 - protein, 726 aa, synthetic construct
SEVEFSHEYWMRHALTLAKRARDEREVPVGAILVLNNRVIGEGWNRAIGLHDPTAHAEIMALRQGGLVMQNYRLIDATLYVTFEPCVMCAGAMVHSRIGRVVFGVRNSKRGAAGSLMNVLNYPGVNHCVEITEGILVDECAALLCDFYRMPRRVLNAQKKAQSSISSGGSSGGCSGSEMPGASESVTPKSSGGSSAGSTKNTITKTLKLRIVRPYNSAEVEKIVADEKNSREKIALERNKDKVKEACSEHLKVAAYCTTQVERNACLFCKARKLDDRFYQKLRGQFPDAVFWQETGEIFRQLQRQAAEIYNQSLIELYYEIFIKGKGFANASSVEHYLSDVCYTRAAELFKNAAIASGLRGKVKSNFRLKELKNMKSGLPTTKSDNFPIPLVKQKGGQYTGFEISSHNDDFIIKIPFGRWQVKKEIDKYRPWEKFDFEQVRKSPKPISLLLSTQRRKRNKGWSKDEGTEAEIRKVMNGDYQTSYIEVKRGSKIGEKSAWMLSLSIDVPKIDKGVDPSIIGGIDVGVKSPLVCAINNAFSRYSIGDNDLFRFNKKVFARRRILLKKNRHKRAGHGAKNKLKPISILTEKSKRFRKKLIERWACEIADFFIKNKVGTVQMENLESMKRKEDSYFNIRLRGFWPYAEMQNRIEFKLEQYGIEIRKVAPHNTSKTCSKCGHLNNYFNFEYRKKNKFPHFKCEKCNFKENADYNAALNISNPKLKSTKEEP

SEQ ID NO: 3415 - protein, 726 aa, synthetic construct
SEDEFSHEYWMRHALTLAKRARDECEVPVGAILVLNNRVIGEGWNRAIGLHDPTAHAEIMALRQGGLVMQNYRLIDATLYVTFEPCVMCAGAMIHSRIGRVVFGVRNSKYGAAGSLVNVLNYPGMNHRVEITEGILADECAALLCDFYRMPRQVFNARKKAQSSINPSGSSGGSSGSVTPGTSESATPESSGGGFGGSAKNTITKTLQLRIVRPYNSAEVEKIVADEKNNREKIALEKNKDKVKEACSKHLKVASYCTTQVERNACLFCKARKLDDKFYQKLRGQFPDAVFWQELGEIFRQLQKQAAEIYNQSLIELYYEIFIKGKGFANASSVEHYLSDVCYTRAAELFKNTAIASGLRGKVKSNFRLKELKNMKSGLPTTKSDNFPIPLVKQKGGQYTGFEISSHNDDFVIKIPFGRWQVKKEIDKYRPWEKFDFEQVRKGPKPISLLLSTQRRKRNKGWSKDEGTEAEIRKVMSGDYQTSYIEVKRGSKTGEKSAWMLNLSIDVPKIDKGVDPSIIGGIDVGVKSPLVCAINNALSRYSISDNDLFHFNKKMFARRRILLKKNRHKRAGHGAKNKLKPISILTEKSERFRKKLIERWACEIADFFIKNKVGTVQMENLESMKRREDSYFNIRLRGFWPYAEMQNKIEFKLKQYGIKIRKVAPNNTSKTCSKCGHLNNYFSFEYRKKNKFPHFKCEKCNFKEDADYNAALNISNPKLKSTKEEP

SEQ ID NO: 3416 - protein, 726 aa, synthetic construct
SEVEFSHEYWMRRALTLAKRARDEREVPVGAVLVLNNRVIGVGWNRAVGLHDPTAHAEIMALRQGGLVLQNYRLIDATLYVTFEPCVMCAGAMIHSRIGRVVFGVRNNKHGAAGSLVNVLNYPGMNHRVEITEGILADECAALLCDFYRMPRQVFNARKKTQSSINPGGSSGGSSGSETPGTSESATPESSGGSSGSSAKNTITKTLQLRIVRPYNSAEVEKIVADEKNSREKIALEKNKDKVKEACSKHLKVASYCTTQVERNACLFCKARKLDDKFYQKLRGQFPDAVFWQELGEIFRQLQKQAAEIYNQSLIELYYEIFIKGKGLANASSVEHYLSDVCYTRAAELFKNAAIASGLRGKVKSNFRLKELKNMKSGLPTTKSDNFPIPLVKQKGGKYTGFEISSHNDDFIIKIPFGRWQVKKEINKFRPWEKFDFEQVRKSPKPISLLLSTQRRKRNKGWSKDEGTEAEIRKVMNGDYQTSYIEVKRGSKIGEKSAWMLNLSIDVPKIDKGVDPSIIGGIDVGVKSPLVCAISNAFSRYSISDNDLFHFNKKMFARRRILLKKSKHKRADHGAKNKLKPITVLTEKSRRFRKKLIERWACEIADFFIKNKVGTVQMENLESMKRKEDSYFNIRLRGFWPYAEMQNRIEFKLKQYGIKIRKVAPNDTSKTCSKCGHLNDYFNFEYRKRNKFPHFKCGKCNFKENADYNAALNISNPKLKGTKEEP

SEQ ID NO: 3417 - protein, 726 aa, synthetic construct
SEVEFSHEYWMRHALTLAKRARDEREVPVGAILVLNNRVIGEGWNRAIGLHDPTAHAEIMALRQGGLVMQNYRLIDATLYVTFEPCVMCAGAMIHSRIGRVVFGVRNNKHGAAGSLVNVLNYPGMNHRVEITEGILADECAALLCDFYRMPRQVFNARKKAQSSINPGGSSGGSSGSETPGTSESATPESSGGSSGSSAKNTITKTLKLRIVRPYNSAEVEKIVADEKNNREKIALEKNKDKVKEACSKHLKVAAYCTTQVERNACLFCKARRLDDKFYQKLRGQFPDAVFWQELGEILRQLQKQAAEIYNQSLIELYYEIFNKGKGFANASSVEHYLSDVCYTRAAELFKNAAIASGLRGKVKSNFRLKELRSMKSGLPTTKSDNFPIPLVRQKGGQYTGFEISSRNDDFIIKIPFGRWQVKKEIDKYRPWEKFDFEQVRKSPKPISLLLSTQRRKRNRGWGKDEGTEAEIKRVMNGDYQTSYIEVKRGSKIGEKSAWMLNLSIDVPKIDKGVDPRIIGGIDVGVKSPLVCAINNAFSRYSVSDNDLFHFNKKMFARRRILLKKNRHKRAGHGAKNKLKPITILTKKSERFRKKLIERWVCEVADFFIKNKVGTVQMENLESMKRKEDSYFNIRLRGFWPYAEMQNRIELKLKQYGIEIRRVAPNNTSRTCSKCGHLNNYFNFEYRKKNKFPHFKCEKCNFREDADYNAALNISNPKLKSTKGEP

SEQ ID NO: 3418 - protein, 726 aa, synthetic construct
SEVEFSHEYWMRHALTLAKRARDEREVPVGAILVLNNRVIGEGWNRAIGLHDPTAHAEIMALRQGGLVMQNYRLIDATLYVTFEPCVMCAGAMIHSRIGRVVFGVRNNKHGAAGSLVNVLNYPGMNHRVEITEGILADECAALLCDFYRMPRQVFNARKKAQSSISSGGSSGGCSGSEMPGASESVTPKSSGGSSAGSTKNTITKTLKLRIVRPYNSAEVEKIVADEKNSREKIALERNKDKVKEACSEHLKVAAYCTTQVERNACLFCKARKLDDRFYQKLRGQFPDAVFWQEAGEIFRQLQKQATEIYNQSLIELYYEIFIKGRGFANASSVEHYLSDVCYTRAAELFKNAAIASGLRGKVKSNFRLKELKNMKSGLPTTKSDNFPIPLVKQKGGQYTGFEISSHNDDFIIKIPFGRWQVKKEIDKYRPWEKFDFEQVRKSPKPISLLLSTQRRKRNKGWSKDEGTEAEIRKVMNGDYQTSYIEVKRGSKTGEKSAWMLNLSIDVPKIDKGVDPSIIGGIDVGVKSPLVCAINNAFSRYSISDNDLFRFNKKMFARRRILLKKNGHKRAGHGAKNKLKPISILTEKSKRFRKKLIERWACEIADFFIRNKVGTVQIENLESMKRKEDSYFNIRLRGFWPYAEMQNKIEFKLKQYGIKIRKVAPNNTSRTCSKCGLLNNYFDFEYRKKNKFPHFKCEKCNFKENADYNAALNISNPKLKSTKEEP

SEQ ID NO: 3419 - protein, 726 aa, synthetic construct
SEDEFSHEYWMRHALTLAKRARDGREVPVGAVLVLNNRVIGEGWNRAIGLHDPTAHAEIMALRQGGLVMQNYRLIGATLYVTFEPCVMCAGAMVHSRIGRVVFGVRNSKRGAAGSLMNVLDYPGMGHRVEITEGILADECAALLCDFYCMPRQVFNAQKRAQSSINSGGSSGGGSSSDTPSTSESTTPESPGGSSGGSAKNTITKTLKLRIVRPYNSAEVEKIVADEKDNRERIALEKNKDKVKEACSKHLMVASYCTTQVERSACLFCKARELDGRFYQKLRGQFPDAVFWQEIGEIFRQLQKQAAGIYNQSLIELYYEIFIKGKGFANASSVEHYLSDVCYARAAELFKNAAIASGLRGKVKSNFRLKELRNMKSGLPTTMSDNFPIPLVKQKGGQYTGFEISNHNSDFIIKIPFGRWQVKKEIDKYRPWEKFDFEQVRKSPKPISLLLSTQRRKRNKGWSKDEGTEAEIRKVMNGDYQTSYIEVKRGSKIGEKSAWMLNLSIDVPKIDKGVDPSIIGGIDVGVKSPLVCAINNAFSRYSISDNDLFHFNKKMFARRRILLKKNRRRRAGHGAKNKLKPITILTEKSGRFRKKLIERWACEIADFFVKNKVGTVQMENLESMKRKEDSYFNIRLRGFWPYAEMQNKIEFKLKQYGIEVRKVAPNNTSRTCSKCGHLNNYFNFEFRKKNKFPHFKCEKCNFKENADYNAALNISNPKLKSTKEEP

SEQ ID NO: 3420 - protein, 726 aa, synthetic construct
SEVEFSHEYWMRHALTLAKRARDEREVPVGAILVLNNRVIGEGWNRAIGLHDPTAHAEIMALRQGGLVMQNYRLIDATLYVTFEPCVMCAGAMIHSRIGRVVFGVRNSKHGAAGSLVNVLNYPGMNHRVEITEGILADECAALLCDFYRMPHQVFGARRKAQSSINPGGSSGGSSGSETPGASESVTPKSSVGSSAGSTKNTITKTLKLRIVRPYNSAEVEKIVADEKDNRERIALEKNKDKVKEACSKHLMVASYCTTQVERSACLFCKARELDGRFYQKLRGQFPDAVFWQEIGEIFRQLQKQAAEIYNQSLIELYYEIFIKGKGFANASSAEHYLSDVCYTRAAELFKNAAIASGLRGKVKSNFRLKELKNMKSGLPTTKSDNFPIPLVRQKGGQYTGFEISNYNGDFIIKIPFGRWQVKKEVDKYRPWEKFDFEQVRKSPKPISLLLSTQRRKRNKGWSKDEGTEAEIRKVMNGDYQTSYIEVKRGSKIGEKSAWMLNLSIDVPKIDKGVDPSIIGGIDVGVKSPLVCAINNAFSRYSISDNDLFHFNKKMFARRRILLKKNRHRRAGHGAKNKLKPITVLTEKSEGFRKKLIERWACEIADFFIKNKVGTVQMENLESMKRKEDSYFNIRLRGFWPYAEMQNKIEFKLKQYGIEIRKVAPNNTSKTCSKCGHLNNYFDFEYRKKNKFPHFKCEKCNFKENADYNAALNISNPKLRSTKEEP

SEQ ID NO: 3421 - protein, 726 aa, synthetic construct
SEVEFSHEYWMRHALTLAKRARVEREVPVGAVLVLNNRVIGEGWNRAIGLHDPTAHAEIMALRQGGLVMQNYRLIDATLYVTFEPCVMCAGAMIHSRIGRVVFGVRNNKHGAAGSLVNALNYPGMNHRVEITEGILADECAALLCDFYRMPRQVFNARKKAQSSINPGGSSGGSSGSETPGTSESPTPESSGGSSGGSAKNTITKTLKLRIVRPYNNAEVEKIVAEEKNNREKIALEKNKDKVKEACSEHLKVATYCTTQVERNACPFCKARKLDDKFYQKLRGQFPDAVFWQELGEIFRQLRKQAAEIYNQSLIELYYEIFIKGKGFANASSVEHYLSDVCYTRAAELFKNAAIASGLRGKVKSNFRLKELRNMKSGLPTTKSDNFPIPLVRQKGGQYTGFEISSRNDDFIIKIPFGRWQVKKEIDKYRPWEKFDFEQVRKSPKPISLLLSTQRRKRNKGWSKDEGTEAEIGKVMNGDYQTSYIEVKRGSKIGEKSAWMLNLSIDVPKIDKGVDPSIIGGIDVGVRSPLVCAINNALSRYSISDNDLFRFNKKMFARRRILLKKNRHKRAGHGAKNKLKPITILTEKSKRFRKKLIERWACEIADFFIKNKVGTVQMENLESMKRKEDSYFNIRLRGFWPYAEMQNKIEFKLKQYGIVVRKVAPNNTSKTCSECGHLNNYFNFEYRKKNKFPHFKCEKCNFKENADYNAALNISNPKLKSTKGEP

SEQ ID NO: 3422 - protein, 726 aa, synthetic construct
SEVEFSHEYWMRHALTLAKRARDEREVPVGAVLVLNNRVIGEGWNRAIGLHDPTAHAEIMALRQGGLVLQNYRLVDATLYVTFEPCVLCAGAMVHSRIGRVVFGARNSKRGAAGSLMNVLDYPGMGHRVEITEGILADECAALLCDFYCMPRQVFNAQKRAQSSINSGGSSGGSCGSDTPGTSGSATPESSSGGSSGSAKNTITKTLQLRIVRPYNSAEVEKIVADEKNNREKIALEKNKDKVKEACSEHLKVAAYCTTQVERNACLFCKARKLDDKFYQKLRGQFPDAVFWQELGEIFRQLQKQAAEIYNQSLIELYYEIFIKGKGFANASSAEHYLSDVCYTRAAELFKNAAIASGLRGKVKSNFRLKELKNMKSGLPTTKSDNFPIPLVRQKGGKYTGFEISSHNDDFIIKIPFGRWQAKKEIDKYRPWEKFDFEQVRKSPKPISLLLSTRRRKRNKGWSKDEGTEAEIRRVMNGDYQTSYIEVKRGSKIGEKSAWMLNLSIDVPKIDKGVDPSIIGGIDVGVKSPLVCAINNAFSRYSISDNDLFHFNKKMFARRRILLKKNRHKRAGHGAKNKLKPLTILTGKSKRFRKKLIERWACEIANFFIKNKVGTVQMENLESMKRKEDSYFNIRLRGLWPYAEMQNKIEFKLKQYGIEVRKVAPNNTSKTCSKCGHLNNYFNFEYRKRNKFPHFKCEKCNFKENADYNAALNISNPKLKGTKEEL

SEQ ID NO: 3423 - protein, 726 aa, synthetic construct
GEVEFSHEYWMRHALTLAKRARDEREVPVGAILVLNNRVIGEGWNRAIGLHDPTAHAEIMALRQGGLVMQNYRLVDATLYVTFEPCVLCAGAMVHSRIGRVVFGVRNSKRGAAGSLMNVLDYPGMNHRVKITEGILADECAALLCDFYRMPRRVFNAQKKAQSSINSGGSSGGGSGSETPSTSENTTPESSGGSSGGPAKSTITKTLKLRIVRPYNSAEVEKIVADEKNNREKIALEKNKDKVKEACSEHLKVAAYCTTQVERNACLFCKARKLDDRFYQKLRGQFPDAVFWQEIGEIFRQLQKQAAEIYNQSLIELYYEIFIKGKGFANASGVEHYLSDVCYTRAAELFKNAAIASGLRGKVKSNFRLKELKNMRSGLPTTKSDNFPIPLVKQKGGQYTGFEISDLNSDFIIKIPFGRWQAKKEIDKYRPWEKFDFEQVRKSPKPISLLLSTQRRKRNKGWSKDEGTEAEIRKVMNGDYQTSYIEVKRGSKIGEKSAWMLNLSIDVPKIDKGVDPSIIGGIDVGVKSPLVCAINNAFSRYSISDNDLFHFNKKMFARRRILLKKNRHKRAGHGAKNKLKPLTILTGKSKRFRKKLIERWACEVADFFIKNKVGTVQMENLESMKRKEDSYFNIRLRGLWPYAEMQNKIEFKLKQYGIEIRKVAPNNTSKTCSKCGHLNNYFNFEYRKKNKFPHFKCEKCNFKENADYNAALNISNPKLKSPKEEP

SEQ ID NO: 3424 - protein, 726 aa, synthetic construct
SEVEFSHEYWMRRALTLAKRARDEREVPVGAVLVLNNRVIGVGWNRAVGLHDPTAHAEIMALRQGGLVMQNYRLIEATLYVTFEPCIMCAGAMIHSRIGRVVFGVRNSKRGAAGSLMNVLNYPGMNHRVEITEGILTDECAALLCDFYRMPHQVLNAQKKAQSSINSGGSSGGSSGSETPGTSGSATPEGSGGSSGGSAKNTITKTLKLRIVRPYNSAEVEKIVADEKNNREKIALEKNKDKVKEACSKHLKVAAYCTTQVERNACLFCRARKLDDKFYQKLRGQFPDAVFWQEIGEIFRQLQRQAAEIYNQSLIELYYEIFIKGKGFANASSAEHYLSDVCYTRAAELFKNAAIASGLRSKVRSNFRLKELKNMKSGLPTTKSDNFPIPLVKQKGGQYTGFEISSHNSDFIIKIPFGRWQVKKEINKYRPWEKFDFEQVRKSPKPISLLLSTQRRKRNKGWGKDEGTEAEIRRVMNGNYQTSYIEVKRGSKIGEKSAWMLNLSIDVPKIDKGVDPSIIGGIDVGVKSPLVCAINNAFSRYSISDNDLFHFNKKMFARRRILLKKNRHKRAGHGAKNKLKRITILTEKSKRFRKKLIERWACEIADFFIKNKVGIVQMENLESMKRKEDSYFNIRLRGFWPYAEMQNRIEFKLKQYGIVVRKVAPNNTSKTCSKCGHLNNYFNFEYRKKNKFPHFKCEKCNFKEDADYNAALNISNPKLKSTKGEP

SEQ ID NO: 3425 - protein, 726 aa, synthetic construct
SEVEFSHEYWMRHALTLAKRARDEREVPVGAILVLNNRVIGEGWNRAIGLHDPTAHAEIMALRQGGLVMQNYRLIDATLYVTFEPCVMCAGAMIHGRIGRVVFGVRNSKHGAAGSLVNVLNYPGMNHRVEITGGILVDECAALLCDFYRMPRHVLNAQKKAQSSISSGGSSGGCSGSEMPGASESVTPKSSGGSSAGSTKNTITKTLKLRIVRPYNSAEVEKIVADEKNSREKIALERNKDKVKEACSEHLKVAAYCTTQVERNACLFCKARKLDDRFYQKLRGQFPDAVFWQETGEIFRQLQRQAAEIYNQSLIELYYEIFIKGKGFANASGVEHYLSDVCYTRAAELFKNAAIASGLRGKVKGNFRLKELRNMKSGLPTTMSDNFPIPLVKQKGGQYTGFEISNHNSDFIIKIPFGRWQVKKEIDKYRPWEKFDFEQVRKSPKPISLLLSTQRRKRNKGWSKDEGTEAEIRKVMNGDYQTSYIEVKRGNKIGEKSAWMLNLSIDVPKTDKGVDPSVIGGIDVGVKSPLVCAVNSALSRYSISDNDLFHFNKKMFARRRILLKKNRHKRAGHGAKNKLKPISILTEKSKRFRKKLIERWACEIADFFIKNKVGTVQMENLESMKRKEDSYFNIRLRGFWPYAEMQNKIEFKLKQYGIGIRKVAPNNTSKTCSKCGHLNNYFNFEYRRKNKFPHFKCEKCNFREDADYNAALNISNPKLKSTKEEP

SEQ ID NO: 3426 - protein, 726 aa, synthetic construct
SEVEFSHEYWMRHALTLAKRARDEREVPVGAVLVLNNRVIGEGWNRTTGLHDPTAHAEIIALRQGGLVMQNHRLVDATLYVTFEPCVMCAGAMIHSRIGRVVFGVRNNKHGAAGSLVNVLNYPGMNHRVEITEGILVDECAALLCDFYRMPRQVLNAQKKAQSSISSGGSSGGCSGSETPGASESVTPKSSGSSSGGSAKNTITKTLKLRIVRPYNSAEVEKIVADEKNNREKIALEKNKDKVKEACSKHLKVAAYCTTQVERNACLFCKARRLDDKFYQRLRGQFPDAVFWQEIGEIFRQLQKQAAETYNQSLIELYYEIFIKGKGITNASRVEHYLSDVCYTRAAELFKNAAIASGLRSKVRSNFRLKELKNMKSGLPTTKSDNFPIPLVKQKGGQYTGFEISSHNSDFIIKIPFGRWQEKEEIGKYRPWEKFDFEQVRRSPKPISLLLSTQRRKKNKGWSKDEGTEAEIKKVMNGDYQTSYIEVKRGSKIGEKSAWMLNLSIDVPKIDKGVDPSIVGGIDVGVKSPLVCAINNALGRYSISDNDLFHFNKKMFARRRILLKKSKHKRAGHGAKNKLKPITILTEKSGRFRKKLIERWACEIADFFIKNKVGTVQMENLEGMKRKEDSYFNIRLRGFWPYAEMQNKIEFKLKQYGIEVRKVAPNNTSKTCSKCGHLNHYFNFEYRKKNKFPHFKCEKCNFKENADYNAALNISNPKLKSTKGEP

SEQ ID NO: 3427 - protein, 726 aa, synthetic construct
SEGEFSHEYWMRHALTLAKRARDEREVPVGAVLVLNNRVIGEGWNRMTGLHDPTAHAEIMALRQGGLVMQNHRLVDATLYVTFEPCAMCAGAMIHGRIGRVVFGVRNNKHGAAGSLVNVLNYPGMNHRVEITEGILANECAALLCDFYRMPRQVFNARKKAQSSINPGGSSGGSSGSETPGTSESATPESSGGSSGGSAKNTITKALKLRIVRPYNSAEVEKIVADEKNNRERIALEKNKDKVKEACSEHLKVAAYCTTQVERNACLFCKARKLDDRFYQELRGQFPGAVFWQEIGEIFRQLQKQAAEIYNQSLIELYYEIFIKGKGFANASSVEHYLSDVCYTRAAELFKNAAIASGLRGKVKSNFRLKELKNMKSGLPTTKSDNFPIPLVKQKGGQYTGFEISNHNSDFIIKIPFGRWQAKEEIDKYRPWEKFDFEQVRKSPKPISLLLSTQRRKKNKGWSKDEGTEAEIRRVMNGDYQTSYIEVKRGSKIGEKSAWMLNLSIDVPKIDKGVDPSIIGGIDVGVKSPLVCAINNSSSRYSICDNDLFRFNKKMFARRRILLKKNRHKRAGHGAKNKLKPISILTEKSKRFRKKLIERWACEIADFFIKNKVGTVQMENLESMKKKEDSYFNIRLRGFWPYAEMQNKIEFKLKQYGIEIRKVAPNNTSKTCSKCGHLNNYFNFEYRKKNKFPHFKCEKCNFIENADYNAALNISNPKLKSTREEP

SEQ ID NO: 3428 - protein, 726 aa, synthetic construct
SENEFSHEYWMRHALTLAKRARDGREVPVGAVLVLNNRVIGEGWNRAIGLHDPTAHAEIMALRQGGLAMQNYRLVDATLYVTFEPCVLCAGAMVHSRIGRVVFGVRNSKRGAAGSLMNVLNHPGMNHRVEITGGILADECAALLCDFYRMPRQVFNVQKKARSNINSGGSSGGSSGSETLGTSESATPESSGGSSGGSAKNTITKTLKLRIVRSYNSAEVEKIVADEKNNREKIAMEKNKDKVKEACSKHLKVASYCTTQVERNACLFCKARKLDDKFYQKLRGQFPDAVFWQELGEIFRQLQKQAAEIYNQSLIELYYEIFIKGKGFANASSVEHYLSDVCYTRAAGLFKNAAIASGLRGKVKSNFRLKELKNMKSGLPTTKSDNFPIPLVKQKGGQYTGFEVSSHNDDFIIKIPFGRWQVKKEIDKYRPWEKFDFEQVRKSPRPISLLLSTQRRKRNKGWSKDEGTEAEIRKVMNGDYRTSYIEVKRGSKIGEMSAWMLNLSIDVPKIDKGVDPSIIGGIDVGVKSPLVCAINNAFSRYSISDNELFHFNKKMFARRRILLKKNRHKRAGHGAKNKLKPISVLTEKSGRFRKKLIERWACEIADFFIKNKVGTVQMENLGSMKRKEDSYFNIRLRGFWPYAEMQNKIEFKLKQYGIEIRKVAPDNTSKTCSKCGHLNNYFNFEYRKKNKFPHFKCEKCNFKEDADYNAALNISNPKLKSTKEEP

SEQ ID NO: 3429 - protein, 726 aa, synthetic construct
SEVEFSHEYWMRHALSLAKRARDEREVPVGAVLVLNNRIIGEGWNRAIGQHDPTAHAEIMALRQGGLVMQNNRLTDATLYVTFEPCVMCAGAMVHSRIGRVVFGVRNSKRGAAGSLMNVLNYPGVNHCVEITEGILVDECAALLCDFYRMPRQVLNAQKKAQSSISSGGSSGGCSGSEMPGASESVTPKSSGGGSAGSTKNTITKTLKLRIVRPYNSAEVEKIVADEKNNREKIALEKNKGKVKEACSKHLEVAAYCTTQVERNACLFCKARKLDDKFYQELRGQFPDAVFWQEIGGIFRQLQKQAAEIYNQSLIELYYEIFIKGKGITNASRVEHYLSDVCYTRAAELFKNAAIASGLRSKVRSNFRLKELKNMKSGLPTTKSDNFPIPLVKQKGGQYTGFEISSHNSDFIIKIPFGRWQEKEEIGKYRPWEKFDFEQVRRSPKPISLLLSTQRRKKNKGWSKDEGTEAEIRRVMNGDYQTSYIEVKRGSKIGEKSAWMLNLSIDVPKIDKGVDPSIIGGIDVGVKSPLVCAINDAFSRYSISDNDLFHFNKKMFARRRILLKKNRRRRAGHGAKNKLKPISILTGKSERFRKKLIERWACEIADFFIKNKVGTVQMENLESMKRKEDSYFNIRLRGFWPYAEMQNKIEFKLKQYGIEIRKVAPNNTSKTCSKCGHLNNYFNFEYRKKNKFPHFKCEKCNFKENADYNAALNISNPKLKSTKEEP

SEQ ID NO: 3430 - protein, 726 aa, synthetic construct
SEVEFSHEYWMRHALTLAKRARDEREVPVGAVLVLNNRVIGEGWNRAIGLHDPTAHAEIMALRQGGLVMQNYRLIDATLYVTFEPCVMCVGAMVHSRIGRVVFGVRNSKRGAAGSLMNVLDYPGMGHCVEITEGILADECAALLSDFYRMPRQVFNAQKKAQSSINSGGSSGGSSGSETPGTSESATPESSGGSSGGSAKNTITKTLQLRIVRPYNSAEVERIVADEKNYREKIALEKNKDKVKEACSKHLKVAAYCTTQVERNACLFCRARKLDDKFYQKLRGQFPDAVFWQELGEIFRQLQKQAAEIYNQSLIELYYEIFIKGKGFANASSVEHYLSDVCYTRAAELFKNAAIASGLRGKVKSNFRLKELKNMKSGLPTTKSDNFPIPLVKQKGGQYTGFEISSHNDDFIIKIPFGRWQVKEEIIKFRPWERFDFEQVRKSPKPISLLLSTQRRKRNRGWSKDEGTEAEIRKVMNGDYQTSYIEVKRGSKIGEKSAWMLNLSIDVPKIDKGVDPGIIGGIDVGVKSPLVCAINNALSRYSISDNDLFHFNKKMFARRRILLRKNRHKRAGHGARNKLKPITVLTEKSERFRKKLIERWACEIANFFIKNKVGTVQMENLESMKRREDSYFNVRLRGFWPYAEMQSKIEFELKQYGIKIRKVAPNNTSKTCSKCGHLNNYFNFEFRKKNKFPHFKCEKCNFKEDADYNAALNIGNPKLKGTKEEP

SEQ ID NO: 3431 - protein, 726 aa, synthetic construct
SEVEFSHEYWMRHALTLAKRARDGREVPVGAVLVLNNRVIGEGWNRAIGLHDPTAHAEVMALRQGGLVMQNYRLIGATLYVTFEPCAMCAGAMVLSRISRVVFGVRNSKRGAAGSLMNVLNYPGMDHRVEITGGILADECAALLCDFYRMPRRVFNAQKKAQSGINSGGSSGGSSGSVTPGTSESATPESSGGGFGGSAKNTITKTLQLRIVRPYNSAEVEKIVADEKNNREKIALEKNKDKVQEACSKHLKVASYCTTQVERNACLFCKARKLDDKFYQKLRGQFPDAVFWQELGEIFRQLQKQAAEIYNQSLIELYYEIFIKGKGLANASSVEHYLSDVCYTRAAELFKNAAIASGLRGKVKSNFKLKELKSMKSGLPSTKSDNFPIPLVKQKGGQYTGFEIRGHNDDLIIKIPFGRWQVKKEIDKYRPWEKFDFEQVRKSPKPISLLLSTQRRKRNKGWSKDEGTEAEIRKVMNGDYQTSYIEVKRGSKIGEKSAWMLNLSIDVPKIDKGVDPGIIGGIDVGVQSPLVCAIDNAFGRYSISDNDLFHFNKKMFARRRILLKKNRHKRAGHGAKNKLKPITILTKKSERFRKKLIERWVCEVADFFIKNKVGTVQMENLESLKRKEDSYFNIRLRGFWPYAEMQNKIEFKLKQYGIEIRKVAPNNTSKTCSKCGHLNNYFNFEYRKKNKFPHFKCEKCNFKENADYNAALNISNPMLKSTKEEP

SEQ ID NO: 3432 - protein, 726 aa, synthetic construct
SEDEFSHEYWMRHALTLAKRARDEREVPVGAILVLNNRVIGEGWNRAIGLHDPTAHAEIMALRQGGLVMQNYRLIDATLYVTFEPCVMCAGAMIHSRIGRVVFGVRNSKHGAAGSLMNVLNYPGMNHRVEITEGILADECAALLCDFYRMPHQVFSARKKAQSSINPGGSSGGSSGSKTPGTSESATPESSGGSSGGSAKNSITKTLKLRIVRPYNSAEVEKIVADEKNNREKIALEKNKGKVKEACSKHLKVATYCTTQVERNACLFCKARKLDDKFYQKLRGQFPDAVFWQEIGEIFRQLQKQAAEIYNQSLIELYYEIFIEGKGFANASSVEHYLSDVCYTRAAELFKNAAIASGLRNKIKSNFRLKELRNMKSGLPTTKSDNFPIPLVRQKGGQYTGFEISSHNDDFIIKIPFGRWQVKKEIDKYRPWEKFDFEQVRKSPKPISLLLSTQRRKRNKGWSKDEGTEAEIRKVMNGDYQTSYIEVKRGSKIGEKSAWMLNLSIDVPKIDKGVDPSIIGGIDVGVKSPLVCAINNAFSRYSVSDNDLFHFNKKMFARRRILLKKNRHRRAGHGAKNKLKPIAVLAKKSEGFRKKLIERWACEVADFFIKNKVGTVQMENLESMKRREDSYFNIRLRGFWPYAEMQNKIEFKLRQYGIEIRKVAPNNTSKTCSKCGHLNNYFDFEYRKKNKFPHFKCEKCNFKENADYNAALNISNPKLRSTKEEP

SEQ ID NO: 3433 - protein, 726 aa, synthetic construct
SEVEFSHEYWMRHALTLAKRARDEREVPVGAVLVLNNRVIGGGWNRAIGLHDPTAHAEIMALRQGGLVMQNCRLIDATLYVTFEPCVMCAGAMIHSRIGRVVFGVRNSKHGAAGSLVNVLNYPGMNHRVEITEGILADECAALLCDFYRMPRQVLNAQKKAQSSISSGGSSGGSSGSETPGASGSVIPKSSGGSSAGSTKDTITKTLKLWIVRPYNSAEVEKIVADEKNNREKIALEKNKDKVKEACSKHLKVAAYCTTQVERNACLFCKARRLDDKFYQKLRGQFPDAVFWQEVGEIFRQLQKQAAEIYNQSLIELYYEIFIKGKGLANASSVEHYLSDVCYTRAAELFKNAAIASGLRGKVKSNFRLKELKSMKSGLPSTKSDNFPIPLVKQRGGQYTGFEISSHNDDFIIKIPFGRWQAKKEIDKYRPWEKFDFEQVRKSPKPISLLLSTQRRKRNKGWSKDEGTEAEIRKVMNGDYQTSYIEVKRGSKVGEKGAWMLNLSIDVPKIDKGVDPSIIGGIDVGVKSPLVCAINNASSRYSISDNDLFRFNKKMFARRRILLGKNRHKRAGHGVKNKLKPITILTEKSGRFRKKLIERWACEIADFFVKNKVGTVQMENLESMKRKEDSYFNIRLRGFWPYAEMQNKIEFKLKQYGIEIRKVAPNNTSKTCSKCGHLNNYFNFEYRKKNKFPHFKCEKCNFKENADYNAALNISNPKLKSTKEEP

SEQ ID NO: 3434 - protein, 726 aa, synthetic construct
SEVEFSHEYWMRHALTLAKRARDEREVPVGAVLVLNNRVIGEGWNRAIGLHDPTAHAEIMALRQGGLVMQNYRLIDATLYVTFEPCVMCAGAMVHSRIGRVVFGVRNSKRGAAGSLMNVLDYPGMGHRVEITEGILADECAALLCDFYCMPRQVFNAQKRAQSSINSGGSSGGSSGSDTPGTSESATPESSGGGSSGSAKNTITKTLQLRIVRPYNSAEVEKIVADEKNNREKIALEKNKDKVKEACSKHLKVASYCTTQVERNACLFCKARKLDDKFYQKLRGQFPDAVFWQEIGEIFRQLQKQAAGIYNQSLIELYYEVFIKGKGFANASSVEHYLSDVCYTRAAELFKNAAIASGLRGKVKSNFRLKELKNMRSGLPTTKSDNFPIPLVKQKGGQYTGFEISSHNDDFIIKIPFGRRQVKKETDKYRPWEKFDFEQVRKSPKPISLLLSTQRRKRNKGWSKDEGTEAEIRKVMNGDYQTSYIEVKRGSRIGEKNAWMLNLSIDVPKVDKGVDPSIIGGIDVGVRSPLVCAINNAFSRYSVSDNDLFRFNKKMFARRRILLKKNKHKRAGHGAKNKLKPITILTEKSGRFRKKLIERWACEIADFFIKNKVGTVQMENLESMKRKEDSYFNIRLRGFWPYAEMQNKIEFKLKQYGIKIRKVAPNNTSKTCSKCGHLNNYFSFEYRKKNKFPHFRCEKCSFMENADYNAALNISNPKLKSTKEEP

SEQ ID NO: 3435 - protein, 726 aa, synthetic construct
SEVEFSHEYWMRHALTLAKRARDEREVPVGAVLVLNNRVIGGGWNRAIGLHDPTAHAEIMALRQGGLVMQNCRLVDATLYVTFEPCVMCAGAMVHSRIGRVVFGVRNSKRGAAGSLMNVLDYPGMDHRVEITEGILADECAALLCDFYRMPRQVFNAQKKAQSSINSGGPSGGSSGSETPGTSESATPESSGGSSGGSAKNTITKTLKLRIVRPYNSAEVEKIVADEKNNREKIALEKNKDKVKEACSQHLKVAAYCTTQVERNACLFCKARRLDDKFYQKLRGQFPDAVFWQEIGEIFRQLQKQAAEIYNQSLIELYYEIFIKGKGFANASSVEHYLSDVCYTRAAELFKNAAIASGLRGKVKSNFRLKELKNMKSGLPSTKSDNFPIPLVKQKGGQYTGFEISSHNDDFIIKIPFGRWQVKKEIDKYRPWEKLDFEQVRKSPKPISLLLSTQRRKRNKGWSKDEGTEAEIRKVMNGDYQTSYIEVKRGSKIGEKSAWMLNLSIDVPKIDKGVDPSIVGGIDVGVKSPLVCAINNAFSRYSISDNDLFHFNKKMFARRRILLKKSKHKRAGHGAKNKLKPITILTEKSGRFRKKLIERWACEIADFFIKNKVGTVQMENLESMKRKEDSYFNLRLRGFWPYAEMQNKIEFKLKQYGIEIRKVAPNNTSKTCSKCGHLNNYFNFEYRKMNKFPHFKCEKCNFKENADYNAALNISNPKLKSTKEEP

SEQ ID NO: 3436 - protein, 726 aa, synthetic construct
SEVEFSHEYWMRHALTLAKRARDEREVPVGAILVLNNRVIGEGWNRAIGLHDPTAHAEIMALRQGGLVMQNYRLIDATLYVTFEPCVMCAGAMIHSRIGRVVFGVRNNKHGAAGSLVNVLNYPGMNHRVEITEGILADECAALLCDFYRMPRQVFNARKKAQSSINPGGSSGGSSGSETPGTSESATPKSSGGSSAGSTKDTITKTLKLRIVRPYNSAEVEKIVADEKNSREKIALEKNKDKVKEACSEHLKVAAYCTTQVERNACLFCKARRLDDKFYQKLRGQFPDAVFWQEIGEIFRQLQKQAAEIYNQSLIELYYEIFIRGKGTANASSVEHYLSDMCYARAAELFKNAAIASGLRNKVKSNFRLKELKNMRSGLPTTKSVNFPIPLVKQKGGQYTGFEVSNHNSDFIIKIPFGRWLVKKEINKYRPWEKFDFERVRKSPKPISLLLSTQRRKRNKGWSKDEGTEAEIRKVMNGDYQISYIEVKRGHKIGEKSAWMLNLSIDVPKIDKGVDSSIVGGIDVGVKSPLVCAINSALGRYSISDNDLFHFNKKVFARRRILLKKNGHKRAGHGAKNKLKPISILTGKSERFRKKLIERWACEIADFFIKNKVGTVQMENLESMKRKEDSYFNIRLRGFWPYAEMQNKIEFKLKQYGIEIRKVAPNNTSKTCSRCGHLNNYFNFEYRKKNKFPHFKCEKCDFREDADYNAALNISNPKLKSTKEEP

SEQ ID NO: 3437 - protein, 726 aa, synthetic construct
SEVEFSHEYWMRHALTLAKRARDEREVPVGAVLVLNNRAIGEGWNRAIGLHDPTAHAEIMALRQGGLVMQNYRLIDATLYVTFEPCVMCAGAMVHSRIGRVVFGVRNSKRGAAGSLMNVLDYPGMGHRVEITEGILADECAALLCDFYRMPRQVFNAQKRAQSSISPGGSSGGSSGSETPGASESVTPKSSGGSSGGSAKNTITKTLKLRIVRPYNSAEVEKIVADEKNNREKIALEKNKDKVKEACSEHLKVAAYCTTQVERSACLFCKARKLDDKFYQKLRGQFPDAVFWQELGEIFRQLQKQAAEIYNQSLIELYYEIFIKGKGFANASSVEHYLSDVCYTRAAELFKNAAIASGLRGKVKSNFRLKELKNMKSGLPTTKSDNFPIPLVKQKGGQYTGFEISSHNDDFIIKIPFGRWQVKKEINKHRPWEKFDFEQVRKSPKPISLLLSTQRRKRNKGWSKDEGTEAEVRKVMNGDYQTSYIEVKRGSKIGEKSAWMLNLSIDVPKIDKGVDPSIIGGIDVGVKSPLVCPINNALSRYSISDNDLFHFNKKMFARRRILLRKNRHKRAGHGAKNKLKPITIMTEKSKRFRKKLIERWACEIADFFIKNKVGTVQMENLESMKRKEDSYFNIRLRGFWPYAEMQNKIEFKLKQYGIVVRKVAPNNTSKTCSKCGHLNNYFNFEYRKKNKFPHFKCEKCNFKEDADYNAALNISNPKLKSTKGEP

SEQ ID NO: 3438 - protein, 726 aa, synthetic construct
SEVEFSHEYWMRRALTLAKRARDEREVPVGAVLVLNNRVIGVGWNRAVGLHDPTAHAEIMALRQGGLVMQNYRLIEATLYVTFEPCIMCAGAMIHSRIGRVVFGVRNSKRGAAGSLMNVLNYPGMNHRVEITEGILADECAALLCDYYRMPRQVFNARKKAQSSINSGGSSDGGSGSETPGTSESATPESSGGSSGGSAKNTITKTLKLRIVRPYNSAEVEKIVADEKNNREKIALEKNKDKVKEACSEHLKVAAYCTTQVERGACLFCKARKLDDKFYQKLRGQFPDAVFWQEIGEIFRQLQKQAAEIYNQSLIELYYEIFIKGKGSANASSVEHYLSDVCYTRAAEQFKNAAIASGLRGKVKSNFRLKELKNMKSGLPTTKSDNFPIPLVKQKGGQYTGFEISSHSDDFIIKIPFGRWQVKKEIDKYRPWEKFDFEQVRKSPKPISLLLSIQRRKRNKGWSKDEGTEAEIRRVMNGDYQTSYIEVKRGSKIGEKSAWMLNLSIDVPKIDKGVDPSIIGGIDVGVRSPLVCAINNAFSRYSISDNDLFRFNKKMFARRRILLKKNRHKRAGHGAKNKLKPITILTKKSERFRKKLIERWVCEVADFFIKNKVGTVQMENLESMKRKEDSYFNIRLRGFWPYAEMQNKIEFKLKQYGIEIRKVAPNNTSKTCSKCGHLNNYFNFEYRKKNKFPHFKCEKCNFKENADYNAALNISNPKLKSTKEEP

SEQ ID NO: 3439 - protein, 726 aa, synthetic construct
SEVEFSHEYWMRHALTLAKRARDGREVPVGAVLVLNNRVIGEGWNRAIGLHDPTAHAEIMALRQGGLVMQNYRLIDATLYVTFEPCAMCAGAMVHSRISRVVFGVRNSKRGAAGSLMNVLNYPGMDHRVEITGGILADECAALLCDFYRMPRRVFNAQKKAQSSINSGGSSGGSSGSVTPGTSESATPESSGGSSGGPAKNTITKTLKLRIVRPYNSAEVEKIVADEKNNREKTALEKNKDKVKEACSKHLKVAAYCTTQVERNACLFCKARKLDDKFYQKLRGQFPDAVFWQEIGEIFRQLQKQAAEIYNQSLIELYYEIFIEGKGFANASSVEHYLSDVCYTRAAELFKNAAIASGLRGKVKGNFRLKELKSMKSGLPTTKSDNFPIPLVKQKGGQYTGFEISSHNDDFIIKIPFGRWQVKKEIDRYRPWEKFDFEQVRKSPKPISLLLSTQRRKRSKGWSKDEGTEAEIRKVMNGDYQTSYIEVKRGSKIGEKSAWMLNLSIGVPKIDKGVDPSIIGGIDVGVKSPLVCAINNAFSRYSISDNDLFHFNKKMFARRRVLLKKNRHKRAGHGAKNKLKPISILTEKSKRFRKKLIERWACEIADFFIKNKVGTVQMEDLESMKRKEDSYFNIRLRGFWPYAEMQNRIEFKLKQYGIEIRKVAPNSTSKTCSKCGHLNNYFNFEYRKRNKFPHFKCEKCNFKENADYNAALNISNPKLKSTKEEF

SEQ ID NO: 3440 - protein, 726 aa, synthetic construct
SEVEFSHEYWMRHALTLAKRARDEREVPVGAILVLNNRVIGEGWNRAIGLHDPTAHAEIMALRQGGLVMQNYRLIDATLYVTFEPCVMCAGAMIHSRIGRVVFGVRNSKHGAAGSLMNVLNYPGMNHRVEITEGILADECAALLCDFYRMPHQVFSARKKAQSSINPGGSSGGSSGSKTPGTSESATPESSGGSSGGSAKNSITKTLKLRIVRPYNSAEVEKIVADEKNNREKIALEKNKGKVKEACSKHLKVATYCTTQVERNACLFCKARKLDDKFYQKLRGQFPDAVFWQEIGEIFRQLQKQAAEIYNQSLIELYYEIFIEGKGFANASSVEHYLSDVCYTRAAELFKNAAIASGLRNKIKSNFRLKELRNMKSGLPTTKSDNFPIPLVRQKGGQYTGFEISSHNDDFIIKIPFGRWQVKKEIDKYRPWEKFDFEQVRKSPKPISLLLSTQRRKRNKGWSKDEGTEAEIRKVMNGDYQTSYIEVKRGSKIGEKSAWMLNLSIDVPKIDKGVDPSIIGGIDVGVKSPLVCAINNAFSRYSVSDNDLFHFNKKMFARRRILLKKNRHRRAGHGAKNKLKPIAVLAKKSEGFRKKLIERWACEVADFFIKNKVGTVQMENLESMKRREDSYFNIRLRGFWPYAEMQNKIEFKLRQYGIEIRKVAPNNTSKTCSKCGHLNNYFDFEYRKKNKFPHFKCEKCNFKENADYNAALNISNPKLRSTKEEP

SEQ ID NO: 3441 - protein, 724 aa, synthetic construct
SDVEFSHEYWMRHALTLAKRARDEREVPVGAVLVLNNHVIGEGWNRAIGLHDPTAHAEIMALRQGGLVMQNYRLTDATLYVTFEPCVMCAGAMIHSRIGRVVFGVRNSRRGAAGSLMNVLNYPGMNHCVEITEGILVDECAALLCDFYCMPRQVFNAQKKAQSSISSGGSSGGSGGGETPGASESVTPKNSGGSSAGSTKNTITKTLKLRIVRPYNSAEVEKIVADEKNSREKIALERNKDKVKEACREHLKVAAYCTTQVERSACLFCKARKLDDRFYQKLRGQFPDAVFWQEISEIFRQLQKAAEIYNQSLIELYYEVLIKGKGIANASRVEHYLSDVCYTRAAELFKNAAIASGLRSKIKSNFRLKELRNMKSGLPTTKSDNFPIPLVKQKGGQCTGFEISNHNSNFIIKIPFGRWQVKKEIDKYRPWEKFDFEQVRKSPKPISLLLSTQRRRRNKGWSKDEGTEAEIRKVMYGDYQTSYIEVKRGSKIGEKSAWMLNLSIDVPKIDKGVDPSIIGGIDVGVKSPLVCAINNAFSRYSISDNDLFHFNKKVFARRRILLKKNRHRRAGHGAKNKLKPITILTEKSKRFRKKLIERWACEIADFFIKNKVGTVQMENLESMKRKEDSYFNIRLRGFWPYAEMNKIEFKLKQYGIKIKKVAPSNTSRTCSECGHLNNYFSFEYRKKNKFPHFKCEKCNFKEDADYNAALNISNPKLKGTKEEL

SEQ ID NO: 3442 - protein, 726 aa, synthetic construct
SEVEFSHEYWMRRALTLAKRARDEREVPVGAVLVLNNRVIGEGWNRAIGLHDPTAHAEIMALRQGGLVMQNYRLTDATLYVTFEPCVMCAGAMIHSRIGRVVFGVRNSKHGAAGSLMNVLNYPGMNHRVEITEGILADECAALLCDFYRMPRQVFNARKKAQSSINPGGPSGGSSGSETPDTSESATPESSGGNSGGSAKNTITKTLKLRIVRPYNSAEVEKIVADEKNNREKIALEKNKDKVKEACSEHLKVAAYCTTQVERNACLFCKARKLDDKFYQKLRGQFPDAVFWQETGEIFRQLQKQAAEIYNQSLIELYYEIFIKGRGFANASSVEHYLSDVCYTRAAELFKNAAIASGLRGKVKSNFKLKELKSMKSGLPSTKSDNFPIPLVKQKGGQYTGFEISSRNDDLIIKIPFGRWQVKKEIDRYRPWEKFDFEQVRKSPKPISLLLSTQRRKRNKGWSKDEGTEAEIRKVMNGDYQTSYIEVKRGSKIGEKSAWMLNLSIDVPKIDKGVDPSIIGGIDVGVKSPLVCAINDAFSRYSISDNDLFRFNKKMFARRRILLKKSKHKRAGHGVKNKLKPITILTEKSRRFRKKLIERWACEIANFFIKNKVGTVQMESLESMKRKGDSYFNIRLRGFWPYAEMQNKIEFKLKQYGIEIRKVAPNNTSKTCSKCGHLNNYFNFEYRKMNKFPHFKCEKCNFKENADYNAALNISNPKLKSTKEEP

SEQ ID NO: 3443 - protein, 726 aa, synthetic construct
SEVEFSHEYWMRHALTLAKRARDEREVPVGAVLVLNNRVIGEGWNRAIGMHDPTAHAEIMALRQGGLVMQNYRLVDATLYVTFEPCVLCAGAMVHSRIGRVVFGVRNSKRGAAGSLMNVLNYPGMNHRVEVTEGILADECAALLCDFYRMPRQVFNARKKARSNINSGGSSGGSSGSETLGTREGATPESSGGSSGGSAKNTITKTLKLRIVRPYNSAEVEKIVVDEKNNREKVALEKNKDKVKEACSEHLKVAAYCTTQVERSACLFCKARKLDDKFYQKLRGQFPDAVFWQEIGEIFRQLQKQAAEIYNQSLIELYYEIFIEGKGSANARSVEHYLSDVCYTRAAELFKNAAIASGLRGKVKGNFRLKELKSMKSGLPTTKSDNFPIPLVKQKGGQYTGFEISSHNDDFIIKIPFGRWQVKKEIDKYRPWEKFDFEQVRKSPKPISLLLSTQRRKKNKGWSKDEGTEAEIRRVMNGDYQTSYIEVKRGSKIGEKSAWMLNLSIDVPKIDKGVDPSIIGGIDVGVKSPLVCAINNSSSRYSICDNDLFRFNKKMFARRRILLKKNRHKRAGHGAKNKLKPITILTKKSERFRKKLIERWVCEVADFFIKNKVGTVQMENLESMKRKEDSYFNIRLRGFWPYAEMQNRIELKLKQYGIEIRRVAPNNTSRTCSKCGHLNNYFNFEYRKKSKFPHFKCEKCNFREDADYNAALNISNPKLKSTKEEP

SEQ ID NO: 3444 - protein, 725 aa, synthetic construct
SEVEFSHEYWMRHALTLARRARDGREVPVGAVLVLNNRVIGEGWNRAIGLHDPTAHAEIMALRQGGLVMQNYRLIDATLYVTFEPCVMCAGAMVHSRIGHVVFGVRNSKRGAAGSLMNVLDYPGMNHRVEITEGILADECAALLCDFYRMPRQVFNARKKAQSSINSGGSSGGSSGGETPGASGSVTPKSSGGSSAGSTKDAITKTLKLRIVRPYNSAEVEKIVADEKNNRERIALEKNKDKVKEACSEHLKVAAYCTTQVERNACLFCKARKLDDKFYQKLRGQFPDAVFWQETGEILRQLQKQAAEIYNQSLIELYYEIFIKGRGFANASSVEHYLSDVCYTRAAELFKNAAIASGLRGKVKGNFRLKELKNMKSGLPTTKSDNFPIPLVKQKGGQYTGFEISSHNDDFIIKIPFGRWQVKKEINKFRPWEKFDFEQVRKSPKPISLLLSTQRRKRNKGWSRDEGTEAEIRKVMNGDYQTSYIEVKRGSKIGEKSAWMLNLSIDVPKIDKGVDPSIIGGIDVGVKSPLVCAINNAFSRYSISDNDLFRFNKKMFARRRILLKKNRHKRAGHGAKNKLRPISILTGKSERFRKKLIERWACEIADFFIKNKVGTVQMESLESMKRKEDSYFNIRLRGFWPYAEMQNKIEFKLKQYGIEIRKVAPNNTSRTCSKCGHLNDYFNFEYRKKNKFPHFKCEKCSFKENADYNAALNISNPKLKSTKEP

SEQ ID NO: 3445 - protein, 726 aa, synthetic construct
SEVEFSHEYWMRHALALAKRARDEREVPVGAILVLNNRVIGEGWNRAIGLHDPTAHAEIMALRQGGLAMQNYRLIGATLYVTFEPCVMCAGAMIHSRIGRVVFGVRNNKHGAAGSLVNVLNYPGMNHRVEITEGILADECAALLCDFYRMPRQVFNARKKAQSSINPGGSSGGSSGSETPGTSESATPESSGGSSGGSAKNTITKALKLRIVRPYNSAEVEKIVADEKNNREKIALEKNKDKVKEACSKHLKVAAYCTTQVERDACLFCKARRLDDKFYQKLRGQFPDAVFWQEIGEIFRQLQKQAAEVYNQSLVELYYEILIKGKGIANASSVEHYLSDVCYTRAAELFKNAAIASGLRNKIKSNFRLKELRNMKSGLPTTKSDNFPIPLVKQKGGQCTGFEISSPNDDFIIKIPFGRWQVKKEIDKYRPWEKFDFEQVRKSPKPISLLLSTQRRKRYKGWSKDEGTEAEIRKVMNGDYQTSYIEVKRGSKTGEKSAWMLNLSIDVPKIDKGVDPSIIGGIDVGVKSPLVCAINNAFSRYSISDNDLFRFNKKMFARRRILLKKNRHKRAGHGAKNKLKPISILTGKSERFRKKLIERWACEIADFFIKNKVGTVQMENLESMKRKEDSYFNIRLRGFWPYAEMQNKIEFKLKQYGIEIRKVAPNNTSKTCSKCGHLNNYFNFEYRKKNKFPHFKCERCNFKENADYNAALNISNPKLKSTKEKP

SEQ ID NO: 3446 - protein, 726 aa, synthetic construct
SEVEFSHEYWMRHALTLAKRARDEREVPVGAVLVLNNRVIGEGWNRAIGLHDPTAHAEIMALRQGGLVLQNYRLVDATLYVTFEPCVLCAGAMVHSRIGRVVFGARNSKRGAAGSLMNILNYPGMNHRVEITEGILADECAALLCDFYRMPRQVFNAQKKAQSSINSGGSSGGSSGSETPSTSESATPESSGGSSGGSAKSTITKTLQLRIVRPYNSAEVEKIVTDEKNNREKIALEKNKDKVKEACSEHLKVAAYCTTQVERSACLFCKARKLDDKFYQKLRSQFPDAVFWQEIGEIFRQLQKQAAEIYNQSLIELYYEIFIKGKGIASTSRVGHYLSDVCYTRAAELFKNAAIASGLRGKVKSNFRLKELRNMKSGLPTTKSDNFPIPLVRQKGGQYTGFEISNHDGDFIIKIPFGRWQVKKEINKHRPWEKFDFEQVRKSPKPISLLLSTQRRKRNKGWSKDEGTEAEIRKVMNGDYQTSYIEVKRGSKIGEKSAWMLSLSIDVPKIDKGVDPSIVGGIDVGVKSPLVCAINNALGRFSISDNDLFHFNKKMFARRRILLRKNRHKRAGHGAKNKLKPISILTEKSRRFRKKLIERWACEIADFFIKNKVGTVQMEDLESMKRRGDSYFNIRLRGLWPYAEMQNKIEFKLKQYGIEIRKVAPNNTSKTCSKCGHLNNYFNFEYRKKNKFPHFKCEKCNFKENADYNAALNISNPKLKNTKEEP

SEQ ID NO: 3447 - protein, 726 aa, synthetic construct
SEVEFSHEYWMRHALTLAKRARDEREVPVGAILVLNNRVIGEGWNRAIGLHDPTAHAEIMALRQGGLVMQNYRLIDATLYVTFEPCVMCAGAMIHSRIGRVVFGVRNSKHGAAGSLVNVLNYPGMNHRVEITEGILADECAALLCDFYRMPRQVFNARKKAQSSINPSGSSGGSSGSVTPGTSESATSESSGGGFGGSAKNAITKTLQLRIVRPYNSAEVEKIVADEKNNREKIALEKNKDKVKEACSKHLKVAAYCTTQVERNACLFCKARKLDDKFYQKLRGQFPDAVFWQEVGEIFRQLQKQAAEIYNQSLIELYYEIFIKGKGIANASSVGHYLSDVCYTRAAELFKNAAIASGLRGKVKSNFKLKELKSMKSGLPSTKSDNFPIPLVKQRGGQYTGFEISSHNDDFIIKIPFGRWQAKKEIDKYRPWEKFDFEQVRKSPKPISLLLSTQRRKRNRGWSKDEGTEAEIRKVMNGDYQTSYIEVKRGSKIGEKSAWMLNLSIDVPKIDKGVDPSIIGGIDVGVKSPLVCAINNAFSRYSISDNDLFRFNKKMFARRRILLGKNRHKRAGHGVKNKLKPITILTEKSGRFRKKLIERWACEIADFFVKNKVGTVQMENLESMKRKEDSYFNIRLRGFWPYAEMQNKIEFKLKQYGIKVRKVAPNNTSKTCSKCGHLNNYFSFEYRKKNKFPHFKCEKCNFKENADYNAALNISNPKLKSTKEEP

SEQ ID NO: 3448 - protein, 726 aa, synthetic construct
SEVEFGHEYWMRHALTLAKRARDEREVPVGAILVLNNRVIGEGWNRAIGQHDPTAHAEIMALRQGGLVMQNYRLIDATLYVTFEPCVMCAGAMIHSRIGRVVFGVRNSKHGAAGSLVNVLNYPGMNHRVGITEGILADECAALLCDFYRMPRQVFNARKKAQSIINPGGSSGGSSCSETPGASESVTPKSSGGSSAGSTKSTITKTLKLRIVRPYNSAEVEKIVADEKNSREKIALEKNKDKVKEACSEHLKVAAYCTTQVERNACLFCKARKLDDRFYQKLRGQFPGAMFWQEIGEIFRQLQKQAAEIYNQSLIELYYEIFIKGKGFANASSVEHYLSDVCYTRAAELFKNAAIASGLRGKVKSNFRLKELKNMKSGLPTTKSDNFPIPLVKQKGGQYTGFEVSSHNGDFIIKIPFGRWQVKKEIDKYRPWEKFDFEQVRKSPRPISLLLSTQRRKRNKGWSKDEGTEAEIRKVMNGDYQTSYIEVKKGSKIGEKSAWMLNLSIDVPKIDKGVDPSIIGGIDVGVKSPLVCAIDNAFSRYSISDNDLFHFNKKMFAKRRILLKKNRHKRAGHGAKNKLKPISILTEKSERFRKKLIERWACEIADFFIKNKVGTVQMENLESMKRKEDSYFNIRLRGFWPYAEMQNKIVFKLKQYGIEIRKVAPNNTSRTCSKCGHLNNYFNFEYRKMNKFPHFKCEKCNFKENADYNAALNISNPKLKSTKEEP

SEQ ID NO: 3449 - protein, 726 aa, synthetic construct
SEVEFSHEYWMRHALTLAKRARGEREVPVGAILVLNNRVIGEGWNRAIGLHDPTAHAEIMALRQGGLVMQNYRLVNATLYVTFEPCVMCAGAMIHSRIGRVVFGVRNSKRGAAGSQMNVLNYPGMNHRVEITEGILTDECAALLCDFYRMPRQVFNAQKKAQSTINSGGSSGGSSGSGTPGTSESPTPESSGGSPGGSAKNTITKTLKLRIVRPYNSAEVEKIVADEKNNREKVALEKNKDKVKEACSKHLKVAAYCTTQVERNACLFCKARKLDDKFYQKLRGQFPDAVFWQEIGEIFRQLQRQAAEIYNQSLIELYYEIFIKGKGSANASSVEHYLSDVCYTRAAEQFRNAAIASGLRGKVKSNFRLKELKNMKSGLPTTKSDNFPIPLVKQKGGQYTGFEISSHSDDFIIKIPFGRWQVRKEIDKYRPWEKFDFEQVRKSPKPISLLLSTQRRKRNKGWSKDEGTEAEIRKVMNGDYQTSYIEVKRGSKAGEKSAWMLNLSIDVPKIDKGVDPSIIGGIDVGVKSPLVCAINNALSRYSISDNDLFHFNKKMFARRRILLGKNRHKRAGHGVKNKLKPITILTEKSGRFRKKLIERWACEIADFFVKNKVGTVQMENLESMKRKEDSYFNIRLRGFWPYAEMQNKIEFKLKQYGIEIRKVAPNNTSKTCSKCGHLNNYFNFEYRKKNKFPHFKCEKCNFKENADYNAALNISNPMLKSTKEEP

SEQ ID NO: 3450 - protein, 727 aa, synthetic construct
SEVEFSHEYWMRHALTLAKRARDEREVPVGAILVLNNRVIGEGWNRAIGLHDPTAHAEIMALRQGGLVMQNYRLIDATLYVTFEPCVMCAGAMIHSRIGRVVFGVRNNKHGAAGSLVNVLNYPGMNHRVEITEGILADECAALLCDFYRMPRQVFNARKKAQSSINPGGSSGGSSGSDTPGTSESATPESSGGGSSGSAKNTITKTLQLRIVRPYNSAEVEKIVADEKNNREKIALEKNKDKVREACSKHLKVASYCTTQVERNACPFCKARKLDDKFYQKLRGQFPDAVFWQELGEILRQLQKQAAEIYNQSLIELYYEIFIKGRGFANASSVEHYLSDVCYTRAAELFKNAAIASGLRGKVKGNFRLKELKNMKSGLPTTKSDNFPVPLVKQKGGQYTGFEISSHNDDFIIKIPFGRWQVKKEIDKYRPWEKFDFEQVRKSPKPISLLLSTQRRKRNKGWSKDEGTEAEIRKVMNGDYQTSYIEVKRGSKIGEKSAWMLSLSIDVPKIDKGVDPSIIGGIDVGVKSPLVCAINNAFCRYSISDNDLFHFNKKMFARRRILLKKSRHKRAGHGAKNKLKPISILTEKSKRFRKKLIERWACEIADFFIKNKVGTVQMENLESMKRKEDSYFNIRLRGFWPYAEMQNKIEFKLKQYGIKIRKVAPNNTSKTCGKCGHLNNHFSFEYRRKNKFPHFKCEKCNFKEDADYNAALNISNPKLKSTKEEPQ

SEQ ID NO: 3451 - protein, 726 aa, synthetic construct
SEVEFSHEYWMRHALTLAKRARDEREVPVGAILVLNNRVIGEGWNRAIGLHDPTAHAEIMALRQGGLVMQNYRLIDATLYVTFEPCVMCAGAMIHSRIGRVVFGVRNSKHGAAGSLVNVLNYPGMNHRVEITEGILADECAALLCDFYRMPRQVFNARKKAQSSINPSGSSGGSSGSVTPGTSESATPESSGGGFGNSAKNTITKTLQLRIVRPYNSAEVEKIVADEKNNREKIALEKNKDKVKEACNKHLKVASYCTTQVERNACLFCKARKLDDKFYQKLRGQFPDAVFWQELGEIFRQLQKQAAEIYNQSLIELYYEIFIKGKGLANASSVEHYLSDVCYTRAAELFKNAAIASGLRGKVKSNFKLKELKSMKSGLPSTKSDNFPIPLVKQKGGQYTGFEISSHNDDLIIKIPFGRWQVKREIDKYRPWEKFDFEQVRKNPKPISLLLSTQRRKGNKGWSKDEGTEAEIRRVMNGDYQTSYIEVKRGSKIGEKSAWMLNLSIDVPKIDKGVDPSIIGGIDVGVKSPLVCAINNAFSRYSISDNDLFRFNKKMFARRRILLKKNRHKRAGHGAKNKLKPITILTEKSGRFRKKLIERWACEIADFFIKNKVGTVQMENLESMKRKEDSYFNIRLRGFWPYAEMQSKIELKLKQYGFKIRKVAPNNTSKTCSKCGHLNDYFNFEYRKKNKFPHFKCEKCNFKENADYNAALNISNPKLKGTKEEP

SEQ ID NO: 3452 - protein, 726 aa, synthetic construct
SEVEFSHEYWMRHALTLAKRARDEREVPVGAILVLNNRVIGEGWNRAIGLNDPTVHAEIMALRQGGLVMQNHRLTDATLYATFEPCVMCAGAMIHSRIGRVVFGVRNSKHGAAGSLMNVLNYPGMNHRVEITEGILADECAGLLCDFYRMPRQVFSARKKAQSSTNPGGSSGGSSSGKAPGTCESATLESSGGSSGGSAKNSITKALKLRIVRPYNSAEVEKIVADEKNNREKTALEKNKGKVKEACSKHLKVATYCTTQVERNACLFCKARKLDDKFYQKLRGQFPDAVFWQEIGEIFRQLQKQAAEIYNQSLIELYYEIFIEGKGSANARSVEHYLSDVCYTRAAELFKNAAIASGLRGKVKSNFRLKELKNMKSGLPTTKSDNFPIPLVKQKGGQYTGFEISSHNDDFIIKIPFGRWQAKKEIDKYRPWEKFDFEQVRKSPKPISLLLSTQRRKRNKGWSKDEGTEAEIRKVMNGDYQTSYIEVKRGSKIGEKSAWMLNLSIDVPKIDKGVDPSIIGGIDVGVKSPLVCAINNAFSRYSISDNDLFHFNKKMFARRRILLKKNRRRRAGHGAKNKLKPITILTEKSVRFRKKLIERWACEIADFFIKNKVGTVQMENLESMKRKEDSYFNIRLRGFWPYAEMQNKIEFKLKQYGIEIRRVAPNNTSRTCSKCGHLNNYFNFEYRRKYKFPHFKCEKCNFKENADYNAALNISNPKLKSTKEEP

SEQ ID NO: 3453 - protein, 726 aa, synthetic construct
SEVEFSHEYWMRHALTLAKRARDEREVPVGAVLVLNNRVIGEGWNRAIGLHDPTAHAEIMALRQGGLVMQNYRLIDATLYVTFEPCVMCAGAMIHSRIGRVVFGVRNSKHGAAGSLVNVLNYPGMNHRIEITEGILADECAALLCDFYRMPRQVFNARKKAQSSINSGGSSGGSSGSETPGTSESATPKNSGGSSGGSAKNTITKALKLKIVRPYNSAEVEKIVADEKNNRERIALEKNKDKVKEACSKHLKVAAYCTTQVERNACLFCKARKLDDKFYQKLRGQFPDAVFWQEIGEIFRQLQKQAAEIYNQSLIELYYEIFIEGKGSASARSVEHYLSDVCYTRAAELFKNAAIASGLRGKVKGNFRLKELKNMKSGLPTTKSDNFPIPLVKQKGGQYTGFEISSHNDDFIIKIPFGRWQVKKEIDKYRPWEKFDFAQVRKSPKPISLLLSTQRRKRNRGWSKDEGTEAEIRKVMNGDYQTSYIEVKRGSKIGEKSAWMLNLSIDVPKIDKGVDPSIIGGIDVGVKSPLVCAINNAFSRYSISDNDLFHFNKKMFARRRILLKKSKHKRAGHGAKNKLKPITVLTKKSERFRKKLIERWVCEVADFFIKNKVGTVQMENLESMKRKEDSYFNIRLRGFWPYAEMQNKIEFKLKQYGIKIRKVAPNNTSKTCSKCGHLNNYFSFEYRKRNKFPHFKCEKCNFKENADYNAALNISNPKLKGTKEEP

SEQ ID NO: 3454 - protein, 726 aa, synthetic construct
SEDEFSHEYWMRHALTLAKRARDGREVPVGAVLVLNNRVIGEGWNRAIGLHDPTAHVEIMALRQGGLVMQNYRLIDATLYVTFEPCVMCAGAMVHSRIGRVVFGVRNSKRGAAGSLMNVLNHPGMNHRVEITGGILADECAALLCDFYRMPRQVFNAQKKARSNINSGGSSGGSSGSETLGTSESATPESSGGSSGGSAKNTITKTLQLRIVRPYNSAEVEKIVADEKNNREKIALEKNKDKVKEACSKHLKVASYCTTQVERNACPFCKARKLDDKFYQKLRGQFPDAVFWQELGEILRQLQKQAAEIYNRSLIELYYEIFIKGRGFANASSVEHYLSDVCYTRAAELFKNAAIASGLRGKVKSNFRLKELKNMKSGLPTTKSDNFPIPLVKQKGGQYTGFEISRHNDDFIIKIPFGRWQVKKGIDKYRPWEKFDFEQVRKSPKPISLLLSTQRRKRNKGWSKDEGTEAEIRKVMNGDYQTSYIEVKRGSKTGEKSTWMLNLSIDVPKIDKGVDPSIIGGIDVGVKSPLVCAINNAFSRYSISDNDLFRFNKKMFARRRILLKKNRYKRAGHGAKNKLRPISILTGKSERFRKKLIERWACEIADFFIKNKVGTVQMENLESMKRKEDSYFNIRLRGFWPYAEMQNKIEFKLKQYGIEIRKVAPNNTSKTCSKCGHLNNYFNFEYRRKNKFPHFKCEKCNFKEDADYNAALNISNPKLKSTKEEP

SEQ ID NO: 3455 - protein, 726 aa, synthetic construct
SEVEFSHEYWMRHALTLAKRARDEREVPVGAVLVLNNRVIGVGWNRAVGLHDPTAHAEIMALRQGGLVMQNYRLIDATLYVTFEPCAMCAGAMVHSRIGRVVFGVRNSKRGAAGSLMNVLDYPGMGHRVEITEGILADECAALLCDFYCMPRQVFNAQKRAQSSINSGGSSGGSSGSETPGASGSVIPKSSGGSSAGSTKDTITKTLKLRIVRPYNSAEVEKVVADEKNNREKIAMEKNKDKVKEACSEHLKVAAYCTTQVERNACLFCRARKLDDRFYQKLRGQFPDAVFWQEIGEIFRQLQKQAAEIYNQSLIELYYEIFIKGKGFANASSVEHYLSDVCYTRAAELFKNAAIASGLRGKVKSNLRLKELKNMKSGLPTTKSDNFPIPLVKQKGGQYTGFEISSHNDDFIIKIPFGRWQVKKEIDKYRPWEKFDFEQVRKSPKPISLLLSTQRRKRNKGWSKDEGTEAEIRKVMNGDYQTSYIEVKRGSRIGEKSAWMLSLSIDVPKIDRGVDPSIIGGIDVGVKSPLVCAINNGLNRYSISDNDLFHFNKKMFARRRILLKKNRHRRAGHGARNKLKPITVLTEKSKRFRKKLIERWACEIANFFVKNKVGTVQMENLESMKRKEDSYFNIRLRGLWPYAEMQNKIEFKLKQYGIEVRKVAPNNTSKTCSKCGHLNNYFNFEYRKRNKFPHFKCEKCNFKENADYNAALNISNPKLKGTKEEP

SEQ ID NO: 3456 - protein, 726 aa, synthetic construct
SEVEFSHGYWMRHALTLAKRARDEREVPVGAVLVLNNRVIGVGWNRAVGLHDPTAHAEIMALRQGGLVMQNYRLIEATLYVTFEPCIMCAGAMIHSRIGRVVFGVRNSKRGAAGSLMNVLNYPGMNHRVEITEGILADECAALLCDFYRVPRQVFNAQKKARSDINSGSSSGGSSGSETPGTSESATPESSGGDSGGSAKNTITKALKLRIVRPYNSAEVEKIVADEKSNREKIALEKNKDKVKEACSEHLKVAAYCTTQVERNACLFCKARKLDDKFYQKLRGQFPDAVFWQEISEIFRQLQKQTAEIYNQSLIELYYEIFIKGKGFANASSVEHYLSDVCYTRAAELFKNAAIASGLRGKVKSNFRLKELKNMKSGLPTTKSDNFPIPLVRQKGGQYTGFEISNHDGDFIIKIPFGRWQVKKEINKHRPWEKFDFEQVRKSPKPISLLLSTQRRKRNKGWSKDEGTEAEIRKVMNGDYQTSYIEVKRGSKIGEKSAWMLNLSIDVPKIDKGVDPGIIGGIDVGVKSPLVCAINNASSRYSISDNDLFHFNKKMFARRRILLKKNRHKRAGHGAKNKLKPITIMTEKSKRFRKKLIERWACEIADFFIKNQVGTVQMENLESMKRKEDSYFNIRLRGFWPYAEMQNKIEFKLKQYGIEIRKVAPNNTSKTCSKCGHLNNYFNFEYRKKNKFPHFKCEKCNFKEDADYNAALNISNPKLKSTKEEP

SEQ ID NO: 3457 - protein, 726 aa, synthetic construct
SEVEFSHEYWMRHALTLAKRARDEREVPVGAVLVLDNRVIGEGWNRAIGLHDPTAHAEIMALRQGGLVMQNYRLIDATLYVTFEPCVMCAGAMVHSRIGRVVFGVRNNKRGAAGSLMNVLDYPGMDHRVEITEGILADECAALLCDFYRMPRQVFNAQRKAQSSINSGGSSGGSSGSETPGTSESATPESSGGSSGGSAKNTITKTLQLRIVRPYNSAEVEKIVADEKNSREKIALEKNKDKVKEACSKHLMVASYCTTQVERSACLFCKARELDDKFYQKLRGQFPDAVFWQELGEILRQLQKQAAEIYNQSLIELYYEIFIKGRGFANASSVEHYLSDVCYTRAAELFKNAAIASGLRGKVKSNFRLKELKNMKSGLPTTKSDNFPIPLVKQKGGQYTGFEISSHNDDFIIKIPFGRWQVKKEIDKYRPWEKFDFEQVRKSPKPISLLLSTQRRKRNKGWSKDEGTEAEIRKVMNGDYRTSYIEVKRGSKTGEKSAWVPNLSIDVPKIDKGVDPSIIGGIDVGVKSPLVCAINNAFSRYSISDNDLFRFNKKMFARRRILLKKNRHKRAGHGAKNKLKPISILTGKSERFRKKLIERWACEIADFFIKNKVGTVQMENLESMKKKEDSYFNIRLRGFWPYAEMQNRIEFKLKQYGIEIRKVAPNNTSKTCSKCGHLNNYFNFEYRKKNKFPHFKCEKCNFKENADYNAALNISNPKLKSTKEEP

SEQ ID NO: 3458 - protein, 726 aa, synthetic construct
SEVEFSHEYWMRHALTLAKRARDEREVPVGAVLVLNNRVIGEGWNRAIGLHDPTAHAEIMALRQGGLAMRNYRLVDATLYVTFEPCVLCAGAMVHSRIGRVVFGVRNSKRGAAGSLMNVLNHPGMNHCVEITEGILVDECAALLCDFYRMPRQVLNAQKKAQSSISSGGSSGGSSGSVTPGTSESATPESSSGGLGGSAKNTITKTLQLRIVRPYNSAEVEKIVADEKNNREKIALEKNKDKVKEACSKHLKVASYCTTQVERNACPFCKARKLDDKFYQKLRGQFPDAVFWQEIGEIFRQLQKQAAEIYNQSLIELYYEIFIKGKGLANASSVEHYLSDVCYTRAAELFKNAAIASGLRGKVKSNFKLKELKSMKSGLPSTKSDNFPIPLVKQRGGQYTGFEISSHNDDFIIKIPFGRWLAKKEIDKYRPWEKFDFEQVRKSPKPISLLLSTQRRRRNKGWSKDEGTEAEIRKVMNGDYQTSYIEVKRGSKIGEKSAWMLNLSIDVPKIDKGVDPSIIGGIDVGVKSPLVCAIDNAFSRYSISDNDLYRFNKKMFARRRILLKKNRRKRAGHGAKNKLKPISILTGKGERFRKKLIERWACEIADFFIKNKVGTVQMENLESMKRKEDSYFNIRLRGFWPYAEMQNKIELKLKQYGIKIRKVAPNNTSKTCSKCGHLNDYFNFEYRKKNKFPHFKCEKCNFKEDADYNAALNISNPKLKSTREEP

SEQ ID NO: 3459 - protein, 726 aa, synthetic construct
SEVEFSHEYWMRHALILARRARDEREVPVGAVLVLNNRVIGEGWNRAIGLHDPTAHAEIMALRQGGLVMQNYRLIDATLYVTFEPCVMCAGAMIHSRIGRVVFGVRNSKRGAAGSLMNVLNYPGMDHRVEITEGILTDECAALLCDFYRMPHQVLNAQKKAQSSTNSSGSSGGSSGSETPGTGGSATPEGSSGSSGGFAKSTITKTLKLRIVRPYNSAEVEKIVADEKNNREKIALEKNKGKVKEACSKHLKVATYCTTQVERNACLFCKARKLDDKFYQKLRGQFPDAVFWQELGEIFRQLQKQAAETYNQSLIELYYEIFIKGKGFANASSVEHYLSDVCYTRAAELFKNAAIASGLRGKVKSNFRLKELKNMKSGLPTTKSDNFPIPLVKQKGGQYTGFEISSHNDDFIIKIPFGRWQVKEEIDKYRPWEKFDFEQVRKNPKPISLLLSIQRRKRNKGWSRDEGTEAEIRKVMNGDYQTSYIEVKRGSKIGEKSAWMLNLSIDVPKIDKGVDPSIIGGIDVGVKSPLICAINNAFSRYGISDNDLFRFNKKVFARRRILLKKNRHKRAGHGTKNKLKPITILAEKSGRFRKKLIERWACEIANFFIKNKVGTVQMENLESMKRKEDSYFNIRLRGFWPYAEMQNKIEFKLKQYGIEIRKVAPNSTSKTCSKCGHLNIYFNFEYRKKNKFPHFKCEKCNFKENADYNAALNISNPKLKSTKEEP

SEQ ID NO: 3460 - protein, 726 aa, synthetic construct
SEVEFSHEYWMRHALTLAKRARDEREVPVGAILVLNNRVIGEGWNRAIGLHDPTAHAEIMALRQGGLVMQNYRLIDATLYVTFEPCVMCAGAMIHSRIGRVVFGARNSKRGAAGSLMNVLSYPGMNHRVEITEGVLADECAALLSDFYRMPRRVFNAQKKAQSSINSGGSSGGSSGSETPGTSESATPKNSGGSSGGSAKNTITKALKLKIVRPYNSAEVEKIVADEKNNRERIALEKNKDKVKEACSKHLKVAAYCTTQVERNACLFCKARKLDDKFYQKLRGQFPDAVFWQEIGEIFRQLQKQAAEIYNQSLIELYYEIFVKGKGFANASSVEHYLSDVCYTRAAELFKNAAIASGLRGKVKSNFRLKELKNMKSGLPTTKSDNFPIPLVKQKGGQYTGFEISSHNDDFIIKIPFGRWQVKEEIDRYRPWEKFDFEQVRKNPKPISLLLSTQRRKRNKGWSKDEGTKAEIRKVMNGDYRTSYIEVKRGSKTGEKSAWMLNLSIDVPKIDKGVDPSIIGGIDVGVKSPLVCAVNNAFSRYSISDNDLFRFNKKMFARRRILLKKNRHKRAGHGAKNKLKPISILTGKSERFRKKLIERWACEIADFFIKNKVGTVQMENLESMKRKEDSYFNIRLRGFWPYAEMQNKIEFKLKQYGIEIRKVAPNNTSKTCSKCGHLNNYFNFEYRKKNKFPHFKCEKCNFKENADYNAALNISNPKLKSTTEEP

SEQ ID NO: 3461 - protein, 726 aa, synthetic construct
SEVEFSHEYWMRHALTLAKRARDEREVPVGAVLVLNNRAIGEGWNRAIGLHDPTAHAEIMALRQGGLVMRNYRLTDATLYVTFEPCVMCAGAMIHSRIGRVVFGVRNSKRGAAGSLMNVLDYPGMGHRVEITEGILADECAALLCDFYCMPRQVFNARKKAQSSINSGGSSDGGSGSETPGTSESATPESSGGSSGGSAKNTITKTLKLRIVRPYNSAEVEKIVADEKNNREKIALEKNKDKVKEACSEHLKVAAYCTTQVERSACLFCKARKLDDKFYQKLRGQFPDAVFWQEIGEIFRQLQKQAAEIYNQSLIELYYEIFIKGKGSANASSVEHYLSDVCYTRAAEQFKNAAIASGLRGKVKSNFRLKELKNMKSGLPTTKSDNFPIPLVKQKGGQYTGFEISSHSDDFIIKIPFGRWQVRKEIDKYRPWEKFDFEQVRKSPRPISLLLSTQRRKRNKGWSKDEGTEAEIRKVMNGDYQTSYIEVKRGSKIGEKSAWMLNLSIDVPKIDKGVDPSIIGGIDVGVKSPLICAINNALSRYSISDNDLFRFNKKMFARRRILLKKNRHKRAGHGAKNKLKPITILTKKSERFRKKLIERWVCEVADFFIKNKVGTVQMENLESMKRKEDSYFNIRLRGFWPYAEMQNRIELKLKQYGIEIRKVAPNNTSKTCSKCGHLNSYFNFEYRKKNKFPHFKCERCNFKENADYNAALNISNPKLKSTKEEP

SEQ ID NO: 3462 - protein, 726 aa, synthetic construct
SEVEFSHEYWMRHALTLAKRARDEREVPVGAILVLNNRVIGEGWNRTTGLHDPTAHAEIMALRQGGLVMQNHRLVDATLYVTFEPCVMCAGAMIHSRIGRVVFGARNSKRGAAGSLMNVLSYPGMNHRVEVTEGILADECAALLCDFYRMPRQVFNARKKAQSSINSGGSSGGSSGSETPGTRESATPKSSGGSSGGSAKNTVTKALKLRIVRPYNSAEVEKIVADEKNNREKIALEKNKDKVKEACSKHLKVAAYCTTQVERNACLFCKARKLDDKFYQKLRGQFPDAVFWQELGGIFRQLQKQAAEIYNQSLIELYYEIFIKGKGITNASSVEHYLSDVCYTRAAELFKNAAIASGLRGKVKSNLRLKELKNMRSGLPTTKSDNFPIPLVKQKGGQYTGFEISSHNSDFIIKIPFGRWQEKEEIGKYRPWEKFDFEQVRRSPKPISLLLSTQRRKKNKGWSKDEGTEAEIRKVMNGDYQTSYIEVKRGSKIGEKSAWMLNLSIDVPKIDKGVDPSIIGGIDVGVKSPLVCAVNNALSRYSISDNDLFHFNKKMFARRRILLKKNRHRRAGHGAKNKLKPIAVLTEKSEGFRKKLIERWACEVADFFIKNKVGTVQMENLESMKRREDSYFNIRLRGFWPYAEMQNKIEFKLRQYGIEIRKVAPNNTSKTCSKCGHLNDYFNFEYRKKNKFPHFKCEKCNFKEDADYNAALNISNPKLKSTREEP

SEQ ID NO: 3463 - protein, 726 aa, synthetic construct
SEVEFSHEYWMRRALTLAKRARDEREVPVGAVLVLNNRVIGVGWNRAVGLHDPTAHAEIMALRQGGLVMQNYRLIEATLYVTFEPCIMCAGAMIHSRIGRVVFGVRNSKRGAAGSLMNVLNYPGVNHRVEITEGILADECAALLCDYYRMPRQVFNARKKAQSSINSGGSSDGSSGSETPGTSESATPKSSGGSSAGSTKNTITKTLKLRIVRPYNSAEVEKIVADEKNSREKIALERNKDKVKEACSEHLKVAAYCTTQVERNACLFCKARKLDDKFYQKLRGQFPDAVFWQEISEIFRQLQKQAAEIYNQSLIELYYEIFIKGRGFANTSSVEHYLSDVCYTRAAELFKNAAIASGLRGKVKSNFRLKELKSMKSGLPTTKSDNFPIPLVKQKGGQYTGFEISSHNDDFIIKIPFGRWQEKKEINKYRPWEKFDFEQVRKSPKPISLLLSTQRRKGNKGWSKDEGTEAEIRKVMNGDYQTSYIEVKRGSKIGEKSAWMLNLSIDVPQIDKGVDPSIIGGIDVGVKSPLVCAINNAFSRYSISDNDLYRFNKKMFARRRILLKKNRHKRAGHGAKNKLKPISILTGKSGRFRKKLIERWACEIADFFIKNKVGTVQMENLGSMKRREDSYFNIRLRGFWPYAEMQNKIELKLKQYGIEIRKVAPNNTSKTCSKCGHLNNYFDFEYRKKNKFPHFKCEKCSFKENADYNAALNISNPKLKSTKEEP

SEQ ID NO: 3464 - protein, 726 aa, synthetic construct
SEVEFSHEYWMRHALTLAKRARDEREVPVGAVLVLNNRVIGEGWNRAIGLHDPTAHAEIMALRQGGLVMQNYRLSDATLYVTFEPCVMCAGAMIHSRIGRVVFGVRNSKRGAAGSLMNVLNYPGMNHCVEITEGILVGECAALLCDFYRMPRQVLSAQKKAQSSVSSGGSSGGSSGSETPGASGSVTPKSSGGSSAGSTKDTITKTLKLRIVRPYNSAEVEKIVADEKNNREKIALEKNKDKVKEACSKHLKVASYCTAQVERNACPFCRARKLDDKFYQKLRGQFPDAVFWQEIGGIFRQLQKQAAEIYNQSLIELYYEIFIKGKGIANASSVEHYLSDVCYTRAAELFKNAAIASGLRNKIKSNFRLKELRNMKSGLPTTKSDNFPIPLVRQKGGQYTGFEISSHNDDFIIKIPFGRWQVKEEIDKYRPWEKFDFEQVRKNPKPISLLLSTQRRKRNKGWSKDEGTEAEIRKVMNGDYQTSYIEVKRGSKIGEKSAWMLNLSIDVPRIDKGVDPSIIGGIDVGVKSPLVCAINNAFSRYSISDNDLFRFNKKMFARRRILLGKNRHKRAGHGVKNKLKPISILTERSRRFRKKLIERWACEIADFFIRNKVGTVQMENLESMKRKEDSYFNIRLRGFWPYAEMQNKIEFKLKQYGIEIRKVAPNNTSRTCSECGHLNNYFNFEHRKKNKFPRFKCEKCNFKENADYNAALNISNPKLKSTKEEP

SEQ ID NO: 3465 - protein, 726 aa, synthetic construct
SEVEFSHEYWMRHALSLAKRARDEREVPVGAVLVLNNRIIGEGWNRAIGLHDPTAHAEIMALRQGGLVMQNYRLTDATLYVTFEPCVMCAGAMVHGRIGRVVFGVRNSKRGAAGSLMNVLNYPGVNHCVEITEGILVDECAALLCDFYRMPRQVLNAQKKAQSSISSGGSSGGCSGSEMPGASESVTPKSSGGSSAGSTKNTITKTLKLRIVRPYNSAEVEKIVADEKNSREKIALERNKDKVKEACSEHLKVAAYCTTQVERNACLFCKARKLDDRFYQKLRGQFPDAVFWQETGEIFRQLQRQAAEIYNQSLIELYYEIFIKGKGFANASSVEHYLSDVCYTRAAELFKNAAIASGLRGKVKSNFRLKELKNMKSGLPTTKSDNFPIPLVKQKGGQYTGFEISNHHDDFIIKIPFGRWQVKKEIDKYRPWEKLDFEQVRKSPKPISLLLSTQRRKRNKGWSKDEGTEAEIRKVMNGDYQTSYIEVKRGSKIGEKSAWMLNLSIDVPKIDRGVDPSIIGGIDVGVKSPLVCAINNGLSRYSISDNDLFHFNKKMFARRRILLKKNRHRRAGHGARNKLKPITVLTEKSKRFRKKLIERWACEIANFFVKNKVGTVQMENLESMKRREDSYFNIRLRGFWPYAKMLNKIEFKLKQYGIKVRKVAPNNTSKTCSKCGHLNNYFSFEYRKKNKFPHFKCEECNFKENADYNAALNISNPKLKSTKEES

SEQ ID NO: 3466 - protein, 726 aa, synthetic construct
SEVEFSHEYWMRHALTLARRARDEREVPVGAVLVLNNRVIGEGWNRAIGLHDPTAHAEIMALRQGGLVTRNYRLIDATLYVTFEPCVMCAGAMIHSRISRVVFGVRNSKRGAAGSLMNVLNYPGMNHRVGITEGILADECAALLCDFYRMPRRVLNAQKKAQSSISSGGSSGGSSGGETPGASGSVTPKSSGGSSAGSTKDAITKTLKLRIVRPYNSAEVEKIVADEKNNREKIAMEKNKDKVKEACSEHLKVAAYCTTQVERNACLFCKARKLDDKFYQKLRGQFPDAVFWQEIGEIFRQLQKQAAEIYNQSLVELYYEILIKGKGFANASSVEHYLSDVCYTRAAELFKNAAIASGLRGKVKSNFRLKELKNMKSGLPTTKSDNFPIPLVKQKGGQYTGFEISSHHDDLIIKIPFGRWQVKEEIDKYRPWEKFDFEQVRKSPKPISLLLSTQRRKKNKGWSKDEGTEAEIRRVMNGDYQTSYIEVKRGSKIGEKSAWMLNLSIDVPKIDKGVNPSIIGGIDVGVKSPLVCAINNSSSRYSICDNDLFRFNKKMFARRRILLKKNRHKRAGHGAKNKLKPITILTKKSERFRKKLIERWVCEVADFFIKNKVGTVQMENLESMKRKEDSYFNIRLRGFWPYAEMQNRIELKLKQYGIEIRRVAPNNTSRTCSKCGHLNNYFNFEFRKKNKFPHFKCEKCNFKEDADYNAALNISNPKLKSTKEEP

SEQ ID NO: 3467 - protein, 726 aa, synthetic construct
SEVEFSHEYWMRHALTLAKRARDEREVPVGAVLVLNNRAIGEGWNRAIGLHDPTAHAEIMALRQGGLVMQNYRLTDATLYVTFEPCVMCAGAMIHSRIGRVVFGVRNSKRGAAGSLMNVLNYPGMNHCVEITEGILVDECAALLCDFYRMPRQVLNAQKKAQSSISSGGSSGGSSGSETPGASGSVIPKSSGGSSAGSAKNTITKTLKLRIVRPYNSAEVEKIVADEKNNREKIALEKNKDKVREACSKHLKVASYCTTQVERNACPFCKARKLDDKFYQKLRGQFPDAVFWQELGEILRQLQKQAAEIYNQSLIELYYEIFIKGRGFANASSVEHYLSDVCYTRAAELFKNAAIASGLRGKVKSNFRLKELKNMKSGLPTTKSDNFPIPLVKQKGGQYTGFEISSHNDDFIIKIPFGRWQVKKEIDKYRPWEKFDFEQVRKSPKPISLLLNTQRRKRNKGWSKDEGTEAEIRKVMNGDYQTSYIEVKRGSKAGEKSAWMLNLSIDVPKIDKGVDPSIIGGIDVGVKSPLVCAINNAFGRYSISDNDLFHFNKKMFARRRILLKRNRHKRAGHGAKNKLKPITILTEKSKRFRRKLIERWACEIADFFIKNKVGTVQMENLESMKRKEDSYFNIRLRGFWPYAEMQDKIEFKLKQYGIEIRKVAPNNTSKTCSRCGHLNNYFNFEYRRKNKFPHFKCEKCNFKENADYSAALNISNPKLKSTKEEP

SEQ ID NO: 3468 - protein, 726 aa, synthetic construct
SEVEFSHEYWMRHALALAKRARDEREVPVGAVLVLNNRVIGGGWNRAIGLHDPTAHAEIMALRQGGLVMQNCRLVDATLYVTFEPCVMCAGAMIHSRIGRVVFGVRNSKRGAAGSLMNVLNYPGMSHRVEITEGILEDECAALLCDFYRMPRRILNAQKKAQSSISSDGSSGGSSGSETPGTSESATPESSGGSFGGSTKNTITKTLKLRIVRPYNSAEVEKVVADEKNNRERIALEKNKDKVKEACSKHLKVAAYCTTQVERNACLFCKARKLDDKFYQKLRGQFPDAVSWQEIGEIFRQLQRQAAEIYNQSLIELYYEIFIKGKGFANASSVEHYLSDVCYTRAAELFKNAAIASGLRSKTKSNFRLKELKNMKSGLPTTKSDNFPIPLVKQKGGQYTGFEISNHNSDFIIKIPFGRWQVKKEIDKYRPWEKFDFAQVRKSPKPISLLLSTQRRKRNKGWSKDEGTEAEIRKVMNGDYQTSYIEVKRGSRIGEKSAWMLNLSIDVPKIDKGVDPSIIGGIDVGVKSPLVCAINNAFSRYSISDNDLFHFNKKMFARRRILLKKSRHKRAGHGAKNKLKPISILTEKSKRFRKKLIERWACEIADFFIKNKVGTVQMENLESMKRKEDSYFNIRLRGFWPYAEMQNKIELKLKQYGIKIRKVAPNNTSKTCSRCGHLNDYFNFEYRKKNKFPHFKCEKCNLKEDADYNAALNISNPKLKSTKEEP

SEQ ID NO: 3469 - protein, 726 aa, synthetic construct
SEVEFSHEYWMRHALTLAKRARVKHEVPVGAVLVLNNRVIGEGWNRAIGLNDPTAHAEIMALRQGGLVMQNYRLIDATLYVTFEPCAMCAGAMIHSRIGRVVFGVRNSKRGAAGSLMNVLNYPGMNHRVEITEGILADECAALLCDFYRMPRQVFNAQEKTQSSINSGGSSGGSSGSVTPGTSESATPESSGGGFGGSAKNTITKTLQLRIVRPYNSAEVEKIVADEKNSREKIALEKNKGKVKEACSEHLKVAAYCTTQVERNAYLFCKARKLDDKFYQKLRGQFPDAVFWQEIGEIFRQLQKQAAEIYNQSLIELYYEIFIKGKGFANASSVEHYLSDVCYTRAAELFKNAAIASGLRGKVKSNFRLKELKNMKSGLPTTKSDNFPIPLVKQKGGQYTGFEISSHNDDFIIKIPFGRWQVKEEIDKYRPWEKFDFEQVRKNPKPISLLLSTQRRKRNKGWSKDEGTEAEIRKVMNGDYQTSYIEVKRGSKIGEKSAWMLNLSIDVPKIDKGVDPSIIGGIDVGVKSPLVCAINNAFSRYSISDNDLFRFNKKVFARRRILLKKNRHKRAGHGTKNKLKPITILTEKSGRFRKKLIERWACEIANFFIKNKVGTVQMEDLDSMKRKGDSYFNIRLRGFWPYAEMQNKIEFKLKQYGIKIRKVAPNNTSKTCSKCGHLNNYFSFEYRKKNKFPHFKCEKCNFKEDADYNAALNISNPKLKSTKEEP

SEQ ID NO: 3470 - protein, 725 aa, synthetic construct
SEAEFSHEYWMRHALTLAKRARDEREVPVGAVLVLNNRVIGEGWNRAIGLHDPTAHAEIMALRQGGLVMQNYRLVNATLYVTFEPCVMCAGAMIHSRIGRVVFGVRNSRRGAAGSLMNVLGYPGMNHRVEITEGILADECAALLCDFYRMPRQVFNTQKKAQSGFNSGGSSGCGSGSETPGTSESAAPKSSGDSSGGSAKNTITKTLKLRIVRPYNNAEVEKIVADEKNNREKIALERNKDKVKEACSEHLKVAACTTQVERNACLFCKARKLDDKFYQKLRGQFPDAVFWQETGEIFRQLQRQAAEIYNQSLIELYYEIFIKGKGFANASSVEHYLSDVCYTRAAELFKNAAIASGLRGKVKGNFRLKELKNMKSGLPTTKSDNFPVPLVKQKGGQYAGFEISSHNDDFIIKIPFGRWQVKKEIDKYRPWEKFDFEQVRKSPKPISLLLSTRRRKRNKGWSKDEGTEAEIKKVMNGDYQTSYIEVKRGSKIGEKSAWMLSLSIDVPKIDKGVDPSIIGGIDVGVKSPLVCAINNAFGRHSISDNDLFHFNKKMFARRRILLKKNRHKRAGHGAKNKLKPITVLTEKSVRFRKKLIERWACEIADFFIKNRVGTVQMENLESMKRKEDSYFNIRLRGFWPYAEMQNKIEFKLKQYGIEIRKVAPNNTSKTCSKCGHLNNYFSFEYRKKNKFPHFKCEKCNFKENADYNAALNISNPKLKSTKEEP

SEQ ID NO: 3471 - protein, 726 aa, synthetic construct
SEDEFSHEYWMRHALTLAKRARDGREVPVGAVLVLNNRVIGEGWNRAIGLHDPTAHAEIMALRQGGLVMQNYRLSDATLYVTFEPCVMCAGAMIHSRIGRVVFGVRNSKRGAAGSLMNVLNYPGMNHCVEITEGIVVDECAALLCDFYRMPRQVLNAQKKAQSSISSGSSSGGSSGSETPGASESATPKSSVGSSAGSTKNTITKTLKLRIVRPYNSAEVEKIVADEKNNREKIALEKNKDKVKEACSKHLKVAAYCTTQVERNACLFCKARKLDDKFYQKLRGQFPDAVFWQELGEIFRQLQKQAAEIYNQSLIELYYEIFIKGKGLASASSVEHYLSDVCYTRAAELFKNAAIASGLRGKVKSNFKLKELKSMKSGLPSTKSDNFPIPLVKQRGGQYTGFEISSHNDDFIIKIPFGRWQAKKEIGKYRPWEKFDFEQVRKSPKPISLLLSTQRRKRNKGWSKDEGTEAEIRKVMNGDYQTSYIEVKRGSKIGEKSAWMLNLSIDVPKIDKGVDPSIIGGIDVGVRSPLVCAINNAFCRYSISDNDLFHFNKKMFARRRILLKKSRHKRAGHGAKNKLKPISILTEKSKRFRKKLIERWACEIADFFIKNKVGTVQMENLESMKRKEDSYFNIRLRGFWPYAEMQNKIEFKLKQYGIEIRKVAPNNTSKTCSKCGHLNNYFNFEYRKKNKFPHFKCEKCNFNEDADYNAALNISNPKLKSTKEEP

SEQ ID NO: 3472 - protein, 725 aa, synthetic construct
SEVEFSHEYWMRHALTLAKRARDEREVPVGAVLVLNNRVIGEGWNRAIGLHDPTAHAEIMALRQGGLVMQNYRLVDATLYVTFEPCVLCAGAMVHSRIGRVVFGVRNSKRGAAGSLMNVLDYPGMNHRVEITEGILADECAALLCDFYRMPRQVFSAQKKARPNINSGGSSGGRSGSGTPGTSGSATPESSGGSSGGFAKNTITKTLKLRIVRPYNSAEVEKIVADEKNNREKVALEKNKDKVKEACSEHLRVAAYCTTQVERNACLFCKARKLDDKFYQKLRGQFPDAVFWELGEIFRQLQKQAAEIYNQSLIELYYEIFIKGKGFANASNVEHYLSDVCYTRAAELFKNAAIASGLRGKVKSNFRLKELKNMKSGLPTTKSDNFPVPLVKQKGGQYTGFEISSHNDDFIIKIPFGRWQVKKEIDKYRPWEKFDFEQVRKSPKPISLLLSTQRRKRNKGWSKDEGTEAEIRKVMNGDYQISYIEVKRGSKIGEKSAWMLNLSIDVPKIDKGVDPSIIGGIDVGVKSPLVCAINNAFSRYSINDNDLFHFNKKMFARRRILLKKNRHKRAGHGAKNKLRPLTILTKKSGRFRKKLIERWACEIANFFIKNKVGTVQMENLESMKRKEDSYFNIRLRGFWPYAEMQNRIEFKLKQYGIKIRKVAPNNTSKTCGKCGHLNNYFNFEYRKKNKFPHFKCEKCNFKENADYNAALNISNPKLKSTKEEP

SEQ ID NO: 3473 - protein, 726 aa, synthetic construct
SEVEFSHEYWMRHALTLAKRARDEREVPVGAILVLNNRVIGEGWNRAIGLHDPTAHAEIMALRQGGLVMQNYRLIDATLYVTFEPCVMCAGAMIHSRIGRVVFGARNSKRGAAGSLMNVLSYPGMNHRVEITEGILTDECAALLCDFYRMPHQVLNAQKKAQSSINSGGSSGGSSGSETPGTSGSATPEGSGGSSGGSAKNTITKTLKLRIVRPYNSAEVEKIVADEKNNREKIALEKNKGKVREACSKHLKVAAYCTTQVERNACLFCKARRLDDKFYQKLRGQFPDAVFWQEIGEILRQLQKQAAEIYNQSLIELYYEIFIKGKGIASASRVGHYLSDVCYTRAAELFKNAAIASGLSGKVKSNFRLKELKNMKSGLPTTKSDNFPIPLVKQKGGQYTGFEISSHNDDFIIKIPFGRWQVKKEIDKYRPWEKFDFEQVRKSPKPISLLLSTQRRKRNKGWSKDEGTEAEIRKVMNGDYQTSYIEVKRGSKTGEKSAWMLNLSIDVPKIDKGVDPSIIGGIDVGVKSPLVCAINNAFSRYSISDNDLFRFNKKMFARRRILLKKNRHKRAGHGAKNKLKPISILTGKSERFRKKLIERWACEIADFFIKNKVGTVQMENLESMKRKEDSYFNIRLRGFWPYAEMQNRIELKLKQYGIEIRRVAPNNTSRTCSKCGHLNNYFNFEYRKKSKFPHFKCEKCNFREDADYNAALNISNPKLKSTKEEP

SEQ ID NO: 3474 - protein, 726 aa, synthetic construct
SEVEFSHEYWMRHALTLARRARDEREVPVGAVLVLNNRVIGEGWNRAIGLHDPTAHAEIMALRQGGLVMQNYRLTDATLYVTFEPCVMCAGAMIHSRIGRVVFGVRNSKRGAAGSLMNVLSYPGMNHCVEITEGILVDECAALLCDFYRMPRQVLNAQKKAQSSISSGGSSGGSSGSETPGASESVTPKSSVGSSASSTKNTITKTLKLRIVRPYNSAEVEKIVADEKDNREKIALEKNKDKVKEACSKHLKVAAYCTTQVERNACLFCKARRLDDKFYQKLRGQFPDAVFWQELGGIFRQLQKQAAEIYNQSLIELYYEIFIKGKGITNASRVEHYLSDVCYTRAAELFKNAAIASGLRSKVRSNFRLKELKNMKSGLPTTKSDNFPIPLVKQKGGQYTGFEISSHNSDFIIKIPFGRWQVKEEIVKYRPWEKFDFEQVRKSPKPISLLLSTQRRKRNKGWSKDEGTEAEIRKVMNGDYQTSYIEVKRGSRIGEKSAWMLSLSIDVPKIDRGVDPSIIGDIDVGVKSPLVCAINNALSRYSISDNDLFHFNKKMFARRRILLKKNRHRRAGHGARNKLKPITVLTEKSKRFRKKLIERWACEIADFFIKNKVGTVQMENLESMKRKEDSYFNIRLRGFWPYAEMQNKIEFKLKQYGIEIRKVAPNNTSKTCSKCGHLNNYFNFEYRRKNKFPHFKCEKCNFKENADYNAALNISNPKLKSTKEEP

SEQ ID NO: 3475 - protein, 726 aa, synthetic construct
SEVEFSHEYWMRHALTLAKRARDEREVPVGAVLVLNNRVIGEGWNRAIGLHDPTAHAEIMALRQGGLVMQNYRLVDATLYVTFEPCVLCAGAMVHSRIGRVVFGVRNSKRGAAGSLMNVLDYPGMGHRVEITEGILADECAALLCDFYCMPRQVLNAQKKAQSSISPGGSSGGSSGSETPGAGESVTPKSSVGSSAGSTKNTITKTLKLRIVRPYNSAEVEKIVADEKNNREKIALEKNKDKVKEACSKHLKVASYCTTQVERNACPFCKARKLDDKFYQKLRGQFPDAVFWQELGEILRQLQKQAAEIYNQSLVELYYEIFIKGKGIANASSVEHYLSDVCYTRAAELFKNAAIASGLRNKIKSNFRLKELRNMKSGLPTTKSDNFPIPLVRQKGGQYTGFEISNHNGDFIIKIPFGRWQVKKEICKHRPWEKFDFEQVRKSPKPISLLLSTQRRKRNKGWSKDEGTEAEIRKVMNGDYQTSYIEVKRGSKIGEKSAWMLNLSIDVPKIDKGVDPGIIGGIDVGVKSPLVCAINNASSRYSISDNDLFHFNKKMFARRRILLKKNRHKRAGHGAKNKLKPITIMTEKSKRFRKKLIERWACEIADFFIKNKVGTVQMENLESMKRKEDSYFNIRLRGFWPYAEMQNKIEFKLKQYGIEIRKVAPNNTSKTCSKCGHLSNHFNFEYRKKNKFPHFKCEKCNFKENAVYNAALNISNPKLKGTKEEP

SEQ ID NO: 3476 - protein, 726 aa, synthetic construct
IEVEFSHEYWMRHALTLARRARDEREVPVGAVLVLNNRVIGEGWNRAIGLHDPTAHAEIMALRQGGLVMRNYRLTGATLYVTFEPCVMCAGAMIHSRIGRVVFGVRNSKRGAAGSLMNVLNYPGMNHCVEITEGILVDECAALLCDFYRMPRQVLNAQKRAQSSINSGGPSGGSSGSETPGTSKSATPESSGGGSGGSTKGTITKTLKLRIVRPYNSAEVEKIVADEKNNREKIALEKNKDKVKEAYSKHLKVAAYCTTQVERNVCLFCKARKLDDKFYQKLRGQFPDAVFWQEIGEIFRQLQKQAAEIYNQSLIELYYEIFIKGKGLANTSSVEHYLSDVCYTRAAELFKNAAIASGLRNKIKSNFRLKELRNMKSGLPTTKSDNFPIPLVRQKGGQYTGFEISNHNGDFIIKIPFGRWQVKKEISKHRPWEKFDFEQVRKSPKPISLLLSTQRRRRNKGWSKDEGTEAEIRKVMNGDYQTSYIEVKRGSKIGEKSAWMLNLSIDVPKIDKGVDPSIIGGIDVGVKSPLVCAINNAFSRYSIGDNDLFHYNKKMFARRRILLKKNRYKRAGHGAKNKLKPITILTKKSERFRKKLIERWACEIANFFIKNKVGTVQMENLESMKRKEDSYFNIRLRGFWPYAEMQNKIEFKLKQYGIKIRKVAPNNTSKTCSKCGHLNNHFSFEYRKKNKFPHFKCEKCNFKENADYNAALNISNPKLKSTKEEP

SEQ ID NO: 3477 - protein, 726 aa, synthetic construct
SEVEFSHEYWMRHALTLAKRARDEREVPVGAVLVLNNRVIGEGWNRTTGLHDPTAHAEIMALRQGGLVMQNHRLVDATLYVTFEPCVMCAGAMIHSRIGRVVFGIRNSKRGAAGSLTNVLNYPGMNHRVEITEGILVDECAALLCDFYRMPRQVFNAQRKAQSTINSGGSSGGSSGSETPGTSESATPESSGGSSGGSAKNTITKALKLRIVRPYNSAEVEKIVADEKNNREKIALEKNKDKVKEACSKHLKVASYCTTQVERNACPFCKARKLDDKFYQKLRGQFPDAMFWQELGEILRQLQKQAAEIYNQSLVELYYEIFIKGKGFANASSVEHCLSDVCYTRAAELFKNAAIASGLRGKVKSNFRLKELKNMKSGLPTTKSDNFPIPLVKQKGGQYTGFEISNLNSDFIIKIPFGRWQVKKEINKYRPWEKFDFEQVRKSPKPISLLLSTQRRKGNKGWSKDEGTEAEIRKVMNGDYQTSYIEVKRGSKTGEKSAWMLNLSIDVPKIDKGVDPSVIGGIDVGVKSPLVCAINNAFSRFSISDNDLFHFNKKMFARRRILLKKNGRKRAGHGAKNKLKPITILTEKSKRFRKKLIERWACEIAGFFIKNKVGTVQMENLESMKRKEDSYFNIRLRGFWPYAEMQNKIEFKLKQYGIEIRKVAPNNTSKTCSKCGHLNSYFNFEYRKKNKFPHFKCEKCNFRENADYNAALNISNPKLKSTKGEP

SEQ ID NO: 3478 - protein, 726 aa, synthetic construct
SEVEFSHEYWMRHALALAKRARDEREVPVGAILVLNNRVIGEGWNRAIGLHDPTAHAEIMALRQGGLVMQNYRLTDATLYVTFEPCVMCAGAMIHSRIGRVVFGVRNSKRGAAGSLMNVLNYPGMNHCVEITEGILVDECAALLCDFYRMPRQVLNAQKKAQSSIGSGGLSGGSSGSETPGASGSVTPKSSGGSSAGPTKDTITKTLKLRIVRPYNSAVVEKIVADEKNSREKIALEKNKDKVKEACSEHLKVAAYCTTQVERNACLFCKARELDDKFYQKLRGQFPDAVFWQEIGEIFRQLQKQAAEIYNQSLIELYYEILIKGKGFANASSVEHYLSDVCYTRAAELFKNAAIASGLRGKVRSNFRPKELKNMKSGLPTTKSDNFPIPLVKQKGGQYTGFEISSHNDDFIIKIPFGRWQVKEEIDKYRPWEKFDFEQVRKNPKPISLLLSTLRRKRNKGWSKDEGTEAEIRKVMNGDYQTSYIEVKRGSKIGEKSAWMLNLSIDVPKIDKGADPSIVGGIDVGVKSPLVCAINNAFSRYSISDNDLFRFNKKVFARRRILLKKNRHKRAGHGAKNKLKPISILTEKSERFRKKLIEKWACEIADFFIKNKVGTVQMENLESIKRKEDSYFNIRLRGFWPYAEMQNKIEFKLKQYGIEIRKVAPNNTSKTCSKCGHLNNYFNFEYRKKNKFPHFKCEKCNFKEDADYNAALNISNPKLKSTKEEP

SEQ ID NO: 3479 - protein, 725 aa, synthetic construct
SEVEFSHEYWMRHALTLAKRARDEREVPVGAILVLNNRVIGEGWNRAIGLHDPTAHAEIMALRQGGLVMQNYRLTDATLYVTFEPCVMCAGAMIHSRIGRVVFGVRNSKRGAAGSLMNVLNYPGMNHCVEITEGILVDECAALLCDFYRMPCQVLNAQKKAQSSISSGGSSGGSSGSETPGTSESPTPESSGGSPGGSAKNTITKTLKLRIVRPYNSAKVEKIVADEKNNREKIAMEKNKDKVKEACSKHLKVASYCTTQVERNACLFCKARKLDDKFYQKLRGQFPDAVFQEIGEIFRQLQKQAAEIYNQSLIELYYEIFIKGKGFANASSVEHYLSDVCYTRAAELFKNAAIASGLRGKVKSNFRLKELKNMRSGLPTAKSDNFPIPLVKQKGGQYSGFEISSHNDDFIIKIPFGRWQVKKEIDKYRPWEKFDFEQVRKSPKPISLLLSTQRRKRNKGWSKDEGTEAEIRKVMNGDYQTSYIEVKRGSKIGEKSAWMLNLSIDVPKIDKGVDPSIIGGIDVGVKSPLVCAINNAFSRYSISDNDLFRFNKKMFARRRILLKKNRHKRAGHGAKNKLKPISILTGKSERFRKKLIERWACEIADFFIKNKVGTVQMENLESMKRREDSYFNIRLRGFWPYAEMQNKIEFKLKQYGIEIRKVAPNNTSKTCSKCGHLNNYFNFEYRKKNKFPHFKCERCNFKEDADYNAALNISNPKLKSTKEEP

SEQ ID NO: 3480 - protein, 726 aa, synthetic construct
SEVEFSHEYWMRHALPLAKRARDEREVPVGAVLVLNNRVIGEGWNRAIGLHDPTAHAEIMALRQGGLVMQNYRLSDATLYVTFEPCVMCAGAMIHSRIGRVVFGVRNSKRGAAGSLMNVLNYPGMNHCVEITEGILVDECAALLCDFYRMPRQVLSAQKKAQSSIGSGGSSGGSSGSETPGASGSVTPKSSVGSSAGSTKNTITKTLKLRIVRPYNSAEVEKIVADEKNNREKVALEKNKDKVKEACSKHLKVAAYCTTQVERNACLFCKARKLDDKFYQKLRGQFPDAVFWQEIGEIFRQLQKQAAEIYNQSLIELYYEIFIKGKGFANASSAEHYLSDVCYTRAAELFKNAAIASGLRGKVKSNFRLKELKNMKSGLPTTKSDNFPIPLVKQKGGQCTGFEISSHNDDFIIKIPFGRWQVKKEIDKYRPWEKFDFEQVRKSPKPISLLLSTQRRKRNKGWSKDEGTEAEIRKVMNGYYQTSYIEVKRGSKIGEKSAWMLNLSIDVPKIDKGVDPSIVGGIDVGVKSPLVCAIDNALSRYSISDNDLFHFNKKMFARRRILLKKNRHRRAGHGAKNKLKPISILTEKSKRFRKKLIERWACEIADFFIKNKVGTVQMENLEGMKRKEDSYFNIRLRGFWPYAEMQNKIEFKLKQYGIEIRKVAPNNTSKTCSKCGHLNNYFNFEYRKKNKFPHFKCEKCNFKENADYNAALNISNPMLKSTKEEL

SEQ ID NO: 3481 - protein, 726 aa, synthetic construct
SEVEFSHEYWMRHALTLAKRARDGREVPVGAVLVLNNRVIGEGWNRAIGLHDPTAHAEIMALRQGGLVMQNYRLVDATLYVTFEPCVMCAGAMVHSRIGRVVFGVRNSKRGAAGSLMNVLDYPGMGHRVEITEGILADECAALLCDFYCMPRQVFNAQKRAQSSINSGGSSGGSSGSDTPGTSESATPESSGGGSSGSAKNTITKTLQLRIVRPYNSAEVEKIVADEKNNREKIALEKNKDKVREACSKHLKVAAYCTTQVERNACLFCKARKLDDKFYQKLRGQFPDAVFWQELGEILRQLQKQAAEIYNQSLIELYYEIFIKGRGFANASSVEHYLSDVCYTRAADLFKNAAIASGLRGKVKSNFRLKELKNMRSGLPTAKSDNFPIPLVKQKGGQYTGFEISSHNDDFIIKIPFGRWQVKKEIDKYRPWEKFDFEQVRKSPKPISLLLSTQRRKRNKGWSKDEGTEAEIRKVMNGDYQTSYIEVKRGSKTGEKSAWMLNLSIDVPKIDKGVDPCIIGDIDVGVKSPLVCAINNAFSRYSISDNDLFHFNKKMFARRRILLKENGHKRAGHGAKNKLKPITIMTEKSKRFRKKLIERWACEIADFFIKNKVGTVQMENLESMKRKEDSYFNIRLRGFWPYAEMQNKIEFKLKQYGIVVRKVAPNNTSKTCSECGHLNNYFNFEYRKMNKFPHFKCEKCNFKEDADYNAALNISNPKLKSTKEEP

SEQ ID NO: 3482 - protein, 726 aa, synthetic construct
SEVEFSHEYWMRHALTLAKRARDEREVPVGAILVLNNRVIGEGWNRAIGLHDPTAHAEIMALRQGGLVMQSYRLIDATLYVTFEPCVMCAGAMVHSRIGRVVFGVRNSKRGAAGSLMNVLDYPGMGHRVEITEGILADECAALLCDFYCMPRRVFNAQKRAQTSINSGGSSGGSSGSETPGTSESATPGSSGGGSSGSAKNTITKTLQLRIVRPYNSAEVEKIVADEKNNREKIALEKNKDKVKEACSEHLKVAAYCTAQVERNACLFCKARKLDDRFYQKLRGQFPDAVFWQEIGEIFRQLQKQAAEIYNQSLIELYYEIFIKGRGFANASSVEHYLSDVCYTRAAELFKNAAIASGLRGKVKGNFRLKELKNMKSGLPSTKSDNFPIPLVKQRGGQYTGFEISSHNDDFIIKIPFGRWQAKKEIDKYRPWEKFDFEQVRKSPKPISLLLSTQRRKRNRGWSKDEGTEAEIRKVMNGDYQTSYIEVKRGSKIGEKSAWMLNLSIDVPKIDKGVDPSIIGGIDVGVKSPLVCAINNAFSRYSISDNDLFHFNKKMFARRRILLKKNRRRRAGHGAKNKLKPITILTEKSVRFRKKLIERWACEIADFFIKNKVGTVQMENLESMKRKEDSYFNIRLRGFWPYAEMQNKIEFKLKQYGIEIRRVAPNNTSRTCSKCGHLNNYFNFEYRRKYKFPHFKCEKCNFKEDADYNAALNISNPKLKSTKEEP

SEQ ID NO: 3483 - protein, 726 aa, synthetic construct
SEVEFSHEYWMRHALTLAKRARDEREVPVGAILVLNNRVIGEGWNRTTGLHDPTAHAEIMALRQGGLVMQNHRLVDATLYVTFEPCVMCAGAMIHSRIGRVVFGVRNSKRGAAGSLTNVLNYPGMNHRVEITEGILVDECAALLCDFYRMPRQVFNARKKAQSSINPGGSSGGSSGSEMPGTSESATPGSSGGSSGGSTKNTITKTLKLRIVRPYNCAEVEKIVADEKNNREKIALEKNKDKVKEACSKHLKVAAYCTTQVERNACLFCRARKLDDEFYQKLRGQFPDAVFWQEIGEIFRQLQRQAAEIYNQSLIELYYEIFIKGKGFANASSAEHYLSDVCYTRAAELFKNAAIASGLRGKVKSNFRLKELKNMKSGLPTTKSDNFPIPLVRQKGGQYTGFEISSHNDDFIIKIPFGRWQVRKEIDKYRPWEKFDFEQVRKSPKPISLLLSTQRRKKNKGWSKDEGTEAEIRKVMNGDYQTSYIEVKRGSKIGEKSAWMLNLSIDVPKIDKGVDPSIIGGIDVGVKSPLVCAINNSSSRYSICDNDLFRFNKKMFARRRILLKKNRHKRAGHGAKNKLKPITILTKKSERFRKKLIERWVCEVADFFIKNKVGTVQMENLESMKRKEDSYFNIRLRGFWPYAEMQNRIELKLKQYGIEIRRVAPNNTSRTCSKCGHLNNYFNFEYRKKSKFPHFKCEKCNFREDADYNAALNISNPKLKSTKENP

SEQ ID NO: 3484 - protein, 726 aa, synthetic construct
SEVVFSHEYWMRHALTLAKRARDEREVPVGAVLVLNNRVIGEGWNRAIGLHDPTAHAEIMALRQGGLVMQNYRLDNATLYVTFEPCVMCVGAMIHSRIGRVAFGVRNSKRGAAGSLMNVLNYPGMNHRVEITEGILAGECAALLCDFYRMPRQVFNAQKKAQSNINSGGSSGGNSGSEAPGTSESPTPESSGGDSSGSAKNTITKTLQLRIVRPYNSTEVEKIVADEKNNREKVALEKNKDKVKEACSKHLKVAAYCTTQVERNACLFCKARKLDDKFYQKLRGQFPDAVFWQEIGEIFRQLQKQAAEIYNQSLIELYYKIFIKGRGFANASSVEHYLSDVCYTRAAELFKNAAIASGLRSKVRSNFRLKELRNMKSGLPTTKSDNFPIPLVKQKGGQYTGFEISNHNSDFIIKIPFGRWRVKKEIDKYRPWEKFDFEQVRKSPKPISLLLSTQRRKRNKGWSKDEGTEAEIRKVMNGDYQTSYIEVKRGSKTGEKSAWMLNLSIDVPKVDKGVDPSIIGGIDVGVKSPLVCAINNAFSRYSISDNDLFRFNKKMFARRRILLRKNRHKRAGHGAKNKLKPITTMTEKSRRFRKKLIERWACEIADFFIKNKVGTVQMENLESMKRREDSYFNIRLRGFWPYAKMQNKIEFKLKQYGIEIRKVAPNNTSKTCSKCGHLSNYFDFEYRKKNKFPHFKCEKCNFKESADYNAALNISNPKLKSTKEEP

SEQ ID NO: 3485 - protein, 726 aa, synthetic construct
SEVEFSHEYWMRHALTLAKRARDEREVPVGAILVLNNRVIGEGWNRAIGLHDPTAHAEIMALRQGGLVMQNYRLIDATLYVTFEPCVMCAGAMIHSRIGRVVFGVRNNKHGAAGSLVNVLNYPGMNHRVEITEGILADECAALLCDFYRMPRQVFNARKRAQSSINPGGSSGGSSGGETPGTSESPTPESSGGSSGGSAKNTITKTLKLRIVRPYNSAEVEKIVAEEKNNREKIALEKNKDKVKEACSKHLKVAAYCTTQVGRNACLFCKARKLDDKFYQKLRGQFPDAVFWQEIGEIFRQLQKQAAEIYNQSLIELYYEIFIKGKGFANASSVEHYLSDVCYTRAAELFKNAAIASGLRGKVKSNFRLKELKNMKSGLPTTKSDNFPIPLVKQKGGQYTGFEISNHNDDFIIKIPFGRWQVKKEIDKYRPWEKFDFEQVRKSPKPISLLLSTQRRKRNKGWSKDEGTEAEIRKVMNGDYQTSYIEVKRGSKIGEKSAWMLNLSIDVPKIDKGVDPSIVGGIDVGVKSPLVCAINNAFSRYDISDNDLFHFNKKMFARRRILLKKNRHKRAGHGAKNKLKPISIPTEKSVRFRKKLIERWACEIADFFIKNKVGTVQMENLESMKRKEDSYFNIRLRGFWPYAEMQNKIEFKLKQYGIEIRKVAPNNTSKTCSKCGHLNNYFNFEYRKKNKFPHFKCEKCNFKENADYNAALNISNPKLKSTKEEP

SEQ ID NO: 3486 - protein, 726 aa, synthetic construct
SEVEFSHEYWMRRALTLAKRARDEREVPVGAILVLNNRVIGEGWNRAIGLHDPTAHAEIMALRQGGLAMQNYRLIDATLYVTFEPCVMCAGAMIHSRIGRVVFGVRNSKHGAAGSLVNVLSYPGMNHRVEITEGILADECAALLCDFYRMPRQVFNARKKTQSSINPGGSSGGSSGSETPGTSESATPESSGGSSGGSAKNTITKTLKLRIVRPYNSAEVEKIVADEKNNREKIALEKNKDKVKEACSEHLKVAAYCTTQVERNACLFCKARKLDDKFYQKLRGQFPDAVFWQEIGEIFRQLQKQAAETYNQSLIELYYEIFIKGKGVANANNVEHYLSDVCYTRAAELFKNAAIASGLRNKIKSNFRLKELRNMKSGLPTTKSDNFPIPLVKQKGGQYTGFEIGNHNSDFIIKIPFGRWQAKKEIDKYRPWEKFDFEQVRKSPKPISLLLSTQRRRRNKGWSKDEGTEAEIRKVMNGDYQTSYIEVKRGSKIGEKSAWMLNLSIDVPKIDKGVDPSIIGGIDVGVKSPLVCAIDNAFSRYSISDNDLYRFNKKMFARRRILLKKNRHKRAGHGTMNKLKPITILTEKSGRFRKKLIERWACEIADFFIKNKVDTVQMENLESMKRKEDSYFNIRLRGFWPYAEMQNKIEFKLKQYGIKIRKVAPDNTSKTCSKCGHLNNYFSFEYRKKNKFPHFKCEKCNFKENADYNAALNISNPKLKSTKEGP

SEQ ID NO: 3487 - protein, 726 aa, synthetic construct
SEVEFSHEYWMRHALTLAKRARDEREVPVGAILVLNNRVIGEGWNRAIGLHDPTAHAEIMALRQGGLVMQNYRLIDATLYVTFEPCVMCAGAMIHSRIGRVVFGVRNSKHGAAGSLVNVLNYPGMNHRVEITEGILVDECAALLCDFYRMPRQVLNAQKKAQSSISSGGSSGGSSGSETPGASGSVIPKSSGGSSAGSTKDTITKTLKLRIVRPYNSAEVEKVVADEKNNREKIAMEKNKDKVKEACSKHLKVASYCTTQVERNACLFCKARKLDDKFYQKLRGQFPDAVFWQELGGIFRQLQKQAAEIYNQSLIELYYEIFIKGKGITNASRVEHYLSDVCYTRAAELFKNAAIASGLRSKVRSNFRLKELKNMKSGLPTTKSDNFPIPLVKQKGGQYTGFEINSHNDDFIIKIPFGRWQVKKEIDKYRPWEKFDFEQVRKSPKPISLLLSTQRRKRNKGWSKDEGTEAEIRKVMNGDYQTSYIEVKRGSKTGEKSAWMLNLSIDVPKIDKGVDPSIIGGIDVGVKSPLVCAINNAFSRYSISDNDLFRFNKKMFARRRILLKKSKHKRAGHGAKNKLKPITILTEKSGRFRKKLIERWVCEVADFFIKNKVGTVQMENLESMKRKEDSYFNIRLRGFWPYAEMQNRIELKLKQYGIEIRRVAPNNTSRTCSKCGHLNNYFNFEYRKRSKFPHFKCEKCNFREDADYNAALNISNPKLKSTKEEP

SEQ ID NO: 3488 - protein, 726 aa, synthetic construct
SEVEFSHEYWMRHALTLAKRARDEREVPVGAILVLNNRVIGEGWNRAIGLHDPTAHAEIMALRQGGLVMQNYRLIDATLYVTFEPCVMCAGAMVHSRIGRVVFGVRNSKRGAAGSLMNVLDYPGMGHRVEITEGILADECAALLCDFYRMPRQVLNAQKKAQSSISSGGSSGGSSGSETPGTSESATPENSGGSSGSSAKNTITKTLKLRIVRPYNSAEVEKIVADEKNNREKIALEKNKDKVKEACSEHLKVAAYCTTQVERNACLFCKARKLDDRFYQKLRGQFPDAVFWQEIGEIFRQLQKQAAEIYNQSLIELYYEIFIKGKGFANASSVEHYLSDVCYTRAAELFKNAAIASGLRGKVKSNFRLKELKNMKSGLPTTKSDNFPIPLVKQKGGQYTGFEISSHNDDFIIKIPFGRWQVKEEIDKYRPWEKFDFEQVRKNPKPISLLLSIQRRKRNKGWSRDEGTEAEIRRVMNGDYQTSYIEVKRGSKIGEKSAWMLNLSIDVPRIDKGVDPSIIGGIDVGVKSPLICAINNAFSRYGISDNDLFRFNKKVFARRRILLKKNRHKRAGHGTKNKLKPITILTEKSGRFRKKLIERWACEIANFFIKNKVGTVQMENLESMKRKEDSYFNIRLRGFWPYAKMQNKIEFKLKQYGIEIRKVAPNNTSKTCSKCGHLNNYFNFEYRKKNKFPHFKCEKCNFKENADYNAALNISNPKLKSTKEEH

SEQ ID NO: 3489 - protein, 726 aa, synthetic construct
SEIEFSHEYWMRHALTLAKRARDEREVPVGAVLVLNNRVIGEGWNRAIGLHDPTAHAEIMALRQGGLVMQNYRLTDATLYVTFEPCVMCAGAMIHSRIGRVVFGVRNSKRGAAGSLMNVLNYPGMNHCVEITEGILVDECAALLCDFYRMPRQVLNAQKKAQSSISSGGSSGGSSGSETPGASGSVTPKSSGGSSAGSTKDTITKTLKLRIVRPYNSAEVEKVVADEKNNREKIAMEKNKDKVKEACSEHLKVAAYCTTQVERNACLFCKARKLDDRFYQKLRGQFPDAVFWQETGEIFRQLQKQAAEIYNQSLIELYYEIFIKGKGFANASSVEHYLSDVCYTRAAELFKNAAIASGLRGKVKSNLRLKELKNMKSGLPTTKSDNFPIPLVKQKGGQYTGFEISSHNDDFIIKIPFGRWQVKKEIDKYRPWEKFDFEQVRKSPKPISLLLSTQRRKRNKGWSKDEGTEAEIRKVMNGDYRTSYIEVKRGSKTGEKSAWMLNLSIDVPKIDKGVDPSIIGGVDVGVKSPLVCAINNAFSRYSISDNDLFRFNKKMFARRRILLKKNRHKRAGHGAKNKLKPISILTGKSERFRKKLIERWACEIADFFIKNKVGTVQMENLESMKRKEDSYFNIRLRGFWPYAEMQNRIEFKLKQYGIEIRKVAPNNTSKTCSKCGHLNNYFNFEYRKKNKFPHFKCERCNFKENADYNAALNISNPKLKSTKEEP

SEQ ID NO: 3490 - protein, 726 aa, synthetic construct
SEVEFSHEYWMRHALTLAKRARDEREVPVGAVLVLNNRVIGEGWNRAIGLHDPTAHAEIMALRQGGLVMQNYRLIDATLYVTFEPCVMCAGAMIHSRIGRVVFGVRNNKHGAAGSLVNVLNYPGMNHRVEITEGILADECAALLCDFYRMPRQVFNARKKAQSSTNPGGSSGGSSGSETPGTSESATPESPGGSSTGSTKNTITKTLKLRIVRPYNSAEVEKIVADEKNSREKIALEKNKDKVKEACSEHLKVAAYCTTQVERNACLFCKARKLDDRFYQKLRGQFPDAVFWQEIGEIFRQLQKQAAEIYNQSLIELYYEIFIKGKGFAIASSVVHYLSCVCYTRAAELFKNAAIASGLRGKVKSNFRLKELKNMKSGLPTTKSDNFPIPLVKQKGGQYTGFEISSHNDDFIIKIPFGRWQVKKEIDKYRPWEKFDFEQVRRSPKPISLLLSTQRRKRNKGWNEDEGTEAEIRKVMNGDYQTSYIEVKRGSKIGEKSAWMLNLSIDVPKIDKGVDPSIIGGIDVGVKSPLVCAINNALSRYSISDNDLFRFNKKMFARRRILLKKNRHKRAGHGAKNKLKPISILTEKSERFRKKLIEKWACEIADFFIKNKVGTVQMENLEGMKRKEDSYFNIRLRGFWPYAEMQNKIEFKLKQYGIEIRKVAPNNTSKTCSKCGHLNNYFNFEYRKKNKFPHFKCEKCNFKENADYNAALNISNPRLKSTKEEP

SEQ ID NO: 3491 - protein, 725 aa, synthetic construct
SEVEFSHEYWMRRALTLAKRARDEREVPVGAVLVLNNRVIGVGWNRAVGLHDPTAHAEIMALRQGGLVMQNYRLTDATLYVTFEPCVMCAGAMIHSRIGRVVFGVRNSKRGAAGSLMNVLNYPGMNHCVEITEGILVDECAALLCDFYRMPRQVLNAQKKAQPSINPGGSSGGSSGSETPGTSESPTPESPGGGSGGSAKNTITKTLKLRIVRPYNSAEVEKIVADEKNNREKIALEKNKDKVKEACSKHLKVAAYCTTQVERNACLFCKARKLDDKFYQKLRGQFPDAVFWEIGEIFRQLQKQAAEIYNQSLIELYYEIFIKGRGFANASSVEHYLSDVCYTRAAELFKNAAIASGLRGKVKSNFRLKELKSMKSGLPTTKSDNFPIPLVKQKGGQCTGFEISSHNDDFIIKIPFGRWQAKKEIDRYRPWEKFDFEQVRKSPKPISLLLSTQRRKRNKGWSKDEGTEAEIRRVMNGDYRTSYIEVKRGSKTGEKSAWMLNLSIDVPRTDKGVDPCIIGGIDVGVKSPLVCAINNAFSRYSISDNDLFHYNKKMFARRRILLKKNRHKRAGHGARNKLKPITVLTEKSERFRKKLIERWACETANFFIKNKVGTVQMENLESMKRREDSYFNIRLRGFWPYAEMQNKIEFKLKQYGIEIRKVAPNNTSKTCSKCGHLNSYFNFEFRKKNKFPHFKCEKCNFKEDADYNAALNISNPKLKSTKEEP

SEQ ID NO: 3492 - protein, 726 aa, synthetic construct
SEVEFSHEYWMRHALTLAKRARDEREVPVGAVLVLNNRVIGEGWNRAIGLHDPTAHAEIMALRQGGLVMQNYRLSDATLYVTFEPCVMCAGAMIHSRIGRVVFGVRNSKRGAAGSLMNVLNYPGMNHCVEITEGILVDECAALLCDFYRMPRQVLSAQKKAQSSVSSGGSSGGSSGSETPGASGSVTPKSSVGSSAGSTKNTITKTLKLRIVRPYNSAEVEKIVADEKNNREKIALEKNKDKVKEACSKHLKVASYCTTQVGRNACPFCKARKLDDKFYQKLRGQFPDAVFWQELGEILRQLQKQAAEIYNQSLIELYYEILIKGRGFANACSVEHYLSDVCYTRAAELFKNAAIASGLRGKVKSNFRLKELKNMKSGLPTTKSDNFPIPLVKQKGGQYTGFEISSHNDDFIIKIPFGRWQVRKEIDKYRPWEKFNFEQVRKSPKPISLLLSTQRRKRNKGWSEDEGTEAEIRKVMNGNYQTSYIEVKRGSKIGEKSAWMLSLSIDVPKIDKGVDPSIIGGIDVGVKSPLVCAINNAFSRYSISDNDLFHFNKKMFARRRILLKKNRHKRAGHGAKNKLKPISILAEKSERFRKKLIEKWACEIADFSIKNKVGTVQMENLGSMKRKEDSYFNIRLRGFWPYAEMQNKIEFKLKQYGIEIRKVAPDNTSKTCSKCGHLNNYFNFEYRKKNKFPHFKCEKCNFKEDADYNAALNISNPKLKSTKEEP

SEQ ID NO: 3493 - protein, 726 aa, synthetic construct
SEVEFSHEYWMRHALTLAKRARDEREVPVGAILVLNNRVIGEGWNRAIGLHDPTAHAEIMALRQGGLVMQNYRLTDATLYATFEPCVMCAGAMIHSRIGRVVFGVRNSKHGAAGSLMNVLNYPGMNHRVEITEGILADECAGLLCDFYRMPRQVFSARKKAQSSINPGGSSGGSSGGKAPGTSESATLESSGGSSGGSAKNSITKTLKLRIVRPYNSAEVEKIVADEKNNREKTALEKNKGKVKEACSKHLKVATYCTTQVERNACLFCKARKLDDKFYQKLRGQFPDAVFWQEIGEIFRQLQKQAAEIYNQSLIELYYEIFIEGKGSANARSVEHYLSDVCYTRAAELFKNAAIASGLRGKVKGNFRLKELKSMKSGLPTTKSDNFPIPLVKQKGGQYTGFEISSHNDDFIIKIPFGRWQVKKEIDKYRPWEKFDFEQVRKSPKPISLLLSTQRRKRNRGWSKDEGTEAEIRKVMNGVYQTSYIEVKRGSKIGEKSAWMLNLSIDVPKIDKGVDPSIIGGIDVGVRSPLVCAIDNASSRYSISDNDLFHFNKKMFARRRILLKKNRHRRADHGAKNKLKPISILTEKSKRFRKKLIERWACGIADFFIKNKVGTVQMENLESMKRKEDSYFNIRLRGFWPYAEMQNKIEFKLRQYGIEIRRVAPNNTSKTCSKCGHLNNYFDFEYRKKNKFPHFKCEKCNFKENADYNAALNISNPKLKSTKGEP

SEQ ID NO: 3494 - protein, 725 aa, synthetic construct
SEVEFSHEYWMRHALTLAKRARDEREVPVGAILVLNNRVIGVGWNRAIGLHDPTAHAEIMALRQGGLVMQNYRLIDATLYVTFEPCVMCAGAMIHSRIGRVVFGVRNSKHGAAGSLVNVLNYPGMNHRVEITEGILADECAALLCDFYRMPRQVFNARKKAQSSINSGGSSGGSSGSETPGTSESATPKSSGGSSGGSAKNTITKALKLRIVRPYNSAEVEKIVADEKNNRERIALEKNKDKVKEACSKHLKVAAYCTTQVERNACLFCKARKLDDKFYQKLRGQFPDAVFWELGEIFRQLQKQAAEIYNQSLIELYYEIFIKGKGFANASNVEHYLSDVCYTRAAELFKNAAIASGLRGKVKSNFRLKELKNMKSGLPTTKSDNFPIPLVKQKGGQYTGFEISSHNDDLIVKIPFGRWQVKKEIDRYRPWEKFDFEQVRKSPKPISLLLSTQRRKRNKGWSKDEGTEAEIRKVMNGDYQTSYIEVRRGSKIGEKSAWMLNLSIDVPKIDKGVDPCIIGGIDVGVKSPLVCAINNASSRYSISDNDLFHFNKKMFARRRILLKKNGHKRAGHGTKNKLKPITIMTEKSKRFRKKLIERWACEIADFFIKNKVGTVQMENLESMKRKEDSYFNIRLRGFWPYAELQNKIEFKLKQYGIVVRKVAPNNTSKTCSKCGHLNNYFNFEYRKKNKFPHFKCEKCNFKENADYNAALNISNPKLKSTKGEP

SEQ ID NO: 3495 - protein, 726 aa, synthetic construct
SEVEFSHEYWMRHALTLAKRARDEREVPVGAVLVLNNRVIGEGWNRAIGLHDPTAHAEIMALRQGGLVMQNYRLIDATLYVTFEPCVMCAGAMIHSRIGRVVFGVRNSKRGAAGSLMNVLNYPGMNHCVEVTEGILVDECAALLCDFYRMPRQVLNAQKKAQSSISPGGSSGGSSGSETPGASESVTPKSSGGSSGGSAKNTITKALKLRIVRPYNSAEVEKIVADEKNNRERIALEKNKDKVKEACSKHLKVAAYCTTQVERNACPFCKARKLDDKFYQKLRGQFPDALFWQEIGEIFRQLQKQAAEIYNQSLIELYYEIFIKGKGFANASSVEHYLSDVCYTRAAELFKNAAIASGLRGKVKSNFRLKELKNMRSGLPTTKSDNFPIPLVKQKGGQYTGFEISSHNDDFIIKIPFGRWQVKEEIDKYRPWEKFDFEQVRKNPKPISLLLSTQRRKRNKGWSKDEGTEAEIRKVMNGDYQTSYIEVKRGSKIGEKSAWMLNLSIDVPKIDKGVDPSIIGDIDVGVKSPLVCAINNALSRYSISDNDLFHFNKKMFARRRILLKKNRHKRAGHGAKNKLKPISILTEKSKRFRKKLIERWACEIADFFIKNKVGTVQMENLESMKRKEDSYFNIRLRGFWPYAEMQNKIEFKLKQYGIEIRKVAPNNTSKTCSKCGHLNNYFNFEYRRKNKFPHFKCEKCNFKEDADYNAALNISNPKLKSTKEEP

SEQ ID NO: 3496 - protein, 726 aa, synthetic construct
SEVEFSHEYWMRHALTLAKRARDEREVPVGAILVLNNRVIGEGWNRAIGLHDPTAHAEIMALRQGGLVMQNYRLTEATLYVTFEPCVMCAGAMIHSRIGRVVFGVRNSKRGAAGSLMNVLDYPGMGHRVEITEGILADECAALLCDFYRMPRQVFNARKKAQSSINPGGSSGGSSGSETPGTSESATLENSGGSSGGSAKNTITKTLKLRIVRPYNSAEVEKIVADEKNHREKIALEKNKDKVKEACSKHLKVAAYCTTQVERNACLFCKARRLDDRFYQKLRGQFPDAVFWQETGEIFRQLQRQAAEVYNQSLVELYYEILIKGKGIANASSVEHYLSDVCYTRAAELFKNAAIASGLRNKIKSNFRLKELRNMKSGLPTTKSDNFPIPLVKQKGGQYTGFEISSHDSDFIIKIPFGRWQVREEIDKYRPWEKFDFEQVRKSPKPISLLLSTQRRKKNKGWSKDEGTEAEIRRVMNGDYQTSYIEVKRGSKIGEKSAWMLNLSIDVPKIDKGVDPSIVGGIDVGVKSPLVCAINNSFSRYSICDNDLFRFNKKMFARRRILLKKNRHKRAGHGAKNKLKPITVLTKKSERFRKKLIERWVCEVADFFIKNKVGTVQMENLESMKRKEDSYFNIRLRGFWPYAEMQNRIELKLKQYGIEIRRVAPNNTSRTCSKCGHLNSYFNFEYRKKNKFPHFKCEKCNFKENADYNAALNISNPKLKSTKEEP

SEQ ID NO: 3497 - protein, 726 aa, synthetic construct
SEVEFSHEYWMRHALTLAKRARDEREVSVGAILVLNNRVIGEGWNRAIGLHDPTAHAEIMALRQGGLVMQNYRLTDATLYATFEPCVMCAGAMIHSRIGRVVFGVRNSKHGAAGSLMNVLNYPGMNHRVEITEGILADECAGLLCDFYRMPRQVFSARKKAQSNINSGGLSGGSSGSETPGASESPTPESSGGSSGGPAKNTITKTLQLRIVRPYNSAEVEKIVADEKNSREKIALEKNKGKVKEACSKHLEVAAYCTTQVERNACLFCKARKLDDKFYQKLRGQFPDAVFWQELGEIFRQLQKQAAEIYNQSLIELYYEIFIKGKGFANASSVEHYLSDVCYTRAAELFKNAAIASGLRGKVKSNFRLKELKNMKSGLPTTKSDNFPIPLVKQKGGQYTGFEISSHDDDFIIKIPFGRWQVRKEIDKYRPWEKFNFEQVRKSPKPISLLLSTQRRKRNKGWSKDEGTEAEIRKVMNGDYQTSYIEVKRGSKIGEKSAWMLNLSIGVPKIDKGVDPSIIGGIDVGVKSPLVCAVNNAFSRYSISDNDLFHFNKKMFARRRILLKKNRHKRAGHGAKNKLKPITIMTERSKRFRKKLIERWACEIADFFIKNKVGTVQMENLESMKRREDSYFNIRLRGFWPYAEMQNKIEFKLKQYGIVVRKVAPNNTSKTCSKCGHLNNYFNFEYRKKNKFPHFKCEKCNFKEDADYNAALNISNPKLKSTKGEP

SEQ ID NO: 3498 - protein, 726 aa, synthetic construct
SEVEFSHEYWMRHALTLAKRARDEREVPVGAVLVLNNRVIGEGWNRAIGLHDPTAHAEIMALRQGGLVMQNYRLTDATLYVTFEPCVMCAGAMIHSRIGRVVFGVRNSKHGTAGSLMNVLNYPDMNHYVEITGGILVDECAALLCDFYRMPRQVLNSQKKAQSSISSGGSSGGSSGGETPGASESPTPESSDGSPGGSAKNTITKTLKLRIVRPYNSAEVEKIVADEKNNREKIALEKNKDKVKEACSKHLKVAAYCTTQVERNACLFCKARRLDDKFYQRLRGQFPDAVFWQEIGEIFRQLQKQAAEVYNQSLVELYYEILIKGKGIANASSVEHYLSDVCYTRAAELFKNAAIASGLRNKIKSNFRLKELRNMKSGLPTTKSDNFPIPLVRQKGGQYTGFEISNHNGDFIIKIPFGRWQVKKEICKHRPWEKFDFEQVRKSPKPISLLLSTQRRKRNKGWGKDEGTEAEIRKVMNGDYQTSYIEVKRGSKIGEKSAWMLNLSIDVPKIDKGVDPSIIGGIDVGVKSPLVCAINNAFSRYSISDNDLFHFNKKMFARRRILLKKNGHKRAGHGAKNKLKPIAIMTEKSKRFRKKLIERWACEIADFFIKNKVGTVQMEDLESMKRKEDSYFNIRLRGFWPYAEMQNKIEFKLKQYGIVVRKVAPNNTSKTCSKCGHLNNYFNFEYRKKNKFPHFKCEKCNFKEDADYNAALNISNPKLKSTKGEP

SEQ ID NO: 3499 - protein, 726 aa, synthetic construct
SEVEFSHEYWMRHALTLAKRARDEREVPVGAILVLNNRVIGEGWNRAIGLHDPTAHAEIMALRQGGLVMQNYRLIDATLYVTFEPCVMCAGAMIHSRIGRVVFGVRNSKHGAAGSLVNVLNYPGMNHRVEITEGILADECAALLCDFYRMPRQVFNARKKAQSSINPSGSSGGSSGSVTPGTSESATPESSGGGFGGSAKNTITKTLQLRIVRPYNSAEVEKIVADEKNNREKIALEKNKDKVKEACSKHLKVASYCTTQVERNACLFCKARKLDDKFYQKLRGQFPDAVFWQELGEIFRQLQKQAAEIYNQSLIELYYVIFIKGKGLANASSVEHYLSDVCYTRAAELFKNAAIASGLRGKVKSNFKLKELKSMKSGLPSTKSDNFPIPLVKQRGGQYTGFEISSHNDDFIIKIPFGRWQAKKEIDKYRPWEKFDFEQVRKSPKPISLLLSTQRRKRNRGWSKDEGTEAEIRKVMNGDYQTSYIEVKRGSKIGEKSAWMLNLSIDVPKIDKGVDPSIIGGIDVGVKSPLVCAINNAFSRYSISDNDLFRFNKKMFARRRILLGKNRHKRAGHGVKNKLKPITILTEKSGRFRKKLIERWACEIADFFVKNKVGTVQMENLESMKRKEDSYFNIRLRGFWPYAEMQNKIEFKLKQYGIKVRKVAPNNTSKTSSKCGHLNNYFSFEYRKKNKFPHFKCEKCNFKENADYNAALNISNPKLKGTKEEP

SEQ ID NO: 3500 - protein, 726 aa, synthetic construct
SEVEFSHEYWMRHALTLAKRARDEREVPVGAVLVLNNRVIGVGWNRAIGLHDPTAHAEIMALRQGGLVMQNYRLIDATLYVTFEPCAMCAGAMVHSRIGRVVFGVRNGKRGAAGSLMNVLDYPGMGHRVEITEGILADECAALLCDFYCMPRQVFNAQKRAQSSINSGGSSGGSSGSETPGTSEGATPGSSGGGSSGSAKNTITKTLQLRIVRPYNSAEVEKIVADEKNNREKIALEKNKDKVKEACSKHLKVASYCTTQVERNAWLFCKARKLDDKFYQKLRGQFPDAVFWQEIGEIFRQLQKQAAEVYNQSLVELYYEILIKGKGIANASSVEHYLSDVCYTRAAELFKNAAIASGLRGKVKSNFRLKELRNMKSGLPTTKSDNFPIPLVRQKGGQYTGFEVSSHNDDFIIKIPFGRWQVRKEIDRYRPWEKFDFEQVRKSPKPISLLLSTQRRKRNKGWSKDEGTEAEIRRVMNGDYQTSYIEVKRGSKIGEKSAWMLNLSIDVPKIDKGVDPGIIGGIDVGVKSPLVCAINNASSRYSISDNDLFHFNKKMFARRRILLKKNRHKRAGHGAKNKLKPITIMTEKSKRFRKKLIERWACEIADFFIKNKVGTVQMENLESMKRKEDSYFNIRLRGFWPYAEMQNKIEFKLKQYGIEIRKVAPNNTSKTCSMCGHLNNYFSFEYRKKNKFPHFKCEKCNFKENADYNAALNISNPKLMSAKEGP

SEQ ID NO: 3501 - protein, 726 aa, synthetic construct
SEVEFSHEYWMRHALALAKRARDEREVLVGAVLVLNNRAIGEGWNRAIGLHDPTAHAEIMALRQGGLVMQNYRLTDATLYVTFEPCVMCAGAMIHSRIGRVVFGVRNSKRGAAGSLMNVLNYPGMNHCVEITEGILVDECAALLCDFYRMPRQVLSARKKAQPSANSGGSSDGGSGSETPGTSESATPESSGGSSGGSAKNTITKTLKLRIVRPYNSAEVEKIVADEKNNREKIALEKNKDKVKEACSEHLKVAAYCTTRVERNACLFCKARKLDDKFYQKLRGQFPDAVFWQETGEIFRQLQRQAAEIYNQSLIELYYEIFIKGKGITNASRVEHYLSDVCYTRAAELFKNAAIASGLRSKVRSNFRLKELKNMKSGLPTTKSDNFPIPLVKQKGGQYTGFEISSHNSDFIIKIPFGRWQVKEEIDKYRPWEKFDFEQVRKSPKPISLLLSTQRRKKNKGWSKDEGTEAEIRRVMNGVYQTSYIEVKRGSKIGEKSAWMLNLSIDVPKIDKGVDPSIIGGIDVGVKSPLVCAINNAFSRYSISDNDLFRFNKKMFARRRILLKKNRHKRAGHGAKNKLKPISILTGKSERFRKKLIERWACEIADFFIKNKVGTVQMENLESMKRKEDSYFNIRLRGFWPYAEMQNKIEFKLKQYGIEIRKVAPNNTSKTCSKCGHLNNYFNFEYRKMNKFPHFKCEKCNFKENADYNAALNISNPKLKSTKEEP

SEQ ID NO: 3502 - protein, 726 aa, synthetic construct
SEVEFSHEYWMRHALTLAKRARDEREVPVGAILVLNNRVIGEGWNRAIGLHDPTAHAEIMALRQGGLVMQNYRLTDATLYVTFEPCVMCAGAMIHSRIGRVVFGVRNSKRGAAGSLMNVLNYPGMNHCVEITEGILVDECAALLCDFYRMPRQVLNAQKKAQPSISSGGSSGGCSGSEMPGASESVTPKSSGGSSAGSTKNTITKTLKLRIVRPYNSAEVEKIVADEKNSREKIALEKNKDKVKEACSEHLKVAAYCTTQVERNACLFCKARKLDDKFYQKLRGQFPDAVFWQEIGEIFRKLQKQAAEIYNQSLIELYYEIFIKGRGFASASSVEHYLSDVCYTRAAELFKNAAIASGLRGKVKSNFRLKELKNMRSGLPTTKSDNFPIPLVKQKGGQYAGFEISSHNDDFIIKIPFGRWQAKKEIDKYRPWEKFDFEQVRKSPKPISLLLSTQRRKRNKGWSKDEGTEAEIRKVMNGDYQTSYIEVKRGSKIGEKSAWMLNLSIDVPKIDKGVDPSIIGGIDVGVKSPLVCAINNAFSRYSISDNDLFRFNKKMFARRRILLRKNRHKRAGHGAKNKLKPISILTGKSERFRKKLIERWACEIADFFIKNKVGTVQMENLESMKRKEDSYFNIRLRGFWPYAEMQNKIEFKLKQYGIKIRKVAPNNTSKTCSKCGHLNNYFSFEYRKKNKFPHFKCEKCSFKENADYNAALNISNPKLKSTKEEP

SEQ ID NO: 3503 - protein, 726 aa, synthetic construct
SEVEFSHEYWMRHALTLAKRARDEREVPVGAVLVLNNRVIGVGWNRAVGLHDPTAHAEIMALRQGGLVMQNYRLIDATLYVTFEPCVMCAGAMIHSRIGRVVFGVRNSKHGAAGSLMNVLNYPGMNHRVEITEGILADECAALLCDFYRMPRQVFNARKKAQSSINPGGPSGGSSGSETPDTSESATPESSGGNSGGSAKNTITKTLKLRIVRPYNSAEVEKIVADEKNNREKIALEKNKDKVKEACSEHLKVAAYCTTQVERNACLFCKARKLDDKFYQKLRGQFPDAVFWQETGEIFRQLQRQAAEIYNQSLIELYYEIFIKGKGITNASRVEHYLSDVCYTRAAELFKNAAIASGLRSKVRSNFRLKELKNMKSGLPTTKSDNFPIPLVKQKGGQYTGFEISSHNSDFIIKIPFGRWQVRKEIDKYRPWEKFNFEQVRMSPKPISLLLSTQRRKGNKGWSKDEGTEAEIKRVMNGDYQTSYIEVKRGSKTGEKSAWMLNLSIDVPKIDKGVDPSIIGGIDVGVKSPLVCAINDAFNRYSISDNNLFHFNKKMFARRRILLKKNRHKRAGHGAKNKLKPISILTGKSERFRKKLIERWACEIADFFIKNKVGTVQMENLESMKRKEDSYFNIRLRGFWPYAEMQNKIEFKLKQYGIEIRKVAPNNTSKTCSKCGHLNNYFNFEFRKKNKFPHFKCEKCNFKENADYNAALNISNPKLKSTKEEP

SEQ ID NO: 3504 - protein, 726 aa, synthetic construct
SEVEFSHEYWMRHALTLAKRARDEREVPVGAVLVLNNRVIGEGWNRTTGLHDPTAHAEIMALRQGGLVMQNHRLVDATLYVTFEPCVMCAGAMIHSRIGRVVFGVRNSKRGAAGSLTNVLNYPGMNHRVEITEGILVDECAALLCDFYRMPRQVFNAQKKAQSTINSGGSSGGSSGSETPGDSESATSESSGGSSGGSAKNTITKTLKLRIVRPYNSAEVEKIVADEKNNREKIALEKNKDKVKEACSRHLKVAAYCTTQVERNACLFCKARKLDDKFYQKLGGQFPDAVFWQEISEIFRQLQKQAAEIYNQSLIELYYEIFIKGKGFANASSVEHYLSDVCYTRAAELFKNAAIASGLRGKVKGNFRLKELKNMKSGLPTTKSDNFPIPLVKQKGGQYTGFEISSHNDDFIIKIPFGRWQVKKEIDKYRPWEKFDFEQVRKSPKPISLLLSTQRRKRNKGWSKDEGTEAEIRKVMNGDYQTSYIEVKRGSRTGEKSAWMLNLSIDVPKIDKGVDPSIIGGIDVGVKSPLVCAINNAFSRYSISDNDLFRFNKKMFARRRILLKKNRHKRAGHGAKNKLKPITILTKKSERFRKKLIERWVCEVADFFIKNKVGTVQMENLESMKRKEDSYFNIRLRGFWPYAEMQNRIELKLKQYGIEIRRVAPNNTSRTCSKCGHLNNYFNFEYRKKSKFPHFKCEKCNFREDADYNAALNISNPKLKSTKEEP

SEQ ID NO: 3505 - protein, 726 aa, synthetic construct; identical to SEQ ID NO: 3476

SEQ ID NO: 3506 - protein, 726 aa, synthetic construct
SEDEFSHEYWMRHALTLAKRARDGREVPVGAVLVLNNRVIGEGWNRAIGLHDPTAHAEIMALRQGGLVLQNYRLVDATLYVTFEPCVLCAGAMVHSRIGRVVFGARNSKRGAAGSLMNILNYPGMNHRVEITEGILADECAALLCDFYRMPRQVFNAQKKAQSSINSGGSSGGSSGSETPSTSECATPESSGGSSGGSAKNTTTKTLQLRIVRPYNSAEVEKIVTDEKNNREKIALEKNKDKVKEACSEHLKVAAYCTTQVERNACLFCKARKLDDGFYQKLRGQFPDAVFWQEIGEIFRQLQKQAAEIYNQSLIELYYEIFIKGKGITNASRVEHYLSDVCYTRAAELFKNAAIASGLRSKVRSNFRLKELKNMKSGLPSTKSDNFPIPLVKQRGGQYTGFEISSHNDDFIIKIPFGRWQAKKEIDKYRPWEKFDFEQVRKSPKPISLLLSTQRRKRNRGWSKDEGTEAEIRKVMNGDYQTSYIEVKRGSKIGEKSAWMLNLSIDVPKIDKGVDPSIIGGIDVGVKSPLVCAINNALGRYSISDNDLFHFNKKMFARRRILLKKNRHRRAGHGARNKLKPITVLTEKSKRFRKKLIERWACEIANFFVKNKVGTVQMENLESMKRKEDSYFNIRLRGLWPYAEMQNKIEFKLKQYGIEIRKVAPDNTSKTCSKCGHLNNYFNFEYRKKNKFPHFKCEKCNFKEDADYNAALNISNPKLKSTKEEP

SEQ ID NO: 3507 - protein, 726 aa, synthetic construct
SEVEFSHEYWMRHALTLAKRARDEREVPVGAVLVLNNRVIGEGWNRAIGLHDPTAHAEIMALRQGGLVMQNYRLTDATLYVTFEPCVMCAGAMVHSRIGRVVFGVRNSKRGAAGSLMNVLNYPGVNHCVEITEGILVDECAALLCDFYRMPRQVLNAQKKAQSSINSGGSSGGNSGNKTPGASESVTPKSSGGSSGGSAKNTITKTLKLRIVRPYNSAEVEKIVADEKNNREKIALEKNKGKVKEACSKHLKVAAYCTTQVERNACLFCKARRLDDKFYQKLRGQFPDAVFWQEIGEIFRQLQKQAAVIYNQGLIELYYEIFIKGKGIANASRVEHYLSNVCYTRAAELFKNAAIASGLRNKIKSNFRLKELRNMKSGLPTTKSDNFPIPLVRQKGGQYTGFEISNHNSDFTIKIPFGRWQVKKEIDKYRPWERFDFEQVRKSPKPISLLLSTQRRKRNKGWGKDEGTEAEIRKVMNGDYQTSYIEVKRGSKIGEKSAWMLNLSIDVPKIDKGVDPSIIGGIDVGVKSPLVCAINNAFSRYSISDNDLFRFNKKVFARRRILLGKNRHKRAGHGVKNKLKPITILTEKSGRFRKKLIERWACEIADFFIKNKVGTVQMENLESMKRKEDSYFNIGLRGFWPYAEMQNKIEFKLKQYGIGIRKVAPNNTSKTCSKCGHLNNYFNFEYRKKNKFPYFKCEKCNFKENADYNAALNISNPQLKSTKGEP

SEQ ID NO: 3508 - protein, 726 aa, synthetic construct
SEVEFSHEYWMRHALSLAKRARDEREVPVGAVLVLNNRIIGEGWNRAIGLHDPTAHAEIMALRQGGLVMQNYRLTDATLYVTFEPCVMCAGAMVHSRIGRVVFGVRNSKRGAAGSLMNVLNYPGVNHCVEITEGILVDECAALLCDFYRMPRQVLNAQKKAQSSISSGGPSGGCSGSEMPGASGSVTPKSSGGSSAGSTKNTITKTLKLRIVRPYNSAEVEKIVADEKNSREKIALERNKDRVKEACSEHLKVAAYCTTQVERNACLFCKARKLDDRFYQKLRGQFPDAVFWQETGEIFRQLQRQAAEIYNQSLIELYYEIFIKGKGFANASSVEHYLSDVCYTRAAELFKNAAIASGLRGKVKSNFRLKELKNMKSGLPTTKSDNFPIPLVKQKGGQYTGFEISSHNDDFIIKIPFGRWQVKKEIDRYRPWEKFDFEQVRKSPKPISLLLSTQRRKRNKGWSKDGGTEAEIRKVMNGDYQTSYIEVKRGSKIGEKSAWMLSLSIDVPKIDKGVDPSTIGGIDVGVKSPLVCAINNAFCRYSISDNDLFHFNKKMFARRRILLKKNRHKRAGHGAKNKLKPITILTKKSERFRKKLIERWVCEVADFFIKNKVGTVQMENLESMKRKEDSYFNIRLRGFWPYAEMQNRIELKLKQYGIEIRRVAPNNTSRTCSKCGHLNNYFNFEYRKMNKFPHFKCEKCNFKENADYNAALNISNPKLKSTKEEP

SEQ ID NO: 3509 - protein, 726 aa, synthetic construct
SEVEFSHEYWMRHALTLAKRARDEREVPVGAILVLNNRVIGEGWNRAIGLHDPTAYAEIMALRQGGLVLQNYRLVDATLYVTFEPCVMCAGAMIHSRIGRVVFGVRNSKHGAAGSLVNVLNYPGMNHRVEITEGILADECAALLCDFYRMPRQVFGARRKAQSSINPGGSSGGSSSSETPGTSESPTPESPGGSSGGSAKNTITKALKLRIVRPYNSAEVEKIVADEKNNRERIALEKNKDKVKEACSKHLKVAAYCTTQVERNACLFCKARKLDDKFYQKLRGQFPDAVFWQEIGEIFRQLQKQAAEIYNQSLIELYYEIFIKGKGFANASSVEHYLSDVCYTRAAELFKNAAIASGLRGKVKSNFRLKELKNMRSGLPTTKSDNFPIPLVKQKGGQYAGFEISSHNDDFIIKIPFGRWQVKKEIDKYRPWEKFDFEQVRKSPKPISLLLSTRRRKRNRGWSKDEGTEAEIRKVMNGDYQTSYIEVKRGSKIGEKSAWMLNLSIDVPKIDKGVDPSIIGGIDVGVKSPLVCAINNAFSRYSISDNDLFCFNKKMFARRRILLGKNRHKRAGHGVKNKLKPITILTEKSGRFRKKLIERWACEIADFFVKNKVGTVQMENLESMKRKEDSYFNIRLRGFWPYAEMQNKIEFKLKQYGIKVRKVAPNNTSKTCSKCGHLNNYFSFEYRKKNKFPPFKCEKCNFKENADYNAALNISNPKLKGTKEEP

SEQ ID NO: 3510 - protein, 726 aa, synthetic construct
SEVEFSHEHWMRHALTLAKRARDEREVPVGAVLVLNNRVIGEGWNRAIGLHDPTAHAEIMALRQGGLVMQNYRLIDATLYVTFEPCVMCAGAMIHSRIGRVVFGVRNSKHGAAGSLVNVLNYPGMNHRVEITEGILADECAALLCDFYRMPRQVLNAQKKAQSSISSGGSSGGSSGSETPGASGSVTPKSSGGSSAGSTKDTITKTLKLRIVRPYNSAEVEKIVADEKNSREKIALERNKDKVKEACSEHLKVAAYCTTQVERNACLFCKARKLDDRFYQKLRGQFPDAVFWQETGEIFRQLQRQAAEIYNQSLIELYYEIFIKGKGFANAGSVEHYLSDVCYTRAAELFKNAAIASGLRGKVKSNFRLKELKNMKSGLPTTKSDNFPIPLVKQKGGQYTGFEISSHNDDFIIKIPFGRWQVKEEIDKYRPWEKFDFEQVRKNPKPISLLLSIQRRKRNKGWSRDEGTEAEIRKVMNGDYQTSYIEVKRGSKIGEKSAWMLNLSIDVPKIDKGVDPSIIGGIDVGVKSPLICAINNAFSRYGICDNDLFHFNKKVFARRRILLKKNRHKRAGHGTKNKLKPITILTEKSGRFRKKLIERWACEIANFFIKNKVGTVQMENLESMKRKEDSYFNIRLRGFWPYAEMQNKIEFKLKQYGIVVRKVAPNNTSKTCSKCGHLNNYFNFEHRKKNKFPHFKCEKCNFKENADYNAALNISNPKLKSTKGEP

SEQ ID NO: 3511 - protein, 725 aa, synthetic construct
SEVEFSHEYWMRHALTLAKRARDEREVPVGAVLVLNNRAIGEGWNRAIGLHDPTAHAEIMALRQGGLVMQNYRLTDATLYVTFEPCVMCAGAMIHSRIGRVVFGVRNSKRGAAGSLMNVLNYPGMNHCVEITEGILVDECAELLCDFYRMPRQVLNAQKRAQSSISSGGSSGGSSGSETPGASESATPKSSGGSSASSTKNTITKTLKLRIVRPYNSAEVEKIVADEKNNREKIALEKNKDKVKEACSEHLKVAAYCTTQVERNACLFCKARKLDDKFYQKLRGQFPDAVFWQETGEIFRQLQRQAAEIYNQSLIELYYEIFIKGKGFANASSVEHYLSDVCYTRAAELFKNAAIASGLRGKVKSNFRLKELKNMKSGLPTTKSDNFPIPLVQKGGQYTGFEISSHNDDFIIKIPFGRWQVKKEIDKYRPWEKFDFEQVRKSPKPISLLLSTQRRKRNKGWSKDEGTEAEIKKVMNGDYQTSYIEVKRGSKTGEKSAWMLNLSIDVPKIDKGVDPCIIGGIDVGVKSPLVCAINNAFSRYCISDNDLFHFNKKMFARRRILLKKNGHKRAGHGAKNKLKPITIMTEKSKRFRKKLIERWACEIADFFIKNKVGTVQMENLESMKRKEDSYFNIRLRGFWPYAEMQNKIEFKLKQYGIVVRKVAPNDTSKTCSKCGHLNNYFNFEYRKKNKFPHFKCEKCNFKENADYNAALNISNPKLKSTKGEP

SEQ ID NO: 3512 - protein, 726 aa, synthetic construct
SEVEFSHEYWMRHALTLAKRARDEREVPVGAVLVLNNRVIGEGWNRAIGLHDPTAHAEIMALRQGGLVMQNYRLVEATLYVTFEPCIMCAGAMIHSRIGRVVFGVRNSKRGAAGSLMNVLNYPGMNHRVEITEGILADECAALLCDYYRMPRQVFNARKKAQSSINSGGSSDGGSGSETPGTSESATPESSGGSSGGSAKNTITKTLKLRIVRPYNSAEVEKIVADEKNNREKIALEKNKDKVKEACSEHLKVAAYCTTQVERNACLFCKARKLDDKFYQKLRGQFPDAVFWQEIGEIFRQLQKQAAEIYNQSLIELYYEIFIKGKGFANASSVEHYLSDVCYTRAAELFKNAAIASGLRGKVKSNFRLKELKNMRSGLPTTKSDNFPIPLVKQKGGQYTGFEISSHNDDFIIKIPFGRWQVKKEIDKYRPWEKFDFEQVRKSPKPISLLLSTQRRKRNKGWSKDEGTEAEIRKVMNGDYQTSYIEVKRGSKIGEKSAWMLNLSIGVPKIDKGVDPGIIGGIDVGVKSPLVCAINNASSRYSISDNDLFHFNKKMFARRRILLKKNRHKRAGHSAKNKLKPITIMTEKSKRFRKKQIERWACEIADFFIKNKVGTVQMENLESMKRKEDSYFNIRLRGFWPYAEMQNRIEFKLKQYGIEIRKVAPNNTSKTCSKCGHLNNYFNFEYRKKNKFPHFKCEKCNFKENADYNAALNISNPKLKSTKEES

SEQ ID NO: 3513 - protein, 726 aa, synthetic construct
SEVEFSHEYWMRHALTLAKRARDEREVPVGAILVLNNRVIGEGWNRAIGLHDPTAHAEIMALRQGGLVMQNYRLIDATLYVTFEPCVMCAGAMIHSRIGRVVFGVRNNKHGAAGSLVNVLNYPGMNHRVEITEGILADECAALLCDFYRMPRQVFNARKKAQSSINPGGSSGGSSGSETPGTSESATPESSGGSSGSSAKNTITKTLKLRIVRPYNSAEVEKIVADEKNNREKIALEKNKDKVKEACSKHLKVAAYCTTQVERNACLFCKARRLDDKFYQKLRDQFPDAVFWQELGEIFRQLQKQAAEIYNQSLIELYYEIFIKGKGITNASRVEHYLSDVCYTRAAELFKNAAIASGLRSKVRSNFRLKELKNMKSGLPTTKSDNFPIPLVKQKGGQYTSFEISSHNSDFIIKIPFGRWQVKEEIDKYRPWEKFDFEQVRRSPKPISLLLSTQRRKKNKGWSKDEGTEAEIRKVMNGDYQTSYIEVKRGSKIGEKSAWMLNLSIDVPKIDKGVDPSIIGGIDVGVKSPLVCAINNAFSRYSISDNDLFRFNKKMFARRRILLKKNRHQRAGHGAKNKLKPITILTEKSGRFRKKLIERWACEIADFFIKNKVGTVQMENLESMKRKEDSYFNIRLRGFWPYAEMQNKIEFKLKQYGIKIRKVAPNNTSKTCSKCGHLNNYFSFEYRKKNKFPHFKCEKCNFKENADYNAALNISNPKLMSTKEEP

SEQ ID NO: 3514 - protein, 726 aa, synthetic construct
SEVEFSHEYWMRHALTLAKRARDEREVSVGAVLVLNNRVIGEGWNRAIGLHDPTAHAEIMALRQGGLVMQNYRLVDATLYVTFEPCVLCAGAMVHSRIGRVVFGVRNSKRGAAGSLMNVLNYPGMNHRVEITEGILADECAALLCDFYRMPRQVFNAQKKARSNINSGGSSGGSSGSETPGTSESATPVSSSGSSGGSAKNTITKTLKLRIVRPYNSAEVEKIVADEKNNREKIALAKNKDKVKEACSEHLKVAAYCTTQVERNACLFCKARKLDDRFYQKLRGQFPDAVFWQEIGEIFRQLQKQAAEIYNQSLIELYYEIFIKGKGFANASSVEHYLSDVCYTRAAELFKNAAIASGLRGKVKSNFRLKELKSMKSGLPTTKSDNFPIPLVKQKGGQYTGFEVSSHNDDFIIKIPFGRWQVKKEIDKYRPWEKFDFEQVRKSPRPISLLLSTQRRKRNKGWSKDEGTEAEIRKVMNGDYQTSYIEVKRGSKIGEKSAWMLNLTIDVPKIDKGVDPSIIGGIDVGVKSPLVCAIDNAFSRYSISDNDLYHFNKKMFAKRRILLKKNRHKRAGHGVKNKLKPISILTGKSERFRKKLIERWACEIADFFIKNKVGTVQMENLESMKRKEDSYFNIRLRGFWPYAEMQNKIEFKLKQYGIEIRKVAPNNTSKTCSKCGHLNNYFNFEYRKKNKFPHFKCEKCNFKENADYNAALNISNPKLKSTKEKP

SEQ ID NO: 3515 - protein, 726 aa, synthetic construct
SEVEFSHEYWMRHALTLAKRARDEREVPVGAILVLNNRVIGEGWNRAIGLHDPTAHAEIMALRQGGLVMQNYRLIDATLYVTFEPCVMCAGAMIHSRIGRVVFGVRNSKHGAAGSLMNVLNYPGMNHRVEITEGILADECAALLCDFYRMPRRVFNARKKAQPSISSGGPSGGSSGSKTPGTSESATPESSGGSSGGSAKNSITKTLKLRIVRPYNSAEVEKIVADEKNNREKIALEKNKDKVKEACSKHLKVASYCTTQVERNACLFCKARKLDDRFYQKLRGQFPDAVFWQELGEILRQLQKQAAEVYNQSLIELYYEIFIKGRGFANASSVEHYLSDVCYTRAAELFKNAAIASGLRGKVKSNFRLKELKNMKSGLPTTKSDNFPIPLVKQKGGQYTGFEISSHNDDFIIKIPFGRWQVKKEIDKYRPWEKFDFEQVRKSPKPISLLLSTQRRKRNKGWSKDEGTEAEIRKVMNGDYQTSYIEVKRGSKTGEKSAWMLNLSIDVPKIDKGVDPSIIGDIDVGVKSPLVCAINNAFSRYSISDNDLFRFNKKMFARRRILLKKNRHKRAGHGAKNKLKPISTLTERSKRFRKKLIERWACEIADFFIKNKVGTVQMENLESMKRKEDSYFNIRLRGFWPYAEMQNRIELKLKQYGIEIRRVAPNNTSRTCSKCGHLNNYFNFEYRKKNKFPHFKCEKCNFREDADYNAALNISNPKLKSTKEEP

SEQ ID NO: 3516 - protein, 726 aa, synthetic construct
SEDEFSHEYWMRHALTLAKRARGEREVPVGAVLVLNNRVIGEGWNRAIGLHDPTAHAEIMALRQGGLVMQNYRLTDATLYVTFEPCVMCAGAMIHSRIGRVVFGVRNSKRGAAGSLMNVLNYPGMNHCVEITEGILMDECAALLCDFYRMPRQVLNAQKKAQSSISSGGPSGGSSCSETSGASESVTPKSSGGSSTGSTKNTITKTLKLRTVRPYNSAEVEKIVADEKNSREKIALEKNKDKVKEACSEHLKVAAYCTTQVERNACLFCKARKLDDRFYQKLRGQFPDAVFWQEIGEIFRQLQKQAAEIYNQSLIELYYEIFIKGKGFAIASSVEHYLSCVCYTRAAELFKNAAIASGLRGKVKSNFRLKELKNMKSGLPTTKSDNFPIPLVKQKGGQYTGFEISSHNDDFIIKIPFGRWQVKKEIDKYRPWEKFDFEQVRKSPKPISLLLSTQRRKRNRGWSKDEGTEAEIRKVMNGDYQTSYIEVKRGSKIGEKSAWMLNLSIDVPKIDKGVDPSIIGGIDVGVKSPLVCAINNAFSRYSISDNDLFRFNKKMFARRRILLKKNRHKRAGHGAKNKLKPISILTRKSERFRKKLIERWACEIADFFIKNKVGTVQMENLESMKRKEDSYFNIRLRGFWPYAEMQNKIEFKLKQYGIEIRKVAPNNTSKTCSKCGHLNNYFNFEYRKKNKFPHFKCEKCNFKENADYNAALNISNPKLKSTKGEP

SEQ ID NO: 3517 - protein, 726 aa, synthetic construct
SEVEFSHEYWMRHALTLAKRARDEREVPVGAVLVLNNRVIGEGWNRAIGLHDPTAHAEIMALRQGGLVMQNYRLIDATLYVTFEPCVMCAGAMVHSRIGRVVFGVRNSKRGAAGSLMNVLDYPGMGHRVEITEGILADECAALLCDFYRMPRQVLSAQKKAQSSISSGGSSGGSSGSETPGTSESATPESSGGSSGSSAKNTITKTLKLRIVRPYNSAEVEKIVVDEKNNREKIALEKNKDKVKEACSKHLKVAAYCTTQVERNACLFCKARRLDDKFYQKLRGQFPDAVFWQEIGEIFRQLQKQAAEVYNQSLVELYYEILIKGKGIANASSVEHYLSDVCYTRAAELFKNAAIASGLRNKIKSNFRLKELRNMKSGLPTTKSDNFPVPLVRQKGGQYTGFEISNHDGDFIIKIPFGRWQVKKEINKHRPWEKFDFEQVRKSPKPISLLLSTQRRKRNKGWSKDEGTEAEIRKVMNGDYQTSYIEVRRGSKIGEKSAWMLNLSIDVPKIDKGVDPSIIGGIDVGVKSPLVCAINNALSRYSISDNDLFHFNKKMFARRRILLRKNRHKRAGHGAKNKLKPITIMTEKSKRFRKKLIERWACEIADFFIKNKVGTVQMENLESMKRKEDSYFNIRLRGFWPYAEMQNKIEFKLKQYGIVVRKVAPNNTSKTCSKCGHLNDYFNFEYRKKNKFPHFKCEKCNFREDADYNAALNISNPKLKSTKGEP

SEQ ID NO: 3518 - protein, 726 aa, synthetic construct
SEVEFSHEYWMRHALALARRARDEREVPVGAILVLNNRVIGEGWNRAIGLHDPTAHAEIMALRQGGLVMQNYRLVDATLYVTFEPCVMCAGVMIHSRIGRVVFGVRNNKHGAAGSLMNVLNCPGMNHCVEITEGILVDECAALLCDFYRMPRQVLNAQKKAQPSISPGGSSGGSSGSETPGASESVTPKSSGGSSAGSTKNTITKTLKLRIVRPYNSAEVEKIVADEKNSREKIALEKNKDKVKEACSEHLKVAAYCTTQVERNACLFCKARKLDDRFYQKLRGQFPDAVFWQEIGEIFRQLQKQAAEIYNQSLIELYYEIFIKGKGFANASSAEHYLSDVCYTRAAELFKNAAIASGLRGKVKSNFRLKELKNMKSGLPTTKSDNFPIPLVKQKGGKYTGFEISSHNDDFIIKIPFGRWQVKKEIDKYRPWEKFDFEQVRKSPKPISLLLSTQRRKRNKGWSKDEGTEAEIRKVMNGDYQTSYIEVKRGSKIGEKSAWMLNLSIDVPKIDKGVDPSIIGGIDVGVKSPLVCAINNAFSRYSISDNDLFHFNKKMFARRRILLRKNRHKRAGHGVRNKLKPITVLTEKSERFRKKLIERWACEIANFFIKNKVGTVQMENLESMKRREDSYFNIRLRGFWPYAEMQSKIEFKLKQYGIKIRKVAPNNTSKTCSKCGHLNNYFNFEFRKKNKFPHFKCEKCNLKEDADYNAALNISNPKLKSTKEEP

SEQ ID NO: 3519 - protein, 726 aa, synthetic construct
SEVEFSHEYWMRHALTLAKRARDEREVPVGAVLVLNNRVIGEGWNRAIGLHDPTAHAEIMALRQGGLVMQNYRLVDATLYVTFEPCVLCAGAMVHSRIGRVVFGVRNSKRGAAGSLTNVLDYPGMNHRVEITEGILVDECAALLCDFYRMPRQVFNAQKKAQSTINSGGSSGGSSGSETPGTSESPTPESSGGSPGGSAKNTITKTLKLRIVRPFNSAEVEKIMADEKNNRERIALEKNKDKVKEACSKHLKVAAYCTTQVERNACLFCKARKLDDKFYQKLRGQFPDAVFWQETGEIFRQLQRQAAEIYNQSLIELYYEIFIKGKGFANASSVEHYLSDVCYTRAAELFKNAAIASGLRGKVKGNFRLKELKNMKSGLPTTKSDNFPIPLVKQKGGQYTGFEISSHNDDFIIKIPFGRWQAKKEIDKYRPWEKFDFEQVRKSPKPISLLLSTQRRKRNKGWSKDEGTEAEIRKVMNGDYQTSYIEVKRGSKIGEKSAWMLNLSIDVPKIDKGVDPSIIGGIDVGVKSPLVCAINNAFSRYSISDNDLYRFNKKMFARRRILLKKNRHKRAGHGAKNKLKPLTILTGKSKRFRKKLIERWACEIAGFFIKNKVGTVQMENLESMKRREDSYFNIRLRGFWPYAEMQNKIEFKLKQYGIEIRKVAPNNTSKTCSRCGHLNNYFNFEYRKRNKFPHFKCEKCNFKENADYNAALNISNPKLKSPKEEP

SEQ ID NO: 3520 - protein, 726 aa, synthetic construct
SEVEFSHEYWMRHALTLAKRARDEREVPVGAVLVLNNRAIGEGWNRAIGLHDPTAHAEIMALRQGGLVMQNYRLTDATLYVTFEPCVMCAGAMIHSRIGRVVFGVRNSKRGAAGSLMNVLNYPGMNHCVEITEGILVDECAALLCDFYRMPRQVLNAQKKAQSSISSGGSSGGSSGSETLGTREGATPESSGGSSGGSAKNTITKALKLRIVRPYNSAEVERIVADEKNNREKIALEKNRDKVKEACSKHLKVAAYCTTQVERNACLFCKARKLDDKFYQKLRGQFPEAVFWQEIGEIFRQLQKQTAEIYNQSLIELYYEIFIKGKGVANASSVEHYLSDVCYTKAAELFKNAAIASGLRGKVKGNFRLKELKNMKSGLPTTKSDNFPIPLVKQKGGQYTGFEISSHNDDFIIKIPFGRWQAKKEIDKYRPWEKFDFEQVRKSPKPISLLLSTQRRKRNKGWSKDEGTEAEIRKVMNGDYQTSYIEVKRGSKIGEKSAWMLNLSIDVPKIDKGADPSVIGGIDVGVKSPLVCAINNAFSRYSISDNDLFRFNKKVFARRRILLKKTRHKRAGHGAKNKLKPITILTEKSGRFRKKLIERWACEIANFFIKNKVGTVQMENLESMKRKEDSYFNIRLRGFWPYAEMQNKIEFKLKQYGIKIRKVAPNNTSKTCSKCGHLNNYFDFEYRKKNKFPYFKCEKCNFKENADYNAALNISNPQLKSTKGEP

SEQ ID NO: 3521 - DNA, 24 bp, synthetic construct
  source 1..24: mol_type = other DNA
tttggttaacctcctggaccccct

SEQ ID NO: 3522 - DNA, 24 bp, synthetic construct
  source 1..24: mol_type = other DNA
tttgttataacccagggcgaagtg

SEQ ID NO: 3523 - DNA, 120 bp, synthetic construct
  source 1..120: mol_type = other DNA
gcactatgactattgcggcctctagaacgatttgatacggcannnyrnnnyrnnnyrnnnyrnnnyrnnnyrnnnyrnnnyrnnnyrnnnyrcctgcagggcgcggtaattgcttgttgc

SEQ ID NO: 3524 - DNA, 20 bp, synthetic construct
  source 1..20: mol_type = other DNA
gcactatgactattgcggcc

SEQ ID NO: 3525 - DNA, 20 bp, synthetic construct
  source 1..20: mol_type = other DNA
gcaacaagcaattaccgcgc

SEQ ID NO: 3526 - DNA, 24 bp, synthetic construct
  source 1..24: mol_type = other DNA
tttggttaacctcctggaccccct

SEQ ID NO: 3527 - DNA, 24 bp, synthetic construct
  source 1..24: mol_type = other DNA
tttggttgacctcctggaccccct

SEQ ID NO: 3528 - DNA, 76 bp, synthetic construct
  source 1..76: mol_type = other DNA
tttgccatatggtagcaatttgtacgtttggttaacctcctggaccccctcgtttgttataacccagggcgaagtg

SEQ ID NO: 3529 - DNA, 83 bp, synthetic construct
  source 1..83: mol_type = other DNA
atgcatttttgccgtatggtagcaatttgtacgtttggttgacctcctggaccccctcgtttgttgtaacccagggcgaagtg

SEQ ID NO: 3530-3532 - skipped (3 entries)

SEQ ID NO: 3533 - DNA, 20 bp, synthetic construct
  source 1..20: mol_type = other DNA
aaatccgtgataacaagctg

SEQ ID NO: 3534 - DNA, 20 bp, synthetic construct
  source 1..20: mol_type = other DNA
gcaaccactttacctgcgat

SEQ ID NO: 3535 - DNA, 36 bp, synthetic construct
  source 1..36: mol_type = other DNA
cccaccctcgtgaccaccctgacctacggcgtgcag

SEQ ID NO: 3536 - DNA, 36 bp, synthetic construct
  source 1..36: mol_type = other DNA
gggtgggagcactggtgggactggatgccgcacgtc

SEQ ID NO: 3537 - DNA, 36 bp, synthetic construct
  source 1..36: mol_type = other DNA
cccaccctcgtgaccaccctgacccacggcgtgcag

SEQ ID NO: 3538 - DNA, 36 bp, synthetic construct
  source 1..36: mol_type = other DNA
gggtgggagcactggtgggactgggtgccgcacgtc

SEQ ID NO: 3539 - DNA, 2181 bp, synthetic construct
  source 1..2181: mol_type = other DNA
agcgaagttgaatttagccacgaatactggatgcgtcatgcgttgacgctggcgaagcgtgcgcgtgacgaacgcgaggtgccggtgggtgctgttctggtgctgaacaatcgtgtaatcggtgaaggttggaatcgcgcgatcggtctgcatgatccaaccgcgcacgcagaaatcatggcgctgcgtcagggtggcctggtgatgcaaaattaccgtctgatcgatgcgacgctgtatgtgaccttcgaaccgtgtgtcatgtgtgccggtgccatgatccacagccgcattggccgtgtggtctttggcgttcgtaacagcaaacgtggcgcagcaggctctctgatgaacgtcctgaattacccgggtatgaaccatcgtgttgagattacggagggcatcttagcggatgaatgtgctgcgctgctgtgcgatttctatcgcatgccgcgtcaagtctttaacgcacagaagaaggcacaatctagcattaactctggcggttcgtctggtggtagcagcggcagcgaaacgccgggtaccagcgagagcgcaaccccggagagctccggtggcagctctggcggctctgccaagaacaccatcaccaagaccctgaagctgaggatcgtgaggccctacaacagcgccgaggtggagaagatcgtggccgacgagaagaacaacagggagaagatcgccctggagaagaacaaggacaaggtgaaggaggcctgcagcaagcacctgaaggtggccgcctactgcaccacccaggtggaaaggaacgcttgcctgttctgcaaggccaggaagctggacgacaagttctaccagaagctgaggggccagttccccgatgctgtgttctggcaagagatcagcgagatcttcaggcagctgcagaagcaggccgccgagatctacaaccagagcctgatcgagctgtactacgagatcttcatcaagggcaagggcatcgccaacgccagcagcgtggagcactacctgagcgacgtgtgctacaccagggccgctgaactgttcaagaacgccgccatcgcaagcggactgaggagcaagatcaagagcaacttcaggctgaaggagctgaagaacatgaagagcggcctgcccaccaccaagagcgacaacttccccatccccctggtgaagcagaagggcggccagtacaccggcttcgagatcagcaaccacaacagcgacttcatcatcaagatccccttcggcaggtggcaggtgaagaaggagatcgacaagtacaggccctgggagaagttcgacttcgagcaggtgcagaagagccccaagcccatcagcctgctgctgagcacccagaggaggaagaggaacaagggctggagcaaggacgaaggcaccgaggccgagatcaagaaggtgatgaatggcgactaccagaccagctacatcgaggtgaagaggggcagcaagatcggcgagaagagcgcctggatgctgaacctgagcatcgacgtgcccaagatcgacaagggcgtggaccccagcatcatcggcggcatcgacgttggagtgaaatctcccctggtttgcgccatcaacaacgccttcagcaggtacagcatcagcgacaacgacctgttccacttcaacaagaagatgttcgccaggaggagaatcctgctgaagaagaacaggcacaagagggccggccacggcgccaagaacaagctgaagcccatcaccatcctgaccgagaagagcgagaggttcaggaagaagctgatcgagaggtgggcctgcgaaatcgccgacttcttcatcaagaacaaggtgggcaccgtgcagatggagaacctggagagcatgaagaggaaggaggacagctacttcaacatcaggctgaggggcttctggccctacgccgagatgcagaacaagatcgagttcaagctgaagcagtacggcatcgagatcaggaaggtggcccccaacaacaccagcaagacctgcagcaagtgcggccacctgaacaactacttcaacttcgagtacaggaagaagaacaagttcccccacttcaagtgcgagaagtgcaacttcaaggagaacgccgactacaacgccgccctgaacatcagcaaccccaagctgaagagcaccaaggaggagccctaa

SEQ ID NO: 3540 - DNA, 76 bp, synthetic construct; identical to SEQ ID NO: 3528
  source 1..76: mol_type = other DNA

SEQ ID NO: 3541 - DNA, 20 bp, synthetic construct
  source 1..20: mol_type = other DNA
cattctatggcacgccatcg

SEQ ID NO: 3542 - DNA, 20 bp, synthetic construct
  source 1..20: mol_type = other DNA
cagcttatgccaatccgacg

SEQ ID NO: 3543 - DNA, 20 bp, synthetic construct
  source 1..20: mol_type = other DNA
cgagatgtcatgcgatgctc

SEQ ID NO: 3544 - DNA, 21 bp, synthetic construct
  source 1..21: mol_type = other DNA
ctcttctcgctaaccaaaccg

SEQ ID NO: 3545 - DNA, 20 bp, synthetic construct
  source 1..20: mol_type = other DNA
cccaactgatcttcagcatc

SEQ ID NO: 3546 - DNA, 84 bp, synthetic construct
  source 1..84: mol_type = other DNA
gatctctttgccatatggtagcaatttgtacgtttggttaacctcctggaccccctcgtttgttataacccagggcgaagtgta

SEQ ID NO: 3547 - DNA, 84 bp, synthetic construct
  source 1..84: mol_type = other DNA
gatctacacttcgccctgggttataacaaacgagggggtccaggaggttaaccaaacgtacaaattgctaccatatggcaaaga

SEQ ID NO: 3548 - DNA, 20 bp, synthetic construct
  source 1..20: mol_type = other DNA
atacgtcagctaccgccttg

SEQ ID NO: 3549 - DNA, 20 bp, synthetic construct
  source 1..20: mol_type = other DNA
gcttgtgaccagactggctc

SEQ ID NO: 3550 - DNA, 20 bp, synthetic construct
  source 1..20: mol_type = other DNA
gcttgtgaccagactggctc
